European Patent Application EP 4 635 975 A1, published October 22, 2025. Title: MODIFIED BACTERIAL STRAINS. Applicant: Institute of Science and Technology Austria. Application EP. The sequence listing filed with the application follows.

SEQUENCE LISTING (219 sequences)

SEQ ID NO: 1 - DNA, 1337 bp, Escherichia coli
  source 1..1337: mol_type = genomic DNA; note = insL-2
ataagcgctaacttaagggttgaaccatctgaagaatgcgacgcctcggtgcctcgttaagacgatgcctcgcgttcttcaattgcgttttgtaggctgtcagggatactgtcccacgaatggccacctgtaagctccagatgaccatttttgttattctccacaacgagttagttcttcttttcggatccggcacttctgggggggaaatccagcgatggctggattatgtcgtcaattaaaaatgcggcgagtagattagcaaatatccacgctttcgcgagttcaggttcctttgcacgcaaagcatccaggtgcagcaaacttttgagccgcttaaaagccagttcaatttgccatcgcagacggtaacaatcagccacttgctctgctgaatattcatcttccggtaatgatgttagcaatagcacatggcccgctgcttccagcgtttccgcctgaactactcgtccttttcgacgattctcgctgagcagtcgggttttactgattaatgctttttcgggaggaagtgatacggcaatgagacgtgccggaaagggagctccggcttttttattacctgaattgcctatcattacagtggtttcaccgttcttaccgcaatccagcccgcgcagaaaacccatcatgtcaaagcgcattccttctgcagttaaccagcgcaatcctcgccagtgaacccggacgatataatcagcttctccaaaagcaagtgagcggatacattcgggacgcgaaccgaatccccggtcagcaatgcgtatctcgtctgccgtttgcgcaaatcggtccagccgttcagcgtctctgctgtcggttagctcaaaatcagtgaactgacaggtatgaggatcatatcccatatgtagtcgccattcagcgctgccgcccccgggcgcactgattgctgttccatcgacaagacgcaatctctttccgcttgtacaacccgtaactgcggcgcgtacagcaagtgtttgtgcggcaagtatgccaaaccagtcggcggcattccgcagccgcttcaggagagccacgtcagataatgttgcaacgtcatggagctgagcccatgcagtgacttcacgtaatgacatccccccggggccgtaagccagccccagacgtagcagagttgcagcatcacgaatttcgcggcggcgggttagagccccggcattacgtgccgaagtatccagttcttcgggcttaccaatatgggccagaattgctgaccagttatcgtgagagtaattcatcggcacgttaaatcatatcaggcgtaataccacaacccttaagttagcgcttat

SEQ ID NO: 2 - DNA, 768 bp, Escherichia coli
  source 1..768: mol_type = genomic DNA; note = IS1A
ggtaatgactccaacttattgatagtgttttatgttcagataatgcccgatgactttgtcatgcagctccaccgattttgagaacgacagcgacttccgtcccagccgtgccaggtgctgcctcagattcaggttatgccgctcaattcgctgcgtatatcgcttgctgattacgtgcagctttcccttcaggcgggattcatacagcggccagccatccgtcatccatatcaccacgtcaaagggtgacagcaggctcataagacgccccagcgtcgccatagtgcgttcaccgaatacgtgcgcaacaaccgtcttccggagactgtcatacgcgtaaaacagccagcgctggcgcgatttagccccgacatagccccactgttcgtccatttccgcgcagacgatgacgtcactgcccggctgtatgcgcgaggttaccgactgcggcctgagttttttaagtgacgtaaaatcgtgttgaggccaacgcccataatgcgggctgttgcccggcatccaacgccattcatggccatatcaatgattttctggtgcgtaccgggttgagaagcggtgtaagtgaactgcagttgccatgttttacggcagtgagagcagagatagcgctgatgtccggcggtgcttttgccgttacgcaccaccccgtcagtagctgaacaggagggacagctgatagaaacagaagccactggagcacctcaaaaacaccatcatacactaaatcagtaagttggcagcatcacc

SEQ ID NO: 3 - DNA, 768 bp, Escherichia coli
  source 1..768: mol_type = genomic DNA; note = IS1B
ggtaatgactccaacttattgatagtgttttatgttcagataatgcccgatgactttgtcatgctgctccaccgattttgagaacgacagcgacttccgtcccagccgtgccaggtgctgcctcagattcaggttatgccgctcaattcgctgcgtatatcgcttgctgattacgtgcagctttcccttcaggcgggattcatacagcggccagccatccgtcatccatatcaccacgtcaaagggtgacagcaggctcataagacgccccagcgtcgccatagtgcgttcaccgaatacgtgcgcaacaaccgtcttccggagcctgtcatacgcgtaaaacagccagcgctggcgcgatttagccccgacgtatccccactgttcgtccatttccgcgcagacgatgacgtcactgcccggctgtatgcgcgaggttaccgactgcggcctgagttttttaaatggcggaaaatcgtgttgaggccaacgcccataatgcgggcggttgcccggcatccaacgccattcatggccatatcaatgattttctggtgcgtaccgggttgagaagcggtgtaagtgaactgcagttgccatgttttacggcagtgagagcagagatagcgctgatgtccggcagtgcttttgccgttacgcaccaccccgtcagtagctgaacaggagggacagctgatagaaacagaagccactggagcacctcaaaaacaccatcatacactaaatcagtaagttggcagcatcacc

SEQ ID NO: 4 - DNA, 763 bp, Escherichia coli
  source 1..763: mol_type = genomic DNA; note = IS1C
tgactccaacttattgatagtgttttatgttcagataatgcccgatgactttgtcatgctgctccaccgattttgagaacgacagcgacttccgtcccagccgtgccaggtgctgcctcagattcaggttatgccgctcaattcgctgcgtatatcgcttgctgattacgtgcagctttcccttcaggcgggattcatacagcggccagccatccgtcatccatatcaccacgtcaaagggtgacagcaggctcataagacgccccagcgtcgccatagtgcgttcaccgaatacgtgcgcaacaaccgtcttccggagcctgtcatacgcgtaaaacagccagcgctggcgcgatttagccccgacgtatccccactgttcgtccatttccgcgcagacgatgacgtcactgcccggctgtatgcgcgaggttaccgactgcggcctgagttttttaaatggcggaaaatcgtgttgaggccaacgcccataatgcgggcggttgcccggcatccaacgccattcatggccatatcaatgattttctggtgcgtaccgggttgagaagcggtgtaagtgaactgcagttgccatgttttacggcagtgagagcagagatagcgctgatgtccggcagtgcttttgccgttacgcaccaccccgtcagtagctgaacaggagggacagctgatagaaacagaagccactggagcacctcaaaaacaccatcatacactaaatcagtaagttggcagcatcacc

SEQ ID NO: 5 - DNA, 768 bp, Escherichia coli
  source 1..768: mol_type = genomic DNA; note = IS1D
ggtgatgctgccaacttactgatttagtgtatgatggtgtttttgaggttctccagtggcttctgtttctatcagctgtccctcctgttcagctactgacggggtggtgcgtaacggcaaaagcactgccggacatcagcgctatctctgctctcactgccgtaaaacatggcaactgcagttcacttacaccgcttctcaacccggtacgcaccagaaaatcattgatatggccatgaatggcgttggatgccgggcaacagcccgcattatgggcgttggcctcaacacgattttccgccatttaaaaaactcaggccgcagtcggtaacctcgcgcatacagccgggcagtgacgtcatcgtctgcgcggaaatggacgaacagtggggatacgtcggggctaaatcgcgccagcgctggctgttttacgcgtatgacaggctccggaagacggttgttgcgcacgtattcggtgaacgcactatggcgacgctggggcgtcttatgagcctgctgtcaccctttgacgtggtgatatggatgacggatggctggccgctgtatgaatcccgcctgaagggaaagctgcacgtaatcagcaagcgatatacgcagcgaattgagcggtataacctgaatctgaggcagcacctggcacggctgggacggaagtcgctgtcgttctcaaaatcggtggagctgcatgacaaagtcatcgggcattatctgaacataaaacactatcaataagttggagtcattacc

SEQ ID NO: 6 - DNA, 768 bp, Escherichia coli
  source 1..768: mol_type = genomic DNA; note = IS1E
ggtgatgctgccaacttactgatttagtgtatgatggtgtttttgaggtgctccagtggcttctgtttctatcagctgtccctcctgttcagctactgacggggtggtgcgtaacggcaaaagcaccgccggacatcagcgctatctctgctctcactgccgtaaaacatggcaactgcagttcacttacaccgcttctcaacccggtacgcaccagaaaatcattgatatggccatgaatggcgttggatgccgggcaacagcccgcattatgggcgttggcctcaacacgattttacgtcacttaaaaaactcaggccgcagtcggtaacctcgcgcatacagccgggcagtgacgtcatcgtctgcgcggaaatggacgaacagtggggctatgtcggggctaaatcgcgccagcgctggctgttttacgcgtatgacagtctccggaagacggttgttgcgcacgtattcggtgaacgcactatggcgacgctggggcgtcttatgagcctgctgtcaccctttgacgtggtgatatggatgacggatggctggccgctgtatgaatcccgcctgaagggaaagctgcacgtaatcagcaagcgatatacgcagcgaattgagcggcataacctgaatctgaggcagcacctggcacggctgggacggaagtcgctgtcgttctcaaaatcggtggagctgcatgacaaagtcatcgggcattatctgaacataaaacactatcaataagttggagtcattacc

SEQ ID NO: 7 - DNA, 768 bp, Escherichia coli
  source 1..768: mol_type = genomic DNA; note = IS1F
ggtaatgctgccaacttactgatttagtgtatgatggtgattttaaggtgcttgcgtggcttccatttccatcagatgtccttcctgctccgctactgaaggcgtggtgcgtaacggcaaaagcactgccggacatcagcgctatctctgctctccttgccgtaaaacatggcaactacagttcacttacaccgcctctcagcccggtaagcaccagaaaatcattgatatggccatgaatggcgtcggatgtcgcgccagtgcacgcattatgggcgttggcctcaacacggttttacgtcacttaaaaaactcaggccgcagtcggtaacctcgcgcatacaaccgggcagtgatgtgattgtctgcgctgaaatggacgaacagtggggctacgtcggtgctaaatcacgtcagcgctggctgttttacgcgtatgacaggatacggaggacggttgtggcgcacgtcttcggtgaacgcactctggccacactggagcgtcttctgagcctgctgtcggcctttgaggtcgtggtatagatgacggatggctggccgctgtatgaatcacgcctgaagggaaagctgcacgttatcagcaagcgttacactcagcgcattgagcgacataatctgaatctgagacaacatctggcaaggctgggacggaagttactgtcgttctcaaaatcggtggagttgcatgacaaggtcatcgggcattatctgaacataaaacactatcagtaagttggagtcattacc

SEQ ID NO: 8 - DNA, 768 bp, Escherichia coli; identical to SEQ ID NO: 2
  source 1..768: mol_type = genomic DNA; note = IS1H

SEQ ID NO: 9 - DNA, 1157 bp, Escherichia coli
  source 1..1157: mol_type = genomic DNA; note = IS5A
ctcagtcatttcatttcttcatgtttgagccgattttttctcccgtaaatgccttgaatcagcctatttagaccgtttcttcgccatttaaggcgttatccccagtttttagtgagatctctcccactgacgtatcatttggtccgcccgaaacaggttggccagcgtgaataacatcgccagttggttatcgtttttcagcaaccccttgtatctggctttcacgaagccgaactgtcgcttgatgatgcgaaatgggtgctccaccctggcccggatgctggctttcatgtattcgatgttgatggccgttttgttcttgcgtggatgctgtttcaaggttcttaccttgccggggcgctcggcgatcagccagtccacatccacctcggccagctcctcgcgctgtggcgccccttggtagccggcatcggctgagacaaattgctcctctccatgcagcagattacccagctgattgaggtcatgctcgttggccgcggtggtgaccaggctgtgggtcaggccactcttggcatcgacaccaatgtgggccttcatgccaaagtgccactgattgcctttcttggtctgatgcatctccggatcgcgttgctgctctttgttcttggtcgagctgggtgcctcaatgatggtggcatcgaccaaggtgccttgagtcatcatgacgcctgcttcggccagccagcgattgatggtcttgaacaattggcgggccagttgatgctgctccagcaggtggcggaaattcatgatggtggtgcggtccggcaaggcgctatccagggataaccgggcaaacagacgcatggaggcgatttcgtacagagcatcttccatcgcgccatcgctcaggttgtaccaatgctgcatgcagtgaatgcgtagcatggtttccagcggataaggtcgccggccattaccagccttggggtaaaacggctcgatgacttccaccatgttttgccatggcagaatctgctccatgcgggacaagaaaatctcttttctggtctgacggcgcttactgctgaattcactgtcggcgaaggtaagttgatgactcatgatgaaccctgttctatggctccagatgacaaacatgatctcatatcagggacttgttcgcaccttcc

SEQ ID NO: 10 - DNA, 1195 bp, Escherichia coli
  source 1..1195: mol_type = genomic DNA; note = IS5B
ggaaggtgcgaataagcggggaaattcttctcggctgactcagtcatttcatttcttcatgtttgagccgattttttctcccgtaaatgccttgaatcagcctatttagaccgtttcttcgccatttaaggcgttatccccagtttttagtgagatctctcccactgacgtatcatttggtccgcccgaaacaggttggccagcgtgaataacatcgccagttggttatcgtttttcagcaaccccttgtatctggctttcacgaagccgaactgtcgcttgatgatgcgaaatgggtgctccaccctggcccggatgctggctttcatgtattcgatgttgatggccgttttgttcttgcgtggatgctgtttcaaggttcttaccttgccggggcgctcggcgatcagccagtccacatccacctcggccagctcctcgcgctgtggcgccccttggtagccggcatcggctgagacaaattgctcctctccatgcagcagattacccagctgattgaggtcatgctcgttggccgcggtggtgaccaggctgtgggtcaggccactcttggcatcgacaccaatgtgggccttcatgccaaagtgccactgattgcctttcttggtctgatgcatctccggatcgcgttgctgctctttgttcttggtcgagctgggtgcctcaatgatggtggcatcgaccaaggtgccttgagtcatcatgacgcctgcttcggccagccagcgattgatggtcttgaacaattggcgggccagttgatgctgctccagcaggtggcggaaattcatgatggtggtgcggtccggcaaggcgctatccagggataaccgggcaaacagacgcatggaggcgatttcgtacagagcatcttccatcgcgccatcgctcaggttgtaccaatgctgcatgcagtgaatgcgtagcatggtttccagcggataaggtcgccggccattaccagccttggggtaaaacggctcgatgacttccaccatgttttgccatggcagaatctgctccatgcgggacaagaaaatctcttttctggtctgacggcgcttactgctgaattcactgtcggcgaaggtaagttgatgactcatgatgaaccctgttctatggctccagatgacaaacatgatctcatatcagggacttgttcgcaccttcc

SEQ ID NO: 11 - DNA, 1195 bp, Escherichia coli; identical to SEQ ID NO: 10
  source 1..1195: mol_type = genomic DNA; note = IS5D

SEQ ID NO: 12 - DNA, 1195 bp, Escherichia coli
  source 1..1195: mol_type = genomic DNA; note = IS5F
ggaaggtgcgaacaagtccctgatatgagatcatgtttgtcatctggagccatagaacagggttcatcatgagtcatcaacttaccttcgccgacagtgaattcagcagtaagcgccgtcagaccagaaaagagattttcttgtcccgcatggagcagattctgccatggcaaaacatggtggaagtcatcgagccgttttaccccaaggctggtaatggccggcgaccttatccgctggaaaccatgctacgcattcactgcatgcagcattggtacaacctgagcgatggcgcgatggaagatgctctgtacgaaatcgcctccatgcgtctgtttgcccggttatccctggatagcgccttgccggaccgcaccaccatcatgaatttccgccacctgctggagcagcatcaactggcccgccaattgttcaagaccatcaatcgctggctggccgaagcaggcgtcatgatgactcaaggcaccttggtcgatgccaccatcattgaggcacccagctcgaccaagaacaaagagcagcaacgcgatccggagatgcatcagaccaagaaaggcaatcagtggcactttggcatgaaggcccacattggtgtcgatgccaagagtggcctgacccacagcctggtcaccaccgcggccaacgagcatgacctcaatcagctgggtaatctgctgcatggagaggagcaatttgtctcagccgatgccggctaccaaggggcgccacagcgcgaggagctggccgaggtggatgtggactggctgatcgccgagcgccccggcaaggtaagaaccttgaaacagcatccacgcaagaacaaaacggccatcaacatcgaatacatgaaagccagcatccgggccagggtggagcacccatttcgcatcatcaagcgacagttcggcttcgtgaaagccagatacaaggggttgctgaaaaacgataaccaactggcgatgttattcacgctggccaacctgtttcgggcggaccaaatgatacgtcagtgggagagatctcactaaaaactggggataacgccttaaatggcgaagaaacggtctaaataggctgattcaaggcatttacgggagaaaaaatcggctcaaacatgaagaaatgaaatgactgagtcagccgagaagaatttccccgcttattcgcaccttcc

SEQ ID NO: 13 - DNA, 1195 bp, Escherichia coli
  source 1..1195: mol_type = genomic DNA; note = IS5H
ggaaggtgcgaataagtggggaaattcttctcggctgactcagtcatttcatttcttcatgtttgagccgattttttctcccgtaaatgccttgaatcagcctatttagaccgtttcttcgccatttaaggcgttatccccagtttttagtgagatctctcccactgacgtatcatttggtccgcccgaaacaggttggccagcgtgaataacatcgccagttggttatcgtttttcagcaaccccttgtatctggctttcacgaagccgaactgtcgcttgatgatgcgaaatgggtgctccaccttggcccggatgctggctttcatgtattcgatgttgatggccgttttgttcttgcgtggatgctgtttcaaggttcttaccttgccggggcgctcggcgatcagccagtccacatccacctcggccagctcctcgcgctgtggcgccccttggtagccggcatcggctgagacaaattgctcctctccatgcagcagattacccagctgattgaggtcatgctcgttggccgcggtggtgactaggctgtgggtcaggccgctcttggcatcgacaccaatgtgggccttcatgccaaagtgccactgattgcctttcttggtctgatgcatctccggatcgcgttgctgctctttgttcttggtcgagctgggtgcctcaatgatggtggcatcgaccaaggtgccttgagtcatcatgacgcctgcttcggccagccagcgattgatggtcttgaacaattggcgggccagttgatgctgctccagcaggtggcggaaattcatgatggtggtgcggtccggcaaggcgctatccagggataaccgggcaaacagacgcatggaggcgatttcgtacagagcatcttccatcgcgccatcgctcaggttgtaccaatgctgcatgcagtgaatgcgtagcatggtttccagcggataaggtcgccggccattaccagccttggggtaaaacggctcgatgacttccaccatgttttgccatggcagaatctgctccatgcgggacaagaaaatctcttttctggtctgacggcgcttactgctgaattcactgtcggcgaaggtaagttgatgactcatgatgaaccctgttccatggctccagatgacaaacatgatctcatatcagggacttgttcgcaccttcc

SEQ ID NO: 14 - DNA, 1195 bp, Escherichia coli; identical to SEQ ID NO: 10
  source 1..1195: mol_type = genomic DNA; note = IS5I

SEQ ID NO: 15 - DNA, 1195 bp, Escherichia coli; identical to SEQ ID NO: 10
  source 1..1195: mol_type = genomic DNA; note = IS5K

SEQ ID NO: 16 - DNA, 1125 bp, Escherichia coli
  source 1..1125: mol_type = genomic DNA; note = IS5LO
gagtcatcaacttaccttcgccgacagtgaattcagcagtaagcgccgtcagaccagaaaagagattttcttgtcccgcatggagcagattctgccatggcaaaacatggtggaagtcatcgagccgttttaccccaaggctggtaatggccggcgaccttatccgctggaaaccatgctacgcattcactgcatgcagcattggtacaacctgagcgatggcgcgatggaagatgctctgtacgaaatcgcctccatgcgtctgtttgcccggttatccctggatagcgccttgccggaccgcaccaccatcatgaatttccgccacctgctggagcagcatcaactggcccgccaattgttcaagaccatcaatcgctggctggccgaagcaggcgtcatgatgactcaaggcaccttggtcgatgccaccatcattgaggcacccagctcgaccaagaacaaagagcagcaacgcgatccggagatgcatcagaccaagaaaggcaatcagtggcactttggcatgaaggcccacattggtgtcgatgccaagagtggcctgacccacagcctggtcaccaccgcggccaacgagcatgacctcaatcagctgggtaatctgctgcatggagaggagcaatttgtctcagccgatgccggctaccaaggggcgccacagcgcgaggagctggccgaggtggatgtggactggctgatcgccgagcgccccggcaaggtaagaaccttgaaacagcatccacgcaagaacaaaacggccatcaacatcgaatacatgaaagccagcatccgggccagggtggagcacccatttcgcatcatcaagcgacagttcggcttcgtgaaagccagatacaaggggttgctgaaaaacgataaccaactggcgatgttattcacgctggccaacctgtttcgggcggaccaaatgatacgtcagtgggagagatctcactaaaaactggggataacgccttaaatggcgaagaaacggtctaaataggctgattcaaggcatttacgggagaaaaaatcggctcaaacatgaagaaatgaaatgactgagtcagccgagaagaatttccccgcttattcgcaccttcc

SEQ ID NO: 17 - DNA, 1195 bp, Escherichia coli; identical to SEQ ID NO: 10
  source 1..1195: mol_type = genomic DNA; note = IS5R

SEQ ID NO: 18 - DNA, 1195 bp, Escherichia coli; identical to SEQ ID NO: 10
  source 1..1195: mol_type = genomic DNA; note = IS5T

SEQ ID NO: 19 - DNA, 1196 bp, Escherichia coli
  source 1..1196: mol_type = genomic DNA; note = IS5Y
ggaaggtgcgaataagcaggtcatttcttcccaagctgactcgctgattaaaatttcgcggatctgggccgatttttttcccgcaaacacatcgaatcagcctatttaggctattttttccaccatttctggcgttatttccggtttttactgagatctctcccactgacgtatcatttggtccacccgaaacaggttggccagggtgaataacatcgccagttggttatcgtttttcagcagccccttgtatctggctttcacgaagccgaactgccgcttgatgatgcgaaacgggtgctccaccctggcacggatgctggctttcatgtattcgatgttgatggccgttttgttcttgcgcggattctgcttcaaggtttttaccttgccgggacgctcggcgatcagccagtccacatccacctcggccagctcctcgcgctgtggcgctccttggtagccggcatcggctgagacaaattgctcctctccatgaagcagattacccagctgattgaggtcatgctcgttggccgcggtggtgaccaggctgtgggtcaggccactcttggcatcgacaccaatgtgggccttcatgccaaagtgccactgattgcctttcttggtctgatgcatctccggatcgcgttgctgctctttgttcttggtagagctgggtgcctcaatgatggtggcatccaccaaagtgccttgggtcatcatgacgcctgcttcggccagccagcgattgatggtcttgaacaattgacgggccagttgatgctgctcgagcaggtggcggaaattcatgatggtggtgcgatccggcagggcgctatccagggataatcgggcaaacaggcgcatggaggcgatttcgtacagggcatcttccatggcaccgtcgctcaggttgtaccaatgctgcatgcagtgaatacgcagcatggtctccagcggatagggccgtcggccattgcccgccttgggataaaacggctcgatgacagcggtcatattctgccatggcagaatctgctccatgcgggagaggaaaatctcttttcgggtctgacggcgcttagtgctgaattcactatcggcgaaggtgagttgatggctcatgatgtccctctgggatgcgctccggatgaatatgatgatctcatatcaggaacttgttcgcaccttcc

SEQ ID NO: 20 - DNA, 1426 bp, Escherichia coli
  source 1..1426: mol_type = genomic DNA; note = IS4
taatgccagtcagttaagcaactgactggctctttttcggggctgtggggtatttccagggcctctcctttaccactctcgggaaggccctttcccttcttgtcggtaatttcacaagttgtcccatacttgcaagatcgcgcatcagctccggtatacgtcccggtgaagcgccctgcaatgtcatcagcattctcatcaccattccgcatgattctgagaaactcagttgattcggccagtaacctttcagatgttccgccattttaatcatctgatatctcaccagattataagccagtaagacaccccacagctcttgctccacaagctccggctttttacttctcagcgtcagcctgctccgttgcatcgtctgttttatctccctgtatcccagttcgatttcccagcgatgactgtacagatcccccatttctcctccggggaagcgcatggcgtccgtcatcgacgtcagcagatggcagacttttcctttgcgcgtcacggtcagcaggcgggcagtcacttcatttcccagtcccggccacttttttcgtgcctgcgggctggttttcagcttcaccagatgatcgcctttacccagttttctgatctcttcatattgcgctccctttctgagaggtatcatccagtggcggtgttctcccgccaggctccaggcatttaacagtcccagtgagtaataacctttatccattaacgtcagagtgttatcgccggtttgttctataagttgctcagcaagctcattttcgctgttcttcatcgtgccgaaggctgcagccgtcagcagatggctggtcagttccatctggcagaccattttgacctgcgggtagagcgccgggttcccggcatgtgtctggcgggggaaggctgcatcgttctctggtgtatccggtgtgcgccagaacacaccatcgatggccagcagggtcaggccgcaccagtgcggatgcggcgtggcgttatgccagagctgcgctgttttcgtgaacacgcggcggacagcctcacttcccaggcgctggcgggcctgaataacggcactgggggcaacgaaggggcgattgcccggcagcatgatgtccaggcgattcacaatctggtgaagaggttctttacgctcaagcgccatgccaacaatacaccagaccatcatttcgaggggaagacggcgcttgcgtagcgttacagtacctgattcggcaaggcaacgagagatgagttcggggtcgaggtaatcccccagagaagtcagtgggttacgcagagaatcgtaacgggataccagatcaagagcctgtccaatgtgcataaaaaaatccggaaacaagtgagcgtttccggattcttacacagccactggatcggtcaactgatccttaactgatcggcatta

SEQ ID NO: 21 - DNA, 1331 bp, Escherichia coli
  source 1..1331: mol_type = genomic DNA; note = IS2A
tagactggccccctgaatctccagacaaccaatatcacttaaataagtgatagtcttaatactagtttttagactagtcattggagaacagatgattgatgtcttagggccggagaaacgcagacggcgtaccacacaggaaaagatcgcaattgttcagcagagctttgaaccggggatgacggtctccctcgttgcccggcaacatggtgtagcagccagccagttatttctctggcgtaagcaataccaggaaggaagtcttactgctgtcgccgccggagaacaggttgttcctgcctctgaacttgctgccgccatgaagcagattaaagaactccagcgcctgctcggcaagaaaacgatggaaaatgaactcctcaaagaagccgttgaatatggacgggcaaaaaagtggatagcgcacgcgcccttattgcccggggatggggagtaagcttagtcagccgttgtctccgggtgtcgcgtgcgcagttgcacgtcattctcagacgaaccgatgactggatggatggccgccgcagtcgtcacactgatgatacggatgtgcttctccgtatacaccatgttatcggagagctgccaacgtatggttatcgtcgggtatgggcgctgcttcgcagacaggcagaacttgatggtatgcctgcgatcaatgccaaacgtgtttaccggatcatgcgccagaatgcgctgttgcttgagcgaaaacctgctgtaccgccatcgaaacgggcacatacaggcagagtggccgtgaaagaaagcaatcagcgatggtgctctgacgggttcgagttctgctgtgataacggagagagactgcgtgtcacgttcgcgctggactgctgtgatcgtgaggcactgcactgggcggtcactaccggcggcttcaacagtgaaacagtacaggacgtcatgctgggagcggtggaacgccgcttcggcaacgatcttccgtcgtctccagtggagtggctgacggataatggttcatgctaccgggctaatgaaacacgccagttcgcccggatgttgggacttgaaccgaagaacacggcggtgcggagtccggagagtaacggaatagcagagagcttcgtgaaaacgataaagcgtgactacatcagtatcatgcccaaaccagacgggttaacggcagcaaagaaccttgcagaggcgttcgagcattataacgaatggcatccgcatagtgcgctgggttatcgctcgccacgggaatatctgcggcagcgggcttgtaatgggttaagtgataacagatgtctggaaatataggggcaaatcca

SEQ ID NO: 22 - DNA, 1331 bp, Escherichia coli
  source 1..1331: mol_type = genomic DNA; note = IS2D
tggatttgcccctatatttccagacatctgttatcacttaacccattacaagcccgctgccgcagatattcccgtggcgagcgataacccagcgcactatgcggatgccattcgttataatgctcgaacgcctctgcaaggttctttgctgccgttaacccgtctggtttgggcatgatactgatgtagtcacgctttatcgttttcacgaagctctctgctattccgttactctccggactccgcaccgccgtgttcttcggttcaagtcccaacatccgggcgaactggcgtgtttcattagcccggtagcatgaaccattatccgtcagccactccactggagacgacggaagatcgttgccgaagcggcgttccaccgctcccagcatgacgtcctgtactgtttcactgttgaagccgccggtagtgaccgcccagtgcagtgcctcacgatcacagcagtccagcgcgaacgtgacacgcagtctctctccgttatcacagcagaactcgaacccgtcagagcaccatcgctgattgctttctttcacggccactctgcctgtatgtgcccgtttcgatggcggtacagcaggttttcgctcaagcaacagcgcattctggcgcatgatccggtaaacacgtttggcattgatcgcaggcataccatcaagttctgcctgtctgcgaagcagcgcccatacccgacgataaccatacgttggcagctctccgataacatggtgtatacggagaagcacatccgtatcatcagtgtgacgactgcggcggccatccatccagtcatcggttcgtctgagaatgacgtgcaactgcgcacgcgacacccggagacaacggctgactaagcttactccccatccccgggcaataagggcgcgtgcgctatccacttttttgcccgtccatattcaacggcttctttgaggagttcattttccatcgttttcttgccgagcaggcgctggagttctttaatctgcttcatggcggcagcaagttcagaggcaggaacaacctgttctccggcggcgacagcagtaagacttccttcctggtattgcttacgccagagaaataactggctggctgctacaccatgttgccgggcaacgagggagaccgtcatccccggttcaaagctctgctgaacaattgcgatcttttcctgtgtggtacgccgtctgcgtttctccggccctaagacatcaatcatctgttctccaatgactagtctaaaaactagtattaagactatcacttatttaagtgatattggttgtctggagattcagggggccagtcta

SEQ ID NO: 23 - DNA, 513 bp, Escherichia coli
  source 1..513: mol_type = genomic DNA; note = IS2E
aagaaagcaatcagcgatggtgctctgacgggttcgagttctgctgtgataacggagagagactgcgtgtcacgttcgcgctggactgctgtgatcgtgaggcactgcactgggcggtcactaccggcggcttcaacagtgaaacagtacaggacgtcatgctgggagcggtggaacgccgcttcggcaacgatcttccgtcgtctccagtggagtggctgacggataatggttcatgctaccgggctaatgaaacacgccagttcgcccggatgttgggacttgaaccgaagaacacggcggtgcggagtccggagagtaacggaatagcagagagcttcgtgaaaacgataaagcgtgactacatcagtatcatgcccaaaccagacgggttaacggcagcaaagaaccttgcagaggcgttcgagcattataacgaatggcatccgcatagtgcgctgggttatcgctcgccacgggaatatctgcggcagcgggcttgtaatgggttaa

SEQ ID NO: 24 - DNA, 1331 bp, Escherichia coli; identical to SEQ ID NO: 22
  source 1..1331: mol_type = genomic DNA; note = IS2F

SEQ ID NO: 25 - DNA, 1328 bp, Escherichia coli
  source 1..1328: mol_type = genomic DNA; note = IS2H
tggatttgcccctatatttccagacatctgttatcacttaacccattacaagcccgctgccgcagatattcccgtggcgagcgataacccagcgcactatgcggatgccattcgttataatgctcgaacgcctctgcaaggttctttgctgccgttaacccgtctggtttgggcatgatactgatgtagtcacgctttatcgttttcacgaagctctctgctattccgttactctccggactccgcaccgccgtgttcttcggttcaagtcccaacatccgggcgaactggcgtgtttcattagcccggtagcatgaaccattatccgtcagccactccactggagacgacggaagatcgttgccgaagcggcgttccaccgctcccagcatgacgtcctgtactgtttcactgttgaagccgccggtagtgaccgcccagtgcagtgcctcacgatcacagcagtccagcgcgaacgtgacacgcagtctctctccgttatcacagcagaactcgaacccgtcagagcaccatcgctgattgctttctttcacggccactctgcctgtatgtgcccgtttcgatggcggtacagcaggttttcgctcaagcaacagcgcattctggcgcatgatccggtaaacacgtttggcattgatcgcaggcataccatcaagttctgcctgtctgcgaagcagcgcccatacccgacgataaccatacgttggcagctctccgataacatggtgtatacggagaagcacatccgtatcatcagtgtgacgactgcggcggccatccatccagtcatcggttcgtctgagaatgacgtgcaactgcgcacgcgacacccggagacaacggctgactaagcttactccccatccccgggcaataagggcgcgtgcgctatccacttttttgcccgtccatattcaacggcttctttgaggagttcattttccatcgttttcttgccgagcaggcgctggagttctttaatctgcttcatggcggcagcaagttcagaggcaggaacaacctgttctccggcggcgacagcagtaagacttccttcctggtattgcttacgccagagaaataactggctggctgctacaccatgttgccgggcaacgagggagaccgtcatccccggttcaaagctctgctgaacaattgcgatcttttcctgtgtggtacgccgtctgcgtttctccggccctaagacatcaatcatctgttctccaatgactagtctaaaaactagtattaagactatcacttatttaagtgatattggttgtctggagattcagggggccagt

SEQ ID NO: 26 - DNA, 1331 bp, Escherichia coli; identical to SEQ ID NO: 21
  source 1..1331: mol_type = genomic DNA; note = IS2I

SEQ ID NO: 27 - DNA, 1331 bp, Escherichia coli; identical to SEQ ID NO: 21
  source 1..1331: mol_type = genomic DNA; note = IS2K

SEQ ID NO: 28 - DNA, 1205 bp, Escherichia coli
  source 1..1205: mol_type = genomic DNA; note = IS3A
tggacacgcggctaagtgagtaaactctcagtcagaggtgactcacatgacaaaaacagtatcaaccagtaaaaaaccccgtaaacagcattcgcctgaatttcgcagtgaagccctgaagcttgctgaacgcatcggtgttactgccgcagcccgtgaactcagcctgtatgaatcacaactctacaactggcgcagtaaacagcaaaatcagcagacgtcttctgaacgtgaactggagatgtctaccgagattgcacgtctcaaacgccagctggcagaacgggatgaagagctggctatcctccaaaaggccgcgacatacttcgcgaagcgcctgaaatgaagtatgtctttattgaaaaacatcaggctgagttcagcatcaaagcaatgtgccgcgtgctccgggtggcccgcagcggctggtatacgtggtgtcagcggcggacaaggataagcacgcgtcagcagttccgccaacactgcgacagcgttgtcctcgcggcttttacccggtcaaaacagcgttacggtgccccacgcctgacggatgaactgcgtgctcagggttacccctttaacgtaaaaaccgtggcggcaagcctgcgccgtcagggactgagggcaaaggcctcccggaagttcagcccggtcagctaccgcgcacacggcctgcctgtgtcagaaaatctgttggagcaggatttttacgccagtggcccgaaccagaagtgggcaggagacatcacgtacttacgtacagatgaaggctggctgtatctggcagtggtcattgacctgtggtcacgtgccgttattggctggtcaatgtcgccacgcatgacggcgcaactggcctgcgatgccctgcagatggcgctgtggcggcgtaagaggccccggaacgttatcgttcacacggaccgtggaggccagtactgttcagcagattatcaggcgcaactgaagcggcataatctgcgtggaagtatgagcgcaaaaggttgctgctacgataatgcctgcgtggaaagcttctttcattcgctgaaagtggaatgtatccatggagaacactttatcagccgggaaataatgcgggcaacggtgtttaattatatcgaatgtgattacaatcggtggcggcggcacagttggtgtggcggcctcagtccggaacaatttgaaaacaagaacctcgc

SEQ ID NO: 29 - DNA, 1258 bp, Escherichia coli
  source 1..1258: mol_type = genomic DNA; note = IS3B
tgatcctacccacgtaatatggacacaggcctaagcgaggttcttgttttcaaattgttccggactgaggccgccacaccaactgtgccgccgccaccgattgtaatcacattcgatataattaaacaccgttgcccgcattatttcccggctgataaagtgttctccatggatacattccactttcagcgaatgaaagaagctttccacgcaggcattatcgtagcagcaaccttttgcgctcatacttccacgcagattatgccgcttcagttgcgcctgataatctgctgaacagtactggcctccacggtccgtgtgaacgataacgttccggggcctcttacgccgccacagcgccatctgcagggcatcgcaggccagttgcgccgtcatgcgtggcgacattgaccagccaataacggcacgtgaccacaggtcaatgaccactgccagatacagccagccttcatctgtacgtaagtacgtgatgtctcctgcccacttctggttcgggccactggcgtaaaaatcctgctccaacagattttctgacacaggcaggccgtgtgcgcggtagctgaccgggctgaacttccgggaggcctttgccctcagtccctgacggcgcaggcttgccgccacggtttttacgttaaaggggtaaccctgagcacgcagttcatccgtcaggcgtggggcaccgtaacgctgttttgaccgggtaaaagccgcgaggacaacgctgtcgcagtgttggcggaactgctgacgcgtgcttatccttgtccgccgctgacaccacgtataccagccgctgcgggccacccggagcacgcggcacattgctttgatgctgaactcagcctgatgtttttcaataaagacatacttcatttcaggcgcttcgcgaagtatgtcgcggccttttggaggatagccagctcttcatcccgttctgccagctggcgtttgagacgtgcaatctcggtagacatctccagttcacgttcagaagacgtctgctgattttgctgtttactgcgccagttgtagagttgtgattcatacaggctgagttcacgggctgcggcagtaacaccgatgcgttcagcaagcttcagggcttcactgcgaaattcaggcgaatgctgtttacggggttttttactggttgatactgtttttgtcatgtgagtcacctctgactgagagtttactcacttagccgcgtgtccactattgctgggtaagatca

SEQ ID NO: 30 - DNA, 1258 bp, Escherichia coli
  source 1..1258: mol_type = genomic DNA; note = IS3C
tgatcttacccagcaatagtggacacgcggctaagtgagtaaactctcagtcagaggtgactcacatgacaaaaacagtatcaaccagtaaaaaaccccgtaaacagcattcgcctgaatttcgcagtgaagccctgaagcttgctgaacgcatcggtgttactgccgcagcccgtgaactcagcctgtatgaatcacaactctacaactggcgcagtaaacagcaaaatcagcagacgtcttctgaacgtgaactggagatgtctaccgagattgcacgtctcaaacgccagctggcagaacgggatgaagagctggctatcctccaaaaggccgcgacatacttcgcgaagcgcctgaaatgaagtatgtctttattgaaaaacatcaggctgagttcagcatcaaagcaatgtgccgcgtgctccgggtggcccgcagcggctggtatacgtggtgtcagcggcggacaaggataagcacgcgtcagcagttccgccaacactgcgacagcgttgtcctcgcggcttttacccggtcaaaacagcgttacggtgccccacgcctgacggatgaactgcgtgctcagggttacccctttaacgtaaaaaccgtggcggcaagcctgcgccgtcagggactgagggcaaaggcctcccggaagttcagcccggtcagctaccgcgcacacggcctgcctgtgtcagaaaatctgttggagcaggatttttacgccagtggcccgaaccagaagtgggcaggagacatcacgtacttacgtacagatgaaggctggctgtatctggcagtggtcattgacctgtggtcacgtgccgttattggctggtcaatgtcgccacgcatgacggcgcaactggcctgcgatgccctgcagatggcgctgtggcggcgtaagaggccccggaacgttatcgttcacacggaccgtggaggccagtactgttcagcagattatcaggcgcaactgaagcggcataatctgcgtggaagtatgagcgcaaaaggttgctgctacgataatgcctgcgtggaaagcttctttcattcgctgaaagtggaatgtatccatggagaacactttatcagccgggaaataatgcgggcaacggtgtttaattatatcgaatgtgattacaatcggtggcggcggcacagttggtgtggcggcctcagtccggaacaatttgaaaacaagaacctcgcttaggcctgtgtccatattacgtgggtaggatca

SEQ ID NO: 31 - DNA, 1258 bp, Escherichia coli; identical to SEQ ID NO: 30
  source 1..1258: mol_type = genomic DNA; note = IS3D

SEQ ID NO: 32 - DNA, 1258 bp, Escherichia coli; identical to SEQ ID NO: 30
  source 1..1258: mol_type = genomic DNA; note = IS3E

SEQ ID NO: 33 - DNA, 1221 bp, Escherichia coli
  source 1..1221: mol_type = genomic DNA; note = IS30A
tgtagattcaattggtcaacgcaacagttatgtgaaaacatggggttgcggaggttttttgaatgagacgaacatttacagcagaggaaaaagcctctgtttttgaactatggaagaacggaacaggcttcagtgaaatagcgaatatcctgggttcaaaacccggaacgatcttcactatgttaagggatactggcggcataaaaccccatgagcgtaagcgggctgtagctcacctgacactgtctgagcgcgaggagatacgagctggtttgtcagccaaaatgagcattcgtgcgatagctactgcgctgaatcgcagtccttcgacgatctcacgtgaagttcagcgtaatcggggcagacgctattacaaagctgttgatgctaataaccgagccaacagaatggcgaaaaggccaaaaccgtgcttactggatcaaaatttaccattgcgaaagcttgttctggaaaagctggagatgaaatggtctccagagcaaatatcaggatggttaaggcgaacaaaaccacgtcaaaaaacgctgcgaatatcacctgagacaatttataaaacgctgtactttcgtagccgtgaagcgctacaccacctgaatatacagcatctgcgacggtcgcatagccttcgccatggcaggcgtcatacccgcaaaggcgaaagaggtacgattaacatagtgaacggaacaccaattcacgaacgttcccgaaatatcgataacagacgctctctggggcattgggagggcgatttagtctcaggtacaaaaaactctcatatagccacacttgtagaccgaaaatcacgttatacgatcatcgttagactcaggggcaaagattctgtctcagtaaatcaggctcttaccgacaaattcctgagtttaccgtcagaactcagaaaatcactgacatgggacagaggaatggaactggccagacatctagaatttactgtcagcaccggcgttaaagtttacttctgcgatcctcagagtccttggcagcggggaacaaatgagaatacaaatgggctaattcggcagtactttcctaaaaagacatgtcttgcccaatatactcaacatgaactagatctggttgctgctcagctaaacaacagaccgagaaagacactgaagttcaaaacaccgaaagagataattgaaaggggtgttgcattgacagattgaatctaca

SEQ ID NO: 34 - DNA, 182 bp, Escherichia coli
  source 1..182: mol_type = genomic DNA; note = IS30B
gagaacacaaatgggctaattcggcagtactttcctaaaaagacatgtcttgcccaatatactcaacatgaactagatctggttgctgctcagctaaacaacagaccgagaaagacactgaagttcaaaacaccgaaagagataattgaaaggggtgttgcattgacagattgaatctacag

SEQ ID NO: 35 - DNA, 1221 bp, Escherichia coli
  source 1..1221: mol_type = genomic DNA; note = IS30C
tgtagattcaattggtcaacgcaacagttatgtgaaaacatggggttgcggaggttttttgaatgagacgaacatttacagcagaggaaaaagcctctgtttttgaactatggaagaacggaacaggcttcagtgaaatagcgaatatcctgggttcaaaacccggaacgatcttcactatgttaagggatactggcggcataaaaccccatgagcgtaagcgggctgtagctcacctgacactgtctgagcgcgaggagatacgagctggtttgtcagccaaaatgagcattcgtgcgatagctactgcgctgaatcgcagtccttcgacgatctcacgtgaagttcagcgtaatcggggcagacgctattacaaagctgttgatgctaataaccgagccaacagaatggcgaaaaggccaaaaccgtgcttactggatcaaaatttaccattgcgaaagcttgttctggaaaagctggagatgaaatggtctccagagcaaatatcaggatggttaaggcgaacaaaaccacgtcaaaaaacgctgcgaatatcacctgagacaatttataaaacgctgtactttcgtagccgtgaagcgctacaccacctgaatatacagcatctgcgacggtcgcatagccttcgccatggcaggcgtcatacccgcaaaggcgaaagaggtacgattaacatagtgaacggaacaccaattcacgaacgttcccgaaatatcgataacagacgctctctagggcattgggagggcgatttagtctcaggtacaaaaaactctcatatagccacacttgtagaccgaaaatcacgttatacgatcatccttagactcaggggcaaagattctgtctcagtaaatcaggctcttaccgacaaattcctgagtttaccgtcagaactcagaaaatcactgacatgggacagaggaatggaactggccagacatctagaatttactgtcagcaccggcgttaaagtttacttctgcgatcctcagagtccttggcagcggggaacaaatgagaacacaaatgggctaattcggcagtactttcctaaaaagacatgtcttgcccaatatactcaacatgaactagatctggttgctgctcagctaaacaacagaccgagaaagacactgaagttcaaaacaccgaaagagataattgaaaggggtgttgcattgacagattgaatctaca

SEQ ID NO: 36 - DNA, 1221 bp, Escherichia coli; identical to SEQ ID NO: 35
  source 1..1221: mol_type = genomic DNA; note = IS30D

SEQ ID NO: 37 - DNA, 1443 bp, Escherichia coli
  source 1..1443: mol_type = genomic DNA; note = IS150
tgtactgcacccattttgttggacgatgaaatggaatagcccctaatatgtcaaagccaaaatacccttttgaaaagcgccttgaagtcgtgaatcactacttcacaactgatgatggttacaggatcatctcggcacgttttggtgtcccccgaacccaggtcaggacatgggttgccctctatgaaaaacatggagaaaaaggtttaattcccaaacctaaaggcgttagtgctgatccagagttgcgtattaaggtcgtgaaagctgtgatcgagcagcacatgtcccttaatcaggctgctgctcactttatgcttgctggtagtggttctgtagccaggtggctgaaggtctatgaagagcgcggagaagctggtttacgcgcgctcaagattggcaccaaaagaaacattgcaatatcagttgatccagaaaaagcggcatcagcattggagctgtcaaaagaccgacgcattgaggatcttgaaaggcaagttcgatttcttgaaacgcggcttatgtatctaaaaaagctgaaagccttagctcatcccacgaaaaagtgaaagtactcaacgagctaaggcagttttatcctcttgatgagcttctcagggctgcggagataccgcgcagtacgttttattatcatctaaaggctctcagcaagcctgacaagtatgcggacgttaaaaagcgtattagtgagatttatcacgagaatagaggccgatacggataccgtagggtaacgctgtctcttcatcgagaagggaaacagattaaccataaagctgttcagcgcctgatgggaaccctctcacttaaagcagcgattaaggtcaagcgataccgctcttacagaggagaggtagggcaaaccgcccctaatgttctccaaagagatttcaaggctacgcggccaaacgagaagtgggttaccgatgttactgaatttgcagtcaatgggcgcaagctgtatttgtctccagtaatagatctcttcaacaacgaagttatttcttacagcctttcggaaagaccagtgatgaacatggttgagaatatgctcgatcaggcattcaaaaagcttaatcctcacgagcatcctgttctgcactctgaccagggatggcagtatcgtatgagaagatatcaaaatatccttaaagaacatggtattaaacaaagcatgtccagaaaaggcaattgtctggataatgctgtggtggagtgtttctttggaaccttaaagtcggagtgtttttatcttgatgagttcagtaatataagcgaactgaaggatgctgttacggaatatattgaatactacaacagcagaagaattagcctgaaattaaaaggtctgactccaattgaatatcggaatcagacctatatgcctcgtgtttaactgtccaactttttggggtcagtaca

SEQ ID NO: 38 - DNA, 1343 bp, Escherichia coli
  source 1..1343: mol_type = genomic DNA; note = IS186A
cccataagcgctaacttaagggttgtggtattacgcctgatatgatttaacgtgccgatgaattactctcacgataactggtcagcaattctggcccatattggtaagcccgaagaactggatacttcggcacgtaatgccggggctctaacccgccgccgcgaaattcgtgatgctgcaactctgctacgtctggggctggcttacggccccggggggatgtcattacgtgaagtcactgcatgggctcagctccatgacgttgcaacattatctgacgtggctctcctgaagcggctgcggaatgccgccgactggtttggcatacttgccgcacaaacacttgctgtacgcgccgcagttacgggttgtacaagcggaaagagattgcgtcttgtcgatggaacagcaatcagtgcgcccgggggcggcagcgctgaatggcgactacatatgggatatgatcctcatacctgtcagttcactgattttgagctaaccgacagcagagacgctgaacggctggaccgatttgcgcaaacggcagacgagatacgcattgctgaccggggattcggttcgcgtcccgaatgtatccgctcacttgcttttggagaagctgattatatcgtccgggttcactggcgaggattgcgctggttaactgcagaaggaatgcgctttgacatgatgggttttctgcgcgggctggattgcggtaagaacggtgaaaccactgtaatgataggcaattcaggtaataaaaaagccggagctccctttccggcacgtctcattgccgtatcacttcctcccgaaaaagcattaatcagtaaaacccgactgctcagcgagaatcgtcgaaaaggacgagtagttcaggcggaaacgctggaagcagcgggccatgtgctattgctaacatcattaccggaagatgaatattcagcagagcaagtggctgattgttaccgtctgcgatggcaaattgaactggcttttaagcggctcaaaagtttgctgcacctggatgctttgcgtgcaaaggaacctgaactcgcgaaagcgtggatatttgctaatctactcgccgcatttttaattgacgacataatccagccatcgctggatttcccccccagaagtgccggatccgaaaagaagaactaactcgttgtggagaataacaaaaatggtcatctggagcttacaggtggccattcgtgggacagtatccctgacagcctacaaaacgcaattgaagaacgcgaggcatcgtcttaacgaggcaccgaggcgtcgcattcttcagatggttcaacccttaagttagcgcttatggg

SEQ ID NO: 39 - DNA, 1343 bp, Escherichia coli; identical to SEQ ID NO: 38
  source 1..1343: mol_type = genomic DNA; note = IS186B

SEQ ID NO: 40 - DNA, 1343 bp, Escherichia coli; identical to SEQ ID NO: 38
  source 1..1343: mol_type = genomic DNA; note = IS186C

SEQ ID NO: 41 - DNA, 327 bp, Escherichia coli
  source 1..327: mol_type = genomic DNA; note = IS600
tgaggtagcctgagtttaacggacactccttcctgaaatagaatggcatcagaaggagctaataatgagcagaaaaacccaacgttactctaaaaagttcaaagccgaagctgtcagaacggttcttgaaaatcaactttcgatcagtgaaggcgcttcccgattatctcttcctgaaggcactttaggacaatgggttaccgccgccagaaaagggctcggtactcctggttcccgcacggtggctgaactggaatctgaaattctgcaactgcgtaaggcgttaaatgaagctcgccttgagcgagatatattaaaaaaagcaac

SEQ ID NO: 42 - DNA, 1744 bp, Escherichia coli
  source 1..1744: mol_type = genomic DNA; note = IS609
ccggtgcgccgtaaaaccccatccttcagggcggggatataaggcgcggttttccacctgaccaggtgtttgctgttgttcaatgtattggcggatgacggatattggcgcacctccgcagctactggcaaaatagccaggactccacaaaacgcctttgtagtaatacctgaatgcaatatctggtcgatctcgtcgcagtcacctacccgatacgcctttgaggctgtttaccagactggatatcgccagtttgggaggatagttaattaacaaatggacgtgatctggttcgccatccatttcaaccagttcagcttcaaaatcagcacatacatttgaaaagtaagtgcgtagtttttctgtcgcgtcatggtcaaaaatctggcgtcggtatctggtgacaaagagcaggtgaacatgcatcaggaaaacacaatgccttccacgccggatatcggtttcttttttcacagaccaaagtatcatttgacctgtgaaacgattacaggcatttaaattccagttaagacccggtggtcaacaggagtgtgaaatgaggcgcttcgcaggcgcatgtcgtttcgttttcaatcgtgctctggcacgtcagaatgagaatcatgaggccggtaataaatacatcccttacgggaaaatggcttcctggctggttgagtggaaaaatgccactgaaacgcaatggcttaaagattctccctcacagccattgcaacagtcactgaaagaccttgagcgggcttacaaaaacttcttccggaagcgggctgcttttccccgattcaaaaagcggggacagaatgatgcattccgctacccgcagggcgttaagctcgatcaggaaaacagccgtatttttctgccgaaactgggctggatgcgctaccggaacagccgtcaggtcacgggtgttgtgaaaaatgtcactgtcagccagtcctgcggtaagtggtacatcagtattcagacagaaagtgaagtatcaactccggttcacccttcagcatcaatggtcgggctggatgctggcgtggctaaactcgccacgctgtcagatggcacagtctttgagcctgtaaacagttttcagaaaaaccagaagaagctggcgagacttcagcgacagttaagccgcaaggtcaaattcagcaacaactggcaaaagcagaaacgcaaaatacagcgactgcattcctgtatcgcaaatatccgcagggactaccttcacaaagtcacaacggccgtcagcaaaaaccacgcaatgatagtcattgaggatttgaaggtcagcaacatgtcaaagtcagcagcgggtacggtcagccagccggggcgcaatgtccgggcaaaatcaggtttaaaccgttcgatactggatcagggctggtatgaaatgcgccgccagcttgcgtataagcagctctggcgtggcggtcaggtgcttgctgttccgccagcgtatacaagccagcgttgcgcgtactgtggtcatacagcgaaagagaaccgcctgtcacaaagtaaattcagatgccaggtatgtggatatacagcgaacgccgatgtaaatggcgctcgcaacattttagcggcggggcacgccgttcttgcctgtggagagatggtgcagtcaggccgcccgttgaagcaggaacccaccgaaatgattcaggcgacagcctgaacgtagcagggatccacgtccttcagggcgtggaggatg

SEQ ID NO: 43 - DNA, 764 bp, Escherichia coli
  source 1..764: mol_type = genomic DNA; note = IS911A
  misc_feature 1..335: note = Equivalent to position 270206..270540 in MG1655 Reference Genome U00096.3; note = IS911A site 1
  misc_feature 336..764: note = Equivalent to position 271672..272190 in MG1655 Reference Genome U00096.3; note = IS911A site 2
tgaagtggtttactgaatttggccacctgaacagaggtgatatgctcacctcagaacaacacaggtgtcataatgaaaaaaagaaatttcagcgcagagtttaaacgcgaatccgctcaactggtcgttgaccagaactacaccgtggcagatgcagccagcgctatggatgtcggcctttccacaatgacgcgatgggtgaaacaattacgtgatgaacggcagggcaaaacaccaaaagcctcccccattaccccggaacaaattgaaatccgtgagctcaggaaaaagctacaacgtattgaaatggaaaatgaaatattaaaaaaggctacaccgcgctcttgatgtcagactccctgaacagttctcgataatcgggaaactcagggcgcgttatcctgtggccactctctgccatgtgttcggggttcatcgcagcagctacaaatactggaaaaaccgtcctgaaaagccagacggcagacgggctgtattacgcagtcaggtacttgaactgcatggcatcagccacggctctgccggagcaagaagcatcgccacaatggcaacccagagaggataccagatggggcgctggcttgctggcagactcatgaaagagctggggctggtcagttgccagcagccgactcaccggtataagcgtggcggtcatgagcacgttgctatcccgaatcatcttgagcgacagttcgccgtaacggaaccaaatcaggtgtggtgcggtgatgtgacctata

SEQ ID NO: 44 - DNA, 1129 bp, Escherichia coli
  source 1..1129: mol_type = genomic DNA; note = IS911B
  misc_feature 1..334: note = IS911B site 1; note = Equivalent to position 4507125..4507458 in MG1655 Reference Genome U00096.3
  misc_feature 335..1129: note = IS911B site 2; note = Equivalent to position 4509007..4509801 in MG1655 Reference Genome U00096.3
tgaagtggcacactgaatttggccacctgaacagaggtgatatgctcacctcagaacaacacaggtgctccaatgaaaaaaagaaatttcagcgcagagtttaaacgcgaatccgctcaactggttgttgaccagaaatacacggtggcagatgccgcgaaagctatggatgttggcctttccacaatgacaagatgggtcaaacaactgcgtgatgagcgtcagggcaaaacaccaaaagcctctccgataacaccagaacaaatcgaaatacgtaagctgaggaaaaagctacaacggattgaaatggagaatgaaatattaaaaaggctacggaaaaaccgtcctgaaaaaccagacggcagacgggctgtattacgcagtcaggtacttgagctacatggcatcagccacggttcggccggagcaagaagcatcgccacaatggcaacccggagaggctaccagatgggacgctggcttgctggcaggctcatgaaagagctggggctggtcagctgtcagcagccgactcaccggtataaacgtggtggtcatgaacatgttgctatccctaactaccttgaaaggcagttcgccgtgaccgagccaaatcaggtgtggtgcggtgatgtgacctatatctggacgggtaagcgctgggcgtacctcgccgttgttctcgacctgttcgcaagaaaaccagtgggctgggccatgtcgttctcgccggacagcaggcttaccatgaaagcactggaaatggcatgggaaacccgtggtaagcccgtcggggtgatgttccaagcgatcaaggcagtcattatacgagcaggcagttccggcagttactgtggcgataccggatcaggcagagtatgagtcggcgtggaaactgctgggataacagcccaatggagcgcttcttcaggagtctgaagaacgaatgggtgccagcgacgggctatgtaagcttcagcgatgcagctcacgcaataacggactatatcgttggatattacagcgcactaagaccgcacgaatataatggtgggttaccaccaaacgaatcagaaaaccgatactggaaaaactctaacgcggaggccagttttagttgaccacaaca

SEQ ID NO: 45 - DNA, 272 bp, Escherichia coli
  source 1..272: mol_type = genomic DNA; note = ISX
cagctttttttaatatgtcccgttcgtcggtaacccgtttcagctctttctggagacggcggatctcggcctgagcatctgactgttctttattagtggaagaatccggaccgtacttctttatccaggcataaaggctgtgggtggtgatatcgagacgtgttgcaacgctggcaacagaataaccgagatcaacaacctgtttgactgcttcagttttaaactcttcgggataacgcttaccgctcatgggcacctctctttaagccatt

SEQ ID NO: 46 - DNA, 999 bp, Escherichia coli
  source 1..999: mol_type = genomic DNA; note = ISZ
caatgccgttcacttaagaggagcggcactatgtttcacaggataacgggtttttgatatcttaaccgacctcggccttgatggtcgggggcgttttgttatgaacaccacttccagagcaccccgaagatgctccagtcgtttcgggatggtccctggtgacgccgtgtttcccagctctatcatttctgatgcgatattcttccacgcaggcagtagccagtggcggttacaacccttctggttcagcgtcagcagcaggtcttcgctgtaaaaaagtttatcaaacaacgtaatagagttatccgggatggtggcgagcatggagtgggccagcacagtttcgctctgccggtaaggtgcggtcacggcattcagcagaatgtgacttcccaggttcattaaggccaccagacgcataaccgggtaggcgttctgccgcttagtggatgtgttggcagacccataatattcacgcagctcgggtttatcaggtgtcctgaactgtgcgccatcaatggcaaaaagttgcaggccgtgccagtcatccttcaggtaacgttccgcgcccctgtctgtgcggtctggcggaagagccattccactggggcggcccccacgcgctgacgcgcctgggtgacagcgctgcgggccagcaggttcatccccgcttcgccatccgcgctcaggttcagacggcgaacaacatcggtaattggctcattgcaccaccatccagataaccatgtcccccggtaaacgacggcggcgaacggtcgcatgagcagaaagcgtcaggcagtgttgtatccactcggtgggaaggtgttctgcaaatagttgtgcagagggcggaggcataagcggatggtcactgaaatcgagcagatcattgagaagtggcataagaaaacggctccctgttgtggaagccgttatagtgcctcagtttaaggatcggtcaactaatccttaactgatcggcattgcccagaaggg

SEQ ID NO: 47 - DNA, 777 bp, Escherichia coli
  source 1..777: mol_type = genomic DNA; note = IS1D + 9bp TSD
  misc_feature 1..9: note = TSD
gacaatacgggtgatgctgccaacttactgatttagtgtatgatggtgtttttgaggttctccagtggcttctgtttctatcagctgtccctcctgttcagctactgacggggtggtgcgtaacggcaaaagcactgccggacatcagcgctatctctgctctcactgccgtaaaacatggcaactgcagttcacttacaccgcttctcaacccggtacgcaccagaaaatcattgatatggccatgaatggcgttggatgccgggcaacagcccgcattatgggcgttggcctcaacacgattttccgccatttaaaaaactcaggccgcagtcggtaacctcgcgcatacagccgggcagtgacgtcatcgtctgcgcggaaatggacgaacagtggggatacgtcggggctaaatcgcgccagcgctggctgttttacgcgtatgacaggctccggaagacggttgttgcgcacgtattcggtgaacgcactatggcgacgctggggcgtcttatgagcctgctgtcaccctttgacgtggtgatatggatgacggatggctggccgctgtatgaatcccgcctgaagggaaagctgcacgtaatcagcaagcgatatacgcagcgaattgagcggtataacctgaatctgaggcagcacctggcacggctgggacggaagtcgctgtcgttctcaaaatcggtggagctgcatgacaaagtcatcgggcattatctgaacataaaacactatcaataagttggagtcattacc

SEQ ID NO: 48 - DNA, 777 bp, Escherichia coli
  source 1..777: mol_type = genomic DNA; note = IS1E + 9bp TSD
  misc_feature 769..777: note = TSD
ggtgatgctgccaacttactgatttagtgtatgatggtgtttttgaggtgctccagtggcttctgtttctatcagctgtccctcctgttcagctactgacggggtggtgcgtaacggcaaaagcaccgccggacatcagcgctatctctgctctcactgccgtaaaacatggcaactgcagttcacttacaccgcttctcaacccggtacgcaccagaaaatcattgatatggccatgaatggcgttggatgccgggcaacagcccgcattatgggcgttggcctcaacacgattttacgtcacttaaaaaactcaggccgcagtcggtaacctcgcgcatacagccgggcagtgacgtcatcgtctgcgcggaaatggacgaacagtggggctatgtcggggctaaatcgcgccagcgctggctgttttacgcgtatgacagtctccggaagacggttgttgcgcacgtattcggtgaacgcactatggcgacgctggggcgtcttatgagcctgctgtcaccctttgacgtggtgatatggatgacggatggctggccgctgtatgaatcccgcctgaagggaaagctgcacgtaatcagcaagcgatatacgcagcgaattgagcggcataacctgaatctgaggcagcacctggcacggctgggacggaagtcgctgtcgttctcaaaatcggtggagctgcatgacaaagtcatcgggcattatctgaacataaaacactatcaataagttggagtcattaccgacattaaa

SEQ ID NO: 49 - DNA, 777 bp, Escherichia coli
  source 1..777: mol_type = genomic DNA; note = IS1H +9bp TSD
  misc_feature 769..777: note = TSD
ggtaatgactccaacttattgatagtgttttatgttcagataatgcccgatgactttgtcatgcagctccaccgattttgagaacgacagcgacttccgtcccagccgtgccaggtgctgcctcagattcaggttatgccgctcaattcgctgcgtatatcgcttgctgattacgtgcagctttcccttcaggcgggattcatacagcggccagccatccgtcatccatatcaccacgtcaaagggtgacagcaggctcataagacgccccagcgtcgccatagtgcgttcaccgaatacgtgcgcaacaaccgtcttccggagactgtcatacgcgtaaaacagccagcgctggcgcgatttagccccgacatagccccactgttcgtccatttccgcgcagacgatgacgtcactgcccggctgtatgcgcgaggttaccgactgcggcctgagttttttaagtgacgtaaaatcgtgttgaggccaacgcccataatgcgggctgttgcccggcatccaacgccattcatggccatatcaatgattttctggtgcgtaccgggttgagaagcggtgtaagtgaactgcagttgccatgttttacggcagtgagagcagagatagcgctgatgtccggcggtgcttttgccgttacgcaccaccccgtcagtagctgaacaggagggacagctgatagaaacagaagccactggagcacctcaaaaacaccatcatacactaaatcagtaagttggcagcatcaccgaggctggc

SEQ ID NO: 50 - DNA, 1199 bp, Escherichia coli
  source 1..1199: mol_type = genomic DNA; note = IS5B + 4bp TSD
  misc_feature 1..4: note = TSD
ttagggaaggtgcgaataagcggggaaattcttctcggctgactcagtcatttcatttcttcatgtttgagccgattttttctcccgtaaatgccttgaatcagcctatttagaccgtttcttcgccatttaaggcgttatccccagtttttagtgagatctctcccactgacgtatcatttggtccgcccgaaacaggttggccagcgtgaataacatcgccagttggttatcgtttttcagcaaccccttgtatctggctttcacgaagccgaactgtcgcttgatgatgcgaaatgggtgctccaccctggcccggatgctggctttcatgtattcgatgttgatggccgttttgttcttgcgtggatgctgtttcaaggttcttaccttgccggggcgctcggcgatcagccagtccacatccacctcggccagctcctcgcgctgtggcgccccttggtagccggcatcggctgagacaaattgctcctctccatgcagcagattacccagctgattgaggtcatgctcgttggccgcggtggtgaccaggctgtgggtcaggccactcttggcatcgacaccaatgtgggccttcatgccaaagtgccactgattgcctttcttggtctgatgcatctccggatcgcgttgctgctctttgttcttggtcgagctgggtgcctcaatgatggtggcatcgaccaaggtgccttgagtcatcatgacgcctgcttcggccagccagcgattgatggtcttgaacaattggcgggccagttgatgctgctccagcaggtggcggaaattcatgatggtggtgcggtccggcaaggcgctatccagggataaccgggcaaacagacgcatggaggcgatttcgtacagagcatcttccatcgcgccatcgctcaggttgtaccaatgctgcatgcagtgaatgcgtagcatggtttccagcggataaggtcgccggccattaccagccttggggtaaaacggctcgatgacttccaccatgttttgccatggcagaatctgctccatgcgggacaagaaaatctcttttctggtctgacggcgcttactgctgaattcactgtcggcgaaggtaagttgatgactcatgatgaaccctgttctatggctccagatgacaaacatgatctcatatcagggacttgttcgcaccttcc

SEQ ID NO: 51 - DNA, 1199 bp, Escherichia coli
  source 1..1199: mol_type = genomic DNA; note = IS5D + 4bp TSD
  intron 1196..1199: note = TSD
ggaaggtgcgaataagcggggaaattcttctcggctgactcagtcatttcatttcttcatgtttgagccgattttttctcccgtaaatgccttgaatcagcctatttagaccgtttcttcgccatttaaggcgttatccccagtttttagtgagatctctcccactgacgtatcatttggtccgcccgaaacaggttggccagcgtgaataacatcgccagttggttatcgtttttcagcaaccccttgtatctggctttcacgaagccgaactgtcgcttgatgatgcgaaatgggtgctccaccctggcccggatgctggctttcatgtattcgatgttgatggccgttttgttcttgcgtggatgctgtttcaaggttcttaccttgccggggcgctcggcgatcagccagtccacatccacctcggccagctcctcgcgctgtggcgccccttggtagccggcatcggctgagacaaattgctcctctccatgcagcagattacccagctgattgaggtcatgctcgttggccgcggtggtgaccaggctgtgggtcaggccactcttggcatcgacaccaatgtgggccttcatgccaaagtgccactgattgcctttcttggtctgatgcatctccggatcgcgttgctgctctttgttcttggtcgagctgggtgcctcaatgatggtggcatcgaccaaggtgccttgagtcatcatgacgcctgcttcggccagccagcgattgatggtcttgaacaattggcgggccagttgatgctgctccagcaggtggcggaaattcatgatggtggtgcggtccggcaaggcgctatccagggataaccgggcaaacagacgcatggaggcgatttcgtacagagcatcttccatcgcgccatcgctcaggttgtaccaatgctgcatgcagtgaatgcgtagcatggtttccagcggataaggtcgccggccattaccagccttggggtaaaacggctcgatgacttccaccatgttttgccatggcagaatctgctccatgcgggacaagaaaatctcttttctggtctgacggcgcttactgctgaattcactgtcggcgaaggtaagttgatgactcatgatgaaccctgttctatggctccagatgacaaacatgatctcatatcagggacttgttcgcaccttccttag

SEQ ID NO: 52 - DNA, 1199 bp, Escherichia coli
  source 1..1199: mol_type = genomic DNA; note = IS5F + 4bp TSD
  misc_feature 1..4: note = TSD
ctaaggaaggtgcgaacaagtccctgatatgagatcatgtttgtcatctggagccatagaacagggttcatcatgagtcatcaacttaccttcgccgacagtgaattcagcagtaagcgccgtcagaccagaaaagagattttcttgtcccgcatggagcagattctgccatggcaaaacatggtggaagtcatcgagccgttttaccccaaggctggtaatggccggcgaccttatccgctggaaaccatgctacgcattcactgcatgcagcattggtacaacctgagcgatggcgcgatggaagatgctctgtacgaaatcgcctccatgcgtctgtttgcccggttatccctggatagcgccttgccggaccgcaccaccatcatgaatttccgccacctgctggagcagcatcaactggcccgccaattgttcaagaccatcaatcgctggctggccgaagcaggcgtcatgatgactcaaggcaccttggtcgatgccaccatcattgaggcacccagctcgaccaagaacaaagagcagcaacgcgatccggagatgcatcagaccaagaaaggcaatcagtggcactttggcatgaaggcccacattggtgtcgatgccaagagtggcctgacccacagcctggtcaccaccgcggccaacgagcatgacctcaatcagctgggtaatctgctgcatggagaggagcaatttgtctcagccgatgccggctaccaaggggcgccacagcgcgaggagctggccgaggtggatgtggactggctgatcgccgagcgccccggcaaggtaagaaccttgaaacagcatccacgcaagaacaaaacggccatcaacatcgaatacatgaaagccagcatccgggccagggtggagcacccatttcgcatcatcaagcgacagttcggcttcgtgaaagccagatacaaggggttgctgaaaaacgataaccaactggcgatgttattcacgctggccaacctgtttcgggcggaccaaatgatacgtcagtgggagagatctcactaaaaactggggataacgccttaaatggcgaagaaacggtctaaataggctgattcaaggcatttacgggagaaaaaatcggctcaaacatgaagaaatgaaatgactgagtcagccgagaagaatttccccgcttattcgcaccttcc

SEQ ID NO: 53 - DNA, 1199 bp, Escherichia coli
  source 1..1199: mol_type = genomic DNA; note = IS5H + 4bp TSD
  misc_feature 1196..1199: note = TSD
ggaaggtgcgaataagtggggaaattcttctcggctgactcagtcatttcatttcttcatgtttgagccgattttttctcccgtaaatgccttgaatcagcctatttagaccgtttcttcgccatttaaggcgttatccccagtttttagtgagatctctcccactgacgtatcatttggtccgcccgaaacaggttggccagcgtgaataacatcgccagttggttatcgtttttcagcaaccccttgtatctggctttcacgaagccgaactgtcgcttgatgatgcgaaatgggtgctccaccttggcccggatgctggctttcatgtattcgatgttgatggccgttttgttcttgcgtggatgctgtttcaaggttcttaccttgccggggcgctcggcgatcagccagtccacatccacctcggccagctcctcgcgctgtggcgccccttggtagccggcatcggctgagacaaattgctcctctccatgcagcagattacccagctgattgaggtcatgctcgttggccgcggtggtgactaggctgtgggtcaggccgctcttggcatcgacaccaatgtgggccttcatgccaaagtgccactgattgcctttcttggtctgatgcatctccggatcgcgttgctgctctttgttcttggtcgagctgggtgcctcaatgatggtggcatcgaccaaggtgccttgagtcatcatgacgcctgcttcggccagccagcgattgatggtcttgaacaattggcgggccagttgatgctgctccagcaggtggcggaaattcatgatggtggtgcggtccggcaaggcgctatccagggataaccgggcaaacagacgcatggaggcgatttcgtacagagcatcttccatcgcgccatcgctcaggttgtaccaatgctgcatgcagtgaatgcgtagcatggtttccagcggataaggtcgccggccattaccagccttggggtaaaacggctcgatgacttccaccatgttttgccatggcagaatctgctccatgcgggacaagaaaatctcttttctggtctgacggcgcttactgctgaattcactgtcggcgaaggtaagttgatgactcatgatgaaccctgttccatggctccagatgacaaacatgatctcatatcagggacttgttcgcaccttccctag

SEQ ID NO: 54 - DNA, 1199 bp, Escherichia coli
  source 1..1199: mol_type = genomic DNA; note = IS5I + 4bp TSD
  misc_feature 1..4: note = TSD
ttaaggaaggtgcgaataagcggggaaattcttctcggctgactcagtcatttcatttcttcatgtttgagccgattttttctcccgtaaatgccttgaatcagcctatttagaccgtttcttcgccatttaaggcgttatccccagtttttagtgagatctctcccactgacgtatcatttggtccgcccgaaacaggttggccagcgtgaataacatcgccagttggttatcgtttttcagcaaccccttgtatctggctttcacgaagccgaactgtcgcttgatgatgcgaaatgggtgctccaccctggcccggatgctggctttcatgtattcgatgttgatggccgttttgttcttgcgtggatgctgtttcaaggttcttaccttgccggggcgctcggcgatcagccagtccacatccacctcggccagctcctcgcgctgtggcgccccttggtagccggcatcggctgagacaaattgctcctctccatgcagcagattacccagctgattgaggtcatgctcgttggccgcggtggtgaccaggctgtgggtcaggccactcttggcatcgacaccaatgtgggccttcatgccaaagtgccactgattgcctttcttggtctgatgcatctccggatcgcgttgctgctctttgttcttggtcgagctgggtgcctcaatgatggtggcatcgaccaaggtgccttgagtcatcatgacgcctgcttcggccagccagcgattgatggtcttgaacaattggcgggccagttgatgctgctccagcaggtggcggaaattcatgatggtggtgcggtccggcaaggcgctatccagggataaccgggcaaacagacgcatggaggcgatttcgtacagagcatcttccatcgcgccatcgctcaggttgtaccaatgctgcatgcagtgaatgcgtagcatggtttccagcggataaggtcgccggccattaccagccttggggtaaaacggctcgatgacttccaccatgttttgccatggcagaatctgctccatgcgggacaagaaaatctcttttctggtctgacggcgcttactgctgaattcactgtcggcgaaggtaagttgatgactcatgatgaaccctgttctatggctccagatgacaaacatgatctcatatcagggacttgttcgcaccttcc

SEQ ID NO: 55 - DNA, 1199 bp, Escherichia coli
  source 1..1199: mol_type = genomic DNA; note = IS5K + 4bp TSD
  misc_feature 1..4: note = TSD
ataaggaaggtgcgaataagcggggaaattcttctcggctgactcagtcatttcatttcttcatgtttgagccgattttttctcccgtaaatgccttgaatcagcctatttagaccgtttcttcgccatttaaggcgttatccccagtttttagtgagatctctcccactgacgtatcatttggtccgcccgaaacaggttggccagcgtgaataacatcgccagttggttatcgtttttcagcaaccccttgtatctggctttcacgaagccgaactgtcgcttgatgatgcgaaatgggtgctccaccctggcccggatgctggctttcatgtattcgatgttgatggccgttttgttcttgcgtggatgctgtttcaaggttcttaccttgccggggcgctcggcgatcagccagtccacatccacctcggccagctcctcgcgctgtggcgccccttggtagccggcatcggctgagacaaattgctcctctccatgcagcagattacccagctgattgaggtcatgctcgttggccgcggtggtgaccaggctgtgggtcaggccactcttggcatcgacaccaatgtgggccttcatgccaaagtgccactgattgcctttcttggtctgatgcatctccggatcgcgttgctgctctttgttcttggtcgagctgggtgcctcaatgatggtggcatcgaccaaggtgccttgagtcatcatgacgcctgcttcggccagccagcgattgatggtcttgaacaattggcgggccagttgatgctgctccagcaggtggcggaaattcatgatggtggtgcggtccggcaaggcgctatccagggataaccgggcaaacagacgcatggaggcgatttcgtacagagcatcttccatcgcgccatcgctcaggttgtaccaatgctgcatgcagtgaatgcgtagcatggtttccagcggataaggtcgccggccattaccagccttggggtaaaacggctcgatgacttccaccatgttttgccatggcagaatctgctccatgcgggacaagaaaatctcttttctggtctgacggcgcttactgctgaattcactgtcggcgaaggtaagttgatgactcatgatgaaccctgttctatggctccagatgacaaacatgatctcatatcagggacttgttcgcaccttcc

SEQ ID NO: 56 - DNA, 1199 bp, Escherichia coli; identical to SEQ ID NO: 51
  source 1..1199: mol_type = genomic DNA; note = IS5R + 4bp TSD
  misc_feature 1196..1199: note = TSD

SEQ ID NO: 57 - DNA, 1199 bp, Escherichia coli; identical to SEQ ID NO: 51
  source 1..1199: mol_type = genomic DNA; note = IS5T + 4bp TSD
  misc_feature 1196..1199: note = TSD

SEQ ID NO: 58 - DNA, 1200 bp, Escherichia coli
  source 1..1200: mol_type = genomic DNA; note = IS5Y + 4bp TSD
  misc_feature 1197..1200: note = TSD
ggaaggtgcgaataagcaggtcatttcttcccaagctgactcgctgattaaaatttcgcggatctgggccgatttttttcccgcaaacacatcgaatcagcctatttaggctattttttccaccatttctggcgttatttccggtttttactgagatctctcccactgacgtatcatttggtccacccgaaacaggttggccagggtgaataacatcgccagttggttatcgtttttcagcagccccttgtatctggctttcacgaagccgaactgccgcttgatgatgcgaaacgggtgctccaccctggcacggatgctggctttcatgtattcgatgttgatggccgttttgttcttgcgcggattctgcttcaaggtttttaccttgccgggacgctcggcgatcagccagtccacatccacctcggccagctcctcgcgctgtggcgctccttggtagccggcatcggctgagacaaattgctcctctccatgaagcagattacccagctgattgaggtcatgctcgttggccgcggtggtgaccaggctgtgggtcaggccactcttggcatcgacaccaatgtgggccttcatgccaaagtgccactgattgcctttcttggtctgatgcatctccggatcgcgttgctgctctttgttcttggtagagctgggtgcctcaatgatggtggcatccaccaaagtgccttgggtcatcatgacgcctgcttcggccagccagcgattgatggtcttgaacaattgacgggccagttgatgctgctcgagcaggtggcggaaattcatgatggtggtgcgatccggcagggcgctatccagggataatcgggcaaacaggcgcatggaggcgatttcgtacagggcatcttccatggcaccgtcgctcaggttgtaccaatgctgcatgcagtgaatacgcagcatggtctccagcggatagggccgtcggccattgcccgccttgggataaaacggctcgatgacagcggtcatattctgccatggcagaatctgctccatgcgggagaggaaaatctcttttcgggtctgacggcgcttagtgctgaattcactatcggcgaaggtgagttgatggctcatgatgtccctctgggatgcgctccggatgaatatgatgatctcatatcaggaacttgttcgcaccttcccaag

SEQ ID NO: 59 - DNA, 1349 bp, Escherichia coli
  source 1..1349: mol_type = genomic DNA; note = IS186A + 6bp TSD
  misc_feature 1..6: note = TSD
atcactcccataagcgctaacttaagggttgtggtattacgcctgatatgatttaacgtgccgatgaattactctcacgataactggtcagcaattctggcccatattggtaagcccgaagaactggatacttcggcacgtaatgccggggctctaacccgccgccgcgaaattcgtgatgctgcaactctgctacgtctggggctggcttacggccccggggggatgtcattacgtgaagtcactgcatgggctcagctccatgacgttgcaacattatctgacgtggctctcctgaagcggctgcggaatgccgccgactggtttggcatacttgccgcacaaacacttgctgtacgcgccgcagttacgggttgtacaagcggaaagagattgcgtcttgtcgatggaacagcaatcagtgcgcccgggggcggcagcgctgaatggcgactacatatgggatatgatcctcatacctgtcagttcactgattttgagctaaccgacagcagagacgctgaacggctggaccgatttgcgcaaacggcagacgagatacgcattgctgaccggggattcggttcgcgtcccgaatgtatccgctcacttgcttttggagaagctgattatatcgtccgggttcactggcgaggattgcgctggttaactgcagaaggaatgcgctttgacatgatgggttttctgcgcgggctggattgcggtaagaacggtgaaaccactgtaatgataggcaattcaggtaataaaaaagccggagctccctttccggcacgtctcattgccgtatcacttcctcccgaaaaagcattaatcagtaaaacccgactgctcagcgagaatcgtcgaaaaggacgagtagttcaggcggaaacgctggaagcagcgggccatgtgctattgctaacatcattaccggaagatgaatattcagcagagcaagtggctgattgttaccgtctgcgatggcaaattgaactggcttttaagcggctcaaaagtttgctgcacctggatgctttgcgtgcaaaggaacctgaactcgcgaaagcgtggatatttgctaatctactcgccgcatttttaattgacgacataatccagccatcgctggatttcccccccagaagtgccggatccgaaaagaagaactaactcgttgtggagaataacaaaaatggtcatctggagcttacaggtggccattcgtgggacagtatccctgacagcctacaaaacgcaattgaagaacgcgaggcatcgtcttaacgaggcaccgaggcgtcgcattcttcagatggttcaacccttaagttagcgcttatggg

SEQ ID NO: 60 - DNA, 1349 bp, Escherichia coli
  source 1..1349: mol_type = genomic DNA; note = IS186B + 6bp TSD
  misc_feature 1344..1349: note = TSD
cccataagcgctaacttaagggttgtggtattacgcctgatatgatttaacgtgccgatgaattactctcacgataactggtcagcaattctggcccatattggtaagcccgaagaactggatacttcggcacgtaatgccggggctctaacccgccgccgcgaaattcgtgatgctgcaactctgctacgtctggggctggcttacggccccggggggatgtcattacgtgaagtcactgcatgggctcagctccatgacgttgcaacattatctgacgtggctctcctgaagcggctgcggaatgccgccgactggtttggcatacttgccgcacaaacacttgctgtacgcgccgcagttacgggttgtacaagcggaaagagattgcgtcttgtcgatggaacagcaatcagtgcgcccgggggcggcagcgctgaatggcgactacatatgggatatgatcctcatacctgtcagttcactgattttgagctaaccgacagcagagacgctgaacggctggaccgatttgcgcaaacggcagacgagatacgcattgctgaccggggattcggttcgcgtcccgaatgtatccgctcacttgcttttggagaagctgattatatcgtccgggttcactggcgaggattgcgctggttaactgcagaaggaatgcgctttgacatgatgggttttctgcgcgggctggattgcggtaagaacggtgaaaccactgtaatgataggcaattcaggtaataaaaaagccggagctccctttccggcacgtctcattgccgtatcacttcctcccgaaaaagcattaatcagtaaaacccgactgctcagcgagaatcgtcgaaaaggacgagtagttcaggcggaaacgctggaagcagcgggccatgtgctattgctaacatcattaccggaagatgaatattcagcagagcaagtggctgattgttaccgtctgcgatggcaaattgaactggcttttaagcggctcaaaagtttgctgcacctggatgctttgcgtgcaaaggaacctgaactcgcgaaagcgtggatatttgctaatctactcgccgcatttttaattgacgacataatccagccatcgctggatttcccccccagaagtgccggatccgaaaagaagaactaactcgttgtggagaataacaaaaatggtcatctggagcttacaggtggccattcgtgggacagtatccctgacagcctacaaaacgcaattgaagaacgcgaggcatcgtcttaacgaggcaccgaggcgtcgcattcttcagatggttcaacccttaagttagcgcttatgggagtaat

SEQ ID NO: 61 - DNA, 1349 bp, Escherichia coli
  source 1..1349: mol_type = genomic DNA; note = IS186C + 6bp TSD
  misc_feature 1..6: note = TSD
ataattcccataagcgctaacttaagggttgtggtattacgcctgatatgatttaacgtgccgatgaattactctcacgataactggtcagcaattctggcccatattggtaagcccgaagaactggatacttcggcacgtaatgccggggctctaacccgccgccgcgaaattcgtgatgctgcaactctgctacgtctggggctggcttacggccccggggggatgtcattacgtgaagtcactgcatgggctcagctccatgacgttgcaacattatctgacgtggctctcctgaagcggctgcggaatgccgccgactggtttggcatacttgccgcacaaacacttgctgtacgcgccgcagttacgggttgtacaagcggaaagagattgcgtcttgtcgatggaacagcaatcagtgcgcccgggggcggcagcgctgaatggcgactacatatgggatatgatcctcatacctgtcagttcactgattttgagctaaccgacagcagagacgctgaacggctggaccgatttgcgcaaacggcagacgagatacgcattgctgaccggggattcggttcgcgtcccgaatgtatccgctcacttgcttttggagaagctgattatatcgtccgggttcactggcgaggattgcgctggttaactgcagaaggaatgcgctttgacatgatgggttttctgcgcgggctggattgcggtaagaacggtgaaaccactgtaatgataggcaattcaggtaataaaaaagccggagctccctttccggcacgtctcattgccgtatcacttcctcccgaaaaagcattaatcagtaaaacccgactgctcagcgagaatcgtcgaaaaggacgagtagttcaggcggaaacgctggaagcagcgggccatgtgctattgctaacatcattaccggaagatgaatattcagcagagcaagtggctgattgttaccgtctgcgatggcaaattgaactggcttttaagcggctcaaaagtttgctgcacctggatgctttgcgtgcaaaggaacctgaactcgcgaaagcgtggatatttgctaatctactcgccgcatttttaattgacgacataatccagccatcgctggatttcccccccagaagtgccggatccgaaaagaagaactaactcgttgtggagaataacaaaaatggtcatctggagcttacaggtggccattcgtgggacagtatccctgacagcctacaaaacgcaattgaagaacgcgaggcatcgtcttaacgaggcaccgaggcgtcgcattcttcagatggttcaacccttaagttagcgcttatggg

SEQ ID NO: 62 - DNA, 1438 bp, Escherichia coli
  source 1..1438: mol_type = genomic DNA; note = IS4 + 12bp TSD
  misc_feature 1427..1438: note = TSD
taatgccagtcagttaagcaactgactggctctttttcggggctgtggggtatttccagggcctctcctttaccactctcgggaaggccctttcccttcttgtcggtaatttcacaagttgtcccatacttgcaagatcgcgcatcagctccggtatacgtcccggtgaagcgccctgcaatgtcatcagcattctcatcaccattccgcatgattctgagaaactcagttgattcggccagtaacctttcagatgttccgccattttaatcatctgatatctcaccagattataagccagtaagacaccccacagctcttgctccacaagctccggctttttacttctcagcgtcagcctgctccgttgcatcgtctgttttatctccctgtatcccagttcgatttcccagcgatgactgtacagatcccccatttctcctccggggaagcgcatggcgtccgtcatcgacgtcagcagatggcagacttttcctttgcgcgtcacggtcagcaggcgggcagtcacttcatttcccagtcccggccacttttttcgtgcctgcgggctggttttcagcttcaccagatgatcgcctttacccagttttctgatctcttcatattgcgctccctttctgagaggtatcatccagtggcggtgttctcccgccaggctccaggcatttaacagtcccagtgagtaataacctttatccattaacgtcagagtgttatcgccggtttgttctataagttgctcagcaagctcattttcgctgttcttcatcgtgccgaaggctgcagccgtcagcagatggctggtcagttccatctggcagaccattttgacctgcgggtagagcgccgggttcccggcatgtgtctggcgggggaaggctgcatcgttctctggtgtatccggtgtgcgccagaacacaccatcgatggccagcagggtcaggccgcaccagtgcggatgcggcgtggcgttatgccagagctgcgctgttttcgtgaacacgcggcggacagcctcacttcccaggcgctggcgggcctgaataacggcactgggggcaacgaaggggcgattgcccggcagcatgatgtccaggcgattcacaatctggtgaagaggttctttacgctcaagcgccatgccaacaatacaccagaccatcatttcgaggggaagacggcgcttgcgtagcgttacagtacctgattcggcaaggcaacgagagatgagttcggggtcgaggtaatcccccagagaagtcagtgggttacgcagagaatcgtaacgggataccagatcaagagcctgtccaatgtgcataaaaaaatccggaaacaagtgagcgtttccggattcttacacagccactggatcggtcaactgatccttaactgatcggcattaatcttggttctg

SEQ ID NO: 63 - DNA, 1223 bp, Escherichia coli
  source 1..1223: mol_type = genomic DNA; note = IS30C + 2bp TSD
  misc_feature 1222..1223: note = TSD
tgtagattcaattggtcaacgcaacagttatgtgaaaacatggggttgcggaggttttttgaatgagacgaacatttacagcagaggaaaaagcctctgtttttgaactatggaagaacggaacaggcttcagtgaaatagcgaatatcctgggttcaaaacccggaacgatcttcactatgttaagggatactggcggcataaaaccccatgagcgtaagcgggctgtagctcacctgacactgtctgagcgcgaggagatacgagctggtttgtcagccaaaatgagcattcgtgcgatagctactgcgctgaatcgcagtccttcgacgatctcacgtgaagttcagcgtaatcggggcagacgctattacaaagctgttgatgctaataaccgagccaacagaatggcgaaaaggccaaaaccgtgcttactggatcaaaatttaccattgcgaaagcttgttctggaaaagctggagatgaaatggtctccagagcaaatatcaggatggttaaggcgaacaaaaccacgtcaaaaaacgctgcgaatatcacctgagacaatttataaaacgctgtactttcgtagccgtgaagcgctacaccacctgaatatacagcatctgcgacggtcgcatagccttcgccatggcaggcgtcatacccgcaaaggcgaaagaggtacgattaacatagtgaacggaacaccaattcacgaacgttcccgaaatatcgataacagacgctctctagggcattgggagggcgatttagtctcaggtacaaaaaactctcatatagccacacttgtagaccgaaaatcacgttatacgatcatccttagactcaggggcaaagattctgtctcagtaaatcaggctcttaccgacaaattcctgagtttaccgtcagaactcagaaaatcactgacatgggacagaggaatggaactggccagacatctagaatttactgtcagcaccggcgttaaagtttacttctgcgatcctcagagtccttggcagcggggaacaaatgagaacacaaatgggctaattcggcagtactttcctaaaaagacatgtcttgcccaatatactcaacatgaactagatctggttgctgctcagctaaacaacagaccgagaaagacactgaagttcaaaacaccgaaagagataattgaaaggggtgttgcattgacagattgaatctacact

SEQ ID NO: 64 - DNA, 1747 bp, Escherichia coli
  source 1..1747: mol_type = genomic DNA; note = IS609 + 3bp TSD
  misc_feature 1..3: note = TSD
tatccggtgcgccgtaaaaccccatccttcagggcggggatataaggcgcggttttccacctgaccaggtgtttgctgttgttcaatgtattggcggatgacggatattggcgcacctccgcagctactggcaaaatagccaggactccacaaaacgcctttgtagtaatacctgaatgcaatatctggtcgatctcgtcgcagtcacctacccgatacgcctttgaggctgtttaccagactggatatcgccagtttgggaggatagttaattaacaaatggacgtgatctggttcgccatccatttcaaccagttcagcttcaaaatcagcacatacatttgaaaagtaagtgcgtagtttttctgtcgcgtcatggtcaaaaatctggcgtcggtatctggtgacaaagagcaggtgaacatgcatcaggaaaacacaatgccttccacgccggatatcggtttcttttttcacagaccaaagtatcatttgacctgtgaaacgattacaggcatttaaattccagttaagacccggtggtcaacaggagtgtgaaatgaggcgcttcgcaggcgcatgtcgtttcgttttcaatcgtgctctggcacgtcagaatgagaatcatgaggccggtaataaatacatcccttacgggaaaatggcttcctggctggttgagtggaaaaatgccactgaaacgcaatggcttaaagattctccctcacagccattgcaacagtcactgaaagaccttgagcgggcttacaaaaacttcttccggaagcgggctgcttttccccgattcaaaaagcggggacagaatgatgcattccgctacccgcagggcgttaagctcgatcaggaaaacagccgtatttttctgccgaaactgggctggatgcgctaccggaacagccgtcaggtcacgggtgttgtgaaaaatgtcactgtcagccagtcctgcggtaagtggtacatcagtattcagacagaaagtgaagtatcaactccggttcacccttcagcatcaatggtcgggctggatgctggcgtggctaaactcgccacgctgtcagatggcacagtctttgagcctgtaaacagttttcagaaaaaccagaagaagctggcgagacttcagcgacagttaagccgcaaggtcaaattcagcaacaactggcaaaagcagaaacgcaaaatacagcgactgcattcctgtatcgcaaatatccgcagggactaccttcacaaagtcacaacggccgtcagcaaaaaccacgcaatgatagtcattgaggatttgaaggtcagcaacatgtcaaagtcagcagcgggtacggtcagccagccggggcgcaatgtccgggcaaaatcaggtttaaaccgttcgatactggatcagggctggtatgaaatgcgccgccagcttgcgtataagcagctctggcgtggcggtcaggtgcttgctgttccgccagcgtatacaagccagcgttgcgcgtactgtggtcatacagcgaaagagaaccgcctgtcacaaagtaaattcagatgccaggtatgtggatatacagcgaacgccgatgtaaatggcgctcgcaacattttagcggcggggcacgccgttcttgcctgtggagagatggtgcagtcaggccgcccgttgaagcaggaacccaccgaaatgattcaggcgacagcctgaacgtagcagggatccacgtccttcagggcgtggaggatg

SEQ ID NO: 65 - DNA, 1336 bp, Escherichia coli
  source 1..1336: mol_type = genomic DNA; note = IS2A + 5bp TSD
  misc_feature 1..5: note = TSD
attactagactggccccctgaatctccagacaaccaatatcacttaaataagtgatagtcttaatactagtttttagactagtcattggagaacagatgattgatgtcttagggccggagaaacgcagacggcgtaccacacaggaaaagatcgcaattgttcagcagagctttgaaccggggatgacggtctccctcgttgcccggcaacatggtgtagcagccagccagttatttctctggcgtaagcaataccaggaaggaagtcttactgctgtcgccgccggagaacaggttgttcctgcctctgaacttgctgccgccatgaagcagattaaagaactccagcgcctgctcggcaagaaaacgatggaaaatgaactcctcaaagaagccgttgaatatggacgggcaaaaaagtggatagcgcacgcgcccttattgcccggggatggggagtaagcttagtcagccgttgtctccgggtgtcgcgtgcgcagttgcacgtcattctcagacgaaccgatgactggatggatggccgccgcagtcgtcacactgatgatacggatgtgcttctccgtatacaccatgttatcggagagctgccaacgtatggttatcgtcgggtatgggcgctgcttcgcagacaggcagaacttgatggtatgcctgcgatcaatgccaaacgtgtttaccggatcatgcgccagaatgcgctgttgcttgagcgaaaacctgctgtaccgccatcgaaacgggcacatacaggcagagtggccgtgaaagaaagcaatcagcgatggtgctctgacgggttcgagttctgctgtgataacggagagagactgcgtgtcacgttcgcgctggactgctgtgatcgtgaggcactgcactgggcggtcactaccggcggcttcaacagtgaaacagtacaggacgtcatgctgggagcggtggaacgccgcttcggcaacgatcttccgtcgtctccagtggagtggctgacggataatggttcatgctaccgggctaatgaaacacgccagttcgcccggatgttgggacttgaaccgaagaacacggcggtgcggagtccggagagtaacggaatagcagagagcttcgtgaaaacgataaagcgtgactacatcagtatcatgcccaaaccagacgggttaacggcagcaaagaaccttgcagaggcgttcgagcattataacgaatggcatccgcatagtgcgctgggttatcgctcgccacgggaatatctgcggcagcgggcttgtaatgggttaagtgataacagatgtctggaaatataggggcaaatcca

SEQ ID NO: 66 - DNA, 1261 bp, Escherichia coli
  source 1..1261: mol_type = genomic DNA; note = IS3B + 3bp TSD
  misc_feature 1259..1261: note = TSD
tgatcctacccacgtaatatggacacaggcctaagcgaggttcttgttttcaaattgttccggactgaggccgccacaccaactgtgccgccgccaccgattgtaatcacattcgatataattaaacaccgttgcccgcattatttcccggctgataaagtgttctccatggatacattccactttcagcgaatgaaagaagctttccacgcaggcattatcgtagcagcaaccttttgcgctcatacttccacgcagattatgccgcttcagttgcgcctgataatctgctgaacagtactggcctccacggtccgtgtgaacgataacgttccggggcctcttacgccgccacagcgccatctgcagggcatcgcaggccagttgcgccgtcatgcgtggcgacattgaccagccaataacggcacgtgaccacaggtcaatgaccactgccagatacagccagccttcatctgtacgtaagtacgtgatgtctcctgcccacttctggttcgggccactggcgtaaaaatcctgctccaacagattttctgacacaggcaggccgtgtgcgcggtagctgaccgggctgaacttccgggaggcctttgccctcagtccctgacggcgcaggcttgccgccacggtttttacgttaaaggggtaaccctgagcacgcagttcatccgtcaggcgtggggcaccgtaacgctgttttgaccgggtaaaagccgcgaggacaacgctgtcgcagtgttggcggaactgctgacgcgtgcttatccttgtccgccgctgacaccacgtataccagccgctgcgggccacccggagcacgcggcacattgctttgatgctgaactcagcctgatgtttttcaataaagacatacttcatttcaggcgcttcgcgaagtatgtcgcggccttttggaggatagccagctcttcatcccgttctgccagctggcgtttgagacgtgcaatctcggtagacatctccagttcacgttcagaagacgtctgctgattttgctgtttactgcgccagttgtagagttgtgattcatacaggctgagttcacgggctgcggcagtaacaccgatgcgttcagcaagcttcagggcttcactgcgaaattcaggcgaatgctgtttacggggttttttactggttgatactgtttttgtcatgtgagtcacctctgactgagagtttactcacttagccgcgtgtccactattgctgggtaagatcagat

SEQ ID NO: 67 - DNA, 1336 bp, Escherichia coli
  source 1..1336: mol_type = genomic DNA; note = IS2D + 5bp TSD
  misc_feature 1332..1336: note = TSD
tggatttgcccctatatttccagacatctgttatcacttaacccattacaagcccgctgccgcagatattcccgtggcgagcgataacccagcgcactatgcggatgccattcgttataatgctcgaacgcctctgcaaggttctttgctgccgttaacccgtctggtttgggcatgatactgatgtagtcacgctttatcgttttcacgaagctctctgctattccgttactctccggactccgcaccgccgtgttcttcggttcaagtcccaacatccgggcgaactggcgtgtttcattagcccggtagcatgaaccattatccgtcagccactccactggagacgacggaagatcgttgccgaagcggcgttccaccgctcccagcatgacgtcctgtactgtttcactgttgaagccgccggtagtgaccgcccagtgcagtgcctcacgatcacagcagtccagcgcgaacgtgacacgcagtctctctccgttatcacagcagaactcgaacccgtcagagcaccatcgctgattgctttctttcacggccactctgcctgtatgtgcccgtttcgatggcggtacagcaggttttcgctcaagcaacagcgcattctggcgcatgatccggtaaacacgtttggcattgatcgcaggcataccatcaagttctgcctgtctgcgaagcagcgcccatacccgacgataaccatacgttggcagctctccgataacatggtgtatacggagaagcacatccgtatcatcagtgtgacgactgcggcggccatccatccagtcatcggttcgtctgagaatgacgtgcaactgcgcacgcgacacccggagacaacggctgactaagcttactccccatccccgggcaataagggcgcgtgcgctatccacttttttgcccgtccatattcaacggcttctttgaggagttcattttccatcgttttcttgccgagcaggcgctggagttctttaatctgcttcatggcggcagcaagttcagaggcaggaacaacctgttctccggcggcgacagcagtaagacttccttcctggtattgcttacgccagagaaataactggctggctgctacaccatgttgccgggcaacgagggagaccgtcatccccggttcaaagctctgctgaacaattgcgatcttttcctgtgtggtacgccgtctgcgtttctccggccctaagacatcaatcatctgttctccaatgactagtctaaaaactagtattaagactatcacttatttaagtgatattggttgtctggagattcagggggccagtctaaaccc

SEQ ID NO: 68 - DNA, 1261 bp, Escherichia coli
  source 1..1261: mol_type = genomic DNA; note = IS3E + 3bp TSD
  misc_feature 1..3: note = TSD
gtctgatcttacccagcaatagtggacacgcggctaagtgagtaaactctcagtcagaggtgactcacatgacaaaaacagtatcaaccagtaaaaaaccccgtaaacagcattcgcctgaatttcgcagtgaagccctgaagcttgctgaacgcatcggtgttactgccgcagcccgtgaactcagcctgtatgaatcacaactctacaactggcgcagtaaacagcaaaatcagcagacgtcttctgaacgtgaactggagatgtctaccgagattgcacgtctcaaacgccagctggcagaacgggatgaagagctggctatcctccaaaaggccgcgacatacttcgcgaagcgcctgaaatgaagtatgtctttattgaaaaacatcaggctgagttcagcatcaaagcaatgtgccgcgtgctccgggtggcccgcagcggctggtatacgtggtgtcagcggcggacaaggataagcacgcgtcagcagttccgccaacactgcgacagcgttgtcctcgcggcttttacccggtcaaaacagcgttacggtgccccacgcctgacggatgaactgcgtgctcagggttacccctttaacgtaaaaaccgtggcggcaagcctgcgccgtcagggactgagggcaaaggcctcccggaagttcagcccggtcagctaccgcgcacacggcctgcctgtgtcagaaaatctgttggagcaggatttttacgccagtggcccgaaccagaagtgggcaggagacatcacgtacttacgtacagatgaaggctggctgtatctggcagtggtcattgacctgtggtcacgtgccgttattggctggtcaatgtcgccacgcatgacggcgcaactggcctgcgatgccctgcagatggcgctgtggcggcgtaagaggccccggaacgttatcgttcacacggaccgtggaggccagtactgttcagcagattatcaggcgcaactgaagcggcataatctgcgtggaagtatgagcgcaaaaggttgctgctacgataatgcctgcgtggaaagcttctttcattcgctgaaagtggaatgtatccatggagaacactttatcagccgggaaataatgcgggcaacggtgtttaattatatcgaatgtgattacaatcggtggcggcggcacagttggtgtggcggcctcagtccggaacaatttgaaaacaagaacctcgcttaggcctgtgtccatattacgtgggtaggatca

SEQ ID NO: 69 - DNA, 1336 bp, Escherichia coli
  source 1..1336: mol_type = genomic DNA; note = IS2F + 5bp TSD
  misc_feature 1332..1336: note = TSD
tggatttgcccctatatttccagacatctgttatcacttaacccattacaagcccgctgccgcagatattcccgtggcgagcgataacccagcgcactatgcggatgccattcgttataatgctcgaacgcctctgcaaggttctttgctgccgttaacccgtctggtttgggcatgatactgatgtagtcacgctttatcgttttcacgaagctctctgctattccgttactctccggactccgcaccgccgtgttcttcggttcaagtcccaacatccgggcgaactggcgtgtttcattagcccggtagcatgaaccattatccgtcagccactccactggagacgacggaagatcgttgccgaagcggcgttccaccgctcccagcatgacgtcctgtactgtttcactgttgaagccgccggtagtgaccgcccagtgcagtgcctcacgatcacagcagtccagcgcgaacgtgacacgcagtctctctccgttatcacagcagaactcgaacccgtcagagcaccatcgctgattgctttctttcacggccactctgcctgtatgtgcccgtttcgatggcggtacagcaggttttcgctcaagcaacagcgcattctggcgcatgatccggtaaacacgtttggcattgatcgcaggcataccatcaagttctgcctgtctgcgaagcagcgcccatacccgacgataaccatacgttggcagctctccgataacatggtgtatacggagaagcacatccgtatcatcagtgtgacgactgcggcggccatccatccagtcatcggttcgtctgagaatgacgtgcaactgcgcacgcgacacccggagacaacggctgactaagcttactccccatccccgggcaataagggcgcgtgcgctatccacttttttgcccgtccatattcaacggcttctttgaggagttcattttccatcgttttcttgccgagcaggcgctggagttctttaatctgcttcatggcggcagcaagttcagaggcaggaacaacctgttctccggcggcgacagcagtaagacttccttcctggtattgcttacgccagagaaataactggctggctgctacaccatgttgccgggcaacgagggagaccgtcatccccggttcaaagctctgctgaacaattgcgatcttttcctgtgtggtacgccgtctgcgtttctccggccctaagacatcaatcatctgttctccaatgactagtctaaaaactagtattaagactatcacttatttaagtgatattggttgtctggagattcagggggccagtctagtggc

SEQ ID NO: 70 - DNA, 1336 bp, Escherichia coli
  source 1..1336: mol_type = genomic DNA; note = IS2I + 5bp TSD
  misc_feature 1332..1336: note = TSD
tagactggccccctgaatctccagacaaccaatatcacttaaataagtgatagtcttaatactagtttttagactagtcattggagaacagatgattgatgtcttagggccggagaaacgcagacggcgtaccacacaggaaaagatcgcaattgttcagcagagctttgaaccggggatgacggtctccctcgttgcccggcaacatggtgtagcagccagccagttatttctctggcgtaagcaataccaggaaggaagtcttactgctgtcgccgccggagaacaggttgttcctgcctctgaacttgctgccgccatgaagcagattaaagaactccagcgcctgctcggcaagaaaacgatggaaaatgaactcctcaaagaagccgttgaatatggacgggcaaaaaagtggatagcgcacgcgcccttattgcccggggatggggagtaagcttagtcagccgttgtctccgggtgtcgcgtgcgcagttgcacgtcattctcagacgaaccgatgactggatggatggccgccgcagtcgtcacactgatgatacggatgtgcttctccgtatacaccatgttatcggagagctgccaacgtatggttatcgtcgggtatgggcgctgcttcgcagacaggcagaacttgatggtatgcctgcgatcaatgccaaacgtgtttaccggatcatgcgccagaatgcgctgttgcttgagcgaaaacctgctgtaccgccatcgaaacgggcacatacaggcagagtggccgtgaaagaaagcaatcagcgatggtgctctgacgggttcgagttctgctgtgataacggagagagactgcgtgtcacgttcgcgctggactgctgtgatcgtgaggcactgcactgggcggtcactaccggcggcttcaacagtgaaacagtacaggacgtcatgctgggagcggtggaacgccgcttcggcaacgatcttccgtcgtctccagtggagtggctgacggataatggttcatgctaccgggctaatgaaacacgccagttcgcccggatgttgggacttgaaccgaagaacacggcggtgcggagtccggagagtaacggaatagcagagagcttcgtgaaaacgataaagcgtgactacatcagtatcatgcccaaaccagacgggttaacggcagcaaagaaccttgcagaggcgttcgagcattataacgaatggcatccgcatagtgcgctgggttatcgctcgccacgggaatatctgcggcagcgggcttgtaatgggttaagtgataacagatgtctggaaatataggggcaaatccagttat

SEQ ID NO: 71 - DNA, 1336 bp, Escherichia coli
  source 1..1336: mol_type = genomic DNA; note = IS2K + 5bp TSD
  misc_feature 1332..1336: note = TSD
tagactggccccctgaatctccagacaaccaatatcacttaaataagtgatagtcttaatactagtttttagactagtcattggagaacagatgattgatgtcttagggccggagaaacgcagacggcgtaccacacaggaaaagatcgcaattgttcagcagagctttgaaccggggatgacggtctccctcgttgcccggcaacatggtgtagcagccagccagttatttctctggcgtaagcaataccaggaaggaagtcttactgctgtcgccgccggagaacaggttgttcctgcctctgaacttgctgccgccatgaagcagattaaagaactccagcgcctgctcggcaagaaaacgatggaaaatgaactcctcaaagaagccgttgaatatggacgggcaaaaaagtggatagcgcacgcgcccttattgcccggggatggggagtaagcttagtcagccgttgtctccgggtgtcgcgtgcgcagttgcacgtcattctcagacgaaccgatgactggatggatggccgccgcagtcgtcacactgatgatacggatgtgcttctccgtatacaccatgttatcggagagctgccaacgtatggttatcgtcgggtatgggcgctgcttcgcagacaggcagaacttgatggtatgcctgcgatcaatgccaaacgtgtttaccggatcatgcgccagaatgcgctgttgcttgagcgaaaacctgctgtaccgccatcgaaacgggcacatacaggcagagtggccgtgaaagaaagcaatcagcgatggtgctctgacgggttcgagttctgctgtgataacggagagagactgcgtgtcacgttcgcgctggactgctgtgatcgtgaggcactgcactgggcggtcactaccggcggcttcaacagtgaaacagtacaggacgtcatgctgggagcggtggaacgccgcttcggcaacgatcttccgtcgtctccagtggagtggctgacggataatggttcatgctaccgggctaatgaaacacgccagttcgcccggatgttgggacttgaaccgaagaacacggcggtgcggagtccggagagtaacggaatagcagagagcttcgtgaaaacgataaagcgtgactacatcagtatcatgcccaaaccagacgggttaacggcagcaaagaaccttgcagaggcgttcgagcattataacgaatggcatccgcatagtgcgctgggttatcgctcgccacgggaatatctgcggcagcgggcttgtaatgggttaagtgataacagatgtctggaaatataggggcaaatccaccttg

SEQ ID NO: 72-73 - skipped (2 entries)

SEQ ID NO: 74 - DNA, 1350 bp, Escherichia coli
  source 1..1350: mol_type = genomic DNA; note = insL-2 + 13bp TSD
  misc_feature 1..13: note = TSD
ggggaaacatcccataagcgctaacttaagggttgaaccatctgaagaatgcgacgcctcggtgcctcgttaagacgatgcctcgcgttcttcaattgcgttttgtaggctgtcagggatactgtcccacgaatggccacctgtaagctccagatgaccatttttgttattctccacaacgagttagttcttcttttcggatccggcacttctgggggggaaatccagcgatggctggattatgtcgtcaattaaaaatgcggcgagtagattagcaaatatccacgctttcgcgagttcaggttcctttgcacgcaaagcatccaggtgcagcaaacttttgagccgcttaaaagccagttcaatttgccatcgcagacggtaacaatcagccacttgctctgctgaatattcatcttccggtaatgatgttagcaatagcacatggcccgctgcttccagcgtttccgcctgaactactcgtccttttcgacgattctcgctgagcagtcgggttttactgattaatgctttttcgggaggaagtgatacggcaatgagacgtgccggaaagggagctccggcttttttattacctgaattgcctatcattacagtggtttcaccgttcttaccgcaatccagcccgcgcagaaaacccatcatgtcaaagcgcattccttctgcagttaaccagcgcaatcctcgccagtgaacccggacgatataatcagcttctccaaaagcaagtgagcggatacattcgggacgcgaaccgaatccccggtcagcaatgcgtatctcgtctgccgtttgcgcaaatcggtccagccgttcagcgtctctgctgtcggttagctcaaaatcagtgaactgacaggtatgaggatcatatcccatatgtagtcgccattcagcgctgccgcccccgggcgcactgattgctgttccatcgacaagacgcaatctctttccgcttgtacaacccgtaactgcggcgcgtacagcaagtgtttgtgcggcaagtatgccaaaccagtcggcggcattccgcagccgcttcaggagagccacgtcagataatgttgcaacgtcatggagctgagcccatgcagtgacttcacgtaatgacatccccccggggccgtaagccagccccagacgtagcagagttgcagcatcacgaatttcgcggcggcgggttagagccccggcattacgtgccgaagtatccagttcttcgggcttaccaatatgggccagaattgctgaccagttatcgtgagagtaattcatcggcacgttaaatcatatcaggcgtaataccacaacccttaagttagcgcttat

SEQ ID NO: 75 - DNA, 75 bp, Synthetic construct
  source 1..75: mol_type = other DNA; note = FP1 IS1A oligomer
tacttccttcatggggatgctgaaaagagtagtaattgcttacctcaatgtgtatgtgtaggctggagctgcttc

SEQ ID NO: 76 - DNA, 75 bp, Synthetic construct
  source 1..75: mol_type = other DNA; note = RP1 IS1A oligomer
ccccacaaagaatatggatattgtgatacacattgaggtaagcaattactactctgtgtaggctggagctgcttc

SEQ ID NO: 77 - DNA, 75 bp, Synthetic construct
  source 1..75: mol_type = other DNA; note = FP1 IS1B oligomer
gctgagtgaggcttcatcgagcgatttatcgatttggcccgagaacacaaatggggtgtaggctggagctgcttc

SEQ ID NO: 78 - DNA, 75 bp, Synthetic construct
  source 1..75: mol_type = other DNA; note = RP1 IS1B oligomer
ttttaggaaagtactgccgaattagcccatttgtgttctcgggccaaatcgataagtgtaggctggagctgcttc

SEQ ID NO: 79 - DNA, 75 bp, Synthetic construct
  source 1..75: mol_type = other DNA; note = FP1 IS1C oligomer
cttcagcggtgatggaggcgatatatctgttaccgggtaagaattttcagcccgggtgtaggctggagctgcttc

SEQ ID NO: 80 - DNA, 75 bp, Synthetic construct
  source 1..75: mol_type = other DNA; note = RP1 IS1C oligomer
tattcgacataggtacgtgaaacatccgggctgaaaattcttacccggtaacagagtgtaggctggagctgcttc

SEQ ID NO: 81 - DNA, 75 bp, Synthetic construct
  source 1..75: mol_type = other DNA; note = FP1 IS1D oligomer
aaagcttgtgtttcataacttttcctttattcatcgcatggacaatacgtacgctgtgtaggctggagctgcttc

SEQ ID NO: 82 - DNA, 75 bp, Synthetic construct
  source 1..75: mol_type = other DNA; note = RP1 IS1D oligomer
ctcaaagtagacaatcctgatctcaagcgtacgtattgtccatgcgatgaataaagtgtaggctggagctgcttc

SEQ ID NO: 83 - DNA, 75 bp, Synthetic construct
  source 1..75: mol_type = other DNA; note = FP1 IS1E oligomer
cggggattatagcatttcaatatttacttatgacattaaaagtaacttttttgaagtgtaggctggagctgcttc

SEQ ID NO: 84 - DNA, 75 bp, Synthetic construct
  source 1..75: mol_type = other DNA; note = RP1 IS1E oligomer
tttctgtgccaatattatctctaatttcaaaaaagttacttttaatgtcataagtgtgtaggctggagctgcttc

SEQ ID NO: 85 - DNA, 75 bp, Synthetic construct
  source 1..75: mol_type = other DNA; note = FP1 IS1F oligomer
tattattgacatcctcactgccctaaaggatggggatttcgaccatgtttatttcgtgtaggctggagctgcttc

SEQ ID NO: 86 - DNA, 75 bp, Synthetic construct
  source 1..75: mol_type = other DNA; note = RP1 IS1F oligomer
aataagaacaatacccacaatgtatgaaataaacatggtcgaaatccccatccttgtgtaggctggagctgcttc

SEQ ID NO: 87 - DNA, 75 bp, Synthetic construct
  source 1..75: mol_type = other DNA; note = FP1 IS1H oligomer
gtattacagcggcgatctctgccgtatggatgaggctggctatataaaaattaccgtgtaggctggagctgcttc

SEQ ID NO: 88 - DNA, 75 bp, Synthetic construct
  source 1..75: mol_type = other DNA; note = RP1 IS1H oligomer
ggacaataatatcttttttgcgtccggtaatttttatatagccagcctcatccatgtgtaggctggagctgcttc

SEQ ID NO: 89 - DNA, 75 bp, Synthetic construct
  source 1..75: mol_type = other DNA; note = FP1 IS5A oligomer
atggaaggtgcgaataagcggggaaattcttctcggctgaggaggcgttatgagcgtgtaggctggagctgcttc

SEQ ID NO: 90 - DNA, 75 bp, Synthetic construct
  source 1..75: mol_type = other DNA; note = RP1 IS5A oligomer
taatcagatacaaaaagggccgccagctcataacgcctcctcagccgagaagaatgtgtaggctggagctgcttc

SEQ ID NO: 91 - DNA, 75 bp, Synthetic construct
  source 1..75: mol_type = other DNA; note = FP1 IS5B oligomer
acctacagcaacgatgtcatcagtgcttacaccgagtgctttagtgaagtcatttgtgtaggctggagctgcttc

SEQ ID NO: 92 - DNA, 75 bp, Synthetic construct
  source 1..75: mol_type = other DNA; note = RP1 IS5B oligomer
attacaaaatcaacctgcttgacaaaaatgacttcactaaagcactcggtgtaaggtgtaggctggagctgcttc

SEQ ID NO: 93 - DNA, 75 bp, Synthetic construct
  source 1..75: mol_type = other DNA; note = FP1 IS5D oligomer
tatcgtctgcaactttattgtgcagtgttgtgcctgttaggtaacatttagtttggtgtaggctggagctgcttc

SEQ ID NO: 94 - DNA, 75 bp, Synthetic construct
  source 1..75: mol_type = other DNA; note = RP1 IS5D oligomer
aaacagcaatatctttacatttagccaaactaaatgttacctaacaggcacaacagtgtaggctggagctgcttc

SEQ ID NO: 95 - DNA, 75 bp, Synthetic construct
  source 1..75: mol_type = other DNA; note = FP1 IS5F oligomer
tcagatcatcaatagtcagggaaggaagtagcaacattagctaactaatcaatgcgtgtaggctggagctgcttc

SEQ ID NO: 96 - DNA, 75 bp, Synthetic construct
  source 1..75: mol_type = other DNA; note = RP1 IS5F oligomer
cctcttagctggatttacaatcaacgcattgattagttagctaatgttgctacttgtgtaggctggagctgcttc

SEQ ID NO: 97 - DNA, 75 bp, Synthetic construct
  source 1..75: mol_type = other DNA; note = FP1 IS5Y oligomer
gactttctccggggattatctccgcgtaactgacaacaaggggaaaacgcacgacgtgtaggctggagctgcttc

SEQ ID NO: 98 - DNA, 75 bp, Synthetic construct
  source 1..75: mol_type = other DNA; note = RP1 IS5Y oligomer
gaccgtcatcacttccggtcagcacgtcgtgcgttttccccttgttgtcagttacgtgtaggctggagctgcttc

SEQ ID NO: 99 - DNA, 75 bp, Synthetic construct
  source 1..75: mol_type = other DNA; note = FP1 IS5H oligomer
cgtaatagaattatccggaatggtggcgactatgcactagaacaccacaatttcggtgtaggctggagctgcttc

SEQ ID NO: 100 - DNA, 75 bp, Synthetic construct
  source 1..75: mol_type = other DNA; note = RP1 IS5H oligomer
ctgtgacagtgccttaccgagagagcgaaattgtggtgttctagtgcatagtcgcgtgtaggctggagctgcttc

SEQ ID NO: 101 - DNA, 75 bp, Synthetic construct
  source 1..75: mol_type = other DNA; note = FP1 IS5I oligomer
cgtatcagaatagatactttctttaggaatttttgttttattaatccctaacatagtgtaggctggagctgcttc

SEQ ID NO: 102 - DNA, 75 bp, Synthetic construct
  source 1..75: mol_type = other DNA; note = RP1 IS5I oligomer
tgctttctgattttattgtgtcatttatgttagggattaataaaacaaaaattccgtgtaggctggagctgcttc

SEQ ID NO: 103 - DNA, 75 bp, Synthetic construct
  source 1..75: mol_type = other DNA; note = FP1 IS5K oligomer
tcaccatactcaacagttgatgccaatgctatgggtgaatataacgctgtagccagtgtaggctggagctgcttc

SEQ ID NO: 104 - DNA, 75 bp, Synthetic construct
  source 1..75: mol_type = other DNA; note = RP1 IS5K oligomer
tgtcgttccgcaatatctgttctggtggctacagcgttatattcacccatagcatgtgtaggctggagctgcttc

SEQ ID NO: 105 - DNA, 75 bp, Synthetic construct
  source 1..75: mol_type = other DNA; note = FP1 IS5LO oligomer
tcatgtttgtcatctggagccatagaacagggttcatcatctaaatcaggtcatagtgtaggctggagctgcttc

SEQ ID NO: 106 - DNA, 75 bp, Synthetic construct
  source 1..75: mol_type = other DNA; note = RP1 IS5LO oligomer
gtttggcgttaagtatctcgaagcgtatgacctgatttagatgatgaaccctgttgtgtaggctggagctgcttc

SEQ ID NO: 107 - DNA, 75 bp, Synthetic construct
  source 1..75: mol_type = other DNA; note = FP1 IS5R oligomer
aaaatgacaatccgggcagcacaggaacagcatcaattagtacttcccccaataagtgtaggctggagctgcttc

SEQ ID NO: 108 - DNA, 75 bp, Synthetic construct
  source 1..75: mol_type = other DNA; note = RP1 IS5R oligomer
accattttgcataaacaccagccaattattgggggaagtactaattgatgctgttgtgtaggctggagctgcttc

SEQ ID NO: 109 - DNA, 75 bp, Synthetic construct
  source 1..75: mol_type = other DNA; note = FP1 IS5T oligomer
aagatctacttaatataaatttcactgacgcaaatttaggtgacactatttttttgtgtaggctggagctgcttc

SEQ ID NO: 110 - DNA, 75 bp, Synthetic construct
  source 1..75: mol_type = other DNA; note = RP1 IS5T oligomer
tttgggggtagggtgttctttatgtaaaaaaatagtgtcacctaaatttgcgtcagtgtaggctggagctgcttc

SEQ ID NO: 111 - DNA, 75 bp, Synthetic construct
  source 1..75: mol_type = other DNA; note = FP1 IS186A oligomer
ttgaagatatgcgagcacctgtaaagtggcggggatcactccccgccgttgctctgtgtaggctggagctgcttc

SEQ ID NO: 112 - DNA, 75 bp, Synthetic construct
  source 1..75: mol_type = other DNA; note = RP1 IS186A oligomer
ttttcacggcttacgaatccgagtaagagcaacggcggggagtgatccccgccacgtgtaggctggagctgcttc

SEQ ID NO: 113 - DNA, 75 bp, Synthetic construct
  source 1..75: mol_type = other DNA; note = FP1 IS186B oligomer
gcttacgaaccgaagaagtagccgttgtgcggggagtaatccccgcatatccggtgtgtaggctggagctgcttc

SEQ ID NO: 114 - DNA, 75 bp, Synthetic construct
  source 1..75: mol_type = other DNA; note = RP1 IS186B oligomer
ggtgccttaccatcctgacctgacaaccggatatgcggggattactccccgcacagtgtaggctggagctgcttc

SEQ ID NO: 115 - DNA, 75 bp, Synthetic construct
  source 1..75: mol_type = other DNA; note = FP1 IS186C oligomer
tggtgctgtaagaccatacataaaaaagccggggataattccccggtttttttacgtgtaggctggagctgcttc

SEQ ID NO: 116 - DNA, 75 bp, Synthetic construct
  source 1..75: mol_type = other DNA; note = RP1 IS186C oligomer
cgcagccattagctgattaacaggcgtaaaaaaaccggggaattatccccggcttgtgtaggctggagctgcttc

SEQ ID NO: 117 - DNA, 75 bp, Synthetic construct
  source 1..75: mol_type = other DNA; note = FP1 IS4 oligomer
taacagttgatgctgaaacgaaataggcatcttggttctggtgtttgtaacaaacgtgtaggctggagctgcttc

SEQ ID NO: 118 - DNA, 75 bp, Synthetic construct
  source 1..75: mol_type = other DNA; note = RP1 IS4 oligomer
attgagcatatttttgtagctgatagtttgttacaaacaccagaaccaagatgccgtgtaggctggagctgcttc

SEQ ID NO: 119 - DNA, 75 bp, Synthetic construct
  source 1..75: mol_type = other DNA; note = FP1 IS911A & IS30A oligomer
tttgctaagagcttcattcatgaatccttttcactagggagtgtgcccggagttcgtgtaggctggagctgcttc

SEQ ID NO: 120 - DNA, 75 bp, Synthetic construct
  source 1..75: mol_type = other DNA; note = RP1 IS911A & IS30A oligomer
tcatttaagcatccatgcccgccctgaactccgggcacactccctagtgaaaagggtgtaggctggagctgcttc

SEQ ID NO: 121 - DNA, 75 bp, Synthetic construct
  source 1..75: mol_type = other DNA; note = FP1 IS30B oligomer
gctgagtgaggcttcatcgagcgatttatcgatttggcccttaaatgactcggaggtgtaggctggagctgcttc

SEQ ID NO: 122 - DNA, 75 bp, Synthetic construct
  source 1..75: mol_type = other DNA; note = RP1 IS30B oligomer
gaatcgccacgggtttaacagacacctccgagtcatttaagggccaaatcgataagtgtaggctggagctgcttc

SEQ ID NO: 123 - DNA, 75 bp, Synthetic construct
  source 1..75: mol_type = other DNA; note = FP1 ISZ oligomer
aagttgctttgggtaaacaaaaaatacggccccagaaggggccgtttatgttgccgtgtaggctggagctgcttc

SEQ ID NO: 124 - DNA, 75 bp, Synthetic construct
  source 1..75: mol_type = other DNA; note = RP1 ISZ oligomer
atccgcttaatcagtagcgctgtctggcaacataaacggccccttctggggccgtgtgtaggctggagctgcttc

SEQ ID NO: 125 - DNA, 75 bp, Synthetic construct
  source 1..75: mol_type = other DNA; note = FP1 IS30C oligomer
ttatgctgattccggtgcgaaaattgttaataaaggtactgttgaaattcagaatgtgtaggctggagctgcttc

SEQ ID NO: 126 - DNA, 75 bp, Synthetic construct
  source 1..75: mol_type = other DNA; note = RP1 IS30C oligomer
caccagtaacaaaagcaaaacctaaattctgaatttcaacagtacctttattaacgtgtaggctggagctgcttc

SEQ ID NO: 127 - DNA, 75 bp, Synthetic construct
  source 1..75: mol_type = other DNA; note = FP1 IS609 oligomer
aaaagtagttccagacgcgccatcgttagatggcgctttttcaatatcggtttctgtgtaggctggagctgcttc

SEQ ID NO: 128 - DNA, 75 bp, Synthetic construct
  source 1..75: mol_type = other DNA; note = RP1 IS609 oligomer
cgtggtgttgaatttaatcgctgacagaaaccgatattgaaaaagcgccatctaagtgtaggctggagctgcttc

SEQ ID NO: 129 - DNA, 75 bp, Synthetic construct
  source 1..75: mol_type = other DNA; note = FP1 IS911, IS30D & IS600 oligomer
catgcgtccagataagtcattgtaaaagtcgaatcagggcgactacctgaagggagtgtaggctggagctgcttc

SEQ ID NO: 130 - DNA, 75 bp, Synthetic construct
  source 1..75: mol_type = other DNA; note = RP1 IS911B, IS30D & IS600 oligomer
actgcaactgccaggcgaccgcggctcccttcaggtagtcgccctgattcgacttgtgtaggctggagctgcttc

SEQ ID NO: 131 - DNA, 75 bp, Synthetic construct
  source 1..75: mol_type = other DNA; note = FP1 IS150 oligomer
tgcggcattcccagcctcctgtgttgatttccaacgagtaaactttgatttataggtgtaggctggagctgcttc

SEQ ID NO: 132 - DNA, 75 bp, Synthetic construct
  source 1..75: mol_type = other DNA; note = RP1 IS150 oligomer
gcagacagagaaaagccccacctgactataaatcaaagtttactcgttggaaatcgtgtaggctggagctgcttc

SEQ ID NO: 133 - DNA, 75 bp, Synthetic construct
  source 1..75: mol_type = other DNA; note = FP1 IS3A oligomer
cgaggtgacctatacgccagtgcctcttacccagcaatagttaggcctgtgtccagtgtaggctggagctgcttc

SEQ ID NO: 134 - DNA, 75 bp, Synthetic construct
  source 1..75: mol_type = other DNA; note = RP1 IS3A oligomer
actttatgatcctacccacgtaatatggacacaggcctaactattgctgggtaaggtgtaggctggagctgcttc

SEQ ID NO: 135 - DNA, 75 bp, Synthetic construct
  source 1..75: mol_type = other DNA; note = FP1 IS2A oligomer
cgccattgctgattattgtgccaggacgaataaacgcataattacctatcaggcagtgtaggctggagctgcttc

SEQ ID NO: 136 - DNA, 75 bp, Synthetic construct
  source 1..75: mol_type = other DNA; note = RP1 IS2A oligomer
gggtccggtagtgattggcgcaaactgcctgataggtaattatgcgtttattcgtgtgtaggctggagctgcttc

SEQ ID NO: 137 - DNA, 75 bp, Synthetic construct
  source 1..75: mol_type = other DNA; note = FP1 IS3B oligomer
tactgttgcgttgaccgaatctactgggtggggggctgattacaacctgtacgccgtgtaggctggagctgcttc

SEQ ID NO: 138 - DNA, 75 bp, Synthetic construct
  source 1..75: mol_type = other DNA; note = RP1 IS3B oligomer
cgccgttagttacggtgatagtattggcgtacaggttgtaatcagccccccacccgtgtaggctggagctgcttc

SEQ ID NO: 139 - DNA, 75 bp, Synthetic construct
  source 1..75: mol_type = other DNA; note = FP1 IS3C oligomer
tgcacaggacgttgccgcggtaacaggcgcaaccgtaatcaccagcataaatcaggtgtaggctggagctgcttc

SEQ ID NO: 140 - DNA, 75 bp, Synthetic construct
  source 1..75: mol_type = other DNA; note = RP1 IS3C oligomer
ctgcccgcgccattttagccgcagcctgatttatgctggtgattacggttgcgccgtgtaggctggagctgcttc

SEQ ID NO: 141 - DNA, 75 bp, Synthetic construct
  source 1..75: mol_type = other DNA; note = FP1 IS3D oligomer
gatgtggtgaatttttgtgagtcaccataaagcggcatttgtgcctggcacacgcgtgtaggctggagctgcttc

SEQ ID NO: 142 - DNA, 75 bp, Synthetic construct
  source 1..75: mol_type = other DNA; note = RP1 IS3D oligomer
gcctgaacgccgtcttccatcaaacgcgtgtgccaggcacaaatgccgctttatggtgtaggctggagctgcttc

SEQ ID NO: 143 - DNA, 75 bp, Synthetic construct
  source 1..75: mol_type = other DNA; note = FP1 IS2D oligomer
caggatattgacagttttgaacatcatgggacaagaaccccagaacttacttatggtgtaggctggagctgcttc

SEQ ID NO: 144 - DNA, 75 bp, Synthetic construct
  source 1..75: mol_type = other DNA; note = RP1 IS2D oligomer
ttaacaattttcgcaccggaatcagcataagtaagttctggggttcttgtcccatgtgtaggctggagctgcttc

SEQ ID NO: 145 - DNA, 75 bp, Synthetic construct
  source 1..75: mol_type = other DNA; note = FP1 IS3E oligomer
ggcgataagcattgtcgtacttccgctgtcgagaataacggtcatcccttcgtgggtgtaggctggagctgcttc

SEQ ID NO: 146 - DNA, 75 bp, Synthetic construct
  source 1..75: mol_type = other DNA; note = RP1 IS3E oligomer
tagcgcaggcggcagtcaaaatgatccacgaagggatgaccgttattctcgacaggtgtaggctggagctgcttc

SEQ ID NO: 147 - DNA, 75 bp, Synthetic construct
  source 1..75: mol_type = other DNA; note = FP1 IS2E oligomer
ccgccatcgaaacgggcacatacaggcagagtggccgtgagtgataacagatgtcgtgtaggctggagctgcttc

SEQ ID NO: 148 - DNA, 75 bp, Synthetic construct
  source 1..75: mol_type = other DNA; note = RP1 IS2E oligomer
ctgtggatttgcccctatatttccagacatctgttatcactcacggccactctgcgtgtaggctggagctgcttc

SEQ ID NO: 149 - DNA, 75 bp, Synthetic construct
  source 1..75: mol_type = other DNA; note = FP1 IS2F oligomer
caactccttggcaggccgtaaacaaatccgcattcgtggcgaagcatcctcccgtgtgtaggctggagctgcttc

SEQ ID NO: 150 - DNA, 75 bp, Synthetic construct
  source 1..75: mol_type = other DNA; note = RP1 IS2F oligomer
cctgaccatcaatgagaattaaaacacgggaggatgcttcgccacgaatgcggatgtgtaggctggagctgcttc

SEQ ID NO: 151 - DNA, 75 bp, Synthetic construct
  source 1..75: mol_type = other DNA; note = FP1 IS2H oligomer
tgagtaaacagatcaatggaagtaaattccaattgtttatctaaacttgctctttgtgtaggctggagctgcttc

SEQ ID NO: 152 - DNA, 75 bp, synthetic construct
  source 1..75: mol_type = other DNA; note = RP1 IS2H oligomer
tctttcaaagataaacaccagaagaaaagagcaagtttagataaacaattggaatgtgtaggctggagctgcttc

SEQ ID NO: 153 - DNA, 75 bp, Synthetic construct
  source 1..75: mol_type = other DNA; note = Fp1 IS2I oligomer
gcgaattgattaaaaatatttattgttcattatccgttatcatcattggttgtgcgtgtaggctggagctgcttc

SEQ ID NO: 154 - DNA, 75 bp, Synthetic construct
  source 1..75: mol_type = other DNA; note = Rp1 IS2I oligomer
gttgaattcaacggcataagctgacgcacaaccaatgatgataacggataatgaagtgtaggctggagctgcttc

SEQ ID NO: 155 - DNA, 75 bp, Synthetic construct
  source 1..75: mol_type = other DNA; note = Fp1 IS2K oligomer
actgacgtaaggagtgctgcagggatttgatggtcccttgtgctgatatgaatacgtgtaggctggagctgcttc

SEQ ID NO: 156 - DNA, 75 bp, Synthetic construct
  source 1..75: mol_type = other DNA; note = Rp1 IS2K oligomer
gaaaagtattctgtataaaatatccgtattcatatcagcacaagggaccatcaaagtgtaggctggagctgcttc

SEQ ID NO: 157 - DNA, 20 bp, Synthetic construct
  source 1..20: mol_type = other DNA; note = Cat-midF oligomer
cgacgatttccggcagtttc

SEQ ID NO: 158 - DNA, 20 bp, Synthetic construct
  source 1..20: mol_type = other DNA; note = Cat-midR oligomer
gccgacatggaagccatcac

SEQ ID NO: 159 - DNA, 20 bp, Synthetic construct
  source 1..20: mol_type = other DNA; note = Kan-midF oligomer
cctgatgatgcgtggttact

SEQ ID NO: 160 - DNA, 20 bp, Synthetic construct
  source 1..20: mol_type = other DNA; note = Kan-midR oligomer
aatccggtgagaatggcaag

SEQ ID NO: 161 - DNA, 1310 bp, Shigella sonnei
  source 1..1310: mol_type = genomic DNA; note = IS629
tgaaccgccccgggaatcctggagactaaacttcctgagaaagaggtaaacaggatgactaaaaatactcgtttttcccccgaagtccgtcaacgggcagtccgtatggttctggaaagtcagggcgaatatgactcacaatgggcgacaatttgttccattgctccaaagattggctgtacgccggagactctgcgtgtccgggttcgccagcatgagcgggataccgggggcggtgatggagggctcaccaccgctgaacgtcagcgtctgaaagagctggagcgtgaaaatcgtgaactgcgccgcagtaacgatatccttcgccaggcttccgcttattttgcgaaggcggagtttgaccgcctctggaaaaaatgatgccactgctggataagctgcgtgagcagtacggggtcggaccgctatgcagcgaactgcatattgccccgtcaacgtattaccactgtcagcaacagcgacatcatccggataaacgcagtgcccgtgcgcagcgcgatgactggctgaagaaagagatacagcgcgtatacgatgaaaatcacaaggtatacggtgtgcgtaaagtctggcgtcagttgttacgggaaggtatcagagtggccagatgcactgtggcacgtctcatggcggttatgggacttgccggtgttctccggggtaaaaaggtccgtacgaccatcagccggaaagccgttgccgcaggcgaccgcgtaaaccgtcagttcgtggcagaacgacctgaccagctgtgggtggctgattttacttacgtcagcacatggcagggcttcgtctatgtggcgttcatcattgatgtgtttgccggatacatcgtggggtggcgggtctcatcgtccatggaaacgacattcgtgctggatgcactggagcaggcgttatgggcccgtcgaccgtccggcacggtccatcacagtgataaaggttctcagtatgtatcgctggcctacacacagcggcttaaggaagccggattactggcatcaacaggaagtacaggcgactcgtatgacaacgcgatggcggagagcatcaatggtctttacaaagcgaaggtaatacaccgtaagagctggaaaaaccgtgcagaagtggaactggccacactcacgtgggtggactggtataacaatcgacgattgctggaaaggctgggccatactcctccggcagaagcagaaaaagcttattatgcttccatcggaaacgatgatctggcagcctgagttcacagataaaacactctccaggaaacccggggcggttca

SEQ ID NO: 162 - DNA, 1329 bp, Escherichia coli
  source 1..1329: mol_type = genomic DNA; note = IS10
ctgatgaatcccctaatgattttggtaaaaatcattaagttaaggtggatacacatcttgtcatatgatcaaatggtttcgcgaaaaatcaataatcagacaacaagatgtgcgaactcgatattttacacgactctctttaccaattctgccccgaattacacttaaaacgactcaacagcttaacgttggcttgccacgcattacttgactgtaaaactctcactcttaccgaacttggccgtaacctgccaaccaaagcgagaacaaaacataacatcaaacgaatcgaccgattgttaggtaatcgtcacctccacaaagagcgactcgctgtataccgttggcatgctagctttatctgttcgggcaatacgatgcccattgtacttgttgactggtctgatattcgtgagcaaaaacgacttatggtattgcgagcttcagtcgcactacacggtcgttctgttactctttatgagaaagcgttcccgctttcagagcaatgttcaaagaaagctcatgaccaatttctagccgaccttgcgagcattctaccgagtaacaccacaccgctcattgtcagtgatgctggctttaaagtgccatggtataaatccgttgagaagctgggttggtactggttaagtcgagtaagaggaaaagtacaatatgcagacctaggagcggaaaactggaaacctatcagcaacttacatgatatgtcatctagtcactcaaagactttaggctataagaggctgactaaaagcaatccaatctcatgccaaattctattgtataaatctcgctctaaaggccgaaaaaatcagcgctcgacacggactcattgtcaccacccgtcacctaaaatctactcagcgtcggcaaaggagccatgggttctagcaactaacttacctgttgaaattcgaacacccaaacaacttgttaatatctattcgaagcgaatgcagattgaagaaaccttccgagacttgaaaagtcctgcctacggactaggcctacgccatagccgaacgagcagctcagagcgttttgatatcatgctgctaatcgccctgatgcttcaactaacatgttggcttgcgggcgttcatgctcagaaacaaggttgggacaagcacttccaggctaacacagtcagaaatcgaaacgtactctcaacagttcgcttaggcatggaagttttgcggcattctggctacacaataacaagggaagacttactcgtggctgcaaccctactagctcaaaatttattcacacatggttacgctttggggaaattatgaggggatctctcag

SEQ ID NO: 163 - DNA, 1534 bp, Escherichia coli
  source 1..1534: mol_type = genomic DNA; note = IS50
ctgactcttatacacaagtagcgtcctgaacggaacctttcccgttttccaggatctgatcttccatgtgacctcctaacatggtaacgttcatgataacttctgctcttcatcgtgcggccgactgggctaaatctgtgttctcttcggcggcgctgggtgatcctcgccgtactgcccgcttggttaacgtcgccgcccaattggcaaaatattctggtaaatcaataaccatctcatcagagggtagtgaagccatgcaggaaggcgcttaccgatttatccgcaatcccaacgtttctgccgaggcgatcagaaaggctggcgccatgcaaacagtcaagttggctcaggagtttcccgaactgctggccattgaggacaccacctctttgagttatcgccaccaggtcgccgaagagcttggcaagctgggctctattcaggataaatcccgcggatggtgggttcactccgttctcttgctcgaggccaccacattccgcaccgtaggattactgcatcaggagtggtggatgcgcccggatgaccctgccgatgcggatgaaaaggagagtggcaaatggctggcagcggccgcaactagccggttacgcatgggcagcatgatgagcaacgtgattgcggtctgtgaccgcgaagccgatattcatgcttatctgcaggacaaactggcgcataacgagcgcttcgtggtgcgctccaagcacccacgcaaggacgtagagtctgggttgtatctgtacgaccatctgaagaaccaaccggagttgggtggctatcagatcagcattccgcaaaagggcgtggtggataaacgcggtaaacgtaaaaatcgaccagcccgcaaggcgagcttgagcctgcgcagtgggcgcatcacgctaaaacaggggaatatcacgctcaacgcggtgctggccgaggagattaacccgcccaagggtgagaccccgttgaaatggttgttgctgaccagcgaaccggtcgagtcgctagcccaagccttgcgcgtcatcgacatttatacccatcgctggcggatcgaggagttccataaggcatggaaaaccggagcaggagccgagaggcaacgcatggaggagccggataatctggagcggatggtctcgatcctctcgtttgttgcggtcaggctgttacagctcagagaaagcttcacgctgccgcaagcactcagggcgcaagggctgctaaaggaagcggaacacgtagaaagccagtccgcagaaacggtgctgaccccggatgaatgtcagctactgggctatctggacaagggaaaacgcaagcgcaaagagaaagcaggtagcttgcagtgggcttacatggcgatagctagactgggcggttttatggacagcaagcgaaccggaattgccagctggggcgccctctgggaaggttgggaagccctgcaaagtaaactggatggctttcttgccgccaaggatctgatggcgcaggggatcaagatctgatcaagagacag

SEQ ID NO: 164 - DNA, 791 bp, Staphylococcus aureus
  source 1..791: mol_type = genomic DNA; note = IS257
ggttctgttgcaaagttgaatttatagtataattttaacaaaaaggagtcttctgtatgaactatttcagatataaacaatttaacaaggatgttatcactgtagccgttggctactatctaagatatgcattgagttatcgtgatatatctgaaatattaagggaacgtggtgtaaacgttcatcattcaacagtctaccgttgggttcaagaatatgccccaattttgtatcaaatttggaagaaaaagcataaaaaagcttattacaaatggcgtattgatgagacgtacatcaaaataaaaggaaaatggagctatttatatcgtgccattgatgcagagggacatacattagatatttggttgcgtaagcaacgagataatcattcagcatatgcgtttatcaaacgtctcattaaacaatttggtaaacctcaaaaggtaattacagatcaggcaccttcaacgaaagtagcaatagctaaagtaattaaagcttttaaacttaaacctgactgtcattgtacatcgaaatatctgaataacctcattgagcaagatcaccgtcatattaaagtaagaaagacaagatatcaaagtatcaatacggcaaaaaatacactcaaaggcattgaatgtatttacgctctatataaaaagaaccgcagatctcttcagatctacggattttcgccatgccacgaaattagggatatgttagccagttaagggaacaacgacatgataaaatggtagttagctatatttttctaactttgcaacagaacc

SEQ ID NO: 165 - DNA, 1648 bp, Escherichia coli
  source 1..1648: mol_type = genomic DNA; note = IS15
ggcactgttgcaaatagtcggtggtgataaacttatcatccccttttgctgatggagctgcacatgaacccattcaaaggccggcattttcagcgtgacatcattctgtgggccgtacgctggtactgcaaatacggcatcagttaccgtgagctgcaggagatgctggctgaacgcggagtgaatgtcgatcactccacgatttaccgctgggttcagcgttatgcgcctgaaatggaaaaacggctgcgctggtactggcgtaacccttccgatctttgcccgtggcacatggatgaaacctacgtgaaggtcaatggccgctgggcgtatctgtaccgggccgtcgacagccggggccgcactgtcgatttttatctctcctcccgtcgtaacagcaaagctgcataccggtttctgggtaaaatcctcaacaacgtgaagaagtggcagatcccgcgattcatcaacacggataaagcgcccgcctatggtcgcgcgcttgctctgctcaaacgcgaaggccggtgcccgtctgacgttgaacaccgacagattaagtaccggaacaacgtgattgaatgcgatcatggcaaactgaaacggataatcggcgccacgctgggatttaaatccatgaagacggcttacgcggcactgttgcaaatagtcggtggtgataaacttatcatccccttttgctgatggagctgcacatgaacccattcaaaggccggcattttcagcgtgacatcattctgtgggccgtacgctggtactgcaaatacggcatcagttaccgtgagctgcaggagatgctggctgaacgcggagtgaatgtcgatcactccacgatttaccgctgggttcagcgttatgcgcctgaaatggaaaaacggctgcgctggtactggcgtaacccttccgatctttgcccgtggcacatggatgaaacctacgtgaaggtcaatggccgctgggcgtatctgtaccgggccgtcgacagccggggccgcactgtcgatttttatctctcctcccgtcgtaacagcaaagctgcataccggtttctgggtaaaatcctcaacaacgtgaagaagtggcagatcccacgattcatcaacacggataaagcgcccgcctatggtcgcgcgcttgctctgctcaaacgcgaaggccggtgcccgtctgacgttgaacaccgacagattaagtaccggaacaacgtgattgaatgcgatcatggcaaactgaaacggataatcaacgccacgctgggatttaaatccatgaagacggcttacgccaccatcaaaggtattgaggtgatgcgtgcactacgcaaaggccaggcctcagcattttattatggtgatcccctgggcgaaatgcgcctggtaagcagagtttttgaaatgtaaggcctttgaataagacaaaaggctgcctcatcgctaactttgcaacagtgccgcttacgccaccatcaaaggtattgaggtgatgcgtgcactacgcaaaggccaggcctcagcattttattatggtgatcccctgggcgaaatgcgcctggtaagcagagtttttgaaacgtaaggcctttgaataagacaaaaggctgcctcatcgctaactttgcaacagtgcc

SEQ ID NO: 166 - DNA, 820 bp, Escherichia coli
  source 1..820: mol_type = genomic DNA; note = IS26
ggcactgttgcaaatagtcggtggtgataaacttatcatccccttttgctgatggagctgcacatgaacccattcaaaggccggcattttcagcgtgacatcattctgtgggccgtacgctggtactgcaaatacggcatcagttaccgtgagctgcaggagatgctggctgaacgcggagtgaatgtcgatcactccacgatttaccgctgggttcagcgttatgcgcctgaaatggaaaaacggctgcgctggtactggcgtaacccttccgatctttgcccgtggcacatggatgaaacctacgtgaaggtcaatggccgctgggcgtatctgtaccgggccgtcgacagccggggccgcactgtcgatttttatctctcctcccgtcgtaacagcaaagctgcataccggtttctgggtaaaatcctcaacaacgtgaagaagtggcagatcccgcgattcatcaacacggataaagcgcccgcctatggtcgcgcgcttgctctgctcaaacgcgaaggccggtgcccgtctgacgttgaacaccgacagattaagtaccggaacaacgtgattgaatgcgatcatggcaaactgaaacggataatcggcgccacgctgggatttaaatccatgaagacggcttacgccaccatcaaaggtattgaggtgatgcgtgcactacgcaaaggccaggcctcagcattttattatggtgatcccctgggcgaaatgcgcctggtaagcagagtttttgaaatgtaaggcctttgaataagacaaaaggctgcctcatcgctaactttgcaacagtgcc

SEQ ID NO: 167 - DNA, 3244 bp, Synthetic construct
  source 1..3244: mol_type = other DNA; note = Acatsac1 template, NCBI Genbank MF124798.1
gtgtaggctggagctgcttcgaagagacgtcaggtggcaaacgcaaaaagccccgagcggttaaactcagggctttatttttattaggcgaccacaggtttgcgtgcaatggaaatttcacactgctcaaccgaagtgtaatccttgttgtgattggttacatccagtttgcggtcaacatagtgataccctggcatcttcacaggcttctttgccttgtaagtagttttaaattcacacaaatagtgaccgcctccttctaacttcagagccataaagttgtttcctagcagcattccatctcgtgcaaagagacgctcagtgttgggttcccagccctgtgtcttcttctgcatgacaggtccattgggaggaaagttcaaaccagagaacttgacatggtagatgaaacagttgccttggatgctggaatcattgctgacagtacacactgcaccatcttcaaagttcatgatcctctcccatgtatagccctccgggaatgactgctttacatagtcagggatgtcttcagggtacttggtgaatggtatgcttccgtactgacactgtggtgataaaatatcccaagcaaatggcagaggtccgcccttggtgacagtgagctttaccgtctgctccccctcgtagggcttaccttttccatcgccttcgacctcaaagtagtgtccattgaccgtgcctgacatataaaccttgtaggtcatttgtttagcgatcacactcatctagtatttctcctctttctctagtaacagtactatgtgattataccagccccctcactacatgtcaagaataaactgccaaagctctagaagcggccgcgaattcgtttacagctagctcagtcctaggtattatgctagcgttgatcgggcacgtaagaggttccaactttcaccataatgaaataagatcactaccgggcgtattttttgagttatcgagattttcaggagctaaggaagctaaaatggagaaaaaaatcacgggatataccaccgttgatatatcccaatggcatcgtaaagaacattttgaggcatttcagtcagttgctcaatgtacctataaccagaccgttcagctggatattacggcctttttaaagaccgtaaagaaaaataagcacaagttttatccggcctttattcacattcttgcccgcctgatgaacgctcacccggagtttcgtatggccatgaaagacggtgagctggtgatctgggatagtgttcacccttgttacaccgttttccatgagcaaactgaaacgttttcgtccctctggagtgaataccacgacgatttccggcagtttctccacatatattcgcaagatgtggcgtgttacggtgaaaacctggcctatttccctaaagggtttattgagaatatgttttttgtctcagccaatccctgggtgagtttcaccagttttgatttaaacgtggccaatatggacaacttcttcgcccccgttttcacgatgggcaaatattatacgcaaggcgacaaggtgctgatgccgctggcgatccaggttcatcatgccgtttgtgatggcttccatgtcggccgcatgcttaatgaattacaacagtactgtgatgagtggcagggcggggcgtaataatactagaggagacatgaacgatgaacatcaaaaagtttgcaaaacaagcaacagtattaacctttactaccgcactgctggcaggaggcgcaactcaagcgtttgcgaaagaaacgaaccaaaagccatataaggaaacatacggcatttcccatattacacgccatgatatgctgcaaatccctgaacagcaaaaaaatgaaaaatatcaagttcctgagttcgattcgtccacaattaaaaatatctcttctgcaaaaggcctggacgtttgggacagctggccattacaaaacgctgacggcactgtcgcaaactatcacggctaccacatcgtctttgcattagccggagatcctaaaaatgcggatgacacatcgatttacatgttctatcaaaaagtcggcgaaacttctattgacagctggaaaaacgctggccgcgtctttaaagacagcgacaaattcgatgcaaatgattctatcctaaaagaccaaacacaagaatggtcaggttcagccacatttacatctgacggaaaaatccgtttattctacactgatttctccggtaaacattacggcaaacaaacactgacaactgcacaagttaacgtatcagcatcagacagctctttgaacatcaacggtgtagaggattataaatcaatctttgacggtgacggaaaaacgtatcaaaatgtacagcagttcatcgatgaaggcaactacagctcaggcgacaaccatacgctgagagatcctcactacgtagaagataaaggccacaaatacttagtatttgaagcaaacactggaactgaagatggctaccaaggcgaagaatctttatttaacaaagcatactatggcaaaagcacatcattcttccgtcaagaaagtcaaaaacttctgcaaagcgataaaaaacgcacggctgagttagcaaacggcgctctcggtatgattgagctaaacgatgattacacactgaaaaaagtgatgaaaccgctgattgcatctaacacagtaacagatgaaattgaacgcgcgaacgtctttaaaatgaacggcaaatggtacctgttcactgactcccgcggatcaaaaatgacgattgacggcattacgtctaacgatatttacatgcttggttatgtttctaattctttaactggcccatacaagccgctgaacaaaactggccttgtgttaaaaatggatcttgatcctaacgatgtaacctttacttactcacacttcgctgtacctcaagcgaaaggaaacaatgtcgtgattacaagctatatgacaaacagaggattctacgcagacaaacaatcaacgtttgcgccaagcttcctgctgaacatcaaaggcaagaaaacatctgttgtcaaagacagcatccttgaacaaggacaattaacagttaacaaataataaatttggcttggactcctgttgatagatccagtaatgacctcagaactccatctggatttgttcagaacgctcggttgccgccgggcgttttttattggtgagaatccaagcactaggaactaaggaggatattcatatg

SEQ ID NO: 168 - DNA, 3229 bp, Synthetic construct
  source 1..3229: mol_type = other DNA; note = Acatsac3 template, NCBI Genbank MF124799.1
gtgtaggctggagctgcttcgaagagacgtcaggtggcaaacgcaaaaagccccgagcggttaaactcagggctttatttttattaggcgaccacaggtttgcgtgcaatggaaatttcacactgctcaaccgaagtgtaatccttgttgtgattggttacatccagtttgcggtcaacatagtgataccctggcatcttcacaggcttctttgccttgtaagtagttttaaattcacacaaatagtgaccgcctccttctaacttcagagccataaagttgtttcctagcagcattccatctcgtgcaaagagacgctcagtgttgggttcccagccctgtgtcttcttctgcatgacaggtccattgggaggaaagttcaaaccagagaacttgacatggtagatgaaacagttgccttggatgctggaatcattgctgacagtacacactgcaccatcttcaaagttcatgatcctctcccatgtatagccctccgggaatgactgctttacatagtcagggatgtcttcagggtacttggtgaatggtatgcttccgtactgacactgtggtgataaaatatcccaagcaaatggcagaggtccgcccttggtgacagtgagctttaccgtctgctccccctcgtagggcttaccttttccatcgccttcgacctcaaagtagtgtccattgaccgtgcctgacatataaaccttgtaggtcatttgtttagcgatcacactcatctagtatttctcctctttctctagtaacagtactatgtgattataccagccccctcactacatgtcaagaataaactgccaaagctctagacatatgaatatcctccttagttcctagtgcttggattctcaccaataaaaaacgcccggcggcaaccgagcgttctgaacaaatccagatggagttctgaggtcattactggatctatcaacaggagtccaagccaaatttattatttgttaactgttaattgtccttgttcaaggatgctgtctttgacaacagatgttttcttgcctttgatgttcagcaggaagcttggcgcaaacgttgattgtttgtctgcgtagaatcctctgtttgtcatatagcttgtaatcacgacattgtttcctttcgcttgaggtacagcgaagtgtgagtaagtaaaggttacatcgttaggatcaagatccatttttaacacaaggccagttttgttcagcggcttgtatgggccagttaaagaattagaaacataaccaagcatgtaaatatcgttagacgtaatgccgtcaatcgtcatttttgatccgcgggagtcagtgaacaggtaccatttgccgttcattttaaagacgttcgcgcgttcaatttcatctgttactgtgttagatgcaatcagcggtttcatcacttttttcagtgtgtaatcatcgtttagctcaatcataccgagagcgccgtttgctaactcagccgtgcgttttttatcgctttgcagaagtttttgactttcttgacggaagaatgatgtgcttttgccatagtatgctttgttaaataaagattcttcgccttggtagccatcttcagttccagtgtttgcttcaaatactaagtatttgtggcctttatcttctacgtagtgaggatctctcagcgtatggttgtcgcctgagctgtagttgccttcatcgatgaactgctgtacattttgatacgtttttccgtcaccgtcaaagattgatttataatcctctacaccgttgatgttcaaagagctgtctgatgctgatacgttaacttgtgcagttgtcagtgtttgtttgccgtaatgtttaccggagaaatcagtgtagaataaacggatttttccgtcagatgtaaatgtggctgaacctgaccattcttgtgtttggtcttttaggatagaatcatttgcatcgaatttgtcgctgtctttaaagacgcggccagcgtttttccagctgtcaatagaagtttcgccgactttttgatagaacatgtaaatcgatgtgtcatccgcatttttaggatctccggctaatgcaaagacgatgtggtagccgtgatagtttgcgacagtgccgtcagcgttttgtaatggccagctgtcccaaacgtccaggccttttgcagaagagatatttttaattgtggacgaatcgaactcaggaacttgatatttttcatttttttgctgttcagggatttgcagcatatcatggcgtgtaatatgggaaatgccgtatgtttccttatatggcttttggttcgtttctttcgcaaacgcttgagttgcgcctcctgccagcagtgcggtagtaaaggttaatactgttgcttgttttgcaaactttttgatgttcatcgttcatgtctcctctagtattattacgccccgccctgccactcatcacagtactgttgtaattcattaagcatgcggccgacatggaagccatcacaaacggcatgatgaacctggatcgccagcggcatcagcaccttgtcgccttgcgtataatatttgcccatcgtgaaaacgggggcgaagaagttgtccatattggccacgtttaaatcaaaactggtgaaactcacccagggattggctgagacaaaaaacatattctcaataaaccctttagggaaataggccaggttttcaccgtaacacgccacatcttgcgaatatatgtggagaaactgccggaaatcgtcgtggtattcactccagagggacgaaaacgtttcagtttgctcatggaaaacggtgtaacaagggtgaacactatcccagatcaccagctcaccgtctttcatggccatacgaaactccgggtgagcgttcatcaggcgggcaagaatgtgaataaaggccggataaaacttgtgcttatttttctttacggtctttaaaaaggccgtaatatccagctgaacggtctggttataggtacattgagcaactgactgaaatgcctcaaaatgttctttacgatgccattgggatatatcaacggtggtatatcccgtgatttttttctccattttagcttccttagctcctgaaaatctcgataactcaaaaaatacgcccggtagtgatcttatttcattatggtgaaagttggaacctcttacgtgcccgatcaacgctagcataatacctaggactgagctagctgtaaac

SEQ ID NO: 169 - DNA, 3400 bp, Synthetic construct
  source 1..3400: mol_type = other DNA; note = Akansac1 template
gtgtaggctggagctgcttcgaagagacgtcaggtggcaaacgcaaaaagccccgagcggttaaactcagggctttatttttattaggcgaccacaggtttgcgtgcaatggaaatttcacactgctcaaccgaagtgtaatccttgttgtgattggttacatccagtttgcggtcaacatagtgataccctggcatcttcacaggcttctttgccttgtaagtagttttaaattcacacaaatagtgaccgcctccttctaacttcagagccataaagttgtttcctagcagcattccatctcgtgcaaagagacgctcagtgttgggttcccagccctgtgtcttcttctgcatgacaggtccattgggaggaaagttcaaaccagagaacttgacatggtagatgaaacagttgccttggatgctggaatcattgctgacagtacacactgcaccatcttcaaagttcatgatcctctcccatgtatagccctccgggaatgactgctttacatagtcagggatgtcttcagggtacttggtgaatggtatgcttccgtactgacactgtggtgataaaatatcccaagcaaatggcagaggtccgcccttggtgacagtgagctttaccgtctgctccccctcgtagggcttaccttttccatcgccttcgacctcaaagtagtgtccattgaccgtgcctgacatataaaccttgtaggtcatttgtttagcgatcacactcatctagtatttctcctctttctctagtaacagtactatgtgattataccagccccctcactacatgtcaagaataaactgccaaagctctagaagcggccgcgaattcgtttacagctagctcagtcctaggtattatgctagcgttgatcgggcacgtaagaggttccaactttcaccataatgaaataagatcactaccgggcgtattttttgagttatcgagattttcaggagctaaggaagctaaaatgagccatattcaacgggaaacgtcttgctcccgtccgcgcttaaactccaacatggacgctgatttatatgggtataaatgggctcgcgataatgtcgggcaatcaggtgcgacaatctatcgcttgtatgggaagcccgatgcgccagagttgtttctgaaacatggcaaaggtagcgttgccaatgatgttacagatgagatggtccgtctcaactggctgacggagtttatgcctctcccgaccatcaagcattttatccgtactcctgatgatgcgtggttactcaccaccgcgattcctgggaaaacagccttccaggtattagaagaatatcctgattcaggtgaaaatattgttgatgcgctggccgtgttcctgcgccggttacattcgattcctgtttgtaattgtccttttaacagcgatcgtgtatttcgtcttgctcaggcgcaatcacgcatgaataacggtttggttgatgcgagtgattttgatgacgagcgtaatggctggcctgttgaacaagtctggaaagaaatgcacaagctcttgccattctcaccggattcagtcgtcactcatggtgatttctcacttgataaccttatttttgacgaggggaaattaataggttgtattgatgttggacgggtcggaatcgcagaccgttaccaggaccttgccattctttggaactgcctcggtgagttttctccttcattacagaaacggctttttcaaaaatatggtattgataatcctgatatgaataaattgcagtttcatttgatgctcgatgagtttttctaataatactagaggagacatgaacgatgaacatcaaaaagtttgcaaaacaagcaacagtattaacctttactaccgcactgctggcaggaggcgcaactcaagcgtttgcgaaagaaacgaaccaaaagccatataaggaaacatacggcatttcccatattacacgccatgatatgctgcaaatccctgaacagcaaaaaaatgaaaaatatcaagttcctgagttcgattcgtccacaattaaaaatatctcttctgcaaaaggcctggacgtttgggacagctggccattacaaaacgctgacggcactgtcgcaaactatcacggctaccacatcgtctttgcattagccggagatcctaaaaatgcggatgacacatcgatttacatgttctatcaaaaagtcggcgaaacttctattgacagctggaaaaacgctggccgcgtctttaaagacagcgacaaattcgatgcaaatgattctatcctaaaagaccaaacacaagaatggtcaggttcagccacatttacatctgacggaaaaatccgtttattctacactgatttctccggtaaacattacggcaaacaaacactgacaactgcacaagttaacgtatcagcatcagacagctctttgaacatcaacggtgtagaggattataaatcaatctttgacggtgacggaaaaacgtatcaaaatgtacagcagttcatcgatgaaggcaactacagctcaggcgacaaccatacgctgagagatcctcactacgtagaagataaaggccacaaatacttagtatttgaagcaaacactggaactgaagatggctaccaaggcgaagaatctttatttaacaaagcatactatggcaaaagcacatcattcttccgtcaagaaagtcaaaaacttctgcaaagcgataaaaaacgcacggctgagttagcaaacggcgctctcggtatgattgagctaaacgatgattacacactgaaaaaagtgatgaaaccgctgattgcatctaacacagtaacagatgaaattgaacgcgcgaacgtctttaaaatgaacggcaaatggtacctgttcactgactcccgcggatcaaaaatgacgattgacggcattacgtctaacgatatttacatgcttggttatgtttctaattctttaactggcccatacaagccgctgaacaaaactggccttgtgttaaaaatggatcttgatcctaacgatgtaacctttacttactcacacttcgctgtacctcaagcgaaaggaaacaatgtcgtgattacaagctatatgacaaacagaggattctacgcagacaaacaatcaacgtttgcgccaagcttcctgctgaacatcaaaggcaagaaaacatctgttgtcaaagacagcatccttgaacaaggacaattaacagttaacaaataataaatttggcttggactcctgttgatagatccagtaatgacctcagaactccatctggatttgttcagaacgctcggttgccgccgggcgttttttattggtgagaatccaagcactaggaactaaggaggatattcatatg

SEQ ID NO: 170 - DNA, 3385 bp, Synthetic construct
  source 1..3385: mol_type = other DNA; note = Akansac3 template
gtgtaggctggagctgcttcgaagagacgtcaggtggcaaacgcaaaaagccccgagcggttaaactcagggctttatttttattaggcgaccacaggtttgcgtgcaatggaaatttcacactgctcaaccgaagtgtaatccttgttgtgattggttacatccagtttgcggtcaacatagtgataccctggcatcttcacaggcttctttgccttgtaagtagttttaaattcacacaaatagtgaccgcctccttctaacttcagagccataaagttgtttcctagcagcattccatctcgtgcaaagagacgctcagtgttgggttcccagccctgtgtcttcttctgcatgacaggtccattgggaggaaagttcaaaccagagaacttgacatggtagatgaaacagttgccttggatgctggaatcattgctgacagtacacactgcaccatcttcaaagttcatgatcctctcccatgtatagccctccgggaatgactgctttacatagtcagggatgtcttcagggtacttggtgaatggtatgcttccgtactgacactgtggtgataaaatatcccaagcaaatggcagaggtccgcccttggtgacagtgagctttaccgtctgctccccctcgtagggcttaccttttccatcgccttcgacctcaaagtagtgtccattgaccgtgcctgacatataaaccttgtaggtcatttgtttagcgatcacactcatctagtatttctcctctttctctagtaacagtactatgtgattataccagccccctcactacatgtcaagaataaactgccaaagctctagacatatgaatatcctccttagttcctagtgcttggattctcaccaataaaaaacgcccggcggcaaccgagcgttctgaacaaatccagatggagttctgaggtcattactggatctatcaacaggagtccaagccaaatttattatttgttaactgttaattgtccttgttcaaggatgctgtctttgacaacagatgttttcttgcctttgatgttcagcaggaagcttggcgcaaacgttgattgtttgtctgcgtagaatcctctgtttgtcatatagcttgtaatcacgacattgtttcctttcgcttgaggtacagcgaagtgtgagtaagtaaaggttacatcgttaggatcaagatccatttttaacacaaggccagttttgttcagcggcttgtatgggccagttaaagaattagaaacataaccaagcatgtaaatatcgttagacgtaatgccgtcaatcgtcatttttgatccgcgggagtcagtgaacaggtaccatttgccgttcattttaaagacgttcgcgcgttcaatttcatctgttactgtgttagatgcaatcagcggtttcatcacttttttcagtgtgtaatcatcgtttagctcaatcataccgagagcgccgtttgctaactcagccgtgcgttttttatcgctttgcagaagtttttgactttcttgacggaagaatgatgtgcttttgccatagtatgctttgttaaataaagattcttcgccttggtagccatcttcagttccagtgtttgcttcaaatactaagtatttgtggcctttatcttctacgtagtgaggatctctcagcgtatggttgtcgcctgagctgtagttgccttcatcgatgaactgctgtacattttgatacgtttttccgtcaccgtcaaagattgatttataatcctctacaccgttgatgttcaaagagctgtctgatgctgatacgttaacttgtgcagttgtcagtgtttgtttgccgtaatgtttaccggagaaatcagtgtagaataaacggatttttccgtcagatgtaaatgtggctgaacctgaccattcttgtgtttggtcttttaggatagaatcatttgcatcgaatttgtcgctgtctttaaagacgcggccagcgtttttccagctgtcaatagaagtttcgccgactttttgatagaacatgtaaatcgatgtgtcatccgcatttttaggatctccggctaatgcaaagacgatgtggtagccgtgatagtttgcgacagtgccgtcagcgttttgtaatggccagctgtcccaaacgtccaggccttttgcagaagagatatttttaattgtggacgaatcgaactcaggaacttgatatttttcatttttttgctgttcagggatttgcagcatatcatggcgtgtaatatgggaaatgccgtatgtttccttatatggcttttggttcgtttctttcgcaaacgcttgagttgcgcctcctgccagcagtgcggtagtaaaggttaatactgttgcttgttttgcaaactttttgatgttcatcgttcatgtctcctctagtattattagaaaaactcatcgagcatcaaatgaaactgcaatttattcatatcaggattatcaataccatatttttgaaaaagccgtttctgtaatgaaggagaaaactcaccgaggcagttccaaagaatggcaaggtcctggtaacggtctgcgattccgacccgtccaacatcaatacaacctattaatttcccctcgtcaaaaataaggttatcaagtgagaaatcaccatgagtgacgactgaatccggtgagaatggcaagagcttgtgcatttctttccagacttgttcaacaggccagccattacgctcgtcatcaaaatcactcgcatcaaccaaaccgttattcatgcgtgattgcgcctgagcaagacgaaatacacgatcgctgttaaaaggacaattacaaacaggaatcgaatgtaaccggcgcaggaacacggccagcgcatcaacaatattttcacctgaatcaggatattcttctaatacctggaaggctgttttcccaggaatcgcggtggtgagtaaccacgcatcatcaggagtacggataaaatgcttgatggtcgggagaggcataaactccgtcagccagttgagacggaccatctcatctgtaacatcattggcaacgctacctttgccatgtttcagaaacaactctggcgcatcgggcttcccatacaagcgatagattgtcgcacctgattgcccgacattatcgcgagcccatttatacccatataaatcagcgtccatgttggagtttaagcgcggacgggagcaagacgtttcccgttgaatatggctcattttagcttccttagctcctgaaaatctcgataactcaaaaaatacgcccggtagtgatcttatttcattatggtgaaagttggaacctcttacgtgcccgatcaacgctagcataatacctaggactgagctagctgtaaac

SEQ ID NO: 171 - DNA, 80 bp, Synthetic construct
  source 1..80: mol_type = other DNA; note = Fp1-STOP IS2A oligomer
cgccattgctgattattgtgccaggacgaataaacgcatacctattaattacctatcagggtgtaggctggagctgcttc

SEQ ID NO: 172 - DNA, 80 bp, Synthetic construct
  source 1..80: mol_type = other DNA; note = Rp1-STOP IS2A oligomer
gggtccggtagtgattggcgcaaactgcctgataggtaattaataggtatgcgtttattcgtgtaggctggagctgcttc

SEQ ID NO: 173 - DNA, 80 bp, Synthetic construct
  source 1..80: mol_type = other DNA; note = Fp1-STOP IS3A oligomer
tactgttgcgttgaccgaatctactgggtggggggctgattaataggtacaacctgtacggtgtaggctggagctgcttc

SEQ ID NO: 174 - DNA, 80 bp, Synthetic construct
  source 1..80: mol_type = other DNA; note = Rp1-STOP IS3A oligomer
cgccgttagttacggtgatagtattggcgtacaggttgtacctattaatcagccccccacgtgtaggctggagctgcttc

SEQ ID NO: 175 - DNA, 80 bp, Synthetic construct
  source 1..80: mol_type = other DNA; note = Fp1-STOP IS3C oligomer
tgcacaggacgttgccgcggtaacaggcgcaaccgtaatctaataggaccagcataaatcgtgtaggctggagctgcttc

SEQ ID NO: 176 - DNA, 80 bp, Synthetic construct
  source 1..80: mol_type = other DNA; note = Rp1-STOP IS3C oligomer
ctgcccgcgccattttagccgcagcctgatttatgctggtcctattagattacggttgcggtgtaggctggagctgcttc

SEQ ID NO: 177 - DNA, 80 bp, Synthetic construct
  source 1..80: mol_type = other DNA; note = Fp1-STOP IS5B oligomer
gacctacagcaacgatgtcatcagtgcttacaccgagtgccctattatttagtgaagtcagtgtaggctggagctgcttc

SEQ ID NO: 178 - DNA, 80 bp, Synthetic construct
  source 1..80: mol_type = other DNA; note = Rp1-STOP IS5B oligomer
ttacaaaatcaacctgcttgacaaaaatgacttcactaaataatagggcactcggtgtaagtgtaggctggagctgcttc

SEQ ID NO: 179 - DNA, 80 bp, Synthetic construct
  source 1..80: mol_type = other DNA; note = Fp1-STOP IS5Y oligomer
gactttctccggggattatctccgcgtaactgacaacaagtaatagggggaaaacgcacggtgtaggctggagctgcttc

SEQ ID NO: 180 - DNA, 80 bp, Synthetic construct
  source 1..80: mol_type = other DNA; note = Rp1-STOP IS5Y oligomer
gaccgtcatcacttccggtcagcacgtcgtgcgttttccccctattacttgttgtcagttgtgtaggctggagctgcttc

SEQ ID NO: 181 - DNA, 80 bp, Synthetic construct
  source 1..80: mol_type = other DNA; note = Fp1-STOP IS2D oligomer
gcaggatattgacagttttgaacatcatgggacaagaacctaataggccagaacttacttgtgtaggctggagctgcttc

SEQ ID NO: 182 - DNA, 80 bp, Synthetic construct
  source 1..80: mol_type = other DNA; note = Rp1-STOP IS2D oligomer
taacaattttcgcaccggaatcagcataagtaagttctggcctattaggttcttgtcccagtgtaggctggagctgcttc

SEQ ID NO: 183 - DNA, 80 bp, Synthetic construct
  source 1..80: mol_type = other DNA; note = Fp1-STOP IS1H oligomer
gtattacagcggcgatctctgccgtatggatgaggctggctaataggtatataaaaattagtgtaggctggagctgcttc

SEQ ID NO: 184 - DNA, 80 bp, Synthetic construct
  source 1..80: mol_type = other DNA; note = Rp1-STOP IS1H oligomer
ggacaataatatcttttttgcgtccggtaatttttatatacctattagccagcctcatccgtgtaggctggagctgcttc

SEQ ID NO: 185 - DNA, 80 bp, Synthetic construct
  source 1..80: mol_type = other DNA; note = Fp1-STOP IS2F oligomer
caactccttggcaggccgtaaacaaatccgcattcgtggctaatagggaagcatcctcccgtgtaggctggagctgcttc

SEQ ID NO: 186 - DNA, 80 bp, Synthetic construct
  source 1..80: mol_type = other DNA; note = Rp1-STOP IS2F oligomer
cctgaccatcaatgagaattaaaacacgggaggatgcttccctattagccacgaatgcgggtgtaggctggagctgcttc

SEQ ID NO: 187 - DNA, 80 bp, Synthetic construct
  source 1..80: mol_type = other DNA; note = Fp1-STOP IS5I oligomer
cgtatcagaatagatactttctttaggaatttttgttttattcctattaaatccctaacagtgtaggctggagctgcttc

SEQ ID NO: 188 - DNA, 80 bp, Synthetic construct
  source 1..80: mol_type = other DNA; note = Rp1-STOP IS5I oligomer
tgtgctttctgattttattgtgtcatttatgttagggatttaataggaataaaacaaaaagtgtaggctggagctgcttc

SEQ ID NO: 189 - DNA, 80 bp, Synthetic construct
  source 1..80: mol_type = other DNA; note = Fp1-STOP IS3E oligomer
cggcgataagcattgtcgtacttccgctgtcgagaataaccctattaggtcatcccttcggtgtaggctggagctgcttc

SEQ ID NO: 190 - DNA, 80 bp, Synthetic construct
  source 1..80: mol_type = other DNA; note = Rp1-STOP IS3E oligomer
agcgcaggcggcagtcaaaatgatccacgaagggatgacctaatagggttattctcgacagtgtaggctggagctgcttc

SEQ ID NO: 191 - DNA, 80 bp, Synthetic construct
  source 1..80: mol_type = other DNA; note = Fp1-STOP IS5K oligomer
tcaccatactcaacagttgatgccaatgctatgggtgaatacctattataacgctgtagcgtgtaggctggagctgcttc

SEQ ID NO: 192 - DNA, 80 bp, Synthetic construct
  source 1..80: mol_type = other DNA; note = Rp1-STOP IS5K oligomer
ttgtcgttccgcaatatctgttctggtggctacagcgttataataggtattcacccataggtgtaggctggagctgcttc

SEQ ID NO: 193 - DNA, 80 bp, Synthetic construct
  source 1..80: mol_type = other DNA; note = Fp1-STOP IS2I oligomer
cgaattgattaaaaatatttattgttcattatccgttatctaataggatcattggttgtggtgtaggctggagctgcttc

SEQ ID NO: 194 - DNA, 80 bp, Synthetic construct
  source 1..80: mol_type = other DNA; note = Rp1-STOP IS2I oligomer
tgttgaattcaacggcataagctgacgcacaaccaatgatcctattagataacggataatgtgtaggctggagctgcttc

SEQ ID NO: 195 - DNA, 80 bp, Synthetic construct
  source 1..80: mol_type = other DNA; note = Fp1-STOP IS5R oligomer
aaatgacaatccgggcagcacaggaacagcatcaattagttaataggacttcccccaatagtgtaggctggagctgcttc

SEQ ID NO: 196 - DNA, 80 bp, Synthetic construct
  source 1..80: mol_type = other DNA; note = Rp1-STOP IS5R oligomer
gaccattttgcataaacaccagccaattattgggggaagtcctattaactaattgatgctgtgtaggctggagctgcttc

SEQ ID NO: 197 - DNA, 80 bp, Synthetic construct
  source 1..80: mol_type = other DNA; note = Fp1-STOP IS1E oligomer
cggggattatagcatttcaatatttacttatgacattaaataataggagtaacttttttggtgtaggctggagctgcttc

SEQ ID NO: 198 - DNA, 80 bp, Synthetic construct
  source 1..80: mol_type = other DNA; note = Rp1-STOP IS1E oligomer
tttctgtgccaatattatctctaatttcaaaaaagttactcctattatttaatgtcataagtgtaggctggagctgcttc

SEQ ID NO: 199 - DNA, 80 bp, Synthetic construct
  source 1..80: mol_type = other DNA; note = Fp1-STOP IS5T oligomer
cgaagatctacttaatataaatttcactgacgcaaatttataataggggtgacactatttgtgtaggctggagctgcttc

SEQ ID NO: 200 - DNA, 80 bp, Synthetic construct
  source 1..80: mol_type = other DNA; note = Rp1-STOP IS5T oligomer
tgggggtagggtgttctttatgtaaaaaaatagtgtcacccctattataaatttgcgtcagtgtaggctggagctgcttc

SEQ ID NO: 201 - DNA, 4641652 bp, Escherichia coli (residues 1-2,320,826 of 4,641,652)
  source 1..4641652: mol_type = genomic DNA; note = U00096.3, strain K-12, substrain MG1655, complete genome
agcttttcattctgactgcaacgggcaatatgtctctgtgtggattaaaaaaagagtgtctgatagcagcttctgaactggttacctgccgtgagtaaattaaaattttattgacttaggtcactaaatactttaaccaatataggcatagcgcacagacagataaaaattacagagtacacaacatccatgaaacgcattagcaccaccattaccaccaccatcaccattaccacaggtaacggtgcgggctgacgcgtacaggaaacacagaaaaaagcccgcacctgacagtgcgggctttttttttcgaccaaaggtaacgaggtaacaaccatgcgagtgttgaagttcggcggtacatcagtggcaaatgcagaacgttttctgcgtgttgccgatattctggaaagcaatgccaggcaggggcaggtggccaccgtcctctctgcccccgccaaaatcaccaaccacctggtggcgatgattgaaaaaaccattagcggccaggatgctttacccaatatcagcgatgccgaacgtatttttgccgaacttttgacgggactcgccgccgcccagccggggttcccgctggcgcaattgaaaactttcgtcgatcaggaatttgcccaaataaaacatgtcctgcatggcattagtttgttggggcagtgcccggatagcatcaacgctgcgctgatttgccgtggcgagaaaatgtcgatcgccattatggccggcgtattagaagcgcgcggtcacaacgttactgttatcgatccggtcgaaaaactgctggcagtggggcattacctcgaatctaccgtcgatattgctgagtccacccgccgtattgcggcaagccgcattccggctgatcacatggtgctgatggcaggtttcaccgccggtaatgaaaaaggcgaactggtggtgcttggacgcaacggttccgactactctgctgcggtgctggctgcctgtttacgcgccgattgttgcgagatttggacggacgttgacggggtctatacctgcgacccgcgtcaggtgcccgatgcgaggttgttgaagtcgatgtcctaccaggaagcgatggagctttcctacttcggcgctaaagttcttcacccccgcaccattacccccatcgcccagttccagatcccttgcctgattaaaaataccggaaatcctcaagcaccaggtacgctcattggtgccagccgtgatgaagacgaattaccggtcaagggcatttccaatctgaataacatggcaatgttcagcgtttctggtccggggatgaaagggatggtcggcatggcggcgcgcgtctttgcagcgatgtcacgcgcccgtatttccgtggtgctgattacgcaatcatcttccgaatacagcatcagtttctgcgttccacaaagcgactgtgtgcgagctgaacgggcaatgcaggaagagttctacctggaactgaaagaaggcttactggagccgctggcagtgacggaacggctggccattatctcggtggtaggtgatggtatgcgcaccttgcgtgggatctcggcgaaattctttgccgcactggcccgcgccaatatcaacattgtcgccattgctcagggatcttctgaacgctcaatctctgtcgtggtaaataacgatgatgcgaccactggcgtgcgcgttactcatcagatgctgttcaataccgatcaggttatcgaagtgtttgtgattggcgtcggtggcgttggcggtgcgctgctggagcaactgaagcgtcagcaaagctggctgaagaataaacatatcgacttacgtgtctgcggtgttgccaactcgaaggctctgctcaccaatgtacatggccttaatctggaaaactggcaggaagaactggcgcaagccaaagagccgtttaatctcgggcgcttaattcgcctcgtgaaagaatatcatctgctgaacccggtcattgttgactgcacttccagccaggcagtggcggatcaatatgccgacttcctgcgcgaaggtttccacgttgtcacgccgaacaaaaaggccaacacctcgtcgatggattactaccatcagttgcgttatgcggcggaaaaatcgcggcgtaaattcctctatgacaccaacgttggggctggattaccggttattgagaacctgcaaaatctgctcaatgcaggtgatgaattgatgaagttctccggcattctttctggttcgctttcttatatcttcggcaagttagacgaaggcatgagtttctccgaggcgaccacgctggcgcgggaaatgggttataccgaaccggacccgcgagatgatctttctggtatggatgtggcgcgtaaactattgattctcgctcgtgaaacgggacgtgaactggagctggcggatattgaaattgaacctgtgctgcccgcagagtttaacgccgagggtgatgttgccgcttttatggcgaatctgtcacaactcgacgatctctttgccgcgcgcgtggcgaaggcccgtgatgaaggaaaagttttgcgctatgttggcaatattgatgaagatggcgtctgccgcgtgaagattgccgaagtggatggtaatgatccgctgttcaaagtgaaaaatggcgaaaacgccctggccttctatagccactattatcagccgctgccgttggtactgcgcggatatggtgcgggcaatgacgttacagctgccggtgtctttgctgatctgctacgtaccctctcatggaagttaggagtctgacatggttaaagtttatgccccggcttccagtgccaatatgagcgtcgggtttgatgtgctcggggcggcggtgacacctgttgatggtgcattgctcggagatgtagtcacggttgaggcggcagagacattcagtctcaacaacctcggacgctttgccgataagctgccgtcagaaccacgggaaaatatcgtttatcagtgctgggagcgtttttgccaggaactgggtaagcaaattccagtggcgatgaccctggaaaagaatatgccgatcggttcgggcttaggctccagtgcctgttcggtggtcgcggcgctgatggcgatgaatgaacactgcggcaagccgcttaatgacactcgtttgctggctttgatgggcgagctggaaggccgtatctccggcagcattcattacgacaacgtggcaccgtgttttctcggtggtatgcagttgatgatcgaagaaaacgacatcatcagccagcaagtgccagggtttgatgagtggctgtgggtgctggcgtatccggggattaaagtctcgacggcagaagccagggctattttaccggcgcagtatcgccgccaggattgcattgcgcacgggcgacatctggcaggcttcattcacgcctgctattcccgtcagcctgagcttgccgcgaagctgatgaaagatgttatcgctgaaccctaccgtgaacggttactgccaggcttccggcaggcgcggcaggcggtcgcggaaatcggcgcggtagcgagcggtatctccggctccggcccgaccttgttcgctctgtgtgacaagccggaaaccgcccagcgcgttgccgactggttgggtaagaactacctgcaaaatcaggaaggttttgttcatatttgccggctggatacggcgggcgcacgagtactggaaaactaaatgaaactctacaatctgaaagatcacaacgagcaggtcagctttgcgcaagccgtaacccaggggttgggcaaaaatcaggggctgttttttccgcacgacctgccggaattcagcctgactgaaattgatgagatgctgaagctggattttgtcacccgcagtgcgaagatcctctcggcgtttattggtgatgaaatcccacaggaaatcctggaagagcgcgtgcgcgcggcgtttgccttcccggctccggtcgccaatgttgaaagcgatgtcggttgtctggaattgttccacgggccaacgctggcatttaaagatttcggcggtcgctttatggcacaaatgctgacccatattgcgggtgataagccagtgaccattctgaccgcgacctccggtgataccggagcggcagtggctcatgctttctacggtttaccgaatgtgaaagtggttatcctctatccacgaggcaaaatcagtccactgcaagaaaaactgttctgtacattgggcggcaatatcgaaactgttgccatcgacggcgatttcgatgcctgtcaggcgctggtgaagcaggcgtttgatgatgaagaactgaaagtggcgctagggttaaactcggctaactcgattaacatcagccgtttgctggcgcagatttgctactactttgaagctgttgcgcagctgccgcaggagacgcgcaaccagctggttgtctcggtgccaagcggaaacttcggcgatttgacggcgggtctgctggcgaagtcactcggtctgccggtgaaacgttttattgctgcgaccaacgtgaacgataccgtgccacgtttcctgcacgacggtcagtggtcacccaaagcgactcaggcgacgttatccaacgcgatggacgtgagtcagccgaacaactggccgcgtgtggaagagttgttccgccgcaaaatctggcaactgaaagagctgggttatgcagccgtggatgatgaaaccacgcaacagacaatgcgtgagttaaaagaactgggctacacttcggagccgcacgctgccgtagcttatcgtgcgctgcgtgatcagttgaatccaggcgaatatggcttgttcctcggcaccgcgcatccggcgaaatttaaagagagcgtggaagcgattctcggtgaaacgttggatctgccaaaagagctggcagaacgtgctgatttacccttgctttcacataatctgcccgccgattttgctgcgttgcgtaaattgatgatgaatcatcagtaaaatctattcattatctcaatcaggccgggtttgcttttatgcagcccggcttttttatgaagaaattatggagaaaaatgacagggaaaaaggagaaattctcaataaatgcggtaacttagagattaggattgcggagaataacaaccgccgttctcatcgagtaatctccggatatcgacccataacgggcaatgataaaaggagtaacctgtgaaaaagatgcaatctatcgtactcgcactttccctggttctggtcgctcccatggcagcacaggctgcggaaattacgttagtcccgtcagtaaaattacagataggcgatcgtgataatcgtggctattactgggatggaggtcactggcgcgaccacggctggtggaaacaacattatgaatggcgaggcaatcgctggcacctacacggaccgccgccaccgccgcgccaccataagaaagctcctcatgatcatcacggcggtcatggtccaggcaaacatcaccgctaaatgacaaatgccgggtaacaatccggcattcagcgcctgatgcgacgctggcgcgtcttatcaggcctacgttaattctgcaatatattgaatctgcatgcttttgtaggcaggataaggcgttcacgccgcatccggcattgactgcaaacttaacgctgctcgtagcgtttaaacaccagttcgccattgctggaggaatcttcatcaaagaagtaaccttcgctattaaaaccagtcagttgctctggtttggtcagccgattttcaataatgaaacgactcatcagaccgcgtgctttcttagcgtagaagctgatgatcttaaatttgccgttcttctcatcgaggaacaccggcttgataatctcggcattcaatttcttcggcttcaccgatttaaaatactcatctgacgccagattaatcaccacattatcgccttgtgctgcgagcgcctcgttcagcttgttggtgatgatatctccccagaattgatacagatctttccctcgggcattctcaagacggatccccatttccagacgataaggctgcattaaatcgagcgggcggagtacgccatacaagccggaaagcattcgcaaatgctgttgggcaaaatcgaaatcgtcttcgctgaaggtttcggcctgcaagccggtgtagacatcacctttaaacgccagaatcgcctggcgggcattcgccggcgtgaaatctggctgccagtcatgaaagcgagcggcgttgatacccgccagtttgtcgctgatgcgcatcagcgtgctaatctgcggaggcgtcagtttccgcgcctcatggatcaactgctgggaattgtctaacagctccggcagcgtatagcgcgtggtggtcaacgggctttggtaatcaagcgttttcgcaggtgaaataagaatcagcatatccagtccttgcaggaaatttatgccgactttagcaaaaaatgagaatgagttgatcgatagttgtgattactcctgcgaaacatcatcccacgcgtccggagaaagctggcgaccgatatccggataacgcaatggatcaaacaccgggcgcacgccgagtttacgctggcgtagataatcactggcaatggtatgaaccacaggcgagagcagtaaaatggcggtcaaattggtaatagccatgcaggccattatgatatctgccagttgccacatcagcggaaggcttagcaaggtgccgccgatgaccgttgcgaaggtgcagatccgcaaacaccagatcgctttagggttgttcaggcgtaaaaagaagagattgttttcggcataaatgtagttggcaacgatggagctgaaggcaaacagaataaccacaagggtaacaaactcagcaccccaggaacccattagcacccgcatcgccttctggataagctgaataccttccagcggcatgtaggttgtgccgttacccgccagtaatatcagcatggcgcttgccgtacagatgaccagggtgtcgataaaaatgccaatcatctggacaatcccttgcgctgccggatgcggaggccaggacgccgctgccgctgccgcgtttggcgtcgaacccattcccgcctcattggaaaacatactgcgctgaaaaccgttagtaatcgcctggcttaaggtatatcccgccgcgccgcctgccgcttcctgccagccaaaagcactctcaaaaatagaccaaatgacgtggggaagttgcccgatattcattacgcaaattaccaggctggtcagtacccagattatcgccatcaacgggacaaagccctgcatgagccgggcgacgccatgaagaccgcgagtgattgccagcagagtaaagacagcgagaataatgcctgtcaccagcgggggaaaatcaaaagaaaaactcagggcgcgggcaacggcgttcgcttgaactccgctgaaaattatgccataggcgatgagcaaaaagacggcgaacagaacgcccatccagcgcatccccagcccgcgcgccatataccatgccggtccgccacgaaactgcccattgacgtcacgttctttataaagttgtgccagagaacattcggcaaacgaggtcgccatgccgataaacgcggcaacccacatccaaaagacggctccaggtccaccggcggtaatagccagcgcaacgccggccaggttgccgctacccacgcgcgccgcaagactggtacacaatgactgaaatgaggttaaaccgcctggctgtggatgaatgctatttttaagacttttgccaaactggcggatgtagcgaaactgcacaaatccggtgcgaaaagtgaaccaacaacctgcgccgaagagcaggtaaatcattaccgatccccaaaggacgctgttaatgaaggagaaaaaatctggcatgcatatccctcttattgccggtcgcgatgactttcctgtgtaaacgttaccaattgtttaagaagtatatacgctacgaggtacttgataacttctgcgtagcatacatgaggttttgtataaaaatggcgggcgatatcaacgcagtgtcagaaatccgaaacagtctcgcctggcgataaccgtcttgtcggcggttgcgctgacgttgcgtcgtgatatcatcagggcagaccggttacatccccctaacaagctgtttaaagagaaatactatcatgacggacaaattgacctcccttcgtcagtacaccaccgtagtggccgacactggggacatcgcggcaatgaagctgtatcaaccgcaggatgccacaaccaacccttctctcattcttaacgcagcgcagattccggaataccgtaagttgattgatgatgctgtcgcctgggcgaaacagcagagcaacgatcgcgcgcagcagatcgtggacgcgaccgacaaactggcagtaaatattggtctggaaatcctgaaactggttccgggccgtatctcaactgaagttgatgcgcgtctttcctatgacaccgaagcgtcaattgcgaaagcaaaacgcctgatcaaactctacaacgatgctggtattagcaacgatcgtattctgatcaaactggcttctacctggcagggtatccgtgctgcagaacagctggaaaaagaaggcatcaactgtaacctgaccctgctgttctccttcgctcaggctcgtgcttgtgcggaagcgggcgtgttcctgatctcgccgtttgttggccgtattcttgactggtacaaagcgaataccgataagaaagagtacgctccggcagaagatccgggcgtggtttctgtatctgaaatctaccagtactacaaagagcacggttatgaaaccgtggttatgggcgcaagcttccgtaacatcggcgaaattctggaactggcaggctgcgaccgtctgaccatcgcaccggcactgctgaaagagctggcggagagcgaaggggctatcgaacgtaaactgtcttacaccggcgaagtgaaagcgcgtccggcgcgtatcactgagtccgagttcctgtggcagcacaaccaggatccaatggcagtagataaactggcggaaggtatccgtaagtttgctattgaccaggaaaaactggaaaaaatgatcggcgatctgctgtaatcattcttagcgtgaccgggaagtcggtcacgctacctcttctgaagcctgtctgtcactcccttcgcagtgtatcattctgtttaacgagactgtttaaacggaaaaatcttgatgaatactttacgtattggcttagtttccatctctgatcgcgcatccagcggcgtttatcaggataaaggcatccctgcgctggaagaatggctgacatcggcgctaaccacgccgtttgaactggaaacccgcttaatccccgatgagcaggcgatcatcgagcaaacgttgtgtgagctggtggatgaaatgagttgccatctggtgctcaccacgggcggaactggcccggcgcgtcgtgacgtaacgcccgatgcgacgctggcagtagcggaccgcgagatgcctggctttggtgaacagatgcgccagatcagcctgcattttgtaccaactgcgatcctttcgcgtcaggtgggcgtgattcgcaaacaggcgctgatccttaacttacccggtcagccgaagtctattaaagagacgctggaaggtgtgaaggacgctgagggtaacgttgtggtacacggtatttttgccagcgtaccgtactgcattcagttgctggaagggccatacgttgaaacggcaccggaagtggttgcagcattcagaccgaagagtgcaagacgcgacgttagcgaataaaaaaatccccccgagcggggggatctcaaaacaattagtgggattcaccaatcggcagaacggtgcgaccaaactgctcgttcagtacttcacccatcgccagatagattgcgctggcaccgcagatcagcccaatccagccggcaaagtggatgattgcggcgttaccggcaatgttaccgatcgccagcagggcaaacagcacggtcaggctaaagaaaacgaattgcagaacgcgtgcgcctttcagcgtgccgaagaacataaacagcgtaaatacgccccacagacccaggtagacaccaaggaactgtgcatttggcgcatcggtcagacccagtttcggcatcagcagaatcgcaaccagcgtcagccagaaagaaccgtaagaggtgaatgcggttaaaccgaaagtgttgccttttttgtactccagcagaccagcaaaaatttgcgcgatgccgccgtagaaaatgcccatggcaagaataataccgtccagagcgaaataacccacgttgtgcaggttaagcagaatggtggtcatgccgaagcccatcaggcccagcggtgccggattagccaacttagtgttgcccataattcctcaaaaatcatcatcgaatgaatggtgaaataatttccctgaataactgtagtgttttcagggcgcggcataataatcagccagtggggcagtgtctacgatcttttgaggggaaaatgaaaattttccccggtttccggtatcagacctgagtggcgctaaccatccggcgcaggcaggcgatttgcagtacggctggaatcgtcacgcgataggcgctgccgctgaccgctttaaccccatttagtgccgcacctacagggcctcccagccccgcgccgcgcagcaaaccatgcccaagtacgctcattgctgcgtgggtgcgtaaaatgcgggtcagttggctggaaagcaaatgcgacacaccttttgccaataatttgtctttcatcagcagcggcagcagctcttccagctcattcaccctggcatcgaccgcgtgcagaaactcctgcttatgttcctcgtccattttcttccaggtattacgcagaaattgttccagtaactgttgctcaatttcaaacgtagacatctctttgtcggctttcagcttcaatcgctttgaaacatcgagcaaaatggcccgatacaatttaccgtgtccgcgcagtttgttggcgatactatcgccaccaaaatgctgtaattctccggcaatcagctgccagttgcggcgatgttgctcgggatgcccttccatcgatttaaacagttcgttgcgcatcagtacgctggagaggcgagttttgcctttttcattatgggtgagcaatcgggcgaaatttgccaactgttcctcactacaatgctgaagaaaatccagatctgaatcattcaggtaattaacattcattttttgtggcttctatattctggcgttagtcgtcgccgataattttcagcgtggccatatccgatgagttcaccgtatgacccgaaaaggtgatttttgagacgcagcgtttattgtcgttatcgctgttaatgttgatccagtcagtggtttgcccttcttttatttctgaaggaatattcaggctctgactggcgctacgggcggctttgaaataaaccgatgcaccgcttaactgtaaatcgccatggtcggcagagagttgtatgcgtttcacaatgcgacaaacaggaagtttcagcgccagatcgttggtttcgttacgcggcattgcaatggcgccgaggagtttatggtcgtttgcctgcgccgtgcagcacagcatcaggctaatcgccaggctggcggaaatcgtaaaaacggatttcataaggattctcttagtgggaagaggtagggggatgaatacccactagtttactgctgataaagagaagattcaggcacgtaatcttttctttttattacaattttttgatgaatgccttggctgcgattcattctttatatgaataaaattgctgtcaattttacgtcttgtcctgccatatcgcgaaatttctgcgcaaaagcacaaaaaatttttgcatctcccccttgatgacgtggtttacgaccccatttagtagtcaaccgcagtgagtgagtctgcaaaaaaatgaaattgggcagttgaaaccagacgtttcgcccctattacagactcacaaccacatgatgaccgaatatatagtggagacgtttagatgggtaaaataattggtatcgacctgggtactaccaactcttgtgtagcgattatggatggcaccactcctcgcgtgctggagaacgccgaaggcgatcgcaccacgccttctatcattgcctatacccaggatggtgaaactctagttggtcagccggctaaacgtcaggcagtgacgaacccgcaaaacactctgtttgcgattaaacgcctgattggtcgccgcttccaggacgaagaagtacagcgtgatgtttccatcatgccgttcaaaattattgctgctgataacggcgacgcatgggtcgaagttaaaggccagaaaatggcaccgccgcagatttctgctgaagtgctgaaaaaaatgaagaaaaccgctgaagattacctgggtgaaccggtaactgaagctgttatcaccgtaccggcatactttaacgatgctcagcgtcaggcaaccaaagacgcaggccgtatcgctggtctggaagtaaaacgtatcatcaacgaaccgaccgcagctgcgctggcttacggtctggacaaaggcactggcaaccgtactatcgcggtttatgacctgggtggtggtactttcgatatttctattatcgaaatcgacgaagttgacggcgaaaaaaccttcgaagttctggcaaccaacggtgatacccacctggggggtgaagacttcgacagccgtctgatcaactatctggttgaagaattcaagaaagatcagggcattgacctgcgcaacgatccgctggcaatgcagcgcctgaaagaagcggcagaaaaagcgaaaatcgaactgtcttccgctcagcagaccgacgttaacctgccatacatcactgcagacgcgaccggtccgaaacacatgaacatcaaagtgactcgtgcgaaactggaaagcctggttgaagatctggtaaaccgttccattgagccgctgaaagttgcactgcaggacgctggcctgtccgtatctgatatcgacgacgttatcctcgttggtggtcagactcgtatgccaatggttcagaagaaagttgctgagttctttggtaaagagccgcgtaaagacgttaacccggacgaagctgtagcaatcggtgctgctgttcagggtggtgttctgactggtgacgtaaaagacgtactgctgctggacgttaccccgctgtctctgggtatcgaaaccatgggcggtgtgatgacgacgctgatcgcgaaaaacaccactatcccgaccaagcacagccaggtgttctctaccgctgaagacaaccagtctgcggtaaccatccatgtgctgcagggtgaacgtaaacgtgcggctgataacaaatctctgggtcagttcaacctagatggtatcaacccggcaccgcgcggcatgccgcagatcgaagttaccttcgatatcgatgctgacggtatcctgcacgtttccgcgaaagataaaaacagcggtaaagagcagaagatcaccatcaaggcttcttctggtctgaacgaagatgaaatccagaaaatggtacgcgacgcagaagctaacgccgaagctgaccgtaagtttgaagagctggtacagactcgcaaccagggcgaccatctgctgcacagcacccgtaagcaggttgaagaagcaggcgacaaactgccggctgacgacaaaactgctatcgagtctgcgctgactgcactggaaactgctctgaaaggtgaagacaaagccgctatcgaagcgaaaatgcaggaactggcacaggtttcccagaaactgatggaaatcgcccagcagcaacatgcccagcagcagactgccggtgctgatgcttctgcaaacaacgcgaaagatgacgatgttgtcgacgctgaatttgaagaagtcaaagacaaaaaataatcgccctataaacgggtaattatactgacacgggcgaaggggaatttcctctccgcccgtgcattcatctaggggcaatttaaaaaagatggctaagcaagattattacgagattttaggcgtttccaaaacagcggaagagcgtgaaatcagaaaggcctacaaacgcctggccatgaaataccacccggaccgtaaccagggtgacaaagaggccgaggcgaaatttaaagagatcaaggaagcttatgaagttctgaccgactcgcaaaaacgtgcggcatacgatcagtatggtcatgctgcgtttgagcaaggtggcatgggcggcggcggttttggcggcggcgcagacttcagcgatatttttggtgacgttttcggcgatatttttggcggcggacgtggtcgtcaacgtgcggcgcgcggtgctgatttacgctataacatggagctcaccctcgaagaagctgtacgtggcgtgaccaaagagatccgcattccgactctggaagagtgtgacgtttgccacggtagcggtgcaaaaccaggtacacagccgcagacttgtccgacctgtcatggttctggtcaggtgcagatgcgccagggattcttcgctgtacagcagacctgtccacactgtcagggccgcggtacgctgatcaaagatccgtgcaacaaatgtcatggtcatggtcgtgttgagcgcagcaaaacgctgtccgttaaaatcccggcaggggtggacactggagaccgcatccgtcttgcgggcgaaggtgaagcgggcgagcatggcgcaccggcaggcgatctgtacgttcaggttcaggttaaacagcacccgattttcgagcgtgaaggcaacaacctgtattgcgaagtcccgatcaacttcgctatggcggcgctgggtggcgaaatcgaagtaccgacccttgatggtcgcgtcaaactgaaagtgcctggcgaaacccagaccggtaagctattccgtatgcgcggtaaaggcgtcaagtctgtccgcggtggcgcacagggtgatttgctgtgccgcgttgtcgtcgaaacaccggtaggcctgaacgaaaggcagaaacagctgctgcaagagctgcaagaaagcttcggtggcccaaccggcgagcacaacagcccgcgctcaaagagcttctttgatggtgtgaagaagttttttgacgacctgacccgctaacctccccaaaagcctgcccgtgggcaggcctgggtaaaaatagggtgcgttgaagatatgcgagcacctgtaaagtggcggggatcactcccataagcgctaacttaagggttgtggtattacgcctgatatgatttaacgtgccgatgaattactctcacgataactggtcagcaattctggcccatattggtaagcccgaagaactggatacttcggcacgtaatgccggggctctaacccgccgccgcgaaattcgtgatgctgcaactctgctacgtctggggctggcttacggccccggggggatgtcattacgtgaagtcactgcatgggctcagctccatgacgttgcaacattatctgacgtggctctcctgaagcggctgcggaatgccgccgactggtttggcatacttgccgcacaaacacttgctgtacgcgccgcagttacgggttgtacaagcggaaagagattgcgtcttgtcgatggaacagcaatcagtgcgcccgggggcggcagcgctgaatggcgactacatatgggatatgatcctcatacctgtcagttcactgattttgagctaaccgacagcagagacgctgaacggctggaccgatttgcgcaaacggcagacgagatacgcattgctgaccggggattcggttcgcgtcccgaatgtatccgctcacttgcttttggagaagctgattatatcgtccgggttcactggcgaggattgcgctggttaactgcagaaggaatgcgctttgacatgatgggttttctgcgcgggctggattgcggtaagaacggtgaaaccactgtaatgataggcaattcaggtaataaaaaagccggagctccctttccggcacgtctcattgccgtatcacttcctcccgaaaaagcattaatcagtaaaacccgactgctcagcgagaatcgtcgaaaaggacgagtagttcaggcggaaacgctggaagcagcgggccatgtgctattgctaacatcattaccggaagatgaatattcagcagagcaagtggctgattgttaccgtctgcgatggcaaattgaactggcttttaagcggctcaaaagtttgctgcacctggatgctttgcgtgcaaaggaacctgaactcgcgaaagcgtggatatttgctaatctactcgccgcatttttaattgacgacataatccagccatcgctggatttcccccccagaagtgccggatccgaaaagaagaactaactcgttgtggagaataacaaaaatggtcatctggagcttacaggtggccattcgtgggacagtatccctgacagcctacaaaacgcaattgaagaacgcgaggcatcgtcttaacgaggcaccgaggcgtcgcattcttcagatggttcaacccttaagttagcgcttatgggatcactccccgccgttgctcttactcggattcgtaagccgtgaaaacagcaacctccgtctggccagttcggatgtgaacctcacagaggtcttttctcgttaccagcgccgccactacggcggtgatacagatgacgatcagggcgacaatcatcgccttatgctgcttcattgctctcttctccttgaccttacggtcagtaagaggcactctacatgtgttcagcatataggaggcctcgggttgatggtaaaatatcactcggggcttttctctatctgccgttcagctaatgcctgagacagacagcctcaagcacccgccgctattatatcgctctctttaacccattttgttttatcgattctaatcctgaagacgcctcgcatttttgtggcgtaattttttaatgatttaattatttaactttaatttatctcttcatcgcaattattgacgacaagctggattatttttgaaatattggcctaacaagcatcgccgactgacaacaaattaattattacttttcctaattaatccctcaggaatcctcaccttaagctatgattatctaggcttagggtcactcgtgagcgcttacagccgtcaaaaacgcatctcaccgctgatggcgcaaattcttcaatagctcgtaaaaaacgaattattcctacactataatctgattttaacgatgattcgtgcggggtaaaatagtaaaaacgatctattcacctgaaagagaaataaaaagtgaaacatctgcatcgattctttagcagtgatgcctcgggaggcattattcttatcattgccgctatcctggcgatgattatggccaacagcggcgcaaccagtggatggtatcacgactttctggagacgccggttcagctccgggttggttcactcgaaatcaacaaaaacatgctgttatggataaatgacgcgctgatggcggtatttttcctgttagtcggtctggaagttaaacgtgaactgatgcaaggatcgctagccagcttacgccaggccgcatttccagttatcgccgctattggtgggatgattgtgccggcattactctatctggcttttaactatgccgatccgattacccgcgaagggtgggcgatcccggcggctactgacattgcttttgcacttggtgtactggcgctgttgggaagtcgtgttccgttagcgctgaagatctttttgatggctctggctattatcgacgatcttggggccatcattatcatcgcattgttctacactaatgacttatcgatggcctctcttggcgtcgcggctgtagcaattgcggtactcgcggtattgaatctgtgtggtgcacgccgcacgggcgtctatattcttgttggcgtggtgttgtggactgcggtgttgaaatcgggggttcacgcaactctggcgggggtaattgtcggcttctttattcctttgaaagagaagcatgggcgttctccagcgaagcgactggagcatgtgttgcacccgtgggtggcgtatctgattttgccgctgtttgcatttgctaatgctggcgtttcactgcaaggcgtcacgctggatggcttgacctccattctgccattggggatcatcgctggcttgctgattggcaaaccgctggggattagtctgttctgctggttggcgctgcgtttgaaactggcgcatctgcctgagggaacgacttatcagcaaattatggtggtggggatcctgtgcggtatcggttttactatgtctatctttattgccagcctggcctttggtagcgtagatccagaactgattaactgggcgaaactcggtatcctggtcggttctatctcttcggcggtaattggatacagctggttacgcgttcgtttgcgtccatcagtttgacaggacggtttaccggggagccataaacggctcccttttcattgttatcagggagagaaatgagcatgtctcatatcaattacaaccacttgtattacttctggcatgtctataaagaaggttccgtggttggcgcagcggaggcgctttatttaactccacaaaccattaccggacagattcgagcgctggaagagcgcctgcaaggcaaattatttaaacgcaagggacgtggtctcgaacccagcgagctgggagaactggtctatcgctatgccgataaaatgttcaccttaagccaggaaatgctggatattgtgaactatcgcaaagaatccaatttattgtttgacgttggcgtggctgatgcactttccaaacgcctggtcagtagcgtacttaacgccgcagtggtagaaggcgagcccattcatcttcgctgcttcgaatccacccacgaaatgctgctggagcaattaagtcagcataaactggatatgatcatttctgactgtccgatagactctacgcagcaggaaggcctgttctccgtgagaattggcgaatgtggcgtgagtttctggtgtacaaatccaccaccagaaaaaccgttcccggcttgtctggaagaacggcgacttttgattcctgggcgacgttcaatgttagggcgcaaattgcttaactggtttaactcccagggattaaacgtagaaatcctcggcgagtttgatgatgccgctttgatgaaagcttttggtgcgatgcacaatgcaatcttcgttgccccaacgctttatgcatatgacttttatgccgataaaactgtcgtagaaattggtcgcgtcgagaatgtgatggaagagtaccatgctatttttgctgagcggatgattcagcacccggcggtacagcgaatctgcaatacggattattctgcgctttttagtccagcggtgcgttaatcggcagctcccccaaagttaaggtgggggagatagattagttgtacattaccacgattttgactcggctcattatttgcccgcttgagacattgtttccatatgtacgcgggcgaataaatagaggaatctgattacttccttcatggggatgctgaaaagagtagtaattgctggtaatgactccaacttattgatagtgttttatgttcagataatgcccgatgactttgtcatgcagctccaccgattttgagaacgacagcgacttccgtcccagccgtgccaggtgctgcctcagattcaggttatgccgctcaattcgctgcgtatatcgcttgctgattacgtgcagctttcccttcaggcgggattcatacagcggccagccatccgtcatccatatcaccacgtcaaagggtgacagcaggctcataagacgccccagcgtcgccatagtgcgttcaccgaatacgtgcgcaacaaccgtcttccggagactgtcatacgcgtaaaacagccagcgctggcgcgatttagccccgacatagccccactgttcgtccatttccgcgcagacgatgacgtcactgcccggctgtatgcgcgaggttaccgactgcggcctgagttttttaagtgacgtaaaatcgtgttgaggccaacgcccataatgcgggctgttgcccggcatccaacgccattcatggccatatcaatgattttctggtgcgtaccgggttgagaagcggtgtaagtgaactgcagttgccatgttttacggcagtgagagcagagatagcgctgatgtccggcggtgcttttgccgttacgcaccaccccgtcagtagctgaacaggagggacagctgatagaaacagaagccactggagcacctcaaaaacaccatcatacactaaatcagtaagttggcagcatcacctacctcaatgtgtatcacaatatccatattctttgtgggggagtctggagattgagtagatattcttgttcagaatgtatcagccgatggttctacgattcttaagccacgaagagttcagatagtacaacggcatgtctcttttgactatctggcaaccggcagtgtgttctctcacgcatcacaaaagcagcaggcataaaaaaacccgcttgcgcgggctttttcacaaagcttcagcaaattggcgattaagccagtttgttgatctgtgcagtcaggttagccttatgacgtgcagctttgtttttgtggatcagacctttagcagcctgacggtccacgatcggttgcatttcgttaaatgctttctgtgcagcagctttgtcgccagcttcgatagctgcgtatactttcttgatgaaagtacgcatcatagagcgacggcttgcgttgtgcttacgagccttttcagactgaatggcgcgcttcttagctgatttgatattagccaaggtccaactcccaaatgtgttctatatggacaattcaaaggccgaggaatatgcccttttagccttcttttgtcaatggatttgtgcaaataagcgccgttaatgtgccggcactcgttacgtagtgatggcgcaggattctaccagcttgcggggtgtgaatacagcttttccgcgataaaaattgcagcaggcggtcagtttcttcccgtgatttgcgccatggcaatgaaaagccacttctttctgatttcggtactcaatcgccggttaaccttgaccgctgtacaaggtatactcggacgattttcactgttttgagccagacatgaagctgatacgcggcatacataatctcagccaggccccgcaagaagggtgtgtgctgactattggtaatttcgacggcgtgcatcgcggtcatcgcgcgctgttacagggcttgcaggaagaagggcgcaagcgcaacttaccggtgatggtgatgctttttgaacctcaaccactggaactgtttgctaccgataaagccccggcaagactgacccggctgcgggaaaaactgcgttaccttgcagagtgtggcgttgattacgtgctgtgcgtgcgtttcgacaggcgtttcgcggcgttaaccgcgcaaaatttcatcagcgatcttctggtgaagcatttgcgcgtaaaatttcttgccgtaggtgatgatttccgctttggcgctggtcgtgaaggcgatttcttgttattacagaaagctggcatggaatacggcttcgatatcaccagtacgcaaactttttgcgaaggtggcgtgcgcatcagcagcaccgccgtgcgtcaggcccttgcggatgacaatctggctctggcagagagtttactggggcacccgtttgccatctccgggcgtgtagtccacggtgatgaattagggcgcactataggtttcccgacggcgaatgtaccgctgcgccgtcaggtttccccggtgaaaggggtttatgcggtagaagtgctgggcctcggtgaaaagccgttacccggcgtggcaaacatcggaacacgcccaacggttgccggtattcgccagcagctggaagtgcatttgttagatgttgcaatggacctttacggtcgccatatacaagtagtgctgcgtaaaaaaatacgcaatgagcagcgatttgcgtcgctggacgaactgaaagcgcagattgcgcgtgatgaattaaccgcccgcgaattttttgggctaacaaaaccggcttaagcctgttatgtaatcaaaccgaaatacggaaccgagaatctgatgagtgactataaatcaaccctgaatttgccggaaacagggttcccgatgcgtggcgatctcgccaagcgcgaacccggaatgctggcgcgttggactgatgatgatctgtacggcatcatccgtgcggctaaaaaaggcaaaaaaaccttcattctgcatgatggccctccttatgcgaatggcagcattcatattggtcactcggttaacaagattctgaaagacattatcgtgaagtccaaagggctttccggttatgactcgccgtatgtgcctggctgggactgccacggtctgccgatcgagctgaaagtcgagcaagaatacggtaagccgggtgagaaattcaccgccgccgagttccgcgccaagtgccgcgaatacgcggcgacccaggttgacggtcaacgcaaagactttatccgtctgggcgtgctgggcgactggtcgcacccgtacctgaccatggacttcaaaactgaagccaacatcatccgcgcgctgggcaaaatcatcggcaacggtcacctgcacaaaggcgcgaagccagttcactggtgcgttgactgccgttctgcgctggcggaagcggaagttgagtattacgacaaaacttctccgtccatcgacgttgctttccaggcagtcgatcaggatgcactgaaagcaaaatttgccgtaagcaacgttaacggcccaatctcgctggtaatctggaccaccacgccgtggactctgcctgccaaccgcgcaatctctattgcaccagatttcgactatgcgctggtgcagatcgacggtcaggccgtgattctggcgaaagatctggttgaaagcgtaatgcagcgtatcggcgtgaccgattacaccattctcggcacggtaaaaggtgcggagcttgagctgctgcgctttacccatccgtttatgggcttcgacgttccggcaatcctcggcgatcacgttaccctggatgccggtaccggtgccgttcacaccgcgcctggccacggcccggacgactatgtgatcggtcagaaatacggcctggaaaccgctaacccggttggcccggacggcacttatctgccgggcacttatccgacgctggatggcgtgaacgtcttcaaagcgaacgacatcgtcgttgcgctgctgcaggaaaaaggcgcgctgctgcacgttgagaaaatgcagcacagctatccgtgctgctggcgtcacaaaacgccgatcatcttccgcgcgacgccgcagtggttcgtcagcatggatcagaaaggtctgcgtgcgcagtcactgaaagagatcaaaggcgtgcagtggatcccggactggggccaggcgcgtatcgagtcgatggttgctaaccgtcctgactggtgtatctcccgtcagcgcacctggggtgtaccgatgtcactgttcgtgcacaaagacacggaagagctgcatccgcgtacccttgaactgatggaagaagtggcaaaacgcgttgaagtcgatggcatccaggcgtggtgggatctcgatgcgaaagagatcctcggcgacgaagctgatcagtacgtgaaagtgccggacacattggatgtatggtttgactccggatctacccactcttctgttgttgacgtgcgtccggaatttgccggtcacgcagcggacatgtatctggaaggttctgaccaacaccgcggctggttcatgtcttccctaatgatctccaccgcgatgaagggtaaagcgccgtatcgtcaggtactgacccacggctttaccgtggatggtcagggccgcaagatgtctaaatccatcggcaataccgtttcgccgcaggatgtgatgaacaaactgggcgcggatattctgcgtctgtgggtggcatcaaccgactacaccggtgaaatggccgtttctgacgagatcctgaaacgtgctgccgatagctatcgtcgtatccgtaacaccgcgcgcttcctgctggcaaacctgaacggttttgatccagcaaaagatatggtgaaaccggaagagatggtggtactggatcgctgggccgtaggttgtgcgaaagcggcacaggaagacatcctcaaggcgtacgaagcatacgatttccacgaagtggtacagcgtctgatgcgcttctgctccgttgagatgggttccttctacctcgacatcatcaaagaccgtcagtacaccgccaaagcggacagtgtggcgcgtcgtagctgccagactgcgctatatcacatcgcagaagcgctggtgcgctggatggcaccaatcctctccttcaccgctgatgaagtgtggggctacctgccgggcgaacgtgaaaaatacgtcttcaccggtgagtggtacgaaggcctgtttggcctggcagacagtgaagcgatgaacgatgcgttctgggacgagctgttgaaagtgcgtggcgaagtgaacaaagtcattgagcaagcgcgtgccgacaagaaagtgggtggctcgctggaagcggcagtaaccttgtatgcagaaccggaactgtcggcgaaactgaccgcgctgggcgatgaattacgatttgtcctgttgacctccggcgctaccgttgcagactataacgacgcacctgctgatgctcagcagagcgaagtactcaaagggctgaaagtcgcgttgagtaaagccgaaggtgagaagtgcccacgctgctggcactacacccaggatgtcggcaaggtggcggaacacgcagaaatctgcggccgctgtgtcagcaacgtcgccggtgacggtgaaaaacgtaagtttgcctgatgagtcaatcgatctgttcaacagggctacgctggctgtggctggtggtagtcgtgctgattatcgatctgggcagcaaatacctgatcctccagaactttgctctgggggatacggtcccgctgttcccgtcgcttaatctgcattatgcgcgtaactatggcgcggcgtttagtttccttgccgatagcggcggctggcagcgttggttctttgccggtattgcgattggtattagcgtgatcctggcagtgatgatgtatcgctcgaaggccacgcagaagctaaacaatatcgcttacgcgctgattattggcggcgcgctgggcaacctgttcgaccgcctgtggcacggcttcgttgtcgatatgatcgacttctacgtcggcgactggcacttcgccaccttcaaccttgccgatactgccatctgtgtcggtgcggcactgattgtgctggaaggttttttgccttctagagcgaaaaaacaataataaaccctgccggatgcgatgctgacgcatcttatccggcctacagattgctgcgaaatcgtaggccggataaggcgtttacgccgcatccggcaaaaatccttaaatataagagcaaacctgcatgtctgaatctgtacagagcaatagcgccgtcctggtgcacttcacgctaaaactcgacgatggcaccaccgccgagtctacccgcaacaacggtaaaccggcgctgttccgcctgggtgatgcttctctttctgaagggctggagcaacacctgttggggctgaaagtgggcgataaaaccaccttctcgttggagccagatgcggcgtttggcgtgccgtcaccggacctgattcagtacttctcccgccgtgaatttatggatgcaggcgagccagaaattggcgcaatcatgctttttaccgcaatggatggcagtgagatgcctggcgtgatccgcgaaattaacggcgactccattaccgttgatttcaaccatccgctggccgggcagaccgttcattttgatattgaagtgctggaaatcgatccggcactggaggcgtaacatgcagatcctgttggccaacccgcgtggtttttgtgccggggtagaccgcgctatcagcattgttgaaaacgcgctggccatttacggcgcaccgatatatgtccgtcacgaagtggtacataaccgctatgtggtcgatagcttgcgtgagcgtggggctatctttattgagcagattagcgaagtaccggacggcgcgatcctgattttctccgcacacggtgtttctcaggcggtacgtaacgaagcaaaaagtcgcgatttgacggtgtttgatgccacctgtccgctggtgaccaaagtgcatatggaagtcgcccgcgccagtcgccgtggcgaagaatctattctcatcggtcacgccgggcacccggaagtggaagggacaatgggccagtacagtaacccggaagggggaatgtatctggtcgaatcgccggacgatgtgtggaaactgacggtcaaaaacgaagagaagctctcctttatgacccagaccacgctgtcggtggatgacacgtctgatgtgatcgacgcgctgcgtaaacgcttcccgaaaattgtcggtccgcgcaaagatgacatctgctacgccacgactaaccgtcaggaagcggtacgcgccctggcagaacaggcggaagttgtgttggtggtcggttcgaaaaactcctccaactccaaccgtctggcggagctggcccagcgtatgggcaaacgcgcgtttttgattgacgatgcgaaagacatccaggaagagtgggtgaaagaggttaaatgcgtcggcgtgactgcgggcgcatcggctccggatattctggtgcagaatgtggtggcacgtttgcagcagctgggcggtggtgaagccattccgctggaaggccgtgaagaaaacattgttttcgaagtgccgaaagagctgcgtgtcgatattcgtgaagtcgattaagtcattagcagcctaagttatgcgaaaatgccggtcttgttaccggcattttttatggagaaaacatgcgtttacctatcttcctcgatactgaccccggcattgacgatgccgtcgccattgccgccgcgatttttgcacccgaactcgacctgcaactgatgaccaccgtcgcgggtaatgtctcggttgagaaaactacccgcaatgccctgcaactgctgcatttctggaatgcggagattccgctcgcccaaggggccgctgtgccactggtacgcgcaccgcgtgatgcggcatctgtgcacggcgaatcgggaatggctggctacgactttgttgagcacaaccgaaagccgctcgggataccggcgtttctggcgattcgggatgccctgatgcgtgcaccagagcctgttaccctggtggccatcggcccgttaaccaatattgcgctgttactttcacaatgcccggaatgcaagccgtatattcgccgtctggtgatcatgggtggttctgccggacgcggcaactgtacgccaaacgccgagtttaatattgctgccgatccagaagctgctgcctgtgtcttccgcagtggtattgaaatcgtcatgtgcggtttggatgtcaccaatcaggcaatattaactcctgactatctctctacactgccgcagttaaaccgtaccgggaaaatgcttcacgccctgtttagccactaccgtagcggcagtatgcaaagcggcttgcgaatgcacgatctctgcgccatcgcctggctggtgcgcccggacctgttcactctcaaaccctgttttgtggcagtggaaactcagggcgaatttacctcaggcacgacggtggttgatatcgacggttgcctgggcaagccagccaatgtacaggtggcattggatctggatgtgaaaggcttccagcagtgggtggctgaggtgctggctctggcgtcgtaacctgtcacatgttattggcatgcagtcattcatcgactcatgcctttcactgatatccctccctgtttatcattaatttctaattatcagcgtttttggctggcggcgtagcgatgcgctggttactctgaaaacggtctatgcaaattaacaaaagagaatagctatgcatgatgcaaacatccgcgttgccatcgcgggagccggggggcgtatgggccgccagttgattcaggcggcgctggcattagagggcgtgcagttgggcgctgcgctggagcgtgaaggatcttctttactgggcagcgacgccggtgagctggccggagccgggaaaacaggcgttaccgtgcaaagcagcctcgatgcggtaaaagatgattttgatgtgtttatcgattttacccgtccggaaggtacgctgaaccatctcgctttttgtcgccagcatggcaaagggatggtgatcggcactacggggtttgacgaagccggtaaacaagcaattcgtgacgccgctgccgatattgcgattgtctttgctgccaattttagcgttggcgttaacgtcatgcttaagctgctggagaaagcagccaaagtgatgggtgactacaccgatatcgaaattattgaagcacatcatagacataaagttgatgcgccgtcaggcaccgcactggcaatgggagaggcgatcgcccacgcccttgataaagatctgaaagattgcgcggtctacagtcgtgaaggccacaccggtgaacgtgtgcctggcaccattggttttgccaccgtgcgtgcaggtgacatcgttggtgaacataccgcgatgtttgccgatattggcgagcgtctggagatcacccataaggcgtccagccgtatgacatttgctaacggcgcggtaagatcggctttgtggttgagtggtaaggaaagcggtctttttgatatgcgagatgtacttgatctcaataatttgtaaccacaaaatatttgttatggtgcaaaaataacacatttaatttattgattataaagggctttaatttttggcccttttatttttggtgttatgtttttaaattgtctataagtgccaaaaattacatgttttgtcttctgtttttgttgttttaatgtaaattttgaccatttggtccacttttttctgctcgtttttatttcatgcaatcttcttgctgcgcaagcgttttccagaacaggttagatgatctttttgtcgcttaatgcctgtaaaacatgcatgagccacaaaataatataaaaaatcccgccattaagttgacttttagcgcccatatctccagaatgccgccgtttgccagaaattcgtcggtaagcagatttgcattgatttacgtcatcattgtgaattaatatgcaaataaagtgagtgaatattctctggagggtgttttgattaagtcagcgctattggttctggaagacggaacccagtttcacggtcgggccataggggcaacaggttcggcggttggggaagtcgttttcaatacttcaatgaccggttatcaagaaatcctcactgatccttcctattctcgtcaaatcgttactcttacttatccccatattggcaatgtcggcaccaatgacgccgatgaagaatcttctcaggtacatgcacaaggtctggtgattcgcgacctgccgctgattgccagcaacttccgtaataccgaagacctctcttcttacctgaaacgccataacatcgtggcgattgccgatatcgatacccgtaagctgacgcgtttactgcgcgagaaaggcgcacagaatggctgcattatcgcgggcgataacccggatgcggcgctggcgttagaaaaagcccgcgcgttcccaggtctgaatggcatggatctggcaaaagaagtgaccaccgcagaagcctatagctggacacaagggagctggacgttgaccggtggcctgccagaagcgaaaaaagaagacgagctgccgttccacgtcgtggcttatgattttggtgccaagcgcaacatcctgcggatgctggtggatagaggctgtcgcctgaccatcgttccggcgcaaacttctgcggaagatgtgctgaaaatgaatccagacggcatcttcctctccaacggtcctggcgacccggccccgtgcgattacgccattaccgccatccagaaattcctcgaaaccgatattccggtattcggcatctgtctcggtcatcagctgctggcgctggcgagcggtgcgaagactgtcaaaatgaaatttggtcaccacggcggcaaccatccggttaaagatgtggagaaaaacgtggtaatgatcaccgcccagaaccacggttttgcggtggacgaagcaacattacctgcaaacctgcgtgtcacgcataaatccctgttcgacggtacgttacagggcattcatcgcaccgataaaccggcattcagcttccaggggcaccctgaagccagccctggtccacacgacgccgcgccgttgttcgaccactttatcgagttaattgagcagtaccgtaaaaccgctaagtaatcaggagtaaaagagccatgccaaaacgtacagatataaaaagtatcctgattctgggtgcgggcccgattgttatcggtcaggcgtgtgagtttgactactctggcgcgcaagcgtgtaaagccctgcgtgaagagggttaccgcgtcattctggtgaactccaacccggcgaccatcatgaccgacccggaaatggctgatgcaacctacatcgagccgattcactgggaagttgtacgcaagattattgaaaaagagcgcccggacgcggtgctgccaacgatgggcggtcagacggcgctgaactgcgcgctggagctggaacgtcagggcgtgttggaagagttcggtgtcaccatgattggtgccactgccgatgcgattgataaagcagaagaccgccgtcgtttcgacgtagcgatgaagaaaattggtctggaaaccgcgcgttccggtatcgcacacacgatggaagaagcgctggcggttgccgctgacgtgggcttcccgtgcattattcgcccatcctttaccatgggcggtagcggcggcggtatcgcttataaccgtgaagagtttgaagaaatttgcgcccgcggtctggatctctctccgaccaaagagttgctgattgatgagtcgctgatcggctggaaagagtacgagatggaagtggtgcgtgataaaaacgacaactgcatcatcgtctgctctatcgaaaacttcgatgcgatgggcatccacaccggtgactccatcactgtcgcgccagcccaaacgctgaccgacaaagaatatcaaatcatgcgtaacgcctcgatggcggtgctgcgtgaaatcggcgttgaaaccggtggttccaacgttcagtttgcggtgaacccgaaaaacggtcgtctgattgttatcgaaatgaacccacgcgtgtcccgttcttcggcgctggcgtcgaaagcgaccggtttcccgattgctaaagtggcggcgaaactggcggtgggttacaccctcgacgaactgatgaacgacatcactggcggacgtactccggcctccttcgagccgtccatcgactatgtggttactaaaattcctcgcttcaacttcgaaaaattcgccggtgctaacgaccgtctgaccactcagatgaaatcggttggcgaagtgatggcgattggtcgcacgcagcaggaatccctgcaaaaagcgctgcgcggcctggaagtcggtgcgactggattcgacccgaaagtgagcctggatgacccggaagcgttaaccaaaatccgtcgcgaactgaaagacgcaggcgcagatcgtatctggtacatcgccgatgcgttccgtgcgggcctgtctgtggacggcgtcttcaacctgaccaacattgaccgctggttcctggtacagattgaagagctggtgcgtctggaagagaaagtggcggaagtgggcatcactggcctgaacgctgacttcctgcgccagctgaaacgcaaaggctttgccgatgcgcgcttggcaaaactggcgggcgtacgcgaagcggaaatccgtaagctgcgtgaccagtatgacctgcacccggtttataagcgcgtggatacctgtgcggcagagttcgccaccgacaccgcttacatgtactccacttatgaagaagagtgcgaagcgaatccgtctaccgaccgtgaaaaaatcatggtgcttggcggcggcccgaaccgtatcggtcagggtatcgaattcgactactgttgcgtacacgcctcgctggcgctgcgcgaagacggttacgaaaccattatggttaactgtaacccggaaaccgtctccaccgactacgacacttccgaccgcctctacttcgagccggtaactctggaagatgtgctggaaatcgtgcgtatcgagaagccgaaaggcgttatcgtccagtacggcggtcagaccccgctgaaactggcgcgcgcgctggaagctgctggcgtaccggttatcggcaccagcccggatgctatcgaccgtgcagaagaccgtgaacgcttccagcatgcggttgagcgtctgaaactgaaacaaccggcgaacgccaccgttaccgctattgaaatggcggtagagaaggcgaaagagattggctacccgctggtggtacgtccgtcttacgttctcggcggtcgggcgatggaaatcgtctatgacgaagctgacctgcgtcgctacttccagacggcggtcagcgtgtctaacgatgcgccagtgttgctggaccacttcctcgatgacgcggtagaagttgacgtggatgccatctgcgacggcgaaatggtgctgattggcggcatcatggagcatattgagcaggcgggcgtgcactccggtgactccgcatgttctctgccagcctacaccttaagtcaggaaattcaggatgtgatgcgccagcaggtgcagaaactggccttcgaattgcaggtgcgcggcctgatgaacgtgcagtttgcggtgaaaaacaacgaagtctacctgattgaagttaacccgcgtgcggcgcgtaccgttccgttcgtctccaaagccaccggcgtaccgctggcaaaagtggcggcgcgcgtgatggctggcaaatcgctggctgagcagggcgtaaccaaagaagttatcccgccgtactactcggtgaaagaagtggtgctgccgttcaataaattcccgggcgttgacccgctgttagggccagaaatgcgctctaccggggaagtcatgggcgtgggccgcaccttcgctgaagcgtttgccaaagcgcagctgggcagcaactccaccatgaagaaacacggtcgtgcgctgctttccgtgcgcgaaggcgataaagaacgcgtggtggacctggcggcaaaactgctgaaacagggcttcgagctggatgcgacccacggcacggcgattgtgctgggcgaagcaggtatcaacccgcgtctggtaaacaaggtgcatgaaggccgtccgcacattcaggaccgtatcaagaatggcgaatatacctacatcatcaacaccacctcaggccgtcgtgcgattgaagactcccgcgtgattcgtcgcagtgcgctgcaatataaagtgcattacgacaccaccctgaacggcggctttgccaccgcgatggcgctgaatgccgatgcgactgaaaaagtaatttcggtgcaggaaatgcacgcacagatcaaataatagcgtgtcatggcagatatttttcatccgctaatttgatcgaataactaatacggttctctgatgaggaccgtttttttttgcccattaagtaaatcttttggggaatcgatatttttgatgacataagcaggatttagctcacacttatcgacggtgaagttgcatactatcgatatatccacaattttaatatggccttgtttaattgcttcaaaacgagtcatagccagacttttaatttgtgaaactggagttcgtatgtgtgaaggatatgttgaaaaaccactctacttgttaatcgccgaatggatgatggctgaaaatcggtgggtgatagcaagagagatctctattcatttcgatattgaacacagcaaggcggttaataccctgacttatattctgtcggaagtcacagaaataagctgcgaagttaagatgatccctaataagctggaagggcggggatgccagtgtcagcgactggttaaagtggtcgatatcgatgagcaaatttacgcgcgcctgcgcaataacagtcgggaaaaattagtcggtgtaagaaagacgccgcgtattcctgccgttccgctcacggaacttaaccgcgagcagaagtggcagatgatgttgtcaaagagtatgcgtcgttaattttatctcgttgataccgggcgtcctgcttgccagatgcgatgttgtagcatcttatccagcaaccaggtcgcatccggcaagatcaccgtttaggcgtcacatccgtcgtcccctgcaaacgggggcgattttcctccatttgcctcagtggctgcgtttcatgtaacgatacatgacagcgcccgacaagatcctgatactctttggtattcaaccgtttccagtgtaactcgtcgtcactaacattgcgtacagcgcgggctggcgtacccatcaacaactggcgtttctcgccgcgaaagcccgctttgacaaagctcatggcggcaacaatgctctcttcgccaatgaccgcgccatccataatcacgctgttcatcccgaccaatgcatcgcgaccaatcaaacaaccatgcaggatcgctccgtgcccgatatggccgttttccccaacgatagtgtcagtgtcgcagtagccatgcataatgcagccatcctgaatattggctcccgcttgcacgatcaaccgcccgtagtcaccacgcagtgaggcgagtgggccgatgtagacaccggctcccacaatcacatcgccaatcaagacggcactgggatggacaaacgccgtcgggtgaaccaccggaattaacccctcaaaggcgtaatagctcacggttgttaacgtcctttccacaccggatcgcgcttctcggcaaacgccagcggcccttcaatggcatcttccgaatgcagaaccgatggatagtgtttcaacacgccgctgcgaatatagcgatacgcttcttctaccggcatttcgctggtggtgcggtagatctctttcagcgccgcaatcgccagcggggcgctgttaaccagctgctgagccagttcgcgggcgttatccatcagttccgcctggctaaccacgcggttgactatcccccaacgcagcgcctcttctgcgcccattcgtctgccggtcatcaccatttcattgacgatggcaggcggcaggatcttcggcagacgcagcacaccgccgctgtcaggaacgatgcccagtttggcttccggcagggcgaagctggcgttatcggcacaaacaataaaatctgccgccagcgccagttcaaagccgccgccaaaggcatagccgttcacagctgcgataaccggtttgtcgagattgaaaatttcggttaatcccgcaaaaccacccggaccaaagtcagcatccggtgcttcgccttctgctgccgcttttaaatcccagcccgcggaaaagaacttctctccggcaccggtaataatggcgacacgtaattgcggatcgtcacggaaatttagaaatacttcgcccatttcaaagctggtttttgcatcaatagcattcgcttttggacgatcaagggtaatttccagaattgatccattgcgggtcagatgtaatgattcactcattccttttctccatttttgctttttcagggacgacaacatccctgcaaaaaatgcatattgttttagagtgtgattattagctggcagggtagttccctgctgtttcatttatttcagattctttctaattattttccccgagcaattacgtggcagatcttttctgatctccagataagagggcactttaaatttcgccatattttgttcgcagaagcggaaaaattcctcttcgctcaatgtttcaccttcattcagcaccacaaatgctttgatggcttcatcgcgaatcgaatctttaatacccacaaccacgatgtcctgaattttcgggtgcgcggcgataatattttccagctccacgcaggagacattctcgccgccacgtttaatcatattgcagcggcgatcgacgaaataaaaaaagtcctcttcgtcgcggtatccggtatcgccggtatgcagccagccatcggcttccagcactttcgcagtggcttgtgggttgagaaagtactctttgaagatggttttcccaggtatgcctttaatgcagatttcaccgatctcaccagccgggagcgggcgattgtgatcgtcgcggatctccgcttcgtagcaaaaccccacccgaccaatcgacggccagcgtcgtttatcgccaggacgatcgccgataatgcccacaatggtttccgtcatcccataagacgtcagcaagcgaacgccgaagcgttcacaaaacgcatctttttcctgctccgacaagttgagataaaacatcacttcccgcaggcggtgttgctgatcgttcgctgaaggcggctgtaccatcaacgtacggatcatcatcggaatacattcggtaacggtggcgcggtacttctgtacctgtccccagaaggcgcgggcgctgtatttctcgaccagcacaaaggtggccccggcagaaaacgccgccatcgccgcagtacactggcaatcgatatgaaacgcaggcattaccgtcaggtagacgtcatcgtcacgcagtgcacactgccaggcggagtaatatccagcgaagcgcaggttgtaatgggtaatcaccacacctttcggtcgggaggtggtgccggaggtgaagagaatttccgccgtatcgtcagtcgatagcggcggtgcatagcacaaggtggcaggttgttgatttttcagttgagtaaacgaactcacgccatcatcagcgggaagtgccacatctgtcaggcaaatgtgccgcaattgagtggcatcttcctgctgaatctgttgatacataggatagaattgcgcactggtcaccagcaggcacgcctggctattttgcaggatccacgcgctttcctcgcacaacaggcgggcgttaatcggcaccataatcgcgccaatttttgccagcccgaaccagcaaaagataaattccgggcagttgtcgagatgtagtgcaaccttgtcgcctttgcgaatccccagcgtataaaacaggtttgccgtgcggttaatctcctgatttaactcaagataactataccggttaacgactccgccgctggattcacaaatcagcgccgttttatgaccgtaaacgtccgcaagatcgtcccacatttgacgtagatgttgtccgccaatgatatccattgcacctctatccatttttgttcgtttgttattgggcgggcgctagtcaggcaagccgactgacgccacgcgtttagtcctcaactttggccagacctttgctgaccaactcctgaatgtcgttttcgctgtagccgatatttttcaaaatggcagccgtgtccatgccatgtgagggcattccgcgccagatttgtccggggttatttttgaatttcggcatgatgttcggccctttgcaggtgcgaccatccatcgtttgccactgagtgattgattcgcgagccacatactgtggattgctttccagttccggtacggtcagcactttggcgcaggcgatattcagttcagcaaagcgttcttttacttccgcgatggtatgtgtcgccagccaggcatcgagtttctcttcaaccagtgggccgtaagggcattcgatacggtggataagctgagtgccttccgggatttctggcgtgccaagcagatgtgcgaggccaatatctttaaagcactcttcaatttgggtaatgcccaccagttccatcacgatgtagccgtcggcacatttatacagaccgcaaccggcgtagtagggatctttacctttgctcatgcgcgggcacatttcgccgccgttgaagtaatccatcatgaagtactggcccatacgcagcatcacttcatacatggcgatgtcgatactttcgcctttaccggtttcacgcactttatgcagtgctgccagcgccgccgtggtggcggtcaggccagaaaagtaatcggcggtatacgggaaggcaggcattggctggtcaacatcaccgttctgaatcaggtaaccactaaaggcctgggcgatagtgttataggccggaagattggtgtactcctcggtgccgtactgaccaaaaccggacaggtgagcgataaccagtttcgggttgtgctgccacagtacttcatcggtaatgccacgacgggcaaaggccggacctttactggcttcgatgaagatatcggtggtttccattaatttcagaaacgcttcgcggccttcatctttgaaaatatttaacgacagcgcgtgcaaattgcggcgggagagttgcgggtagttcggttgaacgcgaatggtgtcggcccaggcgacgttctcgatccagataacttccgcgccccattctgcgaacatttgcccggcaaacggtccggcgatttcgataccggagaagacaacgcgcaatccggccaacggcccgaatttcggcatgggtagatgatccattatttgctcctgaaaaatttatgtagcgcatgactgccggatgcggcgtaaacgctttatccggcctacattcgtgctcccgtaggcctgataagacgcatcagcgtcgcatcaggcagcgcacggacttagcggtattgcttcagcaccgcacgacccagcgtcaggatctgcatttcgtcagatcccccggagacgcggtctacacgcagatcacgccagaagcggctgatgcggtggttgcccgcaatcccgacaccgcccagcacctgcattgcgctatccacaacttcaaatgccgcattggcgcagaagtatttgcacatcgctgcatcgccagaggtgatggtgccgttgtctgctttccacgctgcttcatacagcatgtttttcatggagtttaatttgatcgccatgtgggcgaatttttcctgaatcaactggaaacgaccaatagcctcgccaaactgcacgcgctgattggcgtagcgcgccgcatcttcaaaggcgcacatcgccgtaccgtagttggtgagggctaccaggaaacgttcatggtcgaactcttctttgacgcggttaaagccgttaccttcccgaccgaacatgtctttctcgtccagttccacgtcgtcaaaggtgatttcacagcagctatccatacgcagaccgagcttttcaagtttggtcactttgatgcccggtttgctcatatcaacaaaccattcggtgtagacaggtttgtccggagaagccccgtcgcgcgccatcaccacgatgtacggggtgtaggcgctgctggtaataaaacacttactaccattaagataaatcttaccatttctacgggtataagtcgttttcaggctacccacgtcggagcccgcgcccggttcggtaatcgctgagttccacatctgcttaccggtgccgcggaaagccataattttgtcgatctgctcttgtgtgccttcgcgcaggaaggtgttgaacccgcccggcaactggtacagcacataggttggtgcccccagacgtcccagctccatccacacggcggcgagagtaacaaaccccgcgtccagaccaccgtgctcttcagggatcagcagactgtcgatacccatatccgccagtgctttgacaaaacgttccgggtagacgctgtcacggtcgcactcggcaaaataggcctcccagttttcgctggccatcagttcgcggataccggcgacaaacagttcctgctcatcatttaaattaaaatccatctttcaacctcttgatattttgggggttaattaatctttccagttctgtttcgcgtctttaataaaggagagcgtcaccataatgttgacgaagaacagcgggcatcctccggcgataatggcggtttgaatcggtttcaggccgccgagcgccagcagaacaataccgataatgccaaccagaattgaccaaccgatacgcaccagcagaggtggttcttcaccatcgcgtacttcgcggcaagtggacatcgccagggtataagagcaggcgttaaccagcgtaacggtggcaataaagcagaggatgaagaagccccacatggtggcggtgctgagtggcagagcggcccaggtttcaatgatggcgcgcgccacaccgtactgttcgatcagatttggaatgttgatgatgtttttatctatcaacagcagagtgttactaccgagtacagtccacaggatccaggttgacgctgtcagccccagcaccatgccgaagcacagttcacgcacagtacgaccacgggagatgcgggcgaggaagatactcatctggatagcataaatcacccaccatgcccagtagaacacggtccagccctgcgggaagccgcctttagcgatgggatcggtatagaacaacatgcgcggcagatacatcagcaacatccccaccgaatcggtgaagtagttcatgatgaagctggcaccgctgacaatgaacacccaacccagcatcaggaagctcaggtaactacgcacgtcactggcgatacgtacccctttttgcagaccgcaagcgacgcaaatggcgttgaggataatccagcaggtaatgatgatagcgtccagttgcagggtatgcggaatgccaaacaaccattgcatacactcggtcaccagcggcgtggcaaggcccagactggtacccatcgcgaagatcaaggcgacgagatagaagttgtcgacgatagtgccgaacaaccctttggcgtgtttttcacctaccagcggcaccagtgtcgagctggggcgaatcacttccattttgcggacaaagaagaagtaagcgaaggcgactgaaaggaagctgtaagtggcccacggcagaggtccccagtggaacaagctgtaagccagccccaactctttcgcccctgtcgagttcggttctaagccaaacggcggggtggagatgtagtagtagatctcaatcgatccccagaacagtacggcagcagacgtacaggaggcgaacatcataaagatccaactggcggtgctaaattctggcggttcgttacctaaacgctttttggcatacgggccaaacaccagccagaaccaaccgaaaagcatcaccaccatataccattcaaatgcccatccccatacattggtgacgtaactgaatacagcattaataacgacattcgctgcatccagatctctgactgtaagccaacaaagtatgccgacgattattaacggcggaaagaaaaccttcggttctattcccgtttttctcttttcattcttcatgagttaattccactgtgaaaacgaatatttattttgcgttcccgtttgttttatttttgttaacatttaatataattattattaacctcgtggacgcgttaatggctaactcataatgggtattcaataagctgtattctgtgattggtatcacatttttgtttcgggtgaatagagggcgttttttcgttaattttgattaataatcagtttgttatgctctgttgtgagtaaaaaataacatctgactttcaatattggtgatccataaaacaatattgaaaatttctttttgctacgccgtgttttcaatattggtgaggaacttaacaatattgaaagttggatttatctgcgtgtgacattttcaatattggtgattaaagttttatttcaaaattaaagggcgtgatatctgtaattaacaccaccgatatgaacgacgtttccttcatgatttctggagatgcaatgaagattattacttgctataagtgcgtgcctgatgaacaggatattgcggtcaataatgctgatggttcattagacttcagcaaagccgatgccaaaataagccaatacgatctcaacgctattgaagcggcttgccagctaaagcaacaggcagcagaggcgcaggtgacagccttaagtgtgggcggtaaagccctgaccaacgccaaagggcgtaaagatgtgctatcgcgcggcccggatgaactgattgtggtgattgatgaccagttcgagcaggcactgccgcaacaaacggcgagcgcactggctgcagccgcccagaaagcaggctttgatctgatcctctgtggcgatggttcttccgacctttatgcccagcaggttggtctgctggtgggcgaaatcctcaatattccggcagttaacggcgtcagcaaaattatctccctgacggcagataccctcaccgttgagcgcgaactggaagatgaaaccgaaaccttaagcattccgctgcctgcggttgttgctgtttccactgatatcaactccccacaaattccttcgatgaaagccattctcggcgcggcgaaaaagcccgtccaggtatggtcggcggcggatattggttttaacgcagaggcagcctggtcagaacaacaggttgccgcgccgaaacagcgcgaacgtcagcgcatcgtgattgaaggcgacggcgaagaacagatcgccgcatttgctgaaaatcttcgcaaagtcatttaattacaggggatgctatgaacacgttttctcaagtctgggtattcagcgataccccttctcgtctgccggaactgatgaacggtgcgcaggctttagctaatcaaatcaacacctttgtcctcaatgatgccgacggcgcacaggcaatccagctcggcgctaatcatgtctggaaattaaacggcaaaccggacgatcggatgatcgaagattacgccggtgtcatggctgacactattcgccagcacggcgcagacggcctggtgctgctgccaaacacccgtcgcggcaaattactggcggcaaaactgggttatcgccttaaagcggcggtgtctaacgatgccagcaccgtcagcgtacaggacggtaaagcgacagtgaaacacatggtttacggtggtctggcgattggcgaagaacgcattgccacgccgtatgcggtactgaccatcagcagcggcacgttcgatgcggctcagccagacgcgtcacgcactggcgaaacgcacaccgtggagtggcaggctccggctgtggcgattacccgcacggcaacccaggcgcgccagagcaacagcgtcgatctcgacaaagcccgtctggtggtcagcgtcggtcgcggtattggcagcaaagagaacattgcgctggcagaacagctttgcaaggcgataggtgcggagttggcctgttctcgtccggtggcggaaaacgaaaaatggatggagcacgaacgctatgtcggtatctccaacctgatgctgaaacctgaactgtacctggcggtggggatctccgggcagatccagcacatggttggcgctaacgcgtcgcaaaccattttcgccatcaataaagataaaaatgcgccgatcttccagtacgcggattacggcattgttggcgacgccgtgaagatccttccggcgctgaccgcagctttagcgcgttgatccactctggcagggctgcattttggccctgccgctgacagggagctcttatgtccgaagatatctttgacgccatcatcgtcggtgcagggcttgccggttcggttgccgcactggtgctcgcccgcgaaggtgcgcaagtgttagttatcgagcgtggcaattccgcaggtgccaagaacgtcaccggcgggcgtctctatgcccacagtctggaacacattattcctggtttcgccgactccgcccccgtagaacgcctgatcacccatgaaaaactcgcgtttatgacggaaaagtcagcgatgactatggactactgcaatggtgacgaaacctcgccatcccagcgttcttactccgttttgcgcagtaaatttgatgcctggctgatggagcaggccgaagaagcgggcgcgcagttaattaccgggatccgcgtcgataacctcgtacagcgcgatggcaaagtcgtcggtgtagaagccgatggcgatgtgattgaagcgaaaacggtgatccttgctgatggggtgaactccatccttgccgaaaaattggggatggcaaaacgcgtcaaaccgacggatgtggcggttggcgtgaaggaactgatcgagttaccgaagtcggttattgaagaccgttttcagttgcagggtaatcagggggcggcttgcctgtttgcgggatcacccaccgatggcctgatgggcggcggcttcctttataccaatgaaaacaccctgtcgctggggctggtttgtggtttgcatcatctgcatgacgcgaaaaaatcggtgccgcaaatgctggaagatttcaaacagcatccggccgttgcaccgctgatcgcgggcggcaagctggtggaatattccgctcacgtagtgccggaagcaggcatcaacatgctgccggagttggttggtgacggcgtattgattgccggtgatgccgccggaatgtgtatgaacctcggttttaccattcgcggtatggatctggcgattgccgccggggaagccgcagcaaaaaccgtgctttcagcgatgaaaagcgacgatttcagtaagcaaaaactggcggaatatcgtcagcatcttgagagtggtccgctgcgcgatatgcgtatgtaccagaaactaccggcgttccttgataacccacgcatgtttagcggctacccggagctggcggtgggtgtggcgcgtgacctgttcaccattgatggcagcgcgccggaactgatgcgcaagaaaatcctccgccacggcaagaaagtgggcttcatcaatctaatcaaggatggcatgaaaggagtgaccgttttatgacttctcccgtcaatgtggacgtcaaactgggcgtcaataaattcaatgtcgatgaagagcatccgcacattgttgtgaaggccgatgctgataaacaggcgctggagctgctggtgaaagcgtgccccgcaggtctgtacaagaagcaggatgacggcagtgtgcgcttcgattacgccggatgtctggagtgcggcacctgtcgcattctggggctggggtcggcgctggaacagtgggaatacccgcgcggcacctttggtgtggagttccgttacggctgatgttggtttgatacgtaacgccgcactgactctcattgcaaaaaacaggaataaccatgcaaccgtccagaaactttgacgatctcaaattctcctctattcaccgccgcattttgctgtggggaagcggtggtccgtttctggatggttatgtactggtaatgattggcgtggcgctggagcaactgacgccggcgctgaaactggacgctgactggattggcttgctgggcgcgggaacgctcgccgggctgttcgttggcacatcgctgtttggttatatttccgataaagtcggacggcgcaaaatgttcctcattgatatcatcgccatcggcgtgatatcggtggcgacgatgtttgtttcatcccccgtcgaactgttggtgatgcgggtacttatcggcattgtcatcggtgcagattatcccatcgccacctcaatgatcaccgagttctccagtacccgtcagcgggcgttttccatcagctttattgccgcgatgtggtatgtcggcgcgacctgtgccgatctggtcggctactggctttatgatgtggaaggcggctggcgctggatgctgggtagcgcggcgatcccctgtttgttgattttgattggtcgattcgaactgcctgaatctccccgctggttattacgcaaagggcgagtaaaagagtgcgaagagatgatgatcaaactgtttggcgaaccggtggctttcgatgaagagcagccgcagcaaacccgttttcgcgatctgtttaatcgccgccattttccttttgttctgtttgttgccgccatctggacctgccaggtgatcccaatgttcgccatttacacctttggcccgcaaatcgttggtttgttgggattgggggttggcaaaaacgcggcactagggaatgtggtgattagcctgttctttatgctcggctgtattccgccgatgctgtggttaaacactgccggacggcgtccattgttgattggcagctttgccatgatgacgctggcgctggcggttttggggctaatcccggatatggggatctggctggtagtgatggcctttgcggtgtatgcctttttctctggcgggccgggtaatttgcagtggctctatcctaatgaactcttcccgacagatatccgcgcctctgccgtgggcgtgattatgtccttaagtcgtattggcaccattgtttcgacctgggcactaccgatctttatcaataattacggtatcagtaacacgatgctaatgggggcgggtatctcgctgtttggcttgttgatttccgtagcgtttgccccggagactcgagggatgtcactggcgcagaccagcaatatgacgatccgcgggcagagaatggggtaaattgttcagatttctctcttttctgaatcaatattattgactataagccgcgtgaatatatgactacactttgtgggaaaacaaaggcgtaatcacgcgggctacctatgattcttataatttatgcgcatccgtatccgcatcattcccatgcgaataaacggatgcttgaacaggcaaggacgctggaaggcgtcgaaattcgctctctttatcaactctatcctgacttcaatatcgatattgccgccgagcaggaggcgctgtctcgcgccgatctgatcgtctggcagcatccgatgcagtggtacagcattcctccgctcctcaaactttggatcgataaagttttctcccacggctgggcttacggtcatggcggcacggcgctgcatggcaaacatttgctgtgggcggtgacgaccggcggcggggaaagccattttgaaattggtgcgcatccgggctttgatgtgctgtcgcagccgctacaggcgacggcaatctactgcgggctgaactggctgccaccgtttgccatgcactgcacctttatttgtgacgacgaaaccctcgaagggcaggcgcgtcactataagcaacgtctgctggaatggcaggaggcccatcatggatagccatacgctgattcaggcgctgatttatctcggttcggcagcgctgattgtacccattgcggtacgtcttggtctgggatcggtacttggctacctgatcgccggctgcattattggcccgtgggggctgcgactggtgaccgatgccgaatctattctgcactttgccgagattggggtggtgctgatgctgtttattatcggcctcgaactcgatccacaaaggctgtggaagctgcgtgcggcagtgttcggctgtggcgcattgcagatggtgatttgcggcggcctgctggggctgttctgcatgttacttgggctgcgctggcaggtcgcggaattgatcggcatgacgctggcgctctcctctacggcgattgccatgcaggcgatgaatgaacgcaatctgatggtgacgcaaatgggtcgcagtgcctttgcggtgctgctgttccaggatatcgcggcgatcccgctggtggcgatgattccgctactggcaacgagcagtgcctcgacgacgatgggcgcatttgctctctcggcgttaaaagtggcgggtgcgctggtgctggtggtattgctggggcgctatgtcacgcgtccggcgctgcgttttgtagcccgctctggcttgcgggaagtgtttagtgccgtggcgttattcctcgtgtttggctttggtttgctgctggaagaggtcggcttgtcgatggcgatgggcgcgtttctggcgggcgtactgctggcaagctcggaataccgtcatgcgctggagagcgatatcgaaccatttaaaggtttgctgttggggctgtttttcatcggtgttggcatgtcgatagactttggcacgctgcttgaaaacccattgcgcattgtcattttgctgctcggtttcctcatcatcaaaatcgccatgctgtggctgattgcccgaccgttgcaagtgccaaataaacagcgtcgttggtttgcggtgttgttagggcagggcagtgagtttgcctttgtggtatttggcgcggcgcagatggcgaatgtgctggagccggagtgggcgaaatcgctgaccctggcggtggcgctgtcgatggcagcaacgccgattctgctggtgatcctcaatcgccttgagcaatcttctactgaggaagcgcgtgaagccgatgagatcgacgaagaacagccgcgcgtgattatcgccggattcggtcgttttgggcagattaccggacgtttactgctctccagcggggtgaaaatggtggtactcgatcacgatccggaccatatcgaaaccttgcgtaaatttggtatgaaagtgttttatggcgatgccacgcggatggatttactggaatctgccggagcggcgaaagcggaagtgctgattaacgccatcgacgatccgcaaaccaacctgcaactgacagagatggtgaaagaacatttcccgcatttgcagattattgcccgcgcccgcgatgtcgaccactacattcgtttgcgtcaggcaggcgttgaaaagccggagcgtgaaaccttcgaaggtgcgctgaaaaccgggcgtctggcactggaaagtttaggtctggggccgtatgaagcgcgagaacgtgccgatgtgttccgccgctttaatattcagatggtggaagagatggcaatggttgagaacgacaccaaagcccgcgcggcggtctataaacgcaccagcgcgatgttaagtgagatcattaccgaggaccgcgaacatctgtcattaattcaacgacatggctggcagggaaccgaagaaggtaaacataccggcaacatggcggatgaaccggaaacgaaaccctcatcctaataaagagtgacgtaaatcacactttacagctaactgtttgtttttgtttcattgtaatgcggcgagtccagggagagagcgtggactcgccagcagaatataaaattttcctcaacatcatcctcgcaccagtcgacgacggtttacgctttacgtatagtggcgacaattttttttatcgggaaatctcaatgatcagtctgattgcggcgttagcggtagatcgcgttatcggcatggaaaacgccatgccgtggaacctgcctgccgatctcgcctggtttaaacgcaacaccttaaataaacccgtgattatgggccgccatacctgggaatcaatcggtcgtccgttgccaggacgcaaaaatattatcctcagcagtcaaccgggtacggacgatcgcgtaacgtgggtgaagtcggtggatgaagccatcgcggcgtgtggtgacgtaccagaaatcatggtgattggcggcggtcgcgtttatgaacagttcttgccaaaagcgcaaaaactgtatctgacgcatatcgacgcagaagtggaaggcgacacccatttcccggattacgagccggatgactgggaatcggtattcagcgaattccacgatgctgatgcgcagaactctcacagctattgctttgagattctggagcggcggtaattttgtatagaatttacggctagcgccggatgcgacgccggtcgcgtcttatccggccttcctatatcaggctgtgtttaagacgccgccgcttcgcccaaatccttatgccggttcgacggctggacaaaatactgtttatcttcccagcgcaggcaggttaatgtaccaccccagcagcagccggtatccagcgcgtatataccttccggcgtacctttgccctccagcgatgcccagtgaccaaaggcgatgctgtattcttcagcgacagggccaggaatcgcaaaccacggtttcagtggggcaggggcctcttccggcgattctttgctgtacatatccagttgaccgttcgggaagcaaaaacgcatacgggtaaaagcgttggtgataaaacgcagtcttcccagcccccgcaattccggtgaccagttatttggcatatcgccgtacatggcatcaagaaagaagggataggagtcactcgatagcaccgcttctacatcgcgtgcgcactctttggcggtctgcagatcccactgcggcgtgatccctgcgtgggccatcaccagctttttctcttcgtcgatttgcagcagaggctggcgccgcagccagttaagcagctcgtcggcatccggcgcttccagcagcggtgtcaggcgatctttcggtttattgcggctgatcccggcaaataccgccagcagatgcagatcgtgattgcccagcaccagacgtacgctgtcgcctaaggatttcacatagcgcagaacatccagcgaacccggcccgcgcgcgaccagatcgcccgtcagccagagggtatctttcccaggggtaaattctactttatgcagcaatgcgatcagttcatcgtaacaaccatgaacgtcgccaataaggtatgtcgccatattcttttaatgaatgagtgtgggaacggcgagtcggaatacgggaatgtcgatgctgaaagggacgccattttcatcgatcatttcgtagtgaccctgcatggtgcccagcggggtttcaatgattgcaccgctggtgtactggtactcttcgccaggcgcgataagtggctggacgccaaccactccttcgccctggacttcggtttcacggccattgccattggtgatcagccagtaacgccccaacaactgcactggcgctcgccccagattgcgtatggttacggtataagcaaaaacgtaacgttcattatcaggtgaagattgagcctcaatgtagacgctttgaacctgaatacacactcggggcgaattgatcatcgttaactctcctgcaaaggcgcgttctccgccagatagttcgccatctggcaatattgcgcgacagagatattttccgctcgcatcgccgggtcgatccccattcccgttaacacctcgacgctaaacaggttgccgaggctgttacgaatggttttacgacgctggttaaaggcttcggtggtgatgcggctcaacacacgaacatctttaaccgggtgaggcatcgttgcatgaggaaccaggcgcacgacggcggaatccactttgggtggtggtgtaaaggctgacggcggtacttccagtaccgggatcacattgcaatagtattgcgccatgacgcttaatcgaccatacgctttgctgttcggtcctgcaaccagacgattcaccacctctttttgcaacataaagtgcatgtcggcaatggcatcagtatagctaaacagatggaacatcaacggcgtggagatgttataaggcaggttgccgaaaacacgcagcggctgacccattttctcggccagttcaccaaagttaaaggtcatcgcatcctgctgataaatcgtcagtttcgggcctaagaatggatgcgtttgcagacgtgccgccagatcgcggtcaagttcgatgaccgtcagctggtccagacgttcgccgaccggttcggtcaatgccgccagaccggggccgatttcgaccatcgcctggcccttttgcgggttaatggcagacacaatactgtcgatcacgaactgatcgttgagaaagttttgcccgaagcgtttacgggctaagtggccctggtggactcgattattcattgggtgttaacaatcattttgatggcgagattaagcgccgtaataaaactgccgacatcggctttgccacgtcccgccagttcaagcgcggtgccgtggtccactgatgtgcgaataaagggcaggcccagcgtaatgttcacaccgcgcccgaagccctggtattttagcacgggaagaccctgatcgtggtacatcgccagcacggcgtcggcgttatcaagatatttcggctgaaacagggtatcggcaggcagcggcccgttgagtttcatcccctgcgcccgcagctcattgagcaccggaataatggtgtctatctcttccgtacccatatgaccgccttcgcccgcgtgcggattcagcccgcagaccagaatgcgcggttcggcaataccaaatttggtccgcaaatcgtgatgcaaaatagcaatcacttcgtgcaaaagtgcaggggtgatagcgtctgcgatatcgcgcagcggtaaatgcgtcgttgccagcgccacgcgaagttcttcggtcgccagcatcatcaccacctttttcgcctgcgaacgctcttcgaaaaactcggtatgaccggtaaaaggaatgccagcgtcgttaataacgcctttatgcaccggacctgtgatcagcgcggcaaattcgccgttcagacaaccatcgcacgctcgcgccagcgtttccaccacataatgcccattttcaaccgctaactgccccgcagtgacaggtgcacgtagcgcgacaggaagtagcgttaatgtgcccgcagtttgcggttgtgcaggggagttgggggaataagggcggagggtgagcggcaaaccgagcatcgctgcccggttggtaaggagagtggcatcggcacaaacaaccagttcgaccggccactcacgctgtgcaagctggacaactaagtccgggccaatcccggcgggctcgccgggagtgatcacaacacgttgggttttaaccattagttgctcaggattttaacgtaggcgctggcacgttgttcctgcatccagcttgctgcttcttccgagaacttacggttcatcagcatgcggtatgcacgatctttctgcgcagcgtcggttttatcgacattacgggtatccagcagttcgattaaatgccagccgaatgaagagtgaaccggtgcactcatttgacctttgttcaggcgagtcagggcgtcacggaaggccggatcgaaaatatctggtgtagcccagccgagatcgccgccctggttagcagagcctggatcctgagagaactctttcgctgcggcagcaaaagtcgttttaccactcttgatatcagcagcaatctgttccagtttcacacgggcctgttcgtcagtcatgatcggcgacggtttcagcagaatatggcgagcatgaacttcggtcaccgagatatttttgctttcgccgcgcaggtcgttaactttcagaatatggaagccaacgccggaacgaatcgggccaacaatgtcgcctttcttcgcggtgcttaatgcctgggcgaagatcccgggcaactcctgaatacggccccagcccatctggccgccgttcagcgcctgctggtcggcagaatgagcaatcgccagcttaccgaaatcagcgccgttacgcgcctgatcgacaatggcgcgcgcctggctttccgcttcgttcacctgatcagaggtcgggttttccggcagcgggatcaggatgtggctcaggttcagctcagtgctggcgtcgttttggttacccacctgctgcgccagggattcgacttcctgcggcaggatggtgatgcgacgacgcacctcgttgttacgcacttcagagataatcatctctttgcggatctggttacgataggtgttgtagttcagtccatcgtaagccagacggctgcgcatctgatccagcgtcatgttgttctgtttcgcgatgttagcaatcgcctgatccagctgctcatcggagattttcactcccattttctgccccatctgcaggatgatttgatccatgatcaaacgttccatgatttggtggcgcagcgtcgcgtcatcaggaagttgctgccttgcctgagcagcgttcagttttaccgactgcattaatccatcaacgtcgctttccagcacgacgccgttattgacgacggctgcgactttatcgactacctggggggcagcgaaactggtattcgcgatcatggcgataccgagaagcagcgttttccagttcttcatactttttccatttcaattaaccgcactgcggattacgtggtaaatcaacaaatcacaaagtgttttgatacggcagaatgttcgaacgcagcatctcttgcgtacccagaccgtagttggagctcaggccgcgaagttcgatgttaaagccgattgcgttgtcatataccgcatgttgtttatcgttatcccaaccgttcagcttccgctcgtaaccgacgcgaattgcatagcagcaggagctgtattgcacacctaacatagagtcggcttgcttgttagcattggtgtcgtagtagtaggccccaacaatggaccaacgatcggcaattggccagctggcgacagcacctacctgcgaaataccattcttatattgctcagcagtggaatagtacttaggcagcgtagcctgaatatattccgggctggcgtaacggtaattcagctgtaccagacggtcttcatcccgacggtattcaatgctggagttactggtcgctacgttatccagacgtgtatcgtactgaatcccgccacgcaatccccaacgctcggagatacgccagtaagtatcgcctgcccacaccagtgaacccgttttgtcgtcattctcccatgttatgttgtcatcgccagtgcgagactccgtgaaatagtagatttgaccaacggaaatattaaaacgttcaacggcagcatcatcatatatgcgagatgtgacaccggtcgtcacctggttagcggaggcaatacggtcaagaccgccgtaagtccggtcccggaacaggccagagtagtcagattgcagcagagacgagtcgtagttatagatgtcgctctgatcgcgatacggcacgtacaaatactgcgcgcgcggttccagcgtttgggtataacccggagccagcatttccatatcgcgttcaaagaccattttgccgtcaactttgaattgcggcattacgcggttaacggattcgtccagcttggtcgtgtttctggagttataccagtcaagattggtttgctgataatgggttgccagcaacttcgcttcggtattgatgctgccccagttattagagagcggcaaattgatggtcggttccaggtgaacacgggttgcttcaggcatgtcgtctctggtgttaacaaagtgcactgcctggccgtaaatacgcgtatcaaacggaccaacatcattctggtagtaattaacgtctaactgcggctctgccgagtagctactggtgttctgttcgctgaaaacctggaactgcttggttgaaacggtggcattgaagttttgcaccgcatagccaacgctgaatttttgcgttgcgtagccgtcagtactggaaccgtacttgttatcgaaatcattgaagtagctaggatcgctgaccttggtgtagtcgacgttgaaacgccacacctgatccatgaccccggagtggttccagtagaataaccaacgacgtgaactgtcatcgttcgggtgttcatcttcatagactttatctgaaggcagatagtccagttccatcaagccagcgcccgcctgggagaggtagcggaattcgttctcccacatgatgttgccacgacgatgcatataatgcggcgtgatggtggcatccatatttggcgcgatgttccagtaatatggcaggtagaactcaaagtagttggtggtggtgtacttggcgttcgggatcaagaaaccagagcgacgtttgtcacccaccggcaactgcaaataggggctataaaagatcggtaccggacccaccttaaagcgggcgttccagatctccgcaacttgttcttcgcggtcatgaataatttcgctacctaccacgctccaggtgtcagaacccggcagacaggaggtaaagctaccgttatccagaatggtatagcggttttcgccacgttgtttcatcaggtccgctttaccgcgaccctggcgacccaccatctggtaatcaccttcccagacgttggtatctttggtgttcagattcgcccagcctttcggccctttgaggatcacctggttatcgtcgtaatggacattaccgagcgcatcaacggtacgtaccggctccggttgtcctggtgcctctttttgatggagctgcacttcgtcggcctgcagacggctgttaccctgcatgatatccacgctgccagtaaacacggcgtcatccgggtagtcccctttcgcgtggtcagcattgatagtcacgggtaagtcattggtatcgccctgtaccagaggacggtcatagcttggcacgcccaacatgcactgtgaggcgaggtcggctgccagtccctgttgactataaagggcggtggcaatcatggtggccaggagagtggggatacgttttttcatacgttgattttattgttccatcatcggtaacgttgcgcgtgacaaacggtcagagactaacgtactcgtcatctctacgctagtgttaatcctgtccgaatagcgtcagtggtgttaggcacggcattgaatgacaggtatgataatgcaaattataggcgatgtcccacaattgaccgcagccggaaaacggtaaaagcacctttatattgtgggagatagccctgatatccgtgtgtcgatttggggaatatatgcagtattggggaaaaatcattggcgtggccgtggccttactgatgggcggcggcttttggggcgtagtgttaggcctgttaattggccatatgtttgataaagcccgtagccgtaaaatggcgtggttcgccaaccagcgtgagcgtcaggcgctgttttttgccaccacttttgaagtgatggggcatttaaccaaatccaaaggtcgcgtcacggaggctgatattcatatcgccagccagttgatggaccgaatgaatcttcatggcgcttcccgtactgcggcgcaaaatgcgttccgggtgggaaaatcagacaattacccgctgcgcgaaaagatgcgccagtttcgcagtgtctgctttggtcgttttgacttaattcgtatgtttctggagatccagattcaggcggcgtttgctgatggttcactgcacccgaatgaacgggcggtgctgtatgtcattgcagaagaattagggatctcccgcgctcagtttgaccagtttttgcgcatgatgcagggcggtgcacagtttggcggcggttatcagcagcaaactggcggtggtaactggcagcaagcgcagcgtggcccaacgctggaagatgcctgtaatgtgctgggcgtgaagccgacggatgatgcgaccaccatcaaacgtgcctaccgtaagctgatgagtgaacaccatcccgataagctggtggcgaaaggtttgccgcctgagatgatggagatggcgaagcagaaagcgcaggaaattcagcaggcatatgagctgataaagcagcagaaagggtttaaatgaccctgtaaatgatgctgagtaactgcccacgattaaaggtggccgccctggcggtcacttctttgagaaaaggcgtttactcagaatggtggacaggctcaatgcacggtttacgggaggggttctgtaggttttatcgcgttgaccctgcttaaggttgagagctttacgacgagcggaattatatttttacgtcttaaaaataaaaaacacatacctgaatgagcgatttttgaaagtatatttattcagaacgcgcatcatgagtttttaactcaatgcgaggctattaccatgaaagtatcagttccaggcatgccggttacacttttaaatatgagcaagaacgatatttataagatggtgagcggggacaagatggacgtgaagatgaatatctttcaacgcttgtgggagacgttacgccatctgttctggtcagataaacagactgaggcttataaacttctgttcaatttcgtgaataaccagactggcaacatcaacgcctcagaatactttactggggctatcaacgagaatgagagagaaaagtttatcaatagcctggaattattcaataaacttaaaacatgcgcaaaaaatccggatgagttggtcgcaaagggcaatatgcgctgggtcgcccagaccttcggggatatcgagttaagtgtcacttttttcattgaaaagaataagatatgtactcagacgttgcagctgcataagggccaaggtaacttgggcgttgatcttagaaaggcttaccttcccggcgttgacatgagggattgttaccttggtaaaaaaacaatgaaaggtagcaatgatatcctttatgagagacctgggtggaatgctaacctgggcgtgctaccccggacggtgctaccccggacggtgctaacccggacggtgctaacctggacggtgctaccgtgaacggtgctacctccttatatgatgaggtaattattattaataaaatcccccccaaaaaaattgatactaaaggagttgctactgaagaagttgctactaaaaaagtactgctgaacaaattactgacaacgcaattattgaatgagccagaataagctaaggttgaaggggctggaacgccccttcaaccttagcagtagcgtgggatgatttcacaattagaaagacctgcatgatgagctagagaagaggctagtgacgcaaggcgtcgtgcaggacacggatcaccgagatgggcatcgccaaccagactgctaattagcccatgaataacaatcagaaaggaccataacagacccgttaaaatgaaatataagagacggtcaacgggtgaagaaaaagttcaaaaattcgctgtggagcaggaagggaattaccgaatggaaagcgtagccacacgcaacaactgaaagcagtttggcagaaacaaaaaatccccggactcggggatttatgtacaagaggcagcccttaggatgagggtataaacgtacaggaaaggttaaaaatccgctggcgctttaaacgtcatactattgccatacgccggatgggtaatcgtcaacatctctgcatgtagcaacaaacgtggtgccatcgctctcgcttctggtgatgcataaaaacgatcgccgagaatcggatgacccagcgccagcatatgcacacgcaattgatgcgaacgcccggtaatcggttttaacaccactcttgccgtgttatccgccgcatactccaccacttcatattccgtctgcgcaggtttacccgtttcgtaacagactttctgtttcgggcggtttggccagtcgcaaatcagcggcagatccaccagaccttctgcgggggatggatgcccccagacgcgggccacatactgctttttcggctcgcgctcgcggaactggcgttttaactcccgctccgcggctttggtcagcgccactacaatcacgccgctggtagccatatccagacgatgcaccgattctgcctgcggataatcacgctgaatgcgcgtcatcacgctgtctttgtgctcttccagacgacccggcactgacaacaaaccgctcggcttgttgaccaccataatatggtcatcctgatacaggataaccaaccagggttcctgcggtggattgtagttttccatccccattttcggctccgttactgatgcgttacaacgatcaaacgcagggcatccagacgccaacctgcctgatccaggctttccattacctgctgacggttgctctcaatggcggtcagttcgtcgtcacgaatgttcgggttcactgcacgcagagcttccagacgagacagctcggcagacagtttttcgtcggcttcgttacgcgctgcatcaatcaatgcacgggcagatttctcgatctgcgcttcacccagttgaaggatagcgtgaacatcctgctgcacggcgttaaccagtttgctgccggtgtgacggttaaccgcgttaagctggcggttaaaggtttcaaactctacctgcgccgccaggttgttgccgtttttatccagcagcatacgtaccggcgtcggtggcaggaagcggttgagctgcaactgcttcggagcctgggcttcaaccacataaatcagttccaccaacagcgtacctaccggcaacgctttgttttttaacagtgaaatcgtgctgctaccggtatcgccagaaaggatcagatccagaccgttgcggatcagcggatgctcccaggtaataaactgtgcatcttcacgcgccagcgccacttcacgatcaaaggtgatggtgatgccatcttccgacaggccagggaagtccggcaccagcatatgatcggacggcgtcagcacgatcatgttgtcgccgcgatcgtcctgattgataccgataatatcgaacaggttcatggcgaaggcgatcaggttggtatcgtcatcctgctcttcaatgctttctgccagtgcctgggctttttcgccaccgttggagtggatttccagcaggcggtcacgaccctgttccagctgtgctttcagcgcttcatgttgctcgcggcagtttttgatcagatcgtcaaagccttcggtttgatccggtgaagccagatagttaatcagatcgttgtatacgctatcgtaaatagtgcgtccggtcgggcaggtgtgctcaaatgcatccagaccttcgtgataccagcgcaccagcaccgactgagcggttttctccagataaggcacatggatctgaatatcgtgcgcctggccgatacgatccagacgaccaatacgctgctccagtagatccgggttgaatggcaggtcaaacatcaccatgtggctggcgaactggaagttacgtccttcagaaccgatttctgagcacagcagtacctgtgcgccggtgtcttcttcggcaaaccaggcggcagcgcggtcacgttcgataatcgacataccttcgtggaacaccgcagcgcgaataccttcacgttcgcgcagtacctgctccagttgcagcgcagtggcagctttggcgcagatcaccagcactttctgagagcgatggctggtcaggtagcccatcagccactcaacgcgcggatcgaagttccaccaggtggcgttatcaccttcaaattcctgataaatacgctccgggtagagcatatcgcgagcacgatcttccgcacttttacgtgcgcccataatgccggagactttaatagccgtctgatactgcgtcggtagcggcagcttaatggtgtgcagctcgcgtttcgggaatcctttcacaccgttacgcgtgttacggaacagcacgcggctggtgccgtggcgatccatcagcatcgaaaccagctcctgacgggcgctctgggcatcttcgctgtcgctgtttgctgcctgcaacagcggctcgatatcctgctcgccgatcatctcgccgagcatgttcagttcgtcattgctcagtttgttacctgccagcagcatggcaacggcgtccgcaaccggacgataatttttctgctcttcaacgaactgcgcaaaatcgtggaaacggttcgggtccagcagacgcagacgggcgaagtggctttccatccccagctgttccggggtcgcggtcagcagcagaacgcccggcacgtgctctgccagttgttcaatggcctgatattcacggcttggcgcatcttcgctccacaccaggtgatgcgcttcatcgaccaccagcaggtcccattcggcttcacagagatgttccaggcgctgtttgctacgacgggcaaaatccagcgagcaaatcaccagctgttcggtgtcaaacgggttgtaagcatcgtgctgagcttcggcataacgctcatcatcaaatagcgcaaagcgcaggttgaaacggcgcagcatttctaccagccactgatgctgtaaggtttccgggacgataattagcacacgttcagcagcgccagagagcagttgctgatgcaggatcatcccggcttcaatggttttccctaaacccacttcgtcagccagcaggacgcgcggcgcgtggcggcgaccaacatcatgagcgatgttgagctgatgcgggatcaggctggtacgctgaccgcgcaggccgctgtacggcatacggaactgttcgctggaatatttacgcgcgcgataacgcagcgcaaagcggtccatacggtcaatctgcccggcaaacagacggtcctgcggtttgctgaacaccagtttgctatcaaggaaaacttcacgcagggctacgccggactcttcagtatccaggcgagtaccgatataggtcagcaagccattttcttcttttacttcttcgacttgcatctgccagccgtcatggctggtaatggtatcaccagggttgaacatcacgcgggtcacgggggaatcactgcgtgcgtacagacggttttcaccagtagatgggaaaagtaaagtgacagttcgcgcatccaccgcgacaacggttccaagtcccaattcgctttctgtatcgctgatccagcgttgaccaagtgtaaaaggcatatgtgttcggctctatatctttaattgcaggcaataaccacccgctaccgtgcttatgaggtagtggtgttattcaggtccaggaatggaaagggcgctatggtactggatggcaaagcattcgtcacgcatcaaaatggtatctggcgaactcttttttttgctcaaaatagcccaagttgcccggtcataagtgtagcaaaattatcctcaataaaagggagtattccctccgccacgggttgtagctggcgggtcagatagtgttcgtaatccagtggtgaacgttggtagtccagcggctccgggccgttggtggtccatacgtacttaatggtgccgcgattctgatattgcaaggggcgaccacgcttttggttttcttcatcggcaaggcgagcggcgcgtacatgaggcggcacattacgctgatactcgctcagcggacggcgaaggcgtttacggtaaaccagtcgcgcatccagttcacccgccatcagtttgtcgatggtttcgcgtacatattcctgatatggctcgttgcggaagatgcgcaggtatagctcctgctgaaactgctgggccagcggcgtccagtcggtgcgcacggtttccagccctttaaacaccatccgctgcttgtcgccctcctgaatcagtccggcataacgctttttactgccggtatcggctccgcgaatggttggcatcagaaaacggcagaaatgggtttcatactccagttctaatgcgctggtcagccgttgtttttgcagcgtttccgcccaccaggcgttaacgtgctgcaccagtgcacgaccgattttcgccgcttcttcttccgaatgtgcgcctttcagccagacaaacgttgagtcggtatcgccgtagataacgtcgtagccctgtgcttcaatcaacgctttggtttgccgcatgatctgatgaccacgcatggtgatcgacgatgccagccgcggatcgaagaagcggcaggcggtggtgccgagcacgccataaaaggcattcatgatgattttcagcgcctgcgacagcggtttgttaccctggcgtttggcttcatcgcgcccgtgccagatgttagtcacaatctccggcaggcaatgtttttctcgcgagaaccaggcatcgagaaaaccttcggtactgtgctctggatcaggctgcgccatgccttccaccagcccgacgggatcaatcagaaaggtgcggatgatcgacgggtacaggcttttatagtccagcaccagcactgaatcataaagccctggccgtgaatccatcacgtagccgccagggctggcgtgcggcggcacttcgccgagattaggcgcgacataaccagcgcgatgcattcgcggaaaatagagatgaccaaatgccgccaccgaaccgccgtgtcggtccaccggcaggccgttcaccgttgcccgttcgagtaaaaatggcatgatttcagttttgtggaagatctgcgtcaccagctcgcaatctttcaggttataagttgccagcgcaggtttatcttcggcgaaacggcggtcaatttcgtccattcgatcccacgggttatcgatagattttccttcgcctaatagctcctgagcgacagtttccagcgagaatgaagagaaattccagaacgcggatttcagcgcctcgataccgtcgataattagccgacctttagcctgggcaaaaaagacgccgtttttaaagccgtgctcgcgccactccagctcgctattatcgcgcccaagacgcagcggaagacggtaacgctcggcatgtttttgcagcattcgcagatcgaactgcaccacgttccaaccgatgatcacatcaggatcgtagttggcaaaccaggcgttgagtttttccagcaactgcgggcggctggcgacgtattccagttcgaaatcaagcgaggaggcgtcgccattctccggccccagcatataaacgatgcgctgcccgcagccttccaggccgatgcagtacagctcaccgtggcgggtggtttcaatatctatagaaacccacttgagcggcggacgatagtcgggatgcggtttcagacgggcattaacgatagtgccattgtgcatatcaccctcgacccacaccggtgaggtgataaaccgctccatcagatagcgttctggcggacgcacatcggcctcgtagacggtaacgccaccttcacgcaggcgcttttcgtaattcatcaattggcgatgggcgcgacagtaaaggccatacaccggctggcggtgaaaatcctttaacgccagcggtgtcaggcgaaagccttgttcaccctgcaaaatatgctgagcgcggggaacctgatcggcgggaataaacgccacggactcttgcggtgcaagcgtaacctgcaacggcccgttgtccgtcgccagccagaaggagacttctgtcccttgcggggtgtcccgccagtgtcgggttaagataaaacctgcctgcgccacgctgaaaatccatcaaaaaaccaggcttgagtatagcctggtttcgtttgattggctgtggttttatacagtcattactgcccgtaatatgccttcgcgccatgcttacgcagatagtgtttatccagcagcgtttgctgcatatccggtaactgcggcgctaactgacggcagaatatccccatataagcgacctcttccagcacgatggcgttatgcaccgcatcttcggcatttttgccccatgcaaacgggccgtgggaatggaccagaacgccgggcatttgcgctgcatcgataccctgtttttcaaaggtttctacgatgacgttaccggtttcccactcatattcgccgttgatttctgcgtcggtcattttgcgggtgcagggaatggtgccgtagaaatagtcggcgtgggtggtgccggttgctggaatcgactgacccgcctgcgcccagatggtggcgtggcgcgagtgcgtatgcacaatgccgccaatggaggggaatgcctgatagagcagccggtgagttggcgtgtcggaggagggctttttcgtaccttcaaccacttcaccggtttcgatgctaaccacgaccatatcgtcagcggtcatgacgctgtaatcgacgccggaaggtttgatcacaaagacgccgcgctcgcgatcaacggcgctgacgttgccccatgtgagcgtgaccaggttgtgttttggcagcgccaggttggcttctaatacctggcgtttgagatcttctaacatgttgactccttcgtgccggatgcgctttgcttatccggcctacaaaatcgcagcgtgtaggcctgataagacgcgccagcgtcgcatcaggcgttgaatgccggatgcgctttgcttatccggcctacaaaatcgcagcgcgtaggcctgataagacgcgccagcgtcgcatcaggcgttgaatgccggatgcgctttgcttatccggcctacaaaatcgcagcgtgtaggccagataagacgcgtcagcgtcgcatcaggcgttacataccggatgcggctacttagcgacgaaacccgtaatacacttcgttccagcgcagcgcgtctttaaacgctggcaggcgtgtgtcgttatcaatcaccgtgatttcaatgtcgtgcatctcggcgaattggcgcatatcgttgaggttcagtgcatggctgaagacggtatggtgcgcgccaccagcgaggatccacgcttcggaagcagttggcagatccggttgcgctttccacagcgcattcgccaccggcagtttcggcagggagtgcggtgttttcaccgtgtcgatgcagttaaccagtagacggtaacgatcgccgagatcaatcaagctggcgacaatcgctgggccggtttgggtattgaagatcaggcgggcaggatcgtccttaccaccaataccgagatgctgaacgtcgaggatcggtttctcttctgcggcgatcgacgggcagacttccagcatatgggagccgagcaccaggtcattacctttctcgaagtgataggtgtagtcctccataaaggaggtgccgccctgcagaccggttgacatcaccttcatgatgcgaagcagggcggcagttttccagtcgccttcgcccgcaaagccgtaaccctgctgcatcagacgctgtacggccagaccaggaagctgtttcagaccgtgcaaatcttcaaaggtggtggtgaacgcgtggaagccaccttgttccaggaaacgcttcatccccagctcaatacgcgccgcttccagcacgttctgtcgttttttgccgtggatttgtgtggcaggcgtcatggtgtagcagctttcgtactcatcgaccagcgcgttaacatcgccgtcgctgatggagttcaccacctgcaccagatcgccaaccgcccaggtattgacggagaaaccgaacttgatctgtgcggcaactttatcgccatcggtgaccgccacttcacgcatgttatcgccaaatcggcagactttcagatgacgggtatcctgtttagagaccgcctgacgcatccaggagccgatacgctcatgggcttgtttatcctgccagtgaccggtaaccacggcatgttgctgacgcatacgcgcgccaatgaagccgaactcgcgaccgccatgtgcagtctggttcaggttcataaagtccatatcgatactgtcccacggcagcgccgcgttgaactgggtgtggaattgcagcaacggtttgttgagcatggtcaggccgttgatccacattttggccggggagaaggtgtgcagccacaccaccagaccagcgcaacgatcgtcgtaattcgcgtcgcggcaaatagcggtgatttcatccggcgtggtgcccagcggtttcaacaccagtttgcagggcagtttcgcttccgtattcagcgcattaacgacgtgctcggcatgttgggtgacctgacgcagggtttccgggccatacagatgctggctgccaatgacaaaccacacttcataattatcaaaaatcgtcattatcgtgtccttatagagtcgcaacggcctgggcagcctgtgccggggcggaagttggaagatagtgttgttcggcgctcatcgcccattgctgatagcggcgataaagctgttcaaagcgttgtgcctgctcgctgcacggttgcagggttttctctaccgcactggccattttttgctgagctgatgggatgtctgcgtgcactttcgcggcgacggcagcaaaaatcgccgcaccgagcgcacagcactggtcagaggcaacaatttgcagcgggcgattcagcacgtcgcagcaggcctgcataatgacctggtttttccgcgcgatgccgcccagtgccatcacgttattaacggcgatcccctgatcggtaaagcactccatgattgcgcgtgcgccaaaggcggtggcagcaatcaaaccgccgaacagcagcggagcgtcggtagcgaggttaagatcggtaatcacccctttcaggcgttggttagcgttcggtgtgcggcggccgttaaaccagtcgagcaccaccggcaggtgatccagagacggatttttggcccatgcttcggtcagcgccggaagcagttgtttctggctggcgttgatttgcgttttcagttccggatgctgggcggcaagctgttccagcggccagccgagtacgcgaccaaaccaggcgtagatatcaccaaacgccgattggcctgcttccagaccgataaatccaggcaccacgctgccatcaacctgaccgcaaatacctttaactgcccgctcgccaacgctctgtttgtcggcaatcagaatgtcgcaggtggaagtaccgataacttttaccagtgcgttaggctgtgcgcctgcgccaactgcgcccatatggcagtcaaacgcgccgccggaaatcaccacgctttcaggcaggccgagacgctgcgcccattccgggcataaggtgcccaccggaatatcggcagtccaagtgtcagtgaacagcggggaaggcaaatggcgattgaggatcgggtccagctcatcaaagaaactggctggcggcaggccgccccagctttcgtgccacagagatttatgcccggcgctgcaacgtccgcgacgaatatcctgcgggcgggtggtaccggaaagcagagctggcacccagtcgcacagctcaatccacgatgcggcagattgcgccacggcgctgtcctggcgagtcacatgcaggatttttgcccagaaccattcgctggaataaataccaccaatgtagcgggagtagtcaacgttgcccggcgcgtggcacaaacgggtaatctcttccgcttcttcaaccgcagtgtggtctttccacaatacgaacatcgcgttcgggttttcggcaaactccgggcgcagcgccagcacgtttccgtcggcatcaatcggtgcgggcgtcgagccggtactgtcaacgccaatcccgaccacagctgcgcgctgttcgacgctaagctctgcaagcacggttttcagtgccgcttccattgactcaatgtagtcacgcggatgatgacggaactggttattcggggcatcacaaaattgccctttctgccaacggggataccactctacgctggtggcgatctcttcaccggtagcgcagtccaccgccaaagctcgcacagaatcactgccaaaatcgaggccaattgcaatcgccatcgtttcactccatccaaaaaaacgggtatggagaaacagtagagagttgcgataaaaagcgtcaggtaggatccgctaatcttatggataaaaatgctatggcatagcaaagtgtgacgccgtgcaaataatcaatgtggacttttctgccgtgattatagacacttttgttacgcgtttttgtcatggctttggtcccgctttgttacagaatgcttttaataagcggggttaccggttgggttagcgagaagagccagtaaaagacgcagtgacggcaatgtctgatgcaatatggacaattggtttcttctctgaatggtgggagtatgaaaagtatggctgaagcgcaaaatgatcccctgctgccgggatactcgtttaacgcccatctggtggcgggtttaacgccgattgaggccaacggttatctcgatttttttatcgaccgaccgctgggaatgaaaggttatattctcaatctcaccattcgcggtcagggggtggtgaaaaatcagggacgagaatttgtctgccgaccgggtgatattttgctgttcccgccaggagagattcatcactacggtcgtcatccggaggctcgcgaatggtatcaccagtgggtttactttcgtccgcgcgcctactggcatgaatggcttaactggccgtcaatatttgccaatacgggtttctttcgcccggatgaagcgcaccagccgcatttcagcgacctgtttgggcaaatcattaacgccgggcaaggggaagggcgctattcggagctgctggcgataaatctgcttgagcaattgttactgcggcgcatggaagcgattaacgagtcgctccatccaccgatggataatcgggtacgcgaggcttgtcagtacatcagcgatcacctggcagacagcaattttgatatcgccagcgtcgcacagcatgtttgcttgtcgccgtcgcgtctgtcacatcttttccgccagcagttagggattagcgtcttaagctggcgcgaggaccaacgcattagtcaggcgaagctgcttttgagcactacccggatgcctatcgccaccgtcggtcgcaatgttggttttgacgatcaactctatttctcgcgagtatttaaaaaatgcaccggggccagcccgagcgagtttcgtgccggttgtgaagaaaaagtgaatgatgtagccgtcaagttgtcataattggtaacgaatcagacaattgacggcttgacggagtagcatagggtttgcagaatccctgcttcgtccatttgacaggcacattatgcaagcattgctggaacactttattacccaatccaccgtgtattcattgatggcggtggtgttggtggcctttctggagtcgctggcgctggtcggtttgattctacccggtacggtgctgatggcggggctgggagcgctgattggcagcggcgagttaagtttctggcacgcctggctggcagggattattggctgcttgatgggcgactggatttctttctggctgggttggcgttttaaaaagccgttgcatcgctggtcatttctgaagaaaaacaaagcactacttgataaaactgaacatgcgttgcatcaacacagcatgttcaccattctggtcggtcgttttgttggcccgacgcgtccgctggtgccaatggtggcgggaatgctggatctgccggtggctaaatttattacgccgaatattatcggctgcctgctgtggccgccgttttacttcctgccagggattctggcgggcgcggcgatcgatattcctgccggaatgcagagcggtgagtttaaatggttgctgctggcaacagcggtgtttttgtgggttggtggctggctgtgctggcggttatggcgcagcggtaaagcgactgaccgtttgagtcattatttgtcccgcggtcgtttgttgtggctgacgccgttgatttctgccatcggcgtggtggcgctggtggtgttaattcgccacccgttgatgccggtgtatatcgatattttgcgtaaagtggttggggtttaggagatagtcttgtgcgggttgcctgatgcgacgcttgccgcgtcttatcaggcctacaaaacgcactacccgtaggtcggataaggcgttcacgccgcatccgacagtgcatactaacccgtaatccccaatagtgccgaagcactcgccttaccgctcaacaactcattggtcataccctgccaggcgatgcgcccgtcggcgactactaccgagcgcgtggcgatccgcgccgcatcttccacgctgtgcgacaccatcaatagcgtcattttttgctgctggcagctcgtgctcaccagcgtcaacatctcctgacgtaacgccggatcgagcgcagagaacggttcatcgagcaataaaatcggctgttcgcgtaccagacaacgcgctaacgccactcgctgtcgctgaccgccggaaagctcgcccggtaaccgcgccattaaattatcaatccccatctggcgggcgatagcgtgcattttcccctgctgtaccgcgttcagtttcaatcccggatttagccccagcccgatgttctgtgcgaccgtcaggtggctgaacaggttgttctcctgaaacagcatcgacaccggacggcgtgacggcggcatagttgtgtgatctacgccatcgatagtcagcgaaccgctggctggcgtcagaaaaccggcgatcaaattcagcagggtacttttacccgcgccgcttggcccgaggatcgccacctgctcgccgcgttccaccgttaagctaaaacgcatcggcaaatggtggtaaagccaggtgatatcagtcagttttaacatttcgccccggtagtttttcaatcacggtaaacagcagaaaacagagcagcagcagaattaacgcggtgaccgcaccgtcctggctgcgataggagccaatttgctggtagagataaaacggcagggtgcggaaatcatcgttaccgaacaacgccaccacgccaaaatcaccaatcgacagcacgcatgcaaaggccagcgcctgcgccagtggacgtttcagggcgcgcagctccaccacttttaagcgtgaccagccttcaatccccagcgactgacataacatgctgtagcgggcggtgatatcgcgcatcgggttttccagcactttcagcgcataagggatcgccattaacgcattggtgaaaatcacaatgccgtcagcagattgtggcaggccgatagtgttgttgagcagtaaaaagaagccggtagccagcacaatccccggcatggcgaggatcaacatgccgctcatctccagcacctgacccgccagcattttctgccgcgcccgcagttcgcgactgctccatagcagcatcatggtcagcactacgcacaatacacctgccgccagcgcaatacgcaacgaggtccacagcgcctgccacagcaccggttgtgccagcacttccggcaactggcgatttaccccatcgacgatcaccgccagtaacggtggcagcaacagcagcagcgccagcacaattaacaccgtgtcgcaaatgcggctatgcagacgatcgtccgggtcgcgccagccttgcagcagcgtggtgccgggcgcaatggccttactcaatcgctgactcaacagcaccagcccgaggcagcacaccatctggagcagcgccagcattgccgcgcgggcaggatcgtagtcgtaactcagcgcctgatagattgccagctcgatagtggtcgcctgcggaccgccccccagcgatagcacggtggcgaagctggcgaaacagagcataaagataagcgcagcaaccggcgggatttgtcgccgtaaccacggccattcgacgaagcggaaaaaatgccagctacgcatcccaagctgggcggcaagttgacgctgttcgccggggatgttttccagtgcctggagtaataagcggctcgccatcggcagattaaaaaacacatgggccagcaaaataccttgcaggccgtagggcgaaaaggtccactccagaccgagcgattggcagagtgttgccagccagccctggcgaccatagacgctaagaatgccgaaaacagcgaccaacaccgggaggatcaaggtcattgcacacagacgcaacagcgccagccgacccggaaagcgcctgcgatagagcgcgcgggcgaggaatatcgcgggtatgacagagagcagtgccgagagaaacgcctgccagaaggagaagcgcaccacatgccacagatagctgtcctgccagactgccacccagtcatcctgcggcgcgttccaccacagggcgagaaacgccgccagcgcaaccgctaccaccagcgtggtggcgcttacacctggaattaaccagccgggaattaacggctgacggcgcgttgccattcgctaatccatgcctgacgttgtgccgccacttcggctggcgtgaactccaacgtggttgcgggtttggtcaatttttcaaaaccggcaggcagcgtgacgtttgccaccggatacatccagttgccggttgggatcgcattctggaaagccggagaaaccataaactggaggaatttttgcgccagctccggctgcttgctggcagcggtgcgggcggcgacttccacttgcagatagtgaccttcgctgaagttcgcggcggcgtagttatctttcttctcttcgagaatgtgataagccggagaggtggtgtaactcagtaccagatcgctttcaccttttaaaaacaggccgtaggcttcgctccagcctttggtgaccgtgaccgttttcttcgccagtttctgccaggcttgtggggcgtcatcgccatagactttttgcatccatagcaacagacccagccccggtgtactggtgcgcggatcctgataaatcacccgccagttttgatcgctctcaaccagttctttcaggctttgtggcgggtttttcagtttgttcttgtcataaacgaaggcgaagtagccataatcaaacggtacgaaagtgtcattattccagccgccgggaacgttaacggcatccgctgccacaccgcttttggcaaacagtccggttttactggcggcgtctaacaggttgttatccagccccagcaccacatcggctttactgtttttgccttccatccgtagacggttgagaagcgaaacgccatcttccagcgccaccagtttcagttcgcaattacagtcggcttcaaaggcttttttaaccaccggaccaggcccccagtcggcggcgaaggaatcgtaggtataaacagtcagaacgggtttagcgaaaacgggcgctgtgcacagcaacagcaggggcagacatttttttaacactttgcacctcaaaaaagagtggcaaaggacttgagaaggagcctcaaatcccttcgccggcgttatccggatcaggttcgacgggtattttctcagcgcacgcgtacgcgtggcaccccgttgagaacggcgttagtgtagtgattttgttatcaaccagcaatcatggatccggtggcgcaaaccacgctgatttaaaatcgaaccagccgagggtattcatgcgcaggccgcgcatactgcgttgcccctgaatgatcagccagtggtgcaataatggcaccatcgctttgctggcgaccagttgctggcaccagttcgccagattcatctcgccattgcgccagcgagcagcgtcggcttgccagtcaatgggaatgcaatgttgtagcagtggcacttcgcataaatgtgcgaaaacagagaagtccagcggcagggtaaagttggcgctgtttagccagatatcactttcgatctctcctgtatgccactgatcgtagtcgatctctttgattttcagcgtgacctggtgacttgccagaatctgctgcatgatcccggcaatcacccgatgctcactgtgatcctgataaaaggttagggtgaggctttccaggccagccggtttttcgctctttatggtgcgggcatggtgccaacgggggagcagtccataagccgggaaccacagttgctggtactgttcctcagcgaaatagaccagattagttggagaaagcacatagcttacccagtccctgacttgctgattcgccccgcgatgggtgcggctgtcgaacagtaaatagtagcaaccttcctccaggcggctttcaatctctttttcctcgccctgtggaccttttagcatcagccctccggctggctcgtcggcaatttccggcagaacccagacgttaacttcgtcgattaatgcccggtaaccgaagaagtcatcgaatgcctgaattttcagttgattggtgctgttgcgaatcaccgcatacggaccggtgccgatgggatggctggcaaagttactgagggtttcccattcgcgcggcaggatcatcgccggaacttgccccagcagtaacggtaaccagcggtccggttgcgtgagatggatatccagcgtccagggcgtcggcgacacaatgtcagcaatatgcgaatagagcggcagcgtattgattcgttttaaagaggcgatcacatcgtccatttccagttcacgaccatggtgaaaatggactcctggacgcaaaaagaaacgccagtgaagcggtgaaatttgctgccagtggtgggcgatgtctgcttccagttccccattttcctcatttatgcgcgttagcgaactgaagatttgccgggcgatatgggtttcggaacggcgcaatgcgctgccaggtagcagattacgcaacggacgatagtagagcacgcgcaggatgtgccgcccctggcggaagctgcggcccagatgagaaaccagcatttgccgcacagtcgctttgtcgccaaccaactgcaccagttgatcgatacgatcctgctccagcaggtcttccgcccgctgttgctgaagcgccagcccggtatagaggaatgtcagacgcgagcgtttaccgcgcccgacttccgcttcccacgtcagccagccgcgatcctgcatggtgttgagcagggtgcgcatatgacgacgcgagcagctcaataacgctgccagttcgttgagcgttgtgtcctgcgatttaccctcgcagcattgccacaggcggatgaactgttgttgcagacgagcagatggcataaaaggggaactcctgtgcaaaagacagcaattttattttccctatattaagtcaataattcctaacgatgaagcaagggggtgccccatgcgtcagttttatcagcactattttaccgcgacagcgaagttgtgctggttgcgttggttaagcgtcccacaacgattaaccatgcttgaaggactgatgcagtgggatgaccgcaattctgaaagttgacttgcctgcatcatgtgtgactgagtattggtgtaaaatcacccgccagcagattatacctgctggttttttttattctcgccgcgctaaaaagggaacgtatgatctggataatgacgatggctcgccgtatgaacggtgtttacgcggcatttatgctggtcgcttttatgatgggggtggccggggcgctacaggctcctacattgagcttatttctgagtcgtgaggttggcgcgcaacctttctggatcggcctcttttatacggtgaatgctattgctgggatcggcgtaagcctctggttggcaaaacgttctgacagtcagggcgatcggcgaaaactgattatattttgctgtttgatggctatcggcaatgcgctattgtttgcatttaatcgtcattatctgacgcttatcacctgtggtgtgcttctggcatctctggccaatacggcaatgccacagttatttgctctggcgcgggaatatgcggataactcggcgcgagaagtggtgatgtttagctcggtgatgcgtgcgcagctttctctggcatgggttatcggtccaccgttggcctttatgctggcgttgaattacggctttacggtgatgttttcgattgccgccgggatattcacactcagtctggtattgattgcatttatgcttccgtctgtggcgcgggtagaactgccgtcggaaaatgctttatcaatgcaaggtggctggcaggatagtaacgtacggatgttatttgtcgcctcgacgttaatgtggacctgcaacaccatgtacattattgatatgccgttgtggatcagtagcgagttaggattgccagacaaactggcgggtttcctgatggggacggcagctggactggaaataccagcaatgattctggctggctactatgtcaaacgttatggtaagcggcgaatgatggtcatagcagtggcggcaggagtactgttttacaccggattgattttctttaatagccgtatggcgttgatgacgctgcaactttttaacgctgtatttatcggcattgttgcgggtattgggatgctatggtttcaggatttaatgcctggaagagcgggggcagctaccaccttatttactaacagtatttctaccggggtaattctggctggcgttattcagggagcaattgcacaaagttgggggcactttgctgtctactgggtaattgcggttatttctgttgtcgcattatttttaaccgcaaaggttaaagacgtttgatgacgtggacgatagcggaaagcccggtcatttgaccgggcaaggggattaattcataaacgcaggttgttttgcttcataagcggcaatggcgtcgtcgtgctgcaaggtaagcccaatactgtccagaccgttcatcatgcagtggcggcggaaggcatcgatggtaaagcgataggttttctctcccgctttcacctcttgcgcttccagatccacgtcgaaatggatccccggattagctttcaccagcgcaaacagttcgtccacttctgcatcgcttaatttcaccggcagcagctggttgttaaagctattgccgtagaagatgtcagcaaaactcggcgcaatcaccactttaaaaccgtagtcggtcaatgcccagggcgcgtgctcacgcgaagagccacagccgaagttttctcgtgccagcaaaatggaagcgccctgatactgcgggaagttcagcacgaagtccgggtttggctgttggcctttttcatccagaaaacgccagtcgttaaacagatgcgcgccaaaacccgtacgggtcactttctgcaaaaactgtttcgggatgattgcatcggtatcgacattggcggcatccagcggaaccaccaggcctgtgtgtttgataaatttctctgccatggtgtgctccttatttaatgttgcgaatgtcggcgaaatgtccggtcacagcagcagcggcagccattgccgggctgaccagatgcgtgcgcccgccgcgcccctggcggccttcaaagttacggttgctggtggaggcacaacgttcgcccggattcagacggtcgttgttcatcgccagacacattgagcagccaggcaagcgccattcaaaaccggcttcaataaagattttatccagaccttccgcttccgcctgggcttttaccgggccagagccgggaaccaccagtgcctgcacgcctggcgcgacttttcgccctttggcgatctccgctgccgcgcgtaaatcttcaatgcgcgagttggtacaggaaccgataaacactttgtcgatagccacttcggtcagcggaatacccggtttcagccccatataggccagcgctttttctgccgacgcgcgttcaaccggatcggcaaacgaagccggatcgggaatattgtcgttcacggaaatcacctggccgggattggtgccccaggtgacctgcggtgaaatttcttctgcttgcagagtgacaacggtatcgaaagttgcgccttcgtcggtttgcagggttttccagtaggcaacggcgtcgtcgaaatctttgcctttcggcgcatgcagacggcctttgacatagttaaaggtggtttcgtccggtgcaaccagaccggcttttgcgcccatttcgattgccatattgcacagggtcatacgaccttccatgcttaaatcacggattgcttcgccgcaaaactccaccacatgcccggtgccgcctgcgctaccggttttaccgataattgccagcacgatatcttttgcggtaatgcccggcgcggctttgccctggacttcaattttcatggtttttgcgcggccctgtttcagggtttgcgttgccagtacgtgttcaacttcggaagtgccgataccaaaggccagtgcgccaaacgcgccgtgggtggcggtatgcgagtcgccgcagacaatggtcatccccggcaaggtgacgccctgttccggccccattacgtggacgatcccctgatacgggtgattcaggtcatacagttcgacgccaaattctttgcagtttttgatcagttcctgcatctggatacgcgccatttcaccgcaggcattaatgtctttggtctgggtagagacgttgtgatccatggtagcgaaggttttgcccggctgacgtaccgggcgaccgtgggcgcgcagaccatcgaacgcctgcggtgaggtcacttcatgcaccaggtggcggtcgatatataacagtggggtttcgttttcggcttcgtacacaacgtgagcgtcgaacaatttttcgtataacgtcttagccatgattacaccccttctgctacatagcgggcaatgatatcgcccatttcatcggtactaacggcggcagcgccacgggctaaatccccggtgcgaatgccttcttctaatgcgcggttaatggcgcgttcaatggcgcaagccgcatcatcggcatccaggctgtaacgcagcagcagtgccagcgaaaggatttgtgcaatcgggttggcgatgtttttgcctgcgatatctggtgccgagccgcccgccggttcatacagtccaaaaccttgctcgttcaggctggcggaaggcaacatccccatcgagccagtgatcattgcgcactcgtcagacagaatgtcgccaaacaggttggagcacagcagaacgtcaaactgtgatggatctttaatcagctgcatggtggcgttgtcgatgtacatatgcgccagttcgacatccgggtattccgtggcgatctcgttaacgatctcccgccataaaatagaggattgcagcacgttggctttatcgatcgacgtcactttgtggcgacgcttgcgagcagattcaaacgcgatgcgggcgatacgttcgatctcaaaacggtgatacacctcggtatcaaaggctttttcatattgtccgctaccttcgcggccttttggctgaccgaaatagatgccgccggtcagttcgcgcacacacaggatgtcgaagccgtttgcggcaatgtctgcacgcagcggacagaatgcttccagcccctgatacagttttgccgggcgcaggttgctgaataatttgaagtgcttacgcagaggcagcagcgcgccgcgttctggttgctggtctggtggtaaatgttcccacttcgggccgcctaccgagccaaacagcacggcatcggcttgctcacaaccttcaaccgtcgcaggcggcagtggttgcccgtggttatcaatggctgcgccgcctacatcgtaatggctggtggtgatgcgcatcgcaaagcggttgcgcacggcatccagcactttcagcgcctgggtcatcacttccggaccaataccgtcccccggcaatacggcaatatggtaattcttcgacatcacacggtttccttgttgttttcgttgtgttgagctttgcgttgcaactctttttcgacttctgcggcacgccagatattgttcagaacgtgcaccatggctttggcagatgactcgacaatatcggtagccaggccgacgccgtggaagcggcgaccgttgtagttagcgacgatatccacctgacccagcgcatctttaccgtggcctttggcggtcaggctgtatttcaccagttcgacgttatattcagtgatgcggttaattgcctgatagacggcatcgaccggaccgttaccgttggcggcttctgctttgacttcttcgccacaggccagtttgacggcggcggtggcgatatcgttagagccagactgcacgctgaagtaatccagacggaaatgctccggctcttcttgctgcttaccgatgaaggccagcgcctccagatcgtaatcaaacacctgaccttttttgtccgccagcttcaggaaagcatcgtacaaattgtctaaattatattcactttctttataccccatctcatccatgcgatgtttcaccgccgcacgccccgaacgagaggtcagattcagctggatttggttcagaccaatagattctggtgtcatgatttcgtagttttcgcggtttttcagcacgccatcctggtgtataccggaggagtgtgcgaatgcgccgctgccaacaatggctttgtttgccgggatcggcatattacaaatctggctaactaactggctggtgcgccatatctcctggtgattaatggcggtgtggacgttgagaatatccttacgaactttgatcgccatgatgacttcttccagggaacagtttccggcacgctcgccgatcccgttcattgcgccttccacctggcgtgcaccggcatgtaccgccgccagtgagtttccgaccgccaggcccaaatcgtcgtgggtatgtacggagataatggctttgtcgatgttaggcacgcgttcatacaggccgctgatgattccggcgaactcaaacggcatggtgtagcccacggtgtccggaatgttgatggtggtggcaccggcattaatcgccgcttcgaccactcgcgccagatcggcaatgggtgtacgcccggcatcttcgcaagaaaattcaacatcatcggtgtaattacgggcgcgtttcaccatatagatagcgcgttcgatcacctcgtccagcgtgctgcgcagcttggtggcgatgtgcattggcgaagtggcaataaaggtatgaatacggaaggcttcggcgactttcagggattcggccgccacgtcgatatctttttccacgcagcgagctaacgcacatacgcggctgtttttaacctggcgggcgatggtttgcaccgattcaaaatcgcccggcgaagagacggggaaaccgacttccatcacgtcaacacccatacgctcaagggccagcgcaatttgcagtttttctttcacactcaagcttgcctgtaacgcctgttcaccgtcgcgcaatgtggtatcgaaaataatgacttgctggctcatggtttgggtccttgtctcttttagagcgcctcgcttcgggcataaaaaaacccgcgcaatggcgcgggttttttgtttgactgcgtgctggcttaatgctggatgccgctcactcgtctaccgcgcaaagaagatgcgtttagtagtagtagaccgataaagcgaacgatgtgagtcattaaatcagctccagatgaatgcgatatgcttttagagttactggatacaaaaacggatgtcaaccctgacgcaataaaaacgtcccgccagcgtgagttctgcatccgtaaaattagctaattgtgctgcggtggttaaagtaagcgatattaatttctgcttaactaccgacgcttttcatcggttgacatatttcagcataaatttttgcatctaatcaacgaggaaaaaggggacaaaatgcacgcgttgcaaaacctatcctgatgatttgtattgaattatatgttttgcgattttttttgatattgatttggtgaatattattgatcaattaatgttaagaattaatgcattaaatatataaattaattattaaataagcacatttaatccattttgtagatgattgagtattcgcggtagttatgattagattgttttcgcaacaaaaacattatggattattatgctgtggtaaatgactcattccacggcaatggattctgtttttatcagaacccgtatctttatgttttccgaattttactcattttgctttttcttattttatatgcatgataaatcatattcttcaggattatttctctgcattccaataagggaaagggagttaagtgtgacagtggagttaagtatgccagaggtacaaacagatcatccagagacggcggagttaagcaaaccacagctacgcatggtcgatctcaacttattaaccgttttcgatgccgtgatgcaggagcaaaacattactcgtgccgctcatgttctgggaatgtcgcaacctgcggtcagtaacgctgttgcacgcctgaaggtgatgtttaatgacgagctttttgttcgttatggccgtggtattcaaccgactgctcgcgcatttcaactttttggttcagttcgtcaggcattgcaactagtacaaaatgaattgcctggttcaggttttgaacccgcgagcagtgaacgtgtatttcatctttgtgtttgcagcccgttagacagcattctgacctcgcagatttataatcacattgagcagattgcgccaaatatacatgttatgttcaagtcttcattaaatcagaacactgaacatcagctgcgttatcaggaaacggagtttgtgattagttatgaagacttccatcgtcctgaatttaccagcgtaccattatttaaagatgaaatggtgctggtagccagcaaaaatcatccaacaattaagggcccgttactgaaacatgatgtttataacgaacaacatgcggcggtttcgctcgatcgtttcgcgtcatttagtcaaccttggtatgacacggtagataagcaagccagtatcgcgtatcagggcatggcaatgatgagcgtacttagcgtggtgtcgcaaacgcatttggtcgctattgcgccgcgttggctggctgaagagttcgctgaatccttagaattacaggtattaccgctgccgttaaaacaaaacagcagaacctgttatctctcctggcatgaagctgccgggcgcgataaaggccatcagtggatggaagagcaattagtctcaatttgcaaacgctaactgattgcagaataggtcagacatgaatgtctggtttattctgcattttttattgaatgtagaattttattctgaatgtgtgggctctctattttaggattaattaaaaaaatagagaaattgctgtaagttgtgggattcagccgatttattatcaatttaatcctctgtaatggaggattttatcgtttcttttcacctttcctcctgtttattcttattaccccgtgtttatgtctctggctgccaattgcttaagcaagatcggacggttaatgtgttttacacattttttccgtcaaacagtgaggcaggccatggagatgttgtctggagccgagatggtcgtccgatcgcttatcgatcagggcgttaaacaagtattcggttatcccggaggcgcagtccttgatatttatgatgcattgcataccgtgggtggtattgatcatgtattagttcgtcatgagcaggcggcggtgcatatggccgatggcctggcgcgcgcgaccggggaagtcggcgtcgtgctggtaacgtcgggtccaggggcgaccaatgcgattactggcatcgccaccgcttatatggattccattccattagttgtcctttccgggcaggtagcgacctcgttgataggttacgatgcctttcaggagtgcgacatggtggggatttcgcgaccggtggttaaacacagttttctggttaagcaaacggaagacattccgcaggtgctgaaaaaggctttctggctggcggcaagtggtcgcccaggaccagtagtcgttgatttaccgaaagatattcttaatccggcgaacaaattaccctatgtctggccggagtcggtcagtatgcgttcttacaatcccactactaccggacataaagggcaaattaagcgtgctctgcaaacgctggtagcggcaaaaaaaccggttgtctacgtaggcggtggggcaatcacggcgggctgccatcagcagttgaaagaaacggtggaggcgttgaatctgcccgttgtttgctcattgatggggctgggggcgtttccggcaacgcatcgtcaggcactgggcatgctgggaatgcacggtacctacgaagccaatatgacgatgcataacgcggatgtgattttcgccgtcggggtacgatttgatgaccgaacgacgaacaatctggcaaagtactgcccaaatgccactgttctgcatatcgatattgatcctacttccatttctaaaaccgtgactgcggatatcccgattgtgggggatgctcgccaggtcctcgaacaaatgcttgaactcttgtcgcaagaatccgcccatcaaccactggatgagatccgcgactggtggcagcaaattgaacagtggcgcgctcgtcagtgcctgaaatatgacactcacagtgaaaagattaaaccgcaggcggtgatcgagactctttggcggttgacgaagggagacgcttacgtgacgtccgatgtcgggcagcaccagatgtttgctgcactttattatccattcgacaaaccgcgtcgctggatcaattccggtggcctcggcacgatgggttttggtttacctgcggcactgggcgtcaaaatggcgttgccagaagaaaccgtggtttgcgtcactggcgacggcagtattcagatgaacatccaggaactgtctaccgcgttgcaatacgagttgcccgtactggtggtgaatctcaataaccgctatctggggatggtgaagcagtggcaggacatgatctattccggccgtcattcacaatcttatatgcaatcgctacccgatttcgtccgtctggcggaagcctatgggcatgtcgggatccagatttctcatccgcatgagctggaaagcaaacttagcgaggcgctggaacaggtgcgcaataatcgcctggtgtttgttgatgttaccgtcgatggcagcgagcacgtctacccgatgcagattcgcgggggcggaatggatgaaatgtggttaagcaaaacggagagaacctgattatgcgccggatattatcagtcttactcgaaaatgaatcaggcgcgttatcccgcgtgattggccttttttcccagcgtggctacaacattgaaagcctgaccgttgcgccaaccgacgatccgacattatcgcgtatgaccatccagaccgtgggcgatgaaaaagtacttgagcagatcgaaaagcaattacacaaactggtcgatgtcttgcgcgtgagtgagttggggcagggcgcgcatgttgagcgggaaatcatgctggtgaaaattcaggccagcggttacgggcgtgacgaagtgaaacgtaatacggaaatattccgtgggcaaattatcgatgtcacaccctcgctttataccgttcaattagcaggcaccagcggtaagcttgatgcatttttagcatcgattcgcgatgtggcgaaaattgtggaggttgctcgctctggtgtggtcggactttcgcgcggcgataaaataatgcgttgagaatgatctcaatgcgcaatttacagcccaacatgtcacgttgggctttttttgcgaaatcagtgggaacctggaataaaagcagttgccgcagttaattttctgcgcttagatgttaatgaatttaacccataccagtacaatggctatggtttttacattttacgcaaggggcaattgtgaaactggatgaaatcgctcggctggcgggagtgtcgcggaccactgcaagctatgttattaacggcaaagcgaagcaataccgtgtgagcgacaaaaccgttgaaaaagtcatggctgtggtgcgtgagcacaattaccacccgaacgccgtggcagctgggcttcgtgctggacgcacacgttctattggtcttgtgatccccgatctggagaacaccagctatacccgcatcgctaactatcttgaacgccaggcgcggcaacggggttatcaactgctgattgcctgctcagaagatcagccagacaacgaaatgcggtgcattgagcaccttttacagcgtcaggttgatgccattattgtttcgacgtcgttgcctcctgagcatcctttttatcaacgctgggctaacgacccgttcccgattgtcgcgctggaccgcgccctcgatcgtgaacacttcaccagcgtggttggtgccgatcaggatgatgccgaaatgctggcggaagagttacgtaagtttcccgccgagacggtgctttatcttggtgcgctaccggagctttctgtcagcttcctgcgtgaacaaggtttccgtactgcctggaaagatgatccgcgcgaagtgcatttcctgtatgccaacagctatgagcgggaggcggctgcccagttattcgaaaaatggctggaaacgcatccgatgccgcaggcgctgttcacaacgtcgtttgcgttgttgcaaggagtgatggatgtcacgctgcgtcgcgacggcaaactgccttctgacctggcaattgccacctttggcgataacgaactgctcgacttcttacagtgtccggtgctggcagtggctcaacgtcaccgcgatgtcgcagagcgtgtgctggagattgtcctggcaagcctggacgaaccgcgtaagccaaaacctggtttaacgcgcattaaacgtaatctctatcgccgcggcgtgctcagccgtagctaagccgcgaacaaaaatacgcgccaggtgaatttccctctggcgcgtagagtacgggactggacatcaatatgcttaaagtaaataagactattcctgactattattgataaatgcttttaaacccgcccgttaattaactcaccagctgaaattcacaataattaagtgatatcgacagcgcgtttttgcattattttgttacatgcggcgatgaattgccgatttaacaaacacttttctttgcttttgcgcaaacccgctggcatcaagcgccacacagacgtaacaaggactgttaaccggggaagatatgtcctaaaatgccgctcgcgtcgcaaactgacactttatatttgctgtggaaaatagtgagtcattttaaaacggtgatgacgatgagggattttttcttacagctattcataacgttaatttgcttcgcacgttggacgtaaaataaacaacgctgatattagccgtaaacatcgggttttttacctcggtatgccttgtgactggcttgacaagcttttcctcagctccgtaaactcctttcagtgggaaattgtggggcaaagtgggaataaggggtgaggctggcatgttccggggagcaacgttagtcaatctcgacagcaaagggcgcttatcagtgcctacccgttatcgggaacagctgcttgagaacgctgccggtcaaatggtttgcaccattgacatttatcacccgtgcctgctgctttaccccctgcctgaatgggaaattatcgagcaaaaattatcgcgtctgtcgagcatgaacccggttgagcgccgtgtgcagcgcctactgttaggtcatgccagcgaatgtcagatggatggcgcaggtcgattgttaatcgcgccagtactgcggcaacatgccgggctgacaaaagaagtgatgctggttggacagttcaacaagtttgagctgtgggatgaaacaacctggcatcaacaggtcaaggaagatatcgacgcagagcagttggctaccggagacttatcggagcgactgcaggacttgtctctataaaatgatggaaaactataaacatactacggtgctgctggatgaagccgttaatggcctcaatatccgtcctgatggcatctacattgatgggacttttggtcgcggtggtcactcacgtctgatcctctcgcagcttggcgaagaggggcgtttgctggcgatcgatcgcgacccgcaggctatcgccgttgcgaagactattgatgatccgcgcttctccatcatccacggacctttctccgcgctgggcgaatacgttgccgagcgcgatcttatcggcaagatcgacggcattctcctcgatcttggcgtctcttcaccgcaacttgatgatgctgaacgtggcttttcctttatgcgcgatggtccgctggacatgcgtatggacccaacccgtgggcagtcagccgctgaatggctacaaaccgcagaagaagccgatatcgcctgggtattgaaaacctatggtgaagagcgttttgccaaacgcattgcccgcgccattgtcgagcgtaaccgcgaacagccgatgacccgcaccaaagaactggcggaagtcgtggctgctgcaacgccggtgaaagataagtttaaacatcccgcgacccgtaccttccaggcggtgcgcatttgggtaaacagtgaactggaggagatagagcaggcgctaaaaagctcgctcaacgtgctggccccgggtgggcggctttcgatcatcagcttccactcgctggaagaccgtattgtgaaacgttttatgcgtgaaaacagccgcggtccgcaagttccggcagggttaccgatgactgaagagcagctcaaaaaactgggtggccgtcagctgcgagcactaggcaagttaatgccgggcgaagaagaggtggctgagaaccctcgtgcccgtagttcagttctgcgtattgcagagaggacgaatgcatgatcagcagagtgacagaagctctaagcaaagttaaaggatcgatgggaagccacgagcgccatgcattgcctggtgttatcggtgacgatcttttgcgatttgggaagctgccactctgcctgttcatttgcattattttgacggcggtgactgtggtaaccacggcgcaccatacccgtttactgaccgctcagcgcgaacaactggtgctggagcgagatgctttagacattgaatggcgcaacctgatccttgaagagaatgcgctcggcgaccatagccgggtggaaaggatcgccacggaaaagctgcaaatgcagcatgttgatccgtcacaagaaaatatcgtagtgcaaaaataaggataaacgcgacgcatgaaagcagcggcgaaaacgcagaaaccaaaacgtcaggaagaacatgccaactttatcagttggcgttttgcgttgttatgcggctgtattctcctggcgctggcttttctgctcggacgcgtagcgtggttacaagttatctccccggatatgctggtgaaagagggcgacatgcgttctcttcgcgttcagcaagtttccacctcccgcggcatgattactgaccgttctggtcgcccgttagcggtgagcgtgccggtaaaagcgatttgggctgacccgaaagaagtgcatgacgctggcggtatcagcgtcggtgaccgctggaaggcgctggctaacgcgctcaatattccgctggatcagctttcagcccgcattaacgccaacccgaaagggcgctttatttatctggcgcgtcaggtgaaccctgacatggcggactacatcaaaaaactgaaactgccggggattcatctgcgtgaagagtctcgccgttactatccgtccggcgaagtgactgctcacctcatcggctttactaacgtcgatagtcaagggattgagggcgttgagaagagtttcgataaatggcttaccgggcagccgggtgagcgcattgtgcgtaaagaccgctatggtcgcgtaattgaagatatttcttctactgacagccaggcagcgcacaacctggcgctgagtattgatgaacgcctgcaggcgctggtttatcgcgaactgaacaacgcggtggcctttaacaaggctgaatctggtagcgccgtgctggtggatgtcaacaccggtgaagtgctggcgatggctaacagcccgtcatacaaccctaacaatctgagcggcacgccgaaagaggcgatgcgtaaccgtaccatcaccgacgtgtttgaaccgggctcaacggttaaaccgatggtggtaatgaccgcgttgcaacgtggcgtggtgcgggaaaactcggtactcaataccattccttatcgaattaacggccacgaaatcaaagacgtggcacgctacagcgaattaaccctgaccggggtattacagaagtcgagtaacgtcggtgtttccaagctggcgttagcgatgccgtcctcagcgttagtagatacttactcacgttttggactgggaaaagcgaccaatttggggttggtcggagaacgcagtggcttatatcctcaaaaacaacggtggtctgacatagagagggccaccttctctttcggctacgggctaatggtaacaccattacagttagcgcgagtctacgcaactatcggcagctacggcatttatcgcccactgtcgattaccaaagttgaccccccggttcccggtgaacgtgtcttcccggaatccattgtccgcactgtggtgcatatgatggaaagcgtggcgctaccaggcggcggcggcgtgaaggcggcgattaaaggctatcgtatcgccattaaaaccggtaccgcgaaaaaggtcgggccggacggtcgctacatcaataaatatattgcttataccgcaggcgttgcgcctgcgagtcagccgcgcttcgcgctggttgttgttatcaacgatccgcaggcgggtaaatactacggcggcgccgtttccgcgccggtctttggtgccatcatgggcggcgtattgcgtaccatgaacatcgagccggatgcgctgacaacgggcgataaaaatgaatttgtgattaatcaaggcgaggggacaggtggcagatcgtaatttgcgcgaccttcttgctccgtgggtgccagacgcaccttcgcgagcactgcgagagatgacactcgacagccgtgtggctgcggcgggcgatctctttgtagctgtagtaggtcatcaggcggacgggcgtcgatatatcccgcaggcgatagcgcaaggtgtggctgccattattgcagaggcgaaagatgaggcgaccgatggtgaaatccgtgaaatgcacggcgtaccggtcatctatctcagccagctcaacgagcgtttatctgcactggcgggccgcttttaccatgaaccctctgacaatttacgtctcgtgggcgtaacgggcaccaacggcaaaaccacgactacccagctgttggcgcagtggagccaactgcttggcgaaatcagcgcggtaatgggcaccgttggtaacggcctgctggggaaagtgatcccgacagaaaatacaaccggttcggcagtcgatgttcagcatgagctggcggggctggtggatcagggcgcgacgttttgcgcaatggaagtttcctcccacgggctggtacagcaccgtgtggcggcattgaaatttgcggcgtcggtctttaccaacttaagccgcgatcaccttgattatcatggtgatatggaacactacgaagccgcgaaatggctgctttattctgagcatcattgcggtcaggcgattattaacgccgacgatgaagtgggccgccgctggctggcaaaactgccggacgcggttgcggtatcaatggaagatcatattaatccgaactgtcacggacgctggttgaaagcgaccgaagtgaactatcacgacagcggtgcgacgattcgctttagctcaagttggggcgatggcgaaattgaaagccatctgatgggcgcttttaacgtcagcaacctgctgctcgcgctggcgacactgttggcactcggctatccactggctgatctgctgaaaaccgccgcgcgtctgcaaccggtttgcggacgtatggaagtgttcactgcgccaggcaaaccgacggtggtggtggattacgcgcatacgccggatgcactggaaaaagccttacaggcggcgcgtctgcactgtgcgggcaagctgtggtgtgtctttggctgtggtggcgatcgcgataaaggtaagcgtccactgatgggcgcaattgccgaagagtttgctgacgtggcggtggtgacggacgataacccgcgtaccgaagaaccgcgtgccatcatcaacgatattctggcgggaatgttagatgccggacatgccaaagtgatggaaggccgtgctgaagcggtgacttgcgccgttatgcaggctaaagagaatgatgtggtactggtcgcgggcaaaggccatgaagattaccagattgttggcaatcagcgtctggactactccgatcgcgtcacggtggcgcgtctgctgggggtgattgcatgattagcgtaacccttagccaacttaccgacattctcaacggtgaactgcaaggtgcagatatcacccttgatgctgtaaccactgatacccgaaaactgacgccgggctgcctgtttgttgccctgaaaggcgaacgttttgatgcccacgattttgccgaccaggcgaaagctggcggcgcaggcgcactactggttagccgtccgctggacatcgacctgccgcagttaatcgtcaaggatacgcgtctggcgtttggtgaactggctgcatgggttcgccagcaagttccggcgcgcgtggttgctctgacggggtcctccggcaaaacctccgttaaagagatgacggcggcgattttaagccagtgcggcaacacgctttatacggcaggcaatctcaacaacgacatcggtgtaccgatgacgctgttgcgcttaacgccggaatacgattacgcagttattgaacttggcgcgaaccatcagggcgaaatagcctggactgtgagtctgactcgcccggaagctgcgctggtcaacaacctggcagcggcgcatctggaaggttttggctcgcttgcgggtgtcgcgaaagcgaaaggtgaaatctttagcggcctgccggaaaacggtatcgccattatgaacgccgacaacaacgactggctgaactggcagagcgtaattggctcacgcaaagtgtggcgtttctcacccaatgccgccaacagcgatttcaccgccaccaatatccatgtgacctcgcacggtacggaatttaccctacaaaccccaaccggtagcgtcgatgttctgctgccgttgccggggcgtcacaatattgcgaatgcgctggcagccgctgcgctctccatgtccgtgggcgcaacgcttgatgctatcaaagcggggctggcaaatctgaaagctgttccaggccgtctgttccccatccaactggcagaaaaccagttgctgctcgacgactcctacaacgccaatgtcggttcaatgactgcagcagtccaggtactggctgaaatgccgggctaccgcgtgctggtggtgggcgatatggcggaactgggcgctgaaagcgaagcctgccatgtacaggtgggcgaggcggcaaaagctgctggtattgaccgcgtgttaagcgtgggtaaacaaagccatgctatcagcaccgccagcggcgttggcgaacattttgctgataaaactgcgttaattacgcgtcttaaattactgattgctgagcaacaggtaattacgattttagttaagggttcacgtagtgccgccatggaagaggtagtacgcgctttacaggagaatgggacatgttagtttggctggccgaacatttggtcaaatattattccggctttaacgtcttttcctatctgacgtttcgcgccatcgtcagcctgctgaccgcgctgttcatctcattgtggatgggcccgcgtatgattgctcatttgcaaaaactttcctttggtcaggtggtgcgtaacgacggtcctgaatcacacttcagcaagcgcggtacgccgaccatgggcgggattatgatcctgacggcgattgtgatctccgtactgctgtgggcttacccgtccaatccgtacgtctggtgcgtgttggtggtgctggtaggttacggtgttattggctttgttgatgattatcgcaaagtggtgcgtaaagacaccaaagggttgatcgctcgttggaagtatttctggatgtcggtcattgcgctgggtgtcgccttcgccctgtaccttgccggcaaagacacgcccgcaacgcagctggtggtcccattctttaaagatgtgatgccgcagctggggctgttctacattctgctggcttacttcgtcattgtgggtactggcaacgcggtaaacctgaccgatggtctcgacggcctggcaattatgccgaccgtatttgtcgccggtggttttgcgctggtggcgtgggcgaccggcaatatgaactttgccagctacttgcatataccgtatctgcgacacgccggggaactggttattgtctgtaccgcgatagtcggggcaggactgggcttcctgtggtttaacacctatccggcgcaggtctttatgggcgatgtaggttcgctggcgttaggtggtgcgttaggcattatcgccgtactgctacgtcaggaattcctgctggtgattatggggggcgtgttcgtggtagaaacgctttctgtcatcctgcaggtcggctcctttaaactgcgcggacaacgtattttccgcatggcaccgattcatcaccactatgaactgaaaggctggccggaaccgcgcgtcattgtgcgtttctggattatttcgctgatgctggttctgattggtctggcaacgctgaaggtacgttaatcatggctgattatcagggtaaaaatgtcgtcattatcggcctgggcctcaccgggctttcctgcgtggactttttcctcgctcgcggtgtgacgccgcgcgttatggatacgcgtatgacaccgcctggcctggataaattacccgaagccgtagaacgccacacgggcagtctgaatgatgaatggctgatggcggcagatctgattgtcgccagtcccggtattgcactggcgcatccatccttaagcgctgccgctgatgccggaatcgaaatcgttggcgatatcgagctgttctgtcgcgaagcacaagcaccgattgtggcgattaccggttctaacggcaaaagcacggtcaccacgctagtgggtgaaatggcgaaagcggcgggggttaacgttggtgtgggtggcaatattggcctgcctgcgttgatgctactggatgatgagtgtgaactgtacgtgctggaactgtcgagcttccagctggaaaccacctccagcttacaggcggtagcagcgaccattctgaacgtgactgaagatcatatggatcgctatccgtttggtttacaacagtatcgtgcagcaaaactgcgcatttacgaaaacgcgaaagtttgcgtggttaatgctgatgatgccttaacaatgccgattcgcggtgcggatgaacgctgcgtcagctttggcgtcaacatgggtgactatcacctgaatcatcagcagggcgaaacctggctgcgggttaaaggcgagaaagtgctgaatgtgaaagagatgaaactttccgggcagcataactacaccaatgcgctggcggcgctggcgctggcagatgctgcagggttaccgcgtgccagcagcctgaaagcgttaaccacattcactggtctgccgcatcgctttgaagttgtgctggagcataacggcgtacgttggattaacgattcgaaagcgaccaacgtcggcagtacggaagcggcgctgaatggcctgcacgtagacggcacactgcatttgttgctgggtggcgatggtaaatcggcggactttagcccactggcgcgttacctgaatggcgataacgtacgtctgtattgtttcggtcgtgacggcgcgcagctggcggcgctacgcccggaagtggcagaacaaaccgaaactatggaacaggcgatgcgcttgctggctccgcgtgttcagccgggcgatatggttctgctctccccagcctgtgccagccttgatcagttcaagaactttgaacaacgaggcaatgagtttgcccgtctggcgaaggagttaggttgatgcgtttatctctccctcgcctgaaaatgccgcgcctgccaggattcagtatcctggtctggatctccacggcgctaaagggctgggtgatgggctcgcgggaaaaagataccgacagcctgatcatgtacgatcgcaccttactgtggctgaccttcggcctcgcggcgattggctttatcatggtgacctcggcgtcaatgcccatagggcaacgcttaaccaacgatccgttcttcttcgcgaagcgtgatggtgtctatctgattttggcgtttattctggcgatcattacgctgcgtctgccgatggagttctggcaacgctacagtgccacgatgctgctcggatctatcatcctgctgatgatcgtcctggtagtgggtagctcggttaaaggggcatcgcgttggatcgatctcggtttgctgcgtatccagcctgcggagctgacaaaactgtcgctgttttgctatatcgccaactatctggtgcgtaaaggcgacgaagtacgtaataacctgcgcggcttcctgaaaccgatgggcgtgattctggtgttggcagtgttactgctggcacagccagaccttggtacggtggtggtgttgtttgtgactacgctggcgatgttgttcctggcgggagcgaaattgtggcagttcattgccattatcggtatgggcatttcagcggttgtgttgctgatactcgccgaaccgtaccgtatccgccgtgttaccgcattctggaacccgtgggaagatccctttggcagcggctatcagttaacgcaatcgctgatggcgtttggtcgcggcgaactttgggggcaaggtttaggtaactcggtacaaaaactggagtatctgccggaagcgcacactgactttattttcgccattatcggcgaagaactggggtatgtcggtgtggtgctggcacttttaatggtattcttcgtcgcttttcgcgcgatgtcgattggccgtaaagcattagaaattgaccaccgtttttccggttttctcgcctgttctattggcatctggtttagcttccaggcgctggttaacgtaggcgcggcggcggggatgttaccgaccaaaggtctgacattgccgctgatcagttacggtggttcgagcttactgattatgtcgacagccatcatgatgctgttgcgtattgattatgaaacgcgtctggagaaagcgcaggcgtttgtacgaggttcacgatgagtggtcaaggaaagcgattaatggtgatggcaggcggaaccggtggacatgtattcccgggactggcggttgcgcaccatctaatggctcagggttggcaagttcgctggctggggactgccgaccgtatggaagcggacttagtgccaaaacatggcatcgaaattgatttcattcgtatctctggtctgcgtggaaaaggtataaaagcactgatagctgccccgctgcgtatcttcaacgcctggcgtcaggcgcgggcgattatgaaagcgtacaaacctgacgtggtgctcggtatgggaggctacgtgtcaggtccaggtggtctggccgcgtggtcgttaggcattccggttgtacttcatgaacaaaacggtattgcgggcttaaccaataaatggctggcgaagattgccaccaaagtgatgcaggcgtttccaggtgctttccctaatgcggaagtagtgggtaacccggtgcgtaccgatgtgttggcgctgccgttgccgcagcaacgtttggctggacgtgaaggtccggttcgtgtgctggtagtgggtggttctcagggcgcacgcattcttaaccagacaatgccgcaggttgctgcgaaactgggtgattcagtcactatctggcatcagagcggcaaaggttcgcaacaatccgttgaacaggcgtatgccgaagcggggcaaccgcagcataaagtgacggaatttattgatgatatggcggcggcgtatgcgtgggcggatgtcgtcgtttgccgctccggtgcgttaacggtgagtgaaatcgccgcggcaggactaccggcgttgtttgtgccgtttcaacataaagaccgccagcaatactggaatgcgctaccgctggaaaaagcgggcgcagccaaaattatcgagcagccacagcttagcgtggatgctgtcgccaacaccctggccgggtggtcgcgagaaaccttattaaccatggcagaacgcgcccgcgctgcatccattccggatgccaccgagcgagtggcaaatgaagtgagccgggttgcccgggcgtaattgtagcgatgccttttgcatcgtatgaatttaagaagttaatggcgtaaagaatgaatacacaacaattggcaaaactgcgttccatcgtgcccgaaatgcgtcgcgttcggcacatacattttgtcggcattggtggtgccggtatgggcggtattgccgaagttctggccaatgaaggttatcagatcagtggttccgatttagcgccaaatccggtcacgcagcagttaatgaatctgggtgcgacgatttatttcaaccatcgcccggaaaacgtacgtgatgccagcgtggtcgttgtttccagcgcgatttctgccgataacccggaaattgtcgccgctcatgaagcgcgtattccggtgatccgtcgtgccgaaatgctggctgagttaatgcgttttcgtcatggcatcgccattgccggaacgcacggcaaaacgacaaccaccgcgatggtttccagcatctacgcagaagcggggctcgacccaaccttcgttaacggcgggctggtaaaagcggcgggggttcatgcgcgtttggggcatggtcggtacctgattgccgaagcagatgagagtgatgcatcgttcctgcatctgcaaccgatggtggcgattgtcaccaatatcgaagccgaccacatggatacctaccagggcgactttgagaatttaaaacagacttttattaattttctgcacaacctgccgttttacggtcgtgcggtgatgtgtgttgatgatccggtgatccgcgaattgttaccgcgagtggggcgtcagaccacgacttacggcttcagcgaagatgccgacgtgcgtgtagaagattatcagcagattggcccgcaggggcactttacgctgctgcgccaggacaaagagccgatgcgcgtcaccctgaatgcgccaggtcgtcataacgcgctgaacgccgcagctgcggttgcggttgctacggaagagggcattgacgacgaggctattttgcgggcgcttgaaagcttccaggggactggtcgccgttttgatttcctcggtgaattcccgctggagccagtgaatggtaaaagcggtacggcaatgctggtcgatgactacggccaccacccgacggaagtggacgccaccattaaagcggcgcgcgcaggctggccggataaaaacctggtaatgctgtttcagccgcaccgttttacccgtacgcgcgacctgtatgatgatttcgccaatgtgctgacgcaggttgataccctgttgatgctggaagtgtatccggctggcgaagcgccaattccgggagcggacagccgttcgctgtgtcgcacaattcgtggacgtgggaaaattgatcccattctggtgccggatccggcgcgggtagccgagatgctggcaccggtattaaccggtaacgacctgattctcgttcagggggctggtaatattggaaaaattgcccgttctttagctgaaatcaaactgaagccgcaaactccggaggaagaacaacatgactgataaaatcgcggtcctgttgggtgggacctccgctgagcgggaagtttctctgaattctggcgcagcggtgttagccggactgcgtgaaggcggtattgacgcgtatcctgtcgacccgaaagaagtcgacgtgacgcaactgaagtcgatgggctttcagaaagtgtttatcgcgctacacggtcgcggcggtgaagatggtacgctgcaggggatgctcgagctgatgggcttgccttataccggaagcggagtgatggcatctgcgctttcaatggataaactacgcagcaaacttctatggcaaggtgccggtttaccggtcgcgccgtgggtagcgttaacccgcgcagagtttgaaaaaggcctgagcgataagcagttagcagaaatttctgctctgggtttgccggttatcgttaagccgagccgcgaaggttccagtgtgggaatgtcaaaagtagtagcagaaaatgctctacaagatgcattaagattggcatttcagcacgatgaagaagtattgattgaaaaatggctaagtgggccggagttcacggttgcgatactcggtgaagaaattttaccgtcaatacgtattcaaccgtccggaaccttctatgattatgaggcgaagtatctctctgatgagacacagtatttctgccccgcaggtctggaagcgtcacaagaggccaatttgcaggcattagtgctgaaagcatggacgacgttaggttgcaaaggatggggacgtattgacgttatgctggacagcgatggacagttttatctgctggaagccaatacctcaccgggtatgaccagccacagcctggtgccgatggcggcacgtcaggcaggtatgagcttctcgcagttggtagtacgaattctggaactggcggactaatatgtcgcaggctgctctgaacacgcgaaacagcgaagaagaggtttcttctcgccgcaataatggaacgcgtctggcggggatccttttcctgctgaccgttttaacgacagtgttggtgagcggctgggtcgtgttgggctggatggaagatgcgcaacgcctgccgctctcaaagctggtgttgaccggtgaacgccattacacacgtaatgacgatatccggcagtcgatcctggcattgggtgagccgggtacctttatgacccaggatgtcaacatcatccagacgcaaatagaacaacgcctgccgtggattaagcaggtgagcgtcagaaagcagtggcctgatgaattgaagattcatctggttgaatatgtgccgattgcgcggtggaatgatcaacatatggtagacgcggaaggaaataccttcagcgtgccgccagaacgcaccagcaagcaggtgcttccaatgctgtatggcccggaaggcagcgccaatgaagtgttgcagggctatcgcgaaatggggcagatgctggcaaaggacagatttactctgaaggaagcggcgatgaccgcgcggcgttcctggcagttgacgctgaataacgatattaagctcaatcttggccggggcgatacgatgaaacgtttggctcgctttgtagaactttatccggttttacagcagcaggcgcaaaccgatggcaaacggattagctacgttgatttgcgttatgactctggagcggcagtaggctgggcgcccttgccgccagaggaatctactcagcaacaaaatcaggcacaggcagaacaacaatgatcaaggcgacggacagaaaactggtagtaggactggagattggtaccgcgaaggttgccgctttagtaggggaagttctgcccgacggtatggtcaatatcattggcgtgggcagctgcccgtcgcgtggtatggataaaggcggggtgaacgacctcgaatccgtggtcaagtgcgtacaacgcgccattgaccaggcagaattgatggcagattgtcagatctcttcggtatatctggcgctttctggtaagcacatcagctgccagaatgaaattggtatggtgcctatttctgaagaagaagtgacgcaagaagatgtggaaaacgtcgtccataccgcgaaatcggtgcgtgtgcgcgatgagcatcgtgtgctgcatgtgatcccgcaagagtatgcgattgactatcaggaagggatcaagaatccggtaggactttcgggcgtgcggatgcaggcaaaagtgcacctgatcacatgtcacaacgatatggcgaaaaacatcgtcaaagcggttgaacgttgtgggctgaaagttgaccaactgatatttgccggactggcatcaagttattcggtattgacggaagatgaacgtgaactgggtgtctgcgtcgtcgatatcggtggtggtacaatggatatcgccgtttataccggtggggcattgcgccacactaaggtaattccttatgctggcaatgtcgtgaccagtgatatcgcttacgcctttggcacgccgccaagcgacgccgaagcgattaaagttcgccacggttgtgcgctgggttccatcgttggaaaagatgagagcgtggaagtgccgagcgtaggtggtcgtccgccacggagtctgcaacgtcagacactggcagaggtgatcgagccgcgctataccgagctgctcaacctggtcaacgaagagatattgcagttgcaggaaaagcttcgccaacaaggggttaaacatcacctggcggcaggcattgtattaaccggtggcgcagcgcagatcgaaggtcttgcagcctgtgctcagcgcgtgtttcatacgcaagtgcgtatcggcgcgccgctgaacattaccggtttaacggattatgctcaggagccgtattattcgacggcggtgggattgcttcactatgggaaagagtcacatcttaacggtgaagctgaagtagaaaaacgtgttacagcatcagttggctcgtggatcaagcgactcaatagttggctgcgaaaagagttttaatttttatgaggccgacgatgattacggcctcaggcgacaggcacaaatcggagagaaactatgtttgaaccaatggaacttaccaatgacgcggtgattaaagtcatcggcgtcggcggcggcggcggtaatgctgttgaacacatggtgcgcgagcgcattgaaggtgttgaattcttcgcggtaaataccgatgcacaagcgctgcgtaaaacagcggttggacagacgattcaaatcggtagcggtatcaccaaaggactgggcgctggcgctaatccagaagttggccgcaatgcggctgatgaggatcgcgatgcattgcgtgcggcgctggaaggtgcagacatggtctttattgctgcgggtatgggtggtggtaccggtacaggtgcagcaccagtcgtcgctgaagtggcaaaagatttgggtatcctgaccgttgctgtcgtcactaagcctttcaactttgaaggcaagaagcgtatggcattcgcggagcaggggatcactgaactgtccaagcatgtggactctctgatcactatcccgaacgacaaactgctgaaagttctgggccgcggtatctccctgctggatgcgtttggcgcagcgaacgatgtactgaaaggcgctgtgcaaggtatcgctgaactgattactcgtccgggtttgatgaacgtggactttgcagacgtacgcaccgtaatgtctgagatgggctacgcaatgatgggttctggcgtggcgagcggtgaagaccgtgcggaagaagctgctgaaatggctatctcttctccgctgctggaagatatcgacctgtctggcgcgcgcggcgtgctggttaacatcacggcgggcttcgacctgcgtctggatgagttcgaaacggtaggtaacaccatccgtgcatttgcttccgacaacgcgactgtggttatcggtacttctcttgacccggatatgaatgacgagctgcgcgtaaccgttgttgcgacaggtatcggcatggacaaacgtcctgaaatcactctggtgaccaataagcaggttcagcagccagtgatggatcgctaccagcagcatgggatggctccgctgacccaggagcagaagccggttgctaaagtcgtgaatgacaatgcgccgcaaactgcgaaagagccggattatctggatatcccagcattcctgcgtaagcaagctgattaagaattgactggaatttgggtttcgaggctctttgtgctaaactggcccgccgaatgtatagtacacttcggttggataggtaatttggcgagataatacgatgatcaaacaaaggacacttaaacgtatcgttcaggcgacgggtgtcggtttacataccggcaagaaagtcaccctgacgttacgccctgcgccggccaacaccggggtcatctatcgtcgcaccgacttgaatccaccggtagatttcccggccgatgccaaatctgtgcgtgataccatgctctgtacgtgtctggtcaacgagcatgatgtacggatttcaaccgtagagcacctcaatgctgctctcgcgggcttgggcatcgataacattgttatcgaagttaacgcgccggaaatcccgatcatggacggcagcgccgctccgtttgtatacctgctgcttgacgccggtatcgacgagttgaactgcgccaaaaaatttgttcgcatcaaagagactgttcgtgtcgaagatggcgataagtgggctgaatttaagccgtacaatggtttttcgctggatttcaccatcgattttaaccatccggctattgattccagcaaccagcgctatgcgatgaacttctccgctgatgcgtttatgcgccagatcagccgtgcgcgtacgttcggtttcatgcgtgatatcgaatatctgcagtcccgtggtttgtgcctgggcggcagcttcgattgtgccatcgttgttgacgattatcgcgtactgaacgaagacggcctgcgttttgaagacgaatttgtgcgtcacaaaatgctcgatgcgatcggtgacttgttcatgtgtggtcacaatattattggtgcatttaccgcttataaatccggtcatgcactgaataacaaactgctgcaggctgtcctggcgaaacaggaagcctgggaatatgtgaccttccaggacgacgcagaactgccgttggccttcaaagcgccttcagctgtactggcataacgacatttatactgtcgtataaaattcgactggcaaatctggcactctctccggccaggtgaaccagtcgtttttttttgaattttataagagctataaaaaacggtgcgaacgctgttttcttaagcacttttccgcacaacttatcttcattcgtgctgtggactgcaggctttaatgataagatttgtgcgctaaatacgtttgaatatgatcgggatggcaataacgtgagtggaatactgacgcgctggcgacagtttggtaaacgctacttctggccgcatctcttattagggatggttgcggcgagtttaggtttgcctgcgctcagcaacgccgccgaaccaaacgcgcccgcaaaagcgacaacccgcaaccacgagccttcagccaaagttaactttggtcaattggccttgctggaagcgaacacacgccgcccgaattcgaactattccgttgattactggcatcaacatgccattcgcacggtaatccgtcatctttctttcgcaatggcaccgcaaacactgcccgttgctgaagaatctttgcctcttcaggcgcaacatcttgcattactggatacgctcagcgcgctgctgacccaggaaggcacgccgtctgaaaagggttatcgcattgattatgcgcattttaccccacaagcaaaattcagcacgcccgtctggataagccaggcgcaaggcatccgtgctggccctcaacgcctcacctaacaacaataaacctttacttcattttattaactccgcaacgcggggcgtttgagattttattatgctaatcaaattgttaactaaagttttcggtagtcgtaacgatcgcaccctgcgccggatgcgcaaagtggtcaacatcatcaatgccatggaaccggagatggaaaaactctccgacgaagaactgaaagggaaaaccgcagagtttcgtgcacgtctggaaaaaggcgaagtgctggaaaatctgatcccggaagctttcgccgtggtacgtgaggcaagtaagcgcgtctttggtatgcgtcacttcgacgttcagttactcggcggtatggttcttaacgaacgctgcatcgccgaaatgcgtaccggtgaaggaaaaaccctgaccgcaacgctgcctgcttacctgaacgcactaaccggtaaaggcgtgcacgtagttaccgtcaacgactacctggcgcaacgtgacgccgaaaacaaccgtccgctgtttgaattccttggcctgactgtcggtatcaacctgccgggcatgccagcaccggcaaagcgcgaagcttacgcagctgacatcacttacggtacgaacaacgaatacggctttgactacctgcgcgacaacatggcgttcagccctgaagaacgtgtacagcgtaaactgcactatgcgctggtggacgaagtggactccatcctgatcgatgaagcgcgtacaccgctgatcatttccggcccggcagaagacagctcggaaatgtataaacgcgtgaataaaattattccgcacctgatccgtcaggaaaaagaagactccgaaaccttccagggcgaaggccacttctcggtggacgaaaaatctcgccaggtgaacctgaccgaacgtggtctggtgctgattgaagaactgctggtgaaagagggcatcatggatgaaggggagtctctgtactctccggccaacatcatgctgatgcaccacgtaacggcggcgctgcgcgctcatgcgctgtttacccgtgacgtcgactacatcgttaaagatggtgaagttatcatcgttgacgaacacaccggtcgtaccatgcagggccgtcgctggtccgatggtctgcaccaggctgtggaagcgaaagaaggtgtgcagatccagaacgaaaaccaaacgctggcttcgatcaccttccagaactacttccgtctgtatgaaaaactggcggggatgaccggtactgctgataccgaagctttcgaatttagctcaatctacaagctggataccgtcgttgttccgaccaaccgtccaatgattcgtaaagatctgccggacctggtctacatgactgaagcggaaaaaattcaggcgatcattgaagatatcaaagaacgtactgcgaaaggccagccggtgctggtgggtactatctccatcgaaaaatcggagctggtgtcaaacgaactgaccaaagccggtattaagcacaacgtcctgaacgccaaattccacgccaacgaagcggcgattgttgctcaggcaggttatccggctgcggtgactatcgcgaccaatatggcgggtcgtggtacagatattgtgctcggtggtagctggcaggcagaagttgccgcgctggaaaatccgaccgcagagcaaattgaaaaaattaaagccgactggcaggtacgtcacgatgcggtactggaagcaggtggcctgcatatcatcggtaccgagcgtcacgaatcccgtcgtatcgataaccagttgcgcggtcgttctggtcgtcagggggatgctggttcttcccgtttctacctgtcgatggaagatgcgctgatgcgtatttttgcttccgaccgagtatccggcatgatgcgtaaactgggtatgaagccaggcgaagccattgaacacccgtgggtgactaaagcgattgccaacgcccagcgtaaagttgaaagccgtaacttcgacattcgtaagcaactgctggaatatgatgacgtggctaacgatcagcgtcgcgccatttactcccagcgtaacgaactgttggatgtcagcgatgtgagcgaaaccattaacagcattcgtgaagatgtgttcaaagcgaccattgatgcctacattccaccacagtcgctggaagaaatgtgggatattccggggctgcaggaacgtctgaagaacgatttcgacctcgatttgccaattgccgagtggctggataaagaaccagaactgcatgaagagacgctgcgtgagcgcattctggcgcagtccatcgaagtgtatcagcgtaaagaagaagtggttggtgctgagatgatgcgtcacttcgagaaaggcgtcatgctgcaaacgcttgactccctgtggaaagagcacctggcagcgatggactatctgcgtcagggtatccacctgcgtggctacgcacagaaagatccgaagcaggaatacaaacgtgaatcgttctccatgtttgcagcgatgctggagtcgttgaaatatgaagttatcagtacgctgagcaaagttcaggtacgtatgcctgaagaggttgaggagctggaacaacagcgtcgtatggaagccgagcgtttagcgcaaatgcagcagcttagccatcaggatgacgactctgcagccgcagctgcactggcggcgcaaaccggagagcgcaaagtaggacgtaacgatccttgcccgtgcggttctggtaaaaaatacaagcagtgccatggccgcctgcaataaaagctaactgttgaagtaaaaggcgcaggattctgcgccttttttataggtttaagacaatgaaaaagctgcaaattgcggtaggtattattcgcaacgagaacaatgaaatctttataacgcgtcgcgcagcagatgcgcacatggcgaataaactggagtttcccggcggtaaaattgaaatgggtgaaacgccggaacaggcggtggtgcgtgaacttcaggaagaagtcgggattaccccccaacatttttcgctatttgaaaaactggaatatgaattcccggacaggcatataacactgtggttttggctggtcgaacgctgggaaggggagccgtggggtaaagaagggcaacccggtgagtggatgtcgctggtcggtcttaatgccgatgattttccgccagccaatgaaccggtaattgcgaagcttaaacgtctgtaggtcagataaggcgttttcgccgcatccgacattcgcacacgatgcctgatgcgacgctggcgcgtcttatcaggcctaaagggatttctaactcattgataaatttgtttttgtaggtcggataaggcgttcacgccgcatccgacatttgcacaagatgcctgatgcgacgctgtccgcgtcttatcaggcctacgtgcggcatcagacaaatgtcactgctttggttcttcgctccagtcatcgctttcggaaagatcgccactgctggggattcgtttttcttcagcagcccattctccgaggtcgatcagctgacaacgtttggagcaaaatggccgaaacgggctgatttcaccccacaccaccgttttcccgcaggttgggcaattcaccgtaatagtttctgacatttttactccttagcaacaggccagttcgaaatccagacgttccggtacctgtccgttttcagtgtccagcggcataaaacgaatggcaaaacggctcttatgtccggaaatttgcggataaagctgtgaatcgagcgacagattcaggcgcagcaagtcggcatcgccaccgttatcctgataaaaaccattcaggctggtttgtttacggaagggggccgactggcgaattaaatccagcaccatggtaagtgcctgggtgagcgggttcaggctggcaatccaggtttctacctggctgtcgcgctgcgcctggggtagatgcagccaaatgtgcaatgtaggtaaatcaaagctgcaacagccgcctgggatgctcagtcgctgacgcaccagagcaatcaaacgatcttcacgcagaaattgcccgatacgcggcgcggaaattaatacgctccccgccgcttttaactgctgaattaatgcttcaatacggctctggtccacgccaggcacgccaatccaggtctggagtttacgttgctgccggtcaagttctttcaacagctcagtgcggacttcgccgcgctcgaaaacatccagtaattcactgacattacggaagaaatgcagcgcgccagcgtggtcaacgatgggtaaattaacggtgagttgctgaatcaaaaactcaatgcgcagccatgtacgcattttttcatttagtggatgttcaaaaaggacctgggtctgcattacggtttttcctgtgagacaaactgcgacgcaagctgcaaatagtgtgcgtgcaggcgggcaacatccgatgcgatagcatccggtgcgccgttattatcaatgacgtcatctgccacggcaaggcgggcttcgcgcgttgcctgagcagcaaggatttgttcgacatgctcgcgagttacatcatcgcgctgcatggtgcgcttaagttgcgtttctgggctgacatccaccacaagcactcgattcgcttttttatacagtgagttttctaccagcaatggcacaacccacagtacatagggggaagtagcttgctggatctggtgttgcgtctcttgctgaatcagcggatgcagcagggcgttaagccagtttttctcttccgggttggcgaagatccgctcgcgcaaggcccggcgctgcaatgttccatcagcagcaatcatgttagcgccaaagtgatcagcaatggcatgtagcgcaggtgcacctggttcaaccacctgacgcgcaataatatcggcatcaatgacgttaattccgagatcagcaaacgcattggcaacggtactcttgccactgccaatgcctcccgttaaggcaactatatacctcataatttatattcccgggaattcatcatgattatcaaaacgttaaaaatgagtgcacgaaagcgaaattgatgaaacgttcgctcactatttaccaggtaaatttatgggattgtagcgtaaaaaaagacaatttcgcagtcttgcgccgcattgattagtgcgtatgatagcgtcactggagttgcgctcttacccttatagccattaaccccaggaatccgcacatgcgtattgaagaagatctgaagttaggttttaaagacgttctcatccgccctaaacgctccactcttaaaagccgttccgatgttgaactggaacgtcaattcaccttcaaacattcaggtcagagctggtccggcgtgccgattatcgccgcaaatatggacaccgtaggcacattttctatggcctctgcgctggcttcttttgatattttgactgctgtgcataaacactattctgtcgaagagtggcaagcgtttatcaacaattcttccgctgatgtgctgaaacatgtgatggtttctaccggtacgtctgatgcggatttcgaaaaaactaaacagattctcgacctgaacccggcattaaacttcgtttgtattgacgtggcgaatggttattccgaacacttcgtgcagttcgttgcgaaagcgcgtgaagcgtggccgaccaaaaccatttgtgctggtaacgtagtgactggtgaaatgtgtgaggagcttatcctctcaggtgccgatatcgttaaagttggcattggcccaggttctgtttgtacaactcgcgtcaaaacaggcgtcggttatccgcaactttctgcggtaatcgaatgtgccgatgctgcgcacggtctgggcggaatgatcgtcagcgatggtggctgcaccacgccgggcgatgtggcgaaagcctttggcggcggtgccgatttcgtcatgcttggcggcatgctggcgggccacgaagagagcggcggtcgcatcgttgaggagaacggcgagaaatttatgctgttctacggcatgagctccgagtctgcgatgaaacgtcacgttggcggcgttgcggaatatcgcgcagcagaaggtaaaaccgttaagctgccgctgcgaggcccggttgaaaataccgcgcgagatattttgggcggcctgcgttcagcttgtacatacgttggggcttcacgcctgaaagagctgaccaagcgcaccacgtttattcgtgtgcaggaacaagaaaaccgcatcttcaacaacctgtaatctcccaacgctggcgtggagcaacacgccagcgttatcccatcccactcatcgcatcgcctaaatggaaaattggcagatacattgccaccaccagcgtaccaataattcctcccgttatgatcagcaacgccggttccagtaaggctgcgaggttatccgccagcgccattgtgttttcccgatgatgatgggcgaggttgtctaacatgagatccagagagccggatgcctctcctgttctcactaattgcaaacagagcgggctaaactcaccggtattttttagcgccagccagatgggttgaccgttactgatatcgtgctggatttgtgtcagaagttgcacccagtacgggcagcgcattgtttctctgacgctctctacgccctgtaaaaaagtaatgcctgcactttgtgtcagcgccagaatcgtaaagatctgcgtgagtttttgtccccgcatcagtgaacccataatcgggatgcgtaacagcaatttctgccgcactataagccaggtcggtcggcgcatcagcaacttattggctatcgccagcagaaagccgaacaacaccagcagccagctccattcgccactaaagtctgccagcgtcatgatcccctgcgttagtgccggtagtggggtgttgaaggtcttatagatagcggcaaactccggcagaacaaaatgcagcattgccacaaccaccatgattgccatcgctaaaatgatgatgggataacgtaacgctgatttcactttgtcggtcaactgacgctgggctttttgctgacgcgccagttcaaagcagcattcatccagcttaccggtcagttcacccgtgcggatcatcgcctgatagagcggcggaaatacctctgaccagggtaataaggcattggaaaaagcaatgccctgttcgagatcgtgcgccagcgattgcagcaacgcttgccattgcttactgggatgctgttccgccagcagagccagcccttcagaaagcgttaaccctgctttgagtagcgtcgccagttgatgaatgacttccgcgcttttatctcctcgccactgcgcagaattgatggcgattcgcttcaggcttagtggggtaaccatctgttgctgtagtgccataagcagtaaagtacggctctctgcccatagcatcccatcttgcgcattgccgtcgccggttatgccatgccagcgccagagttgcttactcgccatgcggcatccccagtacgcggattaactcttcaaaggtggttaagccttgctctacggccaggcagccgttttcaaaaagcgtacgcatacccgcctgtcgtgcgtgcgtttccagcgattcaacgtcggtattagcggaaataagctgacgaatgaccggcgttatgggcagaacttcaaataaggccgtacgaccataaaaaccgtggtagcaatgtacacaaccgggtgcctgccagtggggcagcggcgatggccatacattgtctggaatgtggatgggctccccttgctgccggcgacaatgtgggcaaagtttgcgtaccagacgctgggctattaccagcgtaagcgccgatgatagcatccagcgggcgacccccatttgctgtaaacgtaccagcgtttcgcaggtggaattagtgtgtagggtagacaacaccaggtgaccagtttgcgccgctttaatagcgatctctgctgtttcgccatcgcggatctctccgatcatgatgacgtcaggatcctggcgcaataacgcacgcaaaacgccctgaaaggtgagtccggcacgcggatggatttgcgtctggtttagtccggctatggggatctcaactggatcttcgacgctacaaatattaatgtcagcggtattcagcttttgcagggcactataaagcgtgaccgttttgccgctgccggtagggccagttaccagcaccagtccctgtggttgttgcaaggcatgagcaaagtccgccagttgtaacggctgcattccaagcgtgttgacatccagtgcctgacccacctgctgtaacaaccttaataccaccttttcaccaccccgacatggtaaggtcgcaatacgaaatgagacggcgtttcctgccagttcgacagtgaattgcccgtcctgcggcaggcgatgttccgcaatatccaggtttcccagcacttttaatctggcggttaatgcgactccggcatccggtgaaacatccggtaaaggatgcaatacgccgtcgatacgcaagcggatgcggtaggcattgtccgctggttcgatatgaatatcagacgcgcgttgttccagcgcagattgtaacgttcgagttagcaactctgctttgggctgatgcttctcctgaacagctacgggcaatgtctgttgtgtgcgactggcgtgaccttccatttgttggcgcgtccagcaggtgatctcaatacgtttggtggtagcgaaatgcaatgcgtccagtagctcatgcgaaggtgcatcgactaccgcaacatgaaccacctcttcgctggcatccagcaagactccatgataacgcagacacagggcagtgagctgtggaatattcattgccgctccttagttggcgtcatcaaagcggaagacatcttcgcaggcttgctgcaatgcgctgtcactttgaatattgcagttgcgcgtccagccggtgacgccgtttgcgttatcccaacccggtgtcatgacgacgcttagcccattgagactttcttgcccggtcagcgacaccacgccctttgccacactcatggctgaaacatagcgggtggtggtaggcgagggaatgccattgctgccaccgtcgcaggtatctaatccaccatgttccagcgcgcacaactctacggcggtacggtaaggcacaaaggtttgtagcatgtcggtgagtgcggctttgcgcaggtagttttgataagcgggaataccaatggcgcttaaaatggcaatgatgccaataaccaccatcagttcgataagtgtaaaaccgcgttgcttgtccatctgtttcgctccttgatttggttggcgctactttggcaaacgccatcagcacaggcgaggggcaaaaaacgaaacgggaaagcagattccgaggttttttatttcgttgcagcgaaagacaagaaatttgcgaggcgttacgaagaaagttggggaaggggagattatccgcccgcgatggagcggataaatctgtcaactattagcgaaaacgcattgaaaggtcgagtgcttgtacgtgtttagttagcgcaccgacggagataaagtccacgcccgtttcggcaaattcacgcagtgttttgtcagtgacgttgccagacacttccagtagcgccttgccgttggtgcgtttgacggcttcgcgcatctgttctgtttcgaagttatccagcatgatgatatcggctcctgctttcagggcttcatcaagttcttccagattctctacttcgacttctactggcgcatccgggtgcagccaggacgctttttcgaccgcctggcgcactgagccggaggcaataatatggttttctttgatcaggaaggcatcagaaagccccagacggtgattcgctccgccgccgcaaagtaccgcgtatttcagagctgaacgcaggccgggtaaggttttgcgcgtatccaacaactgcgtgttggtgccttccagcaattcgacatagtggcgtaccttactggcaactcctgaaagggtttgcacaaaattaagcgcagtgcgttcgcccgttaacagcacgcgggatgggccttcaagttcgaacaaggattgattggcattgatgacatcgccgtcatccacatgccagattatggtgacatcgtcgcctgccagttgaataaacacctcttcaacccagcgtttgccgcaaaagacgccattctcgcgggtgatcaccgtggcatgagagcgagaattttccggtaaaagttttgccgtaatatcattgttggcatcgactgttccgcctaaatcttcccgcagcgcctgggccaccgcgccggggatatcgagattaatgcgttccagcagctcgtcacgtcgggtgtcagggttatagcggcgaggcggcatgttaaaactccagatagctaacgaatcataaggtagaaacatgctactctgaaccgggtattagcaccacatataaggagatcctgcatgttgttagaacaggggtggctggttggcgcgcgccgcgttccctcaccacattacgattgccgcccggatgacgaaacacccaccctgctggtggtgcacaatattagcctgccgccaggcgagtttggcggtccgtggatcgacgcattattcactggaactattgatccgcaggcacatcctttctttgctgagatcgcccatttgcgcgtctccgctcactgtttgattcgccgtgatggtgaaatagtccagtatgttcctttcgataaacgtgcatggcatgcgggagtctctcagtatcaggggcgcgaacgctgcaatgatttttctattgggattgagcttgaaggcaccgatacgctggcgtataccgatgcgcagtatcaacagcttgcggcggttacgcgggcactgattgattgctatccggatatcgctaaaaacatgacgggccattgtgatattgcgccggatcggaaaaccgatcccggtcctgcatttgattgggcacggtttcgtgtgctggtcagcaaggagacaacatgacgctatttacaaccttactggtgttaattttcgagcgcctgtttaagttgggcgagcactggcagcttgatcatcgtcttgaagcgttctttcggcgggtgaaacatttttctctcgggcgcacgttaggcatgaccattattgcgatgggcgtgacttttttactgttacgcgcattgcagggagtattgttcaacgttcccacgctactggtgtggctgctgattggtttgctgtgtattggcgcaggtaaagttcgtcttcattatcatgcttatctgacagctgcttcacgtaatgatagccatgcccgtgccacgatggctggcgaactcaccatgattcacggcgtcccggcaggctgcgacgaacgtgagtatttgcgtgagctgcaaaatgcattgctgtggattaactttcgtttttatcttgcaccgctgttctggctgattgtggggggaacctggggacccgttacgctgatggggtatgcgtttttgcgtgcatggcaatactggctggcgcgatatcagacgccgcatcatcgtttacagtccggcattgatgccgtgcttcatgtactggattgggtgccggttcgtcttgcgggtgtggtatatgccttgatcggtcatggtgagaaagcgttaccggcctggtttgcttcgctgggtgatttccatacttcgcagtatcaggtgttaacgcgtctggcgcagttctctctggcgcgtgaaccgcatgtcgataaggtggagacgccgaaggcagcggtttcaatggcgaagaaaacctcgttcgtggtcgtggtggtgattgcactactgacgatttacggggcgttggtgtaaagattattgccctcaccctgtacgggtgagggcgtagagagattaatgcgcttttacggctttggcggttttctctttaaacagatagccgatacctaacacgatcagccataccgggatcaggtataccgaaatcgccattcctggggtcatcagcataatcaccagtaccgccgccataaacagcaggcagatccagttacccagcggataaagcagagcagggaagcgagttaccacgccttgttcctgcttggcgcgacggaatttcatatgcgccaggctaatcatcgcccagttgattaccagtgcagataccaccagcgccattaacagtccgaaagcggactctggggcaaggtagttaatcagtacgcacaacgccgttaccagtgcagacaccagaatggtatttactggtacaccacgtttatcgacagacgccagcgcttttggcgcattaccctgttgtgccagaccaaacagcatacggctgttgcaatatacgcagctgttgtacacggagagcgccgcagtcagtaccacgatgttcagcgcattcgccacaaaggtatcgcctaactcgtggaagatcagcacaaacggactggtatcggcggtaacgcgggtccacggcatcagtgagagcagaacggctaacgaaccaatatagaaaatcaggatgcggtagataacctggttagttgctttcggtatactttgctccgggttatcagcttctgctgcggtgatccccaccagttccagaccaccgaacgagaacatgataatcgccatcatcatcaccagcccggtgaagccgtgcggcaggaaaccaccctgatcccacaggttgctaacggtcgcctgcgggccgccgttgccactgaatagcagccagccgccgaagatgatcatcgctaccaccgcgataactttgataatggcaaaccagaactccatctcgccaaacactttaacgttggtcaggttgatggcgttaatcaccacaaagaatacggcggcagaaacccaggtggggatttccggataccagaactgaatgtatttacccacggcagtcagctcagccatggcaactaaaacgtacagtacccagtagttccagccagaggcgaaaccggcaaaactgccccagtatttataagcaaagtggctaaaggagcctgcgacaggttcttcgaccaccatttcacccagctgacgcatgatcagaaaggcgataaaaccagcaatggcgtaacccaggataatccctggccctgcggactgtattacggaggcgctacccaggaataacccggtccctatcgcgccacccagcgcgataagctgaatatggcggtttttaaggccgcgctttagctgctcgccgtgctgttgaccttccatcatgaaacctcgtgcggtggttgtttttttgatctacgcagtgatgcgtgtgtaagtttgcaattccgtttgttgtattaatttgtttacatcaaagaagtttgaattgttacaaaaagacttccgtcagatcaagaataatggtatgcggcagcgaatgcacccgctttatgcatggttgaagatgagttgcttaaaaagaaaccgtttgtaaagctcagcctcaacccctctcaatatgtagaatgaatttaaattcgttttaattgaattaaaaatcacaaaattggtaagtgaatcggttcaattcggatttttatagtttaataatcgttaaaaaactcctttcctacgtaaagtctacatttgtgcatagttacaactttgaaacgttatatatgtcaagttgttaaaatgtgcacagtttcatgatttcaatcaaaacctgtatggacataaggtgaatactttgttactttagcgtcacagacatgaaattggtaagaccaattgacttcggcaagtggcttaagacaggaactcatggcctacagcaaaatccgccaaccaaaactctccgatgtgattgagcagcaactggagtttttgatcctcgaaggcactctccgcccgggcgaaaaactcccaccggaacgcgaactggcaaaacagtttgacgtctcccgtccctccttgcgtgaggcgattcaacgtctcgaagcgaagggcttgttgcttcgtcgccagggtggcggcacttttgtccagagcagcctatggcaaagcttcagcgatccgctggtggagctgctctccgaccatcctgagtcacagtatgacttgctcgaaacacgacacgccctggaaggtatcgccgcttattacgccgcgctgcgtagtaccgatgaagacaaggaacgcatccgtgaactccaccacgccatagagctggcgcagcagtctggcgatctggacgcggaatcaaacgccgtactccagtatcagattgccgtcaccgaagcggcccacaatgtggttctgcttcatctgctaaggtgtatggagccgatgttggcccagaatgtccgccagaacttcgaattgctctattcgcgtcgcgagatgctgccgctggtgagtagtcaccgcacccgcatatttgaagcgattatggccggtaagccggaagaagcgcgcgaagcatcgcatcgccatctggcctttatcgaagaaattttgctcgacagaagtcgtgaagagagccgccgtgagcgttctctgcgtcgtctggagcaacgaaagaattagtgatttttctggtaaaaattatccagaagatgttgtaaatcaagcgcatataaaagcgcggcaactaaacgtagaacctgtcttattgagctttccggcgagagttcaatgggacaggttccagaaaactcaacgttattagatagataaggaataacccatgtcagaacgtttcccaaatgacgtggatccgatcgaaactcgcgactggctccaggcgatcgaatcggtcatccgtgaagaaggtgttgagcgtgctcagtatctgatcgaccaactgcttgctgaagcccgcaaaggcggtgtaaacgtagccgcaggcacaggtatcagcaactacatcaacaccatccccgttgaagaacaaccggagtatccgggtaatctggaactggaacgccgtattcgttcagctatccgctggaacgccatcatgacggtgctgcgtgcgtcgaaaaaagacctcgaactgggcggccatatggcgtccttccagtcttccgcaaccatttatgatgtgtgctttaaccacttcttccgtgcacgcaacgagcaggatggcggcgacctggtttacttccagggccacatctccccgggcgtgtacgctcgtgctttcctggaaggtcgtctgactcaggagcagctggataacttccgtcaggaagttcacggcaatggcctctcttcctatccgcacccgaaactgatgccggaattctggcagttcccgaccgtatctatgggtctgggtccgattggtgctatttaccaggctaaattcctgaaatatctggaacaccgtggcctgaaagatacctctaaacaaaccgtttacgcgttcctcggtgacggtgaaatggacgaaccggaatccaaaggtgcgatcaccatcgctacccgtgaaaaactggataacctggtcttcgttatcaactgtaacctgcagcgtcttgacggcccggtcaccggtaacggcaagatcatcaacgaactggaaggcatcttcgaaggtgctggctggaacgtgatcaaagtgatgtggggtagccgttgggatgaactgctgcgtaaggataccagcggtaaactgatccagctgatgaacgaaaccgttgacggcgactaccagaccttcaaatcgaaagatggtgcgtacgttcgtgaacacttcttcggtaaatatcctgaaaccgcagcactggttgcagactggactgacgagcagatctgggcactgaaccgtggtggtcacgatccgaagaaaatctacgctgcattcaagaaagcgcaggaaaccaaaggcaaagcgacagtaatccttgctcataccattaaaggttacggcatgggcgacgcggctgaaggtaaaaacatcgcgcaccaggttaagaaaatgaacatggacggtgtgcgtcatatccgcgaccgtttcaatgtgccggtgtctgatgcagatatcgaaaaactgccgtacatcaccttcccggaaggttctgaagagcatacctatctgcacgctcagcgtcagaaactgcacggttatctgccaagccgtcagccgaacttcaccgagaagcttgagctgccgagcctgcaagacttcggcgcgctgttggaagagcagagcaaagagatctctaccactatcgctttcgttcgtgctctgaacgtgatgctgaagaacaagtcgatcaaagatcgtctggtaccgatcatcgccgacgaagcgcgtactttcggtatggaaggtctgttccgtcagattggtatttacagcccgaacggtcagcagtacaccccgcaggaccgcgagcaggttgcttactataaagaagacgagaaaggtcagattctgcaggaagggatcaacgagctgggcgcaggttgttcctggctggcagcggcgacctcttacagcaccaacaatctgccgatgatcccgttctacatctattactcgatgttcggcttccagcgtattggcgatctgtgctgggcggctggcgaccagcaagcgcgtggcttcctgatcggcggtacttccggtcgtaccaccctgaacggcgaaggtctgcagcacgaagatggtcacagccacattcagtcgctgactatcccgaactgtatctcttacgacccggcttacgcttacgaagttgctgtcatcatgcatgacggtctggagcgtatgtacggtgaaaaacaagagaacgtttactactacatcactacgctgaacgaaaactaccacatgccggcaatgccggaaggtgctgaggaaggtatccgtaaaggtatctacaaactcgaaactattgaaggtagcaaaggtaaagttcagctgctcggctccggttctatcctgcgtcacgtccgtgaagcagctgagatcctggcgaaagattacggcgtaggttctgacgtttatagcgtgacctccttcaccgagctggcgcgtgatggtcaggattgtgaacgctggaacatgctgcacccgctggaaactccgcgcgttccgtatatcgctcaggtgatgaacgacgctccggcagtggcatctaccgactatatgaaactgttcgctgagcaggtccgtacttacgtaccggctgacgactaccgcgtactgggtactgatggcttcggtcgttccgacagccgtgagaacctgcgtcaccacttcgaagttgatgcttcttatgtcgtggttgcggcgctgggcgaactggctaaacgtggcgaaatcgataagaaagtggttgctgacgcaatcgccaaattcaacatcgatgcagataaagttaacccgcgtctggcgtaagaggtaaaagaataatggctatcgaaatcaaagtaccggacatcggggctgatgaagttgaaatcaccgagatcctggtcaaagtgggcgacaaagttgaagccgaacagtcgctgatcaccgtagaaggcgacaaagcctctatggaagttccgtctccgcaggcgggtatcgttaaagagatcaaagtctctgttggcgataaaacccagaccggcgcactgattatgattttcgattccgccgacggtgcagcagacgctgcacctgctcaggcagaagagaagaaagaagcagctccggcagcagcaccagcggctgcggcggcaaaagacgttaacgttccggatatcggcagcgacgaagttgaagtgaccgaaatcctggtgaaagttggcgataaagttgaagctgaacagtcgctgatcaccgtagaaggcgacaaggcttctatggaagttccggctccgtttgctggcaccgtgaaagagatcaaagtgaacgtgggtgacaaagtgtctaccggctcgctgattatggtcttcgaagtcgcgggtgaagcaggcgcggcagctccggccgctaaacaggaagcagctccggcagcggcccctgcaccagcggctggcgtgaaagaagttaacgttccggatatcggcggtgacgaagttgaagtgactgaagtgatggtgaaagtgggcgacaaagttgccgctgaacagtcactgatcaccgtagaaggcgacaaagcttctatggaagttccggcgccgtttgcaggcgtcgtgaaggaactgaaagtcaacgttggcgataaagtgaaaactggctcgctgattatgatcttcgaagttgaaggcgcagcgcctgcggcagctcctgcgaaacaggaagcggcagcgccggcaccggcagcaaaagctgaagccccggcagcagcaccagctgcgaaagcggaaggcaaatctgaatttgctgaaaacgacgcttatgttcacgcgactccgctgatccgccgtctggcacgcgagtttggtgttaaccttgcgaaagtgaagggcactggccgtaaaggtcgtatcctgcgcgaagacgttcaggcttacgtgaaagaagctatcaaacgtgcagaagcagctccggcagcgactggcggtggtatccctggcatgctgccgtggccgaaggtggacttcagcaagtttggtgaaatcgaagaagtggaactgggccgcatccagaaaatctctggtgcgaacctgagccgtaactgggtaatgatcccgcatgttactcacttcgacaaaaccgatatcaccgagttggaagcgttccgtaaacagcagaacgaagaagcggcgaaacgtaagctggatgtgaagatcaccccggttgtcttcatcatgaaagccgttgctgcagctcttgagcagatgcctcgcttcaatagttcgctgtcggaagacggtcagcgtctgaccctgaagaaatacatcaacatcggtgtggcggtggataccccgaacggtctggttgttccggtattcaaagacgtcaacaagaaaggcatcatcgagctgtctcgcgagctgatgactatttctaagaaagcgcgtgacggtaagctgactgcgggcgaaatgcagggcggttgcttcaccatctccagcatcggcggcctgggtactacccacttcgcgccgattgtgaacgcgccggaagtggctatcctcggcgtttccaagtccgcgatggagccggtgtggaatggtaaagagttcgtgccgcgtctgatgctgccgatttctctctccttcgaccaccgcgtgatcgacggtgctgatggtgcccgtttcattaccatcattaacaacacgctgtctgacattcgccgtctggtgatgtaagtaaaagagccggcccaacggccggcttttttctggtaatctcatgaatgtattgaggttattagcgaatagacaaatcggttgccgtttgttgtttaaaaattgttaacaattttgtaaaataccgacggatagaacgacccggtggtggttagggtattacttcacataccctatggatttctgggtgcagcaaggtagcaagcgccagaatccccaggagcttacataagtaagtgactggggtgagggcgtgaagctaacgccgctgcggcctgaaagacgacgggtatgaccgccggagataaatatatagaggtcatgatgagtactgaaatcaaaactcaggtcgtggtacttggggcaggccccgcaggttactccgctgccttccgttgcgctgatttaggtctggaaaccgtaatcgtagaacgttacaacacccttggcggtgtttgcctgaacgtcggctgtatcccttctaaagcactgctgcacgtagcaaaagttatcgaagaagccaaagcgctggctgaacacggtatcgtcttcggcgaaccgaaaaccgatatcgacaagattcgtacctggaaagagaaagtgatcaatcagctgaccggtggtctggctggtatggcgaaaggccgcaaagtcaaagtggtcaacggtctgggtaaattcaccggggctaacaccctggaagttgaaggtgagaacggcaaaaccgtgatcaacttcgacaacgcgatcattgcagcgggttctcgcccgatccaactgccgtttattccgcatgaagatccgcgtatctgggactccactgacgcgctggaactgaaagaagtaccagaacgcctgctggtaatgggtggcggtatcatcggtctggaaatgggcaccgtttaccacgcgctgggttcacagattgacgtggttgaaatgttcgaccaggttatcccggcagctgacaaagacatcgttaaagtcttcaccaagcgtatcagcaagaaattcaacctgatgctggaaaccaaagttaccgccgttgaagcgaaagaagacggcatttatgtgacgatggaaggcaaaaaagcacccgctgaaccgcagcgttacgacgccgtgctggtagcgattggtcgtgtgccgaacggtaaaaacctcgacgcaggcaaagcaggcgtggaagttgacgaccgtggtttcatccgcgttgacaaacagctgcgtaccaacgtaccgcacatctttgctatcggcgatatcgtcggtcaaccgatgctggcacacaaaggtgttcacgaaggtcacgttgccgctgaagttatcgccggtaagaaacactacttcgatccgaaagttatcccgtccatcgcctataccgaaccagaagttgcatgggtgggtctgactgagaaagaagcgaaagagaaaggcatcagctatgaaaccgccaccttcccgtgggctgcttctggtcgtgctatcgcttccgactgcgcagacggtatgaccaagctgattttcgacaaagaatctcaccgtgtgatcggtggtgcgattgtcggtactaacggcggcgagctgctgggtgaaatcggcctggcaatcgaaatgggttgtgatgctgaagacatcgcactgaccatccacgcgcacccgactctgcacgagtctgtgggcctggcggcagaagtgttcgaaggtagcattaccgacctgccgaacccgaaagcgaagaagaagtaatttttcgtttgccggaacatccggcaattaaaaaagcggctaaccacgccgctttttttacgtctgcaatttacctttccagtcttcttgctccacgttcagagagacgttcgcatactgctgaccgttgctcgttattcagcctgacagtatggttactgtcgtttagacgttgtgggcggctctcctgaactttctcccgaaaaacctgacgttgttcaggtgatgccgattgaacacgctggcgggcgttatcacgttgctgttgattcagtgggcgctgctgtactttttccttaaacacctggcgctgctctggtgatgcggactgaatacgctcacgcgctgcgtctcttcgctgctggttctgcgggttagtctgcattttctcgcgaaccgcctggcgctgctcaggcgaggcggactgaatgcgctcacgcgctgcctctcttcgctgctggatcttcgggttagtctgcattctctcgcgaactgcctggcgctgctcaggcgaggcggactgataacgctgacgagcggcgtccttttgttgctgggtcagtggttggcgacggctgaagtcgtggaagtcgtcatagctcccatagtgttcagcttcattaaaccgctgtgccgctgcctgacgttgggtatctcgtgtaatgactggtgcggcgtgtgttcgttgctgaaactgatttgctgccgcctgacgctggctgtcgcgcgttggggcaggtaattgcgtggcgctcattccgccgttgacatcggtttgatgaaaccgctttgccatatcctgatcatgatagggcacaccattacggtagtttggattgtgccgccatgccatattcttatcagtaagatgctcaccggtgatacggttgaaattgttgacgtcgatattgatgttgtcgccgttgtgttgccagccattaccgtcacgatgaccgccatcgtggtgatgataatcatcattgtcatgatgatgatggtcatgatcgtcgtcgtcccagtcgatgctgctgaatagtgcgtacgtggtagcaacgcccatgctatagccgaatccgcgtacaaagctgtcaacaaacggttctccggctggtggtggcagataaaccggcggatacgcagtattggcccagttcccgtaaaccacggttgggttgtagttgggaatatagaccacatcaggattggcgggctcaatggaaatgacggttgttgccggctctgtaatgacggggttggcagttaaaactgtattggatggtatgacgggtgccgtgactgtctgttttaccggtacagctttcttcgttgtggtaataactttctgttcggttgatgacttcagcgagccggtttgttgcgccagttgccgcaatcgctgtaccgagtccatcacgtcctgcggctgggccagaaaagcatcgcccaggttttgcacccattgcgggttttcgcccatcaatgccatcaattgtggaaaggccaccagtgatttaacgctggcgtcccacggctggtcagataccgcctgaatagcagcatcgccttgtttaagtggattatcgtgcgaccattgcactgcttgagcaacgtttgtcggataggttgatgccatcagcacctgcgaaagtagggcgtcgggatacagcgcgacgggcgcgacccattgatctatttgtgcagtgctgaatgcggatttgacgacggcgggtgttacgggaggtgcggaaaccgttgcaggaaacgtaaccgcggcagcgtcagacacagccagttgtgtcgattgcggttccacaggcgcttccactgtgcggctttttatatatagcccggtagaggcggcacaaagcccggcactgcaaattagcgccagcacatggggtttaaacggcaaagtcattttcataattcggatctcaaggaaatcgcaatggtcggcgaactgccacccgcaggtgctgtgaatccgagtataaagaggcggtagtttaaattttgactaatcttgggattcgttgagaaaggtgattatcaccatgcgaattaacgaagtttttacggagggaaacaatctctagaccatccttaacgattcagccacttttttatgttgcttttttgtaaacagattaacacctcgtcaaaatcctgctattctgcccgttgcggtactgggcatttaccctacaaactgctgtctcacaggagcgtgaagagaatcgcctgccgcactatgacaatgagagcgaggagaaccgtcgtgctagaagaataccgtaagcacgtagctgagcgtgccgctgaggggattgcgcccaaacccctggatgcaaaccaaatggccgcacttgtagagctgctgaaaaacccgcccgcgggcgaagaagaattcctgttagatctgttaaccaaccgtgttcccccaggcgtcgatgaagccgcctatgtcaaagcaggcttcctggctgctatcgcgaaaggcgaagccaaatcccctctgctgactccggaaaaagccatcgaactgctgggcaccatgcagggtggttacaacattcatccgctgatcgacgcgctggatgatgccaaactggcacctattgctgccaaagcactttctcacacgctgctgatgttcgataacttctatgacgtagaagagaaagcgaaagcaggcaacgaatatgcgaagcaggttatgcagtcctgggcggatgccgaatggttcctgaatcgcccggcgctggctgaaaaactgaccgttactgtcttcaaagtcactggcgaaactaacaccgatgacctttctccggcaccggatgcgtggtcacgcccggatatcccactgcacgcgctggcgatgctgaaaaacgcccgtgaaggtattgagccagaccagcctggtgttgttggtccgatcaagcaaatcgaagctctgcaacagaaaggtttcccgctggcgtacgtcggtgacgttgtgggtacgggttcttcgcgtaaatccgccactaactccgttctgtggtttatgggcgatgatattccacatgtgccgaacaaacgcggcggtggtttgtgcctcggcggtaaaattgcacccatcttctttaacacgatggaagacgcgggtgcactgccaatcgaagtcgacgtctctaacctgaacatgggcgacgtgattgacgtttacccgtacaaaggtgaagtgcgtaaccacgaaaccggcgaactgctggcgaccttcgaactgaaaaccgacgtgctgattgatgaagtgcgtgctggtggccgtattccgctgattatcgggcgtggcctgaccaccaaagcgcgtgaagcacttggtctgccgcacagtgatgtgttccgtcaggcgaaagatgtcgctgagagcgatcgcggcttctcgctggcgcaaaaaatggtaggccgtgcctgtggcgtgaaaggcattcgtccgggcgcgtactgtgaaccgaaaatgacttctgtaggttcccaggacaccaccggcccgatgacccgtgatgaactgaaagacctggcgtgcctgggcttctcggctgacctggtgatgcagtctttctgccacaccgcggcgtatccgaagccagttgacgtgaacacgcaccacacgctgccggacttcattatgaaccgtggcggtgtgtcgctgcgtccgggtgacggcgtcattcactcctggctgaaccgtatgctgctgccggataccgtcggtaccggtggtgactcccatacccgtttcccgatcggtatctctttcccggcgggttctggtctggtggcgtttgctgccgcaactggcgtaatgccgcttgatatgccggaatccgttctggtgcgcttcaaaggcaaaatgcagccgggcatcaccctgcgcgatctggtacacgctattccgctgtatgcgatcaaacaaggtctgctgaccgttgagaagaaaggcaagaaaaacatcttctctggccgcatcctggaaattgaaggtctgccggatctgaaagttgagcaggcctttgagctaaccgatgcgtccgccgagcgttctgccgctggttgtaccatcaagctgaacaaagaaccgatcatcgaatacctgaactctaacatcgtcctgctgaagtggatgatcgcggaaggttacggcgatcgtcgtaccctggaacgtcgtattcagggcatggaaaaatggctggcgaatcctgagctgctggaagccgatgcagatgcggaatacgcggcagtgatcgacatcgatctggcggatattaaagagccaatcctgtgtgctccgaacgacccggatgacgcgcgtccgctgtctgcggtacagggtgagaagatcgacgaagtgtttatcggttcctgcatgaccaacatcggtcacttccgtgctgcgggtaaactgctggatgcgcataaaggtcagttgccgacccgcctgtgggtggcaccgccaacccgtatggacgccgcacagttgaccgaagaaggctactacagcgtcttcggtaagagtggtgcgcgtatcgagatccctggctgttccctgtgtatgggtaaccaggcgcgtgtggcggacggtgcaacggtggtttccacctctacccgtaacttcccgaaccgtctgggtactggcgcgaatgtcttcctggcttctgcggaactggcggctgttgcggcgctgattggcaaactgccgacgccggaagagtaccagacctacgtggcgcaggtagataaaacagccgttgatacttaccgttatctgaacttcaaccagctttctcagtacaccgagaaagccgatggggtgattttccagactgcggtttaaaaagtcagcgcacgcgctgcgcataaacgacacaatgcccggtgaatgagattcccgggcatttttttatttctaaaccatcgccgttccgctgtttttctccggtaaggctgcgataattacatcaatggcgcaatgcgatttcggtgcattgccgggagcagaggaacacactatggattacgaatttctgcgcgatattaccggagtggtaaaggtgcgtatgtccatggggcatgaagtggtcgggcactggtttaatgaagaggtgaaagaaaacctggccttgcttgatgaagtggaacaagcagcgcacgcactgaaaggtagcgaacggtcctggcaacgggcagggcatgaatacaccctgtggatggacggtgaagaggtgatggttcgcgccaatcaactggaattcgctggcgatgaaatggaagaggggatgaactactacgacgaagaaagcctgtcgctatgcggcgttgaggattttctgcaggtcgtggcggcttaccgcaatttcgtgcagcagaagtaaataaatctggcggagcctgggagctccgccagagccgttaaacagctggcatattgcgcccgtaataaatctcgcgcatttctttccacagcgcagcggtaatttcctggcgctcgctgtcggttaagtcttccggtttggtgtggaacatgtagtgcttaaggtcgaactctttaagcaacatcttggtatggaagatattttcctgatagacgttcacatccaccatgtcatacagcgccttcatatcgtcagacataaagttctgaatcgaattaatctcatggtcgataaagtgcttcataccgttaatgtcgcgggtaaaaccgcgcacgcgataatcaatggttacgatatcggactcaagctggtggatcaggtaattcagcgccttcagcggagaaatcacgccgcaggtagagacttcaatatcggcgcggaaggtacataaaccgccttcaggatgactttccgggtaggtatgtacgcaaatatgacttttatcaagatgggcaacgaccgtttctggcagtgggccggggtgttctgttttgtcgatgagtttcgggtcaaccggttcttcactcaccagaatagtgacgctggcaccctgtggttcgtaatcctggcgggcgatgttaagaatattagccccgataatggaacaggtttctgacaggatttcggtcagacggttggcattatagagttcatcgatataagcaatataaccgtcgcgctcttcggcagttttggcgtagcagatatcgtaaatacaaaaactcagacttttggtcagattattaaagccatgcagtttcagttttttcaatttcttatcttctccttaggacggctgtgaagccagtgcgtcttgcagatactgaggtaaggcaaaagctgccgtatggattgccggattgtaataacggcatttcaggccagaggcgagaaaacgcgcctgaataatttcggttgagagatggcgtaaggcgtcgttatctgtcgcccatgcaaaagtcatgataccgccgtaataggtcgggatcgccgcctgataaaagccaacgtcgctgaagtaatggctgagtttgcgatggctgtcgatggcttcttcctgctgtaaaaagcagacgccgttttgtgcgacgaagataccgccaggattcaggcaacgtttgcagccttcataaaatgccgaagtgaaaaggctttcgccgggaccgataggatcggtgcagtcggagataatgacatcaaaggtctggctggtttgattaacgaaattgacgccatcgtcgatcaccagcttaaagcgcggatcgtcgtagctaccggcgttatggttgggtagatactgacggcagaacgatacgacacccgcatcgatttccaccatcgtgattgactcaacgtttttatgtcgggttacttcacgcagcatggcaccgtcgccgccgccgataatcagcacatgtttcgcgtgaccatgggccagtagcggaacatgggtcatcatctcatgatagataaactcgtcgcgctcggtggtttgtactacgccatccagcgccattacgcgaccaaatgcagcgttctcaaaaatgatcagatcctggtgatcggtcttttcatgatacagaacgttatctaccgcaaagtactgcccaaactggtcgtgtagcgtttcatgccactgttttttttcggccatgggttgatacctcctttgttaacacccgtaaaaaaagggcgcaacataatagctaacattgaccgcggatgcacggtcaatatttctacaaaaaggtatcagggattatttgacgtaggcaagcaggcttaaggaatcgcgggccagggctttgcattttttagcgacgggaatgccaatgccgctgagatcgcggtagctgtcttcaccgagggctttcatgtcgaaggtgtcgtaattactgaggtcccactggttttgctgagcgaaaaagaccagtgcgcgacgaatttgcccgttaggtaagttctggtaaccacaatcgttcttcagaaagacaaaaactgccgttaaatcggccatatcttcggcttcagactcgctgagcgcgtaactgtttgcgcagacggccatcaggctgccgaataacactgttctgaaaaacgtcttcattgcttctaccaggggcttaaagaagataaacgttagcacactgcgagcgaggcgacgaccattattgtcgattaaattgtgtctgcggcttgaccttcccgtaaggggaaggactatgctcaacgtttgattttgtttcgcctgcttaagaataaggaaataactatgcaacgtcgtgatttcttaaaatattccgtcgcgctgggtgtggcttcggctttgccgctgtggagccgcgcagtatttgcggcagaacgcccaacgttaccgatccctgatttgctcacgaccgatgcccgtaatcgcattcagttaactattggcgcaggccagtccacctttggcgggaaaactgcaactacctggggctataacggcaatctgctggggccggcggtgaaattacagcgcggcaaagcggtaacggttgatatctacaaccaactgacggaagagacaacgttgcactggcacgggctggaagtaccgggtgaagtcgacggcggcccgcagggaattattccgccaggtggcaagcgctcggtgacgttgaacgttgatcaacctgccgctacctgctggttccatccgcatcagcacggcaaaaccgggcgacaggtggcgatggggctggctgggctggtggtgattgaagatgacgagatcctgaaattaatgctgccaaaacagtggggtatcgatgatgttccggtgatcgttcaggataagaaatttagcgccgacgggcagattgattatcaactggatgtgatgaccgccgccgtgggctggtttggcgatacgttgctgaccaacggtgcaatctacccgcaacacgctgccccgcgtggttggctgcgcctgcgtttgctcaatggctgtaatgcccgttcgctcaatttcgccaccagcgacaatcgcccgctgtatgtgattgccagcgacggtggtctgctacctgaaccagtgaaggtgagcgaactgccggtgctgatgggcgagcgttttgaagtgctggtggaggttaacgataacaaaccctttgacctggtgacgctgccggtcagccagatggggatggcgattgcgccgtttgataagcctcatccggtaatgcggattcagccgattgctattagtgcctccggtgctttgccagacacattaagtagcctgcctgcgttaccttcgctggaagggctgacggtacgcaagctgcaactctctatggacccgatgctcgatatgatggggatgcagatgctaatggagaaatatggcgatcaggcgatggccgggatggatcacagccagatgatgggccatatggggcacggcaatatgaatcatatgaaccacggcgggaagttcgatttccaccatgccaacaaaatcaacggtcaggcgtttgatatgaacaagccgatgtttgcggcggcgaaagggcaatacgaacgttgggttatctctggcgtgggcgacatgatgctgcatccgttccatatccacggcacgcagttccgtatcttgtcagaaaatggcaaaccgccagcggctcatcgcgcgggctggaaagataccgttaaggtagaaggtaatgtcagcgaagtgctggtgaagtttaatcacgatgcaccgaaagaacatgcttatatggcgcactgccatctgctggagcatgaagatacggggatgatgttagggtttacggtataaaaagaccgtattcggaaatatgcccggatctctccgggcattaaactgatgacaaacgcaaatctgcctgatgcgctacgcttatcaggcctacgctagctgtgcaatccattgattttgcacaattttgtaggctggataaggcgttcacgccgcatccggcatgaacaacgcgcacgttgtcagcaatctgagcaagtcttacttcacatcatccggcagcgcataagccacaatatagtcgcccatcttcgtaccaaatgaaccgtgaccgcctgcggagatcaccacatactgcttaccattcacttcataggtcattggcgtagcctgaccacccgctggtaaacgaccctgccacagtttttcaccgttgctcatgttgtaagcgcgcaggtagttatctgccgtagcggcgataaacagcacgttacccgccgtggagattggcccgcccagcatcggcatacccatattgaacggcaccggaaccggcatcgggaacggcatactgtcctgcggcgtaccaatacgtttcttccacaccacttcattagttttcagatccagcgccgagatataaccccatgctggctgtttacatggcagaccaaatggtgagaggaacgggttgagcgtgacaccatacggtacaccgtactgtggctgaatgccggattccgtacccgtgcctttggcatctttcggctgctccatcgggttgccaggaccacgcgggatcagtttcgaaacaaacggcagtgccattgggttggcaatcgccacttcacgatttggatcaacggaaatcccgccccattcgaacatccccaggttacccgggaagaccagcgtaccctgttcagatggcggggtgaaaatgccttcatagcgcatctggtggaacatcacgcggcacaccagttggtcaaacatggtggctccccacatatccgcaccgctcaaatctttcgtcggacggaagctcagttcagaaaacggttgagttggggttacgtaatcgcctttcgctgcaccttggggaaccggtttttccggtgccggaaccaccagttcgccattacgacgatcgagcacaaaaatgttgccggttttcgccggagcgtaaataactggcactttctgaccattaacggtgatgtccgccagcgtcggctgtgccggaagatccatgtcccacaggtcgtggtgaacggtctggtagctccacgccagtttcccggtagtggcattcagcgccagaatcgagctggcataacgttcctgttccggtgtgcggttaccgccccagatatccggcgtggtcacgcccatcggcagatagaccagatccagcttcgcgtcataggccgctggtgcccaggagtttggcgagttaaaggtaaaggtgtgttcgtcagacgggattgcgttcggatctttcgcgccgggatcaaaagcccacagcagctccccggtgttgacatcaaaaccacggatcacgccagacgtttcgcgggttgagaagttatcggtaactgaaccggccatcacgatggttttatcggtgataatcggtggcgaagtcggttcatacagacccggtttggtgtctggcatattgctttgcagattgagcacgcctttattggcgaaggtttcgcacagtttgccgttttcagcgttaatcgcaatcagtcgaccatcattgaccggaagaatgatacgacgcgggcaatccgccatcacttccggcgaagcggtttctgctttggcttcatgataagagacaccacggcaggttacgtgctggaaagactcgttggttttcagctcaggatcgtaatgccatttctctttgccgctggcggcatcaagcgcaaacaggcgctggtgagcggtacacaggtaaagggtgtcgcccactttaatcggcgtcacttcattggtgatttcacccggatcgttcggctgcttcacatcgccagtacggaacacccaggcttctttcagattatggacgttatcggcgttaatttgtttcagcggcgaaaagcgttgaccttcctgattacgaccataggcaggccagtcctgatcggctacgggggagatagcttcagcaggtgtggcatcggcgcttaaggtgccgttgatctcctgcggatcgttaaatccggcccaggtcaggataccaccgctaatcagcagtgcgaccaccagtgcggcaactgcgccgctggcaggaatgaccaggcgacgccagacaaacggcaggatcagccagatgccgaagaagaccagaatgtcgctgcgcggagtcagcgcccagaagtcgaaaccaacttcccagacgccccaaatcatggtgccgagcagcagggctgcgtatagccaaagcgcggcgcgtttactgcgccacagcatccaggcgacgccgagcatcacaaggccagcgatagggtagtaccaggagccgccaatcgcgaccagccagcctccgccaatgagtagatacagcccgcaaagcgctgcaaaaagggctgttagcgtgacgagtaatcgtcgcgagcctgtattgttaattgccataaagagacaccatttcaattcattaatattttagtagcaattaattataggttttaacatgtgtgatcgtcatcacaattcgagctttattaacagattccgcgaatgaatagttttactggtatactgcgtgtcttgcgctttgttgcggtgccaaaacctgcccgtgcgaagtgatttgtttttaaatcatatggttagagatatgaaacatactgtagaagtaatgatccccgaagcggagattaaagcgcgtatcgccgaactgggtcgtcagattactgagcgttacaaagacagcggcagcgatatggtgctggtgggtctgctgcgtggctcatttatgtttatggcggacctgtgccgtgaagttcaggtatctcatgaagtcgactttatgaccgcctccagctacggtagcggcatgtccaccacccgtgatgtgaaaatcctcaaagatctggatgaagatatccgtggcaaggacgtgctgattgttgaagatatcatcgactcggggaatacactgtcgaaagtgcgtgagatcttaagcctgcgcgaaccgaagtcgctggcgatttgtacgctgctggataaaccgtcccgtcgtgaagtgaacgtcccggtagaatttatcggtttctcgatcccggatgagtttgtggtgggttacggcattgattacgcacagcgttaccgtcatctgccgtatatcggcaaagtgattctgctggacgagtaagtgtgaagttgccggatgtgttgcatccggcatggcatttttatttgtggttggcgtgtttcagcttgaggttggaaatcccgtgacggtaacgttgctcaagggtttcgcggttggtggcggtaacatccagatcacgcagcaagccgtcgtgaatgccgtaggcccagccgtgaatggtaactttctgcccgcgtttccacgctgattgcataatggtggagtggcccaggttatacacctgttccatgacgttcagttcacacaaggtatccagacggcgctcttgcggcatttcgccgagcaatgagctatgtttgaaccagatatcgcggatatgcagcagccagttgttgataagccccagttccgggttttcaactgcggcttgtacgccgccgcaaccgtagtggccacagataataatgtgttcaacttcgagtacatccactgcatactgaaccacggaaaggcagttcaggtcagtgtgaatgaccaggttagcaacattacggtgaacaaagagttcgcccggctcaagaccggttaaacgttctgcaggaacgcgactgtcggaacatccaatccatagaaagcgcggtttttgcgcttgtgccagtttctcaaaaaacccgggatcctcttccaccagcatttttgaccatagtgcattgttgctgatgagtgtatctatgtctttcatggaggttaacgacctgtaaccaaataattacgtttggctaatatagggcaactccgggacgatttaaaccacagataaagtgtaagaacgtaaggtaagtaaaaatttatgaccattgcactggaacttcaacagcttaaaaaaacctatccaggcggcgttcaggcgcttcgtgggatagatttgcaggtcgaagcgggtgatttttatgcgcttctcgggccgaacggggccgggaaatcgaccactatcggtattatcagctctctggtaaataaaacctccgggcgggtcagcgtatttggttacgatctcgagaaggatgtcgtgaacgctaaacgtcagttgggactggtgccgcaggaatttaacttcaacccgtttgaaaccgtgcagcaaattgtggtgaatcaggcagggtactacggcgtggagcgcaaagaagcgtacatccgcagcgaaaagtatcttaaacaactcgatctatggggaaaacgcaacgaacgtgcgcgtatgttatctggcgggatgaagcgccgtttaatgattgcccgtgcgttaatgcatgaacctaaactactgattctcgacgaaccgaccgcaggcgtggatattgaacttcgccgctcaatgtggggctttttgaaggatttaaacgacaaaggcaccaccatcattctcaccacacactacctggaagaagcagaaatgctgtgccgcaatatcggcattattcaacacggtgagctggtggaaaatacctcgatgaaggcgctgctggcgaagctgaaatcggaaacctttattctcgatctcgcaccgaaaagcccgttaccgaagctcgatggctatcagtatcgactggtcgataccgcgacgctggaagttgaagtgctgcgtgagcaggggatcaacagcgtatttacgcagttaagtgagcagggcattcaggtattaagtatgcgtaacaaagctaaccgtctggaagagctgtttgtttcactggttaatgaaaaacaaggagatcgcgcatgatgcatctttactgggtggcgctaaaaagcatctgggcgaaagagatccatcgctttatgcgtatctgggtgcagacgctggtgccgccagtcatcaccatgaccctttactttattatcttcggtaacctgattggttcgcgtattggcgatatgcatggcttcagctatatgcagttcatcgtaccggggctgatcatgatgtcggtgatcaccaatgcctacgccaacgttgcgtcatcattttttggtgccaagttccagcgtaatattgaagagctgctggtagcgccggttccgactcacgtcattattgccggatatgtcggcggtggcgtggcgcgtggtctgtttgttggcattctggtgacggcaatttcactgttttttgtgccatttcaggtgcattcgtgggtattcgttgccttaacgctggtgctcacggcggtgttgttctcccttgcgggtttgctgaacggtgtgtttgccaaaacgttcgatgacatcagcctggtgccaacctttgtgttaacgccactcacgtatttgggcggggtcttttactcactgactttgttgccgccgttctggcaagggctgtcgcacctgaacccaatcgtttatatgatcagtggtttccgctacggcttcctcggtatcaatgatgttccgctggtcactacctttggcgtactggtggtctttattgtggcgttttatttgatctgttggtcgctgatccaacgtggacgtggtttgcgtagctaaggctatttcctctcctctggatttgggggagaggagttttgacggctatcaccctttatcaacaatggtcagggtagactgattttcggctaaggaggaaggcgatgttaggttgggtaattacctgtcacgatgaccgggcgcaagagatactggatgcgctggagaaaaaacatggggcacttcttcagtgccgggccgtgaatttctggcgcggattaagctctaatatgctcagccgcatgatgtgcgatgctctgcatgaagcggactctggtgagggtgtcatcttcttaaccgatatagccggagcgccaccgtatcgcgtggcttcattattaagccacaaacactcccgttgcgaagtgatttctggtgtcacgttaccgttaattgaacagatgatggcttgccgtgaaaccatgaccagttcagagtttcgcgagcgtattgtcgaactgggtgcgccggaggtgagtagtctttggcaccaacaacaaaaaaatccgcctttcgtcctcaaacataatttgtatgagtattaacccgcgattctgatggcgcttttgctacaataaaagcgttgtttcaccctcggttattttttcatgtacaaacaagctgttattctcctgctgatgctgtttaccgcaagtgtcagtgccgcgttacctgcccgttatatgcaaaccatcgaaaatgctgcggtctgggcgcaaattggtgacaagatggtgaccgtggggaatattcgggccggacaaatcattgccgtggagcccactgccgcaagttattacgcatttaattttggctttggcaaaggttttatcgataaaggtcatctcgagccggttcaggggcgacaaaaagttgaagacggtttgggcgacctcaacaagccgctgagtaatcagaacttagttacctggaaagatacgccggtctataacgcgccgagtgcgggaagtgcgccatttggggtactggcggacaatttgcgctacccgattttgcataaactgaaagacaggttaaatcaaacctggtatcagatccgtattggcgatcgactggcctatatcagcgcactggatgcccaacccgataatggcctgtcggtgctaacctatcaccatattctgcgcgacgaagaaaacacccgttttcgccatacttcgacgaccacatcggtacgcgctttcaataaccagatggcctggctgcgtgacaggggatacgcgacactgagcatggtgcagctggaaggctacgtgaagaataagatcaatctccctgcgcgagcggtggtgattacctttgatgatggcctcaagtcggtgagccgctatgcgtatcctgtgttgaaacaatatggcatgaaggcgacggcgtttattgttacctcacgcatcaaacgtcacccgcagaagtggaacccaaaatcgctgcaatttatgagcgtttctgagcttaacgaaattcgcgatgtatttgatttccagtcacatacccattttttgcatcgggtagatggttatcgccgacccatattactgagccgtagtgagcacaatattctgtttgattttgcacgttcacgccgcgctctggcgcaatttaatccgcatgtctggtatctttcgtatccgtttggcggatttaatgacaacgccgtgaaggcagcaaacgatgccggatttcacctggcggtgacaaccatgaaaggcaaagtaaaaccgggggataatccgttgttactaaaacgactttatatcttaagaacggattcgctggagacgatgtcgcggctggtgagtaaccagccgcagggataacaatcaagcaacctgtaccggaatcgctttcgcggtacgtttcatttcattgtcgccttcaaaataggcgacgttgggtcgccaggtgcgagcttcttcatctggcatggtaacgaagctggcgatgatgacaatatcgccgacactggcgcagtgggccgccgcaccgttaacagaaataattctcgaaccgcgttctgccgcgatggcataagtggagaaacgcttgccgttggtgacattccagatatcaatggcttcgttttcgagaataccggctgcgtcaagaaaatcctggtcaatggcgcaagaaccttcatagtgcaggtccgcatgagtcactttcacgcggtggagtttgccctgcagcatcgtgcgaatcataacttctacctttctaccctgtcgttaacgaagcaggcgatgcctgctttgaggaaattctcacgcagtattgcccgatttttgtttagtgtctactcatctgacggcatttgcgtcagcagtttgcgtaccgcgccgaagcgtgccatgtatcgcctgtaacgaattgatatttctctgaacgctgctcggtaaacaataaagaggtggctgacgatagcgcgccttgactggatactgccttcacgcaaagccacacggaagacagggaagatggatgcaccgagtaccacaccgcatgacgcggtatttaaacaatttttaatgcatgcggagacggctcgcgactttctggagatacatttgccagtggaattacgcgaactttgtgacctcaacacgcttcatttagagtcggggagtttcattgaagagagcctgaaaggacacagcacggacgtgctctattccgtgcaaatgcagggcaatcccggttatctgcatgttgtgattgaacaccaaagcaagccggataagaaaatggcctttcgcatgatgcgttattctatagccgccatgcaccggcatctggaggctgaccacgataagctgccgctggtggtgccgatactgttttatcagggcgaggccacaccttatccgctatcaatgtgctggtttgatatgttttactcgccggagctggcgcgacgcgtctataacagtcctttcccgctggtggatatcaccatcacaccggatgacgaaatcatgcaacatcggcggattgcgattctcgaactactgcaaaaacatattcgccagcgcgacttaatgttattgcttgagcaactggtcacgctgatcgacgaagggtacactagcggaagtcagttagttgccatgcaaaactatatgctgcaacgcggtcatactgaacaagcggatttgttttacggtgtgttgagagacagggaaacgggaggggagtctatgatgacgctggcgcagtggtttgaagagaaagggattgagaaggggattcagcagggaagacaggaagtaagtcaggaattcgcccagcgtcttctgagtaaaggaatgtctcgggaagacgttgcagagatggcaaatttacctcttgctgagattgataaggtaattaaccttatttaagttacctgtgttatgacagatgacgtggggtaaattaataactggcgccatcagccgtagcgccagttaagtattacgccagctcgaccattttgttgtcgatcaggcgagcatcgccaagccaggcggctaccagaattactgcccgtttgctggtttcagaaacttccagcaatgtgtcggcatcgcgaatctgaatatcatcggcgcggaagcctttttcattcagttcttgccccgcaatggtaataatttcatcgagatcccgttccccagcctgcaatttgtcagcaatcgaacttaaaactttgtacagaccaggcgcaattttgcgttgttccgccgtcagataaccgttacgggaacttagcgccagaccgtctttggcgcgcataattggcacaccgacaatctcaatatcgaagcccatatcggcaaccattttgcggatcagcgccagttgctgaaaatctttttcaccgaagcaggcgatgtccggctggaccaggttgaacagcttgctgacaatagtcgaaacgccgcgaaaatgtcccggacggctggcaccttccagcatggtcgaaaggccaggaacgtcaacgtaagtgtgggtttcagtaccgttcgggtagatctcttttaccgaaggggcgaaaactaaatccactttacgtttgtttagcttctcgcagtcctcctgcaaggtccgtggataacgagccagatcttccgggcggtcgaactgcatcgggttaacgaaaatactgacgacgaccacatcggcgcgggctttggcttcgtcgaccagcttcatatggccatcgtgcaggttacccatggtaggcaccagcgccacgcgcttgccttccatacgcaggcggcgaatttgctgacgcagcagcggcagggtttcgataattaacacaacgtgactccttaatggaaactgtgttcttcgcccggataaacgccggactccacttcagccatatactgccgcacagccgcgcggatgtcgcccgtttcggcgaggaaatttttagcgaatttaggaatgtgaccgccggtaataccaaaggcgtcgtgcatcacgaggatctgcccgtcagtgacgttgcctgcgccaatgccaataaccgggatcgccagtgcttcggtaatacgttttgccagttcaaccggcacgcattccagcaccagcagctgtgccccagcagcttctaaggctaatgcatcgctgagcagttgatcgcccgcttcatcgccgcgcccctgaactttgtagccaccgaaaatattcactgactgtggtgttaaacctaagtgaccacatacaggaacggcacgttcggtcagcatttgtacggtttctaccagccactcaccgccttcaattttgaccatgttagcaccggcacgcataaccgttgcggcgttttcgaaggcttgttccggcgtggcatacgccataaacggcaggtcagccagcagcaggcagtttggtgcgccgcgacgtacggcggcagtgtggtaggcgatatcggcaacggtaactggcagggtggagtcgtgcccctgaaccgtcatgcccagcgaatcgcccaccagcatgacgttaagcccttcatcagcaaagagtttggcgaagctatagtcataagcggtgatggtcgcgaaacgttttttttcctgtttgtacttctgcagtaaggagatggtggtcggtttcataacgtatcctgataaattgatgttgtgctgtctggcattttatcagtcacattggtgggggcaatgatttatccgtagcagcactgccagaaggtgacagtgctgctacgttatcagggataggttacctggaaagtactggtggctttaaattcgccgggttcgatagcaatattcccgtcttgctttaatgttgcctggaaatgaagaggctgtgatgtgccgttaccttgattagggtaaaccccatcggaggtgtcatcttcggtttcataatctatataaacagaattcgtatcattaggttttaatgtcattagcggatttttactggttgctaaaccttcaatgagtacgccaacgcctttggcggcagtgcttccagtaagcgtattaccaagcagttgtgtgttttgagtacctacttttccagtgacgagttttgtttcaatattacgcacacgaatacaattctgaagcgagatatcaaagggaacaggtgaagcgccatttttaattgtcccagagctatattctcccattctaaccgttgaaccattgactgatggcccggtaagtatggaggtaaaacatgttggtaaggttaatttgacattattcagtgtgaaattgacataaatgtggttgctgtgatctacaacttttgtaccaggactgtaggccttaaacgaataaaggtaatttgatgaactggataactggacttgctgattaagtgtaggatcgaaattagtatctgtataaaattcaacagttatgttgtgtactataccaccaatagcccaaaacttatcgtagtcgtctgctttgttgcaacccttagtttgtagatcgctgtctgtgacggaaaagaaaaattcttggttggaaggatctccgatatagattcctggcgattgaatgtcagttattgtatcgtatgcagaccagacccttgatattaacatggtgtaatacagaccaggaacagatgtattaaatagtttatgtccgccataatctttacctgaatagaccatggcattttcaatagttattggaccaggattcgctctgccagatgtattgcagtaaagaataccaccaccggtacctgtatccaggtatgaccagtacatttttaccccagtcgggccgagctgcgtgggtttataaaaaaccaagttgcttgctgttgatgtgtaattaaaggtcatctgtgcggcagtggaggggcctcgatagttatcaactcctgcattatttcccacaataaaacttgtatatgcactgactgtattacaacaagaatacagtgctaaaaaaagaatgtacctgaagatagtcttcatttttactccaatgtttctttattgttatggtttgcgctgtttttgtttgttattcgtagtaaatatccactaacacatggctcataagttgaccagatgtaacactcaatgcaggatcgattttttgcattcgggtgctaaatttccaggatgaaccattcatgtcatccgacattactggataaacggaacgagatccgcctgaagcattaagaacattgaatgtattcgccgaatcctgagtagaaaatataactactcctacattacttgctcctgacgaaatttcattagcaaatatttgcctagagccagcagccatgacaccgctaagggctctaaaatcaatatgtaactgatttagcacatcgccagttccctgtaatgcacagtcggatacagtgatagtgaactcttttccacctggttgataactttcaggagtaacattacctgaaaaatatcccaccccaacgacgccaagatcaatattaccctggttactgattccgcttttgcaggtgctgttttttacattggcaacaaggtcaatatcctgtccagcaatggctggacaggcgatgcaaaacagtaatgacagaaacagaattattctcttcatcagcttacgttgagtgggatgcatatatagttcctgaatctgtaagtctgttagttataggttactgtaaatgtggctggtgcagaaaacttacccgcagtgacattgtttacggttttatttttttccacgaccaggcgtgcactcatcggataataaacgaccgcattggctgcagtggagattgttacctcttgtgatgctggtgttacacagctaaattgtgttgcactccctgttgccggagttacagtgctccagacttcaacggcgacagcacttgctttatctgcggctgtggaaccatttgcaaaccccgcaccgtcattagcagttccctcgcatgtggctcgcttggttaattttatttgcgcttttttattggggatacccgcacagtctttgaatttgagtttgaatgtttttactttggtcttggcattgatttcagaaatatatacatcaccaaaatcaacaacagaaatgtcctgatcagagtcatttactaatgtagcggtacaagtacccatttctacagtagtaataacggtcagtccaatactgtctgttgccgcataagagagtacgctgaacaatgaggcagccaaaacgacactgctggataatccataacgtaaatttttaaatgtcatcataattatccttcttattgatagatgaaattaaacgtcgccagtgcacgaaaattccccggtacgccttgccctgcatctgtttcacgtagcgcaacggtcatttcaagacccttatcgggctgcatctcgtctgtgctccagcgtatcttttccgcactgttaggtttaaggaaagtggcatcatcagtagtccgttttttgaaacccataccgatattacttgtcgtcgaagatgaatcaccagactgcggtataataagcttaggtgagcttgatgatgcatttccggtcagagtggtatcaatccaactgatgccactgctgcacccactggcaaccagtttaaaatcagcctgagattctgtcgttttattcgcgatcttatccagacccatcttagggattctcaatgtgtagttattattgccatcattcgtgacgttattaccagtaagtgtgatgttacaggttgtcgctttgacagtggctgtaaactctacattaatatccgttgcaaatactgagggtgataataatattcccatcagtatcactattttatgtggcgttgtttttatcatttgacgtcccttgtagttactgaatctgacaccgaattccattcagaataatagattgtgctattttttctgcttctgggctttgttgataatgcgcaagacaacttacgggtttactttgttcgagccatttaatgctgatatttccctgctgctcaataccacgaacaaatgcttgtccaccctgtccaacattaccaatgacattgccttgctcatcataaatatctgcagcaaatggaatatttttaccatcacttcgtgtgatgttcataatggctgattgcccttgcacggtttcaaaatcagcaaagacgactgaaccctgacgcggtacagctactgcactggtactttttaattcaacatcgttctcaagatcgttgatatccagcgcgatacggttttcatgataaggagaaagagcgctggtgacaccataaccccatcgatcgatagtactgttgccataatttattcgcgctccttgagcacctggagcctgaactaccgccagtgtatcggagtcgctaaaactatcattactgaaagtcagtccaccgctatgcaatacaaaaccaccgtcggtgctgagagaaacttgacggctgttatcgctatttgcagaaattgaacctgccagcgttccccatggtgactcatagctggcataacccccaacataactcaaatctttgctggctttattcatcgtatagccagtattcacgctataactgacgcgagcgttatcgctatagccactgctgctaacgttgagttggttattacccttaaagtcactgcttatttgagtatcaatactctggaaacctgaagtacgttgttcagtgccaagtaatttttcaattggaatggtgaaactaagataaacgctatcgtcagtgtcgccgtcttcattccatgaacgctgggcactgacactgtagctgccccaggatgtactgttactgtagccaatagagtaattgctacgattttgtccggaagcccagtaatcggaccaacttccggaaagataaaatgaaccgtaatcttttttctcaaatttcaacggttggttaatactgaccgtaacctgatttttcatgcgtgagtaattacgcatggatttcggttcaagatcttgttcgggatgtttcacttcatcaattagagttagtgcatcattaagaccaaggtaattctgtgtcgaatagcgataggccgcgatattcagtgaagtacttgtttcttcgaataacttgttccaggaaacacgataactttgcccctggtatgttttatcatccgggatacgaacattggaatgagtcacatcgaaagaaaatgcaccaactgaagtattcagaccaagacctaacaaaccagcggtatagttattatcggttatctgaataccggtataacccgtcagatagttattcaggccgtagtagtagcttgcttgaaataaattaggctcatcctgaatatcatcttttaagacctgaccgccgctaatatcccaacgtccaacgccagggcgtaacatttgaacaacggatgagaaaggttgcgagaatgtccgctttgagccatcggattcttcgatggtaacaataagatcgctgccgtaccctgacggactcagatcatcaatgacgaaagcgcctggcggcaccgtcgtttcataaatcttatagccaccttgcgtaatagtgactttggcgttggtattggcaacgccatgaatgataggcgcaaagctggctaaagtcggaggcaacatgcggctgtcactgtataaacgaatgcctcggatactgacggaatcaaaggtttcgcccgtcgtataagactcaccaagaatgagttgagaacgcagcgaggcgatatcacgctgaacataccgattcttaaaatcataattactgccagaatcggtcatccagttgtagttgcccgaggcacgcagtcgccatgcacctaaattcatcccaccgttaaatgcagcataaatgctttcattttttcgaccaggggtttcactatgatatccgttgaggttgtatgacaacatggccgcattaatgccgttttcccataacgatggatcaacatagttttggtaatttttcattacccaggcttgaggaacgtctatatccagacgttgatcgttaacgtcataacgaacagaagcctgagggataatttccgtcaaattgaggcaattgccgagcgtttcatccctggcaagcagaacggctttttcgttatttatatcgggagaattaatatgaaactgcaataaattctttaatgtgatacaagcctgggcgttcttttttccttcaattgcgacaaatgtaatactttggttaatgattggttggtcgtttacataaacactgacgtcgtaaacacccggtatagcggggttaccttcactgtaccggctgagatcaatattagatgcattctgccccatcaggaaggtatggtcatattcaacgagttcagcactgaaagcagtattgcaatacagcagcgcgcaaaacgtggcgatacgggtcagatgatgataatttttagtatattctatagtcacgctatgcttcctgcggaattatatccttgcctgattacagcctggcattaccttcaattgcgccaccaaagtcattaatggcgtaaaaatgcacttttgcagaattcgctttgccattaaggccattgactttcatgacctcatcactaaatggtgcaatcattttcacatcaatcggatagcgtttaccgctagcttctaaatcaccactgctaaaagagacgtagtaaggggttggattggtcactcgtaatgacgccttaccttctgaacctgaccagaaccacttcagggctaacggggcttcagagggatttcccttcaatccatccgggcgatagaaaagttttatacgtgtgcgaaatgccagttgcagcaggctttgattcgcgaccttttctgcatctggttttggtggaacttccagtacgttaaaccagaacacgctctctctgtctttaggcagtgaggtgctggctgtgtacattaatttgattgtttgcccacgtttggcatcaatacgcgatactggcggcgtagcagtaaaagggactgtaatactgccaggctcagcgttgtcatcgccagtatctaaccaactctggacaagcaacgggttattccctttattttccagacgtacgttgacacttttttgatcgcttttatatattacgcgagtacccgaaatgacaatgtccgcaatagacgatgaactaaaagccatacaggttacgaagcataaagctgttgtatgtttggtgttaaaaaacataaaccatccctgatagagttaattaaaacagggaataatataaaatagaaattattattccctgtatattcattcaatcaatttaactggtgaatacttactgataagtaatggtgtatgcagtgttagtttttacataaccagcagttgctgtttggtctgcgacggcacgaacgtaagacgctttaaaatcataaacagcagattttgtcgttgcatccagggctttagtatacacatcgccagggttgttaatttgaacctgtttgatagtggaaccatcaatattgtgtagagcgatattaacgccgtcagatgggttgttaatagacatgtcgttgttcaaagtccctttgctgttaccaaagaaaacagaaccgaaggtcattttagccgtgctacctggattcggatttgctttgctgcagtcaacggtgatgctgaaaggtttagctttagcgccaacggtgtcattcagtacgccagcatcgatttcaccaacggttgcggtttgcagcaggatcagaccatccttgttaccgccgtcaacgcgggtttcacaggtgttatcaacaaccagaccactgatatttaactgaccgccgtccatatcagcagaagcagtacctgcaaccatcgccagcataagaccagacagggcaaaacctaattttttagacataaaaatcctttaataaaattccattagtcagactacatgtttgaagaatgactattcatgacacaaataggagaaacaaatgttagatattaatgagcaatgatatttgttacccaaatttacaaccattgttcattaggtcgcctattgtgcactttagaagcttttgaacaaattaaatttacttaattcaaaattaagtaaaaataagttcacaagtgcaattggttagggtatggagatgggattgatatttatttataggaagttatattatttccgcaaagagatgtttaaactaaaatcgtaattaaggaaagagatgagatatgattttcagaaaatatttatattcgcaatataaataaattaccatttgtttaatttgtcaaatgctcttgtatgtaagatttgacgcaacatctccccatcaggaaacaccaactccggcgcgatttcaaacagcggccacagcataaatccacgattcttcatatcgtagtgcggaacggtcaggcgttcagtatttatcacttcattaccaaacagcatgatgtcgagatccagcgtgcgtggtccccagcgttcagctttgcggacgcgaccttgctgcaattcaatacgctgtgtgtgattgagtagctcttcaggtgcaagagaggtttccagcgccacggctgcgtttaagtaatcgggttgatcttgcggccccagcggtggggtgcggtaaaacgaagaaacggtaagaatgtggctttcagggatatcgcctaatgctttcagggcagcattgacctgctccagcggagaggccagattgctgcctatggcaatatacgccactgtcatgcggtaccctcacgacgtggtgcgcgtttgcgtggacgacgagtacgacgacgcggtgacggttcttcatccagctcgttgagcatccctttttggtctggtggcgcggaaacctggaactcaccccaccatttcaccagacgctgcagttcagcgttacgctcaacttcagctcgcaaggccaacaggtcataagccgcacggaacttaggatgctccagcagtttccatgcgcgtttaccctgacgacgggacatacgcaactgcaactgccagatatcgcgggttaatgtcgtcagacgtttcgggattgccagtgaacggcaggcttcgtccagcacgtcgttcatcgccagcgcgaaagcgtcgtgataggtcaggccgctttcctgggcgatcttctgtgccgtctccagcagtgggtaccagaacatggcggcaaacaggaacgccgggttcacgcgcatatcgttatggatacgcgtatcggtattcttcagcacctgttcaatgatccgctccatcgggctgtcgccattttccgtgaagtagcgggtaatggtcgggaacagcggctggaacagatgatattcacacaacagcttataggtttcgtaaccgtagcccgcttgtagcagtttaagcgattcttcaaacaggcgtgccggtgggatatcgttcagcagggtagcgaggcgagggatcggttctgcggtttccgggctgatgcgcatacccaatttggcggcaaaacgtaccgcgcgcagcatacgtaccggatcttcacggtagcgcgtttccgggttaccaatcagacggataacgccgtccttcagatccttcatgccgccaacgtaatcacggacggtaaaatccgctacgctgtaatacaggctgttgatagtgaaatcgcggcgctgggcgtcttcttcgatggagccgaaaatgttgtcgcgcagcaacatgccgttttgcccgcgttgggaggtcgtgcggtcgctgacgttaccttcgtggtgtccacggaaggtcgcaacttcgataatctccgggccaaacattacatgagccagacggaaacggcgacccaccaggcggcagttacggaacagtttgcgcacctgctcaggcgtggcgttagtggttacgtcaaaatctttcggctttttgccaagtaacaggtcgcgcacgccgccgccaaccagccaggcttcgtatcccgctttattgagcctgtacattaccttcagggcattttcactgatatctttgcgggaaatagcatgctgctcacgcgggatcaccgtcacctgtggacgggcgactgcctgttcagcctcgctttcctcgcggcttagcaccttgcggcaaaaattagcgactcgggtaaaaatagtacacctcggtagtgtcaaacatcattcaggacaaaaaaatagcggctaatcatagctcagcatgacgcatttgagaatgttgaatttacaattgccgactcgggcacggcggtaagccgccagtttttgacggctgactgaaggatttgctcgacgctgaaatcctgccagtgtgcttctgcctgctgccccagaaattgaagtgccgcgattagtaccgggcgtggatcgcctttcggcaacgcaggcgcatgattctgcttggaaagtttagcgccttgtggattaagcgccagcggcagatgaatgtaatctggcactttccagccaaaaagctggtacagcgagatttgccttactgttggttcaatcagatcagccccacgcactatttctgtaacgccctggaaatgatcatcaaccacaacagccaggttgtaggcgaacaacccatcacggcgatgaatgataaaatcttcccgtgccagtttttcgtcggcgtgaataatgccgcgcagctggtcagtaaattgcgtgaccggatgctgctggcggatacgcactgcggcgttgtctggtccatgatgcaacacccggcaatgaccgtcgtaaataccgccaatgctttgaatacgcgcacgcgtacaggtgcagtaataacttagtccttgttcatgtaaccaggcgagtgcttcacgataggcgtcgtgacgttgcgattgccagagaacatcgccgtcccagtgcagaccgtaatgttccagctggcgcaggatagtttctgcggcaccgggaacttcacgaggcgggtcgatatcttctatgcgtaccagccagcgaccttgccgggcgcgagcctgcaaatagctgccgagcgcggcgatcagagagccaaaatgaagctcgccggaaggagagggggcgaagcggccaatatactgtgtgtctgtcatctctttgaacaaaaaataaggcgggagcatttcccgcctgtggtaaacgtgatggaacggctgtaattagccagccatctgtttttcgcgaatttcagccagcgttttgcagtcgatgcacagatcggctgtcgggcgcgcttccagacggcgaataccaatttcaacaccgcaggattcgcagtagccgaaatcttcgtcttccacttttttcagcgtcttctcgatctttttgatcagcttacgctcgcgatcgcggttacgcagttcgaggctgaactcttcttcctgggctgcacggtctaccgggtccgggaagttggctgcttcatcctgcatatgtgtaacggtgcgatcgacttcatccctgagttgattacgccatgcttccagaatacgacggaagtgcgccagctgggcttcattcatatactcttcgcccggcttctcctgatatggttccaccccagcgatggcgagaatactcagggacgatgttttacggttttgcccttcttgcatgttgcttctccttaacacgcactatcgatccccatgttcgggggaaaaatgaggccgctataaatagcagatgcttttccggatagcaattatctaaacgtaacacttgacaactgtgtgaggaaaagcgtatttgcgcacgcgaccagaatgtaaattaaccagttacttactttactacaatgtaaccggcagtgattttttaagagccatgccttcagcagaaatttccgctttgtaagccagaatttctacccccctctgttgagcttctgacaatagttgcgcgtatttctcatcgatgtggcgcgcgggtgaaaaccgtgtaatggctgaatgcagcacggcgaaaaagataaccgcacgctggccttcagccgctacgctcatcaactcccgaaggtgtttctgacctcgttcagtgaccgcatcgggaaaatatccctgttcgttctccgctaacgtaaccgatttcacttcaatatagcagtctggacgcgaatccgcctgcaacataaagtcaatacggctgcgttctgcgccgtattttacttcgcttttcagcgagctatagcctgacagttctgaaattgattcattaaggatagcctctttcgtcaacctgttagcccaaagcgtgttgacgcaaataaatgcgccgctctggctttgagttaattcccaggtgtgtgggtatttccgtttggtgttgtctgaagtcgaataccagacggtatcgccaggcgttgcacaaccggtcatcgcacccgtattcgggcagtgtagcgttaattcgcgaccatcgggtgtgatcacatcggctaaaaaacgtttgtaacgctgaattagcgtcgcgcgctgtagagggggagaaaattccattgcgacaatccttgttattgcgttagcgcccagcgttttagcggcgtgtagcgtgtgcgtccacgggcaaacgaggaggcgtaaagggtgaactccgtcaccgcatacgaccagttaaaacctggcggcgggattgtcaccgcctcgctggcgtcgcgcaataaggtaatatgtggatgaaacggacgattgctttgaaaacaaccgctgcgggcagcctgtgaacggagcatattcgccagctggattaagccgcgtggcggctgacgcatccctaaccacaccacacgcgaacgcagccattgtccggcgtcatcaagcgtgagtgtgaaaccaggttgacgaatccgtccggctaaaagagaaagcgccttctctttctcggcgctcacttcgcctaaaaatgccagagtcagatgcaaattatcggcggcgaccggacgtcccgcctcaggtgggaagtgtgtggcgcgccaatggataatctgttcgcggatttctgcaggtaagtcgatagcaaagaacagacgttgcggttcagacatgtgaggcactcggttatgaattaccgcgatgctacaatgtggcgcgaagaatgttaaccctctggagcgttttgtgtcgtcgttgcccgttgctgccgtcttacctgaattacttaccgctctcgattgtgcgccgcaggtattattaagtgcgccgaccggggccgggaaatcaacctggctgccgctgcaactgctggcgcatcccggcattaacgggaaaattatcctgctggagccgcgtcgtctggcggcgcgtaacgtcgcgcaacggctggcggagctgcttaacgaaaagccaggcgataccgttggctaccggatgcgtgcgcaaaactgcgtcgggccgaatacccgcctggaagtggttaccgaaggcgtgctgacgcgcatgatccagcgtgacccggaactgagcggtgttggactggtgatccttgatgaatttcatgagcgcagcttgcaggcggatttggcgttggcgctgttactcgatgtgcaacaaggtctgcgtgatgaccttaaactgctgattatgtcggctaccctggacaacgaccgcttgcagcaaatgctgccagaagcgcctgtcgtcatctcagaagggcgctcgtttccggttgaacgccgttatttaccgctgcccgcgcatcagcgttttgacgatgccgttgcggtagccaccgctgaaatgctgcgtcaggaaagcggatcattactgttatttttacctggcgtcggagaaattcagcgtgtgcaggaacaactggcttcgcgcatcggcagtgatgtattgctctgcccgctgtatggcgcgttgtcgctgaacgatcagcgaaaagcgatcctcccggcaccgcaagggatgcgcaaagtggtgctggcgaccaatattgctgaaaccagtttaaccattgaaggtattcgtctggtggtggattgtgcccaggagcgtgtggcgcgttttgatccgcgcacggggcttacgcgactgattactcaacgcgttagccaggcatccatgacgcagcgtgccgggcgcgccgggcgtctggagccgggtatcagcctgcatttaatcgccaaagaacaagcagaacgcgccgcggcgcaaagtgaaccggagatcttacaaagcgatctttccggtttgctgatggaattactgcaatggggatgcagcgatccggcgcagatgagctggctggatcaaccgccagtagtgaatctactggccgcgaaacgtctgttacaaatgctgggggcactggagggtgaacggcttagtgcgcaagggcaaaaaatggcagcgctgggtaacgatccgcgtttagcggcaatgctggttagcgcgaagaacgacgacgaagctgctaccgcggcaaaaattgccgccattctcgaagagccgccacggatgggcaatagtgacctgggcgtggcgttttcgcgcaatcaaccagcctggcagcaacgtagtcagcaactgttaaaacgcttaaacgtacgtggcggtgaggcagacagttcgcttatcgcgccgctacttgccggggcgtttgccgatcgcattgctcgtcgccgtgggcaagatggacgctatcaactggcaaacggcatgggagcgatgctcgatgccaacgacgcgctaagccgccacgaatggttgatcgcaccgttattattgcagggcagcgcctcgccggatgcgcggattttactggcgctgctggtcgatattgatgagttagtacaacgctgcccgcagctggtacagcagtctgacactgtggagtgggatgacgcgcaaggtacgctgaaagcctggcgtcggctacaaatcggtcagttgacggtgaaagtgcagccgctggcgaaaccgtcagaagacgagttgcatcaggcgatgcttaatggcatccgtgataaaggtttaagcgtgctcaactggacggcggaagcggaacagctacgcttgcgtttgttatgcgccgcaaagtggttgccggaatatgactggccagcggttgatgatgaaagtttattggcagcgctggaaacgtggctgctgccacatatgactggcgtacattcactacgcggcctgaaatcactcgacatttatcaggcactacgcggattacttgattggggaatgcagcaacgtctggatagtgaattgcctgcgcattacactgtgccgacgggaagccggatcgccattcgttatcatgaagataacccgcccgcgctggcggtgagaatgcaagagatgtttggcgaggccaccaatccgacgatcgcccaggggcgcgtgccgctggtgctggagttgctttcacctgcccaaaggccattacaaatcacacgagatttgagcgacttctggaaaggagcgtaccgtgaggtgcaaaaagagatgaaagggcgttatcccaaacatgtctggccggacgacccggcaaatactgcaccgacgcgacggacgaaaaagtattcgtaaggttggttttctccctctccctgtgggagagggccggggtgagggcatcagcgcgcacgttcaccctcaccctaaccctctccctcaagggagaggggaccgatcgagcacaaattttgagagatatcttcttctgtcttgtaacagaagaacagaaaatcgggcttttgcgcctgaatattgcggagaaaaagcatggccgggaatgaccgcgagccaattggacgcaaagggaaaccgacgcgtccggtcaaacaaaaggtaagccgtcgtcgttacgaagatgacgatgattacgacgattatgatgactatgaggatgaagaaccgatgccgcgcaaaggtaagggcaaaggcaaagggcgtaagcctcgtggcaaacgcggctggctatggctactgctaaaactggctatcgtttttgccgtgctgatcgccatttacggcgtttatctcgatcaaaaaattcgtagccgtattgatggcaaggtctggcaactgcctgcggcagtttatggccgaatggtcaatcttgagccagacatgaccatcagcaagaacgagatggtgaagctgctggaggcgacccagtatcgtcaggtgtcgaaaatgacccgtcctggcgaatttaccgtgcaggccaacagcattgagatgattcgccgtccgtttgatttcccggacagtaaagaaggacaggtgcgcgcgcgtctgacctttgatggcgatcatctggcgacgatcgtcaatatggagaacaaccgtcagttcggtttcttccgtcttgatccgcgtctgatcaccatgatctcttcgccaaacggtgagcagcgtctgtttgtgccgcgcagtggtttcccggatttgctggtggatactttgctggcgacagaagaccgtcatttttacgagcatgatggaatcagtctctactcaatcggacgtgcggtgctggcaaacctgaccgccggacgcacggtacagggtgcgagtacgctgacgcaacagctggtgaaaaacctgttcctctccagcgagcgttcttactggcgtaaagcgaacgaagcttacatggcgctgatcatggacgcgcgttacagcaaagaccgtattcttgagctgtatatgaacgaggtgtatctcggtcagagcggcgacaacgaaatccgcggcttcccgctggcaagcttgtattactttggtcgcccggtagaagagctaagcctcgaccagcaggcgctgttagtcggtatggtgaaaggggcgtccatctacaacccgtggcgtaacccaaaactggcgctggagcgacgtaatctggtgctgcgtctgctgcaacagcaacagattattgatcaagaactctatgacatgttgagtgcccgtccgctgggggttcagccgcgcggtggggtgatctctcctcagccagcctttatgcaactggtgcgtcaggagctgcaggcaaaactgggcgataaggtaaaagatctctccggcgtgaagatcttcactacctttgactcggtggcccaggacgcggcagaaaaagccgccgtggaaggcattccggcactgaagaaacagcgtaagttgagcgatcttgaaactgcgattgtggtcgtcgaccgctttagtggtgaagttcgtgcgatggtcggaggttctgagccgcagtttgcgggctacaaccgtgcgatgcaggcgcgtcgttcgattggttcccttgcaaaaccagcgacttatctgacggccttaagccagccgaaaatctatcgtctgaatacgtggattgcggatgcgccaattgcgctgcgtcagccgaatggccaggtctggtcaccgcagaatgatgaccgtcgttatagcgaaagcggcagagtgatgctggtggatgcgttgacccgttcgatgaacgtgccgacggtaaatctggggatggcgctggggctgcctgcggttacggagacctggattaaactgggcgtaccgaaagatcagttgcatccggttccggcaatgctgctgggggcgttgaacttaacgccaatcgaagtggcgcaggcattccagaccatcgccagcggtggtaaccgtgcaccgctttctgcgctgcgttcggtaatcgcggaagatggcaaagtgctgtatcagagcttcccgcaggcggaacgcgctgttccggcgcaggcggcgtatctgacactatggaccatgcagcaggtggtacaacgcggtacgggtcgtcagcttggggcgaaatacccgaacctgcatctggcagggaaaacagggactaccaacaataacgtagatacctggtttgcgggcattgacggcagcacggtgaccatcacctgggtcggccgtgataacaaccagccgaccaaactgtatggtgccagcggggcaatgtcgatttatcagcgttatctggctaaccagacgccaacgccgctgaatcttgttccgccagaagatattgcagatatgggcgtggactacgacggcaactttgtttgcagcggtggcatgcgtatcttgccggtctggaccagcgatccgcaatcgctgtgccagcagagcgagatgcagcagcagccgtcaggcaatccgtttgatcagtcttctcagccgcagcaacagccgcaacagcaacctgctcagcaagagcagaaagacagcgacggtgtagccggttggatcaaggatatgtttggtagtaattaacatctaagcgtgaaataccggatggcgagttgccatccggtaaaataacatcccatctaagatattaaccctttcttttcatctggttgtttattaacccttcaggaacgctcagattgcgtaccgcttgcgaacccgccagcgtttcgaatattatcttatctttataataatcattctcgtttacgttatcattcactttacatcagagatataccaatggcgcgttccaaaactgctcagccaaaacactcactgcgtaaaatcgcagttgtagtagccacagcggttagcggcatgtctgtttatgcacaggcagcggttgaaccgaaagaagacactatcaccgttaccgctgcacctgcgccgcaagaaagcgcatgggggcctgctgcaactattgcggcgcgacagtctgctaccggcactaaaaccgatacgccgattcaaaaagtgccacagtctatttctgttgtgaccgccgaagagatggcgctgcatcagccgaagtcggtaaaagaagcgcttagctacacgccgggtgtctctgttggtacgcgtggcgcatccaacacctatgaccacctgatcattcgcggctttgcggcagaaggccaaagccagaataactatctgaatggcctgaagttgcagggcaacttctataacgatgcggtcattgacccgtatatgctggaacgcgctgaaattatgcgtggcccggtttccgtgctttacggtaaaagcagtcctggcggcctgttgaatatggtcagcaagcgtccgaccaccgaaccgctgaaagaagttcagtttaaagccggtactgacagcctgttccagactggttttgactttagcgattcgttggatgatgacggtgtttactcttatcgcctgaccggtcttgcgcgttctgccaatgcccagcagaaagggtcagaagagcagcgttatgctattgcaccggcgttcacctggcgtccggatgataaaaccaattttaccttcctttcttacttccagaacgagccggaaaccggttattacggctggttgccgaaagagggaaccgttgagccgctgccgaacggtaagcgtctgccgacagactttaatgaaggggcgaagaacaacacctattctcgtaatgagaagatggtcggctacagcttcgatcacgaatttaacgacacctttactgtgcgtcagaacctgcgctttgctgaaaacaaaacctcgcaaaacagcgtttatggttacggcgtctgctccgatccggcgaatgcttacagcaaacagtgtgcggcattagcgccagcggataaaggccattatctggcacgtaaatacgtcgttgatgatgagaagctgcaaaacttctccgttgatacccagttgcagagcaagtttgccactggcgatatcgaccacaccctgctgaccggtgtcgactttatgcgtatgcgtaatgacatcaacgcctggtttggttacgacgactctgtgccactgctcaatctgtacaatccggtgaataccgatttcgacttcaatgccaaagatccggcaaactccggcccttaccgcattctgaataaacagaaacaaacgggcgtttatgttcaggatcaggcgcagtgggataaagtgctggtcaccctaggcggtcgttatgactgggcagatcaagaatctcttaaccgcgttgccgggacgaccgataaacgtgatgacaaacagtttacctggcgtggtggtgttaactacctgtttgataatggtgtaacaccttacttcagctatagcgaatcgtttgaaccttcttcgcaagttgggaaggatggtaatattttcgcaccgtctaaaggtaagcagtatgaagtcggcgtgaaatatgtaccggaagatcgtccgattgtagttactggtgccgtgtataatctcactaaaaccaacaacctgatggcggaccctgagggttccttcttctcggttgaaggtggcgagatccgcgcacgtggcgtagaaatcgaagcgaaagcggcgctgtcggcgagtgttaacgtagtcggttcttatacttacaccgatgcggaatacaccaccgatactacctataaaggcaatacgcctgcacaggtgccaaaacacatggcttcgttgtgggctgactacaccttctttgacggtccgctttcaggtctgacgctgggcaccggtggtcgttatactggctccagttatggtgatccggctaactcctttaaagtgggaagttatacggtcgtggatgcgttagtacgttatgatctggcgcgagtcggcatggctggctccaacgtggcgctgcatgttaacaacctgttcgatcgtgaatacgtcgccagctgctttaacacttatggctgcttctggggcgcagaacgtcaggtcgttgcaaccgcaaccttccgtttctaatttctcttttggggcacggatttccgtgcccatttcacaagttggctgttatgcaggaatacacgaatcattccgataccacttttgcactgcgtaatatctcctttcgtgtgcccgggcgcacgcttttgcatccgctgtcgttaacctttcctgccgggaaagtgaccggtctgattggtcacaacggttctggtaaatccactctgctcaaaatgcttggccgtcatcagccgccgtcggaaggggagattcttcttgatgcccaaccgctggaaagctggagcagcaaagcgtttgcccgcaaagtggcttatttgccgcagcagcttcctccggcagaagggatgaccgtgcgtgaactggtggcgattggtcgttacccgtggcatggcgcgctggggcgctttggggcggcagatcgcgaaaaagtcgaggaagctatctcgctggttggcttaaaaccgctggcgcatcggctggtcgatagtctctctggcggcgaacgtcagcgggcgtggatcgccatgctggtggcgcaggatagccgttgtctgttgctcgacgaaccgacctcggcgctggatatcgcccaccaggttgatgtgctgtcgctggtgcaccgtttaagtcaggagcgtggcctgacggtcattgccgtgttgcacgatatcaatatggcggcacgctactgtgattatctggtcgccctgcgcggcggtgaaatgattgctcagggaacgcctgcggaaattatgcgcggcgaaaccctcgaaatgatttatggcatcccgatgggtattttgccgcatccggcgggtgctgcacctgtgagttttgtttattgatgagcggcttacctcttatttcgcgccgtcgactgttaacggcgatggcgctttctccgttgttatggcagatgaataccgcccacgcggcggctattgatcccaatcgtattgtggcgctggagtggttgccggtggaattactgctggcgctcggcatcgtgccttacggcgtggcggataccatcaactatcgcctgtgggtcagcgaaccaccattgccggactcagtgatcgacgtcggtttgcgcacagaacctaaccttgaactgctgaccgaaatgaaaccatcgtttatggtctggtcggcaggatatggcccttcaccagaaatgctggctcgtattgcgccgggtcgcggatttaacttcagtgacggcaaacagccgttggcgatggcgcgtaaatcgctgacggaaatggcagatttacttaacctgcaaagcgcagcggaaacgcatttagcgcaatatgaagactttatccgcagcatgaaaccccgctttgtgaagcgtggtgcgcgtccgttattgctgacgacgcttatcgatccgcgccatatgctggtcttcggtccaaacagcttgttccaggaaattcttgatgagtacggcatcccaaatgcctggcaaggggaaaccaacttctggggcagtaccgccgtcagtatcgatcgtctggcggcgtataaagacgttgatgtgctctgttttgatcacgacaacagcaaagacatggatgcgctaatggcaacgccgctgtggcaggccatgccgtttgtccgcgccggacgctttcagcgcgtacctgcagtctggttttatggtgcgacgctctcggcaatgcactttgtgcgcgttctggataacgccatcggaggtaaagcgtgagtaaacgaattgcgcttttcccggcgttattgctggcgctgttagtgattgtcgctacggcgctcacctggatgaacttctcgcaggcgctgccgcgtagccagtgggcgcaggctgcctggtcgccggatattgacgtcatcgagcagatgatttttcactacagcttgttgccgcgtctggcgatttcgctgctggtgggcgcgggtctggggctggtgggcgtgctgtttcagcaagtgctgcgtaacccgctggcggagccgacgacgcttggcgttgctacaggcgcgcaactggggattaccgtcactacgctctgggcgatccctggtgcgatggcgagccagtttgctgcgcaggcaggggcttgtgttgttggcttaattgtctttggcgtcgcgtgggggaaacggctgtcgccggtaacgctgattctcgcggggttggtagtgagcctttattgcggcgcaatcaatcagttactggttatcttccatcatgaccaactgcaaagcatgtttctgtggagcactggaacgctgacgcaaaccgactggggcggcgttgagcgtttatggccgcagctgctgggcggtgtgatgctgacgttgctgctacttcgtccgttaaccctgatggggcttgatgatggcgtggcgcgcaatctcgggctggccttgtcgcttgcgcgtctggcagcgctgtcgctggcgattgtcatcagtgcgctgctggtgaacgctgtggggattatcggctttatcgggttgttcgcgccgctgctggcaaaaatgctgggggcgcggcgtctgctgccacgactgatgctggcgtcgttgattggtgcgctgatcctctggctttccgatcaaatcatcctctggctgactcgcgtgtggatggaagtgtccaccggttcggtcactgcgttgatcggtgcgccgctgctactgtggctgttgccgcgtttacgcagcattagcgcgccggatatgaaggtcaacgatcgtgtcgcggctgaacgccaacatgtgctggcgtttgccctcgcgggcggcgtgctgctgttgatggctgtggtggtggcgctgtcgtttggtcgtgatgcgcacggctggacgtgggcgagcggggcgttgctcgaggatttaatgccctggcgctggccgcgaattatggcggcgctgtttgcgggcgtcatgctggcggtggcgggctgtattattcagcgactgaccggaaacccgatggcaagcccggaagtgctggggattagctccggcgcggcgtttggcgtggtgttgatgctgtttctggtgccgggtaatgcctttggctggctgttacctgcaggcagtctcggcgcggcggtgacgctgttgatcattatgatcgccgccggccgcggtggattttccccacaccgtatgttactggcggggatggcgttaagcaccgcgttcaccatgcttttgatgatgttgcaggcaagtggtgacccgcgaatggcgcaagtgctgacctggatttccggttcgacctacaacgcgaccgatgcgcaggtctggcgcaccggaattgtgatggtgattttgctggcgattaccccgctgtgccgccgctggctgaccattttaccgctgggtggtgataccgcccgagccgtaggaatggcgctgacgccgacgcgaattgcgctgctgctgttagcggcttgcctgacggcgaccgcgacgatgactattggaccgttgagttttgttggtttaatggcaccgcatattgcgcggatgatgggctttcgacggacgatgccacacatcgtaatttcggcgctggtgggtggtttactgctggtgttcgctgactggtgtgggcggatggtgctgtttccattccagatcccggcggggctgctgtcaacctttatcggcgcgccatattttatctatttgttgagaaagcagagccgttaatttttccatataacggccctgtacgcctggacggataaagcgtttacgcgacaacggatgcccgatgcgacgctggcgcgtcttatcgggcctacaaacggccccgaatcgtaggtcggataaggcgttcacgccgcatccgacaaaccatgctggatcacaacttcgcaaacacccgacgtgcagcatcgatggtgttattgatatcttccatgctgtgcgccacggacataaagcccgcttcaaacgctgacggtgccaggtaaacaccttcgtccagcatcatatggaagaaacgcttaaagcgttccacgtcacaggccatcacatcctgatagcacgtcacggactcggcgtcggtaaagaaaataccgaacatgccgccaacgtggttaacgaccagcggaattccggcttcttctgccgcttccagcagaccttctgccagacgtgttgtcagctcatccagcgtttcgtgaacgcccggctgcgcgacttcattcagacaggcgaaacccgctgccatcgcaatcgggttaccggaaagcgtacccgcctgatagaccggacccgtcggggccagcgcatccattacatcacgacgaccaccgaatgcgcctaccggcattccaccgccgatgattttgccgaggcaggttaaatctggcactacgccgtaataatcctgtgcgccagctagcgctacgcggaaaccggtcatcacttcatcgatgatcagcaacgcgccaaattcgtcgcacagcgcgcgcagacctggcaggaactctggcagcggcggaacacagttcatattgcctgccaccggctcgacgataatacaggcaatctcttgcgggtattgctcaaatgcggcgcgtacagaagccagatcattataagtacaggttaaggtatatttggcgaaatctgccggaacgcccggcgagtttggctggcctaacgtgagtgcgccagaaccggctttcaccagcaggcagtcagcgtgaccatggtaacacccttcaaatttaataattttgtcgcgaccggtaaaaccacgggccaggcggatggcgctcatggtcgcttcagtgccggagttcaccatgcgcaccatatccatggtcgggaccagttcggtcaccagttgcgccattttcacttccatttcggttggtgcaccaaagcttaaaccacgctcggcggcttcaatcacggcattgcggattgccggatggttatggcccagcaccatcggcccccaggaaccgacataatcgatataggctttgccatcaacatcgtacagataagcgccgtccgctttttcgataaacagtggagtgccgcccacgccagtaaaggcgcgaacaggggagttcacaccgccagggatcagctcgcgcgctgcgctgtaaagattttcagacttactcatggagggttcctgattcgtagaaaaagtgaatggctgctattctatgttattcataacaagttaaatactcgtcaaacatcaggctgcttgtactggtgcaatcctgatttcttagagtataaaagttttgtgcatttgaaacattacgctttgcaaaggattttcatggaacgtgcgagtaaaatgccgtcatcttatttgtatgaccaataagtgatcattggatgaaaactgatactccctctttagaaacaccgcaggccgcgcgcctgcgacgcagacaactgattcgccaacttcttgagcgcgataaaaccccgttagccattttgtttatggcggcagtcgtcggcacgcttgttgggctggcagcggttgcttttgacaaaggtgtcgcctggttgcagaaccaacgtatgggggcgctggtacatactgctgataattatccgcttctgttaaccgtcgcttttctctgttcggcggtgctggcgatgtttggctactttttggtgcgcaaatacgcgccggaagcaggtggttcggggatcccggaaattgaaggggcgctggaagatcaacgtcccgttcgctggtggcgtgtattgccggtgaagttctttggcgggctggggacactcggcggaggcatggtgttggggcgcgaagggccaaccgtgcagatcggcggtaacattggccgtatggtgcttgatattttccgcctgaaaggtgacgaagctcgccatacgctgctggcaaccggtgctgctgcggggctggctgcggcctttaacgcgccgctggcgggtattttgtttattatcgaagagatgcgtccgcagtttcgctatacgttaatttcgattaaagcggtatttattggtgtcattatgtcgaccattatgtaccggatttttaatcatgaagttgcgttgattgacgtcggtaaactttctgatgcgccgcttaatacgctgtggctttatctgatcctcggtattatttttggcattttcggccctatttttaataaatgggtgctggggatgcaggatttgctgcaccgtgtgcacggcggcaatattaccaaatgggtgctaatgggcggtgcgattggcggtctgtgtggattgctggggtttgtggcaccagcaacgtcgggcggcggttttaacctgattcctatcgctaccgcggggaatttcagcatgggaatgctggtgtttatcttcgtcgcgcgggtcattaccaccttactctgcttctcttccggcgcgccgggcggtatttttgccccgatgctggcgctgggtactgtgctgggaaccgctttcggaatggttgccgttgagctgtttccgcaatatcaccttgaggcggggacgtttgctattgccggaatgggggcattactggcggcatctattcgcgcgccgttaacggggatcattctggttctggagatgaccgataactaccagctcattttgccaatgattattaccggtcttggcgcaacactattagcgcaatttaccggcgggaaaccgctatactcggcgattcttgcgcgcacgctggcaaaacaggaagctgagcaactggcgcgaagcaaggccgcatcagccagcgagaatacttgaacgaaataccagggtattagataatggcgattattattgggttagaatttgcccaattgccgatgtcgtttggagcaaaatatgagtgatgacgtagcactgccgctggagtttaccgacgcagcagccaacaaagttaaaagcctgatcgctgacgaagataacccgaatctgaaattacgcgtgtatatcaccggtggcggttgcagcggcttccagtatggtttcacctttgatgatcaggtgaacgaaggcgatatgaccatcgaaaaacagggcgttggcctggtggttgatccgatgagcctgcaatatctggtcggcggttccgttgattataccgaaggtctggaaggttctcgtttcatcgtgaccaacccgaacgcgaaaagcacctgcggttgcggttcttcctttagtatctaatctgttgttcatgtgccggataaactatccggcacatcttctctcttcaacgcccattctcatccagcgcaaacgtcggtagcttaagatgccaacgaatagccgccagccgaatcaatagcgtcacgaccatgcccatcatactggctgtttccagtggtacggaaaatgtgtaataagccgtagcgtggacaataccgccgataatacaggcagttgcgtagatttctgtacgtaaaatcatggggatttcgcgggccagaacatcacgaatgatcccgccgccaacgccagtaatgacgcccatacaaaccgcgattaacggaccggcttccgcattaaaggctttattcacgccaatgccgacaaacaccgccagaccaacggcgtccagcaccggcaacatccattttggtaagcgtcttggctggcgcaccagcacgatggtcagcatgctggtgaccattgcaacgaccagatcggtgggatctttcacccaaaataccgggccgtgatccagcgccatgtcgcgaattgtcccgccgcctactgcggttaccacgcccagtaccagaacaccaaaagggtccatacgcaattttccggctaacaaaacgccggagatggcaaataccgctgtgccgactatatccagccaatagacgagcattgttcaatccccactgagcacctgaaaaggtcaggcgctaatctacctgtgaaagcgcattacagagctgttgtgcagcgaggataatacgtgggcttgcacgttcaaaccagtcactcgtgagaggaataacgggaattttgagctgttcaccccagtattgtttgattttaggaatttggtccggtccgcctgtaatgacaatcgcctgtggcgagcgtgctaacacctgttcgcggctaacttgcggccagggaacccggctgtctttaaagatgttttctccgccacaaacttcgagtacctggttctgaatcgactcttttccactggtaaatggcggattaatgccgaattgcagaaaaacacgttttttaggtttatcagcatattgcgctttcaattgcgcgtactgatccagcagggattgcgcggcttgttcggccttgtctggttgcggactccagggggccagttgacgtaacgcattggcaatttgttcaatgcttgtcgcatcgacccacatcacttttattcccagcgaagccagctggtcaacctgccgctcggcattacctccacgccaggcaatcaccagatcgggtttcagcgcgacaatgcgttccagattcatcccctgccaggtggaaacctgctcaatcttttgcgcttgtggaggatagtcggaatagctgctgaccccaaccggcgtgatcccggcggcaaaggcaagttcagtgttggcgggagaaagcgtgatgacgcgcggcgcggcgttgagccacagtggcgcaagaaaagacagggcgaccagcgccctgaacagtgacttagccatgtgcaagtttctgcaccagtgactcaaccatcaggctggactgtttagcggcaacagccaggaactcatcgaagctaagatgagactgttgatcggccacgtcggagatggcgcgtacgacaacaaacgggacgttgaaattgtggcagacatgggcgattgccgtcgcttccatctctacagcaatggcctgtgggaagttgtggcggattttcgccagaccaacagaaccgttgatgaaagcgtcgccgctaacaatcaggccacgtacagcgttaagattcagttcggcaatgcaggcctcagcggcagcgatcagtttatcgtcagctttaaagcctgccggacagcctggtaactgaccgtattcataaccaaatgccgtgacatccgcgtcgtgataacgtgcttcgtccgagacaacgatatcgcccactttcaacgttggtgccaggccaccggcagaaccggtgttaataatcacatctggcttgcagtgttccaacagcaaagtggcacccagcgccgcagcgactttaccgatgcccgatttcagaagcgcaacctcggttccattcagttggccggtatagatttcgcaaccgccgagactgatagtttgacggttttcgattttgtcacgcagcagcgtaacttcttcttccattgcaccaatgatgccgattttcatagatttactcgcgataagcccgatttgaaggcatagtttaccatgcgcttacggggaagcgtatttctcacgcgggagaggacatggcacagattgatttccgaaaaaaaataaactggcatcgtcgttaccgttcaccgcagggcgttaaaaccgaacatgagatcctgcggatcttcgagagcgatcgcgggcgtatcatcaactctccggcaattcgtcgtctgcaacaaaagacccaggtttttccactggagcgcaatgccgccgtgcgcacgcgtcttacccactcgatggaagtccagcaggtggggcgctacatcgccaaagaaattttaagccgtctgaaagagcttaaattactggaagcatacggcctggatgaactgaccggtccctttgaaagcattgttgagatgtcatgcctgatgcacgatatcggcaatccgccgtttggtcattttggcgaagcggcgataaatgactggtttcgccaacgtttgcacccggaagatgccgaaagccagcctctgactgacgatcgctgcagcgtggcggcactacgtttacgggacggggaagaaccgcttaacgagctgcggcgcaagattcgtcaggacttatgtcattttgaggggaatgcacaaggcattcgcctggtgcatacattgatgcggatgaatctcacctgggcacaggttggcggtattttaaaatatacccgtccggcgtggtggcgtggcgaaacgcctgagacacatcactatttaatgaaaaagccgggttattatctttctgaagaagcctatattgcccggttgcgtaaagaacttaatttggcgctttacagtcgttttccattaacgtggattatggaagctgccgacgacatctcctattgtgtggcagaccttgaagatgcggtagagaaaagaatatttaccgttgagcagctttatcatcatttgcacgaagcgtggggccagcatgagaaaggttcgctcttttcgctggtggttgaaaatgcctgggaaaaatcacgctcaaatagtttaagccgcagtacggaagatcagttttttatgtatttacgggtaaacaccctaaataaactggtaccctacgcggcacaacgatttattgataatctgcctgcgattttcgccggaacgtttaatcatgcattattggaagatgccagcgaatgcagcgatcttcttaagctatataaaaatgtcgctgtaaaacatgtgtttagccatccagatgtcgagcggcttgaattgcagggctatcgggtcattagcggattattagagatttatcgtcctttattaagcctgtcgttatcagactttactgaactggtagaaaaagaacgggtgaaacgtttccctattgaatcgcgcttattccacaaactctcgacgcgccatcggctggcctatgtcgaggctgtcagtaaattaccgtcagattctcctgagtttccgctatgggaatattattaccgttgccgcctgctgcaggattatatcagcggtatgaccgacctctatgcgtgggatgaataccgacgtctgatggccgtagaacaataaccaggcttttgtaaagacgaacaataaatttttaccttttgcagaaactttagttcggaacttcaggctataaaacgaatctgaagaacacagcaattttgcgttatctgttaatcgagactgaaatacatgaaaaaaaccacattagcactgagtgcactggctctgagtttaggtttggcgttatctccgctctctgcaacggcggctgagacttcttcagcaacgacagcccagcagatgccaagccttgcaccgatgctcgaaaaggtgatgccttcagtggtcagcattaacgtagaaggtagcacaaccgttaatacgccgcgtatgccgcgtaatttccagcagttcttcggtgatgattctccgttctgccaggaaggttctccgttccagagctctccgttctgccagggtggccagggcggtaatggtggcggccagcaacagaaattcatggcgctgggttccggcgtcatcattgatgccgataaaggctatgtcgtcaccaacaaccacgttgttgataacgcgacggtcattaaagttcaactgagcgatggccgtaagttcgacgcgaagatggttggcaaagatccgcgctctgatatcgcgctgatccaaatccagaacccgaaaaacctgaccgcaattaagatggcggattctgatgcactgcgcgtgggtgattacaccgtagcgattggtaacccgtttggtctgggcgagacggtaacttccgggattgtctctgcgctggggcgtagcggcctgaatgccgaaaactacgaaaacttcatccagaccgatgcagcgatcaaccgtggtaactccggtggtgcgctggttaacctgaacggcgaactgatcggtatcaacaccgcgatcctcgcaccggacggcggcaacatcggtatcggttttgctatcccgagtaacatggtgaaaaacctgacctcgcagatggtggaatacggccaggtgaaacgcggtgagctgggtattatggggactgagctgaactccgaactggcgaaagcgatgaaagttgacgcccagcgcggtgctttcgtaagccaggttctgcctaattcctccgctgcaaaagcgggcattaaagcgggtgatgtgatcacctcactgaacggtaagccgatcagcagctttgccgcactgcgtgctcaggtgggtactatgccggtaggcagcaaactgaccctgggcttactgcgcgacggtaagcaggttaacgtgaacctggaactgcagcagagcagccagaatcaggttgattccagctccatcttcaacggcattgaaggcgctgagatgagcaacaaaggcaaagatcagggcgtggtagtgaacaacgtgaaaacgggcactccggctgcgcagatcggcctgaagaaaggtgatgtgattattggcgcgaaccagcaggcagtgaaaaacatcgctgaactgcgtaaagttctcgacagcaaaccgtctgtgctggcactcaacattcagcgcggcgacagcaccatctacctgttaatgcagtaatctccctcaaccccttcctgaaaacgggaaggggttctccttacaatctgtgaacttcaccacaactccatacatcttcatcatcctttaggcatttgcacaatgccgtacgttacgtacttccttatgctaagccgtgcataacggaggacttatggctggctggcatcttgataccaaaatggcgcaggatatcgtggcacgtaccatgcgcatcatcgataccaatatcaacgtaatggatgcccgtgggcgaattatcggcagcggcgatcgtgagcgtattggtgaattgcacgaaggtgcattgctggtactttcacagggacgagtcgtcgatatcgatgacgcggtagcacgtcatctgcacggtgtgcggcaggggattaatctaccgttacggctggaaggtgaaattgtcggcgtaattggcctgacaggtgaaccagagaatctgcgtaaatatggcgaactggtctgcatgacggctgaaatgatgctggaacagtcgcggttgatgcacttgttggcgcaggatagccgtttgcgggaagaactggtgatgaacctgattcaggcagaggagaatactcccgcacttactgaatgggcgcaacggctggggatcgatctcaatcaaccgcgagtggtggctattgttgaggtcgacagcggtcagcttggcgtggacagcgcaatggcggagttacaacaactgcaaaacgcgctgactacgcccgagcgtaataatctggtggcgattgtctcgctaaccgaaatggtggtgttgaaaccggcgttgaactcttttgggcgctgggatgcagaagatcatcgtaagcgagttgaacaactgattacccgcatgaaagagtacggccagctgcgttttcgcgtttcactgggcaactattttaccggtcctggcagtattgcccgatcctatcgtacggcgaaaacgacgatggtggtgggtaaacagcggatgccagaaagtcgctgctatttttatcaggatctgatgttacctgtgttactcgacagtttgcgtggcgactggcaggccaacgaactggcgcgaccgctggcgcggctgaaaacgatggacaataacggcttgctgcgacgaacgctggcggcgtggtttcgccacaatgtgcaaccgctggcaacgtcaaaggcgttgtttattcatcgtaataccctggagtatcggcttaatcgtatatcggaactgaccgggcttgatttgggcaattttgatgacaggttgctgctgtatgtggcgttacaactggatgaagagcggtaggttatgcgttaaggttgaggcggcgctggctcattcccctcagcccgaagggtagaggggaatgcccgaattaaccgtcagttcgggattatttacgcgttagtttttccagatcggcttcaatctcgctgatcttattggttacgactgactccaggtgacgtaagtcgtcgaggatcttacgcttaagatcaacttcgctgcggtcacgctggcagatttgatcaagctcatcaatgatataccgtagattcgggctgatttcctggacttctttataaccctgacccacaccatcagcgacgaccgttttacgctgacgcggatatttaaacttaacgctcttggcgaaaaactcgcctttgtctttctggaaatagattttcagaatatcgttgttggcttcctgccggaggctgtaacgatcaatttcttcaggattggtaatacccagacttttcagattgtcgtacatagcgttacctcaaaatgagtcagtaaattgtgcttattttagcatttggcctggcccgcccggctcgactgtgatcgcagaaagcctttttcttccagacttctatcatggcgtaaaaatcaaaaaattacctgctttattctggtgataaaattcacgatctacaccagttccagcatcgttacttccgggcggcagttcagacgcaaaccatacaaactgcccacgccacgggttgtgtagatgtgtctttcgccaaaggcatttaatccggcgacgtaacgtttatcttcgacaggggcaaaaggttcaccaaccaacggtacgcgcagttgcccgccgtgagtatggccgcacagcatcagatcccagggttcatcacgcatgacttctttgctgtcgggattatgcgccagcaccagtcttggcagattggcttcgctggcgggaggcggtttgcattgtccggcccataagtcaccagtgcctaccagttcgaattgcctgttcggcgtggcgatcaccgtagcctggttaaacaacaccgtgatgcccgctgatttcaacgtctcgccaattaagtgatttttttctgtaccaacagggcgatcgtggttgccgaagcaggcaaacgtcggcgcacattcggcaaggggggagagtacgtcactaaacgccgaaaaattcagcgacatatcaaataatacgtaatcgccgcccagtaatatcaaatcgggcttttgttctatgccaagagcaatcgcgtcagaaatcaggcttaaaggaacaaaacgagagtaatggagatcggccagaaaaagaattttgaatggtgctgcgttgtctttaaaaaaggcgaggcggtgacggattaattcaaaccagcctggctcacagtaatgcatataaccgaaacctgagctcgtggctatcgtcgcggcagtagcctgcaaaaatcggcggcgtgaaatcatcgctcatccctgcaaaaaaatcgggcagcgtcgtgctgcccgtgtgcatacttttagtcgatggtacgcagcagttcgttaatgccgactttgccgcgagttttcgcgtcaactttcttaacgataaccgcacagtagaggctgtatttgccatcttttgacggcagattacctgaaacaaccacagaccccgccggaacgcgaccgtagtggatttcgccggtttcacggtcgtaaatacgggtgctctgaccaatgtatacgcccatggaaatgacggaaccttcttcgacaatcaccccttcaaccacttcagagcgcgcgccgatgaagcaattatcttcaatgatggttgggttagcctgcagcggttccagcacgccgccgatgcccacgccaccggaaaggtggacgtttttaccaatctgcgcacaagaaccgacggtcgcccaggtatcaaccatggtgccttcatcaacatatgcgccgatgttgacgtaagacggcatcagcacggtgttacgggcaataaacgcaccctgacgtaccgccgctggtggcacaacgcggaagccttctttctggaaacgtgcttcgtcgtagtcggcgaatttcatcggcactttgtcgaagtagcggctttctgccccttcgatcacctgattatcattaatacggaaagagagcagcaccgcttttttcaaccactgatgcgtcacccactgaccgtcaattttttccgctacacgcagtgcgccggaatccagcagggcgatcacctgatttaccgcttcgcgggtaacggtgtctgcattggctggcgtgatctcggcacggcgttcaaaagcggtttcaataatgttctgtaactgctgcattgttaaactcttttcatatcagtaaacacatcaccctttatcgtttggattgagggcctctgtcaaccgctgatgcacttcctgctgcaactcgttattaagcgcacgccggtcagcggtggcaattatgaataaatcttctactcgctcgccaatggttgtaattcgggcaccatgaagcgaaattcccagatcggcaaaaattttcccgactcgcgccagcagtccaggttggtcgagggcgatcagttcgaggaacgatttgcggtcggtatgggtcggcaaaaacgttacttcggtttcaacagtaaaatggcgtaatttggcgggttggcgacggggctgcggtggctgccagctactttgcgtcagtacttgctccagaccaaaccgaataacctcatgacgatctgcggacagcgggttgccatcgggttccagcacgataaaggtatccatcgccataccgtcgcgagtggtgaaaatttgtgcgtcgtgaacacttaaattgcggcggtctaattcggcacagacggcggcaaacagataagggcggtccgggctccagataaaaatctcggtgcctccacgcgtagcctgcgggctaagcaataccagcggtttgcttaaatcatgctgtaataaatggcgggcatgccaggccagttgatttgggctatggcggacaaaatagttagcacgacagcgtgaccaaatttggtgcagcgcctcttcgtcgatgttatccatgcgcagtagtgccagtgcctggagttggtgatggcgaacccgttcgcgcatatccggcgtgttttgcattccgcgtcgtagctgcttttcggtggcaaagtagagctcacgcaacagactttgcttccagctattccacagcgtttcgttggtggcgcaaatgtcagccacagtcaggcataccagatagcgcagacgattttccgtttgcacttcttcggcaaactgcttgatgacttccgggtcctgaatatcgcggcgttgggcggtcaccgacatcaacaggtgctggcgaaccagccaggcgaccagctgtgtttcgcgtgagttcagcccgtggagttcggcaaaatgcactacatcctgagcaccgagaatggagtggtcgccgccgcgtcctttggcgatatcgtgaaacagcgcggcgatgaaaatcagctcagttgacggcaggcgcggccagacgtccacacacaacggatggcgctggcgcgtttcttcactggcaaaactctccagtttcagcatcacgcggatagtatgttcatccaccgtgtaggcgtggaacagatcaaactgcatctgcccgacgatatgcgaccattgcggcatatacgcgccgagcacgctatggcgatgcattggcaatagcccgcgccgcaccgctccggggtgacgcagaatgctcaaaaacagttttcgtgcttccggaatattacacagcggttgttgcagatggcgacgggcatggcgtaactggcgcagcgtggtggagtaaatgccggtgatcgcactgttgtgcaccatggtgtagaacatacgcaagatggcttccggctggcgcataaatagtgtttcatcacgcaggtcgattagcgtaccgcgtagctgaaactcatcgtcgattggacgtggtttttcgtcggcgggaagggcgaggatggcttcatcgaacagttgcagcagcatctggttgagttcactgacgcggcgtgtaacgcggaagtaatccttcatcatccgctcgaccggttcgttaccttcaccactgtaattcagacgctgggcgacgctaagctggcgatcgaataacaggcgattatcgtaacggctgacgaccagatgcagggcaaagcgaatacgccacaatatatgcagacattcgtttaattccgcccgctccgctgaggttaagaagccaaacccgaccatttcatccagcgatgttgcgccaaaatgacggcgggccacccattgcagagtgtggatatcgcgcaagccgccagggctgcttttgatgtctggttcaaggttgtagctggtgccatggtaacgctgatggcgctggttctgttcttcaactttcgccgcgtagaacttgtcggaaggccagaatccttcgctgaaaatatgtttttgcagttcgaggaacagcgcaacatcgccaattaataagcgggattcgattaaattggtggcgacggttaaatccgataacccttccagcatgcactcttcaagcgtgcgcacgctatgaccgacttccagctttacatcccagagcagcgttaacagctcgcccactttttgcgcctgatcgtccgggagctttttacggcttaaaatcagtaaatcgacgtctgaaagtggatgcagctcgccacgaccgtagccaccgacggcgaccaatgccaggtcggcaatctggctgaatcccgcttcaatccataatcgttgcaggagctggtcgataaactcggtgcgcgcctcaatcaactgttctgcagagatcccattgtcaaaggcatcacccagccaacgctggaaagtatcgatatgggcttttatcccaccgacggttaattcatcacggggccagacgcatggattttgcggttgaccgggcagggtggggagagcggtgtttgcgtactgttctggaagggtattcattgtgcgccacccataagattaaattatcgcattaaaaaagccggcattcgccggcttcatcttattcgtcgtgcgagattatcgccgggatggtgtcatccttgcgtagcgtcagaatttcgcagccgttatcagtcaccacaatagtatgctcatattgtgcagacaagctgcgatctttggtttttaccgtccagccatctttcatggtgcggatctcttttttacccgcgttgaccattggctcgatggtgaacgtcatcccaggtttcagtacgacgttggtttcacgggagtcatagtgcagcacctgcggttcttcatggaagccgcgaccaataccgtgtccgcaatattcacgaacgacggagaagccttctgcttcgacaaatttctgaatcgccgcaccgatttcgcgcagattaatgcctggttttaccatgcgtagcgccaggtacaggctttcttgcgtgatgcggcacagacgttcgcccatgatggtcggcttaccgacgataaacattttcgaggtatcgccgtggaaaccatctttgattacggtgacatcaatgttaacgatatcgccatctttcagcagcttagcatcgtccgggataccgtggcacaccacttcattaatagagatgcaaacggatttcggatagccgtgatagccgaggcaggcagaaaccgcgtgttgttcattaacaatgtaatcattacagatgcgatccagctcgccggtgctgacgcccggtttaacatacggttcgatcatctccagcacttcggcagccagtcggccagcgacgcgcattttttcgatatcttctggggtcttgattgagatagccattaattctgtccatcagcgtcggtgataccgacaatatatatgtaagtgccgtcaatggtatcacacccgggcaaattgagaatcattctgaatttcgccaaacgtgccactgaaggttttctataatagaaaattcgacgtctgatgctgtacacagcgccaacaattattggtgtccacgacgtatttgtggtataaagcgcgccggacttccgatccatttcgtatacacagactggacggaagcgacaatctcactttgtgtaacaacacacacgtatcggcacatattccggggtgccctttggggtcggtaatatgggatacgtggaggcataaccccaacttttatatagaggttttaatcatggcaactgtttccatgcgcgacatgctcaaggctggtgttcacttcggtcaccagacccgttactggaacccgaaaatgaagccgttcatcttcggtgcgcgtaacaaagttcacatcatcaaccttgagaaaactgtaccgatgttcaacgaagctctggctgaactgaacaagattgcttctcgcaaaggtaaaatccttttcgttggtactaaacgcgctgcaagcgaagcggtgaaagacgctgctctgagctgcgaccagttcttcgtgaaccatcgctggctgggcggtatgctgactaactggaaaaccgttcgtcagtccatcaaacgtctgaaagacctggaaactcagtctcaggacggtactttcgacaagctgaccaagaaagaagcgctgatgcgcactcgtgagctggagaaactggaaaacagcctgggcggtatcaaagacatgggcggtctgccggacgctctgtttgtaatcgatgctgaccacgaacacattgctatcaaagaagcaaacaacctgggtattccggtatttgctatcgttgataccaactctgatccggacggtgttgacttcgttatcccgggtaacgacgacgcaatccgtgctgtgaccctgtacctgggcgctgttgctgcaaccgtacgtgaaggccgttctcaggatctggcttcccaggcggaagaaagcttcgtagaagctgagtaataaggcttgataactcccccaaaatagttcgagttgcagaaaggcggcaagctcgagaattcccgggagcttacatcagtaagtgaccgggatgagcgagcgaagataacgcatctgcggcgcgaaatatgaagggggagagcccttatagaccaggtagtacacgtttggttagggggcctgcatatggccccctttttcacttttatatctgtgcggtttaatgccgggcagatcacatctccgaggattttagaatggctgaaattaccgcatccctggtaaaagagctgcgtgagcgtactggcgcaggcatgatggattgcaaaaaagcactgactgaagctaacggcgacatcgagctggcaatcgaaaacatgcgtaagtccggtgctattaaagcagcgaaaaaagcaggcaacgttgctgctgacggcgtgatcaaaaccaaaatcgacggcaactacggcatcattctggaagttaactgccagactgacttcgttgcaaaagacgctggtttccaggcgttcgcagacaaagttctggacgcagctgttgctggcaaaatcactgacgttgaagttctgaaagcacagttcgaagaagaacgtgttgcgctggtagcgaaaattggtgaaaacatcaacattcgccgcgttgctgcgctggaaggcgacgttctgggttcttatcagcacggtgcgcgtatcggcgttctggttgctgctaaaggcgctgacgaagagctggttaaacacatcgctatgcacgttgctgcaagcaagccagaattcatcaaaccggaagacgtatccgctgaagtggtagaaaaagaataccaggtacagctggatatcgcgatgcagtctggtaagccgaaagaaatcgcagagaaaatggttgaaggccgcatgaagaaattcaccggcgaagtttctctgaccggtcagccgttcgttatggaaccaagcaaaactgttggtcagctgctgaaagagcataacgctgaagtgactggcttcatccgcttcgaagtgggtgaaggcatcgagaaagttgagactgactttgcagcagaagttgctgcgatgtccaagcagtcttaattatcaaaaaggagccgcctgagggcggcttctttttgtgcccatcttgtaaattcagctaacccttgtggggctgcgctgaaaagcgacgtacaatgtcgctagtattaattcatttcaatcgttgacagtctcaggaaagaaacatggctaccaatgcaaaacccgtctataaacgcattctgcttaagttgagtggcgaagctctgcagggcactgaaggcttcggtattgatgcaagcatactggatcgtatggctcaggaaatcaaagaactggttgaactgggtattcaggttggtgtggtgattggtgggggtaacctgttccgtggcgctggtctggcgaaagcgggtatgaaccgcgttgtgggcgaccacatggggatgctggcgaccgtaatgaacggcctggcaatgcgtgatgcactgcaccgcgcctatgtgaacgctcgtctgatgtccgctattccattgaatggcgtgtgcgacagctacagctgggcagaagctatcagcctgttgcgcaacaaccgtgtggtgatcctctccgccggtacaggtaacccgttctttaccaccgactcagcagcttgcctgcgtggtatcgaaattgaagccgatgtggtgctgaaagcaaccaaagttgacggcgtgtttaccgctgatccggcgaaagatccaaccgcaaccatgtacgagcaactgacttacagcgaagtgctggaaaaagagctgaaagtcatggacctggcggccttcacgctggctcgtgaccataaattaccgattcgtgttttcaatatgaacaaaccgggtgcgctgcgccgtgtggtaatgggtgaaaaagaagggactttaatcacggaataattcccgtgatggataaataagggtaagattccgcgtaagtatcgcgggggcgtaagtctggttataaggcgttattgttgcaggcagtttggtcacggccagcgcgcagcaaccggagcgtacaaaagtacgtgaggatggcgagcactgcccggggccaaaatggcaaataaaatagcctaataatccagacgattacccgtaatatgtttaatcagggctatacttagcacacttccactgtgtgtgactgtctggtctgactgagacaagttttcaaggattcgtaacgtgattagcgatatcagaaaagatgctgaagtacgcatggacaaatgcgtagaagcgttcaaaacccaaatcagcaaaatacgcacgggtcgtgcttctcccagcctgctggatggcattgtcgtggaatattacggcacgccgacgccgctgcgtcagctggcaagcgtaacggtagaagattcccgtacactgaaaatcaacgtgtttgatcgttcaatgtctccggccgttgaaaaagcgattatggcgtccgatcttggcctgaacccgaactctgcgggtagcgacatccgtgttccgctgccgccgctgacggaagaacgtcgtaaagatctgaccaaaatcgttcgtggtgaagcagaacaagcgcgtgttgcagtacgtaacgtgcgtcgtgacgcgaacgacaaagtgaaagcactgttgaaagataaagagatcagcgaagacgacgatcgccgttctcaggacgatgtacagaaactgactgatgctgcaatcaagaaaattgaagcggcgctggcagacaaagaagcagaactgatgcagttctgatttcttgaacgacaaaaacgccgctcagtagatccttgcggatcggctggcggcgttttgctttttattctgtctcaactctggatgtttcatgaagcaactcaccattctgggctcgaccggctcgattggttgcagcacgctggacgtggtgcgccataatcccgaacacttccgcgtagttgcgctggtggcaggcaaaaatgtcactcgcatggtagaacagtgcctggaattctctccccgctatgccgtaatggacgatgaagcgagtgcgaaacttcttaaaacgatgctacagcaacagggtagccgcaccgaagtcttaagtgggcaacaagccgcttgcgatatggcagcgcttgaggatgttgatcaggtgatggcagccattgttggcgctgctgggctgttacctacgcttgctgcgatccgcgcgggtaaaaccattttgctggccaataaagaatcactggttacctgcggacgtctgtttatggacgccgtaaagcagagcaaagcgcaattgttaccggtcgatagcgaacataacgccatttttcagagtttaccgcaacctatccagcataatctgggatacgctgaccttgagcaaaatggcgtggtgtccattttacttaccgggtctggtggccctttccgtgagacgccattgcgcgatttggcaacaatgacgccggatcaagcctgccgtcatccgaactggtcgatggggcgtaaaatttctgtcgattcggctaccatgatgaacaaaggtctggaatacattgaagcgcgttggctgtttaacgccagcgccagccagatggaagtgctgattcacccgcagtcagtgattcactcaatggtgcgctatcaggacggcagtgttctggcgcagctgggggaaccggatatgcgtacgccaattgcccacaccatggcatggccgaatcgcgtgaactctggcgtgaagccgctcgatttttgcaaactaagtgcgttgacatttgccgcaccggattatgatcgttatccatgcctgaaactggcgatggaggcgttcgaacaaggccaggcagcgacgacagcattgaatgccgcaaacgaaatcaccgttgctgcttttcttgcgcaacaaatccgctttacggatatcgctgcgttgaatttatccgtactggaaaaaatggatatgcgcgaaccacaatgtgtggacgatgtgttatctgttgatgcgaacgcgcgtgaagtcgccagaaaagaggtgatgcgtctcgcaagctgaggataatccggctacagagagtcgcgctatttgttagcgtagggcttcagtgatatagtctgcgccatctgatcgtaagtagttggctttataaggtcagatatgccgtggttttacacggcttttttttgtataggcttcagtattcctgagtaccgtaaaccctgtcagggaataaaaaacgcgtgatgttgtctgctactcaaccacttagcgaaaaattgccagcgcatggctgccgtcatgttgcgatcattatggacggcaatggccgctgggcaaaaaagcaagggaagattcgtgcctttgggcataaagccggggcaaaatccgtccgccgggctgtctcttttgcggccaacaacggtattgaggcgttaacgctgtatgcctttagtagtgaaaactggaaccgaccagcgcaggaagtcagtgcgttaatggaactgtttgtgtgggcgctcgatagcgaagtaaaaagtctgcaccgacataacgtgcgtctgcgtattattggcgataccagtcgctttaactcgcgtttgcaagaacgtattcgtaaatctgaagcgctaacagccgggaataccggtctgacgctgaatattgcggcgaactacggtggacgttgggatatagtccagggagtcaggcaactggctgaaaaggtgcagcaaggaaacctgcaaccagatcagatagatgaagagatgctaaaccagcatgtctgtatgcatgaactggcccctgtagatttagtaattaggactgggggggagcatcgcattagtaactttttgctttggcaaattgcctatgccgaactttactttacagatgttctctggcccgatttcgatgaacaagactttgaaggggcgttaaatgcctttgctaatcgagagcgtcgtttcggcggcaccgagcccggtgatgaaacagcctgatgggggtcgcttttgctgaagtatcgcctgatatctgcttttgtgttaatacccgtcgtcatcgcggcgttgtttctgttgccgccggtggggttcgccattgtaacgctggtggtctgcatgctggcagcgtgggaatggggacagcttagcggttttaccactcgttcgcagcgagtatggttggcggtgttatgcgggttattgttggcgctgatgctttttctgttgccggaatatcaccgaaatattcatcaaccgctggttgaaatctcactttgggcttcgctgggttggtggattgtcgcgctattgctggtgctgttttacccaggttccgcagcaatctggcgtaactctaaaacattgcgccttatttttggcgtgctaaccattgttcccttcttctggggcatgctggcgttacgggcctggcactatgacgagaatcattacagtggcgcaatatggctgctctatgtcatgatcctggtatggggcgctgactccggcgcatatatgtttggcaaattgtttggtaaacataagctggcaccgaaggtttctccgggtaaaacctggcaaggctttatcggtggactcgctactgcagcggtaatctcatggggttatggcatgtgggcgaatctcgacgtcgctcccgtcaccttactcatttgctctattgtcgcagcgttagcctcagtgctcggcgatctgaccgagagtatgtttaagcgtgaagcaggaattaaggacagcggtcatttaattccaggacacggtggtattttagatcgtattgatagcctgacggctgcggtaccggtctttgcttgcttgttgttactggtattcaggacgctttaacggaaggtaatatgctgagttttctctgggatttggcttcgttcatcgttgcactgggtgtacttatcaccgtgcatgaatttggtcatttctgggttgcccggcgttgtggtgttcgcgttgagcgtttctcaatagggtttggtaaggcgctctggcggcgaactgataagctcggcaccgaatatgttatcgccctgatcccgttgggcggttatgtcaaaatgctggatgagcgcgcagaaccggtcgttccggaactccgccaccatgccttcaataataaatctgtcggccaacgagcggcgattattgccgcaggtccggttgcaaacttcatttttgctatctttgcctactggctggtttttattattggtgtgcctggcgtacgtccggtggttggcgaaatagcagccaattcgatagctgcggaagcacaaattgcaccaggtacggaactaaaagccgtagatggtatcgaaacgcctgattgggatgccgtgcgtttgcagttggtcgataaaattggcgatgaaagcaccaccattacagtagcgccatttggcagcgaccaacggcgggatgtaaagctcgatttacgtcactgggcgtttgagcctgataaagaagatccggtatcttcgctggggattcgtcctcgtgggccgcaaattgaacctgtactggaaaatgtgcagccaaactcggcggcaagcaaggcaggtttgcaagcaggcgacaggatcgttaaagtcgatggtcagcccttaacgcagtgggtgacctttgtgatgcttgtccgggataacccgggtaaatccttagcgttagaaatcgaaaggcaggggagtcccttgtctttgacattaatcccggagagtaaaccgggtaatggtaaagcgattggttttgtcggtattgagccgaaagtcattcctttgccagatgagtataaagttgtacgccagtatgggccgttcaacgccatcgtcgaagccacggacaaaacgtggcagctgatgaagctgacggtcagtatgctgggaaaattgatcaccggtgatgtgaaactgaacaacctcagtgggccgatctctatcgccaagggggctgggatgacagcggaactcggggttgtttattacctgccgtttcttgcgcttattagcgtgaacttagggataattaacctgtttccgttgcccgtacttgacggggggcatctgctgttccttgcgatcgaaaagatcaagggcggaccggtatccgagcgggttcaagacttttgttatcgcattggctcgattctgctggtgctgttaatggggcttgcacttttcaatgatttctctcggttatgagagttagttaggaagaacgcataataacgatggcgatgaaaaagttgctcatagcgtcgctgctgtttagcagcgccaccgtatacggtgctgaagggttcgtagtgaaagatattcatttcgaaggccttcagcgtgtcgccgttggtgcggccctcctcagtatgccggtgcgcacaggcgacacggttaatgatgaagatatcagtaataccattcgcgctctgtttgctaccggcaactttgaggatgttcgcgtccttcgtgatggtgatacccttctggttcaggtaaaagaacgtccgaccattgccagcattactttctccggtaacaaatcggtgaaagatgacatgctgaagcaaaacctcgaggcttctggtgtgcgtgtgggcgaatccctcgatcgcaccaccattgccgatatcgagaaaggtctggaagacttctactacagcgtcggtaaatatagcgccagcgtaaaagctgtcgtgaccccgctgccgcgcaaccgtgttgacctaaaactggtgttccaggaaggtgtgtcagctgaaatccagcaaattaacattgttggtaaccatgctttcaccaccgacgaactgatctctcatttccaactgcgtgacgaagtgccgtggtggaacgtggtaggcgatcgtaaataccagaaacagaaactggcgggcgaccttgaaaccctgcgcagctactatctggatcgcggttatgcccgtttcaacatcgactctacccaggtcagtctgacgccagataaaaaaggtatttacgtcacggtgaacatcaccgaaggcgatcagtacaagctttctggcgttgaagtgagcggcaaccttgccgggcactccgctgaaattgagcagctgactaagatcgagccgggtgagctgtataacggcaccaaagtgaccaagatggaagatgacatcaaaaagcttctcggtcgctatggttatgcctatccgcgcgtacagtcgatgcccgaaattaacgatgccgacaaaaccgttaaattacgtgtgaacgttgatgcgggtaaccgtttctacgtgcgtaagatccgttttgaaggtaacgatacctcgaaagatgccgtcctgcgtcgcgaaatgcgtcagatggaaggtgcatggctggggagcgatctggtcgatcagggtaaggagcgtctgaatcgtctgggcttctttgaaactgtcgataccgatacccaacgtgttccgggtagcccggaccaggttgatgtcgtctacaaggtaaaagagcgcaacaccggtagcttcaactttggtattggttacggtactgaaagtggcgtgagcttccaggctggtgtgcagcaggataactggttaggtacaggttatgctgttggtatcaacgggaccaaaaacgattaccagacctatgctgaactgtcggtaaccaacccgtacttcaccgtagatggcgtaagcctcggtggtcgtctcttctataatgacttccaggcagatgacgccgacctgtccgactataccaacaagagttatggtacagacgtgacgttgggcttcccgattaacgaatataactcgctgcgtgcaggtctgggttatgtacataactccctgtccaacatgcagcctcaggttgcgatgtggcgttatctgtactctatgggtgaacatccgagcacctctgatcaggataacagcttcaaaacggacgacttcacgttcaactatggttggacctataacaagcttgaccgtggttacttcccgacagatggttcacgtgtcaacctgaccggtaaagtgaccattcctggatcggataacgaatactacaaagtgacgttagacacggcgacttatgtgccgatcgatgacgatcacaaatgggttgttctggggcgtacccgctggggttatggtgatggtttaggcggcaaagagatgccgttctacgagaacttctatgccggtggttccagcaccgtgcgtggcttccagtccaataccattggtccgaaagcagtttacttcccgcatcaggccagtaattatgatccggactatgattacgaatgtgcgactcaggacggcgcgaaagacctgtgtaaatcggatgatgctgtaggcggtaacgccatggcggttgccagcctcgagttcatcaccccgacgccgtttattagcgataagtatgctaactcggttcgtacttccttcttctgggatatgggtaccgtttgggatacaaactgggattccagccaatattctggatatccggactatagtgatccaagcaatatccgtatgtctgcgggtatcgcattacaatggatgtccccattggggccgttggtgttctcctacgcccagccgttcaaaaagtacgatggagacaaggcagaacagttccagtttaacatcggtaaaacctggtaagtgttctccacaaaggaatgtagtggtagtgtagcgatgactttaggcgatcaatataagatcgccgggccacgcaaagaactgcaccctccggtgcaaatgggatggtaaggagtttattgtgaaaaagtggttattagctgcaggtctcggtttagcactggcaacttctgctcaggcggctgacaaaattgcaatcgtcaacatgggcagcctgttccagcaggtagcgcagaaaaccggtgtttctaacacgctggaaaatgagttcaaaggccgtgccagcgaactgcagcgtatggaaaccgatctgcaggctaaaatgaaaaagctgcagtccatgaaagcgggcagcgatcgcactaagctggaaaaagacgtgatggctcagcgccagacttttgctcagaaagcgcaggcttttgagcaggatcgcgcacgtcgttccaacgaagaacgcggcaaactggttactcgtatccagactgctgtgaaatccgttgccaacagccaggatatcgatctggttgttgatgcaaacgccgttgcttacaacagcagcgatgtaaaagacatcactgccgacgtactgaaacaggttaaataagtaatgccttcaattcgactggctgatttagcgcagcagttggatgcagaactacacggtgatggcgatatcgtcatcaccggcgttgcgtccatgcaatctgcacaaacaggtcacattacgttcatggttaacccaaaataccgtgagcatttaggcttgtgccaggcgtccgcggttgtcatgacccaggacgatcttcctttcgcgaaaagtgccgcactggtagtgaagaatccctacctgacttacgcgcgcatggcgcaaattttagataccacgccgcagcccgcgcagaacattgcacccagtgcggtgatcgacgcgacggcgaagctgggtaacaacgtatcgattggcgctaacgcggtgattgagtccggcgttgaactgggcgataacgtgattatcggtgccggttgcttcgtaggtaaaaacagcaaaatcggtgcaggttcgcgtctctgggcgaacgtaaccatttaccatgagatccagatcggtcagaattgcctgatccagtccggaacagtggtaggcgcagacggctttggttatgccaacgatcgtggtaactgggtgaagatcccacagattggtcgcgtaattattggcgatcgcgtggagatcggtgcctgcacaaccatcgatcgcggcgcgctggatgacactattattggcaatggcgtgatcattgataaccagtgccagattgcacataacgtcgtgattggcgacaatacggcggttgccggtggcgtcattatggcgggcagcctgaaaattggtcgttactgcatgatcggcggagccagcgtaatcaacgggcatatggaaatatgcgacaaagtgacggttacgggcatgggtatggtgatgcgtcccatcactgaaccaggcgtctattcctcaggcattccgctgcaacccaacaaagtctggcgcaaaaccgctgcactggtgatgaacattgatgacatgagcaagcgtctgaaatcgcttgagcgcaaggttaatcaacaagactaacgttccatcttttgttcgccaaactttacggcctgtctcattcttacgattgcggcaggccgtgttattattgtcgtttcttatattttgacaggaagagtatcttgactactaacactcatactctgcagattgaagagattttagaacttctgccgcaccgtttcccgttcttactggtggatcgcgtgctggattttgaagaaggtcgttttctgcgcgcagtaaaaaatgtctctgtcaatgagccattcttccagggccatttccctggaaaaccgattttcccgggtgtgctgattctggaagcaatggcacaggcaacaggtattctggcgtttaaaagcgtaggaaaactggaaccgggtgagctgtactacttcgctggtattgacgaagcgcgcttcaagcgcccggtcgtgcctggcgatcaaatgatcatggaagtcactttcgaaaaaacgcgccgcggcctgacccgttttaaaggggttgctctggtcgatggtaaagtagtttgcgaagcaacgatgatgtgtgctcgtagccgggaggcctgatacgtgattgataaatccgcctttgtgcatccaaccgccattgtggaagagggcgcgtcaattggcgcgaacgcacacattggtcctttttgtatcgttggaccccatgtcgaaattggtgagggtaccgtactgaaatctcacgttgtcgtgaatggtcatactaaaattggccgcgataatgagatttatcagttcgcctccatcggcgaagttaaccaggatctgaaatatgctggcgaaccgacccgtgtggaaatcggcgatcgtaaccgcattcgcgaaagcgtcaccattcatcgtggcacagtccagggcggtggattgacgaaggtgggcagcgacaacttactgatgatcaacgcgcacattgcgcacgattgtacggtaggtaaccgctgtattctcgccaacaacgcaacgctggcgggtcacgtatcggttgacgacttcgcgatcatcggcggcatgaccgcagtccatcagttctgcatcattggtgcgcacgtgatggttggcggctgctccggtgtggcgcaggacgtccctccttatgtcattgcgcagggtaaccacgcaacgccgttcggtgtcaatatcgaagggctgaagcgccgcggattcagccgtgaggcgattaccgctatccgcaatgcgtataagctgatttatcgtagcggtaaaacgctcgatgaagtgaaaccggaaattgctgaactggcggaaacatatccggaagtgaaagcctttaccgatttctttgcacgctcaacgcgcggtctgattcgttaatgactgaacagcgtccattaacgattgccctggtcgccggagaaacctccggcgatatcctgggggccggtttaatccgcgctctgaaagaacatgtgcccaacgcccgctttgttggtgttgccgggccacgaatgcaggctgaaggctgcgaagcctggtacgaaatggaagaactggcggtgatgggcattgttgaagtgctcggtcgtctgcgtcgcttactgcatattcgtgccgatctgacaaagcgttttggcgaactgaagccagatgtttttgttggtattgatgcgcctgacttcaatattactcttgaaggtaacctcaaaaagcagggtatcaaaaccattcattacgtcagtccgtcagtctgggcgtggcgacagaaacgtgttttcaaaataggcagagccaccgatctggtgctcgcatttctgcctttcgaaaaagcgttttatgacaaatacaacgtaccgtgccgctttatcggtcataccatggctgatgccatgccattagatccagataaaaatgccgcccgtgatgtgctggggatccctcacgatgcccactgcctggcgttgctaccggggagccgtggtgcagaagttgaaatgcttagtgccgatttcctgaaaacggcccagcttttgcgccagacatatccggatctcgaaatcgtggtgccactggtgaatgccaaacgccgcgagcagtttgaacgcatcaaagctgaagtcgcgccagacctttcagttcatttgctggatgggatgggccgtgaggcgatggtcgccagcgatgcggcgctactggcgtcgggtacggcagccctggagtgtatgctggcgaaatgcccgatggtggtgggatatcgcatgaagccttttaccttctggttggcgaagcggctggtgaaaactgattatgtctcgctgccaaatctgctggcgggcagagagttagtcaaagaattattgcaggaagagtgtgagccgcaaaaactggctgcggcgctgttaccgctgttggcgaacgggaaaaccagccacgcgatgcacgataccttccgtgaactgcatcagcagatccgctgcaatgccgatgagcaggcggcacaagccgttctggagttagcacaatgatcgaatttgtttatccgcacacgcagctggttgcgggtgtggatgaagtcggacgcgggccgttagttggcgcggtcgtcaccgctgcggtgatccttgacccggcgcgcccgattgccgggctgaatgattccaaaaagctgagcgaaaaacgccgtctggcgctctatgaagagatcaaagagaaagcgttgagctggagtctgggccgcgcggaaccccacgaaatcgacgagctgaacattcttcatgcgaccatgctggcgatgcagcgtgccgtcgctgggctgcatattgcgccggaatatgtgttgattgatggtaaccgctgcccgaaattaccgatgcctgcgatggctgtggtgaaaggcgatagccgcgtaccggaaatcagtgccgcgtctatcctggcgaaagtgacgcgtgacgccgaaatggcggcgctggatattgttttcccgcaatatggttttgcccaacacaaagggtacccaaccgcttttcatctggaaaaactggctgaacacggcgcgaccgaacaccatcggcgcagctttgggcctgtcaaacgcgcactgggacttgcgtcctgattcttgtgtcgagattaagtaaaccggaatctgaagatgtctgaaccacgtttcgtacacctgcgggtgcacagcgactactcgatgatcgatggcctggccaaaaccgcaccgttggtaaaaaaggcggcggcgttgggtatgccagcactggcgatcaccgatttcaccaacctttgtggtctggtgaagttctacggagcgggacatggcgcagggattaagcctatcgtcggggcagattttaacgtccagtgcgacctgctgggtgatgagttaacccacctgacggtactggcggcgaacaataccggctatcagaatctgacgttgctgatctcaaaagcgtatcagcgcgggtacggtgccgccgggccgatcatcgatcgcgactggcttatcgaattaaacgaagggttgatccttctttccggcggacgcatgggcgacgtcggacgcagtcttttgcgtggtaacagcgcgctggtagatgagtgtgtcgcgttttatgaagaacacttcccggatcgctattttctcgagctgatccgcaccggcaggccggatgaagaaagctatctgcacgcggcggtggaactggcggaagcgcgcggtttgcccgtcgtggcgaccaacgacgtgcgctttatcgacagcagcgactttgacgcacacgaaatccgcgtcgcgatccacgacggctttaccctcgacgatcctaaacgcccgcgtaactattcgccgcagcaatatatgcgtagcgaagaggagatgtgtgagctgtttgccgacatccccgaagcccttgccaacaccgttgagatcgccaaacgctgtaacgtaaccgtgcgtcttggtgaatacttcctgccgcagttcccgaccggggacatgagcaccgaagattatctggtcaagcgtgcaaaagagggcctggaagagcgtctggcctttttattccctgatgaggaagaacgtcttaagcgccgcccggaatatgacgaacgtctggagactgaacttcaggttatcaaccagatgggcttcccgggctacttcctcatcgttatggaatttatccagtggtcgaaagataacggcgtaccggtagggccaggccgtggctccggtgcgggttcactggtggcctacgcgctgaaaatcaccgacctcgatccgctggaatttgacctgctgttcgaacgtttccttaacccggaacgtgtctccatgcctgacttcgacgttgacttctgtatggagaaacgcgatcaggttatcgagcacgtagcggacatgtacggtcgtgatgcggtatcgcagatcatcaccttcggtacaatggcggcgaaagcggtgatccgcgacgtaggccgcgtgctggggcatccgtacggctttgtcgatcgtatctcgaaactgatcccgcccgatccggggatgacgctggcgaaagcgtttgaagccgagccgcagctgccggaaatctacgaagcggatgaagaagttaaggcgctgatcgacatggcgcgcaaactggaaggggtcacccgtaacgccggtaagcacgccggtggggtggttatcgcgccgaccaaaattaccgattttgcgccgctttactgcgatgaagagggcaaacatccggtcacccagtttgataaaagcgacgttgaatacgccggactggtgaagttcgacttccttggtttgcgtacgctcaccatcatcaactgggcgctggagatgatcaacaagcggcgggcgaagaatggcgagccgccgctggatatcgctgcgatcccgctggatgataagaaaagcttcgacatgctgcaacgctcggaaaccacggcggtattccagcttgaatcgcgcggcatgaaggacctgatcaagcgtctacaacctgactgcttcgaagatatgatcgccctagtggcactgttccgccccggtccgttgcaatcagggatggtggataactttatcgaccgtaaacatggtcgtgaagagatctcctatccggacgtacagtggcagcatgaaagcctgaaaccggtactggagccaacctacggcattatcctgtatcaggaacaggtcatgcagattgcgcaggtgctttctggttataccctcggtggcgcggatatgctgcgtcgtgcgatgggtaagaaaaagccggaagagatggctaagcaacgttctgtatttgctgaaggtgcagaaaagaacggaatcaacgctgaactggcgatgaaaatcttcgacctggtggagaaattcgctggttacggatttaacaaatcgcactctgcggcctatgctttggtgtcatatcaaacgttatggctgaaagcgcactatcctgcggagtttatggcggcggtaatgaccgccgatatggacaacaccgagaaggtggtgggtctggtggatgagtgctggcggatggggctgaaaatcctgccaccagatataaactccggtctttaccatttccacgtcaacgacgacggcgaaatcgtgtatggtattggcgcgatcaaaggggtcggtgaaggtccgattgaggccatcatcgaagcccgtaataaaggcggctacttccgcgaactgtttgatctctgcgcccgtaccgacaccaaaaagttgaaccgtcgcgtgctggaaaaactgatcatgtccggggcgtttgaccgtcttgggccacatcgcgcagcgctgatgaactcgctgggcgatgcgttaaaagcggcagatcaacacgcgaaagcggaagctatcggtcaggccgatatgttcggcgtgctggccgaagagccggaacaaattgaacaatcctacgccagctgccaaccgtggccggagcaggtggtattagatggggaacgtgaaacgttaggcctgtacctgaccggacaccctatcaaccagtatttaaaagagattgagcgttatgtcggaggcgtaaggctgaaagacatgcacccgacagaacgtggtaaagtcatcacggctgcggggctcgttgttgccgcgcgggttatggtcaccaagcgcggcaatcgtatcggtatctgcacgctggatgaccgttccgggcggctggaagtgatgttgtttactgacgccctggataaataccagcaattgctggaaaaagaccgcatacttatcgtcagcggacaggtcagctttgatgacttcagcggtgggcttaaaatgaccgctcgcgaagtgatggatattgacgaagcccgggaaaaatatgctcgcgggcttgctatctcgctgacggacaggcaaattgatgaccagcttttaaaccgactccgtcagtctctggaaccccaccgctctgggacaattccagtacatctctactatcagagggcggatgcacgcgcgcggttgcgttttggcgcgacgtggcgtgtctctccgagcgatcgtttattaaacgatctccgtggcctcattggttcggagcaggtggaactggagtttgactaatacaggaatactatgagtctgaatttccttgattttgaacagccgattgcagagctggaagcgaaaatcgattctctgactgcggttagccgtcaggatgagaaactggatattaacatcgatgaagaagtgcatcgtctgcgtgaaaaaagcgtagaactgacacgtaaaatcttcgccgatctcggtgcatggcagattgcgcaactggcacgccatccacagcgtccttataccctggattacgttcgcctggcatttgatgaatttgacgaactggctggcgaccgcgcgtatgcagacgataaagctatcgtcggtggtatcgcccgtctcgatggtcgtccggtgatgatcattggtcatcaaaaaggtcgtgaaaccaaagaaaaaattcgccgtaactttggtatgccagcgccagaaggttaccgcaaagcactgcgtctgatgcaaatggctgaacgctttaagatgcctatcatcacctttatcgacaccccgggggcttatcctggcgtgggcgcagaagagcgtggtcagtctgaagccattgcacgcaacctgcgtgaaatgtctcgcctcggcgtaccggtagtttgtacggttatcggtgaaggtggttctggcggtgcgctggcgattggcgtgggcgataaagtgaatatgctgcaatacagcacctattccgttatctcgccggaaggttgtgcgtccattctgtggaagagcgccgacaaagcgccgctggcggctgaagcgatgggtatcattgctccgcgtctgaaagaactgaaactgatcgactccatcatcccggaaccactgggtggtgctcaccgtaacccggaagcgatggcggcatcgttgaaagcgcaactgctggcggatctggccgatctcgacgtgttaagcactgaagatttaaaaaatcgtcgttatcagcgcctgatgagctacggttacgcgtaattcgcaaaagttctgaaaaagggtcacttcggtggcccttttttatcgccacggtttgagcaggctatgattaaggaaggattttccaggaggaacacatgaacatcattgccattatgggaccgcatggcgtcttttataaagatgagcccatcaaagaactggagtcggcgctggtggcgcaaggctttcagattatctggccacaaaacagcgttgatttgctgaaatttatcgagcataaccctcgaatttgcggcgtgatttttgactgggatgagtacagtctcgatttatgtagcgatatcaatcagcttaatgaatatctcccgctttatgccttcatcaacacccactcgacgatggatgtcagcgtgcaggatatgcggatggcgctctggttttttgaatatgcgctggggcaggcggaagatatcgccattcgtatgcgtcagtacaccgacgaatatcttgataacattacaccgccgttcacgaaagccttgtttacctacgtcaaagagcggaagtacaccttttgtacgccggggcatatgggcggcaccgcatatcaaaaaagcccggttggctgtctgttttatgattttttcggcgggaatactcttaaggctgatgtctctatttcggtcaccgagcttggttcgttgctcgaccacaccgggccacacctggaagcggaagagtacatcgcgcggacttttggcgcggaacagagttatatcgttaccaacggaacatcgacgtcgaacaaaattgtgggtatgtacgccgcgccatccggcagtacgctgttgatcgaccgcaattgtcataaatcgctggcgcatctgttgatgatgaacgatgtagtgccagtctggctgaaaccgacgcgtaatgcgttggggattcttggtgggatcccgcgccgtgaatttactcgcgacagcatcgaagagaaagtcgctgctaccacgcaagcacaatggccggttcatgcggtgatcaccaactccacctatgatggcttgctctacaacaccgactggatcaaacagacgctggatgtcccgtcgattcacttcgattctgcctgggtgccgtacacccattttcatccgatctaccagggtaaaagtggtatgagcggcgagcgtgttgcgggaaaagtgatcttcgaaacgcaatcgacccacaaaatgctggcggcgttatcgcaggcttcgctgatccacattaaaggcgagtatgacgaagaggcctttaacgaagcctttatgatgcataccaccacctcgcccagttatcccattgttgcttcggttgagacggcggcggcgatgctgcgtggtaatccgggcaaacggctgattaaccgttcagtagaacgagctctgcattttcgcaaagaggtccagcggctgcgggaagagtctgacggttggtttttcgatatctggcaaccgccgcaggtggatgaagccgaatgctggcccgttgcgcctggcgaacagtggcacggctttaacgatgcggatgccgatcatatgtttctcgatccggttaaagtcactattttgacaccggggatggacgagcagggcaatatgagcgaggaggggatcccggcggcgctggtagcaaaattcctcgacgaacgtgggatcgtagtagagaaaaccggcccttataacctgctgtttctctttagtattggcatcgataaaaccaaagcaatgggattattgcgtgggttgacggaattcaaacgctcttacgatctcaacctgcggatcaaaaatatgctacccgatctctatgcagaagatcccgatttctaccgcaatatgcgtattcaggatctggcacaagggatccataagctgattcgtaaacacgatcttcccggtttgatgttgcgggcattcgatactttgccggagatgatcatgacgccacatcaggcatggcaacgacaaattaaaggcgaagtagaaaccattgcgctggaacaactggtcggtagagtatcggcaaatatgatcctgccttatccaccgggcgtaccgctgttgatgcctggagaaatgctgaccaaagagagccgcacagtactcgattttctactgatgctttgttccgtcgggcaacattaccccggttttgaaacggatattcacggcgcgaaacaggacgaagacggcgtttaccgcgtacgagtcctaaaaatggcgggataacttgccagagcggcttccgggcgagtaacgtgctgttaacaaataaaggagacgttatgctgggtttaaaacaggttcaccatattgcgattattgcgacggattatgcggtgagcaaagctttctactgcgatattcttggtttcacgctgcaaagcgaagtctatcgcgaagcgcgcgactcatggaaaggggatttggcgcttaatgggcaatatgtgattgagcttttctcatttccgttcccgccggaacgacccagccgaccggaagcttgcggtctgcgtcatctggcttttagcgttgatgacatcgatgcggcagtggcgcaccttgaaagccataacgtgaagtgtgaaaccatccgtgtcgatccatacacgcaaaaacgcttcaccttctttaacgatccggacgggctgccgttggaactgtatgagcagtaaggcttgtcatcgccgcatttgcccggtaacgtgccgggcattgctactgtaaaatcgcaccatcatgacactcacgctcaatagacaacttctcacctcacgccagattctggtggcctttagcggcgggcttgactccaccgttctgctgcatcagttggtgcagtggcggacggaaaatccgggtgtcgctctgcgcgctattcatgtgcatcacggtttaagtgccaatgccgatgcctgggttacgcattgcgaaaacgtctgccaacagtggcaggtgccgctggtggtcgaacgcgtacaacttgcgcaagaaggactgggcattgaggcccaggcgcggcaggcacgttatcaggcatttgcccgcaccttgttgcccggtgaagtgctggtcaccgcgcaacatctcgacgatcaatgtgaaacctttctgctggcgctaaaacgcggcagtggccctgccgggctttcggctatggcggaagtctcggagtttgccggaacgcggcttattcgcccgttgctcgcccgcacgcggggggaactggtgcagtgggcgcgtcagtatgatttacgctggattgaagacgaaagtaatcaggacgactcatacgatcgtaactttctgcgcctgcgcgtagtgccgttattgcagcagcgttggccgcattttgccgaagcaacggcccgcagcgccgcactttgtgctgaacaagagagcctgctggatgaactgctggcagatgatttagcacactgtcaatcgccgcaggggacgctgcagattgtgccaatgctggcgatgagtgatgcccgccgcgcggcgattatccgccgctggctggcagggcagaatgcaccgatgccttcccgcgacgcgttggtgaggatctggcaggaagtggcgctggcgcgggaagatgcctcaccctgtttacgtttgggcgcgtttgaaatccgacgctatcagtcgcaactgtggtggattaaatccgtcaccgggcaaagcgaaaacattgtgccgtggcagacgtggcttcaaccgctggaattaccggcggggctgggaagtgtacagcttaatgcgggaggcgatattcgccctccgcgtgcagacgaagcggtcagcgtgcgtttcaaagcgccaggattgctgcatattgtcgggcgtaacggcggacgtaagctaaagaaaatctggcaagagctgggcgtgccgccgtggctacgtgacaccacgccactgctgttttatggcgaaacgctgattgcggcggcaggggtatttgtgacgcaagaaggtgtggctgaaggtgagaatggcgtaagttttgtctggcagaaaacgcttagttaagtgaaagccggataagacgcatcaaacgtcgcatccggcgaaagtcaatcaggattcgcttaccaccaccgtaccgatttccgggtggctaaagctggtaattttatccagacgcagctcgcgggtttcgccagcggcctcgacgaccaggtactccacatttttgcgggagactaaatcactggcttttgcctgcaatttttcgccatctttcagctcaagtgtcagcattaaatgatgctggcaggcgagctcaagattatcgtaatcatcacaattgattggttgatacgtatcattcattgacataatcgctcaccagtaagtttgccgcagcgtatgctgctttttccctgacagcctcagaaagggcgtcgtcggcagccatttcattcagcactttcaaaacgcagcccagcgcgtccggaacgtatcctaagtctccgctggcgatttccgcgtaccgcttgcgtattaactcacaatatttttccacatgccctcctgtcagcactctgacttaaccgtggatgcaagtctaagcctacgaagataaactctgtttcgcaaggtgactataccacactcatttctgcaatatcagcgccgcaactgcacgtattccgttacaatggcctcctgattcgaaaggagttttcttatggcgcttaaagcgacaatttataaagcgacggttaatgtggccgatctcgaccgcaaccagtttctcgatgcctctctgacgctggcgcgccatccttcagaaacccaggagcgtatgatgctgcgcttgctggcgtggctgaaatatgctgatgaacgtctgcaatttacccgtggtttgtgtgccgatgatgagccggaagcgtggctgcgtaacgatcacctgggcattgatttgtggattgagctggggctgccggatgagcggcggattaagaaagcctgcacccaggccgcagaagtggcgctgtttacctataatagtcgggcggcgcaaatctggtggcagcaaaatcagagcaaatgtgtgcagtttgccaatctttccgtctggtatctggacgatgaacaactggcgaaagtaagcgcctttgccgatcgtaccatgacgctgcaggcaacgattcaggatggcgtgatctggttatcggatgataagaataatctggaagtgaacttaaccgcctggcaacaaccttcatgattgtgatttcccgacatgttgctattcccgatggtgagcttgagatcaccgccattcgtgcgcagggcgcgggcgggcagcatgttaataagacctcaacggctattcatctgcgttttgacattcgggcgtccagcctgccagagtattacaaagagcgtctgctcgccgccagccatcatttgatcagcagtgatggcgtgattgtcattaaggcacaggaataccgcagtcaggaactgaaccgcgaagcagctctggcccggctggtggctatgattaaagaattaacaacagaaaaaaaagcccgacgacccacgcggcccacccgtgcatcgaaagagcgcaggctggcatcgaaagcacaaaaatcaagcgtgaaggcgatgcgcggcaaagtgcgcagcggtcgggaataaaaagaaggaatggatggtgaaaaaagcgatagtgacagcgatggctgtaatcagcctctttactctgatgggatgtaataatcgggccgaagtcgatacgctttctccggcgcaggctgccgaactgaaaccgatgccgcaaagttggcgcggcgtgctgccgtgtgccgattgcgaaggaatcgaaacctctctgttcctcgaaaaagacggaacatgggtgatgaatgagcgttatctcggtgctcgtgaagaaccttcctccttcgcttcctacggtacatgggcgcgaaccgctgacaagctggtattaaccgacagcaaaggtgaaaagtcatattatcgggcgaaaggcgatgcgctggagatgctcgatcgtgaaggcaatccgattgaatcgcagttcaactatacgctggaagcggcacaatccagtttacctatgacgccgatgaccctgcggggcatgtatttttatatggctgatgcggcgaccttcactgattgcgcgaccggaaaacgtttcatggtagcgaataacgcagagctggagcgtagctacctggctgcgcgcggtcacagtgaaaaaccggtgttactgtcagtagaaggtcactttacgcttgagggtaatccggataccggtgcgccgactaaagtattggcacccgatacggcagggaaattttaccccaaccaggattgcagtagtttggggcagtaacccgtcttgagacagaaacaaacgcaaaacaggccagaaggatatatttcaacattttgaatttgcacgttttttgtaggccggataaggcgtttacgccgcatccggcaatggtgctcaacgcctgatgcgacgctggcgcgtcttatcatgcctacaacccccctcataccttaaggcggataaggcatttactttatcaccgggtcaaaccaacaaagcgacccgccttgatataaatcccaggcttcaggtgcccaacatactgtaactgcgtttctggcttaaacgcagagacatcaccaatacgcatatgcatcagatcggcagggctaatccagcccgattgcgccagtgtaagtggatgcccggctttggcaaaggcatccgtgacaaattccgaacaaaaccacgactttttgtctccttcgcccacactgcttaactgcgctttcgccaggccgctgacgcactgttggcgaaaatcctcggagaacggattcagtgagcacatctggcgagtcaccataaagggaataaattcgacaatgccgcgatagttataaccgctatctttgattttattggcaaacgcggtgatatctgtggcttgttgcggggtaagatccgggactcgtaagacgaaaagcttatcactatgcttcatcgcttttttaagggaaacgatctggacgccagcgcctgtcgcttctgcaacgttattatcacccagaaagattgcaacgtgactcacagaggaagtgctgaagacgcggattccaaatgaggttaccccaaggcttgaggagaacagcaaatcgccgggtttgagatcaggtgccgttatttcttttattgattgttcggtgaaagagctttgatgctggaatttgacagcccatgtttttgcctcggcatctactgctgtggctgatgggtctggctggctgatatcaacggtacaagccgaaagtaaaagaaagctggggagaaacaggcggcagtacgcctttggtttatccattttatacaatccatgtaaaaaaagggccctgaaattcaggaccctttctggcatcagcctttaatctgtttcaccagatattcgacgatgtcaccagtcttaattaactgtttctcgccgttgcgacgatatttatattcgatatcgtcgttgtcgaggttacggtcgcccagcacaatagtgtgcggaataccgatcagttccatatcagcaaacatcacgcccggacgctctttgcggtcatccagcagcacttcgataccttgtgcacgcagttcgctgtacagtttctcagcaagctcttgtacgcggaaggatttgtgcatgttcatcggcagaatcgccacctggaacggcgcgatagcgtcaggccatacgatgcctcgttcgtcgtagttctgctcaatcgccgcagctaccacacgcgttaccccgataccgtagcaacccatcgtcaggatttggttacggccatcttcaccctgtacggaggctttcagtgcttcggagtacttggtacccagctggaagatgtgaccaacttcgataccacgtttgatcagcagcctaccctggccatccgggcttggatcgccagccaccacgttacggatatctgcaacttccggggtagcgacatcgcgatcccagttgatgccgaagtagtgtttaccatcgatgttagcaccagcagcgaaatcactcatcgccgcaacggtacggtcaatcaccaccggaatcggcatgtttaccggacccagtgaacccggaccggctttaaccacggcacgaatttcttcttcggtcgcgaaagtcagcgggcttgcaacctgcggcagtttttctgctttaacttcgttcagctcgtgatcaccgcgcaccagcagcgcaacctgcgggaagctgctgccttcaaccgctttaaccagcagagtcttaaccgttttctcaatcggcagattgaactgttcaaccagttccgcgatggttttcgcgttcggcgtatcaaccagcgtcatttcctgggtagcagcagcgcgcggttctttcggcgcgatagcttctgccagttcaatgttcgctgcatagtcagaggtgtcggagaagaccacatcgtcttcaccgctctgcgccagcacctggaattcgtgagaggcgctgccgccgatagaaccggtgtcggcttgtacggcgcggaaatccagccccatgcggctgaagattttgctgtaggccgcatacattgcatcgtaggtttcctgcagggattcctgagaagtatggaaagagtaagcatctttcatcaggaattcgcgggaacgcatgacgccgaaacgcggacgcacttcgtcgcggaacttggtctggatctgatagaagttcagcggcagctgtttgtaagagctaagctcgttacgaatcaggtcagtgataacttcttcatgagttgggccgagtacgaacggacgctcgccacggtcaacaaaacgcagcagttccggaccgtactgttcccaacgaccactctcttgccacaaatcggctggctgaaccaccggcatcgacacctcgatcgcaccggcgttgttcatctcttcacgcacgatgttttcgacttttttcagaacgcgcacgccggtcggcagccaggtatataacccggaggccagcttgcggatcatcccggcgcgcagcatcagctgatggctgatcacctcggcgtcggcaggtgtctccttgagagtggagagcaggtattggctagtacgcatgttgttacggttccagttggaaggtagaacaggctcaaggcgagcctgggacaaaaaaaagtgatttagtttaccagtgcaaaagaaatgtcaaaagagaagggcgtgaatttaacgcggttccagcgcaaagacttcaaaacctgcgtcggtgacgcgccagcgaacgttaaaatcatgtagccagacggcataggttttgcccgtttcctcacctttacgataggccgggcgcgggtcctgcgccagtacttcgcggataaacagcgttaactgcggataacgcttctccagcgtcaaaagctgcttttcgacctctgcggtaaaactcaccgccatctctgcagctggcgcactttgcgcatagctggcactggcatcgggaagcgattcggcaaaggggagatacggtttgatatccactaccggcgtaccatcgaccagatccagactgccgagcttcagaatcacgctgtctttatggcaaacaacctctttcagctctaccagcgacatgccaattgggttagggcggaaagtagagcgtgttgcgaaaacccccattctggcgttaccgccgaggcgcggtggacgcacagtcggacgccagccgccttccatcgtttgatgaaagacgaaaaggatccataaatggctgaacgcttccaggccgcgaacggcgtcggcctggttgtagggagcaatgagatgcagttcgccgttggcgctttttaccagacctggctggcgcggaacggcgaacttttctttatagggcgagcgaataacgcctatttgctcgaactggaaactgctcatttcgccgtaatgttaagcgcagaaccgatacatacagcctgacgatagcagcctggcgtaccgctggtgacttcgcagctatgcagtaatacagcattggctttcattttagaggcgttgatttgcatccgcttacgtgcggttggaatgctcggcggagagtcctgattagaggcctggcaagagtcgccactgacttcaccgagatcgcggaacggtttgccgactaattcttctgcattggtataaattcggaccggcgtggcgcgcggcgctttcggttttgcaggctccgctttcggctggggtgcagtgctttgaacgggttcgacaggggatctgcttaacatggaacagccgcttagcatgagtgctactaaacagatcggtaaagcacgcatagtatttcctcaatgtatgatcaaaacgtcaatattgaatcaggagcttgtaaaaatgacaagacgggcaagcgcccgtcctgaatgatattacaaattgtggaaacagcctaaaaattaccagcctttaacagctccgccgttaaacactttgtttgctgcttcgtaaacttcgtcagactgataagcctggacgaatttcttcacgttctcggcgtctttgttatcttcacgcgtcacgatcaggtttacgtacggggactctttatcttcaacaaagataccgtctttcgccggagtcaggccaatctggctggcataggtggtattgataactgccagagcgatttgcgcgtcgtccagagaacgcggcagttgcggtgcttccagttcaacaattttcagatttttggggttctcaacaacatcaagaacggtcggcagcaggccaacgccatctttcagtttgatcaagcccactttttgcagcagcagcagtgaacgaccaaggttagttgggtcgtttggcacggcaacctgcgaaccatcctgcagttcatccagtgatttgattttcttggagtaaccagcaatcggataaacaaaagtgttgcctactgcgaccagtttgtagccacgatctttcagttgctgatcaaggtacggtttatgctggaaggcgttggcgtcgatatcgcctttgctcaatgcttcgtttggcagaacatagtcgttgaaggttaccagctcaacgtccaggccatatttgtctttcgcaactttctgcgcgacttctgcaacctgctgttcggcaccaacaatcacgccgactttaatgtggtttggatctttttcatcctgaccgcagcctaccagtgccagtgatccgatcagggctcccactgccgcaaaggttttgaatttgaacgccataccttattccttcttcaattatttatgttgtgttgaacgttacttgcgagtgacagcccggacgatgcggtcgcctgcgaactgaattaaataaaccagaatgaccagcaataccagtaccgtattcatcaccgtcgcgttatagccgatgtagccatactgatagccaatctgacctaaaccaccggcaccgactgcaccacccatcgcggaataaccgaccagggtaatcagggtgatagttgccgcattcaccagacccggcagcgcttccggtaacagcaccttacggacgatctgcatcggcgtggcacccattgcgcgggaagcttcaattaacccggttgggatctccagcagagcgttctcgaccatacgggcaataaacggtgctgcaccaacggttaacggaacaatcgctgcctgcaaaccaatcgatgtaccgacaataacgcgggtaaacggaatcatccatacaagcaagataatgaacgggatggaacggaaaatgttcacaatcgcagaaacggtacgatacagcttcgcgttagcaataatttgccccggacgcgtgacataaagcagaacgccaaccggcagaccaatcacaaagccaaaaaaaccggatacgaaggtcattgccagcgtttcccatacgccacgaaccagcagccacatcatcggctcagacataacccagtacctctacttttacatggtgttcctgcagccaggcaatggcggcttgcgtatcttgttgtgtgccgtgcatttcagtcagcatgatgccgaacttaacgccaccggcgtaatccatctgcgcgctaataatgttgttgttgacgttgaaacgacgcgcggtttcagaaagcagtggggcatcgaccgattgaccggtaaactccagacgcagcatcggcacgcagtcagtaaatggctccgcttgcagacgttcctggtaatcttccgggatatccagatgcagggtcgactgaataaacttctgcgccagcggcgttttcggatgcgagaacacttcacttaccgtgtcctgctcgatcagttctccattgctgatgaccgccacgcaatcacaaatgcgcttcacaacgtccatttcgtgggtgatcaacagaatcgtcaaccccagacggcggttgatgtctttcagcagttcgagaatagaacgtgtcgttgccgggtccagcgcgctggtggcttcatcacacagcaatactttgggattgctggctaacgcacgggcaattgccacacgttgtttctgcccaccggaaagattcgacgggtagctatcatgcttatcgccaagaccaaccaatgacagcaattccgtcacgcgacgtttgacctcgtctttcggtgtgttgtccagctccagcggcagagccacgttgccaaaaacagtacgcgaagagagcaggttaaaatgctggaaaatcataccaatctggcggcgagctttggtcaactcggattctgacagcgtggtcagttcctggccatcgaccagcacgctaccctcggttgggcgctccagcaggtttacacaacgtataagcgtactcttacccgcgcctgaggcaccgataacgccataaatttgtccagctggcacatgcaggctgacgttgttcaacgcctggatggtgcgggtgccctggtggaacactttggtgatattcgaaagttttatcattgattatttattatcgtcattaagttagtcgtggcatctcgaatgcctgaaacgggcaacgccgtcaatgaaatggatgttaaggcatccagacgtctaaatcaatcaggtttatgcgaagagcactttcttgcaggtcgaaacatgcgatactagcgtcacatgccttattaaggagctataaaaggtggcgaagagcgtacccgcaatttttcttgaccgtgatggcaccattaatgtcgatcacggctatgtccatgagatcgacaactttgaatttatcgacggtgttattgacgccatgcgcgagctaaaaaaaatgggctttgcgctggtggtagtaaccaaccagtctggcattgctcgcggtaaatttaccgaagcacagtttgaaacgctgaccgagtggatggactggtcgctggcggaccgagatgtcgatctggatggtatctattattgcccgcatcatccgcagggtagtgttgaagagtttcgccaggtctgcgattgccgcaaaccacatccggggatgcttttgtcagcacgcgattatttgcatattgatatggccgcttcttatatggtgggcgataaattagaagatatgcaggcagcggttgcggcgaacgtgggaacaaaagtgctggtgcgtacgggtaaacctattacgcctgaagcagaaaacgcggcggattgggtgttaaatagcctggcagacctgccgcaagcgataaaaaagcagcaaaaaccggcacaatgattaaaagatgagcggttgaaataaaaatgcatttttccgcttgtcttcctgagccgactccctataatgcgcctccatcgacacggcggatgtgaatcacttcacacaaacagccggttcggttgaagagaaaaatcctgaaattcagggttgactctgaaagaggaaagcgtaatatacgccacctcgcgacagtgagctgaaagccgcgtcgcaactgctctttaacaatttatcagacaatctgtgtgggcactcgaagatacggattcttaacgtcgcaagacgaaaaatgaataccaagtctcaagagtgaacacgtaattcattacaaagtttaattctttgagcatcaaacttttaaattgaagagtttgatcatggctcagattgaacgctggcggcaggcctaacacatgcaagtcgaacggtaacaggaagaagcttgcttctttgctgacgagtggcggacgggtgagtaatgtctgggaaactgcctgatggagggggataactactggaaacggtagctaataccgcataacgtcgcaagaccaaagagggggaccttcgggcctcttgccatcggatgtgcccagatgggattagctagtaggtggggtaacggctcacctaggcgacgatccctagctggtctgagaggatgaccagccacactggaactgagacacggtccagactcctacgggaggcagcagtggggaatattgcacaatgggcgcaagcctgatgcagccatgccgcgtgtatgaagaaggccttcgggttgtaaagtactttcagcggggaggaagggagtaaagttaatacctttgctcattgacgttacccgcagaagaagcaccggctaactccgtgccagcagccgcggtaatacggagggtgcaagcgttaatcggaattactgggcgtaaagcgcacgcaggcggtttgttaagtcagatgtgaaatccccgggctcaacctgggaactgcatctgatactggcaagcttgagtctcgtagaggggggtagaattccaggtgtagcggtgaaatgcgtagagatctggaggaataccggtggcgaaggcggccccctggacgaagactgacgctcaggtgcgaaagcgtggggagcaaacaggattagataccctggtagtccacgccgtaaacgatgtcgacttggaggttgtgcccttgaggcgtggcttccggagctaacgcgttaagtcgaccgcctggggagtacggccgcaaggttaaaactcaaatgaattgacgggggcccgcacaagcggtggagcatgtggtttaattcgatgcaacgcgaagaaccttacctggtcttgacatccacagaactttccagagatggattggtgccttcgggaactgtgagacaggtgctgcatggctgtcgtcagctcgtgttgtgaaatgttgggttaagtcccgcaacgagcgcaacccttatcttttgttgccagcggtccggccgggaactcaaaggagactgccagtgataaactggaggaaggtggggatgacgtcaagtcatcatggcccttacgaccagggctacacacgtgctacaatggcgcatacaaagagaagcgacctcgcgagagcaagcggacctcataaagtgcgtcgtagtccggattggagtctgcaactcgactccatgaagtcggaatcgctagtaatcgtggatcagaatgccacggtgaatacgttcccgggccttgtacacaccgcccgtcacaccatgggagtgggttgcaaaagaagtaggtagcttaaccttcgggagggcgcttaccactttgtgattcatgactggggtgaagtcgtaacaaggtaaccgtaggggaacctgcggttggatcacctccttaccttaaagaagcgtactttgcagtgctcacacagattgtctgatgaaaatgagcagtaaaacctctacaggcttgtagctcaggtggttagagcgcacccctgataagggtgaggtcggtggttcaagtccactcaggcctaccaaatttgcacggcaaatttgaagaggttttaactacatgttatggggctatagctcagctgggagagcgcctgctttgcacgcaggaggtctgcggttcgatcccgcatagctccaccatctctgtagtggttaaataaaaaatacttcagagtgtacctgcaaaggttcactgcgaagttttgctctttaaaaatctggatcaagctgaaaattgaaacactgaacaatgaaagttgttcgtgagtctctcaaattttcgcaacacgatgatggatcgcaagaaacatcttcgggttgtgaggttaagcgactaagcgtacacggtggatgccctggcagtcagaggcgatgaaggacgtgctaatctgcgataagcgtcggtaaggtgatatgaaccgttataaccggcgatttccgaatggggaaacccagtgtgtttcgacacactatcattaactgaatccataggttaatgaggcgaaccgggggaactgaaacatctaagtaccccgaggaaaagaaatcaaccgagattcccccagtagcggcgagcgaacggggaggagcccagagcctgaatcagtgtgtgtgttagtggaagcgtctggaaaggcgcgcgatacagggtgacagccccgtacacaaaaatgcacatgctgtgagctcgatgagtagggcgggacacgtggtatcctgtctgaatatggggggaccatcctccaaggctaaatactcctgactgaccgatagtgaaccagtaccgtgagggaaaggcgaaaagaaccccggcgaggggagtgaaaaagaacctgaaaccgtgtacgtacaagcagtgggagcatgcttaggcgtgtgactgcgtaccttttgtataatgggtcagcgacttatattctgtagcaaggttaaccgaataggggagccgaagggaaaccgagtcttaactgggcgttaagttgcagggtatagacccgaaacccggtgatctagccatgggcaggttgaaggttgggtaacactaactggaggaccgaaccgactaatgttgaaaaattagcggatgacttgtggctgggggtgaaaggccaatcaaaccgggagatagctggttctccccgaaagctatttaggtagcgcctcgtgaactcatctccgggggtagagcactgtttcggcaagggggtcatcccgacttaccaacccgatgcaaactgcgaataccggagaatgttatcacgggagacacacggcgggtgctaacgtccgtcgtgaagagggaaacaacccagaccgccagctaaggtcccaaagtcatggttaagtgggaaacgatgtgggaaggcccagacagccaggatgttggcttagaagcagccatcatttaaagaaagcgtaatagctcactggtcgagtcggcctgcgcggaagatgtaacggggctaaaccatgcaccgaagctgcggcagcgacgcttatgcgttgttgggtaggggagcgttctgtaagcctgtgaaggtgtactgtgaggtatgctggaggtatcagaagtgcgaatgctgacataagtaacgataaagcgggtgaaaagcccgctcgccggaagaccaagggttcctgtccaacgttaatcggggcagggtgagtcgacccctaaggcgaggccgaaaggcgtagtcgatgggaaacaggttaatattcctgtacttggtgttactgcgaaggggggacggagaaggctatgttggccgggcgacggttgtcccggtttaagcgtgtaggctggttttccaggcaaatccggaaaatcaaggctgaggcgtgatgacgaggcactacggtgctgaagcaacaaatgccctgcttccaggaaaagcctctaagcatcaggtaacatcaaatcgtaccccaaaccgacacaggtggtcaggtagagaataccaaggcgcttgagagaactcgggtgaaggaactaggcaaaatggtgccgtaacttcgggagaaggcacgctgatatgtaggtgaagcgacttgctcgtggagctgaaatcagtcgaagataccagctggctgcaactgtttattaaaaacacagcactgtgcaaacacgaaagtggacgtatacggtgtgacgcctgcccggtgccggaaggttaattgatggggttagcgcaagcgaagctcttgatcgaagccccggtaaacggcggccgtaactataacggtcctaaggtagcgaaattccttgtcgggtaagttccgacctgcacgaatggcgtaatgatggccaggctgtctccacccgagactcagtgaaattgaactcgctgtgaagatgcagtgtacccgcggcaagacggaaagaccccgtgaacctttactatagcttgacactgaacattgagccttgatgtgtaggataggtgggaggctttgaagtgtggacgccagtctgcatggagccgaccttgaaataccaccctttaatgtttgatgttctaacgttgacccgtaatccgggttgcggacagtgtctggtgggtagtttgactggggcggtctcctcctaaagagtaacggaggagcacgaaggttggctaatcctggtcggacatcaggaggttagtgcaatggcataagccagcttgactgcgagcgtgacggcgcgagcaggtgcgaaagcaggtcatagtgatccggtggttctgaatggaagggccatcgctcaacggataaaaggtactccggggataacaggctgataccgcccaagagttcatatcgacggcggtgtttggcacctcgatgtcggctcatcacatcctggggctgaagtaggtcccaagggtatggctgttcgccatttaaagtggtacgcgagctgggtttagaacgtcgtgagacagttcggtccctatctgccgtgggcgctggagaactgaggggggctgctcctagtacgagaggaccggagtggacgcatcactggtgttcgggttgtcatgccaatggcactgcccggtagctaaatgcggaagagataagtgctgaaagcatctaagcacgaaacttgccccgagatgagttctccctgactccttgagagtcctgaaggaacgttgaagacgacgacgttgataggccgggtgtgtaagcgcagcgatgcgttgagctaaccggtactaatgaaccgtgaggcttaaccttacaacgccgaagctgttttggcggattgagagaagattttcagcctgatacagattaaatcagaacgcagaagcggtctgataaaacagaatttgcctggcggccgtagcgcggtggtcccacctgaccccatgccgaactcagaagtgaaacgccgtagcgccgatggtagtgtggggtctccccatgcgagagtagggaactgccaggcatcaaattaagcagtaagccggtcataaaaccggtggttgtaaaagaattcggtggagcggtagttcagtcggttagaatacctgcctgtcacgcagggggtcgcgggttcgagtcccgtccgttccgccacttattaagaagcctcgagttaacgctcgaggttttttttcgtctgtatatctattattgccagaatcgcaaaaatcctctgcattttacgctctttttcctcaacagtctgaagcccataatcacctcagttaacgaaaatagcattaaaagaggcatattatggctatccctgcatttggtttaggtactttccgtctgaaagacgacgttgttatttcatctgtgataacggcgcttgaacttggttatcgcgcaattgataccgcacaaatctatgataacgaagccgcagtaggtcaggcgattgcagaaagtggcgtgccacgtcatgaactctacatcaccactaaaatctggattgaaaatctcagcaaagacaaattgatcccaagtctgaaagagagcctgcaaaaattgcgtaccgattatgttgatctgacgctaatccactggccgtcaccaaacgatgaagtctctgttgaagagtttatgcaggcgctgctggaagccaaaaaacaagggctgacgcgtgagatcggtatttccaacttcacgatcccgttgatggaaaaagcgattgctgctgttggtgctgaaaacatcgctactaaccagattgaactctctccttatctgcaaaaccgtaaagtggttgcctgggctaaacagcacggcatccatattacttcctatatgacgctggcgtatggtaaggccctgaaagatgaggttattgctcgtatcgcagctaaacacaatgcgactccggcacaagtgattctggcgtgggctatgggggaaggttactcagtaattccttcttctactaaacgtaaaaacctggaaagtaatcttaaggcacaaaatttacagcttgatgccgaagataaaaaagcgatcgccgcactggattgcaacgaccgcctggttagcccggaaggtctggctcctgaatgggattaagcctctctgacagctcctccgggagctgtttttacatgctcgctaaggaaatcgataaaagcccggatgcgcgtacttaccgcacggtcgctgtaatagacggcactgaatggcatttccactggcaacactttatctgccattaactccaccaattctccgcgagcgatttctttgtcgatcatgtagtcggacaaacacgcaatcccgttgccactcaggcaaagctgtttcagtgtttccccactattggatgacaaaccgtacttcacctcatgtaattgtccatcgctacgggctatcggccaggtattgagggaagcgggttcagtgaatcccaggcaaatatgttgctttaaatcgtcgatcgtttctggcttcccgtagcgggaaatataatcgggggaggcgataatttttcgataactgttaaataacggcctggcacgtaagctggaatccgttaacgtaccagcgcgtatcgcgacatccacttttctttcgatcaaattaataatcgtttcggaggagactagcgacaaagtgacttccggatagcgttcacggaaaggcttaattaacggcatcagaaagtgcagcaccactggagttgcggcatcgatccgtaacagtccacgcggtgtattacgcgtctccataatttctgattctgccgctgccatctcctgcaaaattgactgtacgcgacgaaaataacgctcgccttcttccgtcaggctaagttgtcgcgtggtccgattaagcaggctaacgccaagtttcatctccagctttttcaccgcccggcttaccgctgagtttgcttgccctaattgttccgctgcccggctaaagctgccgctttcgacgaccgaaacaaaaatggcgagttcttccgacgtggctttcatttttgctcctgttgcaaaatagaagagatattttgaatttatttgtcattaaaccatcaggatgcgtgatatgtcatgcgatttaatgttctccataatgagcaaaattctgaccggtgtaagcacttgcttacataacaatatacaattgctcgttgaaagagtgagctaaaatccctataacagtagaaccctcccgagtgcggaagggttgacgtaatagaggtttcaaagtcaaaagtgcgaaaaaacacctatgccatgcgctatgttgccggacaacctgcggaaaggatcttaccgccggggtcttttgcgagcatcggccaggcattaccacctggggaaccgttaagtaccgaagagcgtattcggatcctggtgtggaacatatacaaacagcaacgcgctgaatggttgtcggtattaaagaactacggcaaagatgcacatctggtgttattgcaggaagcgcagacaacgccagagttagtacagtttgcgaccgctaactatcttgccgccgatcaggtacccgctttcgtgctgccacaacatccttctggcgtaatgaccctttcggcggcacatccagtgtattgctgcccgttacgtgaacgagaacccattttgcgtctggcgaagtcggcactggtgacggtctatccattacctgacacccgcctgttgatggtggttaatatacacgccgtcaacttcagtctgggcgtggatgtctatagtaagcagttacttcctattggcgatcagatagctcaccacagcggcccggtcattatggcgggagatttcaatgcctggagccgtagaaggatgaacgcgttatatcgctttgcgcgggaaatgtcgctgcgccaggtgcgttttaccgatgatcagcgccgtcgggcgtttggtcgcccgctcgattttgttttctaccgtggtctgaacgtcagtgaagcttctgtactggttacgcgcgcttccgatcacaatccgctactcgttgaattcagtcccggcaagcctgataaataaggtatgtcaggtctgccacagggcagaccaacgtttggcgctgcgcaaaacgtgagcgcggtggtggcgtatgacttatctgcccacatgctggatgtcgtggcacaagctgccgaagcccggcaactgaaaaatatcaccacccgccagggatatgccgaaagtctgccatttgccgataacgcatttgatattgttatcagccgttattctgcccatcactggcatgatgttggtgcagcactgcgagaagtgaataggatattgaaacctggcggtaggctgattgtgatggacgtaatgtctccgggtcacccagtgcgcgacatctggttacagacggtagaagcattacgcgatacctctcacgtacgaaactacgccagcggtgagtggttgacgttaatcaatgaagccaatctgatagttgataatttaattacagataagttaccgctggaattttcttcatgggtcgcgagaatgcgtacgccagaagcgttagtagacgctattcgcatttaccaacagagcgcatcgacagaggtgagaacgtattttgccttgcagaatgatggctttttcaccagtgatatcatcatggtagatgcacataaagcggcataaataaaaaaggcaccgggggaatcggtgcctttttattatctggtttgtcaggaatctggcatgttgttgtttttcacaaacaacgtcagcttatcgcctggttgcagattcgcagtgtcgctgttccagcgcatcacatctttgatgttcacgccgtggcgtttagcaatgcttgaaagcgaatcgcctttgcgcacacgatacgtaatgctatcgctgttgtttgccagtcgctgtgcgctactgcctgcaccaatcgtcaaactttggcctggcttcagcttagatccgcgcagtttgttccactgctgcaaatctttggtgcttacgccgagacgtgaagcgatacttgaaagcgtgtcgccagagcgtacggtgtaaacacggctgttaagcggcgtattgtcggcaaccagcgtcgactgtacagcagcaatttcgcctgaagccagagattcacgcagttgatctgcatgcttctttggcaccatcacgtactgcgggccacttgcgcccagcgtggagccttttacgccagcgttgaatgtcttcagcttgctgacggaaatccccgccatatctgctaccttcgccatttcaaccgggctgctcaggtgcacacgcgccagagcacggctttcatcggtcgttggcagacgtacgccataacgcttgctgtttttgagaatatcactcaatgccagcattttaggcacgtactgcttcgtttcctgcggcaacggtaacgaccagaagtccgtggatttcccacgcgctttgttcgttttaattgccttcatgacccgaccttcgccgctgttataagccgctacggtcagaagccagtcgccgtcaaacattttgttcagacgctgcatcatattcagcgcggcagttgttgaagcaacaacatcgcgacgcgcgtcataattgcgggtctgtttcaaaccataattgcgccccgtgctcggaatgatctgccagatgcctgcggcattggcgccagacgttgcgtgaggatcaaaagcgctctccactatgggtagtagtaccagttccataggcatgttacgttttttaacttgccctgctatccagtacatatacggctctgcccgtaaagttacatcgtggagatagctcttattgcgtaaatatttctgtttctgttcgcgaatccggtcattttccggaattcccatctttagctcgtcgccaatgaaagcccacaagtcaccatctggcgcgatagacgtcccatcgtccatccatcgtgcctgacttgtaaactttgctgcttccccttgaccagctgcagaaaggctctgtgcgtgctgttgaacgttgccggtactctggcaacccacgagcaggacagaggcgagtaatatcgcttttgccttcatgtgtgtgtcaatagttgcttaaaagacgaccgatcataacggcgaacggagccgatgacaagaaagttttatcagaacctatctttctttgaccttaaccatgcaaaacgctcttcaggttgttgcaataatgtttcttcattaattacattaattaaatcaatatcttccgttcttaaaaaaacattaatttgccgctcatttttcagaattacgggtagtgttatttgattttttgcccgtaactccttaactttacgataataatcatttatggacaaatcgtgcggaagaatactcaaagcaaacttcatatttgataaggtatattcatgagcacaacataccaatgtatcgtcaggtaacgcacttaactttttaagtgattgatacatttgtgatgctgtcccttcaaacaaccgaccacacccaccagaaaacagtgtgtcgccgcaaaatagataaggtttactgaagtaacagatatgtcctaaagtgtgacccggcgtagcaattacactaaattcatgccccaaaacgaaggcagtttcgccatctttgactacctgtgttgttcccttatcttgtgtctcttgtggaccatacaccacaatttgtggaaacttttccaccagttcttttacgccgccaacgtgatcgtggtgatggtgggtgagaaatatggcctccggttgccagttattggcggcaatggcgtttaatactggctctgcgtctccgggatcgacaatcaggcagcgacctgcttcatcattcaaaacccagatgtaattgtcatcaaaggcgggaatactgttaagattcatagattacctctcagtgtgaaacggaaggttgtgatgaaaccggcaagagtccctcaaactgtcgtggctcctgattgctggggcgatttgccctggggaaagctttatcgcaaggcgctggagcgccagctcaacccgtggttcactaaaatgtatggttttcatctgcttaagattggcaatttaagcgcagaaatcaattgcgaagcgtgcgcggtttctcatcaagtgaatgtttctgcgcaaggaatgcccgtccaggtacaggcggacccacttcatcttccttttgccgataaatccgttgatgtttgtctactggcacatacattgccgtggtgcaccgatccgcatcgtttattgcgtgaagccgatcgggtattgattgatgatggctggctggtcattagtggcttcaatcccatcagttttatgggattacgcaaacttgtgccggtattgcgcaaaacctcgccctataacagccggatgtttactctgatgcggcagctggactggctctctttgttgaattttgaagtgctacacgccagccgtttccacgttctcccgtggaacaaacacggaggaaaactattgaatgcgcatattcctgcgcttggttgcttacaacttattgttgcccggaaacggactattcctttaacgctaaatccgatgaaacagagtaaaaacaagccacgaattcgccaggcggttggagccacccggcaatgtcgtaaaccacaggcttaaacttcaacttggtagcctgtatcttccagtgtgggattcatcgccgcggcacgagccagttcatcacagcgttcgttttccgggtgtccggcatggcctttaacccattcccatttgatttgatgctgccccaatgcagcatcaagacgttgccagagatcgacattttttactggttttttgtctgcggttttccagccacgttttttccagttatggatccactgggtgataccctggcggacatactggctgtcggtactcaaaatgacttcgcaatgttcttttaacgcctccagcgcgacaatagcggccatcaactccatacggttgttggtggtgcgggtgtagccagcgctaaaggttttctcgcgtccgcgatagcgtaaaatagcgccgtaacccccaggtcctggattgcccagacacgaaccatcggtgaaaatttctacctgtttaagcatctctggtagacttcctgtaattgaatcgaactgtaaaacgacaagtctgacataaatgaccgctatgagcactgcaattacacgccagatcgttctcgataccgaaaccaccggtatgaaccagattggtgcgcactatgaaggccacaagatcattgagattggtgccgttgaagtggtgaaccgtcgcctgacgggcaataacttccatgtttatctcaaacccgatcggctggtggatccggaagcctttggcgtacatggtattgccgatgaatttttgctcgataagcccacgtttgccgaagtagccgatgagttcatggactatattcgcggcgcggagttggtgatccataacgcagcgttcgatatcggctttatggactacgagttttcgttgcttaagcgcgatattccgaagaccaatactttctgtaaggtcaccgatagccttgcggtggcgaggaaaatgtttcccggtaagcgcaacagcctcgatgcgttatgtgctcgctacgaaatagataacagtaaacgaacgctgcacggggcattactcgatgcccagatccttgcggaagtttatctggcgatgaccggtggtcaaacgtcgatggcttttgcgatggaaggagagacacaacagcaacaaggtgaagcaacaattcagcgcattgtacgtcaggcaagtaagttacgcgttgtttttgcgacagatgaagagattgcagctcatgaagcccgtctcgatctggtgcagaagaaaggcggaagttgcctctggcgagcataaatacctgtgaaaggcgctaaaaatagcgacttgggcgatttttgcagcaaacgattcaaaagatgagaaaaaccgttgacgaaggtcgaggcaatccgtaatattcgcctcgttcccaacggaacacaacgcggagcggtagttcagtcggttagaatacctgcctgtcacgcagggggtcgcgggttcgagtcccgtccgttccgccactattcactcatgaaaatgagttcagagagccgcaagatttttaattttgcggtttttttgtatttgaattccaccatttctctgttcaatgattttactctggcgtaggtgcgtgattctcgcttgttgtctcattcattaaaattcaataatgatatcgaaccattcagcttaaatatatttctagagaataaatttatattgattaaatgaatgtatatttcaaattgattttgtttgttattatttaagtgaggtatataattagagtccgttatcaatgctaaatattctaatcattatgacaggcgagggagtgtccaattatgaattcaaaaaagctttgttgcatatgtgtgttattctcgctgcttgcaggatgtgcctctgaatcttctattgatgaaaagaagaaaaaagctcaagtcacacaaagtaatattaataaaaacactccccagcaactgacagacaaagatttattcggtaatgaaaccactctggccgtatccgaagaggatattcaagctgcgcttgatggagatgagttccgcgttccccttaattctcctgtaatacttgttcaatccggcaaccgcgcaccggaaaccattatgcaggaggagatgcgaaaatattatactgtttccacattctctggtatcccggacaggcaaaagcctctgacttgtaacaaaaacaaagataaaaatgagaacgaggatgttgccagtgctgagaatatgaactggatgcaggcactgcgttttgtggctgcaaaaggacatcagaaagcgattattgtttaccaggatatgttgcagacaggaaaatatgactctgcgctgaaatcaacagtatggtccgactataaaaatgacaaactcactgacgctatctccctgcgctacctggtacgtttcacgctggtggatgtggcaacaggtgagtgggctacctggtcgccggtgaattatgaatataaagtgcttccaccattgcccgacaagaatgaagccagtacgactgatatgacagagcagcaaatcatgcaacttaagcaaaagacctataaagcgatggtaaaagatttggttaaccgctatcaataataaattatatctgccgccaggaatttctggcggcaataatacaaaattctttgcataagaaatttttcttgacaaagacagtgcaagaaaggacatggaatccggagttaaaaactgtttgttttagaatatttaattatttaactgctgaatcttccttgcgagaaatatatccattattacatttcatgccatttttaatatagattgctcctgggaaaattcccgtattattaccgcaggggtgataattagtattgacatatcctgtgacaaaaggagctattaaaggtgctattacgatagctattagtaaaaatataagagttagctgtattgttatgtctgtggcgaaattgactaccttcgtttttttgattaagaatgattttattatcgtaagtaaaattacatgaatatttaaaaaggaaaacgacatgaaaccgaagcacagaatcaacattctccaatcataaaatatttccgtggagcattttattattgaatatagaggtttaactccggtaaaaaacaaagaagcattgaatgcagggaaaaataatatggccataaaaaacatcgaaagaaactcttttaatttaacatgtaaacgcatggttaatcctcatatcacgggtggagtgttaagaacatacataaatggagtcatgttttcccttttccatttatcaagttcctgttgccgttttagtccatctctaattgcatattttaatttttctgataaatggcattgagcatcgatttcatttaaaacaactgtacacactatccctgtcagtaaaattgctcctccgacaagaattactggaaagccaaagctaacacaggcaaaagaagccagacttccaatagcggttgcaacaccaccggctataactgctttggccacatccattgaaaaatcgccaagaaaattaaccagatctcgctctgaactcataataaattctatggttctgctgatttaaccgcagagaagttcgccacagcaatccgaaaccactggcacgtggagaataagctgcacaggcgtctggacgtggtaatgaatgaagacgactacaaaataagaagaggaaacgcagcagaattattttcagggatacggcacattgctattaatattttgacgaatgagaaggtattcaaggcagggttaagacgtaagatgcgaaaagcagccatggacagaaactacctggcgtcagtccttgcggggagcgggctttcgtagtaataccccgactctccccgtccttaaacacaacccccactcaccacaacctaaactcatccgcatcctgccatgccggaaacttttctctatattcccgcaatgctgccatcgacagctccgcatcaatgcgcgttgcctgatgcgcgtcggcagtagcgataatctctccttgcggattaatcacccggctgtcaccgcgataatggcagccgttgccatcgctgccgacgcgattgcatcccgccacatacgcctgattctcaatcgcgcgggccgtcagcaatgcctgccagtgcagagagcgcggagcaggccagttggcgacgtacagggcgaggtcataatcgttgagattgcgcgaccacacaggaaaacgtaagtcgtagcacaccagcggcaaaatacgccagccgcgccattccacaatcactcgcgcattgcccgctttataatgtagatgctcatctgccatgcggaacagatgacgcttatcataaaaatgtaccgtgccgcccggctcaaccagcaaaaagcggttaaccgaaccagactccgtttgtaatgcaacactgcctgcaatcagcgcattgcactgctgcgccttagctgtcatccagttcactacgtcatcttgtgctagcgacgaagctgccgcttccatggcaaagccgctggtaaacatctccggtagaacgatcacatcgcgcccggtaataccttccagttgacgatcaaaatgacgcaggttggcaggaccatccatccacaccagtggttgctgcaaaagcgtaatcttcaaaccaggcacggtgtacaactcctttatgcgaagggttttataactttaacaccttatcaggcagttgccttagcgcagaataaattgataacaaatgctgatattggaaatatctgatttgcaaattatcgtgttatcgccaggctttaggaggttaataacatgggcaggataagctcgggaggaatgatgtttaaggcaataacgacagtcgccgctctggtcatcgccaccagtgcaatggcgcaggatgatttaaccattagcagccttgcaaagggcgaaaccaccaaagctgcatttaatcagatggtacaagggcataagctgcctgcctgggtgatgaaaggcggtacttatactcccgcacaaaccgtaacgttgggagatgagacgtatcaggtgatgagcgcgtgcaaaccgcatgactgtggctcgcaacgtatcgctgtgatgtggtccgagaaatctaatcagatgacggggctgttctcgactattgatgagaaaacgtcgcaagagaaactcacctggctgaatgtgaacgatgcgctttcgattgatggtaaaacggtgttgttcgcggcgttgaccggcagcctggaaaaccatccggatggctttaattttaaataattagcggataaagaaacggagcctttcggctccgttattcatttacgcggcttcaactttccgcactttctccggcaactttaccggcttcgtcgccagctcttccggatcaaagtcatcaacgttaatactgcgcagacggctttcttcagctttcaccagaatagcggcttcatctttatcaatcagccccttcaccagcgcgttgtgcgccagttcatccagacgggtaaacggcaggtttttacccagctctttacagatccgctgatgaattgggtcggcggcaatcacatccaccagcgcctcttccagcaagccaaccggattatgctcgctcggcgtcaggtactgaccgcgaccaatgcgggaacgggtggcgttcggcacttgtaaaatcttcgccactttatgatccagcttgtcagaaggtgccagataatgacgtccggtcgggaagatcaccacattcagcagcccggcaaccacgcggttcgggaagttttgcagtaaatcatccatcgcctgttcagcctgatacagcgcatcttgtacgccccagtgcaccagcggcaggtcggcttcattacggccttcgtcgtcataacgcttcagcacggcagaggcgaggtagagctggcttaaaatatcccccagacgggccgagatgcgctcgcgacgtttcaggctgccgcccagcactgccatcgagacatcagaaagcagggcgaggttggcgctcaggcggttcaggtgctgatagtagcgtttagtggcatcgccggttggcgtgctgctggttaaaccgcgcgtcaggcccagccagaagctgcgaactttgttgctaccgacgtgaccgatatgtttgaacaacagtttatcgaacgcgttgacgtcattgttcttcgccgcttccatctcttccagcacgtacggatggcaacgaatcgctccttgtccgaagatcatcatgctgcgggtcagaatgttagccccttcaacggtgatggcaatcggtgcgccctggtaagcacgcgccaggaagttgctttgcccgagcataatgcctttaccgccggtaatatccatcgcatcaataatcgactgctgcccgcggtgggtacagtgatacttaacgatagccgacagcacggcaggtttttcgccgagcataatgccgtaggtaatcagcgatgccgcagcatccatcacgtaggcattaccggcaatacgcgccagcggctcttcaatcccttccatcttaccaatagagattttgaactgacggcgaatgtgagcatacgcgccggttgccagcgctaccgatttcacgccgccggttgagttggaaggcagggtgatgccgcggcctaccgagaggcactccaccagcatccgccagccttgcccggccattttcggcccgccgatgatgtaatcgatcggcacgaagacatctttaccgcgcgtcggtccgttctggaacggtacgttcagcgggaagtggcgacgaccaatttccacgcccggcgtggtggttgggatcagcgcacaggtaatgcctaaatcttctgcaccgccgagtaatttttccgggtcggagagtttaaacgccagcccaagcacggtcgcaatcggtgccagcgtaatgtagcgtttgttccaggtcagacgcatccccagcacctgctggccctgccattcgcccatgcagacaatcccggtgtccggaatcgcgcccgcatcggaacccgcttccgggctggtcagtgcaaagcaggggatctcctgaccacgcgccagacgcggcagatagtgatctttctgctcgtcagtgccgtaatgttgcaacagttcgcccgggcctaatgagtttggcacgccgacggtaatcgccaggatcccgctcacgccggagagtttttgcagcacgcgagactgggcataagccgagaactccagcccgccgtactcttttttgatgatcatcgcgaagaaacgatgctctttaaggtacgcccacaactccggcggcagatccgccagctcatgggtgatctggaaatcattcgccatccggcaggcttcttctaccgggccgtcgagaaacgcttgctcttcggcggtcaggcgcggctgcggatagttatgcagctttttccagtccggcttgccctggaacaagtcgccctcccaccaggtggtgcccgcatcaatcgcttctttctcagtgcgcgacatcggcggcatcaccttacggaaaccgcgaaataccggcgcggaaatcatcgacttacgcataggcgcaaagttaaatggcacgaggataatggccagaggcaccagtacccacgccgaccacagaccagcaacgccgagggcggctgtccaggcgagcaaaatcagactgctgataaataagctcacgcggtgatagaacaacgcgccgagcaggacaaccgtagcgagaatactcaaaatcatcataacgaaaagccccttacttgtaggaggtctgaccacttgtgatgatatggttgtagtggatgtaaaaacatttagcaatatgtttacaatataattacaacaaagctcacattgttgctgtttttatccgcacttcaggtcaaaaagtcctggtcatagcacctgcccgtacttctcgcttttggcggtatccggtacactgcattttgtctattacatttatgctgaaggatatcctcatgtaccaggatcttattcgtaacgaactgaacgaagcggcggaaacgctggctaactttttaaaagatgacgccaatattcacgccattcagcgcgcggcggtcctgttagcagacagctttaaagccggtggcaaagtgctttcctgcggcaacggcggttcccattgcgacgctatgcactttgccgaagagttgaccggtcgctaccgtgaaaaccgtccgggctacccggcgattgctatttctgacgttagtcatatttcctgcgtcggtaatgatttcggtttcaatgatattttctcccgctacgttgaagcggtaggtcgcgaaggcgatgtactgctggggatctccacctccggtaactctgcaaacgtgatcaaagcgatcgcagcggcgcgtgagaagggaatgaaagtgatcaccctgaccggtaaagacggcggcaaaatggctggcacggcggatatcgaaattcgcgtaccgcactttggttatgccgaccgcattcaggagattcacattaaagtgatccatatcctgatccagttgattgaaaaagagatggttaagtaagtctggcgtaggccggataagacgtttacgccgcatccggcatttgtgcgctgatgcctgatgcgacgctgacgcgtcttatcatgcctacaaatctgtacgcgaaccgtaggccgaataatgcgttcacgccgcatccgacctgaaaattcttaaatcaatcttcgccgggggccatgcgctcccgctgttgtggaggttacccatgtgcgaattgctcgggatgagcgccaacgtccctaccgatatctgctttagtttcaccgggcttgtacagcgtggtggtggaaccgggccacataaagatggctggggcattaccttttacgaaggtaaaggctgtcgcacatttaaagatccacaacccagctttaattcccccatcgccaaacttgtccaggactacccgataaaatcctgttcggtggtggctcatattcgccaggctaatcggggcgaggtggcgctggaaaatactcacccatttacccgcgagttatgggggcgtaactggacttatgcccataacggacaactgacgggctacaaatcactggaaaccggcaacttccgcccggtaggcgaaaccgacagcgaaaaagccttctgctggctcctgcataaattaacgcagcgttacccgcgcacaccgggcaacatggcggcggtatttaaatatatcgcctcactggcggatgaactgcggcagaagggcgttttcaacatgctgctttcggacgggcgctatgtaatggcgtattgctcgactaatttacactggatcacccgccgcgcgccgtttggcgtggcaacgttgctggatcaggatgtggaaatcgacttcagctcgcagaccacaccgaatgatgtggtcacggtgattgcaacacagccgctgacgggcaatgaaacctggcaaaagattatgccaggcgaatggcgcttattttgcctcggggagcgtgtagtttgatgccagttgtggctgcacaacttcgtggcttaacggcttgctgaccacgtaacgaccattgaccacagaaacggttggtggcttacgggtttgctcaaagtagtcgtaacccggcttcagttgctcccagaagtccttaaagttggaatatttatggcgcttcatattggcgtcggtcatgcggaacgggtaaatactcacttgcacgctcggctgaccaaacaccagcgcaccagtaacgaactggaatatctcatcaataccctgattggtcattgcgtagcagccgatggaaacacaatcgccgtggatcatcaggtatttcccttcataaccatgcgcacggtcataggcattggggaaaccaatattaatcgctttgtagtaacggctgtctggttttaactgattacgctggacgctataaaacccttccgggcttttgaaatcgccctgacgctgttttggccctaagccgccggaatatttacagattttatagctgtcgagcagttgatattgctcgcccattttgacgtagagatcgagcgtacgttcttccttgaagatctggatgtagacaggggatcccatcaactgctgcttatactctttgctcacaggcgtggtagagctactgctgcccagcaaaccggcaaatgaaacgcacgggatcaacaacatcgcaagaattaatgcgattttacgcatactgcttattccttgataaaacggttacacacgccaggacggcaaaatggatcccaaatcggaatagtctggatttggaaggctcacattatcaccaaaagagttttacgcaagcctgtcggcgcagggtttacaaatttcatcggaagcgggctttacccaaagagcgccgcgtgagttccagttctctcaaatcgtaaaagtttatcggtaagtttgtaaatcaggatccagtccggttcgacatgagcatcgcgataacctttccatgaaccttgcagcgggtggtctttataaacagctggaagcggtaaagtattattgataagaagcgtcataagatatttcaatttattcatatccttatgacgcttttgtgcaagttttacatcctttgaatattgtcccgagtattcaatatccctttgaatcatatttaaattcctaatttatcaaataaatcatcggcgtctttggccttatgaacatcaatgccagcttcgctgtttttgattgattgaatggttaattgattaggctcgcgtaaatcaaacggcaatgccttttcacgcgcgacctttgtgagggttatgcgaaccaggtcagagatggtcagccccatcccggccagtacgtccgctgcctgattcttcagatcttcatcgattcgggcgcgaacaaacgcgttagcagccattggggtatctcctgtgctgtatatttattcagcttgaattgtagctcaaatgagcaacagcgacaatccatgagtaatttaataaacggatgtttttacataattaactgaaatatatatgttaattttataataatggtttattaagtttgttcagaaacgatccgggatacactgcaacattaaagcatgaccagccattattgagtatgtccttgccgtcgattccatcctttgtattgtcgggattactgttgatttgtttgccgttttcttcatttgccagcgccaccacatcacatatctctttcagctacgccgcccgccagcggatgcaaaaccgtgcgcgtttattaaaacagtaccaaactcatctgaaaaagcaggccagctatattgtggaaggcaatgccgaaagcaaaagggcgctacgccagcacaaccgggagcagataaaacagcatccagaatggtttcctgctccgctcaaggcgagtgacagacgctggcaggcgctggcggaaaacaaccactttttaagcagcgaccatctgcataacattaccgaagtggcgattcaccgcctggagcagcagcttggcaagccttacgtctggggcggtacgcggcctgataaaggctttgactgtagcgggttggttttttatgcctacaacaagatccttgaggctaagctcccgcgcacggccaatgagatgtaccactatcgccgggcaacgattgtggcgaacaacgacctgcgccggggagatttgctgtttttccatatccacagccgcgagatagccgatcatatgggcgtgtatttgggcgatgggcaatttatcgagtcgccacgtaccggcgaaaccattcggataagccgattagccgaacctttctggcaggaccattttttgggcgcgcgcaggattttgacggaagagacgattttgtaggacggataaggcgtttacgccgcatccggcagttgtacgcaggtgcctgatgcgacgctggcgcgtcttatcatgcctacgagcccgcgaatatttgcgagccgctttcccgatataaaacaacctcattgccaacctttccttttcttcttaccgttgagaaaaaggagtcgccatgtctgaatatcgtcgttattacatcaaggggggaacatggtttttcacggtgaatttacgaaatcgtcgaagccaacttttgaccacccagtaccagatgctccgtcacgccattattaaagttaagcgagacaggccttttgaaatcaacgcctgggtcgttttgccagagcatatgcactgtatctggacattacctgaaggcgatgatgatttttcctcgcgctggcgggaaattaaaaagcaatttacccatgcttgtggattgaaaaatatctggcaaccacgtttttgggagcacgccatccgcaataccaaagattataggcatcatgttgattatatttatataaatccagtaaagcatggttgggtaaagcaagtgagtgattggccattctcaacgttccatcgcgatgtcgcgcgagggttatatcccatcgattgggcgggggacgtaacggattttagtgccggggagcgtatcatttcataattgtgcgcagatgcctgatgcgacgctagcgcgtcttatcatgcctacaaacttgtgccggatcggtaggccggataaggcgtttatgccgcatccggcagttatgcgcagatgcctgatgcgacgctggcgcgtcttatcatgcctacaaacttgtgcctgaacggtaggacggataaggcgttcacgccgcatccggcagttgtgcaccaatgctggatacttacatcaacgcccccataatcttcaactccagctcatccggcacttcgttatacgacagcacatgcagccccggcgcaaacaaccttgcataacgcgccagcaaagggcgcagctgcggtggcaccagcagcaccgggtctttccccgccgctttcatctgctctttcacctgtggcatcgtactctggaactggttgagcatattcggatcgaccggcacgctgtcgagcatcactttcccgccctgttgcgcctgattcaccacgttggtcagcagattttccagctcattattcagcgtatacaccgtcagctcctgcttgcgaacgaacggatgggtaatgctgcgccgcaatgccaggcgcacatcggccgccagcagaatatgatctttcgtcaccgtgctactggcgaccagcacggtggcgatggtgacgatatcgcgcagggaaacgccttcggtcagcagcgcccggtacactttcagcaactggctgtaattgagcgccgcgctcaaatcttccgccagacgcggtgccgtcgacgataaacggttatgcaactgcgtaatatcatcatagttaaacaaatcaggaatatagctgcgcacaatcttatttacatgggtagcgatcacgctggcgctgtcgatcacctgataccccatattcagcgccttcgctttctgcgccgcctggatccaggtgaccggcatcccgtacgccgggtcgttcccctgcacgccgtcaatctcgccgtaggtttcgctggagggcagggccatcagtttatccgccggaatatccgcttcatcagcctttatgccgttgatgaaaatggcgtactgactgggcttaaggcggaagttttcccgaatgcggatctccggcagcagcacgccgttgccgtcagaaatcacctgccgcacgccgcgaatccgctgggtgagcgggttaccctgtgctttgtccaccagcgccaccagtttgtaaccgaggcttaaactgataggctcgatcagcggaatggtttcccaactgacctgctgctcgctggtttcggtgatggtgcgggtcagcgtttcgaggcttttctcttccgcctccgccgccagcggctgtttgctcatccgccagccggtaaaaccaagcagggcgctgaacagcaaaaacggcaggtgcggcattcccggtaccaccgccagcacgaacataatcccggtggcggtgtagagcaccgacgggcttgccagcagctggttacgcacgtcatgggcgatatcgccgttgtcgctgacgcgggtgacgataatcgccgccgcggtggagagcagcagggaagggatctgcgccaccaggccgtcgccgatggtcatcagcacatactgctggaaggcagcatcggcgctcaggttgtatttgaagatcccgatacagacgccgccgatcaggttgatcgccagaatcatcatcccggcgatggcgtccccgcgcacaaacttcgatgccccgtccatcgcgccgtagaaatcggcctcgctggcaacatctttacgccgggtttgcgcctgcgcctggttgatcaatccggcgttaagatcggcgtcaatcgccatctgtttgccgggcatcgcgtctaaggtaaagcgggcagaaacctcggaaatacgctcggcccctttggtgacgacaataaagttgattgtcaacagcgtcagtaaatccgagcgtgaaagcattatcgccgcgctgcacgggcagtcgatttttaacggtggtgggctgtcgccgttaaataaaatcagcccgtctcatccgccaaaacctgccaccgtggcggtgccggaagagacggagaaaaaagcgcgtgatgtgaatgagaaaacggcgctgctgaagaagaaatccgccaccgagcttggtgagctggcaaccagtatcaacaccattgcccgtgatgcgcatatggaagcgaatctggagatggagattgttccccagggattacgcgtgctgattaaagacgaccagaaccgcaatatgtttgaacgcggcagcgcgaagattatgccgttctttaaaacgctgctggtggagctcgcgccagtgttcgactcgctcgataataaaattattattaccgggcataccgatgcgatggcctacaaaaacaatatctacaacaactggaacctttcgggtgaccgcgcgctttcggctcgtcgggtgctggaagaggccggaatgccggaagataaagtgatgcaggtaagcgcaatggcggaccagatgctgctggattccaaaaatccgcaaagcgcgggcaaccggcgcattgagattatggtgctgaccaaaagtgcgtccgatacgctgtatcaatactttggtcagcatggggataaagtggtgcagccgctggtgcaaaagctggataagcagcaggtgctttcgcagcgaacgcgttaaatgctgaatctttacgcatttctcaaaccctgaaatcactgtatactttaccagtgttgagaggtgagcaatgcgtaaaatcattcatgtggatatggactgctttttcgccgcagtggagatgcgcgacaatcccgccctgcgcgatatccctattgctattggcggcagccgcgaacgtcggggggtgatcagcaccgccaattatcccgcgcgtaaatttggcgtacgtagcgctatgccgacagggatggcgctcaaattatgcccacatctcaccttgcttccggggcgctttgacgcctacaaagaagcctcaaatcatatccgtgaaatcttctcgcgctacacctcgcgcattgaaccgttgtcactggatgaggcttatctcgatgtcaccgatagcgtccattgccacggttctgcgaccctcatcgcccaggaaatccgccagacaatcttcaacgagctgcaactgacggcgtctgcgggcgtggcaccagtaaagtttctcgccaaaatcgcctccgacatgaataaacccaacggccagtttgtgattacgccggcagaagttccggcatttttacaaaccttaccgctggcaaaaatccccggcgtcggcaaagtctcagcggcaaaactggaagcgatggggctgcggacctgcggtgatgtacaaaagtgtgatctggtgatgctgcttaaacgctttggcaaatttggccgcattttgtgggagcgtagtcaggggattgacgaacgcgatgttaacagcgaacggttgcgaaaatccgtcggcgtggaacgcacgatggcggaagatattcatcactggtctgaatgtgaagcgattatcgagcggctgtatccggaacttgaacgccgtctggcaaaggtaaaacctgatttactgattgctcgccagggggtgaaattaaagttcgacgattttcagcaaaccacccaggagcacgtctggccgcggctgaataaagctgatctaatcgccaccgcgcgtaaaacctgggatgaacgccgcggcgggcgcggtgtgcgtctggtggggctgcatgtgacgttgcttgacccgcaaatggaaagacaactggtgctgggattatgatgtatactattatgtatattctggtgtgcattattatgagggtatcactgtatgcatcgaattctcgctgaaaaatcggtcaatatcactgagttacgtaaaaacccagctaaatactttattgatcaaccggttgcggttctttctaataatcgccccgcaggatatctcttaagtgccagcgcattcgaagcgttaatggacatgcttgctgaacaagaggagaaaaagcccataaaggcgcgcttccgtccaagtgctgcaagattagaggaaattacacgccgcgctgaacaatatcttaatgatatgacggatgatgatttcaatgactttaaggaataaggatgcgggtattcaaaacaaaacttattcgcctgcaacttacagcagaggaacttgatgcgttaacggcggattttatttcctataagcgtgacggtgttttgccagatatatttggtcgcgatgcactctacgacgactcctttacctggccattaatcaaatttgagcgagttgctcatattcatctggcaaatgagaataatccatttccgccacagttgcgccaattcagcagaacgaatgacgaagcgcatttggtatattgtcagggggcgtttgatgagcaagcatggttgctcattgccattctgaaacctgaacctcataaactggctcgagataacaaccaaatgcataaaattgggaaaatggcagaagcgtttcgcatgcgtttttgaatttatattatgaataacatacaaataagaaactatcagcctggcgattttcagcaactatgcgctattttcattagagcggttacgatgaccgccagtcagcattattcaccacaacaaatttccgcctgggcgcagattgacgaatctcgctggaaggagaaactcgcgaaatcacaagtgtgggttgcgatcattaatgcacaaccggttggttttatttcccgcattgaacattatatcgatatgttatttgttgaccctgaatacacccgccgtggggttgccagcgctttgttaaaacctttgattaagtctgaatccgaacttacggtggacgcaagcataaccgcaaaacccttttttgaacgttatggttttcagacagttaagcagcagcgcgttgaatgccggggagcgtggtttactaatttttatatgcgatataaaccgcaacattaaatccagcttgcaatgaaaataacgcccgcctggtatgtgcgcgttttctgattccacaaactgcaaggaggtaaatcatgacaaatcctttatcaatgactctttgcagacctttccaggattaattctttttttcttgccctggattcgtctgccatttcctgatttttatatttatatactctaaataattcgagttgcaggaaggcgacaagcgagtgaatcgccaggagcttacataagtaagtgactggggtgaacgaacgcagtcgcagtacatgcaacttgaagtatgacgagtataaatggaatggtacatgggcaaatatattcgtcccttatccgatgcggtatttaccatcgcatctgatgacctgtggatcgagagtttagcgatccaacaattacacaccacggcaaatttacccaacatgcagcgcgtagtggggatgccagatttacaccccggacgcggctacccgattggcgcagcgttcttctctgttggtcgtttttacccggcaagacgtcgcggtaacggtgctggaaacagaaacgggccgctactctgacacactgcgttcggcgctggtttctctcgatggcgataacgcatgggcattaagcgaaagctggtgtggcactattcagtggatttgtccgagtccgtatcggcctcatcatgggcgcaaaaactggtttctgggcattgggcgttttaccgctgatgagcaggaacaatcggatgcaatccgttatgagacgctgcgttcgtcggggccgggcggtcaacatgtcaataaaaccgactcggcggtacgcgccacgcatttggcatccggtattagcgtgaaggttcagtcagagcgtagtcagcatgctaacaagcggctggcacgattgctgattgcctggaagctggagcaacagcaacaggaaaatagcgcggcgctgaaatcgcagcggcgaatgttccatcaccagattgaacgtggcaacccgcgacggacatttacagggatggcttttatcgaaggataatgaaggatgaaactgccggaaggcgattaaacgccatccggcagcaaatcaaataattacttcgccggaatttctttcagcagttcagtcagcagtgtccagtaatgacctacgctttcgatgtgaacttgctcatccggagagtgtggaccggtgatagttggcccgatagaaaccatgtccatttccggatacggttttttgaacagaccacattccaggcccgcgtggataatctggatgttcggcgtcttgttgaacaggcgctgataggtttcacgtaccagatgcatcaccggagaattagcgtccggctgccagccaggatatgcgcctttcgcttcggttttcgcgccagccagtttacccagcgaatccagcatgctcaccacgtagtctttaccgctgtcgatcagtgaacggatcaggcagtgaatttctacgttattgtcagtcatggtcaccacaccgacgttcagggaggtttcaaccacacctttggctacatcggagttacgaatcacaccgttcggggtggcgttcagcagacgaataaaggtatcgcgagatttcgcaatcagggcagctttatcgttcgctacagagtccagcaacaaggccagatttttctctttttctgccagctcgtttttcaggatctcctgataggtattcaccagagatttcaggacgtcgactttatcagctgcgacagcaatggtcgcaaaggcttcacgcgggatggcgttacgcagtgtgccgccgttgaaatcgataaggcgcagatccagttcttccgcatgacccgccaggaagcgcaccagcagtttgttggcattacccagcccaacgtggatttccccgccggagtgaccgcctttcagaccttttaaggttaacttgaaggtttcaaaaccagctggaaccgcttcacgatctaaatgcaggttggaggtgaagtcgataccccccgcacaacccatgtagatttcaccttcttcttcggagtcggtgttaatcagaatatcagcctgcaaccagttgccctgtaagccgaacgcaccgtccataccggcttcttcggtcatggtcagcagcacttccagcgggccgtgaaccacgttttcgtcagccagaaccgccagcgcagaggccataccaatgccgttatccgcacccagcgtggtgccgcgcgctttaacccattcgccatcaatataaggctggataggatctttcgtgaagtcatgcacggtgtcgttatttttctgcggcaccatatcgaggtgggcctgtaagacgaccggtttacgattttccatacctgcggtagcaggtttacgaatcaggatattacctacctgatcgcgttcgacatggaaacctttctcttttgcccaaccaacaatgtattcagcgagttgctcttcatgataggacgggtgaggaatagaacagattttggcaaaaatatcccacagcggctgtggagataattgagacagttcagacacgttaagtctccttgtcgatcacccgcaaaacagtattgcaggtcacagggttagcagaaaatgttgtcaacacaagacaggcttgcgagatatgtttgagaataccactttatcccgcgtcagggagaggcagtgcgtaaaaagacgcggactcatgtgaaatactggtttttagtgcgccagatctctataatctcgcgcaacctattttcccctcgaacactttttaagccgtagataaacaggctgggacacttcacatgagcgaaaaatacatcgtcacctgggacatgttgcagatccatgcacgtaaactcgcaagccgactgatgccttctgaacaatggaaaggcattattgccgtaagccgtggcggtctggtaccgggtgcgttactggcgcgtgaactgggtattcgtcatgtcgataccgtttgtatttccagctacgatcacgacaaccagcgcgagcttaaagtgctgaaacgcgcagaaggcgatggcgaaggcttcatcgttattgatgacctggtggataccggtggtactgcggttgcgattcgtgaaatgtatccaaaagcgcactttgtcaccatcttcgcaaaaccggctggtcgtccgctggttgatgactatgttgttgatatcccgcaagatacctggattgaacagccgtgggatatgggcgtcgtattcgtcccgccaatctccggtcgctaatcttttcaacgcctggcactgccgggcgttgttctttttaacttcaggcgggttacaatagtttccagtaagtattctggaggctgcatccatgacacaggcaaacctgagcgaaaccctgttcaaaccccgctttaaacatcctgaaacctcgacgctagtccgccgctttaatcacggcgcacaaccgcctgtgcagtcggcccttgatggtaaaaccatccctcactggtatcgcatgattaaccgtctgatgtggatctggcgcggcattgacccacgcgaaatcctcgacgtccaggcacgtattgtgatgagcgatgccgaacgtaccgacgatgatttatacgatacggtgattggctaccgtggcggcaactggatttatgagtgggccacccaggcgatggtgtggcaacaaaaagcctgtgcggaagacgatccgcaactcagtggtcgtcactggctgcatgcggctacgttgtacaacattgccgcctatcctcatctgaaaggagatgacctggccgagcaagcgcaggctttgtcaaaccgcgcctatgaagaggccgctcagcgtctaccgggcacgatgcggcagatggagtttaccgtacccggcggtgcgcccatcaccggctttttgcatatgccgaaaggcgatggcccgttcccgacggtattaatgtgtggtggtctggatgcgatgcagacggactattacagcctgtatgaacgttattttgcgccgcgcggcattgcgatgctgactattgatatgccgtcggtgggcttttcttcaaaatggaagctcacccaggactccagcctgttgcatcagcacgtcttaaaggcgctgcctaacgtaccgtgggtggatcacactcgcgtcgcggcctttggtttccgtttcggcgctaacgttgccgtgcgtctggcataccttgaatcgccgcgtctgaaagcggttgcctgtcttggtccggtagttcataccctgttgagtgattttaagtgccagcaacaggtgccggaaatgtatcttgacgttctggccagtcgtttggggatgcatgatgcttccgatgaagcgttgcgcgtggagctgaatcgctattcattaaaagtgcaaggattgctgggacgtcgctgcccaacgccaatgttatcaggctactggaagaacgatccgttcagcccggaagaggactcacgcttaatcacctcatcatctgctgacggtaaattattagagatcccatttaacccggtgtatcggaattttgacaaaggtcttcaggaaatcaccgactggatcgaaaaacgcttgtgttaaaaatttgctaaattttgccaatttggtaaaacagttgcatcacaacaggagatagcaatgacgttaccgagtggacacccgaagagcagattgatcaaaaaatttaccgcactaggcccgtatattcgtgaaggtaggtaatgactccaacttattgatagtgttttatgttcagataatgcccgatgactttgtcatgcagctccaccgattttgagaacgacagcgacttccgtcccagccgtgccaggtgctgcctcagattcaggttatgccgctcaattcgctgcgtatatcgcttgctgattacgtgcagctttcccttcaggcgggattcatacagcggccagccatccgtcatccatatcaccacgtcaaagggtgacagcaggctcataagacgccccagcgtcgccatagtgcgttcaccgaatacgtgcgcaacaaccgtcttccggagactgtcatacgcgtaaaacagccagcgctggcgcgatttagccccgacatagccccactgttcgtccatttccgcgcagacgatgacgtcactgcccggctgtatgcgcgaggttaccgactgcggcctgagttttttaagtgacgtaaaatcgtgttgaggccaacgcccataatgcgggctgttgcccggcatccaacgccattcatggccatatcaatgattttctggtgcgtaccgggttgagaagcggtgtaagtgaactgcagttgccatgttttacggcagtgagagcagagatagcgctgatgtccggcggtgcttttgccgttacgcaccaccccgtcagtagctgaacaggagggacagctgatagaaacagaagccactggagcacctcaaaaacaccatcatacactaaatcagtaagttggcagcatcacctgaaggtaagtgcaaagataatcgattctttttcgattgtctggctgtatgcgtcaacgtgaaaccggcaccggaagtgcgtgaattctggggctggtggatggagctggaagcgcaggaatcccgttttacctacagttaccagtttggtctgttcgataaagcaggcgactggaagagtgttccggtaaaagacactgaagtggttgaacgactggagcacaccctgcgtgagtttcacgagaagctgcgtgaactgctgacgacgctgaatctgaagctggaaccggcggatgattttcgtgacgagccggtgaagttaacggcgtgagtgaaatgtgccggatgcatcacatccggcaatattcattaaaactgatacgtcatgccaaccgcgacaatatcatcattattaatattcaatttgttatcgctatccagttggttgattttataatcaacaaacgctgacatatttttgttgaaataatacgtagcaccgacgtcgatataattgaccagatcttcatcaccgataccttcaatatctttccctttcgataagacataacccagcgatggacgcagaccaaagtcaaactggtattgagcgaccgcttcaaagttctgtgtcttattggcaaagccgccagttattggcgtcattttgcgtgtttcagaatagaaagttgccagataaatattattggcatcgtatttcagacctgttgcccatgcttctgcacgcttgcctgtgccacggctttgcaggttctgctcgttggtgcgatctgagttggtataggccccactaatggcgaaatcgctgccgccaaagtcatatgtcaatgacgtgccgaagccatcgccgttttgctttttaacgtcgcggttttcgtttttcccttgatattgcagggttaagttcaggccatcgataacgccgaagaagtcggtgttccgatacgtcgccagaccgctggcgcgtttggtcataaagttgtcggtctgcgccgaggaatcgccaccaaattccgggaacatatcggtccaggcttccacgtcatacaacgcccccaggttacgaccataatcgaaagaacccaaatctttatatttcaacccggcaaaagcgagacgcgttttttgctgtgcagtatcactctctgctttattaccggcaaactctgcttcccaacgaccataaccagtcagttgatcgttaatttgtgtttcgcctttgaaaccaaaacggatataactctggtcgccatctttactggcgttatcactcatataatgcatggctttaactttgccatagacatccagtttattaccgtctttattatatatttctgcagcctgtacagatgcagatgccacaatgcccatcaccactaatgccagagtgctctttttcattttcattcctgattttaattaacgcgcgaatattcagcgggagagtcccgttgaaaacaggaaagtttttaacctgagattgttaaagatatattacagattaataatattcttaaaatgtggtaatttattaaatctgtaataaaagcgtaaacaactgccgctaggcttgctgatcccgcgcaacaaaacgccatgctttgctcgcagatggttggcaaccgacgacagtcctgctaaaacgttcgtttgatatcatttttcctaaaattgaatggcagagaatcatgagtgacagccagacgctggtggtaaaactcggcaccagtgtgctaacaggcggatcgcgccgtctgaaccgtgcccatatcgttgaacttgttcgccagtgcgcgcagttacatgccgccgggcatcggattgttattgtgacgtcgggcgcgatcgccgccggacgtgagcacctgggttacccggaactgccagcgaccatcgcctcgaaacaactgctggcggcggtagggcagagtcgactgattcaactgtgggaacagctgttttcgatttatggcattcacgtcgggcaaatgctgctgacccgtgctgatatggaagaccgtgaacgcttcctgaacgcccgcgacaccctgcgagcgttgctcgataacaatatcgttccggtaatcaatgagaacgatgctgtcgctacggcagagattaaggtcggcgataacgataacctttctgcgctggcggcgattcttgcgggtgccgataaactgttgctgctgaccgatcaaaaaggtttgtataccgctgacccgcgcagcaatccgcaggcagaactgattaaagatgtttacggcattgatgacgcactgcgcgcgattgccggtgacagcgtttcaggcctcggaactggcggcatgagtaccaaattgcaggccgctgacgtggcttgccgtgcgggtatcgacaccattattgccgcgggcagcaagccgggcgttattggtgatgtgatggaaggcatttccgtcggtacgctgttccatgcccaggcgactccgcttgaaaaccgtaaacgctggattttcggtgcgccgccggcgggtgaaatcacggtagatgaaggggcaactgccgccattctggaacgcggcagctccctgttgccgaaaggcattaaaagcgtgactggcaatttctcgcgtggtgaagtcatccgcatttgcaacctcgaaggccgcgatatcgcccacggcgtcagtcgttacaacagcgatgcattacgccgtattgccggacaccactcgcaagaaattgatgcaatactgggatatgaatacggcccggttgccgttcaccgtgatgacatgattacccgttaaggagcaggctgatgctggaacaaatgggcattgccgcgaagcaagcctcgtataaattagcgcaactctccagccgcgaaaaaaatcgcgtgctggaaaaaatcgccgatgaactggaagcacaaagcgaaatcatcctcaacgctaacgcccaggatgttgctgacgcgcgagccaatggccttagcgaagcgatgcttgaccgtctggcactgacgcccgcacggctgaaaggcattgccgacgatgtacgtcaggtgtgcaacctcgccgatccggtggggcaggtaatcgatggcggcgtactggacagcggcctgcgtcttgagcgtcgtcgcgtaccgctgggggttattggcgtgatttatgaagcgcgcccgaacgtgacggttgatgtcgcttcgctgtgcctgaaaaccggtaatgcggtgatcctgcgcggtggcaaagaaacgtgtcgcactaacgctgcaacggtggcggtgattcaggacgccctgaaatcctgcggcttaccggcgggtgccgtgcaggcgattgataatcctgaccgtgcgctggtcagtgaaatgctgcgtatggataaatacatcgacatgctgatcccgcgtggtggcgctggtttgcataaactgtgccgtgaacagtcgacaatcccggtgatcacaggtggtataggcgtatgccatatttacgttgatgaaagtgtagagatcgctgaagcattaaaagtgatcgtcaacgcgaaaactcagcgtccgagcacatgtaatacggttgaaacgttgctggtgaataaaaacatcgccgatagcttcctgcccgcattaagcaaacaaatggcggaaagcggcgtgacattacacgcagatgcagctgcactggcgcagttgcaggcaggccctgcgaaggtggttgctgttaaagccgaagagtatgacgatgagtttctgtcattagatttgaacgtcaaaatcgtcagcgatcttgacgatgccatcgcccatattcgtgaacacggcacacaacactccgatgcgatcctgacccgcgatatgcgcaacgcccagcgttttgttaacgaagtggattcgtccgctgtttacgttaacgcctctacgcgttttaccgacggcggccagtttggtctgggtgcggaagtggcggtaagcacacaaaaactccacgcgcgtggcccaatggggctggaagcactgaccacttacaagtggatcggcattggtgattacaccattcgtgcgtaaataaaaccgggtgatgcaaaagtagccatttgattcacaaggccattgacgcatcgcccggttagttttaaccttgtccaccgtgattcacgttcgtgaacatgtcctttcagggccgatatagctcagttggtagagcagcgcattcgtaatgcgaaggtcgtaggttcgactcctattatcggcaccattaaaatcaaattgttacgtaagatcttatcattctcccaccaaaaaattatcttaatgtaacagctggtgtaagtaaattctatcaacgaagatcaatcttatctactgaccaaaaaggcctgatagggcttcgctcactatacatccttggctgcaggtttagttgtacaccactcctaaatttaatgtgttggcaatgtgttcaataaagctcgaacaaattagctcattatgatcggttaatacttcaacttctggttgcatgattgtttgtccgtaaaaagataacgcgcctgccgggtagtagcaggcgcattacgcaataggtaaacaagggaggaagttcagaaatgtaaatcgggaaggttgtacgcaatgttcatcgtactacgttgttacggctttgccgcaacaagccagttgcctgccgcgctcgcagaatgtctgcagcccggagataaggagattgttcctgccagctaaatcccttcctgtcgatacgaaccagctcgtatttttctaccagaaaattcacggcatcggctagggtgataccggcatcgatgtgttccttaatcacagcctcattgcagaatggcgtgtcgtttattgtcagaccatagtgctgttccagcagacgtgtcagtaacatttgccagacagccacgggtgacaggcagggcttcaccgcccgctgagttattgcaggtaaagttttcatgtttgctctcgtgtaggtaattaacgctgagtggggtaaatggcgatgtatacgtagccgcaactgccaagggtgtcggcttcgcaggttaaatcgttgtggtacagggtaacgcagtgggcatggtgggggctgagttcaccggtggtcagcatcgattccatctggaggataaagtgcgggaatgtttcatccagcttccggcattcgatgtcactgaacttgccggtgatgctggcccggtcagccagataatgcagtcggttgccttcctgcaccagacgggctcccaggcgcagtgtaatctcccgctgcaggcccctggtagggttgctcattacagttctccactattgtcagttcagggtgatgctcatcaggcaggtatagggcccattgcggtcctggcggcgttcggcgtataccgcgaggactccggcgatatccggaacgtccctgccggtgtaatgacagacgctaccgtgccactggtatttgccggtgcagtagcgaaagattcgggactcaggatgctggcggtatatcgtcattgccctgcgtttactgataattttcatgtaatacctcaaagcagaccgtgttctgcgaacgaatagatttgcctgccaccgacaatcagatggtcagggacacggatatccaccagctgaagcacctgaaccagtcgctgcgtgagggttttgtcggcctggctaggtgtcgtctcgccggaaggatggttatgcgcgagtatcaccgccgccgcgttgaagtgcagagcacgtttgaccacctcccggggatgcacctcggtgcggttaatcgtgccggtgaagagcgtttcatgggcaatcaactgattctggttgtccagatacaacacccggaactcttcccgctcaagcgcggccatatgcagtcgcagccattcacgtacggcgtgggtagaggtgaaggctacgccgggctcatgcaggtggcggtccagagccctgagcgcccgctgaatgagacgccggtcctgtggcgtcatctcgccgggtaaaaaggaaagctgtttcatctgttgctccttcggtcagtcgataatacgcagaatggcgtgagcctctggatgttgcatggcatactcccgcaggcggtaatagtgtgcggtcatcgcgtcacattctgtacggcaggcatggtggctatacgcaatcaggcagacagcaatacctgctgcttctgcactcatttgggcatcgttaccgttcaggcagttaaacagacgccatgtctcatcgttgtcaggctcgggggacataaatgcgccgccattgctgagggtgtagaacgaccagataccaccgctgtagccctcacagaagcggtccatccaggcgaagatatgcggctccaggagtagccactgcgggatagcgccaaagtactgtggccagaaatcgatacgctgttcatcggggaccggcgtgacggtcagttcaaattcgggttggttagcgggtgcgaggtcgtgctgcgtctgtgttgtcatgggtatgtctccgtcaataaaaacgccagcggcgatggctggcgtatggggatataaagtgtgttcggggaggtgaatgcgggtaaatgcttcgcgatcagcgggtggccgtgtctgtacggatgcctgaggtgcggatatagcggttaagaccttcaccggcatccggctcaaagttccatgcccgccagaccatccggccttcagtatcacgaaccaccagacggaagtgactgccctggtcgtcttcgagtgtgatattgctgtacgtggtagtgaccgcttgcgcttgtctccgggtgaaaggccccggtggcagcaacacggattgggtcattttcgggctcctgataaaagaaaaccccggcagcctgctagctgtcggggtgaatttgctggggaagatactactatcagtcgttgctgcagtctccgagagtggacagaactttctcagcgttcttccggtccgcagtgaaggtccctgctttgtggtcattgacgtagacgtcgaactgcccggcctcagagatattgctgatgaagtcaaaccaggcgttatcgccgttacgccagcccaggctggacggaataatgtactgctggtgatccatcactacggtgatagtagtgtcgtcatcgtgcgaactgaccatcttgtcatcggcaagggtaagaaagactgaatgctgatagaaaccattctggtccgggttccctgtgcagttgatggtaaacgtctttccgctggcttcggtcacgctgtattccgtattgccctgaccgtaaccctgctgccagaaccccgggatagcagaggcattaaagctcgcgagcagtacacccgccagcataaaccgacttagtgaaagtattgtcattcttgtctcctttgtcgttgttttattcctgattgtcagggttcgagggtatcagtagctgccccatcagtttgccgtcatgggcgtactcaaagtatttttctttggtatacgggtccgtcacctcctggtattccagtttgatgttatcggcaatacacagcgcattcatcagtggctggacggttttttcctgcatatccacgaggtagtagtaactgccatcctcgcagccatcgggcgactggcgggtacgtaaaacctgcaaggtgggaccggataagtagtcaacctgtgaccattcttcgctgacatcatcctggtggctgaccacatcactgaaacgcggtggggtgaggtccttaaatttactgatggccttcaggtcatcacttctgtcatcgcatgcgatgagaaacagagtggtggcaaccagcgccagcagaggcagtgttttacgtttcattatttttttcctgaaatcagacgaaccactttggcaaagacataaatgcccacgaaaatacccaccggcacgccgacgaacggtgtcagcgcgacactggcagcaccggctgcgccacctcccgtcagcagtgcggcaacagtggcaagggtcagggccgcgagactgtcggacaccccggttttgttcagaatgatgacgatgacaacaatggcgataatggcaatatccggactgatactccaggtccagatacatcagccgctcacgaaaatcacgccgcagcgtgcgcaccgacacaccaaactcagcggcaagcttacgcacactcagcgtttcccctgccaccagacggctgattatcagtgacagcctgacagccagccggtcatggcggcgttctgcctgtgtcatgagacgttctccgtgaaagttaactgactgaaaatgatgtgattactttaaagagggggtcggacagggtatggacaccacagaaactatttttcatttctgcaaaagccagaggcagcgggggttacaggccttccctcggtgagtgaggaccgtcagcacggtgcgatgcggacaggtggtgtccgatattaacaaagcagcaacattaaacggtcactgcagttgcgtgagcagggcttccgccatcacccacagtgcccggttaagtttcacgtccccgtcgataccgcgaacggcacgggtatgtgaccgtcctcctttggcattacggccactgagcccgcccttaatcaggttctcctgaatacgctggtacgtggtccacaggtcattgctctcatcctgccagcggcgaggggagaggatctgcgattcagtcaccggctggtggtcttcaccaaagcggtatgtgagggcggcttttgccagtgcctgctgtgccgggggtggcaacagcaacgactgcatggcatcccgtttctcctccacccggtcaaaaatccccagcacctcatacgcgccttcaatcacctgactcaccacgtcccccttgtgtggcacccgcacctcgccaaacgactcaccgcagacgagcccgttctgacaaaccgcacgaaatagtcccggcaacatctgatacgaactggttccatcgtgagagttgagtagaataatttccggcacctgtttaccggtgatctgcccttcccgccgcagacgcagcatatgctttgtatgttcacgacgacccgggtcacgcacgcgggtctgacaggcaaagaatggctggaagccttctcgctgtaggctgtcgagcagggagatggtgggtatataggtataacgctcactacgggactcgtgtttgtcctcactgaatacactgggcactacgcgaaacagctcttcacgggttaacggacggtcgcgacggataaggtttgctgcgccaaagcgcgaagccagacgggtcataagcagactcctcataacgggaaaacaaataaaagggatccccgtcgcatcggcgacaggggcagggaagtaacagggatgggttaaatactcagaagaagaaatcccagacggcgcgggccactgacaccaccgtggtgcgcacggcctgaatgacggcccgcaccggggcgggtatcaggggaaaggcactgatgctatcgagtacggccccgacggtttcaccaaaatcgctacgagcctgttcccggactaccgtcgtgcgaaaggaaggatggagttgcgacaccaccgggctggtggcctcacgtggcaggcacttaatcatccgctcggccatcaccttaagcccccattgtagacggaccgacacagcacacaccggatggacgggctggaacagctcatgcagcaggcagattttgcggctgatattctgcttctgcgccgtggacaactgtcccccaccgctggtaggttcggccttatccgactggctgataacaaacagcaccttatgccggtatacctctccaatcacctgatgataaaaatgttcatccaccgtcagcgcccggtcatcggccttaatcagccacagtaccaggtcgaggcgaggaagctgttcgcggtacagcgcagcatactcggtatcgcgagcgccactttcgcccacgccgggcagatccatcagcgttatatagcggtcgccgacttgcaggcgaaagcgcagtggctcacgtgtacaggccgccacatcgctgaccggtgatatatctccggcaaacagggcattgcacagactgctcttcccaacaccggttttacccataatgccgatcactggctcgtagttagttaactggttaatttgctgcagaagccgctctgatacccattgcggcagatcagcaagcgattgctgaaacgacttcaaaccttcagaattattcatcactactcctctgaaaaataataaaaaacggtagaatcgtgagattccgccgttaattgcgtatgttcagagtgatgatatatatctgaagattttttcaatcctctgcgcttgaggcagctgcgcgactgctggctcaggcaatgaatgagttataatagcagcatttactaacagggatttattgagagtatgagccgccgtgatacaccttaaaatctcaacccagcaaagtttcggagccgcgagcaaaagtgagagccttcacaaaataatgcttagtaataaagttactttgaattcagagccccgattaatgtgaacatgatcaacgaattttacccagattgagttcattcagtagccaggttttgaacacatcaagcgcagaatgcatgtgttggtgctgggggaaaaccaaataatgaccgatgtaatgtatttcgctggtactgtttacaagtgggcataccagtttaccgctagcgatttcacgttcagccagtagttttgattcaagcacaactcccaagccgtcaactgcggcagcaatcgccataaagctacggtcaaatcgaaggccataattattgggtggcgtcatcttattcgcctcaaaccatcctttccactggtacaactgcacatcgcactgaatcaatgtcaacgcatagagatcctctggtttctttagccgctcagccagttggggagaacacagtggcgtaagttcttcaacagcaagcgggatcttctcatagggtgatgggcggggttcaccgtagactatatcgagatcaaaatcatcctgttcaaaacgtgcatattctgtgctggctgaaagtcgcagatcgatgcttgggttctcacgtatgaacttaccaagacgtggtaaaagccattgatgggcaaaactcggtgcagtatgaaggcgcaaaggcctggattcatcagccgtcactaatgccaacccctgctgtaattcgttaaatccccgctgtatgtgctcaagcagtatttcaccttctttcgtcagcgtaatttctcgcgtactgcgctgaaaaaggcgtacatcaagcaagttttccagtttgcggatggcatggctgatcgcactgggtgacagttccaactcagaggcggccaacgcaaaagctccggtacgaccagccgcttcaaaggcgcgtaacagatttagaggtgcttttgctaagagcttcattcatgaatccttttcactagggatgaagtggtttactgaatttggccacctgaacagaggtgatatgctcacctcagaacaacacaggtgtcataatgaaaaaaagaaatttcagcgcagagtttaaacgcgaatccgctcaactggtcgttgaccagaactacaccgtggcagatgcagccagcgctatggatgtcggcctttccacaatgacgcgatgggtgaaacaattacgtgatgaacggcagggcaaaacaccaaaagcctcccccattaccccggaacaaattgaaatccgtgagctcaggaaaaagctacaacgtattgaaatggaaaatgaaatattaaaaaaggctactgtagattcaattggtcaacgcaacagttatgtgaaaacatggggttgcggaggttttttgaatgagacgaacatttacagcagaggaaaaagcctctgtttttgaactatggaagaacggaacaggcttcagtgaaatagcgaatatcctgggttcaaaacccggaacgatcttcactatgttaagggatactggcggcataaaaccccatgagcgtaagcgggctgtagctcacctgacactgtctgagcgcgaggagatacgagctggtttgtcagccaaaatgagcattcgtgcgatagctactgcgctgaatcgcagtccttcgacgatctcacgtgaagttcagcgtaatcggggcagacgctattacaaagctgttgatgctaataaccgagccaacagaatggcgaaaaggccaaaaccgtgcttactggatcaaaatttaccattgcgaaagcttgttctggaaaagctggagatgaaatggtctccagagcaaatatcaggatggttaaggcgaacaaaaccacgtcaaaaaacgctgcgaatatcacctgagacaatttataaaacgctgtactttcgtagccgtgaagcgctacaccacctgaatatacagcatctgcgacggtcgcatagccttcgccatggcaggcgtcatacccgcaaaggcgaaagaggtacgattaacatagtgaacggaacaccaattcacgaacgttcccgaaatatcgataacagacgctctctggggcattgggagggcgatttagtctcaggtacaaaaaactctcatatagccacacttgtagaccgaaaatcacgttatacgatcatcgttagactcaggggcaaagattctgtctcagtaaatcaggctcttaccgacaaattcctgagtttaccgtcagaactcagaaaatcactgacatgggacagaggaatggaactggccagacatctagaatttactgtcagcaccggcgttaaagtttacttctgcgatcctcagagtccttggcagcggggaacaaatgagaatacaaatgggctaattcggcagtactttcctaaaaagacatgtcttgcccaatatactcaacatgaactagatctggttgctgctcagctaaacaacagaccgagaaagacactgaagttcaaaacaccgaaagagataattgaaaggggtgttgcattgacagattgaatctacaaccgcgctcttgatgtcagactccctgaacagttctcgataatcgggaaactcagggcgcgttatcctgtggccactctctgccatgtgttcggggttcatcgcagcagctacaaatactggaaaaaccgtcctgaaaagccagacggcagacgggctgtattacgcagtcaggtacttgaactgcatggcatcagccacggctctgccggagcaagaagcatcgccacaatggcaacccagagaggataccagatggggcgctggcttgctggcagactcatgaaagagctggggctggtcagttgccagcagccgactcaccggtataagcgtggcggtcatgagcacgttgctatcccgaatcatcttgagcgacagttcgccgtaacggaaccaaatcaggtgtggtgcggtgatgtgacctatagtgtgcccggagttcagggcgggcatggatgcttaaatgaaccgcgagtctgtctggaatattgaaccggtaactcacgatgagaaacccaacaatcccaccgggtgtgacggtggagaacctgagcggcagtgacctgcggcatgcccgcagggtgatgtaacccgctgacaacggggattgaggcgagatcactaagccgagatgatcctcaaggttaagtactgaaaggttgaagaacatgaacccgttaatccgcctctgtgggttgaaaacgtcaccacggcctacgtgatctgacaggccgtgcaggaggaactggcagtgatacgtaagcactgccggtcgaaggtgttttgacatgtatgcgaaacaccggggcagcagcgtctatcacgcttgcgttgctgacttctgccaacttgcggcaagcaaggataaagagtgcgacgggcagcctcctcagtatgcctgagtccaggcaggtaaaccggggaaggtcagcgacggatgttaagggggcatggctccgatgacgcgctggctggcggagcttccgtagtagtccgcgatggggaaagcccattacatggcgaagggaagcagtttgaatgtgtttgcgacgtgaattaactgacctaacgaggtgaagacctttgataatcagcgaaatgcaacgcaagcttgccacatgggcagccaccgatccgtccctacggattcaacggctgctgcgtctgataacacaaccagaatggctggctgaagcggcgcggatcacgctttcatcaaagggggcccatacccccggcgttgatggcgtgaacaaaacaatgctacaggccagactggctgttgagctgcaaatcctcagggatgaattactctcaggccactaccagcccttgcccgccagacgggtttacatccctaaaagcaacggcaaactgcgaccactgggtatccccgcgttgcgggatcgtattgttcagcgggccatgctgatggcgatggagccgatatgggagagtgattttcatacgctctcatatggcttccggcctgagcgcagtgtccaccacgcgatccgcacggtgaaattacagctcacagactgtggtgaaacccggggacgctgggtgattgaaggcgacctgtccagttacttcgacaccgtacatcatcgactgctgatgaaggctgtacgccgcaggatcagtgacgcacgtttcatgactctgctgtggaaaaccatcaaggcgggacatatcgatgtcggtctctttcgggcggccagtgaaggtgtgccacagggcggtgttatatcgccgctattatcgaacatcatgctgaatgagttcgatcaatacctgcatgagcgctacctgagcgggaaagccagaaaagatcggtggtactggaataacagtatccaacggggccgaagtacggcggtcagagaaaactggcagtggaaacccgcggtggcgtactgccgctatgccgatgattttgtcctcatcgtcaaaggcaccaaagcacaggtggaagccatcagggaggagtgtcggggtgtgctcgaaggcagtctgaaactcaggctgaacatggataagactaaaatcccccatgttaatgacggctttatctttctggggcacaggctcattcgcaaacgcagtcgttatggcgagatgcgagtggtctcaacgatcccgcaggagaaagccagaaacttcgccgcatcgctgacagcactgttatggaaggtgcgaataagcggggaaattcttctcggctgactcagtcatttcatttcttcatgtttgagccgattttttctcccgtaaatgccttgaatcagcctatttagaccgtttcttcgccatttaaggcgttatccccagtttttagtgagatctctcccactgacgtatcatttggtccgcccgaaacaggttggccagcgtgaataacatcgccagttggttatcgtttttcagcaaccccttgtatctggctttcacgaagccgaactgtcgcttgatgatgcgaaatgggtgctccaccctggcccggatgctggctttcatgtattcgatgttgatggccgttttgttcttgcgtggatgctgtttcaaggttcttaccttgccggggcgctcggcgatcagccagtccacatccacctcggccagctcctcgcgctgtggcgccccttggtagccggcatcggctgagacaaattgctcctctccatgcagcagattacccagctgattgaggtcatgctcgttggccgcggtggtgaccaggctgtgggtcaggccactcttggcatcgacaccaatgtgggccttcatgccaaagtgccactgattgcctttcttggtctgatgcatctccggatcgcgttgctgctctttgttcttggtcgagctgggtgcctcaatgatggtggcatcgaccaaggtgccttgagtcatcatgacgcctgcttcggccagccagcgattgatggtcttgaacaattggcgggccagttgatgctgctccagcaggtggcggaaattcatgatggtggtgcggtccggcaaggcgctatccagggataaccgggcaaacagacgcatggaggcgatttcgtacagagcatcttccatcgcgccatcgctcaggttgtaccaatgctgcatgcagtgaatgcgtagcatggtttccagcggataaggtcgccggccattaccagccttggggtaaaacggctcgatgacttccaccatgttttgccatggcagaatctgctccatgcgggacaagaaaatctcttttctggtctgacggcgcttactgctgaattcactgtcggcgaaggtaagttgatgactcatgatgaaccctgttctatggctccagatgacaaacatgatctcatatcagggacttgttcgcaccttccggaggcgttatgagctggcggccctttttgtatctgattattaatccccacccgctattaagcgcccggcgcgggcatctgcgtctggtgcagggttgactttgcattctgttaacaaacgcggtataacaaaccttctttggatgtttagatgtccatacgtttagaaggttatatgcaaacaacacaacaaaatgcgccactgaagcgcacaatgaaaacgcgtcacctgattatgctttccttgggcggcgtgattggcacaggattattcttcaataccgggtacatcatttccaccactggagcggcgggaacgctgctggcctatctgattggtgcgctggtggtctggctggttatgcagtgtctgggcgagctgtcggtcgcgatgccggagaccggagcgtttcacgtttatgccgcgcgctatcttggtccggctaccgggtataccgtggcctggctttactggctgacctggaccgtggcgctgggttcgagctttaccgccgctggattctgtatgcagtactggtttccacaggtgccggtatgggtctggtgcgtggtgttctgcgcgattatttttggtctgaatgttatctccacgcgcttttttgccgaaggggagttctggttctcgctggtcaaagtggtcactatcatcgcctttatcatcctcggtggggcggcgattttcggctttattccgatgcaggatggctcgcccgcgccggggctgagtaatatcacggcagaaggctggttcccgcacggtggcttaccgattttgatgactatggtggcagtgaactttgctttttcgggtaccgagcttatcggcattgccgccggtgaaacggaaaacccgcgcaaagttatcccggtagcgattcgtactaccatcgcgcgactgattattttctttatcggcaccgtgtttgtgctggcagcgctgatcccgatgcagcaggtgggcgtggagaaaagcccgtttgtgctggtatttgagaaagtagggatcccgtacgccgctgatatttttaacttcgtgatcctgacggctattctttctgcagcgaactccgggttatatgcctccgggcgcatgctgtggtcgttgtcgaatgaacgtacgctaccggcctgttttgcgcgagtaacgaaaaacggcgtgccactgacggcgctgtcggtcagtatgctcggtggtgtgctggcgctgttttccagcgtggtggccccggacacggtatttgttgcgctgtcggcaatctccgggtttgcggtggtagcggtgtggctgagtatctgcgcctcgcattttgtttttcgtcgccgtcatctgcaacaaggtaaggcattgagtgaattacattatcgcgcgccgtggtatccgctggtgccagtattaggttttgtgctgtgcctggtggcctgtgttgggctggcattcgatccagcgcagagaattgcgttgtggtgcgggttaccgtttgttgcgttgtgctatggtgcttatttccttactcaaccccgaaacgcaaaacaggagccagaacatgtcgcagaataatccgttacgcgctcttcttgataaacaggatatcctgctgctggatggcgcgatggcgacggagctggaagcgcgagggtgtaacttagccgacagcctgtggtcagccaaagtgctggtagaaaacccggagcttatccgcgaagtgcatcttgattactaccgggcgggggcgcaatgcgcgatcactgccagctatcaggcgacgccggcgggcttcgccgcgcgaggtctggatgaagcgcagtcgaaagcgctgattggcaaaagcgtggagctggcgcgtaaagcccgtgaagcgtatctggcagagaacccgcaggcgggaacgcttctggtggcgggatccgtcgggccttacggcgcgtatctggcggatggctctgaataccgtggcgattatcattgtagcgttgaggcatttcaggcgtttcatcgcccgcgcgtggaagccttgctggatgccggggccgatctgctggcctgcgaaaccctgccgaatttttccgagattgaggcgttggccgagctgttgaccgcatatccgcgtgcgcgggcgtggttctcatttaccctgcgcgacagcgaacacctgagcgacggtacgccgctgcgtgacgtggttgcgttgctggcgggttatccgcaggtggtggcgctaggcattaactgtattgcgctggaaaacaccaccgctgcgttgcagcatttacacggtttaacggtgctgccgctggtggtgtatccgaactcgggcgagcattacgatgccgtgagcaaaacctggcatcatcacggtgaacattgcgcgcagctggcggattatctgccgcagtggcaggccgctggcgcacggttgattggcgggtgctgtcgcaccacgcctgcggatatcgccgcgttaaaagcgcgaagctgagggtttatcgggtctacatcgttcattgtaggcctgataagcgcagcgcatcaggcattgccggatggcggcacaagcgccttatccggcctacaaaaccacaaaacgttatgccgcatccgccagaacaaacatgccgtacggatggatttcaagataatactgctcgccgacgtccggttgcagacgcgtagcgttgacctgcaataatatctcctgcccgtgccattccaccgtcacttcatactgcggccccatataggcgacatggcggatcacgcagcgctggctctcttcgccgcgatcgctgagcgtgatcgcttccgggcgcacaccgaccatcccttcaccctgtgtaccaaagtgcagcgggcgcggcagatgatagccgtagatatcaacgtatccgtcgctgaaggttgccgggaacaggttggcatcgcccataaagctcgccataaagcgggaggcgggctggcggtaaagatcctgcggtgagccgatctgcatgatgtgtcccttgttcatcaccagcacagtatcagaaaccgcaaaggcttcgctctgatcgtgggtgacgtacagcgaggtgatatcaaactgcttttgcaactcgcggatcttgtcgcgcatgctgcgacgcaggttggcgtcgaggttactcaacggctcatcaaacagcagcactttcggcttgaggatcagcgcgcgggccagcgccacgcgctgctgctgcccgccggagatctgatcgacaaagcggtcttcgaatccttccagatccaccatcgccaacgcctctttgacgcgggctttcagctctgcgcgcggtacgccgagcattttcaggccataaccgacattctctcccagcgacatatgcgggaacagggcataggactgaaacaccatacagatatcgcgctgctgaatagagcgatgggtgacgtcttcgccatcaatgaaaatttgcccttcgctcggtttttccagcccggcaaccaggcgcaaaatagtggttttgccgcagccggacgggccgagcagcgtcaccatttgcccctgcgggatggtgaggttgatattgtcgattaccgtattactgccaaatcgtttagtgacgttgcgcagttcaacgaaatttttctgagtcatagtgcgctccattacgcctggtttttggcttttgaacgggaggtacgtgattcaccgatcagccagtcaaagatgaaaataatcgccagcatcaccacgatcagaatggaaccgtaggcaatcgctacaccgtattcgccatcttccacgcggttgaggatgtaagccgtcgctacgcgggtatccggcgtgacgaggaacacaatggcgctgacggtggtaatggcgcgcacaaagctgtaaatcagcgccgagaggatcgccgggcgcagcagcggcagcaggatgtgcgtaatggtacgcagggaaccggcgcgcaggctgagtgaggcttcatcgagcgatttatcgatttggcccggtaatgactccaacttattgatagtgttttatgttcagataatgcccgatgactttgtcatgctgctccaccgattttgagaacgacagcgacttccgtcccagccgtgccaggtgctgcctcagattcaggttatgccgctcaattcgctgcgtatatcgcttgctgattacgtgcagctttcccttcaggcgggattcatacagcggccagccatccgtcatccatatcaccacgtcaaagggtgacagcaggctcataagacgccccagcgtcgccatagtgcgttcaccgaatacgtgcgcaacaaccgtcttccggagcctgtcatacgcgtaaaacagccagcgctggcgcgatttagccccgacgtatccccactgttcgtccatttccgcgcagacgatgacgtcactgcccggctgtatgcgcgaggttaccgactgcggcctgagttttttaaatggcggaaaatcgtgttgaggccaacgcccataatgcgggcggttgcccggcatccaacgccattcatggccatatcaatgattttctggtgcgtaccgggttgagaagcggtgtaagtgaactgcagttgccatgttttacggcagtgagagcagagatagcgctgatgtccggcagtgcttttgccgttacgcaccaccccgtcagtagctgaacaggagggacagctgatagaaacagaagccactggagcacctcaaaaacaccatcatacactaaatcagtaagttggcagcatcaccgagaacacaaatgggctaattcggcagtactttcctaaaaagacatgtcttgcccaatatactcaacatgaactagatctggttgctgctcagctaaacaacagaccgagaaagacactgaagttcaaaacaccgaaagagataattgaaaggggtgttgcattgacagattgaatctacagcagctttttttaatatgtcccgttcgtcggtaacccgtttcagctctttctggagacggcggatctcggcctgagcatctgactgttctttattagtggaagaatccggaccgtacttctttatccaggcataaaggctgtgggtggtgatatcgagacgtgttgcaacgctggcaacagaataaccgagatcaacaacctgtttgactgcttcagttttaaactcttcgggataacgcttaccgctcatgggcacctctctttaagccattttaaatgactcggaggtgtctgttaaacccgtggcgattcaaaattgcgatatatacatacccatgactgcccagcgtatcggcttcaccagtcagcccgttacggtacagtgtgacacagtgcgcgtacctgggattcagctcacaggagagcagcatcagctccagatgtgcgacaaaatgcgggaaggcttcatccagttgtagagtctgcacctcactgaatgagccggtgaatccagcccggtcagccagaaaatgcagacgatgaccttcctgcaccagtcgtgctccgaaacacggtgtgatatctcgtttaagcccccaagtttgagtagagtctttattcataattttattcctgttaaagaagaccatgttcggcgaatgagaatatttgcctgccgccgacaatcaggtggtcggggacatggtgaacactttttaacatcctttacccatggtgatcgactttttcttcaggtcgatcacccccactttcgtgctgtaccaccacacctcgtagctgccgtcttcctgcatctccttcagcccgacccgttctcccctgaacgccttgcctgcgctcagacttacccctttcacgctcagctttccgctgatatccactttcctgaccatcaccccttcatcgtattccgggggcgttgtgttgccgctgtactgccgcgctgacggctgataccgcgagcccggtaccgccatatccagcgcctcgtgcgggcgttcaaggttatagaccgtccgccagtggtcgaaggcgcgctgcagttcaccgctgtctgcgaaccattttccctgcagcacttccgccttcaggctgcggtgaaaacgctccagcttcccctgcgtctgcggatgataaggccgggagtgccccacccggatacccaggcgcatcagccacagctccagcgccgtccaggtgccggtggtgtcgccccacggtgagccgttatccatggtcatccggtccggcaggccgtaacgctcaaacacgctgaccagctgctgctgcacggtctcgcgccgttcatcggtacagtgcgccaggcacagggaaaaacgggagtggtcgtccagcagggtgagcggatggcagcgtccaccgccaaaaggaaagtggcccttaaaatccatctgccagaggcggttcggcgcgtcgtgttcgaaccggcccgtggcgggaatgcccggtgaagcgcccggcagcaggccatggcgggccatcaggttatggacggtgctgaaggcgggcatggtgtgcccctggtcctcgagccagcgcttaatcttgcgggctccccagcgttcatgacggtcatgggccatacgcagcagggccgtgatgtcgtcagatgagcggttcggggaatggtgcggaatgcgcgggcggtcctgaagaccggcggcaccttcctgagcccagcgctggagccacttgtagccggtggcaggtgaaatgccgaagcgacggcagagggaacggatgttcgccccgtcctgcgaggcgaacaaaacaaactcagtacgtaatgacatggtatctctcgcatcccagggcataagcgactccataaacgggttcttatgccttagttgtaagtgtctaccatgtccccgaacaagtgttcactatgtccccggaccgtacaccccaaaggggagaggggactgcaccgagccatcttttccccctcgcccctttggggagagggccggggtgaggggcaatatgtgatccagcttaaatttcccgcactccctcttcccttccgatttacctctccttgttctgcgtcatagtatgatcgttaaataaacgaacgctgttctataatgtagaacaaaatgattcagcaaggagatctcatgccgcagtccgcgttgttcacgggaatcattccccctgtctccaccatttttaccgccgacggccagctcgataagccgggcaccgccgcgctgatcgacgatctgatcaaagcaggcgttgacggcctgttcttcctgggcagcggtggcgagttctcccagctcggcgccgaagagcgtaaagccattgcccgctttgctatcgatcatgtcgatcgtcgcgtgccggtgctgatcggcaccggcggcaccaacgcccgggaaaccatcgaactcagccagcacgcgcagcaggcgggcgcggacggcatcgtggtgatcaacccctactactggaaagtgtcggaagcgaacctgatccgctatttcgagcaggtggccgacagcgtcacgctgccggtgatgctctataacttcccggcgctgaccgggcaggatctgactccggcgctggtgaaaaccctcgccgactcgcgcagcaatattatcggcatcaaagacaccatcgactccgtcgcccacctgcgcagcatgatccataccgtcaaaggtgcccatccgcacttcaccgtgctctgcggctacgacgatcatctgttcaataccctgctgctcggcggcgacggggcgatatcggcgagcggcaactttgccccgcaggtgtcggtgaatcttctgaaagcctggcgcgacggggacgtggcgaaagcggccgggtatcatcagaccttgctgcaaattccgcagatgtatcagctggatacgccgtttgtgaacgtgattaaagaggcgatcgtgctctgcggtcgtcctgtctccacgcacgtgctgccgcccgcctcgccgctggacgagccgcgcaaggcgcagctgaaaaccctgctgcaacagctcaagctttgctgagccggacgataacgatgaccattgagaaaattttcaccccgcaggacgacgcgttttatgcggtgatcacccacgcggcggggccgcagggcgctctgccgctgaccccgcagatgctgatggaatctcccagcggcaacctgttcggcatgacgcagaacgccgggatgggctgggacgccaacaagctcaccggcaaagaggtgctgattatcggcactcagggcggcatccgcgccggagacggacgcccaatcgcgctgggctaccacaccgggcattgggagatcggcatgcagatgcaggcggcggcgaaggagatcacccgcaatggcgggatcccgttcgcggccttcgtcagcgatccgtgcgacgggcgctcgcagggcacgcacggtatgttcgattccctgccgtaccgcaacgacgcggcgatcgtgtttcgccgcctgatccgctccctgccgacgcggcgggcggtgatcggcgtagcgacctgcgataaagggctgcccgccaccatgattgcgctggccgcgatgcacgacctgccgactattctggtgccgggcggggcgacgctgccgccgaccgtcggggaagacgcgggcaaggtgcagaccatcggcgcgcgtttcgccaaccacgaactctccctgcaggaggccgccgaactgggctgtcgcgcctgcgcctcgccgggcggcgggtgtcagttcctcggcacggcgggcacctcgcaggtggtcgcggaggcgctgggtctggcgctgccgcactccgcgctggcgccgtccgggcaggcggtgtggctggagatcgcccgccagtcggcgcgcgcggtcagcgagctggatagccgcggcatcaccacgcgggatatcctctccgataaagccatcgaaaacgcgatggtgatccacgcggcgttcggcggctccaccaatttactgctgcacattccggccatcgcccacgcggcgggctgcacgatcccggacgttgagcactggacgcgcatcaaccgtaaagtgccgcgtctggtgagcgtgctgcccaacggcccggactatcacccgaccgtgcgcgccttcctcgcgggcggcgtgccggaggtgatgctccacctgcgcgacctcggcctgctgcatctggacgccatgaccgtgaccggccagacggtgggcgagaaccttgaatggtggcaggcgtccgagcgccgggcgcgcttccgccagtgcctgcgcgagcaggacggcgtagagccggatgacgtgatcctgccgccggagaaggcaaaagcgaaagggctgacctcgacggtctgcttcccgacgggcaacatcgctccggaaggttcggtgatcaaggccacggcgatcgacccgtcggtggtgggcgaagatggcgtataccaccacaccggccgggtgcgggtgtttgtctcggaagcgcaggcgatcaaggcgatcaagcgggaagagattgtgcagggcgatatcatggtggtgatcggcggcgggccgtccggcaccggcatggaagagacctaccagctcacctccgcgctaaagcatatctcgtggggcaagacggtgtcgctcatcaccgatgcgcgcttctcgggcgtgtcgacgggcgcctgcttcggccacgtgtcgccggaggcgctggcgggcgggccgattggcaagctgcgcgataacgacatcatcgagattgccgtggatcgtctgacgttaactggcagcgtgaacttcatcggcaccgcggacaacccgctgacgccggaagagggcgcgcgcgagctggcgcggcggcagacgcacccggacctgcacgcccacgactttttgccggacgacacccggctgtgggcggcactgcagtcggtgagcggcggcacctggaaaggctgtatttatgacaccgataaaattatcgaggtaattaacgccggtaaaaaagcgctcggaatttaattattttaagagataaaaccgtctgcggaatatttcccgcagacggctttgttgtttttgaaatttattaatttaaacaattagttgagatatatcgttggcgtcacaaaagcaaaataacgtaattcggaaataagatatgaccattgctggttaattgaatagctcattacactccattaacacgatgttgtaattcggcacactacataagggtgtaattctgatgacgcaattaaccatgaaagacaaaattggctacgggctgggagacaccgcctgcggcttcgtctggcaggccacgatgttcctgctggcctatttctacaccgacgtcttcggcctgtcggcggggattatgggcacgctgtttttggtctcccgcgtgctcgacgccgtcaccgacccgctgatggggctgctggtagaccgcacccgcacgcggcacggccagttccgcccgttcctgctgtggggggccatcccgttcggcatcgtctgcgtgctgaccttctacacgccggacttctccgcacagggcaagatcatctacgcctgcgtgacctacattctcctgaccctggtctacaccttcgttaacgtgccgtactgcgccatgccgggcgtcatcaccgccgacccgaaagagcgtcacgccctgcagtcctggcgcttcttcctggcggcggcgggctcgctcgctatcagcggcatcgcgctgccgctggtgagcatcatcggcaaaggggacgagcaggtgggctacttcggcgccatgtgcgtgctggggctgagcggcgtggtgctgctctacgtctgcttcttcacgaccaaagagcgctacacctttgaggtgcagccgggctcgtcggtggcgaaagaccttaagctgctgctgggcaacagccagtggcgcatcatgtgcgcgttcaagatgatggcgacctgctccaacgtggtgcgcggcggggcgacgctctacttcgtgaaatacgtgatggatcacccggagttggcgacccagtttttactttacggcagcctcgccaccatgttcggctcgctttgctcctcacgcctgctgggccgcttcgaccgcgtcaccgccttcaagtggatcatcgtcgcctactcgctgatcagcctgctgattttcgtcaccccggcggagcacatcgcgctcatttttgccctcaacatcctgttcctgttcgtctttaataccaccacgccgctgcagtggctgatggcttctgacgtggtggactacgaggagagccgcagcggtcgccgcctcgacgggctggtgttctccacctacctgttcagcctgaagattggcctggcgattggcggggcggtggtgggctggatcctggcgtacgtcaactattccgccagcagcagcgtgcagccggttgaggtgctcaccaccatcaaaattctgttctgcgtggtgccggtggtgctctacgcgggcatgttcatcatgctgtcgctctacaagctcaccgatgcccgcgtggaggccatcagccggcagctgattaagcaccgcgcggcgcagggcgaggccgttcccgacgccgcgacagccgcatcccattaaccggaggcaatatggaaatcactaacccgatactcaccggcttcaacccggacccgtccctgtgccgccagggcgaggactactacatcgccacctcgaccttcgagtggttcccgggcgtgcgcatctaccactcccgtgacctgaaaaactggtcgctggtcagcaccccgttggaccgcgtgtcgatgctggacatgaagggcaacccggactccggcggcatctgggcgccgtgcctgagctacgccgacggtaaattctggctgctctacaccgacgtgaagattgtcgactcgccgtggaaaaacggccgcaacttcctcgtcaccgcgccctccatcgaggggccatggagcgagccaatcccgatgggcaacggcgggtttgacccgtccctgttccacgacgacgatggccgcaaatactatatctaccgcccgtgggggccgcgccaccacagcaacccgcacaacaccatcgtgttacaggcgtttgacccgcagaccggcacgctctcgcccgagcgcaaaacgctgtttaccggcacgccgctctgctacaccgaaggcgcgcacctgtatcgccacgcgggatggtactacctgatggccgccgagggcggcaccagctacgagcacgccgtcgtggtgctgcgttccaaaaatatcgacgggccgtacgagctgcacccggacgtaacgatgatgaccagctggcacctgccggagaacccgctgcagaagagcggccacggctcgctgctgcagacgcatacgggtgaatggtacatggcctacctcaccagccgcccgctgcgcctgcccggcgtgccgctgctggcctccggcggacgcggctactgcccgctggggcgcgagaccggcatcgcccgcattgaatggcgcgacggctggccgtacgtggaaggcggcaagcacgcgcagctgaccgtgaaaggcccgcaagtagccgagcagcctgcagccgttccgggcaactggcgggacgatttcgacgccagttcgcttgacccggagctgcagaccctgcgcattccgttcgacgacaccctcggctcgctcaccgcgcgcccgggcttcttacggctctatggcaacgactcgctcaattcgaccttcacccaatcgaccgtggcgcgccgctggcagcacttcgccttccgggcagaaacgcggatggagttctcgccggtgcacttccagcagagcgcggggctgacctgctactacaacagcaaaaactggagctactgctttgtggactacgaggagggacagggtagaaccatcaaagttatccagctcgaccacaacgtgccgtcgtggccgctgcacgagcagcccattccggtgccggaacatgcggagagcgtctggctgcgggtggacgtggatacgctggtctaccgctacagctactcgtttgatggcgagacgtggcacaccgtgccggtgacgtatgaggcgtggaagctgtcggacgactacatcggcgggcgcggcttcttcaccggcgcgtttgtgggcctgcactgcgaggacatcagcggcgacggctgctacgcggacttcgactacttcacctacgagccggtctaacggctcaggccgggtagcccagcgcgcgcgagagcgcgagcccggcctgctgaagctgctcgcggaaattagccagctccgcgtcgtccacgcgggaggtcagcgtcgacaggctcagggcggcgatgacgcgggactcgtggttccacaccggcaccgccacgcagcgcacgccctgctcgttctcttcgctgtccagggcgtagccttgctcgcgggtctgcgccagggcgctcattaaggcttcgcgagacgcgagggtggcgggcgtaaaggtagtgtactgatagccctccagcagggcgttcagctcggcctcgcccagccaggcaatcaacaccttgccgatggcggtggcgtgcaccggcaggcggcggccgatgcgtgaataggcgatggcggccagcttgccttcaatcttctcgatatagaccccttcacgcccgtccaggatccccagatgggtggtctgcccggtccgccgggacagctccgtcagccagccttttgccttctgccgaatatcgatggagcccacgacaaaatggccgcgctcgaccagcttcatgccgaggcgatacttgccgttctccgggttctgatcgatatagccgtgaagctgcagggtttttagcagcgagtggagggtactcttgctcagccccatcagtttgctgatgtcggtgatcttaagctcggtggcctgctcgttgaacaggtcgaggatctgcaacgcacgttcaacagactgaataatcggcataatgctggcatgtccacgctggaattaaggcgaaaacgtacctttttcgggatgaaaaatcaatgaaatggagccggtgttctccctctccctgtgggagagggccggggtgagggcaccaacgcgcagcggacccaatcactccccaagcgttgccatcatcaccgccttaatcgtatgcatccggttttccgcctggtcgaacacgatgctcgccgccgactcaaacacctcgtccgtcacctccatcccgccgtgcagatcgaactccttcgccatctgcttgccgagcgtagtctggtcgtcatggaacgccggcagacagtgcaggaacttcacgttcgggttgtcggtcagcgccatcatctgcgcgttcacctgatacccgcgcagcagcgcaatccgctctgcccacttctctttggcctcgcccatcgacacccacacgtcggtatagataaagtccgcgcccttaacgcctgccgccacgtcttccgtcagagtaattttcccgccgtgcttctccgccagcgcgctgcactccgccaccaggctctcttccggccagcaggctttcggggccaacaggcgcagatccagcccggtcagcgccgccgcttccagcatcgagttgcccatgttgttgcgcgcatcgcccgcgtagaccagcgtcatctcgttaaacgccttgcccggcaggtgctcctgcatggtcatcaggtccgccagcagctgggtcgggtggaactcgttggtcagcccgttccacaccggcacgcccgcatactgcgccagcgtttcgaccacttcctggccgtgaccgcgatactgaatgccgtcatacatccgcccgagaacccgcgcggtgtccttaattgactctttatgcccaatctggctgccgctcggccctaaataggtaacgcgcgcgccctggtcaaatgcggcaacttcgaaagagcaacgggtacgagtcgagtctttttcgaagatgagcgcgatgtttttaccggtaagcttctgtacttccttgccattttttttatcggctttgagctgtgcggcaagggtcagcagagaagtgaactgtgcaggggtaaagtcgagcagtttcagaaagtgttttttgtataaatcggacattttatcctcgcatggcgaacgccacttattgaattaaaattcactttatatgtgtaattattcatttgcaaccccatttcacaattctttcttacaaaggtggaggcaaacccgtccgtgtgtgaaaataatcgtatctgcctccgattctctgcagaagcagaaagacattggatcgaattctacaaccaggtcgagtcagaaatgagaatgattggccttctttatgattttaaggattatgcttctaaaatggcggagaacatggcgaggcttgctgccttacttcattacttcagcggtgatggaggcgatatatctgttaccgggtaatgactccaacttattgatagtgttttatgttcagataatgcccgatgactttgtcatgctgctccaccgattttgagaacgacagcgacttccgtcccagccgtgccaggtgctgcctcagattcaggttatgccgctcaattcgctgcgtatatcgcttgctgattacgtgcagctttcccttcaggcgggattcatacagcggccagccatccgtcatccatatcaccacgtcaaagggtgacagcaggctcataagacgccccagcgtcgccatagtgcgttcaccgaatacgtgcgcaacaaccgtcttccggagcctgtcatacgcgtaaaacagccagcgctggcgcgatttagccccgacgtatccccactgttcgtccatttccgcgcagacgatgacgtcactgcccggctgtatgcgcgaggttaccgactgcggcctgagttttttaaatggcggaaaatcgtgttgaggccaacgcccataatgcgggcggttgcccggcatccaacgccattcatggccatatcaatgattttctggtgcgtaccgggttgagaagcggtgtaagtgaactgcagttgccatgttttacggcagtgagagcagagatagcgctgatgtccggcagtgcttttgccgttacgcaccaccccgtcagtagctgaacaggagggacagctgatagaaacagaagccactggagcacctcaaaaacaccatcatacactaaatcagtaagttggcagcatcaccgaattttcagcccggatgtttcacgtacctatgtcgaatatctggccgataaggttgcggatcgagaagaggatgcagaggaatatctggaagcaatcatggaggctcgtgttaccgttgctggcatggggctggtgatggaggtgcaggattacttcgatggcgaggccgatagactggcgaaggcgtggctggccgagtacacaccgcaaatcaagtcgttgaaagatgagcgtaaagaggcctatcgtcaaatcgtcgaaatgagtaccgaaccgcaggatgtggatctggtcaggccggcgaacaagtttgaaatgaccagggtgcgtgaaggtgaaaaggaagctgaccttccagtctggaaacaccatttgttgtgtgacgaaagcgggaactatccggctctgttgaaccattgggaaaccaaggtttttgagatcgaaaccaaacgtgaaggatttgctttctggtatcgtaatccacagtacacagggcagtcgtcactgggaatcgcttatgttgaagctgaacagtacaagattgttcgtcccgatttcctgttctttgccgaacaggatggcaaaatggttgtggacctggtagatccacatagcctacatctggctgatgctttgcccaaactggaaggacttgcgctatatgccgaacatcattctgatgcttacaggcgaatcgaatctgtcgccgaagtaaagggtaaattacgagtgttagatttgaaacggcaggatgtgcaggatgctgttgctaccgctgaaaatgcagaaacgttatttagtagcggacttgctgatgactatcagtaatctatagaaaattgcgtaacgaaactgcattttagtaattttttgaaacaatacaaataaggccttctcactgagaaggccattaccgacttacagttcgatttggctacagccgaagttacggtctccttcaccaaacactttgctttcaactttggtcaggtagtccagtcgggttaacagcgcctggtagttctgctggaagtcagtactattggtgtctagcacatacttacagttttcaggaaaatggaccagaccagggtgatcgtctctctccagtctcagggcgctgtaccaggctcctgtgatcatccctctaaggttatcgtcctgatcgtaatccccgaggtggtagtaagcgtctttgttgaacaacaggcaaatgtgatagtggcatttacctgattcagaatactctttcgcccatataataaataaagggcaacggtaaatgcgtttatcctcacgcaccttacgggtacggtcagcctccagcttagctctgagggattcacgcatccgggatatcaccccaggttccaggttagggaagcaacagatattgtcaccgttatcaactattttgggatagtggagatcgacacgtacagcaattaacctaggataccggttagtcaaataacataataatttattaatcttactctgatattcgaggatatgtactccatgagtaccttgatatgttttcataatatatacctgtatttggtcctacggtctatagcagaccgtacagggatgccatacaggcagggctattcctggtcactgttgtcggtatatactggtatcagattttagtacggacatactgatctgattactactcttactggtgaatacaggtagtaagagtacacaatgccattatataatacctatccaacatctaaatttgagacgaaggtagccccagcctgtgatggctgttaaaaagttactctgcaattagcttctggaattaaccgatgattccgttattccagtgccgcttcacagtcgataaactgatactcaatttctttgcaatctcagcctgagtaaatccacctttcttaagtattgtgatatcacgtcggtatttgcttccctcctttcgtcctaattttttcttaacatgtcgatatcggcttttagttgatttcagattgtgaatgtcaatcgtatcctgacgagcaatcaaaaaagacaagcaactttcagcagaaggctctatccttgaagctggatggtagctgtagataaacatttctttttgaaggcaaaaaaataaaatattctgtaagtcctccacagttctgccaagacagcttagatctggaatgacaagcgtgtcctgccggttcatttcatgatgaatcaattgtctgagtaaacgttgctctgaaacaacctctttaatatctacctgctcgatcacaacatgttcaggtagaatattaaatttttggcatatctcagcaagtgagtgatgatctgtaatgctttcttgctgttcgctactgcatatggtgtaaaaaaatgaacgcatctgatgcactccggtgtcataaattattttttgatacctgaataatgtcattttgcataaaaaacaaccaaaaatagagagtgattgccagcgatactttaactggtaaagtagtattttacctctcataattgtttgtccttctttgttacctcttaggttctgctctcttgtgagtatgggtttataatgatgtcatccggtacattaacacggttggaaacatctgttttgcggagcactggcagcataaccaccatttcattgacatggtaaatatcaatccaacaaacaaccggataaggcataacaatcccctttcttctaagaacttcatttatcccgaatataatcaattgggatgttgacaagagtagagcctgcccggcatcaaagtaataaccctcaaaggttgttctatgaataagaataatgtttgaatatcctgagacactttgatgctttacatcaaaatgtctttgattgtaaatgtaaatggctttttccatatcgtaattttcccttagcgaggatagcctttcacgtataactgttttttcatctttccccatgaattcatcattagcgttcagttgaaagtaatctgcaatggggatttttaatggactcatgatgttcgttttccagattaacgaacagtactcttccagagttacttctgttttacctcggcttcgattgatgctttcttttatagagaactttaacaggtcattttttatttcatttattgaccagttatgacgattgcatttttctaatatagggatagccaaatccacaacttccgctattacggaagagtgagatttatttgttagtctggcataatgatcaattactcctaatgaagattgatttttgaacgtgactgagtgtttttttatgggagtagtctgtactacctgtgactcattgtttttgccttgacaaggtttttttcctggtagaacgctgctcatctcaaaattagtaacactattagacatttttaaggaaacctctttgttatctcaatataaaactactatctgaaatttctcagtgttgccccatttttctcggggcaacatcgctataaatcaataaaattaaatctgtaatttattacagactttctcgtacagaaaatgtatctataaaatcgaggacatctttacgtaaccagtaatggcggccattgatttgttttgggcgaggtagcccctcaggcaatttgtcctgacaaagccatttacgaatggtttgagatttgtagctaatgattttagctaactcagctgttgaaatgagctgtgattgagatgtatccgggagtttgaatgcgctcattttgccacctcagtgattgagatattggcaaagaaagctttaagcattattgaattagtaggggtagtaatgaaggcagaaggaaacgtttcgggctcggggtcggggtcactaccatcacctgaatctgatgataaggcacttttagctgatttagccgtactgtgatgcgatctggatgcctgatttttacatgacatcagacgcgcgagaaagttagtagcattttgcattctttgtttaagatgtaaaattttcagtttggcgcatgcgacagacttgcgaagagctgagtatgttcctttgagatactcgacaacctcttccatggacgcaggatcgttaaaggattgagttgttttacttgaattaatacaccagcgagctctgatagctgccagagtgggttctatggatacagttgctggggttgccattggcttatctcctgtgtagttgctgtatcattgactaaactgtgtattacgatacatgaaaatctatcttgatcaatagttgatgatattttgtaatatgttgatttttaatggaatcaacgcatatcaacgttgttttttatggtaatacctgcttcatttaagatccatgtctcaattttctcgtgccattttcgtaacagatctaacggacgacggcgatagtgtttttcggcaagagcgctgggtttgtgtcccataatttgagcaacaataccagtgggaacttcaacccactcggccaaagtaccaaaactacgacgtaaaccgtgaaggctgatatgtggtaactcagccagcactaatgctctgttgtgcgctgaacgcggctcaataattttgccacttttactgttacttctgaaaacccaaccctccttatttacgtcagaatttggggattgcgctagtacatttaacaattcagaaacataaggagtgagagggatgatacgttcaccttcgatcttgtctttaattcgcatgcttgaccatttgaaatctacgtctgaccagcgaagcgacgcaatttcttcacgccgagcaccagtgagcaaaagtacttggagataggccgatgcaataggattattgaggctacgcacggcactaaaccagctttttagttgttccttttgcaggcaatcatcagctttactcgctgacacgggaaccatttttcttacgttgtaatcttgtgccagatcgccaggaatgatcccttgatattttttctgataattactccatttgatgaaagcacgtagtaggcgataagcgtgagcagtgacggtaggtctattttgcctttctgtactcagccacgctgctatgtaatctggggttagctccgataacggcaggttgagcaaactagccaatggtccagccgaagtcgggccttggcctctttttttactttcgcctccacgactggacaagttaatgtgatcggcaatgtatcgagtagaatatgggcgtttagtttttgcactgataccggttctcaattcttgaagatagtcttcccaggcgacggagaaagtcacttttgttttacgtgattctgcctgcagggattctgcttctgcgatttttacagccttagcaattcgtggatctatccctgtatcgatcaatgtttgtaaccgtcttgcctcggctctcgcatcatcaatcttccagtcgttaatgttgccaatagtcatgcgaagggttttccccgcatatacgctttggaatacaaaggcttttgctccgctagttgctcggcatgccagggttgttacatctgcatcccaaagaaaagtttgttttttcccttccggtaaggtgaatctgcgaagtctttcgaaggtaaatttttgtcttgaaagcgccatttttcggctccagttgagaattgctgtcttacaataatgtaactgctggtgtaagtaaatggagggaataaacatcaacttttgttaatttcaatcaacgggtttattgctataacttggtgttttataatataaagtatgttgttttgattgattgctcaagtagttaaaaatgcattaacatcgcattcgtaatgcgaaggtcgtaggttcgactcctattatcggcaccattaaaatcaaagagttaccccatatttaaatacaccacgtttcctcctgtgccgtatttgtgccattgtaaccttggcaattcatcaaaatactgttctgacatcaggcagtgcaggtgcagacatttaagccaattgctgccgccattctttgacgtagtcaatcagggcgcggagctttggtgcaatattgcgacgctgtgggaaatacagatagaagcccggaaattgtggaagaaagtcatcaagcagcgatacaagcttaccgctttcaatatatggcctgaaagtttcctgagtggcaattgttattcctccgccggcaagagccagcctcaacatcagacgcagatcattagtcgtaatctgcggttcaatcgcaaggtcgaaagttctcccgttttcttcaaatggccagcgataaggcgcaacctccggggactgacgccagccgatacacttatgggtatttcccccggaggcgagaaagcactctccacgcccggccgcaaggatcaggacgacgggggcaggcatgaatcctcctcctgatggagacgtacagaggcgacttctgccagcacggagagtgccagagtatgcgcatcccgggctttggggaatatcccgacgggtgcccggatttgcgttgtttcctccctggaccatcccagctcgtggagcttttgcagacgtaacgtgtgggttcgatagctgcccaatgcgccgagataaaagggttttgcttctcgcgcggcctgcaacactggcagctcccggttgagatcatggcacagcaaaatgaccgccgtatcggtatcgatctgagcgctggctgaggccggaaaaagatcgaagatatggctgtcatagcctgtggctgctgcaagactcgcggttgcctgcgcctcaagagaacgtccgtaaatcatcagcctgacgcatggcctgaaccccacctcaaagccattgagattccagcccgtccgggtttgcgtgggcaggcacaccagcgattgtgcttgcggatcgtagcgcagccccaccggttttctctgttccaggcggttcagcacggcgagcagaggctgtgccgagcgtagtttatggagcgtcagcgtgatcccaccgccgcagggcagaacgatgtcaaaccacggcgaaccttcgccatagcgaatttcgcgatcgcggcctgagcccatcatctccagcgcttcaaaagcggcagcggcctccacgcagccgccagagacaaaaccgcagtaacgaccatcttcgcgcaccaccatctgcgccccgagcgggcgcgccgcgccgccgcgtatctccaccagcgtcaccagcaccgctcctttaccggacattagcgcctctacggcgaagcgcagaatggtccggtggtcatcggtgagaaacgcctgctctggcttatgccagtgttcgtctttgtcaaaaagcgggtatgacattgttcctccttaaaccacatccggcagcttatcgagcagcttatccagagtgatgggataatcccgtacccgaataccggtggcgttatacaccgcgttggcgatagccgcgctcacgccgcacaggcccagctcaccgacacctttggccttcatcggggaggatatggggtcggtatcatccaggaaaatcacctcctgttttgggatatccgcatgaaccggcacctcataccccgccatatcgtgattaacgaagtagcccaaacggtcatccaccgccagctcctccatcagtgccgcgcccatgcccatagtcattgcgccaatgacctggctgcgcgcagttttcggattcaggatgcgtcctgcagcacacacagcgagcatacgccggacccgaacttctcccgtcgcgctatgcacgccgacctccacaaaatgcccggcaaaggtcgactgctggtactctttgctcagtgttccgaattcaatgctctcttccgctgtcagtctgccgcctgcggtggcttcatgtagcgtggcgcttcgggtaccgttggtaatcttgccgtcggcaaactgcgactgctcaggatcaaacccgactgccgaggcaatcatttcgcgaagcttcatacaggcggcgtaaacgccggaggtggaggtattcgcgccccattgtccaccagaacccgcagaaaccgggaaactggaatcgccgaggtgaaccgcaacctgctccagcggtacgccaagcatttccgctgccgtctgggccagaatggtgtagctgccggtgccaatgtcggtcatgtccgtttctacggtaacggtgccgttttgttcgaggtgaacccgagcacccgatttttccagcagattattgcgaaagcccgccgcaacaccgtggccgactagccactccccgtcgcgcacctgtccgggtgtggcgttgcgctgcttccagccaaatttatccgctccggtgcgcaagcactcgataagctgacggcgagagaagcagcgcgtcgggtcggcggggtcaacctgagtgtcattcaggatgcgaaactcgacgggatcgatgcccgctttttccgccagttcgtcgatcgcgatttcgagcgccatcagaccgggggcttcgccgggcgcacgcatggcgttcccttccggcaaatcaagcgtggcgagccgcaggccggtatgacgattcgccccggcgtagagtaattcgctttgctgtaccgccgtttccggcgtgccgccgggcaggtttccagaccagctttcatgtgagatagcggtgattttcccgctctggtcggcaccgatacgcaagtgctgaagggtggcggggcggtgcgtggtgttattgggaatagaggggcgggggagcatcactttaaccggacgtttcaccgctcgggcggcgagggccgccagcagcgcatcgcttctcaggaacagcttgccgccaaaccctccgccgatatacggggagataatacgcacattctccacgggaactttcagcgtttttgccagatcggtgcggcaccagtcaatcatctgatttgaggtccagagggtaagcttatttccatcccagacggccatcgaggcatgcggctccatcgccatatggctctggtccggggtcgtgtaggtagcatcaatcttcaccgcagcggaggtgaaagccccgtcaaagtcaccgacgtttttgtcgggcgtgtcttccggcggctgattgacggcctgtttttcgtccgccagggagtaagctcctttattacggcgatagtgtgcctgcaccagcgaggccgccgctcgcgcctgttcgaaggtctcggccactaccagcgcaatggcctgatgatagtgctcaatagtggggccgcctaacagcctggcggtgtttttgtcgcctttgccgagtgccccggcgttactggcggtaatgacagccagtacgcccggcgctttttgcgcggcgtccgtatcaagggcggtgaggcgtcctttggcaatggcggaaccgacgatatagccataggcggcgttgggggcttcttcatgccattcgtaggcgtagcgtgccgtgccggtagttttcagcggtccgtcgatgcggtcatggggacgaccgacaaccttcagctgatcgatcgggttttcccctgcgggtttatcaaatttcatgcctgtgccctcgcttcagccagtacggaggcaagcgttcgcttcgccaacaggagtttaaaggtgttttcagcggtgggatgggcgctggcgaacagcgtgtcatatacggcctgcgccccctgggatagctgagcatccgcagcctcaatgcgccagggcttatgtgctactccgcccagcgcgacgcgcccgctgccgtcaggctgaataatcgccgcgaccgataccagggcaaaggcgtaggaggcgcgatcgcgcaccttacggtagatatgttttccgccgagcggtggaggtaacgtcaccgcaacgataagctcaccgggaagcagggcggtttcaatgtgcggcgtttttcccggagggtgataaaaatcagccagtgtgatactgcgagtctttccctccggcgtgatggtttccaccaccgcatccagcaaccgcattgcgaccgccatatcgctcggatgggtggcaatgcaggcttcgcttacgcctaccaccgcgtgctgacggctaaagccttcaagcgccgcgcagccgctcccgggcaggcgcttattgcagggctgattggtgtcgtaaaaataggggcagcgcgtgcgctggagcagattacctgcggtggttgcctgattacgtaactgaccagacgcgccagcgagcagggcgcgggagagtaccgcgtaatcacgacgcacgcgctcgtgagccgccaggtcggtgttccgtaccagtgcgccgatgcgcagcccacccgcgtcggtcacttcaatcttatcgagcccgaggccgttcacatcgataaggtgggtgggcgtttcaatttccagcttcatcaggtccagcagattggtcccgcccgcgataaattttgcgccgggtacgcgctgagcgctaagtgccgcctcggctggggtattcactcgttcataggtaaacgccttcatgattttatctcccccgcagcatcttcaatggcggcaaggatgttagcgtatgcaccacagcgacagatgttgccgctcatacgttcacggatctcatcggcagttgtttctggagcggaaaccaaatcgaccgtgacgtgactgggaatgccgtcctgaatctcttttagcaccgctactgatgagcaaatttgcccggaggtgcagtagccgcactggaagccatcatgcttgataaaggccgcctgcatggggtgaagattatctggcgaacccaggccttcaatggtggtgatctcggccccctgatgcatgactgcaagcgtcaggcaggcattaagcctgcgaccattgaccagcacggtacaggctccgcactgtccgtgatcgcaacctttcttggtaccgatcaaatgcagattttcacgcaaagtgtccagtagcgtggttcgggtatccacctcaagctgctcggttttgccgttcaccttcagtgtcaggggcattatctctggcgcgggtgtagctgccggaacgcttgccgccagcgtagaatgaggataaaccacggcggtcgccgctgttgcggcgctcactttaatcagatcgcgacgggtcaaacttaaatcgtgcggctcgtgcttcccaacccgattatcttcggggtattcgccttggttgctcataccaggcctccggtattctaaaggggaaaataagagtgcgttgcgagagtgctgatgcttttttaaacgttaagcatagtcggcgacagcaggaggattattcttaaaacgcgaatgcagctatgagcccggctaataaattcatgttcgccgggatgttgatgatgatgggagctggtttattgctttagttgtacgatgcaaaaaccaataaggaaacctgtgattttcagctctacatcaccctgcaaatctctgtcacttctaatataaaaatagggagaaatgatggagcttatattcattggcgattaggaaactatcttgttatacaaaacaatacagttctttacatttgccttgttttatgaatactcctgaagaggtgtataacataatggtacaagcagggtagatatgaatatatttgaacaaactccaccgaaccgcagacgttatggtcttgctgcattcattgggctgattgctggcgttgtttccgcattcgtgaagtggggggctgaagttccattgccgccacgtagcccggtggatatgtttaatgcagcgtgtggcccggaatcattaatcagggctgcaggccaaattgattgctcgcgtaattttctcaatccaccgtatatttttcttcgagactggttggggctgacagatcccaatgcggctgtttatacctttgccgggcatgtctttaactgggttggtgttacgcacattatcttttcgatagtgtttgctgtcggttattgtgtggtcgctgaagtatttccaaaaattaaactctggcagggcttactggcaggtgctttagcccaactttttgttcatatgatttcattccctctcatgggactgacgccacctctgtttgatctcccgtggtatgagaatgtttctgaaatttttggacatttagtctggttctggtctattgaaattattcgcagagatttacgaaacagaattactcatgagccagaccctgagatccctttaggctcaaacagataatgcattgaatgataaaaatggcgcaaatacagcgccatttttataggttaaaaacattgctttttatattctgatgcagatagtcagtgagtatatcgcgctacttcaggatgatgtagatccgaagaacgctacagaagagaggcattgttgctggcaaatagaagaagtatcgggttttgttacccctgaaaaacgaagccccgctattatcgctggcggggcagtgcaattaattattgtatgtttataacggtgtcagcccgtatttagcccttgcacgattgcaagcctcattgacgactccgttctcaccagacatggcgaattctctgcatgtggacgatcgatttttatatatcgtgcagcaggcatttttgcccggggttcctgcaagggcaatacatcgggggtttttctgattggtaccgctcatgcatcggtgaaaaggggatatttgttcagtgagcctggcgggaatagtaccgccagcatcgtcggcttcggcccagtaaaaagagacgcggaaaaatgcacaacaggcaccacacgtcatgcatggattcagattgctcataattcaccagtacagctaaaaatcgtaaagagaacagcggtacatcgtatgtaagaacgtaccgcggttggctggggaactttcgatagtgtgagtattgaatgatttccagccgttaccgattttacgtactaattcgtgattaaaccactcgttagcaggctgcctgatacctttccgtgtctcctgaacactatggtgtgcatatgagaaagcccatcgttacaggtgatattgacgatcgcttccacatcatttaaacgatttttggggctctgaggtggaattcttccctcgaccgatggataagtcttagtccgccgaagggggcttagccggacaggaatcgctaatcttaatgaatttgtcgttatagaccagatagtgattccccggctgacgtaactcaggctgatgaaccacgtctcccggacgtagataccaggcatcgccttcctcttcggtcgaatcacatcctggcttaatcagtagcttaaaccatgtgttgccagtgttacttaccgttcctgtcaccttgtcgaaggaccatttaaactgaacctgacgtggtcgtactaccagaatggtatccatcaccaccaccggctccgtgctgaccacgccgccggttgggctgcgtcttgtatggttacgagtggggacctcgcgaaatgagacccggtagtagcgctcgcggttatcccgtggaccatgatagtaaaatttaaaatactcgctctcaccagcctgcaacgccagctggcggggggcgaaaagcagttcaccatccaccggtcgggtgcgcaattcactgctgcccgggctatcaatagcactgatggcaatacggtatatccgtgcgcttttgttgttattcactacacgtttgctgacaaagtcagtctcggacggcagcgaaaatgtcagattgccgaccgaaatcgcctgtgtcaaaggtgccgccagcatacagaccgctgtcagcagggccttagttaatgttacgccacgtcgcctgaacatgaatctctcctgaagcgctgacttcgccaaaccagccgttatcatctaccgtacgcagcgaaatggcgttatccattggaatcgaaaatttgactgtggtcttatccatctgccccacttcgccagagatatcagtccacggtgtggtcaaccacagcgcatcggtcatatcccgccagctatcatcgcacccggcatcgtaggtttttgtagctccgttgcgggtaataaaggaaagtgtcgccgggaacggtactttcgccttaccgtcatcggagctgaagacacaataggagcgcccgccaatcacctgcgcgggtccggtcaccttgatcagcacttcgtcggcagctgttttaccgctggtggttacgatatagccgaaatcgagtgccgactcgccgctgccaacatatccctcccgcgacggtgtctgagtatattcatcggagataatactgatgctgaaatcacggggtttgataatcagcgtgttggaggtagaaaattcataccagccagactccggtgatgtggtgttctgaaagcgaaagttgaatagatctttggtgttgatatcgctgatcccgaggttcaccatctgcttaaagaagttgctcgagaagaaaacatagatcgagtctgcgctcttcatctcgttgaaggtgtagtaataggcggtattgctcaccggtttccatgaactgccattcagactgaactgcatatcgtacgccccgacggccgaggctaacgacgagttggcgatcgccgggaatatatggattgaggtgttgctgagtccgtttgtttgcagggtatagttaaccatcttacaacttaatcctgaacggctgccgatggtttgcgtccggcagtcggcgttcccttcgcccagagtcggtactccgtcgctgttgataaatacttccgccagcgagtgggtatttatcaaccgtagatttgctgctttcgtatgggtgacgttgcgaacataccagttgccggaggcctgatccttacagcgtgcgccgctgctggcgtcatagttcacagaggtctggcaggcattgatggtcattgtaaagctgctgccgacgggcatttgttgcatatactggtaaaacgcgtctgacaacatgccgtgcatccacttcgcgccgccgctggtcaccgtcgcgccataaaatccactggcgtcggtggtttgcggcaggataagactggtggtcatattacacccagcgtaccagttgatgcagcgcaagccagttaaaggagatgaaactggtgaattttccagccacatatcaaacttccagttggtataaaggccggtgttgtaaccgttatcaatgtagccgaggctttgctgatagatggttcctgaaccagtgtattttaaaccggtccagcggttggcaccggtcaggcgcggatccagcgccccgccaggagtgacgaaaaagttgtcgtctgagttgttttcgacaaacacaaactcgcgtgccggtgcatccgcccaggttgttttgctcactgccgctctgagcgcagttactggccagattagcgcgaaaattatcatcgttattagtaggttaactctcattctcttctcctgtctgcgtcaccgccgcccacgatgagaggccgctgcagaccacatcaccgacccagacggcaccgcgcgcctggttgagttccagagccacttcgcaggttttattgccactgtagcgaaaatcgatagtggggtatttcttatccacgtccatgacaaactcgccgttttcatcggttcgggttcggccgatatggttgttaatccgtgcgttagccagcagtgtgccgtcttccgcacggatacgaccggagacggtaaccatctgcttcacctctggctcaatgacagcgacattgcctggatagagagtcagacgacttttgcggccgctgacgatatcgtaactgtcgagtgagtttttgctgttctgtaactccacctcatatcttccatagggagagagcgggagatagttacgcttgccgttaagcgggaaaatccgcccgttgattttggcgctgatctgaccgtcgtcctccagcccggtgttgaatatcaccccagcgttgccatcagtccgcccgctggcagcaatgtttttaccctgccagccgacgctgccattggcggtcaagttggtattgacgtagccgtccgccgcgctattgacgttcagcgttccgctggcgtaacgagcgtcgaattgtgcatacgccccgccgctgagggttttgtcatcaccggtatcgccggagatggcacgtgacagattggcaccaacagtgcgaatggttccttcatcaaactgtttgcgtgctgacaggtttgccatggtgtagccgttttgatgagtcatccctgcgctaaaccagttgcccagtggtagcgagagatcgagagcgatatattttcctgtattggcgttgctgtcgccgttgttatagcgctgaataccggcccgcaggccaagcgaaccaaaggtaccgctgtagacattttgatagtaatctgccgtgtaataatggctgttgtaacggcggtcatcattgtagctgatgctgaatgtgcccagcttcgaccacagtgagttcaggttgagtgtgccgccgattgcacggttgtcggcatcgctacgtcgcaattgattgccaatgcgggttttttcctgattaacccacagcgaactaaagcctcccggtagagtggcgctgatgctgccgatgctgctccatgagctgtcactggccagcatattttgcaggttaacgttgatcgcccccccaagcggcagcgtcagacgggtttcacccaccgcctgattatcgtatccatatcccgttgccgcccagctaagcgtactcaatgagccggaggtcgaggcacctgctagccaactctctttagctggtcgcgtctttttcccgttttccgaccagcgatccatatgaaagctaccgccccatacctgccacgccagtggtgcaccgacgccgcgcccccggctaaacagcttattgacccgctgggtgcgtttgctgatcacgcgaccgttaacgatcacctcaacttccacatcgtaaatcccgtacggtagaccccgggtatccacttcatgattgcccatagtgaagttctgaacgcttagtagccgcccatcacgggtgagatgtacttcgcccgccgccggtaaaaaggcgatcactggcgtggctgactggctgctgtcgaagatggtggagctggcctggtttccccaggaaaggccgtaaatcttccctgctgaaatggcggtcatcggccctaaggactgcaagttccaggtgtcgagcattccaccggcaaatcggtgaccggcaaaatcgcgttcatacatcgctttatataattcactgtcctgttgaccgctaccgatcccgtacagcgagccgtcgagcaccacatgatgttcgcgcagtgcagtaacgttattcagcgacagatagctggatgtgttgctcccgccgttacgcaactggttgttatagacgcccaagttatagctcagattactgctgagggtgttaacactggactgcccgatgtcttcgctacgtgagcgtagtacggtgcccagcgcttcgcgcttgaccactagctgcagcagcagttggcgcaagctgagatccagctgcgcgttgtcagtcagggggatggtaagggcctcattgaacggggcgttggccagagccatcagctgctgtcgagtttgttcgctgacactggcgttatcttcactctcttccagctgtattttccggatgcgtagctgtccatcgtccagccagataaaagcgctgccgattcgctgatcgtcctggcgaccctggctaccggcgagatgaatatagagcgggacgctcatgccgtcctgaagcgcctgactgaaggcctgcggaataatcaccccacctatttgctgcgcacttatgtcagcagcgctggcatcgggctgaacgaacaaaaagaccatgccgaaggcaaactgggctttcagtcctggggagaaccgtcgtaaaggcattgtcgttatccatctgcacagctatctatttcacgggaatgaacttatcaccctgccaaagtgcaacccgtcctttgttatccgcagtgtccacgcgggtaaaacgacgcgacttgcccggcatcaggtagtaattctctttacactccttaccgttggcggctttcaggcaaggtccgtaggcgaggatccgcagcgtcgcatttcctgtatttgtcagggagccgttggcgtactgaaagtggtagttcgcctgacgaggggcgacgaccagaatggtgccgatgcgggcggaagcagtggccacagcgctgcggttggcattatcgcgctgcgcatcactgagggcctgatcaaaccagacaatgcggtagtagcgctctttttcatctgcgggtcccttatagaagaagcggatcacttcgctggcttgggcgggtagcagcaagctggcgggagtgagtagcaactcatccggcttgtccattgagataacctgcccgtcgtcaagcggtgaagagagccgttcgagacggatattgataaggcgaccactgtcggtactgtttttgatcgttttgctcagcgtgctgctgtcactgttcataaacgatgatatatcgccgacatccagcgcctgggccggagatattccggaaaacagcagagcgagaggcagaaggtgctttttcataacaattccgtccaggaataaagcaggggggctacccctgctggtacatcagagagattaactggtccaggtcgcgtcgaactgtacgctaacgtcgccgctccagatgccttccggtagagtgctgtaatctgttactgcggtggtaccattggtggtaccgctgatgatggagaaggtgaaaccatcctgtgcggtggtacgattgctggcattgtaaccgttagccagcgggctaaggttgccgcccagtacgccgttggcggtatcgatcatcacggtatcgccagttttttcgactgccgcgccgttataatccacgcccacattcagtgtggaacctgaggtatccaactgggttaatgtgttggtgataagacgtgaggtcagtttaaaggcggtagccgttgagtcaccctcgatagccacgtcaaatagacctttctgtgagttaaaacctttaatgccttcggcatactggaacgccaggctaccgagtggcgtcacaaccagcttactggtggtgtcttttttggctgttgccgaccaggtcgctacagcctgagctgttacgtcagcagcctgcgccacacccatgccggtaaacaccgttaccagagctattgccagaaccttttttttcattgcatttcttcccgagttgaattgaggacgtgatgtcccagtgagtcattttttaaaactaacttgcctggagtttactgaaccaacttatatatttttgagtacagcttggcctcagcattacgccgatgggtatacactgtcttcacactacaattttcaattctggcaatcgatttaggttgcattccctgggccgtcatgcggataatttccatttcccggtccgtgattttatctttcttaatatcttttctcaggaacctgccattaatcacatagaccagttcttttctaatatcacgactcagtccagcgtataccacgcccctaatattgctattgtaataccaataatttgctaaggcctctgactttctggccgcaatcaatacgacctgtttcccctttaccgcggataaccattcattatcacggtttataaattcagataaagaatccgtactgagattgataaacacgaaatcttttctaattttctccaacgatagataaattaatctgtcgatatccacaatcagttcagatagtcctttatagaagtaggcgtcatggggagaccagatgtatttatcagaacggttttgacattccatatggtttttaacctcatagtccctactgtaatcactttgccatgtcactactttccaaacctgtaatttttacaggtgcattcagtttccttagtaaaccggaagtaaataagatacgtagtacatatcaataaaggttaaacgagattaagtttaattattttcgattgggcttaaatttatgttttttttcccgatgagtgtcaatatgtgaacggaaaaggaattcaatggttaagtcaatatttagaaaaactgaaaatattgcttttttgataagaagaaaaagacatttggtttcataaggttattggcaatataacgttcaattcttacttgcattttatattggtcaggaactttgccctgaagtgttaggaatagtcttaatgcgctgtgtgatggactagtaaaaaaacaagttttaagggtaagggatagaatataaaactatgatgagctgtcattgaagatgatttgccaatcagtaagatattttaatggattaacatgccgcacaaaatggttacaggtgttcattccaataagtaatggaaaattgaacgggcgtatgtacgtcatctgttcggtaagcccccaagagccagattaagtgaagttaaacgaaggctgccagctgtcacaggaacgatggcctttttgtcagggcactgcattcagttatctgtgcgcgttactctaactggcactcgaacgtcggcgacggggttaccggtggatcagactgttcctgtggcgtaaacgtttttatgttagtaccaacagatttaccacatttatcatcttaacagtttgagtgaaaatgcaggctgcgccgcaaagggaggagactgagtggcgtgttcagtctaaaagagggttgatgccagcatacaggggcgaagctggtcaacaagtcaacattaagataatggaatattcggagagaaacgtcaggcagttggcctcaaatgaacaggaagaatatatccccaggaaaattaatgttggtgttataaacacaccaacattaatccgatctgattattaatcagacaaatatcgttaatccgtcgaattttgaatcaacgttttttcttacgaccctgaacggccttaaaacgtggattagatttacaaatcacatatagccgtccttttcgcttcacaatctgacagtctggatggcgttcttttgcggtacgcagagagttaagaactttcatcacgccccctttttcgtgctaacaaaacgaccaaaacgttgggtgaatcgtgcaacatttccttctgatgccactgttctcagcttccctgtatagaacgggtgcgatttagaagagacatcaattgtcacgtatggatacgttacgccatccagctcaatctcacggtctgttttgatagtcgagccgattttaaagtactcatcaacactggtgtcgtggaacaccacagtacgatactcaggatggatattgggcttcatcatttttacctgttatgttataacataaccataaagatacatgctcatccggatcatttcaacactcaatccctgtgactctttgtggatgtggaattttcgcaacggggaactctggcattgttagcagccattggtgacgctcccataaacgcctggatgagtgattgatgatggttttgctgagagtatggatttttcgagaatggaggttatctccactttactggccgataatttatcgcagtatgattgattacctgacagcgtgtattcctctcccacggatataataattacttacaaaaaagggagaggatgcatattttaaatatcactgaagtgaacagtttatttccgttattaatagaaatggagaaataaataggcgtattctacaattgcgacaaaaacaacgatattaatcagtttatgactgatttgctgtactttattctctttcattggtacttcctcgctttaaaaaagagtgcacttcgtaagtgcccttatataaataacgagtttggtcaaccaattttttgacatgtatcacaaatttgaatagatgtattacatcaactatcttttattgcaccaacgtcattgatatatgtcgcctgaagtcagttccgggaatgagtctgatctcaagactggcccagtccgggcgttgattggtgctgaggagcatatcgcatctcatcataatgtcgtatctcctggggtgttatacaagatatcgttgttggtgacctgggagaggaattgagttctattaaaccgtcaactatgccggatacatactggattacactgcaggcacgccttatgagagaacgtgccgcagtgacgggttaattatctgaaagaatttgtgaggctgtatcggttactcattgatttgatagttttactctcgggagaataatagatatttaatccattaacggaaaccagccagttcctttcgatgcctgaatttgatcccatagtttatccggaatggttaattcatgaacaagttgtgttatcgttcatgagaagcataacgtaaagggaaaagctcgattagacggcagaatttgtcaggggttatgaacgaaattcataaatctgtttgagtgttgcgatgggtagtgcaagttcgatatctccgcaatttacagtccgatgaaggaaaatgaatatccataaaaaatatattggtttatcctggcatatatacctatttcgacgtatttccaatagttttaattaaaggcaggtcattgttattcactctgaatagtgaattattcactgtccgcagagtaagaaatataacttaggtatctatttaatgacttgcacaaaaagctaaattttcccccataaataaaaatataatcccgcgcccaaccacctgatgagtggctataggcactggatatattaggtggcggtgcactttcttacataaaggtatttccttttctgcggaaaaggaaatcgggaaatccccggtttttctgacaagcagacgccattatttgtgtctgcctatgttcgttaattcgttcatcaggaaattatctcaatgtcacattataaaacaggtcataaacaaccacgatttcgttattcagttctggcccgctgcgtggcgtgggcaaatatctctgttcaggttctttttccactcgctgtcacctttaccccagtaatggcggcacgtgcgcagcatgcggttcagccacggttgagcatgggaaatactacggtaactgctgataataacgtggagaaaaatgtcgcgtcgtttgccgcaaatgccgggacatttttaagcagtcagccagatagcgatgcgacacgtaactttattaccggaatggccacagctaaagctaaccaggaaatacaggagtggctcgggaaatatggtactgcgcgcgtcaaactgaatgtcgataaagatttctcgctgaaggattcttcgctggaaatgctttatccgatttatgatacgccgacaaatatgttgttcactcagggggcaatacatcgtacagacgatcgtactcagtcaaatattggttttggctggcgtcatttttcaggaaatgactggatggcgggggtgaatacttttatcgatcatgatttatcccgtagtcatacccgcattggtgttggtgcggaatactggcgcgattatctgaaactgagcgccaatggttatattcgggcttctggctggaaaaaatcgccggatattgaggattatcaggaacgcccggcgaatggctgggatattcgtgctgagggctatttacccgcctggccgcagcttggcgcaagcctgatgtatgaacagtattatggcgatgaagtcgggctgtttggtaaagataagcgccagaaagacccgcatgctatttctgccgaggtgacctatacgccagtgcctcttacccagcaatagtggacacgcggctaagtgagtaaactctcagtcagaggtgactcacatgacaaaaacagtatcaaccagtaaaaaaccccgtaaacagcattcgcctgaatttcgcagtgaagccctgaagcttgctgaacgcatcggtgttactgccgcagcccgtgaactcagcctgtatgaatcacaactctacaactggcgcagtaaacagcaaaatcagcagacgtcttctgaacgtgaactggagatgtctaccgagattgcacgtctcaaacgccagctggcagaacgggatgaagagctggctatcctccaaaaggccgcgacatacttcgcgaagcgcctgaaatgaagtatgtctttattgaaaaacatcaggctgagttcagcatcaaagcaatgtgccgcgtgctccgggtggcccgcagcggctggtatacgtggtgtcagcggcggacaaggataagcacgcgtcagcagttccgccaacactgcgacagcgttgtcctcgcggcttttacccggtcaaaacagcgttacggtgccccacgcctgacggatgaactgcgtgctcagggttacccctttaacgtaaaaaccgtggcggcaagcctgcgccgtcagggactgagggcaaaggcctcccggaagttcagcccggtcagctaccgcgcacacggcctgcctgtgtcagaaaatctgttggagcaggatttttacgccagtggcccgaaccagaagtgggcaggagacatcacgtacttacgtacagatgaaggctggctgtatctggcagtggtcattgacctgtggtcacgtgccgttattggctggtcaatgtcgccacgcatgacggcgcaactggcctgcgatgccctgcagatggcgctgtggcggcgtaagaggccccggaacgttatcgttcacacggaccgtggaggccagtactgttcagcagattatcaggcgcaactgaagcggcataatctgcgtggaagtatgagcgcaaaaggttgctgctacgataatgcctgcgtggaaagcttctttcattcgctgaaagtggaatgtatccatggagaacactttatcagccgggaaataatgcgggcaacggtgtttaattatatcgaatgtgattacaatcggtggcggcggcacagttggtgtggcggcctcagtccggaacaatttgaaaacaagaacctcgcttaggcctgtgtccatattacgtgggtaggatcataaagtcctcgggtcgttgtccactcttttggcatgtcagcatattcacataccgtaccagcaaaagtttcaaccgtgagcaaatcgaccgattttgttgacggttcaaacgtggaaacgaaatagatatccgtcttaaaattcttcatacatctggctaaatgatgacgtcgtagtttgacttcttcatccggtgatttattcgacacttcaatgtcatatttaaatgagttgccaaaaataggtgtctcaggaaagttgattaatctacactccgtcttttgctgttgacgtattaaaaaagaagggaagatatttgcgagatcccaataatcacggtggcggtattcacggggagagcagccgaataactttttaaattcgcggctgaatgactgctgtgaatcaaaatgcaaagagagtgcaatatcaagcatagatttcgcggtgagccggacaagaatggcggcacgacaaagccttcgtttgcgaatgtattctcccaaaggcacatgcatgaaatttcggaacagaagctggatgttgcgtctgctgtagccagatttctgtgcgatatcttcgattgaaatagggtgctcaagattgcactcaatccactccaggagctgctgtagaatcttctgcctgatcatctcattctccgttaattctttgtcatatcgcacattttcgttataccctgggccctaagtgtatcaaaaatagcaagggcgaaggcaaaagcactggtagcgtctgcttcgttgtccccgaaaatagagaggtttcagtcctacattattaatgaattttttgcataagtgatatcaaaatccacatactactttgaggttacgttttaacgtagactcattgttcatgcctaatggagggactgacagtggaattttccgtatagtctgcttcagagtattgcagatgcccatcaaaaatcgatttctcactgacagataaagaaatggcacaaattagttcgcttgatttgggttatgttggggagtcggtaaaacattttaatcctgaatttgttcgtggttgtcttgctgtaaaaatacatgattgatattaatcatgtattttacctaagacgacaaaaaccttttaacagggagtgatattgatcttcactctgtcatatctccggtaatatggcgtcaggcttcatcatcagaaagggggcctgacgcctgaaaaagtgaacaacagacagtgttcggattatcaatattcagtttttaacgttgaactggattcattactgcgttgtttaagaatttcccgcgccgaatctgccattatcatgactgcacctgccagcatcagagtatctttcaataccaggcgaccagcaccggataaataagggaaaccatgatgagcgtcacccaatgcgggtacccatgcctccggggtggtgattaaaaatgagagtgttaccagcggcgtggtaaatgccatcagtcctcccaataaacctaaccagcgattgacaggattagccaaaaccagcagagcaataatcacctccacgacgccaagaccgttggaaaaaccataggtattattggccgtttgccatgcccttgcttctggtttgtattcgccttcgtgagtcagatactgtttatagtcttccgggtgttcataaaagaacgacattagtggactgtttgcgacgaatggtgtaatgctgtctgcctcgtaagggacaaactttaataacccaatccacataaaaacaattgcaatactcagacgaatcaatgtcaggccaattttatctccccgacttaacaggtgcaggtatttttccattgtgaacatccttatttatacaatactgctgttgcggttgaattattatcaattcgcatcgatgtgactttccaggatgaagcattatattttctggctatatcagcaatggtatcctccagaactgtcggtgatgctgatactgacgagacgctgatatgtttcagaattattttatcatctgcattggtggaaaatgccataacgccagataatagtgttgcaaataaaacagattttttaaacatataaaataccatcaatgaagtgattaagaagttatagagtaacagagaattaataagattcttttctctgagacgccagaatatttgttctggcgtctgattttgagtttatttgactaatgaaaatagatcattgagtgattcgctcatcgacggatgagtaaatatctgatcgcgtaatatgctataaggcagcccggcatccatcaccattttcactatattgatcatctcgtgggagtcaacacacagcagtgatgcccctaacatacgttgggttttattatcaacaatcgcttttaataccccacgagtatcattcatcactctggcacgcggaattgcagctacaggcaatgtcaccacctgaatatcagcaccactctctctggcttgttcttctgtcataccaaccctggacaggggcggtgtcataaatacggaataaggcacatttttccgatcatcagtactacgtttgccttcacccagtaactcatcacgtacaatgcggtaatcatccagtgatatgtaagtaaattgcagcccgccggtaacatctcccatcgcccaaatattgtctgcggtggtatgtaatcgcttgtcaacgacaattgccccgcgctcgtttactgcgataccggcattttctggatgtaacgaagcggtagccggttgacgaccggaagctattaacagtgcatccaccgccagttgggcgtgctcgctatgcacttgcacttgattttcatggtgactgattcgctccacatgggcattgaggataatatcgacgccctgatcgcgtaaaatcgtcgcgatattatcagcaatatcccgatcttcccgaggcaaaaacagcgaagctgcttctaaaatggttaccttgctgccaaaattagcgaacatagaggcgaactcaacgccaatatatccgccgcccaaaatacctaaatgcccaggcaattcttttagattaagtaatccggtgctgtcatatactcctggcgtggtggtaattccaggaattggcggaaccacggtttgtgcaccggtattaataaaaattttctcgccatgaatttccagatttccctcaggccgatgaacacgcaggctatgattattgataaactccgcctggccgtcgatcacgtcgatattgggcatatccgcaagattatgaaaattcttattacgtaaaaaattaaccacttcatttttacgctgtatggcacggacaaaatctgtgtgctgctgtgcgtcatgaaccaatgttttggttgggatgcagccgatattaatacaggtcccgccatacattgcatttgattgttcgatgagagccactcgccaacctgcttttgccagcgtgacggctaatgtttttccagccttgccaaaaccaataatcactgcctgatatttattcatgatgatttcctgtcgaaacgcgttcatttgacatcatgactatagacgcaaaagagcaaataacatttcttcacaacgcttgatattttgtcttatcgtctgatattttctttttcttaatcagaatcacaaaacaaaaatcatgattaactatttgatggtattagattagttatttactaagattgttggtgtttgtaatcaaaaaccactcaggagtctgatatggatgcccttagccgtttgttgatgcttaacgctccacaaggaacgatcgataagaattgcgtgttaggaagtgactggcagcttccacatggtgccggggaattatcggttattcgttggcatgcgttaacgcaaggagcggcgaagctggaaatgccgacgggggagatttttacattacgcccgggaaatgtggtcctgctaccacaaaattcagctcatcgcctgagtcatgtcgataatgaatcgacctgtattgtctgcggcactcttcggttgcaacattcggcgcgttattttttaacgtctttgccggaaacgctgtttttagcaccggttaaccacagcgtggaatataactggctgagggaggcgatcccgtttttacaacaggaatccagatcggcaatgccgggagtggatgcactgtgtagccagatctgcgctacattctttaccctcgcggtgcgtgagtggattgcacaggttaatactgagaaaaacattctcagtttgcttctgcatccacgtcttggtgcggtaatacagcaaatgctggaaatgccaggacacgcctggaccgtcgaatcgctggccagcatcgctcacatgtcccgggcaagttttgcccagcttttccgtgatgtttccggaaccacgccgctggctgtattaacaaagttgcgtctacaaatagcggcccagatgttttcccgggaaacgctccctgttgtggtgatcgctgagtcagtaggctatgccagtgaatcatcttttcacaaggcgtttgtccgcgagtttggttgtaccccgggagaatatcgggaaagggtcagacagcttgcaccctgaataaaaccgccagaaatcagggcaaagataatccgcattccgggagttgtgagcctttcaactatttctatttccaacggtggtttgggctttatatattttttctgatggactctagctcagtttttaaataaaaatgcaaactaaattgcttcaattaaataaaatcccgactattacttgatacgtgattattgtcggtgatttttttgtacaccatcagtgtatatctcaataacccctgaataagtagctctgaataggtataagggatgtagccatttttaaatggatttcttatgccaaaaatgatcgtcgatttccccataaaatgtgagcgatgccgaaagaaataaaattagttattgcatttgacgtttggatgaaagattatcatttgtcatacaaatgaggggtggtatgttgctagccaattaaaaaagaacgccatatttattgatgattgatcccccggtgggggggaaacatcgggcataaatgggcatgaagtaatggagtattagttgtgaatgtcaatttctttgtcacctgtattggtgacgccctgaaatcaagaatggcacgagactccgtgctgctactggaaaaactcggctgtcgcgtaaatttcccggagaaacagggatgctgcggtcagcctgcgatcaatagcggttatatcaaagaagcgattccagggatgaaaaatctgatcgccgcactggaggataacgacgatcccattatttcaccggctggctcttgcacctatgccgtaaaaagttacccgacgtatctggcggatgaacctgaatgggcatcacgtgccgcaaaggttgccgcgcgtatgcaggatctcacctcttttattgttaataaattaggggtagtcgatgtaggtgccagtttgcaagggagagcggtgtatcacccatcttgtagcctggcccgtaagctgggagtgaaggacgagccacttacgctgctgaaaaatgtgcgtggactggagctgttgacctttgctgaacaggatacctgctgcggatttggcggcacgttctcggtcaaaatggccgaaatatccggcgagatggtgaaagaaaaggttgcgcacctgatggaagtccgccctgagtatttaattggtgctgacgtgagttgcctgctaaacatcagtgggcgattacaacgggaagggcagaaagtcaaagtgatgcatattgctgaagtgttgatgagccgctgaggatataaagatgtcgatcaaaaccagtaatacagattttaagacacgcatccgtcagcaaattgaagatccgatcatgcgcaaagcggtggcaaacgcgcagcagcgtattggggcaaatcggcaaaaaatggtcgatgaattggggcactgggaggagtggcgcgatcgggccgcccagatacgtgatcatgttctgagtaatctcgacgcttatctgtaccagctctcagaaaaagtgacgcaaaacggcggtcacgtctattttgcaagaaccaaagaagacgctacccgctacattttacaggttgcccaacgcaaaaatgcccggaaggtggtgaaatctaaatcgatggtgaccgaagagattggtgtcaatcatgtgttgcaggatgctggcattcaggtgattgaaaccgatctgggtgaatatattctccagctggatcaagatccgccatctcatgttgtggtcccggcaattcataaagatcgccatcagatccgtcgagtgctacacgaacgtctgggctatgaggggccggaaacgcctgaagcgatgaccttattcatccggcaaaaaatccgcgaagatttcctcagtgctgaaataggtattaccggctgtaatttcgcggtggcagagaccggttcggtatgcctggtgaccaatgaaggtaatgcgcgaatgtgtaccacgctgcctaaaacgcatattgcagtgatgggaatggagcgtattgcccccacgtttgccgaggtagatgtattgatcaccatgctggcgcgcagtgccgttggtgcacgtttgacgggatacaacacctggctgacaggaccgcgcgaagctgggcacgttgatggtcctgaagagtttcatctggttattgtcgataacgggcgttctgaggtgctggcctctgaatttcgggatgtgctgcgctgtattcgctgcggggcttgtatgaatacttgtccggcatatcgccatattggcggtcatggatatggctctatttatccagggccaattggtgcggtgatttctccgctacttggcggctataaagattttaaagatttaccctacgcctgctctttatgcacagcttgtgacaacgtgtgtccggtgcgtattccgctgtcaaaactgattttgcgtcatcgtcgggtgatggctgaaaaagggatcaccgcaaaagcagagcaacgggcgataaaaatgttcgcttatgccaatagtcatccaggattgtggaaagtcgggatgatggccggtgctcatgcggcaagctggtttatcaatggcggcaaaacaccactcaaatttggcgcgattagcgactggatggaagcacgcgatcttcctgaagctgacggagagagtttccgtagttggtttaagaaacatcaggcgcaggagaaaaagaatggataatcgaggcgaatttttgaataacgttgctcaggcactgggtcgcccgctgcgacttgaaccgcaagcagaagatgcgccgcttaacaactatgctaacgagcggcttacccaacttaaccaacagcagcgctgtgacgcgtttattcagtttgccagcgatgttatgttgacgcgctgtgagctgaccagcgaggcgaaggcggcagaagctgcaatacgtctgtgtaaagagctgggagatcagtcggtcgtgattagcggtgacacgaggctggaggaattggggattagcgaacgtttgcagcaggaatgcaatgccgttgtttgggatccggcgaaaggtgccgagaatatctcgcaggcagagcaggctaaagtgggtgttgtgtatgctgaatatggtttaaccgaatcgggaggcgtggttcttttttccgccgccgagcgcgggcgttcattgagcctgctcccggaatattctctttttatcctgcgtaaaagcactatcctgccgcgtgtagcgcaactcgcagaaaaattgcatcagaaagcgcaggccggtgaacgaatgccttcctgcattaacatcattagcggccccagttcaacggcggatattgagcttatcaaagtcgtcggagttcatggcccggtgaaagcggtgtatctgattattgaggattgttgagagagatatgaagtctggacataaacctgaagaaggcatacgaggttgaaaatagcgtttaggacaacctgacttaaccccgttccgtcatggttatgctgctcttctgtaaatatcctggtattaccaatgccaggatatttacagtgaaaaagacaggcatccattcctgaaaacgggttcccttcccggtcattgtcacttcagctttatacaggcactctctatcagaatgttgtttattactgcccagagttttgttggtattcatctaccatttttttgacaaggcaaaacattacagaaattacaatgcttagaaaaaatcccagagccaggcaaatggcagcagggtatttattttttatttctggtgagcttatagttacacagccatcaccgttcggatacaatgaccagttcctggtcaggtatatcatttttgtataaagctcactgttaattgctgaaggcgtttgtatctcatcgagaacttgcctgccattatgatattctgacgcataccatttgataatagaggcctgcacgcgagatatttcctcttcagcagttggtaaagctctcttatctcctgaccattccagccttatttctctgttcttgacatctgggctggtgtgaaaaaatgtagtaattcgctgaataacatcttcagtcattgtagtctgacaggcaaaattattattgctatcacagctaacaagtatacctggcgttgtctggtttatttttaggctgtaaatcacttttatattgtctttattgatatacagaaacaacagcaccatagccatacatatagccataataaaaaggataacacgaatctttttcttcagataaaataaaatctcaatcagatcgatatcctgtttgatttgttcacgcataatatatccagagaataaaatctgtcgcagataaggttgtattaatagtctgtatcaggaatgttcgggttaaatatcagcaaaaagcccgcatcatgaatactggatatgaagcatgagagttacctcagtgtttatataaggattcggtccccctctctggaacggtaactctcaatctgatcggttcctgcgttagttcacatcacgactcattttttcgctctcaccggcatcccatttgccacaaaatatcccgccgtgctcctcggcagcgcttcctgtccacgaatcatatccgctattttctcgccaatcataattgtcgtggcgttcaaattcccggtgataatctgcggcataatcgacgcatccaccacacgcaggccttctaacccgtgtacgcggccttcgccgtcaaccacggacatctcgtcgtaacccattttgcaggtaccgcacggatggaaggcggtttcggcgtggttacgcacgaactcatcgagctgttcatccgtctggcattcgacaccggggctgatttcgcggccacgatactgatccagcgcgggttgatgcatgatctcgcgggtgatgcgaattgcgtcgcggaactcctgccagtcctgctcgtgcgacatgtagttaaacagaatcgccggatgctggtgcgggtcgcgggatttaatccgcacatgcccacggcttggcgagcgcattgagccgacgtggcactggaaaccgtgctctttcactgcattcgagccgttatagttaatcgctactggcaggaaatggtactgaatattcggccacgcaaattcctcacggctgcgaataaatccacctgcttcaaagtggttgctggcaccaacgccagtgccgccaaacagccactccgcaccgattttcggctggttccaccactgcagggcagggtagagggaaaccggttctttgcactcatattgcagatacatctccagatgatcctgaagattttcgccgacgccgggtaattcatgcaccagcggaatatcaaactccgccagcagttcagcgttgccgacgccggagcgttgcaggatctgcggtgaggcaatcgcgcctgcacataacagcacttctttgttggccgttgcgcgggttgggatggtgctgtcgccttccagccattcgacgcccaccgcgcgtttgccgtcaaaaatgatgtgatcggtcatagcgtgagtacgaatggtcaggttaggacgcgatttggcctgatcgagatagccacgcgcggtgctggcgcgacggccctgcggcgtgacggtgcgatccatcggaccaaaaccttcctgctgataaccgttgagatcgtccgtgcgcgggtagcccgcctgcacgcccgcttcaatcatcgcttcaaacagcggattgacgccgggtttggaggtagtgacgctcaccgggccatcaccgccgtgatagtcgttttcacccatatcgcgagtctcggccttgcggtagtagggcaggcagtcgaggtagctccagttctccagaccgggttcttgcgcccagttatcgagatccagcgcattgccacggatgtagcacatgccgttgatcagcgacgatccacccagacctttaccgcgtccgcactccatgcggcggttattcataaacggttcaggttccgtttcataggcccagttgtagcgtttaccctgtagcgggaatgccagggcagcgggcatctgggtgcggaagtcaaagcgatagtccgggccgcccgcttcaagcagcagcacggaggtattcggatcttcagtcagacgggtagcgagaacgttgccggctgagccggcaccaataatgatgtagtcaaattgcaaataaacctcctggttagaatatggactggaatttagccatctcaacctggatggacttcacctgggtgtaactctggagcgtcatcacgccgttctcgcgaccaatgccggagtgtttgtagccgccaacgggcatctctgccggggattcgccccaggtgttgatccagcaaatacccgcttccagctgatgaatgacgcgatgcgcgcggttcaggtccgctgtcacgatgcccgccgccaggccgtagtcggtatcgttagcgcggcgaatgacttcgtcttccgactcgtaggtcagaatggacatcactggcccgaagatctcttcacgcacgatggtcatatcgtcgctgcaatcggtgaacactgtcggtgcaacccatgcgccgttatcgaagccatcgcctttcagtacatcgccgccgcacagtacgcgcgcgccttcctctttgcctttggcgatatagcgcagcacgttatcgcgatgcgggaagctgaccagcgggccgaagttagtttgcggatcgaaaacgtcgcccgcgcgaatgcgctcaacgcgcgccagaattttctgctcaaatgcggctttgcatttcgccggaacgaagacgcgggtgccattggtacacacctgaccggagctgaagaagtttgccatcatggcgatatcggcggcgagatcgagatccgcatcatcgaaaacgatcagcggtgatttaccgcccagttccatggtcacttctttcagggaagaggccgccgagttagccatcacttttttgccgctggcgacaccgccggtaaatgacactttggcaatgcccggatgctcggtcagatattgcccggtctccgcgcccacgcccggcaacacgttaaatacgccgtccggcaggcccgcttcgctgtaaatttcagccagctttaacgcggtaagcggggtaacttcgctcggtttgaaaatcattgcgttgcctgccgccagcgccggggcggatttccacagggcaatctggatcgggtagttccatgcgccaatccctgccactacgcccagcggttcgcggcgggtatacacaaaggacgtttcacgcaacgggatctggctgccttccagcgccgggatcagcccggcgtagtactccagcacgtccgcaccggtaacgatatcgacggttgaggtttccgaatatgcttttccggtgtcgagggtttccagttttgcgagttcgtcattgcgttcacgcagaatatcaacggcccgacgcagaatacgcgagcgctccatggcggtcatcgacgcccagattttttgcccctgctgggcgcttttcacggcgcgatcgacatcctcgcgcccggcggcctgcacggtcgccagcacgttaccgttggccgggttaatggtctcgaaggtgcgaccgctggtggcggaggtataaccaccatgtatataaagctgctgttctgccattcgggacatcacgtctcctcggttaatcggtgggtagatgctgagtgataaagtggcgggtcagggaattagcgcgggttttatccagcggtttgccgctcagagccgcgcgcagccataatccatcaatcagcgcggccaggccgtagcccgcttcctgtgcctgttcgcgcggcaattcgcgacgaaactcgctcaccagattcgacagcaagcggcggctgctgacctgctgtaaacgatagagcatcggctgatgcatactgctggcccagaacgccagccaggctttcatcgccgcactgctcacctgcgtttcatcgaagtttccgccaacaatcgcctgtaatcgctgctctgcactgccctgcggaagtgcatgtaatcgattcaaaaccgcgtcacgcagctgactggtgatatcgcgcatggttgcttccagcagaccatttttgtccctgaaatagtggctgatgatccccgtagaaacgcctgcacggcgggcgatctgcgcgatcgttgcatcgtgcatgcccacttcatttattgcttccagtgtggcgtcgatcagttgtctgcgccggatcgactgcatccccaatttgggcattttcgccactccattcatcagcggtgtttatctattaaagcggttattgattggacgttcaatataaaatgtgtcttaattgttacgaatttgattttaaatagtaacaataacagtggggatactggatgacagacctttcacacagcagggaaaaggacaaaatcaatccggtggtgttttacacctccgccggactgattttgttgttttccctgacaacgatcctgtttcgcgacttctcggccctgtggattggccgcacgctggactgggtttctaaaaccttcggttggtactatctgctggcggcaacgctctatattgtctttgtggtctgtatcgcttgttcgcgttttggttcggtgaagctcgggccagaacaatccaaaccggaattcagcctgctgagttgggcggcgatgctgtttgctgccgggatcggtatcgacctgatgttcttctccgtagccgaaccggtaacgcagtatatgcagccgccggaaggcgcgggacagacgattgaggccgcgcgtcaggcgatggtctggacgctgtttcactacggcttaaccggctggtcgatgtatgcgctgatgggcatggcgctcggatactttagctatcgttataatttgccgctcaccatccgctcggcgctgtacccgatcttcggtaaacggattaacgggccgataggtcactcagtggatattgcagcggtgatcggcactatcttcggtattgccactacgctcggtatcggtgtggtgcagcttaactatggcttgagcgtactgtttgatattcccgattcgatggcggcgaaagcggcactgatcgccttgtcggtgataatcgccacgatctctgtcacctccggtgtcgataagggcattcgcgtgttatcggagcttaatgtcgcgctggcgctgggattgatcctgttcgtattgtttatgggcgacacttcgttcctgcttaatgcactggtgctgaatgttggcgactatgtgaatcgctttatgggcatgacgctcaacagttttgccttcgaccgtccggttgagtggatgaataactggacgctcttcttctgggcatggtgggtggcatggtcgccgtttgtcggcttgttcctggcgcgtatctcgcgtgggcgtaccattcgccagttcgtgctgggcacgttgattattccgtttaccttcacgctgttatggctctcggtgttcggcaatagcgcgctgtatgaaatcatccacggcggcgcggcatttgccgaggaagcgatggtccatccggagcgcggcttctacagcctgctggcgcagtatccggcgtttacctttagcgcctccgtcgccaccattactggcctgctgttttatgtgacctcggcggactccggggcgctggtgctggggaatttcacctcgcagcttaaagatatcaacagcgacgcccccggctggctgcgcgtcttctggtcggtggcgattggcctgctgacgctcggcatgctgatgactaacgggatatccgcgctgcaaaacaccacggtgattatggggctgccgttcagctttgtgatcttcttcgtgatggcggggttgtataaatctctgaaggtagaagattaccgccgtgaaagtgccaaccgcgataccgcaccgcgaccgctggggcttcaggatcgcctgagctggaaaaaacgtctctcgcgcctgatgaattatccgggcacgcgttacactaaacagatgatggagacggtctgttacccggcaatggaagaagtggcgcaggagttgcggttgcgcggcgcgtacgtggagctaaaaagcctgccaccggaagagggacagcagttgggtcatctggatttgttggtgcatatgggcgaagagcaaaactttgtctatcagatttggccgcagcaatattcggtgccgggctttacctaccgcgcacgcagcggtaaatcgacctactaccggctggaaaccttcctgttagaaggcagccagggcaacgacctgatggactacagcaaagagcaggtgatcaccgatattcttgaccagtacgagcggcaccttaactttattcatctccatcgtgaagcgccgggccatagcgtgatgttcccggacgcgtgattgttattgcataaaaccgcgccatgtctgcatatggcgctgtttctcctacctcttgatacgttatatctatacggttaagcccttagtatctattgatgattaccagacaacagataataaaaaagaaaagaactattgcagcccaaaacctacatttgggctgttgcgaatgttcaataagtttagtcttatttaatgtaaatattgctgatcatttgaaatgacgcattattcatgagaaatgtgtatcgtaaatcaactgaaattaacgcaaccatttgttatttaaggtttaattatctgtgtgtgatattttattgaatgttttaaatattgtttttattggcattgctataatattggttatcatttgctgaatggattcagtcttaatgagtgggtttttaagggacaggcatagagtaatgatacgtatgcataaccaacatctttactcattatgtcattgaatgttgacgctatgtgtttatgagggagaggtattttcagttgatctggattgttaaattcatataatgcgcctttgctcatgaatggatgccagtatgtagtgggaaattataaatattgaaatagtccaactacttctttattaccaaaaatgagtatctgaattttaatattgcattcttgcgtgattatctcctgagtttgacttgtgattacctttttaaggtatttagcgtaactgtttttgagcgagcatcagaggtaaagataatcttcttgatagtgatgtgggatgttatacgtatggcatcgctgatgtttatggttaccccttatgtgtgctcaggaatcgacaggtaatcactcatactgaacagcgataaaagataaaggtgtgttcatgaattcatgtgattttcgtgtttttctgcaagagttcggtacaacggttcatttgtcattgcctggtagcgtatccgagaaagaacgactgctactcaagctgctgatgcagggaatgtctgtaacagaaatatcacagtacagaaatcgcagtgcaaagacaatttcacatcaaaagaaacagctctttgagaaactggggattcagagcgatattactttctggcgcgatattttctttcagtacaatccggagatcatatccgccacggggagtaatagtcacagatatattaatgataatcactatcaccatatcgtcacgcctgaagccatcagtctggcgttggaaaaccacgaattcaaaccgtggatccaaccggttttctgcgcgcagactggcgtactgacgggctgtgaggtgcttgtccgctgggaacatccacaaacgggaattatcccaccggatcagtttattcctctggcggagtcatccggtcttattgtcataatgacccgccaactgatgaaacagactgcggatattctgatgccggtaaaacatttgctgccggacaatttccatattggcatcaacgtctcggcgggttgttttttggcagcgggatttgaaaaagagtgtctgaacctggttaataaattaggtaacgataaaatcaagctggttctcgagctaacggaacgtaaccctattccggtaacgccagaagccagagcgatatttgacagccttcatcagcacaacattacctttgcgctggatgactttggtacgggttatgcgacctatcgttacttgcaggcgttcccggtcgattttattaagatcgataagtcatttgtgcaaatggcgagtgtcgacgaaatctccggtcatattgtggacaatattgtcgaactagcgcgtaagcctggtctgagtatcgtggcggaaggggtagaaacccaggagcaggcggatttaatgatcggtaaaggcgttcactttttgcagggctatttgtactctccgccagtaccgggtaataaatttatctctgaatgggtaatgaaagcaggtggttgatgtaaaccgctattcacagcgcatcgggaggttggcagcgattaattctcccgatgcagtaaatcctgatagatccccgttaatatgccatttggcgcaaattgttttttaatccactgcgtcacctgacccgtagcagaatgctgagtcgccagtaacatgcgcgaatcctggcgcggattatggatttgtcgggtaaccagcagggattgcgtcatcgcctcacggaccatgtaatccggcaaaaaaccaattccttcacctaaaatctggcactgacatttggtgttgaaatctggcaccagaattgactcctgcccgtgcagcaaccagcccacttttttattaatcgtatgcgcggtgtcctccaccataatattagggtagagacgcagttggctttcggcgatgggttccggcacaaaggctaacgggtgatccggggcgatagcaaaagcccagcgaatcgcgccaatttcagtgtaatcaataccgccgccgtccagtagtgtatcgggtgcgccgatggcgatattggcctgattattaataatcgcatcccagacgccgttatacacttcggtggtgacggtaatctggcaggtaggaaactgctttttcagcacctgtaacaagcgtgcggtgtgtttgggcgtataaagcagctgattaatacaaatgcgcacacgcgcttctatgccctgcgaaatagtatcgattctgcgtttgatggcataaaaatcattcagcaggtcggtagctttgcggaaaaaataacgcccggactccgttaactcaatgctgcgggtactgcgagtgaacagcaccacatccagccccgtctccatacgcttaatggtgtagctaatggcggaagtggttaaacccaactcttctgcggctttactgaagctgccaaaacgcgcagcggtagtaaatgccaacagattctcttcggtaaaaattgagttcattaaaccattctcgccattatctactatgaatttctccagctatgactgtagaggtatcggttaaagatagataatcatttttgaataacttttaatacccgtcgcgtttagtcgtcgcttcgcttaatttttgtccaccatattctgaaattacccccacgcagttacccgccagaaaacccagtaacgtcaccgtccagttcatcccgctggcaaaaaacagcgtcatgccgagaaagccaccgggaataaaggacagtaaccagaaacgcccttgccagaccactaccgccgagaagggtacggtagtaattacgctcgcccagaacgcggacagtccacttacagaggccagccaaccagcagtcagcgcggcgaaaaacgcccacaccatcccggaataattaaccgccagacttctgataaaccccgatttaccgccgcctgcggcataaaaactgcaaaaggcgacgaagccaatggttcctaataattcccatccttgagagagcccgacatgtgaagacactaactgccaaagccctgcacaaataccgacggtgacacccgttgccgtgagtccgttcatcttgttcccctctggttagacatggacgaaagctactcttacatgtgcagactatagagaaataaaacctgattgagtgaaagggtatcgggtcaaagaaacaaatattgcactaccgcacactgcgaaaagattgttgaatattattcaacaaaaaggcgagatacggcgaattaaatttaagcgggttcttttatcagattatcgttgctattctcaattcatcgaaaacagccacaaaaaccaggggaatgtgaatgagtataaaaaatctacctgccgactatttattggctgcacaacagggtgatatcgataaagtaaaaacctgccttgcgctgggtgtcgatattaatacctgcgatcgtcaggggaaaacggcaattacgctggcaagtttatatcagcaatatgcttgcgttcaggcattaattgatgccggagcggatattaataagcaagatcatacctgtttaaatccttttttaattagctgtctgaacgatgatttaacgctactacgaattattttaccggctaaacccgatcttaattgcgtaacccgttttggcggtgtcggcctgacgcctgcctgtgaaaaaggccatttaagtattgtaaaagagcttttggcgcatacggagattaacgttaaccagaccaaccatgtaggctggacgccgctactggaagcgattgtgcttaatgatggtggtattaaacagcaggcgattgtgcagttattgctggaacacggtgccagcccgcatctgaccgataaatatggcaaaacgccactggaactggcgcgggaacggggctttgaagagattgcgcagttactgattgccgcaggtgcataaaccgggaggcttgctatcaacacaccagaaagacggtgtgtgtgggcgctaactgcggatgcggattttctggcgcagcgggggcaaggacaggttgaacaggtctttgccagagcggtaaatatcgcactcccggctcgccagcagttgctgacgctgctttgtgaagagtacgacaatgcgccaaacagttgtcggttggcactcactcactttgatgatctgttccggcatggtgataaggttcagtttgacgatcaaggtattacggttggtcaacatcttcatatagagatgagtcgttgtcggcgttggctgtccccaaccttgcaaatgaccgctgtgaattttcaccttatcgcctggctacagtggcacgacattattcatcagcacctgggggaaaatgaaaccctgtttaattatcgcggcgataatccgttttatcaggcgttaaataaagaattacatattaaacgacgggcagttattcaggccgtaaacgataaacaaaatatcgcctcagcggtcgccagtatgatggggttagggattggccttacgccatcagccgacgattatttaacaggtctggcgcttattttatttattcccgggcatccggcggaaaaatacaaagaggaattttatctcggtctgcaacgcggcaaaaataataccacattattaagtgccataacgctggaagccgcattacaacaacgctgccgggaaaatattcatcgttttattcacaacattatttatgacatccctgggaacgcaactcaggcaatagaaaaaattaaacatattggctccagttccggctgcgacatgctgtatggcatggccgatggttgtgcgctgagccaaacctacggagggaattatgtcagttaaaatagtcattaaaccgaatacctattttgattctgtctcgctgatgtctatctccacgcgtgcaaataaactcgacggcgtcgagcaggcatttgtggcgatggcgaccgaaatgaataaaggcgtgctgaagaatttaggactgctgacgccggagctggagcaggcgaaaaacggcgacctgatgattgtcatcaatggtaaatcgggtgcggacaacgagcagttactggtggagattgaagaactgttcaacaccaaagcgcaaagcggctcgcacgaggcgcgttacgccactattggcagcgccaaaaagcatatcccggaaagtaacctggcggtgatttcggtcaacggtctgtttgccgctcgcgaagcgcgtcaggcgctgcaaaacgatctcaacgtgatgctgttttccgataacgtctcagttgaagatgaactggcgctcaagcaactggcccacgaaaaagggctgctgatgatggggccagactgtggcacggcgattatcaacggcgcggcgctctgttttggtaacgccgtgcgtcgcggcaacatcggtattgttggcgcatccggcaccggcagtcaggagttgagcgtccgcattcatgaatttggcggcggcgtttcgcaactgattggcaccggcgggcgcgacctgagcgagaaaatcggcggcctgatgatgctcgacgccatcgggatgctggaaaacgatccgcaaactgaaatcattgcgcttatctccaaaccgcctgcgcctgcggtggcccgcaaagtgctggaacgtgcgcgcgcctgccgcaagccggtggtcgtctgcttcctcgatcgtggcgaaacgccagtggatgagcaggggctacagtttgcccgcggcaccaaagaggcagcgctaaaagcggtgatgctctccggcgtgaaacaggaaaatctcgacctgcatacgcttaaccagccgttgattgcggatgtgcgtgcgcgtctgcaaccgcagcagaaatacattcgtggcctgttctgcggcggcacgctgtgcgacgaaaccatgttcgcggtgatggaaaaacatggcgatgtctacagcaacattcagcccgatccggaattccgcctgaaagatatcaaccgcagcatcaaacacaccttcctcgactttggcgatgacgacttcaccaatggcaagccgcacccgatgattgaccccaccaaccgcatcagtcgcttgatcgaagaggcgcgcgatccagaagtggcggtgatcgtgatggattttgtgctcggatttggatcgcatgaagatccggtcggctccaccatcgagacgatcaaagaagcgaaagcgatcgccgctgccgaaggacgcgagttgatcattctcgcctatgtgctgggtaccgatcttgatacgccatcgttagaacaacaaagccagatgctgcttgatgccggagtgattctggcgagcagcagcaccaataccggattgctggcgcgtgaatttatctgcaaaggggaggaagcctgatgagccagtcactgtttagccaaccattgaacgttattaacgtcggcatcgccatgtttagcgatgacctgaaaaagcagcatgtagaagtgactcaactcgactggacgccgccggggcagggcaatatgcaggtggtgcaggcgctggataacattgccgattcgccgctggcggacaaaatcgccgccgctaaccagcaggcgctggagcgtattatccagtcgcatccggtgctgattggttttgatcaggcgattaacgtggtgccgggcatgacggcgaaaaccattcttcacgccgggccgccgatcacctgggaaaaaatgtgcggcgcgatgaaaggcgcggtcaccggagcgctggtgttcgaaggactggcgaaagatctcgacgaggcggctgaactggcggcttccggggagatcaccttctcgccgtgtcacgagcacgactgcgtgggatcgatggcgggtgttacctcggcctcgatgtttatgcacatcgtaaaaaacaaaacctacggcaacatcgcttataccaacatgagcgagcagatggcgaagattttgcgtatgggcgctaacgaccagagcgtgattgaccgcctgaactggatgcgtgatgtgcagggaccaatactgcgcgacgcgatgaaaattatcggcgaaatcgatctgcgcttaatgctggcgcaggcgctgcatatgggcgatgagtgccataaccgcaataacgccgggacgacactgctgattcaggcgctgacgccggggattattcaggcgggttattccgtcgagcaacagcgcgaagtgtttgagtttgtcgccagcagcgactacttctccggcccgacgtggatggcgatgtgtaaagcggcgatggatgcggcgcatggcatcgaatacagcaccgtggtcaccaccatggcgcgtaacggcgtcgagttcggcctgcgggtcagcggcctgccggggcaatggtttaccggcccggcgcagcaggtgatcggcccgatgtttgccggttataagccggaagattcggggctggatatcggcgacagcgccatcaccgaaacctacggtattggcggatttgctatggcgaccgcgcccgctatcgtcgcgctggtgggcggcacggtggaagaagctattgatttctcccgtcagatgcgcgaaatcaccctcggtgaaaaccccaacgtcaccattccgctgctcggttttatgggcgtgccgtcggcaatcgacatcacccgcgtgggtagcagcggcattctgccggtgatcaacaccgccatcgcccataaagatgcgggcgtcggcatgattggcgcgggcattgtgcatccaccttttgcctgcttcgagaaagccattcttggctggtgcgaacgttacggcgtctgacctacatgttcatgccggatgcggcgtgaacgccttatccggcctacgaatggcgcaagaatctgtaggcctgataagcgtagcgcatcaggcatttgtcaccattgccggatgcggcgtgaacgccttatccggcctacgaatggcgcaagaatctgtaggcctgataagcgtagcgcatcaggcatttgccaccactgccggatgcggcgtggacgccttatccggcctacgagtggcgcgagaatctgtaggcctgataagcgtagcgcatcaggcatttgtcaccattgccggatgcggcgtgaacgccttatccggcctacgagtggcgcgagaattgtaggcctgataagcgtagcgcatcaggcagtctggcgttggtcataaccccatcaccctctgtagcggacataacaacatgaaagagcttgtggtcgttgccattggtggcaacagcattatcaaagataacgccagccagtcgattgagcatcaggcggaggcggtgaaagccgtcgccgatacggtgctggaaatgctggcttccgattacgacattgtgctgacccacggcaacgggccgcaggtcgggctggatttacgccgtgcggagattgcccacaagcgcgaagggctgcccttaacgccgctggcgaactgtgtggcagatacgcagggcggcatcggctatctgatccaacaggcgctgaataaccggctggcgcgtcacggcgagaagaaagccgtcaccgtggtgactcaggtggaagtggataaaaacgatccaggttttgcccatcccaccaagcccatcggcgcattctttagtgacagccagcgtgacgaattacaaaaggcaaaccctgactggtgttttgttgaagatgccgggcggggctatcgccgcgtggtcgcctcgccggaaccgaaacgtattgtcgaagcacctgccattaaagcgctgatccaacaaggttttgtcgtaattggcgcgggcggcggtggaattccggtagtgcgtactgacgcgggagattaccaaagcgtggacgcggttatcgacaaagatctctctaccgcgctgctggcccgtgaaattcacgccgacattcttgtgatcaccactggcgtcgaaaaagtgtgtattcactttggcaaaccgcagcagcaggcgctcgatcgggtggatattgccaccatgacccgctatatgcaggaagggcatttcccgcccggcagcatgttgccaaaaatcatcgccagcctgacatttttagaacaaggcggcaaagaagtgattatcaccacgccggaatgcctgcctgcggcgctgcgcggcgaaacgggcactcatattattaaaacgtaaggacgtaagatgaaagaaagcaatagccgccgtgaatttctgagccagagcggtaagatggtcaccgccgccgcgctgtttggtacctctgtgccgctcgcccatgcggcggtagctggcaccctaaactgcgaagcgaacaacaccatgaaaatcactgacccgcattactatctcgataacgtgctgctggaaaccggttttgactacgaaaatggcgtggcggtgcagacccgcacggcgcgccagaccgtggagattcaggacggcaaaattgtcgccctgcgcgagaacaagctgcatccggacgccacgctgccgcactatgacgctggcggtaagctgatgctgcccaccacccgcgacatgcatattcatctcgacaaaaccttttacggcgggccgtggcgctcgctcaatcgtccggcaggcaccaccatccaggacatgatcaaactcgagcagaaaatgctgccggaactgcaaccgtacactcaggagcgggcagaaaaactgattgatttattgcagtcgaaaggcaccaccattgcccgcagccactgcaatatcgaaccggtttccggcctgaaaaatctgcaaaatttgcaggcggtgctggcgcgacgtcaggcgggctttgagtgtgaaatcgtcgccttcccgcagcacggtttgctgctgtcgaaatctgaacctttaatgcgtgaagcgatgcaggcgggggcgcattacgtcggcggcctggacccgaccagtgttgatggcgcgatggaaaaatccctcgacaccatgttccagattgcgctggactacgacaaaggcgtcgatattcacctgcacgaaaccactccggcaggcgtggcagccatcaattatatggttgaaacggtagagaaaacgccacagctgaagggcaagctgaccatcagtcacgcctttgcgctggcaacgctcaacgagcaacaggtagatgaactggcgaaccggatggtggtgcaacaaatttctatcgcctcgacggtgccgattggcacgctgcatatgccgctcaaacagttgcacgacaaaggcgtaaaagtgatgactggcactgacagcgttatcgaccactggtcgccttatggtctgggcgacatgctggaaaaagccaatctgtacgcgcagctctatattcgtcctaacgaacagaacctctcccgctcgctgtttttagccactggcgatgtattgccgctgaatgaaaaaggcgagcgtgtatggccaaaagcgcaggatgacgccagctttgtgctggtggacgcctcctgttccgccgaggcggtggcgcgtatctcgccgagaaccgcaacgttccataaagggcaactggtgtgggggagtgtggcaggttgatgcgcatttgaaacgcctgcaacggtgaatagtaagagatttaagccccagggagtggggcaatctgaatatgagtgtgtcggcagaaatggacattatctttgaggaatatgcccttattgacgttgtgtagataactatttgtctacgtgaaaagatcatcagttttgccgattttagtcttttacagatagcaaatatcacacttacaggcgctcgccttatggggaacgttgctgctctgtttcattcaggctcgcggcatgttggggctggatcgggtggtttaaatattggctatattcaatggacgcgttttgccgcgatgacatatcaggcgttgccaaatacacatagctaatcaggagtaaacacaatgaagatcaaagctgttggtgcatattccgctaaacaaccacttgaaccgatggatatcacccggcgtgaaccgggaccgaatgatgtcaaaatcgaaatcgcttactgtggcgtttgccattccgatctccaccaggtccgttccgagtgggcggggacggtttacccctgcgtgccgggtcatgaaattgtggggcgtgtggtagccgttggtgatcaggtagaaaaatatgcgccgggcgatctggtcggtgtcggctgcattgtcgacagttgtaaacattgcgaagagtgtgaagacgggttggaaaactactgtgatcacatgaccggcacctataactcgccgacgccggacgaaccgggccatactctgggcggctactcacaacagatcgtcgttcatgagcgatatgttctgcgtattcgtcacccgcaagagcagctggcggcggtggctcctttgttgtgtgcagggatcaccacgtattcgccgctacgtcactggcaggccgggccgggtaaaaaagtgggcgtggtcggcatcggcggtctgggacatatggggattaagctggcccacgcgatgggggcacatgtggtggcatttaccacttctgaggcaaaacgcgaagcggcaaaagccctgggggccgatgaagttgttaactcacgcaatgccgatgagatggcggctcatctgaagagtttcgatttcattttgaatacagtagctgcgccacataatctcgacgattttaccaccttgctgaagcgtgatggcaccatgacgctggttggtgcgcctgcgacaccgcataaatcgccggaagttttcaacctgatcatgaaacgccgtgcgatagccggttctatgattggcggcattccagaaactcaggagatgctcgatttttgcgccgaacatggcatcgtggctgatatagagatgattcgggccgatcaaattaatgaagcctatgagcgaatgctgcgcggtgatgtgaaatatcgttttgttatcgataatcgcacactaacagactgaaaaaattaataaataccctgtggtttaacatattaacttcgctctccacttaactttttagttaaggagagcgaaataatatcaaagtagcagtaaaacctataacgtaaatttaaattgttaaattaacgccctccagtacacaatacttcacacgttagttatgagcgatttctgatagtgcctggtttaatcagagctttattatctgcgacgtttatttttatttaagagagatcgcgatgatatcattaaaagctccgcacaataatttgatgccatatacgcaacaaagcatacttaatacggttaaaaacaatcagttaccagaggatatcaaaagctccctggtttcctgtgtcgatatattcaaggttttgattaaacaatattatgattatccttatgattgtcgtgatgatttagtcgatgacgacaaactcattcatctcatggctgccgtacgagactgtgagtggtcagacgataacgcactcaccataaatgtgcagtttaatgatttccctggattttatgactggatggattaccctgatcacccggttaagtttgtttttcacatacttgaaaatcaaaaagggacagtttgggtatatgaccaggatgatgcgtttcttgatattaaagcaaacgtgcaggctggacgctttaccgggcttaagaaattagtgcagtttatcgattcagtgcgaacagattgcaaatgtattcttcttgaataccatatgcctttgctgagaattttccctaaagggaaagagtgtatgcatgtggaaaaatggcttcgcgaaatgtcgtctattccggagacagacgcgcccattaagcaggcgcttgcgcatggattattattacacttaaaaaatatctaccctgtttttcctgaatcactggtgatgttattgctctctgttctggacgtaaaaacatacagagatgatgcgcgattaaatgaatggatatctaatagagtgcaggaattaggtgacagatattatcctgtaaataagcacgttaaaatccgctacactctttagttcagaaagggttccacctgcaagttgttattccacctgagagtgaatcgcaatgcaggtaatcatttcatctgtatatctgtatgccaactggcattccatctcttttttcgccgatattttgttgtgatcggcgacacttcgcttaaaaaagcaccagtagtggtttcgcagccatgcggtgtataaaaaatgatctcatgcagatgttttgtgaatgtgttggttgacattcatatgaaaaaaatcataattccatcatgtttgtgtggggtcttttctgtatcttacgcatcgcactcaagcctgacagaaaatatgctgtaaggctcatatcaaaaaccgccattagctcatcaggaagagcagacgacaaccaggattgttgtatggtacggggttcgaggcctcgatggcggtccaacttttcaaaactcttctgaatcagatccccttattatcatccctgcaaagtggaacattgccattgtttggctattcaggatggggcagaccaatgaaaaaagcccacacaggggagagtgggctgaaatgggaagctaaagactcaagtaaacttatcggaaataaggaccacgcattacgggggctatcatcgccgatggccgtgattcggcaaatcaggttgattacgtagagagtaaattatctgctcaccgctgcgtcaccccttcgtaaatcaggcgtagcgcgaatacaccaataattgcaccaataacccgactggcaacgcgttgcatacgcccataagcacgacgcacagcgggcaaagaaaacgcctgactaagaaaaactcgccagataattgatgcgagcacaatccccgcccaggccattaaacgtgcccatgttggtgtttcggcatttaatgttactgagaaaatactgataaaaaataaaacggtttgcgggttagagagatcggtaattaatccgcggcgaaaaaagacataccagggggcgctaatcggttgttgtagtgtgctcatttgcggtgttgactggcggcgcatgctgcaccacgcaaaccataagagataagcgccgccgacgattctgataagcgaaaaaatctcctcacactgcgtaattagcgttgcaagaccaaacaaacccaacccggaataaaatgcatcgcccagcgccacgcccagcccggtcagcacccctgcgcgtcgaccggaagccaggctggtttgtactaccacaaagagattggctcccggattaaaaaaagtaatcacgaacagtcctacggtcaggtaaacggcatgcaaaggatccatagtgatttcatccataaataagtgaactaactgcatcatatttctaccaaaaataatcgggtgcgagagagatcacaaagtgtcttatttccggttactggcgtttatgccctgactgaactaattattaatcaacccaataatgtgggtgggtgatagtgtgataacaactctggagccgtaatatgaaaataatctctaaaatgttagtcggtgcgttagcgttagccgttaccaatgtctatgccgctgaattgatgaccaaagcggaatttgaaaaagttgaatcgcagtatgaaaaaataggtgatatttcaaccagcaatgaaatgtcgactgcagatgcaaaagaagatttgatcaaaaaagcggatgaaaaaggggctgatgtgttggtactgacctccggtcaaactgacaataagatccacggcacggcaaatatttataagaagaagtaattctgaatcctatgtaaacatctccgatgcgtaagtttatcggtgatcatctattgaaatttatgccggataaagcgttcgcgctgcattcggcagttcagcttttcagccgccgccagaacgtcgtccggctgatgcctaaataattcgccgctgctgttttatcgccattaaatttctccagtgcctgttgtggtgtcagtaagcgtggagcgggagttttcgccgactcgcgcgccagttccggcagtagcagttgcataaactgcggcgttaaatccggcgtcggttccacacttaaaaacagcgccagtcgttccatcatattgcgcagttcacgaatattgcctggccagtcgtagtgcagcagcacagtttcacttgcctgtaacccctggcgtaatgcagcagaaaatggggcggagagcgccgccagagacactttcaaaaagctttccgccagcggaagaatatccgccacccgctcgcgcagtggtggcaattgcagacgcaaaatactcagccgataaaacagatcacggcgaaaacgtccttgctgcatatcttcttccagattgcagtgagtggcgctaatgacccgtacatctaccggaacaggctgatgcccgccgacgcgggtgacctctttttcttccagcacccgcagcagccgggtctgcaaaggtagcggcatttcgccaatctcatccagaaacagcgtaccgccgtgggcaatttcgaacagcccggcgcgacctccgcgtcgcgagccggtaaacgccccttcctcatagccaaacagttctgcttccagcagcgattcggcaatcgccccgcagttgacggcaacaaacggatgcgactttttgccctgtcgcgcatcgtggcgggcaaaatattcccgatgaatcgcctgggccgccagctctttgcccgtccccgtttccccctcaatcaacaccgccgcactggagcgggcatacagcaaaatagtctgccgtacttgttccatctgtggtgattgaccgagcatatcgcccagcacgtaacgagtacgcagggcgttgcgggtggcatcgtgagtgttatggcgtaacgacatgcgcgtcatatccagcgcatcgctgaacgcctggcgcacggtggcggcggaatagataaaaattccggtcattccggcttcttctgccaaatcggtaatcagccctgcgccgaccaccgcttcggtgccgttagcttttagctcgttaatctgcccgcgtgcgtcttcctcggtaatgtagctacgttggtcgaggcgcaaattaaaggttttttgaaacgccaccagcgctggaatggtttcctgataggtgacaacgccgatagaagaggtgagttttccggcttttgccagtgcctgtaacacatcgtagccgctcggtttaatcaaaataactggcactgacaggcggcttttcaggtacgcgccgttagagccagccgcgatgatggcgtcacagcgttcgtttgccagtttcttgcggatgtaggtcactgctttttcaaagccaagctgaataggggtaatgttcgccaggtgatcaaactcgaggctgatatcgcgaaacagctcgaacaggcgcgttacagataccgtccagataaccggtttgtcgtcattaagccgtggtggatgtgccatagcgcaccgcaaagttaagaaaccgaatattgggtttagtcttgtttcataattgttgcaatgaaacgcggtgaaacattgcctgaaacgttaactgaaacgcatatttgcggattagttcatgactttatctctaacaaattgaaattaaacatttaattttattaaggcaattgtggcacaccccttgctttgtctttatcaacgcaaataacaagttgataacaaaggatgggctatgtctctacactctccaggtaaagcgtttcgcgctgcactgactaaagaaaatccattgcagattgttggcaccatcaacgctaatcatgcgctgttggcgcagcgtgccggatatcaggcaatttatctttctggcggtggcgtggcggcaggttcgctggggctgcccgatctcggtatttctacccttgatgatgtgctgaccgacattcgccgtatcaccgacgtttgttcgctgccgctgctggtggatgcggatatcggttttggttcttcggcctttaacgtggcgcgcaccgtgaaatcgatgattaaagccggtgcggcaggattgcatattgaagatcaggttggtgcgaaacgctgcggtcatcgtccgaataaagcgatcgtctcgaaagaagagatggtggatcggatccgcgcggcggtggatgcgaaaaccgatcctgattttgtgatcatggcgcgcaccgatgctctggcggtagaggggctggatgcggcgatcgagcgtgcgcaggcctatgttgaagcgggtgccgagatgttgttcccggaggcgattaccgaactcgccatgtaccgccagtttgccgatgcggtgcaggtgccgatcctcgccaacatcaccgaatttggtgccacgccgctgtttaccaccgacgaattacgcagcgcccatgtcgcaatggcgctgtacccactttcagcgttccgcgccatgaaccgcgccgctgaacatgtctacaacgtcctgcgccaggaaggcacgcagaaaagcgtcatcgacaccatgcagacccgcaacgagctgtacgaaagcatcaactactaccagtacgaagagaagctcgacaacctgtttgcccgtagccaggtgaaataaaaaacgcccgttgattgtattcgacagccgatgcctgatgcgtcgctgacgcgacttatcaggcctacgaggtgcactgaactgtaggtcggataagacggatggcgtcgcatccgacaaccgatgcctgatgcgccgctgacgtgacttatcaggcctacggggtgcactgaactgtaggtcggataagacgcatagcgtcgcatccgacaaccgatgcctgatgcgccgctgacgcgacttatcaggcctacggggtgcactgaactgtaggtcggataagacgcatagcgtcgcatccgacaaccgatgcctgatgcgccgctgacgcgacttatcaggcctacggggtgaactgaactgtaggtcggataagacgcatagcgtcgcatccgacaacaatctcgaccctacaaatgataacaatgacgaggacaacatgagcgacacaacgatcctgcaaaacagtacccatgtcattaaaccgaaaaaatctgtggcactttctggcgttccggcgggcaatacggcgctctgcaccgtgggtaaaagtggcaatgacctgcattaccgcggctacgatattcttgatctggcgaaacattgcgaatttgaagaagtggcgcatctgctgatccacggcaaactgccgacccgtgacgaactcgccgcttacaaaacgaaactgaaagccctgcgcggtttaccggctaacgtgcgtaccgtgctggaagccttaccggcggcgtcgcacccgatggatgttatgcgcaccggtgtttccgcgctcggctgcacgctgccagaaaaagaggggcataccgtctctggcgcgcgggatattgccgacaaactgctggcgtcgcttagctcgattctcctttattggtatcactacagccacaacggcgaacgcatccaaccggaaaccgatgacgactccatcggcggtcacttcctgcatctgctgcacggcgaaaagccatcgcaaagctgggaaaaggcgatgcatatctcgctggtgctgtacgccgaacacgagtttaacgcctccacctttaccagtcgggtgattgcgggcaccggctctgatatgtattccgcgattattggcgcgattggcgcactgcgcgggccaaaacacggcggggcgaatgaagtgtcgctggagatccagcaacgctacgaaacgccggacgaagccgaagcagatatccgcaagcgcgtggaaaacaaagaagtggtcattggttttggtcatccggtttacaccatcgctgacccgcgccaccaggtgattaaacgtgtggcgaagcagctctcgcaggaaggcggctcgctgaagatgtacaacatcgccgatcgcctggaaacggtgatgtgggagagcaaaaagatgttccccaatctcgactggttctctgctgtttcctacaacatgatgggcgttcccaccgagatgttcacaccactgtttgttatcgcccgcgtcaccggctgggcggcgcacattatcgaacaacgtcaggacaacaaaattatccgtccttccgccaattatgttggaccggaagaccgcccgtttgtcgcgctggataagcgccagtaaacctctacgaataacaataaggaaacgtacccaatgtcagctcaaatcaacaacatccgcccggaatttgatcgtgaaatcgttgatatcgtcgattacgtcatgaactacgaaatcagctctaaagtggcctacgacaccgcacattactgcctgctcgacacgctcggctgcggtctggaagctctcgaatacccggcctgtaaaaaactgctggggccaattgttcccggcaccgtcgtacccaacggcgtgcgcgtccccggaactcagttccagctcgaccccgtccaggcggcatttaacatcggcgcgatgatccgctggctcgatttcaacgatacctggctggcggcggagtggggccatccttccgacaacctcggcggcattctggcaacggcggactggctttcgcgcaacgcggtcgccagcggcaaagcgccgttgaccatgaaacaggtgctgaccgcaatgatcaaagcccatgaaattcagggctgcatcgcgctggaaaactcctttaaccgcgtcggcctcgaccacgttctgttagtgaaagtggcttccaccgccgtggtcgccgaaatgctcggcctgacccgcgaggaaattctcaacgccgtttcgctggcgtgggtggacggtcagtcgctgcgcacctatcgccatgcgccgaacaccggcacgcgtaaatcctgggcggcgggcgatgccacttcccgcgcggtacgtctggcactgatggcgaaaacgggcgaaatgggttacccgtcagccctgactgcgccggtgtggggcttctacgacgtctcctttaaaggtgaatcgttccgcttccagcgcccgtacggttcctacgttatggaaaatgtgctgttcaaaatctccttcccggcggagttccactcccagacggcagttgaagcagcgatgacgctctatgaacagatgcaggcagcaggcaaaacggcggcggatatcgaaaaagtgaccattcgcacccacgaagcctgtattcgcatcatcgacaaaaaagggccgctcaataacccggcagaccgcgatcactgcattcagtacatggtggcgatcccgctgctattcgggcgcttaacggcggcagattacgaggacaacgttgcgcaagataaacgcattgacgccctgcgcgagaagatcaattgctttgaagatccggcatttaccgctgactaccacgacccggaaaaacgcgccatcgccaatgccattacccttgagttcaccgacggcacacgatttgaagaagtggtggtggagtaccccattggtcatgctcgccgccgtcaggatggtattccgaaactggtcgataaattcaaaatcaatctcgcgcgccagttcccgactcgccaacagcagcgcattctggaggtttctctcgacagagctcgcctggaacagatgccggtcaatgagtatctcgacctgtacgtcatttaagtaaacggcggtaaggcgtaagttcaacaggagagcattatgtcttttagcgaattttatcagcgttcgattaacgaaccggagcagttctgggccgagcaggcccggcgtattgactggcagacgccctttacgcaaacgctcgatcacagcaatccgccgtttgcccgttggttttgtgaaggccgaaccaacttgtgccacaacgccatcgaccgctggctggagaaacagccagaggcgctggcgctgattgccgtctcttcggaaacagaagaagagcgcacctttacctttcgtcagctgcatgacgaagtgaacgcggtggcctcaatgttgcgttcattgggtgtgcagcgcggcgatcgggtgctggtgtatatgccgatgattgccgaagcgcatattactctgctggcctgcgcgcgcattggcgctattcactcggtggtgtttggtggatttgcctcgcacagcgtggcggcgcgaattgatgacgctaaaccggtgctgattgtctcggctgatgccggagcgcgcggtggcaaaatcattccctataaaaaattgctcgacgatgcgataagtcaggcgcagcaccagccacgccatgttttgctggtggatcgcgggctggcgaaaatggcgcgcgtcagcgggcgggatgtcgatttcgcgtcgttgcgccatcaacacatcggcgcgcgggtaccggtggcgtggctggaatccaacgaaacctcctgcattctctacacttccggcacgaccggcaaacctaaaggcgtgcagcgtgacgtcggcggatatgcggtggcgctggcgacctcgatggacaccatttttggcggcaaagcgggcagcgtgttcttttgcgcatcggatatcggctgggtggtggggcattcgtatatcgtttacgcgccgctgctggcggggatggcgactatcgtttacgaaggattgccgacctggccggactgcggcgtgtggtggacaatcgtcgagaaatatcaggttagccggatgttctcagcgccgaccgccattcgcgtgctgaaaaaattccctaccgctgaaattcgcaaacacgatctctcgtcgctggaagtgctctatctggctggagaaccgctggacgagccgaccgccagttgggtgagcaatacgctggatgtgccggtcatcgacaactactggcagaccgaatccggctggccgattatggcgattgctcgcggtctggacgacaggccgacgcgtctgggaagccccggtgtgccgatgtatggctataacgtgcagttgcttaatgaagtcaccggcgaaccgtgtggcgtcaacgagaaagggatgctggtggtggaagggccgctgccgccggggtgtattcagaccatctggggcgacgacggccgctttgtgaagacttactggtcgctgttttcccgcccggtgtacgccacctttgactggggcatccgtgacgctgacggttatcactttattctcgggcgcactgacgatgtaattaacgttgccgggcatcggctggggacgcgcgagattgaagagagtatctccagccatccgggcgttgccgaagtggcggtggttggggtgaaagatgcgctgaaagggcaggtggcggtggcgtttgtcattccgaaagagagcgacagtctggaagatcgtgatgtggcgcactcgcaagagaaggcgattatggcgctggtggacagccagattggcaactttggccgcccggcgcacgtctggtttgtctcgcaattgccaaaaacgcgatccggaaaaatgctgcgccgcacgatccaggcgatttgcgaaggacgcgatcctggagatctgacgaccattgatgatcctgcgtcgttggatcagatccgccaggcgatggaagagtaggttattgtcggatgcgtcgcgcggtgcatccggcactgtgtgccgatgcctgatgcgacgctgacgcgttttatcatgcctacggacctgaaccgtaggtcggataaggcgctcgcgtcgcatccgacaccatgctcagatgcctgatgcgacgctgacgcgtcttatcaggcctacccactgtttttacaccgataatttttcccccacctttttgcactcattcatataaaaaatatatttccccacgaaaacgattgctttttatcttcagatgaatagaatgcggcggattttttgggtttcaaacagcaaaaagggggaatttcgtgtcgcaagataacaactttagccaggggccagtcccgcagtcggcgcggaaaggggtattggcattgacgttcgtcatgctgggattaaccttcttttccgccagtatgtggaccggcggcactctcggaaccggtcttagctatcatgatttcttcctcgcagttctcatcggtaatcttctcctcggtatttacacttcatttctcggttacattggcgcaaaaaccggcctgaccactcatcttcttgctcgcttctcgtttggtgttaaaggctcatggctgccttcactgctactgggcggaactcaggttggctggtttggcgtcggtgtggcgatgtttgccattccggtgggtaaggcaaccgggctggatattaatttgctgattgccgtttccggtttactgatgaccgtcaccgtcttttttggcatttcggcgctgacggttctttcggtgattgcggttccggctatcgcctgcctgggcggttattccgtgtggctggctgttaacggcatgggcggcctggacgcattaaaagcggtcgttcccgcacaaccgttagatttcaatgtcgcgctggcgctggttgtggggtcatttatcagtgcgggtacgctcaccgctgactttgtccggtttggtcgcaatgccaaactggcggtgctggtggcgatggtggcctttttcctcggcaactcgttgatgtttattttcggtgcagcgggcgctgcggcactgggcatggcggatatctctgatgtgatgattgctcagggcctgctgctgcctgcgattgtggtgctggggctgaatatctggaccaccaacgataacgcactctatgcgtcgggtttaggtttcgccaacattaccgggatgtcgagcaaaaccctttcggtaatcaacggtattatcggtacggtctgcgcattatggctgtataacaattttgtcggctggttgaccttcctttcggcagctattcctccagtgggtggcgtgatcatcgccgactatctgatgaaccgtcgccgctatgagcactttgcgaccacgcgtatgatgagtgtcaattgggtggcgattctggcggtcgccttggggattgctgcaggccactggttaccgggaattgttccggtcaacgcggtattaggtggcgcgctgagctatctgatccttaacccgattttgaatcgtaaaacgacagcagcaatgacgcatgtggaggctaacagtgtcgaataacgctttacaaacaattattaacgcccggttaccaggcgaagaggggctgtggcagattcatctgcaggacggaaaaatcagcgccattgatgcgcaatccggcgtgatgcccataactgaaaacagcctggatgccgaacaaggtttagttataccgccgtttgtggagccacatattcacctggacaccacgcaaaccgccggacaaccgaactggaatcagtccggcacgctgtttgaaggcattgaacgctgggccgagcgcaaagcgttattaacccatgacgatgtgaaacaacgcgcatggcaaacgctgaaatggcagattgccaacggcattcagcatgtgcgtacccatgtcgatgtttcggatgcaacgctaactgcgctgaaagcaatgctggaagtgaagcaggaagtcgcgccgtggattgatctgcaaatcgtcgccttccctcaggaagggattttgtcgtatcccaacggtgaagcgttgctggaagaggcgttacgcttaggggcagatgtagtgggggcgattccgcattttgaatttacccgtgaatacggcgtggagtcgctgcataaaaccttcgccctggcgcaaaaatacgaccgtctcatcgacgttcactgtgatgagatcgatgacgagcagtcgcgctttgtcgaaaccgttgctgccctggcgcaccatgaaggcatgggcgcgcgagtcaccgccagccacaccacggcaatgcactcctataacggggcgtatacctcacgcctgttccgcttgctgaaaatgtccggtattaactttgtcgccaacccgctggtcaatattcatctgcaaggacgtttcgatacgtatccaaaacgtcgcggcatcacgcgcgttaaagagatgctggagtccggcattaacgtctgctttggtcacgatgatgtcttcgatccgtggtatccgctgggaacggcgaatatgctgcaagtgctgcatatggggctgcatgtttgccagttgatgggctacgggcagattaacgatggcctgaatttaatcacccaccacagcgcaaggacgttgaatttgcaggattacggcattgccgccggaaacagcgccaacctgattatcctgccggctgaaaatgggtttgatgcgctgcgccgtcaggttccggtacgttattcggtacgtggcggcaaggtgattgccagcacacaaccggcacaaaccaccgtatatctggagcagccagaagccatcgattacaaacgttgaacgactgggttacagcgagcttagtttatgccggatgcggcgtgaacgccttatccggcctacgtagagcactgaactcgtaggcctgataagcgtagcgcatcaggcaattccagccgctgatctgtgtcagcggctaccgtgattcattcccgccaacaaccgcgcattcctccaacgccatgtgcaaaaatgccttcgcagcggctgtctgccagctgtagtttatgccggatgcggcgtgaacgccttatccggcctacgtagagcactgaactcgtaggcctgataagcgtagcgcatcaggcaattccagccgcagacctgtgtcagcggctaccgtgattcatttccgccaacaaccgcgcatttatccaacgccatgtgcaaaaatgccttcgcggcggctgtctgccagctatttttccgccgcaacaaaaccgccgttctctccagtagtggcggggcaagagaaatagctttaagcccgtcatgttgtgtggcaatcgctgctggtaacaatgtggaaagggaagtgcggcgaatcagctccagaaccgcgctaattgagttcgcctcaatgaccacctgtggatgtagccccgctttctcgcagtagtggtcaatttgctctctggtggcaaattccgcgctgagcaggaccagtttttcatcatgcaagcgactcaacgccacctgttcatggacggccagcggatgatgttgcgccacgactaacgctaaactttctgtcagtaaaggaattgcctccagctccggcgaatgcacaggcgcgaaggcaatcccaacgtccaactcgtcgcggcaaagcatatcctcgattttctcctgcgacatttcctgtagctggagcgtgatgctgggatagcgcgcatagaaatccgccattaaggggccgataaagtagctcgtaaaggtgggggtgacggcgatacgcagcgatcctcgcgtcagatcggcaacatcatgaatcgcccgtttacccgcccccagttcctgtaacgcccggctggcgtactgtcgccagacttctcctgcatcagtgagacgaatcgttcgcccgctacggtcaaacagcggcacgcctaaactctcctctaactggcgaatctgctgggaaagcgcaggttgggagacgtgcaacgcactggcggcacgggtgaagctgccatgttcagccacggcaagaaaataattgatatgtcgagagagcattcgcaacctataagtaaatccaatggaactcatcataaatgagacttttaccttatgacaatcggcgagtagtctgcctctcattccagagacagacagaggttaacggtgaaagagattattgatggattccttaaattccagcgcgaggcatttccgaagcgggaagccttgtttaaacagctggcgacacagcaaagcccgcgcacactttttatctcctgctccgacagccgtctggtccctgagctggtgacgcaacgtgagcctggcgatctgttcgttattcgcaacgcgggcaatatcgtcccttcctacgggccggaacccggtggcgtttctgcttcggtggagtatgccgtcgctgcgcttcgggtatctgacattgtgatttgtggtcattccaactgtggcgcgatgaccgccattgccagctgtcagtgcatggaccatatgcctgccgtctcccactggctgcgttatgccgattcagcccgcgtcgttaatgaggcgcgcccgcattccgatttaccgtcaaaagctgcggcgatggtacgtgaaaacgtcattgctcagttggctaatttgcaaactcatccatcggtgcgcctggcgctcgaagaggggcggatcgccctgcacggctgggtctacgacattgaaagcggcagcatcgcagcttttgacggcgcaacccgccagtttgtgccactggccgctaatcctcgcgtttgtgccataccgctacgccaaccgaccgcagcgtaaccttatttttaaaccatcaggagttccaccatgattcagtcacaaattaaccgcaatattcgtcttgatcttgccgatgccattttgctcagcaaagctaaaaaagatctctcatttgccgagattgccgacggcaccggtctggcagaagcctttgtaaccgcggctttgctgggtcagcaggcgcttcctgccgacgccgcccgcctggtcggggcgaagctggatctcgacgaagactccattctactgttgcagatgattccactgcgtggctgcattgatgaccgtattccaactgacccaacgatgtatcgtttctatgaaatgttgcaggtgtacggtacaaccctgaaagcgttggttcatgagaaatttggcgatggcattattagcgcgattaacttcaaactcgacgttaagaaagtggcggacccggaaggtggcgaacgtgcggtcatcaccttagatggtaaatatctgccgaccaaaccgttctgacagccatgcgcaaccatcaaaagacgttcacgatgctgctggtactggtgctgattggtcttaatatgcgaccactgctcacctccgtcgggccactgctaccgcaattgcgccaggcgagcggaatgagctttagcgtggctgccctgttgaccgctctgccggtggttaccatgggcgggctggcgctggccggaagctggcttcatcagcatgtcagcgaacgtcgcagtgtcgccatcagtctgttgctgattgccgtcggtgcattgatgcgtgagctttacccgcaaagtgcgctgctgcttagcagcgcactgcttggtggggtggggatcggcatcattcaggcggtgatgccttcggtgattaaacggcggtttcagcagcgcacgccactggtgatggggctgtggtccgcggctctgatgggcggcggtgggcttggtgccgccataacgccctggttagttcaacatagcgaaacctggtatcaaacactcgcctggtgggcgctgcctgccgttgttgcgctctttgcctggtggtggcaaagcgcccgcgaggtcgcctcttcccacaagacaacaaccactccggttcgcgtggtattcactccccgcgcgtggacgctgggtgtttacttcggtctgattaacggcggttacgccagcctgattgcctggttacccgctttctatattgagattggtgccagcgcgcagtacagcggttccttactggcattgatgacgcttgggcaagccgcaggagctttgctgatgcctgctatggctcgccatcaggatcggcgcaaactgttaatgctggcgctggtgttacaactggtggggttctgcggctttatctggctgccgatgcaattgccggtattgtgggcgatggtgtgtgggttaggtctgggcggcgcgtttccgctctgtttgctgctggcgctcgatcactctgtgcaaccggctattgctggcaagctggtggcgtttatgcagggaatcggttttatcatcgccgggcttgccccgtggttttctggcgtgctgcgtagtatcagcggcaattacctgatggactgggcatttcatgcgctgtgcgtcgttgggctgatgatcataaccctgcgttttgcaccagtacgttttccgcagctgtgggtcaaagaggcatgatgcgacgcttgttcctgcgctttgttcatgccggatgcggctaatgtagatcgctgaacttgtaggcctgataagcgcagcgtatcaggcaatttttataatttaaactgacgattcaactttataatctttgaaataatagtgcttatcccggtcgtttatttcgcgaataacccgacaaggaacgccagccgccacgacgtttggtggaatgtcttttgtgacgatactacccgcgccaataacagaattatccccgatggtgacgcctggattaataaccacatgacttccgatccagacgttattgccaatcgttatcggaaaagagtacatctcgccgttttttctcaattcatggtgtacagggtgtcccgtaacggaaagagtaacgttgggtgcaatcagtacgttatcaccgattgttaccgtgtagtcatcgacaatggttaaattgaaatttgcataaaaattgcggcctatatggatgttggaaccgtaagagaaatagacaggcggttctacccaggcgttttcccctaccgtggcaaacatttctttaatcaggctttctcttttttcaacttctgatggatgcgagtgattaaactcatacattaacgttttcccacgaagtcttttttccggtaagccttcgcacatatcggtaaatagcttgcctgctcttattctttcggtcattggcatgttcaatgcgatcactccgttatgatatgttggtcggataaggcgctcgcgccgcatccgacattgattgcttaagcgacttcattcacctgacgacgcagcagggaaagcgggccggggccgctaagcgtgaacacggaaattaaggtgaagcccagcgccaccagacccagcaccagataagcgccctggaaaccgatgctttcatacatattgcccgccagtacagacataaaaatcatcgccagttgcttaaagaagcagaaacagaccagataaatcgtcgctgaaaaacgcacttcaaactggctggtaatatatttaaagcagcccaccagcaggaacggtacttcaaacatatgcagcgttttcagaataaccacttccagcgctgaggtggcgaacgatgagccaataatacgtacagacataatagtgccagccagcagcagggcgtttttcccaccgatgcgattaatgatcagtggcgcaaagaacataatcgaggcgttaagtaattcgcccattgtcgttacgtagccaaatacccgcgtaccctgttcaccggtagcaaagaacgaagtaaagaaattagcaaactgttggtcaaaaacatcgtaggtgcaggaaacgccaataacatacagtgacaaaaaccacagttttggctgtctgaacagttccagtgccagcttaaggctaaatgccgaatggttggcacctaccgcattggcaaccgtggcagaagagggcgcatccgttttggcgaaaaagagtaaaacggcgaggatgagtgcacagccagagcccagccagaaaacaaactgattattgatggtgaacatgatgccgacaatcgaggcacacagcgcccagccaacacagccaaacatccgcgcgcgaccaaattcgaaattactgcgacggctgactttctcaataaatgcctctactgctggcgcaccggcgttaaaacaaaagcctagataaataccaccaacaatcgatcctactaaaatgttgtattgtaacagtggcccgaagataaaaataaagaacggcgcaaacatcactaacatgccggtaataatccacagcaggtatttgcgcagcccgagtttgtcagaaagcagaccaaacagcggttggaataatagcgagaacagagaaatagcggcaaaaataatacccgtatcacttttgctgatatggttgatgtcatgtagccaaatcgggaaaaacgggaagtaggctcccatgataaaaaagtaaaagaaaaagaataaaccgaacatccaaaagtttgtgttttttaaatagtacataatggatttccttacgcgaaatacgggcagacatggcctgcccggttattattatttttgacaccagaccaactggtaatggtagcgaccggcgctcagctggaattccgccgatactgacgggctccaggagtcgtcgccaccaatccccatatggaaaccgtcgatattcagccatgtgccttcttccgcgtgcagcagatggcgatggctggtttccatcagttgctgttgactgtagcggctgatgttgaactggaagtcgccgcgccactggtgtgggccataattcaattcgcgcgtcccgcagcgcagaccgttttcgctcgggaagacgtacggggtatacatgtctgacaatggcagatcccagcggtcaaaacaggcggcagtaaggcggtcgggatagttttcttgcggccctaatccgagccagtttacccgctctgctacctgcgccagctggcagttcaggccaatccgcgccggatgcggtgtatcgctcgccacttcaacatcaacggtaatcgccatttgaccactaccatcaatccggtaggttttccggctgataaataaggttttcccctgatgctgccacgcgtgagcggtcgtaatcagcaccgcatcagcaagtgtatctgccgtgcactgcaacaacgctgcttcggcctggtaatggcccgccgccttccagcgttcgacccaggcgttagggtcaatgcgggtcgcttcacttacgccaatgtcgttatccagcggtgcacgggtgaactgatcgcgcagcggcgtcagcagttgttttttatcgccaatccacatctgtgaaagaaagcctgactggcggttaaattgccaacgcttattacccagctcgatgcaaaaatccatttcgctggtggtcagatgcgggatggcgtgggacgcggcggggagcgtcacactgaggttttccgccagacgccactgctgccaggcgctgatgtgcccggcttctgaccatgcggtcgcgttcggttgcactacgcgtactgtgagccagagttgcccggcgctctccggctgcggtagttcaggcagttcaatcaactgtttaccttgtggagcgacatccagaggcacttcaccgcttgccagcggcttaccatccagcgccaccatccagtgcaggagctcgttatcgctatgacggaacaggtattcgctggtcacttcgatggtttgcccggataaacggaactggaaaaactgctgctggtgttttgcttccgtcagcgctggatgcggcgtgcggtcggcaaagaccagaccgttcatacagaactggcgatcgttcggcgtatcgccaaaatcaccgccgtaagccgaccacgggttgccgttttcatcatatttaatcagcgactgatccacccagtcccagacgaagccgccctgtaaacggggatactgacgaaacgcctgccagtatttagcgaaaccgccaagactgttacccatcgcgtgggcgtattcgcaaaggatcagcgggcgcgtctctccaggtagcgaaagccattttttgatggaccatttcggcacagccgggaagggctggtcttcatccacgcgcgcgtacatcgggcaaataatatcggtggccgtggtgtcggctccgccgccttcatactgcaccgggcgggaaggatcgacagatttgatccagcgatacagcgcgtcgtgattagcgccgtggcctgattcattccccagcgaccagatgatcacactcgggtgattacgatcgcgctgcaccattcgcgttacgcgttcgctcatcgccggtagccagcgcggatcatcggtcagacgattcattggcaccatgccgtgggtttcaatattggcttcatccaccacatacaggccgtagcggtcgcacagcgtgtaccacagcggatggttcggataatgcgaacagcgcacggcgttaaagttgttctgcttcatcagcaggatatcctgcaccatcgtctgctcatccatgacctgaccatgcagaggatgatgctcgtgacggttaacgcctcgaatcagcaacggcttgccgttcagcagcagcagaccattttcaatccgcacctcgcggaaaccgacatcgcaggcttctgcttcaatcagcgtgccgtcggcggtgtgcagttcaaccaccgcacgatagagattcgggatttcggcgctccacagtttcgggttttcgacgttcagacgtagtgtgacgcgatcggcataaccaccacgctcatcgataatttcaccgccgaaaggcgcggtgccgctggcgacctgcgtttcaccctgccataaagaaactgttacccgtaggtagtcacgcaactcgccgcacatctgaacttcagcctccagtacagcgcggctgaaatcatcattaaagcgagtggcaacatggaaatcgctgatttgtgtagtcggtttatgcagcaacgagacgtcacggaaaatgccgctcatccgccacatatcctgatcttccagataactgccgtcactccagcgcagcaccatcaccgcgaggcggttttctccggcgcgtaaaaatgcgctcaggtcaaattcagacggcaaacgactgtcctggccgtaaccgacccagcgcccgttgcaccacagatgaaacgccgagttaacgccatcaaaaataattcgcgtctggccttcctgtagccagctttcatcaacattaaatgtgagcgagtaacaacccgtcggattctccgtgggaacaaacggcggattgaccgtaatgggataggtcacgttggtgtagatgggcgcatcgtaaccgtgcatctgccagtttgaggggacgacgacagtatcggcctcaggaagatcgcactccagccagctttccggcaccgcttctggtgccggaaaccaggcaaagcgccattcgccattcaggctgcgcaactgttgggaagggcgatcggtgcgggcctcttcgctattacgccagctggcgaaagggggatgtgctgcaaggcgattaagttgggtaacgccagggttttcccagtcacgacgttgtaaaacgacggccagtgaatccgtaatcatggtcatagctgtttcctgtgtgaaattgttatccgctcacaattccacacaacatacgagccggaagcataaagtgtaaagcctggggtgcctaatgagtgagctaactcacattaattgcgttgcgctcactgcccgctttccagtcgggaaacctgtcgtgccagctgcattaatgaatcggccaacgcgcggggagaggcggtttgcgtattgggcgccagggtggtttttcttttcaccagtgagacgggcaacagctgattgcccttcaccgcctggccctgagagagttgcagcaagcggtccacgctggtttgccccagcaggcgaaaatcctgtttgatggtggttaacggcgggatataacatgagctgtcttcggtatcgtcgtatcccactaccgagatatccgcaccaacgcgcagcccggactcggtaatggcgcgcattgcgcccagcgccatctgatcgttggcaaccagcatcgcagtgggaacgatgccctcattcagcatttgcatggtttgttgaaaaccggacatggcactccagtcgccttcccgttccgctatcggctgaatttgattgcgagtgagatatttatgccagccagccagacgcagacgcgccgagacagaacttaatgggcccgctaacagcgcgatttgctggtgacccaatgcgaccagatgctccacgcccagtcgcgtaccgtcttcatgggagaaaataatactgttgatgggtgtctggtcagagacatcaagaaataacgccggaacattagtgcaggcagcttccacagcaatggcatcctggtcatccagcggatagttaatgatcagcccactgacgcgttgcgcgagaagattgtgcaccgccgctttacaggcttcgacgccgcttcgttctaccatcgacaccaccacgctggcacccagttgatcggcgcgagatttaatcgccgcgacaatttgcgacggcgcgtgcagggccagactggaggtggcaacgccaatcagcaacgactgtttgcccgccagttgttgtgccacgcggttgggaatgtaattcagctccgccatcgccgcttccactttttcccgcgttttcgcagaaacgtggctggcctggttcaccacgcgggaaacggtctgataagagacaccggcatactctgcgacatcgtataacgttactggtttcacattcaccaccctgaattgactctcttccgggcgctatcatgccataccgcgaaaggttttgcgccattcgatggtgtcaacgtaaatgcatgccgcttcgccttccggccaccagaatagcctgcgattcaaccccttcttcgatctgttttgctacccgttgtagcgccggaagatgcttttccgctgcctgttcaatggtcattgcgctcgccatatacaccagattcagacagccaatcacccgttgttcactgcgcagcggtacggcgatagaggcgatcttctcctcctgatcccagccgcggtagttctgtccgtaaccctctttgcgcgcgcgcgccagaatggcttccagctttaacggttcccgtgccagttgatagtcatcaccggggcgggaggctaacatttcgattaattccttgcggtcttgttccgggcaaaaggccagccaggtcaggcccgaggcggttttcagaagcggcaaacgtcgcccgaccattgcccggtgaaaggataagcggctgaaacggtgagtggtttcgcgtaccaccattgcatcaacatccagcgtggacacatctgtcggccataccacttcgcgcaacagatcgcccagcagtggggccgccagtgcagaaatccactgttcgtcacgaaatccttcgcttaattgccgcactttgatggtcagtcgaaaactatcatcggaggggctacggcggacatatccctcttcctgcagcgtctccagcagtcgccgcacagtggtgcgatgcaggccgctgagttccgccagcagcccgacgctggcaccgccatcaagtttatttaacatatttaataacattagaccgcgggttaagccgcgcacggttttgtattccgtctgctcattgttctgcatattaattgacatttctatagttaaaacaacgtggtgcacctggtgcacattcgggcatgttttgattgtagccgaaaacacccttcctatactgagcgcacaataaaaaatcatttacatgtttttaacaaaataagttgcgctgtactgtgcgcgcaacgacattttgtccgagtcgtgaggtactgaaatggcaatacaacaccctgacatccagcctgctgttaaccatagcgttcaggtggcgatcgctggtgccggcccggttgggctgatgatggcgaactatctcggccagatgggcattgacgtgctggtggtggagaaactcgataagttgatcgactacccgcgtgcgattggtattgatgacgaggcgctgcgcaccatgcagtcggtcggcctggtcgatgatgttctgccgcacactacgccgtggcacgcgatgcgttttctcaccccgaaaggccgctgttttgctgatattcagccaatgaccgatgaatttggctggccgcgccgtaacgcctttattcagccgcaggtcgatgcggtgatgctggaaggggtgtcgcgttttccgaatgtgcgctgcttgttttcccgcgagctggaggccttcagtcagcaagatgacgaagtgaccttgcacctgaaaacggcagaagggcagcgggaaatagtcaaagcccagtggctggtagcctgtgacggtggagcaagttttgtccgtcgcactctgaatgtgccgtttgaaggtaaaactgcgccaaatcagtggattgtggtagatatcgccaacgatccgttaagtacgccgcatatctatttgtgttgcgatccggtgcgcccgtatgtttctgccgcgctgcctcatgcggtacgtcgctttgaatttatggtgatgccgggagaaaccgaagagcagctgcgtgagccgcaaaatatgcgcaagctgttaagcaaagtgctgcctaatccggacaatgttgaattgattcgccagcgtgtctacacccacaacgcgcgactggcgcaacgtttccgtattgatcgcgtactgctggcgggcgatgccgcgcacatcatgccggtatggcaggggcagggctataacagtggtatgcgcgacgcctttaacctcgcatggaaactggcgttggttatccaggggaaagcccgcgatgcgctgctcgatacctatcaacaagaacgtcgcgatcacgccaaagcgatgattgacctgtccgtgacggcgggcaacgtgctggctccgccgaaacgctggcagggtacgttacgtgacggcgtttcctggctgttgaattatctgccgccagtaaaacgctacttcctcgaaatgcgcttcaagccgatgccgcaatattacggcggtgcgctgatgcgtgagggcgaagcgaagcactctccggtcggcaagatgtttattcagccgaaagtcacgctggaaaacggcgacgtgacgctgctcgataacgcgatcggcgcgaacttcgcggtaattggctggggatgcaatccactgtgggggatgagcgacgagcaaatccagcagtggcgcgcgttgggcacacgcttcattcaggtggtgccggaagtgcaaattcataccgcacaggataaccacgacggcgtactacgcgtgggcgatacgcaaggtcgcctgcgtagctggttcgcgcaacacaatgcttcgctggtggtgatgcgcccggatcgctttgttgccgccaccgccattccgcaaaccctgggcaagaccctgaataaactggcgtcggtgatgacgctgacccgccctgatgccgacgtttctgtcgaaaaggtagcctgatatgcacgcttatcttcactgtctttcccactcgccgctggtggggtatgtcgacccggcgcaagaggtgctcgatgaggtcaatggcgtgattgccagcgcccgcgagcgtattgcggcattctcccctgaactggtggtgctgtttgcgccagatcactacaacggctttttctatgacgtgatgccaccgttctgtttaggcgttggagcgacggcaattggtgatttcggcagtgcggcaggagagctgcccgtgcctgtggagctggcggaggcctgtgcgcatgccgtcatgaagagcgggatcgatcttgccgtttcttactgtatgcaggtggaccacgggttcgcccagccgctggagttcctgctcggtgggctggataaggtgccagttctgcctgtgttcatcaacggtgtcgccacgccgctgcccggtttccagcgtacccgcatgttgggtgaagccattggacgtttcaccagcactctcaataaacgcgtgctgttcctgggttccggtgggctttcccatcagccgccggtgcccgaactggcgaaagccgatgcccatatgcgcgaccgtctgttggggagcgggaaagatttacccgccagtgagcgcgaattgcgtcagcaacgggtgattagcgccgctgagaagtttgttgaggatcagagaacgctgcatccgctcaacccgatttgggataaccagttcatgactttgctggagcagggacgcatacaggaactggatgccgtcagtaacgaagagctttccgccattgccggaaagtcgacacatgaaatcaaaacctgggtcgccgcttttgccgctatttctgcgtttggcaactggcgtagcgaagggcgttattaccgcccaatcccggagtggattgccggatttggctcgttaagcgccagaacagagaactgaatatgcaggagaagatgatgagttatcagccacaaaccgaagccgccaccagccgttttctgaatgtagaagaagcgggtaaaacgctgcgcatccattttaatgactgcggacaaggcgacgaaaccgttgtcctgctgcatggttccggcccgggtgctactggctgggcgaacttcagccgcaatatcgatccgctggtagaggcgggctatcgggtgatcctgctggattgtccgggttggggcaagagcgattcggtcgttaatagtggttcgcgatcggatcttaatgcacgaatcctgaaaagcgtggtggatcaactggatatcgccaaaatccacctgctgggcaactcgatggggggccatagttctgtggcgttcacccttaaatggccggagcgcgtcggcaaactggtgctgatgggcggcggtacgggcggcatgagtttgtttacgccgatgccaaccgaaggtattaagcgactgaatcagctttatcgtcagccgactatcgaaaacctgaagctgatgatggatatcttcgtttttgataccagcgatttgaccgacgccctgtttgaagcgcgcctgaataatatgctgtcgcgccgcgatcacctggaaaacttcgttaagagcctggaagctaatccgaaacagttcccggattttggcccacgtctggcggaaatcaaagcgcaaaccctgattgtctgggggcgcaacgaccgctttgtgccgatggatgcgggtctgcgtctgctgtccggcattgccggttctgaactgcatatcttccgcgactgtggtcactgggcgcagtgggaacatgccgacgctttcaatcaactggtgctgaatttcctcgcacgcccttaaggaatggtcatgacgaagcatactcttgagcaactggcggcggatttacgccgcgccgcagagcagggcgaagcgattgcaccgctgcgcgatctgattggtatcgataacgctgaagcggcttacgccattcagcacataaatgtgcaacatgacgttgcgcaggggcgtcgcgtggtagggcgtaaagtgggcctgacacatccgaaagtgcaacaacaactgggcgttgatcaaccggattttgggacgttatttgccgacatgtgttatggcgataacgaaatcattcctttttcccgtgttctgcaaccccgcattgaagcggagatcgcactggtgttgaaccgcgatttgcccgcaaccgatatcaccttcgacgaattgtataacgccattgaatgggtacttccggcgctggaagtggtggggagccgcattcgcgactggtcgattcagtttgtcgataccgtggcagataacgcctcctgtggggtgtatgtcatcggcggtccggcgcaacgtccggcggggttagacctgaaaaactgcgccatgaagatgacgcgtaataacgaagaggtttctagcgggcgcggcagcgaatgcctgggacatccgcttaatgcggccgtctggctggcacgcaaaatggccagtctgggtgaaccgctgcgcaccggagatatcattcttaccggggcattaggtccgatggtggcggtgaatgcgggcgatcgttttgaagcccatattgaaggcataggttcagttgctgcgacattttcaagcgcagccccaaaaggaagtctgtcatgagtaagcgtaaagtcgccattatcggttctggcaacattggtaccgatctgatgattaaaattttgcgtcacggtcagcatctggagatggcggtgatggttggcattgatcctcagtccgacggtctggcgcgcgccagacgtatgggcgtcgccaccacccatgaaggggtgatcggactgatgaacatgcctgaatttgctgatatcgacattgtatttgatgcgaccagcgccggtgctcatgtgaaaaacgatgccgctttacgcgaagcgaaaccggatattcgcttaattgacctgacgcctgctgccatcggcccttactgcgtgccggtggttaacctcgaggcgaacgtcgatcaactgaacgtcaacatggtcacctgcggcggccaggccaccattccaatggtggcggcagtttcacgcgtggcgcgtgttcattacgccgaaattatcgcttctatcgccagtaaatctgccggacctggcacgcgtgccaatatcgatgaatttacggaaaccacttcccgagccattgaagtggtgggcggcgcggcaaaagggaaggcgattattgtgcttaacccagcagagccaccgttgatgatgcgtgacacggtgtatgtattgagcgacgaagcttcacaagatgatatcgaagcctcaatcaatgaaatggctgaggcggtgcaggcttacgtaccgggttatcgcctgaaacagcgcgtgcagtttgaagttatcccgcaggataaaccggtcaatttaccgggcgtggggcaattctccggactgaaaacagcggtctggctggaagtcgaaggcgcagcgcattatctgcctgcctatgcgggcaacctcgacattatgacttccagtgcgctggcgacagcggaaaaaatggcccagtcactggcgcgcaaggcaggagaagcggcatgaacggtaaaaaactttatatctcggacgtcacattgcgtgacggtatgcacgccattcgtcatcagtattcgctggaaaacgttcgccagattgccaaagcactggacgatgcccgcgtggattcgattgaagtggcccacggcgacggtttgcaaggttccagctttaactatggtttcggcgcacatagcgaccttgaatggattgaagcggcggcggatgtggtgaagcacgccaaaatcgcgacgttgttgctgccaggaatcggcactattcacgatctgaaaaatgcctggcaggctggcgcgcgggtggttcgtgtggcaacgcactgtaccgaagctgatgtttccgcccagcatattcagtatgcccgcgagctcggaatggacaccgttggttttctgatgatgagccatatgaccacgccggagaatctcgccaagcaggcaaagctgatggaaggctacggtgcgacctgtatttatgtggtggattctggcggtgcgatgaacatgagcgatatccgtgaccgtttccgcgccctgaaagcagagctgaaaccagaaacgcaaactggcatgcacgctcaccataacctgagtcttggcgtggcgaactctatcgcggcggtggaagagggctgcgaccgaatcgacgccagcctcgcgggaatgggcgcgggcgcaggtaacgcaccgctggaagtgtttattgccgccgcggataaactgggctggcagcatgggaccgatctctatgcgttaatggatgccgccgacgacctggtgcgtccgttgcaggatcgaccggtacgagtcgatcgcgaaacgctggcgctgggatacgctggtgtttactcgagcttcctgcgtcactgtgaaacggcggcggcgcgttatggcttaagtgcggtggatattctcgttgagctgggcaaacgccggatggttggcggccaggaggatatgatcgttgacgtggcgctggatctgcgcaacaacaaataatgatgactgccgagaacgtgcattttgtatgcccatcccagcacgactgccggatgcggcgtgaacgccttatccggcctacggatggcgtgagaatttgtaggtctgataagacgcgttagcgtcgcatcaggcatctgcgcacgactgccggatgcggcgtgaacgccttatccggcctacggatggcgcgggaatttgtaggcctgataagacgcgttagcgtcgcatcaggcatctgcgcacgactgccggatgcggcgtgaacgccttatccggcctacgggtggcgcgagaatttgtaggcctgataagacgcgttagcgtcgcatcaggcatctgcgcacgactgccggatgcggcgtaaacgccttatccggcctacggatggcgcgggaatttgtaggcctgataagacgcgttagcgtcgcatcaggcatctgcacacgactgccggatgcgataaacgtcttgtccggcctacatttcgcccgtaggcagtcattaaatagttctgattacgcggctggcaatgtatcagtcgcgattcacctgcactcgcaacgaggttcatcttatgtcgactcgtaccccttcatcatcttcatcccgcctgatgctgaccatcgggctttgttttttggtcgctctgatggaagggctggatcttcaggcggctggcattgcggcgggtggcatcgcccaggctttcgcactcgataaaatgcaaatgggctggatatttagcgccggaatactcggtttgctacccggcgcgttggttggcggaatgctggcggaccgttatggtcgcaagcgcattttgattggctcagttgcgctgtttggtttgttctcactggcaacggcgattgcctgggatttcccctcactggtctttgcgcggctgatgaccggtgtcgggctgggggcggcgttgccgaatcttatcgccctgacgtctgaagccgcgggtccacgttttcgtgggacggcagtgagcctgatgtattgcggtgttcccattggcgcggcgctggcggcgacactgggtttcgcgggggcaaacttagcatggcaaacggtgttttgggtaggtggtgtggtgccgttgattctggtgccgctattaatgcgctggctgccggagtcggcggttttcgctggcgaaaaacagtctgcgccaccactgcgtgccttatttgcgccagaaacggcaaccgcgacgctgctgctgtggttgtgttatttcttcactctgctggtggtctacatgttgatcaactggctaccgctacttttggtggagcaaggattccagccatcgcaggcggcaggggtgatgtttgccctgcaaatgggggcggcaagcgggacgttaatgttgggcgcattgatggataagctgcgtccagtaaccatgtcgctactgatttatagcggcatgttagcttcgctgctggcgcttggaacggtgtcgtcatttaacggtatgttgctggcgggatttgtcgcggggttgtttgcgacaggtgggcaaagcgttttgtatgccctggcaccgttgttttacagttcgcagatccgcgcaacaggtgtgggaacagccgtggcggtagggcgtctgggggctatgagcggtccgttactggccgggaaaatgctggcattaggcactggcacggtcggcgtaatggccgcttctgcaccgggtattcttgttgctgggttggcggtgtttattttgatgagccggagatcacgaatacagccgtgcgccgatgcctgacgtgccttattaggcaggggcgaaagggacttcaccccaatacacctacggcgtttacaggtatactcgctaaaaattattcagcgggtttggaaacaaagatggcaaaacttaccttacaagagcagttgctcaaagcaggattagtcaccagcaaaaaagcggcgaaggtggagagaacggcgaaaaaatcgcgcgttcaggcgcgtgaagctcgggcggcggtagaagaaaataaaaaggcacagcttgagcgtgataaacagcttagcgaacagcaaaaacaagcggcgttggcgaaagaatataaagctcaggtgaagcagcttattgaaatgaaccgaatcaccattgccaatggcgatattggttttaacttcactgacggcaatctgattaagaagatttttgtcgataagctcacacaggcgcagttgattaatggtcgtctggcgattgcccgcttgttggtcgataacaatagcgaaggtgaatacgccattattcccgccagcgttgccgataaaattgctcagcgcgatgccagcagtatagtgttgcacagcgcgctcagcgccgaagagcaggatgaagacgacccgtatgccgacttcaaagtgcctgatgatttgatgtggtaaacatagataagtcgtgcgcagatgcctgatgcgacgctatgcgcgtcttatcaggcctacggtttatgggcgaagtgtagaccggataaggcgttcacgccgcatccggcagtcgtgcgccatgcctgatgcgacgctttgcgcgtcttatcaggcctacggcttacgggcgaagtgtaggccggataaggcgttcacgccgcatccggcagtcgtgctattatcaacgcatattcagtttattggcgtggtaggcaatatgctcgccaataaaactggagacaaaataatagctgtgatcataaccctcgtgataacggattaacgtcttgatattcatctcctggcagatcttttcaagatttggagtccgcagctgttctgcgtaaaaatcatcactcaacccctgatcaaccatgatttccgcaacgcgttgaccttgtgaaataagactcaccgggtcgtaatccaaccaggcatctttattttcagcaagatatgcagcaaaggcttgctgtccccacggcacttgcgatggggagacaatgggcgaaaacgccgagacgctgacatattcatctgggttacgtaacgccagcaccagcgcgcccagcccgcccatagaatgaccagagatagactttttggccgttgccggaaaatgatgcatcactaaatccggcagctcgttgcggatatagtcatacattttgtaatgttcattccacggcgcttgcgtcgcgttcaggtaaaacccggcaccttgcccgagatcgtaacggtcagcatctgcgacatgactgcctcgcggactggtgtccggcgcaacaacaataatgttgtgctcagccgcgtaacgctgcatccccgatttagtaatgaaattctgctcgttgcaggtcaggcctgaaagccagtacagcaccggcaatttttcattcgcggcttttggtgggagatagacgccgacattcatttcacatttcagtgattgggaataatgccgatacatattttgccagccgccaaagctgacatgtttttcaatgagttccatcagtcattatctcagggttaatcccccggacggctgcccggggagagtattaagaacccccgcctgaagtggacggggtaaacctgcgggaaatcagtaacgaattacggttcgaatggatttgccttcatgcatcaggtcgaaggcgtcattaatttcatccaggctcatggtatgcgtgacaaacggttccagatcgatatcacctttcatcgcatcttcaaccatgcccggtaactgggaacgacctttcacgccgccaaacgcggaacctttccatacgcgaccagtgaccaactggaatggacgggtggagatttcctgaccggcaaccgcgaccccgatgatcaccgactgaccccagccgcggtgcgcactttccagcgccgcacgcatcacgttgacgttaccgatgcattcaaaggtatggtcgataccccatttgttgatatccaacaggacatcttttatcggtttgtcgtagtcattcgggttaatgcagtcggtagcaccgaagcgacgcgccagatcgaatttcttcgggttggtatcgatagcgataatccgacccgctttcgcctgacgcgcgccctgaaccactgccagaccaatcgcgccaagaccaaacacggcaacagaatcacctggctggactttagctgtgttgtgtaccgcgccaataccggtggtcacgccacagcccagcaggcagacgtgttcatggtttgcttctggattaatttttgccagagacacttccgcgactacggtgtattcactgaatgtagagcaccccatgtagtgataaagcggctgcccgttgtaagaaaaacgggtggtgccgtctggcatcaggcctttaccctgggtttcgcgaaccgcaacacagaggttagttttgccagaacgacagaactcacactcgccgcactccgcggtgtaaagcgggatcacatggtcgccaggtttgacgctggttacgccttcaccgacttcaaccacaacgccggccccttcgtgaccgagaaccaccgggaatacaccttccgggtcatcgccggagagggtaaatgcgtcggtatggcaaacgccggtatgggtgactttaattagcacttcaccttttttcggtggtgcaacgtcaatttcaacgatttccagcggtttaccgggagcaaatgcaacggcagcacgtgatttcatctctcgctcttcctcaatatggtaatagattcagctatttaagataggcacgaaccagttcaatagtgtcgtcaacggattggctgacttcgcggctgtagcagtcatttcggtcaaacgtttcccggatatggctttcaagcacttctgccatcagcccattagccgcgccccgaacggcagcgatctgttggagtatggcacggcattcggcatcaccctccagcgaccgttccagagcatcaatctgcccccgaatacgacgaactcgagtaaggacctttttcttctcttccggagtactgggcatttcgcacctcatcatctgcatgcaatatactataggggggtattctatatgtcaatgcatacccccctatagtatataacactggagaataaaatttatccggtgaatgtggtcggaaaacaaagaggaaaggggggggggctaatcggcagggaaggccgccccggatagcgggcggcagaaggaatcagaatttccaggtcagacgggctgcaagttgcagaccgttaaaatcatcggttggggtgtcgtaccacactttacctgccgtcagcccgagattaagttgctcagtcagcggttgaatacgttgcagactgacgctcttcatgctgccgtagcgtgtttctggcgtccagtcataggtgtaagcacctgttccgcggcttagccatagttgcgtataaccagtgccgcgcgggtcattcagacgcacggaaatcatattgctataactaccacctgcatcgctggagtcataatgggtatagcggtagctggtgatcaccgggccagtatagagtgatacgccgccttgccaggcatcgacttcgacatcatcgtaatatttagtgtagcgataaccggtcgtgaaaagcgtttttggtaacagggccaggttaatatcctgacgaaaatcctggcgggcaaagaccggcgtattatccgcaaaggcaatacccgttcgggttgtcagccagttattccatttataccagaccgcaccctgaccgcgagtggcattgaaatgttcagtttcataatcacgacgcccctgggaaagattaaaaagcagcgttgcgttttcaactttcgccaccagttcagcatacgctaaattacggttgccatgatcgccagaataatcggtaaaatcgtagcccgcggtaatggaagttaacccggcataagcgggcaatgcgctaaaaatggccgccgctaataacgtccgttttatcattttaatctcctgtacggataagttcttgtcggagtgaataagttccggtaggtaaattacgttctacaatcacgcgcgggccaagttgcgtgttcggggaaataattcgcccaggcaaaataataacttgtacgccaaggcgtgaacgctgcccgatataacaacctaatttatcgcatccggtagcgataattccctctggagttcgaacagacacgggctgttcatccagacgatgattactggtacgtacttgtgcgcctaaatatgcctggtttgcaactaccgagtcggcaataaaacattgcggaccaatcgttgcttccgcttcaataaccgcatttttaatctcggtggcaaaaccaatttttacgccattgctgattattgtgccaggacgaataaacgcataattactagactggccccctgaatctccagacaaccaatatcacttaaataagtgatagtcttaatactagtttttagactagtcattggagaacagatgattgatgtcttagggccggagaaacgcagacggcgtaccacacaggaaaagatcgcaattgttcagcagagctttgaaccggggatgacggtctccctcgttgcccggcaacatggtgtagcagccagccagttatttctctggcgtaagcaataccaggaaggaagtcttactgctgtcgccgccggagaacaggttgttcctgcctctgaacttgctgccgccatgaagcagattaaagaactccagcgcctgctcggcaagaaaacgatggaaaatgaactcctcaaagaagccgttgaatatggacgggcaaaaaagtggatagcgcacgcgcccttattgcccggggatggggagtaagcttagtcagccgttgtctccgggtgtcgcgtgcgcagttgcacgtcattctcagacgaaccgatgactggatggatggccgccgcagtcgtcacactgatgatacggatgtgcttctccgtatacaccatgttatcggagagctgccaacgtatggttatcgtcgggtatgggcgctgcttcgcagacaggcagaacttgatggtatgcctgcgatcaatgccaaacgtgtttaccggatcatgcgccagaatgcgctgttgcttgagcgaaaacctgctgtaccgccatcgaaacgggcacatacaggcagagtggccgtgaaagaaagcaatcagcgatggtgctctgacgggttcgagttctgctgtgataacggagagagactgcgtgtcacgttcgcgctggactgctgtgatcgtgaggcactgcactgggcggtcactaccggcggcttcaacagtgaaacagtacaggacgtcatgctgggagcggtggaacgccgcttcggcaacgatcttccgtcgtctccagtggagtggctgacggataatggttcatgctaccgggctaatgaaacacgccagttcgcccggatgttgggacttgaaccgaagaacacggcggtgcggagtccggagagtaacggaatagcagagagcttcgtgaaaacgataaagcgtgactacatcagtatcatgcccaaaccagacgggttaacggcagcaaagaaccttgcagaggcgttcgagcattataacgaatggcatccgcatagtgcgctgggttatcgctcgccacgggaatatctgcggcagcgggcttgtaatgggttaagtgataacagatgtctggaaatataggggcaaatccaattacctatcaggcagtttgcgccaatcactaccggaccctgaataacggcaccatgacaaatacgggtattcgcgccgataacaacttcacctgcagtttcatcaataattacctggtctgcaatctgaatatttttctctttaacattaagcttcagatagtttttcagttcctgtgacagaaggttgggaataagcggttgacgcttccaccagtgcggaatagcgggtgggtttgtcgcgctgaggttcgcgtccagtaaaaaaggcaataagtccataaataatccagatggcataagctaataatacatacacaacggaaagcggcgctaaaggcaccaacaaccagcaacgatgaaaccaggcgctaaaagcaccaataacacaaactacgccgacccagataagcggaaacattgccaacaccactccatgcggcccggtggtgatgaattcattaaaccaggtagtgagataaatcccaacgccataaagcacaaccaacagcataggaaatatactgaagataccgaagcggctaaataaaagtcttttatgcaggcgcatacagaccgcgtatcccacaatccaacgccgccagcgacgccactcctcacgcgggctgttgcattcctgtgggtatacgatgcagcgattcgcctgccgaatacggtagccgtttgccaccaatgtccaggtgagatcaaggtcttcgactttagtacgatccgagaaaccgaacttacgcaatacatcagtacggaacatcccgcaggcaccgctgataataaacggtgcgccacccaggagctgctgtagcgtgcgcttcataacaatcatcggcaactttacggtcgcgcggatgtgcggtaacagacccgcgcctttcaacgcagtagagggaatgccgcctacggcatcggcaccgcgctcaatttctgccagcatatagcccattccgtcttgatcgggcggaacataggtgtcggcatcacttaaaaaaacctggtcgcaggtggcgtaattgaggccattcatcagcgcaccacctttaccggtatttttttgcgtgacggcaacaaagcggtcgccccatttgcgtttgacttccgccatgaccgcttcggtattgtccgtggagccgtcgttaacgcaaattacccggcaaaaataagggttacgcagtagattatccagtgactgcgccagacacgggccttcgttatacgcaggtataatggcgtcaatacagcctttcttttgactgggtttacgtcttagcgtacttaaaaaccatagcaacattgctatggacatacagataaatatccaggttttcatgcaatttgctcaaagaatcattttatgaattacaaagccttcacccagatcgctattgacctgttgtccgcgaaattgtgcaactgcacgcaggcgatcatgacgcatataatcgcgtcgttcctagcttttatgtttttttaatgcagcaagtttgactgtgaaatattcttctttaacggattcaaaaacctgaggcataaatgaaagccaggtacttggggtttcgtagccgagaatttgcggaatagttcggcaggcaaccattgaagcttgataaacagcaagatgatcctgatggcggtcggcatcatgcatggtatatacccgcatgatttcaacatcagaaggaatttgatttttaatgatgtcttccagggcggaaatcatatcattgagctgtaaatgagcgcgggtgtcagcaaaattaagatgaatagtttggtggcaccctaatatctttagggcgttgcgcgattcttcatggcgatcgattattccatctgtgccagagttgccggtagtcatcaccacggctgcgatataaattcctttttgcgcaagacgagcaagcgatgcgccacagcctaattctatatcgtcaggatgtgcgccaatagcaaggataccctttcttttatttgccgaagaaaggagggctgaatctaaaaccttatccacttaatgacactccattttatttattatactacaagcacaacgatgcactcagagacgtaatctctggcgcagccagatgttaatttataaatgttaaatgttgctaataactgaaaagcaagggctttcagacccgtgggttcgactgggtaatgtttctatgcaattcatatgttaagtgtttgtatgtttggtatgtatagttattttgttttatacattgtatttagatgtgatttagtttgtcaattaattgcatttaaaaaatatgttctgtgaacaagcattgtttatatacattatgtgaatgtaatatgcgagtgattgagaatgatacagtgatatatacaatgcgaatataatagttttattatatgtattgatattgatagaaataatgaagtaataaatctcgtaatgtggttgtttatgcatcactaaaatgaagtgtagtaattttcccaattgttagaacggagtaattgcatatttaatctttccttagccgtttttttgctaagaataaaatcatctgtgcgataacgactaattcttttaatgaatgtttttattcctgaatactgctcccataacaagacaggggagcagacaatcatggcaatttcatcgcgtaacacacttcttgccgcactggcattcatcgcttttcaggcacaggcggtgaacgtcaccgtggcgtatcaaacctcagccgaaccggcgaaagtggctcaggccgacaacacctttgctaaagaaagcggagcaaccgtggactggcgtaagtttgacagcggagccagcatcgtgcgggcgctggcttcaggcgacgtgcaaatcggcaacctcggttccagcccgttagcggttgcagccagccaacaggtgccgattgaagtcttcttgctggcgtcaaaactgggtaactccgaagcgctggtggtaaagaaaactatcagcaaaccggaagatctgattggcaaacgcatcgccgtaccgtttatctccaccacccactacagcctgctggcggcactgaaacactggggcattaaacccgggcaagtggagattgtgaacctgcagccgcccgcgattatcgctgcctggcagcggggagatattgatggtgcttatgtctgggcaccggcggttaacgccctggaaaaagacggcaaggtgttgaccgattctgaacaggtcgggcagtggggcgcgccaacgctggacgtctgggtggtgcgcaaagattttgccgagaaacatcctgaggtcgtgaaagcgttcgctaaaagcgccatcgatgctcagcaaccgtacattgctaacccagacgtgtggctgaaacagccggaaaacatcagcaaactggcgcgtttaagcggcgtgcctgaaggtgacgttccggggctggtgaaggggaatacctatctgacgccgcagcaacaaacggcagaactgaccggaccggtgaacaaagcgatcatcgacaccgcgcagtttttgaaagagcagggcaaggtcccggctgtagcgaatgattacagccagtacgttacctcgcgcttcgtgcaataaaaggaggcgcagatgctgcaaatctctcatctttacgccgattatggcggcaaaccggcactggaagatatcaacctgacgctggaaagcggcgagctactggtggtgctggggccgtccggctgcggtaaaaccaccctgctgaatctgattgccggttttgtgccttatcagcatggcagcattcaactggcgggtaagcgtattgagggaccgggagcagagcgtggcgtagtttttcagaatgaagggctactaccgtggcgcaatgtacaggacaacgtggcgttcggcctgcaattggcaggtatagagaaaatgcagcgactggaaatcgcgcaccagatgctgaaaaaagtggggctggaaggcgcagaaaaacgctacatctggcagctttccggtggtcaacgtcagcgggtggggattgctcgtgcgctggcggcgaatccccagctgttattactcgacgaaccgtttggtgcgctggacgccttcacccgcgaccagatgcaaaccctgctgctgaaactctggcaggagacgggcaagcaggtgctgttgattacccacgatatagaagaagcggtgtttatggcgactgaactggttctgctttcatccggccctggccgtgtgctggagcggctgccgctcaactttgctcgccgctttgttgcgggagagtcgagccgcagcatcaagtccgatccacaattcatcgccatgcgcgaatatgttttaagccgcgtatttgagcaacgggaggcgttctcatgagtgtgctcattaatgaaaaactgcattcgcggcggctgaaatggcgctggccgctctcgcgtcaggtgaccttaagcattggcacgttagcggttttactcaccgtatggtggacggtggcgacgctgcaactgattagcccgctatttttgccgccgccgcaacaggtactggaaaaactactcaccattgccggaccgcaaggctttatggacgccacgctgtggcagcatctggcagccagtctgacgcgcattatgctggcgctatttgcagcggtgttgttcggtattccggtcgggatcgcgatgggacttagccctacggtacgcggcattctggatccgataatcgagctttatcgtccggtgccgccgctggcttatttgccgctgatggtgatctggtttggtattggtgaaacctcgaagatcttactgatctatttagcgatttttgcaccggtggcgatgtcggcgctggcgggggtgaaaagcgtgcagcaggttcgcattcgtgccgcccagtcgctgggtgccagccgtgcgcaggtgctgtggtttgtcattttgcccggtgcgctgccggaaatcctcaccggattacgtattggtctgggggtgggctggtctacgctggtggcggcggagctgattgccgcgacgcgcggtttaggatttatggttcagtcagcgggtgaatttctcgcaactgacgtggtgctggcggggatcgcggtgattgcgattatcgcctttcttttagaactgggtctgcgcgcgttacagcgccgcctgacgccctggcatggagaagtacaatgagtgaacgtctgagcattaccccgctggggccgtatatcggcgcacaaatttcgggtgccgacctgacgcgcccgttaagcgataatcagtttgaacagctttaccatgcggtgctgcgccatcaggtggtgtttctacgcgatcaagctattacgccgcagcagcaacgcgcgctggcccagcgttttggcgaattgcatattcaccctgtttacccgcatgccgaaggggttgacgagatcatcgtgctggatacccataacgataatccgccagataacgacaactggcataccgatgtgacatttattgaaacgccacccgcaggggcgattctggcagctaaagagttaccttcgaccggcggtgatacgctctggaccagcggtattgcggcctatgaggcgctctctgttcccttccgccagctgctgagtgggctgcgtgcggagcatgatttccgtaaatcgttcccggaatacaaataccgcaaaaccgaggaggaacatcaacgctggcgcgaggcggtcgcgaaaaacccgccgttgctacatccggtggtgcgaacgcatccggtgagcggtaaacaggcgctgtttgtgaatgaaggctttactacgcgaattgttgatgtgagcgagaaagagagcgaagccttgttaagttttttgtttgcccatatcaccaaaccggagtttcaggtgcgctggcgctggcaaccaaatgatattgcgatttgggataaccgcgtgacccagcactatgccaatgccgattacctgccacagcgacggataatgcatcgggcgacgatccttggggataaaccgttttatcgggcggggtaatacgagagtggacggtcccctcgcccccttggggagagggttagggtgagggggcgttcaccgtactttcaacaggttaactccccctttctgagaggaaacaaaattaacgcagaatcttcttctcagccaaatccagcgcaaagtagctgaaaatcagatccgcacccgcacgcttaatcgaacctaagctttcgagcacgactttctcttcatctatagcacccgccagcgcggcgaacttaatcatcgcatactcaccgctcacctgatacgcgccaatcggcaattcagtacgttcacgcagctcacgcacgatgtcgaggtacgctccagcaggtttaaccatcaggcagtctgcgccctgggcttcatccagcagtgattcacgaatcgcctcacgacggttcattgggttcatctgatagcttttgcggtcgccttttaatgcgcttccggcagcttcacggaacgggccataaaaggaggaggcgaacttggtcgaatacgacataatcgccgtatctttaaatcccgcagcgtccagcgcctgacgaatcgcctgtacctggccgtccatcgcggcggaaggggcgatgaagtctgcacctgcagcagctgcaaccacggcttgcttgcctaaattttccagagtcgcgtcgttgtcgacgccatgctcgcacagcacaccgcagtgaccgtgagaagtgtattcacagaagcaggtgtctgacataacgatcatttctggcacggtctgcttgcagatgcgcgacatacgcgccaccagtccatcttcccgccaggcatcgctgccggtttcatcggtatggtgagagatgccaaaagtcatcacggaacgaataccggcgttggcgatgcgttcaatttcgcgtgccagatgtttctctggaatgcgcatcacgcctggcatggcttcaacggctttgtagtcgtcaatttcttcttcaacaaagatcggcaacaccaggtcgttaaggctaagtgttgtctcttcaaacatagcgcgcagcgcaggagatttgcgcaggcgacgagggcgttggattaagtctgtcatggtctgcctgatgtttgtggaatcgaggggcatagtatacctgaagcagggtagggatgttttacgaaagttgtcgcgatgttgacaagaagagaatggaagagaggccaggacatctttttaatagaaacagcaataattttatattcactgaaaatatttttaatctttatttatagctgttggttattattttttggagtttggttgcgctgctataaattgaataattaaaactttgttgcatattcataggatatttatctggtttgtgtttgtgatatttattatgcgtatgcttcaaaaacaaaattatctgcaacatgttgaaatactgtgcttttatgaatttgatgcgtgtttttctccataaattatatatgtccacattcggacttaggggaaagaataattgaaccattcgtctgtaacgcagcataatcgttagcgcgaaacataatatgttttctatgcattgataattgatggatcaacttattacgtccctgaggagggatgacaaatgcactcctggaaaaagaaacttgtagtatcacaattagcattggcttgcactctggctatcacctctcaggctaatgcagcaaactatgatacctggacttatatcgataatcccgttacagcacttgattgggatcatatggataaggcaggcactgtagatggcaactatgtaaactatagtggttttgtctattacaacaacaccaatggtgatttcgatcagtcctttaacggcgataccgttaacggcacgatctcaacctattatttgaaccatgattatgcagacagtactgctaatcagcttgatatcagtaattcagtgattcacggttcgattacttctatgctgcctggcggttattatgatcgttttgatgcagatggtaataatctgggtggatatgatttttacactgatgcggttgttgatacacactggcgtgatggtgatgttttcactttgaacattgctaacactactattgatgatgattatgaagctctttacttcactgattcttataaagatggtgatgtaaccaagcacacaaatgagacatttgatacaagtgaaggcgttgctgttaatcttgatgtagaaagtaacatcaatatttccaataactcccgcgttgcaggtattgcattatctcaaggtaatacttacaacgaaacctacactaccgaatctcatacttgggataacaatatctctgtaaaagattccacagtgacttcgggttcaaattatatcctggatagcaatacttatggcaaaactggtcactttggcaattctgatgaaccgagtgattatgctggcccgggtgatgttgcaatgtcctttactgcttcaggttccgactatgcgatgaagaacaatgtattcctcagcaattcaacgctgatgggtgatgttgcctttaccagcacctggaatagtaattttgatccgaatggtcatgattccaacggtgacggggtgaaagataccaacgggggttggactgatgatagcctcaacgttgatgaactaaatctcactctcgataacggaagcaagtgggttggtcaggcaatttataacgttgctgaaacgtcagcaatgtatgatgttgctacaaacagccttactcctgatgcaacatatgaaaacaatgactggaaacgtgttgttgatgacaaggtcttccagagcggtgtatttaacgtagcgttgaataacggttctgaatgggatactacaggtcgttccatcgttgataccttgacagttaataatggttctcaggttaatgtttcggaatctaaattaacttcagatactatcgatttaactaacggttcttcgctgaacattggtgaagatggctacgttgataccgatcatctgactattaactcctacagtactgttgcgttgaccgaatctactgggtggggggctgattgatcctacccacgtaatatggacacaggcctaagcgaggttcttgttttcaaattgttccggactgaggccgccacaccaactgtgccgccgccaccgattgtaatcacattcgatataattaaacaccgttgcccgcattatttcccggctgataaagtgttctccatggatacattccactttcagcgaatgaaagaagctttccacgcaggcattatcgtagcagcaaccttttgcgctcatacttccacgcagattatgccgcttcagttgcgcctgataatctgctgaacagtactggcctccacggtccgtgtgaacgataacgttccggggcctcttacgccgccacagcgccatctgcagggcatcgcaggccagttgcgccgtcatgcgtggcgacattgaccagccaataacggcacgtgaccacaggtcaatgaccactgccagatacagccagccttcatctgtacgtaagtacgtgatgtctcctgcccacttctggttcgggccactggcgtaaaaatcctgctccaacagattttctgacacaggcaggccgtgtgcgcggtagctgaccgggctgaacttccgggaggcctttgccctcagtccctgacggcgcaggcttgccgccacggtttttacgttaaaggggtaaccctgagcacgcagttcatccgtcaggcgtggggcaccgtaacgctgttttgaccgggtaaaagccgcgaggacaacgctgtcgcagtgttggcggaactgctgacgcgtgcttatccttgtccgccgctgacaccacgtataccagccgctgcgggccacccggagcacgcggcacattgctttgatgctgaactcagcctgatgtttttcaataaagacatacttcatttcaggcgcttcgcgaagtatgtcgcggccttttggaggatagccagctcttcatcccgttctgccagctggcgtttgagacgtgcaatctcggtagacatctccagttcacgttcagaagacgtctgctgattttgctgtttactgcgccagttgtagagttgtgattcatacaggctgagttcacgggctgcggcagtaacaccgatgcgttcagcaagcttcagggcttcactgcgaaattcaggcgaatgctgtttacggggttttttactggttgatactgtttttgtcatgtgagtcacctctgactgagagtttactcacttagccgcgtgtccactattgctgggtaagatcagattacaacctgtacgccaatactatcaccgtaactaacggcggtgtattggatgtgaacgttgatcagttcgatactgaagctttccgtactgacaaactggaactgaccagcggcaacatcgctgaccataacggtaacgtagtatctggtgtgttcgatatccatagcagcgattacgttctgaacgctgatctggtgaacgaccgtacctgggatacttccaagtctaactacggttacggtattgttgctatgaactctgatggtcacctgactatcaacggtaacggcgacgtagacaacggtactgaactggataacagctctgtagacaatgttgttgctgcaaccggtaactacaaagttcgtatcgacaacgcaactggcgctggcgctatcgctgattacaaagataaagaaattatctacgtaaacgacgtcaacagcaacgcgaccttctctgctgctaacaaagctgacctgggtgcatacacctatcaggctgaacagcgcggtaacaccgttgttctgcaacagatggagctgaccgactacgctaacatggcgctgagcatcccgtctgcgaacaccaatatctggaacctggaacaagacaccgttggtactcgtctgaccaactctcgtcatggcctggctgataacggcggcgcatgggtaagctacttcggtggtaacttcaacggcgacaacggcaccatcaactatgatcaggatgttaacggcatcatggtcggtgttgataccaaaattgacggtaacaacgctaagtggatcgtcggtgcggctgcaggcttcgctaaaggtgacatgaatgaccgttctggtcaggtggatcaagacagccagactgcctacatctactcttctgctcacttcgcgaacaacgtctttgttgatggtagcttgagctactctcacttcaacaacgacctgtctgcaaccatgagcaacggtacttacgttgacggtagcaccaactccgacgcttggggcttcggtttgaaagccggttacgacttcaaactgggtgatgctggttacgtgactccttacggcagcgtttctggtctgttccagtctggtgatgactaccagctgagcaacgacatgaaagttgacggtcagtcttacgacagcatgcgttatgaactgggtgtagatgcaggttataccttcacctacagcgaagatcaggctctgactccgtacttcaaactggcttacgtctacgacgactctaacaacgataacgatgtgaacggcgattccatcgataacggtactgaagggtctgcggtacgtgttggtctgggtactcagtttagcttcaccaagaacttcagcgcctataccgatgctaactacctcggtggtggtgacgtagatcaagactggtccgcgaacgtgggtgttaaatatacctggtaatattcttcactccgaagaaatactggtaatttaatctaaataatgcccgtcaaggatttgacgggcattactgcaaaggacgcgcaaatgttatctgtagttaaacctcttcaggaatttggtaagctcgataaatgtttgtccagatacggtacgcgcttcgagtttaataatgaaaagcaagttatattttccagtgatgtcaataacgaagatactttcgttattttagagggagttatctctctgcgtagagaagaaaacgtacttatcggtattacccaggctccttatattatggggctggctgatggtttaatgaaaaacgatataccatacaaattaatatcagaaggaaattgtacgggatatcatctaccagccaaacaaaccattacgcttattgaacaaaatcaactctggcgagacgctttttactggttagcctggcaaaatagaattctggaattacgcgacgtgcagctcattgggcataattcctacgaacaaatccgcgcaacattattatcaatgattgactggaatgaagaattgcgatcacgtattggtgtgatgaattatatccatcaacgtacacgcatatcgcgttctgtcgtcgcagaagttctcgctgctttgcgtaaaggcggctatatcgaaatgaataaaggcaaactggtcgctatcaaccgtttgccttcagagtattaatcaggacgcggggataaccaacggtttattcccgcttagctcggtcaccaggtcattgatgccatcgctcatatttttaaagcgcgtcaacggcgaacgagtgaccaccacaaacgcgccaatattcttctgcgggatcatcgccatataggtaatgaaaccgccaccaccgcctgtcttctgaataatccccggacgaccctctttcggggccatatatacccaacctaaaccaagcgcatccgctttgccggggacatccatgccaatcactttcgtaaactgcgcgcgctgataaatcaacgtctgcatgcgatctgcctggttactgcgctgataaaaatcagatgacaaatactgctgcatccagcgcatcatatcgccaggcgtggaatagacgccgccgctgccaattgccgccagcgtgttattgcacggactggcaccgcgctcagcaaccattaaacggcggcactgatccggtgagggggtgtaggtggtgtctttcatccccaatggacgggtaatctgctcttcaaacaactgggtataaggcttgccggacgcattcgccagtgcatctgccagcaggtcgaacgcaaggttagagtacgccgcctgactgcctggcgcggctttcagcttcgccgtagaaaggtatttccagcgttgctcgcgcgttggccagacaaacaccggacgatgtgccgcgccaccgggctgttcacggggcagggcgctggtatgggttgccagattgaccagcgtaatgggcgtcccattgtaggttggcacgcgtgcgcctggcggagcatatttacttagcggatcgtttaacttcacggtcccctggtcgagcaatttcaccagcatctcactggtcattagcttggtgagggaagcaatacgcacgaccgaatccagctgcgggcgaacgttattaccaggtcgcgtttcgccataactgcgaaagacgcgctggttaccgtcgataacaaccagagccatccccgtggcaccgctgccgtaaaaaatatgatcggcataacgatcgacaatatcagaggcaaactccggttcagtgatcggctgcgccgcatggacggaggtcaatgacgccgcacacagcacggcagaaaaaagcagactacgtttcaacggtggtgtccatagattgaatgaaggtaactgagcgtatttatactactcattgatagattgcaaagggcgaattagtgcaataatagtgttaaaaacgtaacggcgcgtaaacacgatctttttcctgctcaccaatgcctgcatttgtgatcctgcgcgtgttaatccgcttatgtaaacaatctttggtttgtgaaatccgtcgaaacaattcttatggtcaggctggcgaactaagcgccttgctatgggtcacaatgggcggtttcatttggctgacgctttgtagcggtcatgcggttaatacacagcagttgttaaaacgataagaagttagcaggagtgcatatgtttaagtcttttttcccaaagccgggaacgttttttctctcggccttcgtttgggcattgattgccgttatcttctggcaagccggtgggggtgactgggtggcgcgtatcaccggcgcttccgggcagatcccgattagcgccgcgcgtttctggtcgttggatttcctgattttttacgcttactacattgtttgcgtaggactttttgcattgttctggtttatctacagcccgcatcgttggcaatactggtcaatactcggtactgcactgatcatcttcgtcacctggtttttggtggaagtcggggtcgccgtcaacgcctggtatgcgccgttctatgatctgattcaaaccgcgctaagttcgccgcataaagtcaccatcgaacaattttaccgcgaagtgggcgtctttctggggattgcgctgatcgctgtggtgatcagtgtgctgaacaacttctttgtcagtcactacgtgttccgctggcgtacagcgatgaacgaatattacatggcgaactggcaacaactgcgtcatatcgaaggggccgcacagcgtgtgcaggaagacaccatgcgttttgcttcaacgctggagaatatgggcgtcagttttatcaacgccatcatgacgttgatcgccttcctgccggtgctggtaacgctctccgcgcatgtgccggagctgccgattatcgggcacattccgtatggtctggtgattgccgcaatcgtctggtcgctgatggggaccggattgctggcagtggtagggatcaaactgccggggctggagtttaaaaaccagcgtgtagaggctgcctaccgtaaagagctggtttatggtgaagacgatgccacgcgcgcgacgccgcctacggtacgcgagctgtttagcgccgtacggaaaaactatttccgcctctattttcactatatgtatttcaacatcgcccgcattctctatttgcaggtcgataacgttttcggtttgttcttgctgtttccgtcaattgttgccggtacgattacgctcggcctgatgacgcagattaccaacgtttttggtcaggttcgcggtgctttccagtacctgattaactcatggaccacactggttgagttgatgtctatctacaaacgtctgcgcagctttgaacatgagctggatggtgacaaaattcaggaagtaacccataccttgagctaaaaaggagaagtaatgtcgcgcgtcaatcctctatcttcgctgtcattgttggcggttctggttttagcggggtgtagtagtcaggctccgcaaccgttgaaaaagggcgaaaaagcgatagatgtagcgagcgtcgtgcggcagaagatgcctgcgagcgtgaaagaccgcgatgcctgggcgaaagatctcgccaccacctttgaaagtcaggggctggcaccgacgctggaaaacgtctgctcggtgctggcggtggcgcagcaggagtcaaattatcaggcagatccggccgttccgggcttaagcaagatcgcctggcaagagattgaccgtcgtgctgaacggatgcacattcctgcttttctggttcataccgcgctaaaaatcaaatcgccaaacggcaaaagttatagcgaacggttagattcggtgcgtacagaaaagcaattgagcgcgatttttgacgatctgatcaacatggtgccaatggggcagacgctgtttggttcgctcaatccggtgcgcaccggtgggccgatgcaggtcagcattgcttttgccgaacagcataccaaagggtatccgtggaaaatggacggtacagtccgtcaggaagtcttcagtcgccgcggcgggttgtggtttggtacttaccatttactgaattatcccgccagttatagcgcaccgatataccgttttgctgattttaacgctggctggtacgccagccgtaatgccgcgtttcagaacgcggtcagtaaggccagcggcgtgaagctggcactggacggtgatttaattcgttacgacagtaaagaacccgggaaaaccgaactggcaacgcgcaaactggctgcaaaactggggatgagcgacagcgaaattcgccgtcagttagagaaaggtgacagcttctcttttgaggagacggcgctgtacaagaaagtttatcaacttgccgaaacgaaaacgggtaaatcactcccccgcgaaatgttgcctggcattcaactggaaagcccgaaaatcacccgcaacctgactacggcctggtttgcgaagcgcgtagacgaacggcgggcgcgttgtatgaaacagtgatcaaacaggaatgtcaggccagataaggcgtttcaggccgcatctgacaatgtaaaacttactggcggcgatgtcgccagtgcagccatagcgccaccactgcaaaaatgaggcagcctactaaaaacgggatcagcccgaaaatggtgccgacacctaaaccaatttccacccgtgggcgacctgtttcctggacctgcattaaacgctcatagacgccgggcgcatgcactaacaggttcagcaattgcgccccagcccaaaagcaaaacagcacaaacaacgcataggcaatgttgccaggcgttgaagaggcattgcgatattttccgctaaacagcgattttgacagggtgaaatcagccataaaaacctccggaagtcatctgcttctcttctggtgtgataccagcggcttatggcaagtctgacaggtcatttagattgtcaatatcagaatcatggtaaattgatgttgggaatattcccgaagcgtgaatcttcgttgtgagtcacaaaatggcaaccttaagttaaatttattaacaattacgaaaatgttgtctacaccacagacggttgttgcagaatatgcaaggatgttgtttttcgttaacggagctgccatgaatctgcctgtaaaaatccgccgtgactggcactactatgcgttcgccattggccttatattcattcttaatggcgtggtggggttactgggatttgaagcaaaaggttggcagacctatgccgtcggtctggtgacgtgggtgattagtttctggctggcggggttgattattcgtcgtcgcgatgaagaaactgaaaacgcccaataagaatattatcgggcgttaaaatattacattgtggttttcaatgcgttatccgcagcgtgacgctccagcgccagttcaatcaaacgtgtgatcagatcggtgtaacccagaccgctggcttgccacagcttcggatacatactgatattagtgaagccaggcagggtgttgatctcgttgatcaccacttcgttctctggggttaaaaacacgtctacacgcgccatgcctgcgcatcccaacgtttgataagcctgaacggcaatcgcccggatcttatcgttgatttctggcgcaatggctgccggaactaccactttcgcgccatcttcgtcaatgtacttggtgtcgtaggcatagaaatcgctggtgagtacgatctctccacaggtgctggcttgcggattgtcgttgcccagaactgcgcattcgatctcacgacctttgatcccttgctcaacgatcactttatgatcgaactcgaacgccagatcgacggcaattgcgtactgttcttcactggttactttgctgacaccaacagaagagccctgattagccggttttacaaacagtggtaaccccagtttagactccacttcggcaaaactaatgttgtgacgattggcgcgcgtcagggtaataaatggcgcaatgttcagcccggcatcgcgtagcagacgtttggtgacatctttgtccatacaggctgctgaagccagaacatcagaacctacaaacggtaaattggcgacccgcagcattccctgcaaggaaccatcttcgcccagcgtaccgtggacaatcgggaaaatgacatccaccgtcggcaacggctgaccgttttgcgcgtcgataagctgatgctcatgtttacctggcacctgcgcaaggctggtcgccgaagggcgcaacgcaatatgggcaggatcgtctgcatttagcagataattgctggcatcgctgacgtgccattgcccttgtttatcaatgcccagcagcacaacgtcgaagcgacttttatcaatggcatcgacaatgttttttgccgattgcagagacacttcatgttccgctgatttaccaccaaaaacgattcctacccgcagtttttccatcttaaaaacctatcccgtctaacacaaagtgcatacattaccacgacaaaacgggggattcgcggccttctgaaagattgttgcaatcttctgctgacaaagcgtgcaacgtactggtgaagaaagtgcgttatctcaaagatgtgcgcaagatcacaaaaatgatgaacgggaagctaatttattcctggcttaaatggccatgcggtgagtttttttctcttaattataagttaacgaagagaatatatttcataacttttatttataataaaggttgataattaaaagcctatattttgtgtgggtaattatttaaataagagaaacgtttcgctggtaatcaaacaaaaaatatttgcgcaaagtatttcctttgtcataaaaataatacttccagacactatgaagttgtgaaacataatgttaacttctccatactttggataaggaaatacagacatgaaaaatctcattgctgagttgttatttaagcttgcccaaaaagaagaagagtcgaaagaactgtgtgcgcaggtagaagctttggagattatcgtcactgcaatgcttcgcaatatggcgcaaaatgaccaacagcggttgattgatcaggtagagggggcgctgtacgaggtaaagcccgatgccagcattcctgacgacgatacggagctgctgcgcgattacgtaaagaagttattgaagcatcctcgtcagtaaaaagttaatcttttcaacagctgtcataaagttgtcacggccgagacttatagtcgctttgtttttattttttaatgtatttgtacatggagaaaataaagtgaaacaaagcactattgcactggcactcttaccgttactgtttacccctgtgacaaaagcccggacaccagaaatgcctgttctggaaaaccgggctgctcagggcgatattactgcacccggcggtgctcgccgtttaacgggtgatcagactgccgctctgcgtgattctcttagcgataaacctgcaaaaaatattattttgctgattggcgatgggatgggggactcggaaattactgccgcacgtaattatgccgaaggtgcgggcggcttttttaaaggtatagatgccttaccgcttaccgggcaatacactcactatgcgctgaataaaaaaaccggcaaaccggactacgtcaccgactcggctgcatcagcaaccgcctggtcaaccggtgtcaaaacctataacggcgcgctgggcgtcgatattcacgaaaaagatcacccaacgattctggaaatggcaaaagccgcaggtctggcgaccggtaacgtttctaccgcagagttgcaggatgccacgcccgctgcgctggtggcacatgtgacctcgcgcaaatgctacggtccgagcgcgaccagtgaaaaatgtccgggtaacgctctggaaaaaggcggaaaaggatcgattaccgaacagctgcttaacgctcgtgccgacgttacgcttggcggcggcgcaaaaacctttgctgaaacggcaaccgctggtgaatggcagggaaaaacgctgcgtgaacaggcacaggcgcgtggttatcagttggtgagcgatgctgcctcactgaattcggtgacggaagcgaatcagcaaaaacccctgcttggcctgtttgctgacggcaatatgccagtgcgctggctaggaccgaaagcaacgtaccatggcaatatcgataagcccgcagtcacctgtacgccaaatccgcaacgtaatgacagtgtaccaaccctggcgcagatgaccgacaaagccattgaattgttgagtaaaaatgagaaaggctttttcctgcaagttgaaggtgcgtcaatcgataaacaggatcatgctgcgaatccttgtgggcaaattggcgagacggtcgatctcgatgaagccgtacaacgggcgctggaattcgctaaaaaggagggtaacacgctggtcatagtcaccgctgatcacgcccacgccagccagattgttgcgccggataccaaagctccgggcctcacccaggcgctaaataccaaagatggcgcagtgatggtgatgagttacgggaactccgaagaggattcacaagaacataccggcagtcagttgcgtattgcggcgtatggcccgcatgccgccaatgttgttggactgaccgaccagaccgatctcttctacaccatgaaagccgctctggggctgaaataaaaccgcgcccggcagtgaattttcgctgccgggtggtttttttgctgttagcaaccagacttaatggcagatcacgggcgcatacgctcatggttaaaacatgaagagggatggtgctatgaaaataacattactggttaccttgcttttcggtctggtttttttaaccaccgtcggcgctgccgagagaactttaaccccacaacaacagcgtatgacctcctgtaatcagcaggcgacggcgcaggcgttgaaaggggatgctcgtaagacctacatgagtgattgcctgaagaacagcaagtctgcgcctggcgaaaaaagtttgacgccacagcagcaaaagatgcgcgaatgcaataatcaagcaacacaacaatctctgaaaggtgatgatcgtaataagtttatgagtgcctgcctcaagaaagccgcctgatacctgatagtgctaacgggtgagctacgaaaatggctcacccgaaatatcatacttctgcctttagctccgtctctataatttgggaaaattgtttctgaatgttcccaaaaataatgaatgatgaaaactttttcaaaaaagcggcggcgcacggggaggaacctcctttaactcctcaaaacgaacatcagcggtccgggctgcgcttcgcccgtcgcgtcagactaccccgtgcggttggcctggctggcatgttcttaccgattgcttcaacgctggtttcacacccgccgccgggctggtggtggctggtgttggtcggctgggcgttcgtctggccgcatttagcctggcagatagcgagcagggccgtcgatccgcttagccgggaaatttacaacttaaaaaccgatgcagtattagcgggaatgtgggtaggcgtaatgggcgtaaacgtgctgccttccaccgcgatgttgatgattatgtgtctgaatttgatgggggcaggcggcccccgtctgtttgtcgcgggtctggtgttgatggtggtttcctgccttgtcaccctcgagctgacgggcattaccgtgtcgttcaatagtgcgccgctggaatggtggctctcccttcccattattgtcatttatcctctgctgtttggctgggtcagctaccagacggcaaccaaactggcggaacataaacgcaggttgcaggtcatgagtacccgcgacggcatgacgggcgtgtataaccgacgtcattgggaaactatgttacgcaatgaatttgataactgtcggcggcataatcgcgatgcaacgttactgattatcgatatcgaccatttcaagagcatcaacgatacctggggccatgatgtgggcgatgaagcgattgtggcgcttacccgacagttacaaattaccctgcgcggtagcgatgtgattggtcggtttggcggcgatgagtttgcagtaatcatgtccggtacgccagctgagagcgccattaccgccatgttacgggtgcatgaagggctaaatacattacgtttgccgaatacgccacaggtaactttacggattagtgtgggggttgcgccgctgaacccacaaatgagtcactatcgtgagtggttgaaatcggcagatttggcgctttacaaagcaaagaaagccggacgtaaccgcaccgaagtggcggcctgacgtccggcgaaagtcatcaggatttgctgagtttttctgatttttccatacacttcgtcatcgcttcgatcactgcagcacggaagcctttctcttccagtacgcgtaccgcttcaatggtggtgcctcccggtgagcagaccatatctttcagtgcccccggatgttctcccgtttccagcaccatttttgcggaacccattaccgcctgagcggcaaatttatacgcctgggcgcgtggcatcccgcccagcacggcggcgtcggccatcgcttcgataaacataaatacgtaggctggcgaagaaccgctcacaccgaccaccgggtggatcatcggctcagcaattacttccgcttcgccaaagcagcggaaaatattcagcacatcagcggtatcttctggggttaccagcgcgtttggcgttacggaggtcatcccggcattaaccagtgcgggagtgttcggcatggcgcggataattttccggtcatggcccagcgcgcgggcaagctggtcgagcgtgacacctgcagcaatagaaacgaccagagagtctttattcaggctggaggtgatttcgctaagcactttaatcatgatgccaggtttaacggcagcaaaaatgatgtcggcgatttgcgccacttcttgcgccgattctgcggcgttgatgccgaactggtcatgcagggcggcgactttatccggggagggggtgtatacccagatttgccctggaagcacctgaccgctggcaatcagaccgccgagaatggcttttcccatattgccgcagccaataaaaccgattttcttttccattgcctcactcctgccgtgaaattcattgttttgataatcgctggcagaagcataaacagaactatgccggaaggcaaaagcgcgacacaatagaggattacccaacaaaggatgactttatgacaatttgggtggatgccgacgcgtgtcccaatgtaattaaagagattttgtatcgcgcggcggaacgtatgcagatgccgctggtactggtagcaaaccagagtttacgcgtgccgccatcgcgatttattcgtacgctgcgcgtcgcggcaggtttcgacgttgccgataacgaaattgtccggcagtgtgaagcgggcgatttggtgatcaccgcagatatacctttggctgctgaagccatcgagaaaggcgctgcggcgcttaatccgcgcggcgaacgttacacgccagcgaccattcgtgagcgcctgacgatgcgcgattttatggataccttacgtgccagtgggatccagaccggcggaccagatagcctttcacaacgtgaccgccaggcctttgccgcggagctggagaagtggtggctggaagtgcaacgtagtcgtggctaaatgtaatttattatttacacttcattcttgaatatttattggtatagtaaggggtgtattgagattttcactttaagtggaattttttctttacaatcgaaattgtactagtttgatggtatgatcgctattctcatgacaccggctttcgccgcattgcgacctattggggaaaacccacgatgacacaacctctttttctgatcgggcctcggggctgtggtaaaacaacggtcggaatggcccttgccgattcgcttaaccgtcggtttgtcgataccgatcagtggttgcaatcacagctcaatatgacggtcgcggagatcgtcgaaagggaagagtgggcgggatttcgcgccagagaaacggcggcgctggaagcggtaactgcgccatccaccgttatcgctacaggcggcggcattattctgacggaatttaatcgtcacttcatgcaaaataacgggatcgtggtttatttgtgtgcgccagtatcagtcctggttaaccgactgcaagctgcaccggaagaagatttacggccaaccttaacgggaaaaccgctgagcgaagaagttcaggaagtgctggaagaacgcgatgcgctatatcgcgaagttgcgcatattatcatcgacgcaacaaacgaacccagccaggtgatttctgaaattcgcagcgccctggcacagacgatcaattgttgattttcgagcgcctatacttaacgttcatcccgtgaaataaggaagaacgatgccaacgaaaccgccttatcctcgtgaagcatatatagtgacgattgaaaaaggaaagccaggacagacggtaacctggtaccaactcagagccgatcatcctaaaccagactcgttgatcagtgaacatccgaccgctcaggaagcgatggatgcgaaaaaacgctatgaggaccctgacaaagagtgaccgcatcagactgctcggaagggattctgagtgccactacaagggatctgcgtcacatttttcataattcatgtttttctaataattagaatattaaacaataacaatccattactggaatcatttggaatctttacattatgccgtgcacgtctgctgctacgctttttgtcatttgtagcacaagtaagtgtcagcagtggtgcttcacacttgcccggtaattaacgacgaaagaaaagtaaggtggatgaacaatgagtgcgtcgttggcgatcctgaccatcggcattgtacctatgcaggaagttttgccgctcctgacggaatacattgacgaagataatatttcccatcatagcctgctggggaagttaagtcgtgaagaagtgatggcggagtacgcgccagaagcaggcgaagacaccattctcacattattaaatgacaaccagctggcccatgtttcgcgtcgcaaagtggagcgtgacctgcaaggtgtggttgaagtgctcgataatcagggttatgacgtcattttattaatgagtacagcaaacattagtagtatgactgcgcgtaatacgatctttcttgagccgtcgcgaatattgcctccactggtttcctctattgttgaagatcatcaggtgggggttatcgttccggttgaggagatgctgcccgttcaggcgcaaaaatggcaaattttgcagaaatcgccggtattttcattgggtaaccccattcatgattcagaacaaaaaatcattgatgccgggaaagaattactggcaaaaggggctgatgtcatcatgctggattgtttaggatttcaccaacgtcatcgcgatttactgcaaaaacagctcgatgttcctgtcttgctgtctaacgtattgattgcacggctggctgcggaattactggtgtaattttgcgtgacagccagcgcctctggcccctatagtgaagtagatgttcaactaccaaacagggccagtttatgcttcaaagtaatgagtacttttccggcaaagtgaaatcaatcggcttttccagcagcagcactggtcgcgccagcgtgggtgttatggttgaaggcgaatacaccttcagcaccgctgagccggaagagatgacggtaatcagtggcgcgctgaatgtgttactgcctgacgcgaccgactggcaggtgtatgaagccggttcggtgtttaatgttcccggtcacagtgagtttcatctgcaagttgccgaacccacctcttatctgtgccgctatctgtaattcctcgccttccccttgaacgggagggcatttttctgaaatatcctttctttagcccataataatatttcctttgctgcgattttttcaatttccgatatattcataatttatcaaggttgatataaatatcagtgaagatctccagatattgttgcggaactggctacgataaaagataaatcagatgatgaatggtggcgtgcattgctgcaaagtcgcaatgatcatttacgccaaacggcattgcgcaacgcacataccccggcgttgttgttaacgacattgactgagcctcaggatcggtcgctggctattaataatccacagctggctgccgatgtgaaaacggcgtggttaaaagaggatccatcattactcttatttgtcgaacaacccgatctttcgctgttacgtgatttagtgaaaaccggggcaacgcggaaaattcgcagtgaagcgcgtcaccggcttgaggaaaaacaatgacacaacgtccatggagcaagttacagcgtaaaacgcataatattgctgcgctaaaaattattgctcgccgtagcgaataattatatgcctggtgtggcttcgtacgccggataagacgcggcaggcgtcgcatccggcattaaaggaaaatcagcaattaacgttgtgcttcgccacctaatccttcaatcaggttttgaattaacgctgccagttcaccagtcatcaggatgaaatcggcatcaaaacgctgggcgaaatcttcacggtcgatatcttcgttttgatcgcgcagctcgtcgcagaacttcagacgcttgagcgaaccatcgtcgcacatcacaaactgaatgcgctgctgccagtcgagcgccagtttagtcaccacttttccggcttcaatgtgattggtgatctcttcgctggtcagatcttgtttcttcgcgcggatcacgccgccatcttccagcaacgatttcagctcggcttcatcaagcagctggaagccctgtgccgcactaccggagcgaacccattcggtcagcgtcagttcaatcgggttttccatgctcaatggtacaaccggtaacgaccccaggcttttacgcagtaatgccagcgtatcttccgcttttttggcactggcgcagtccaccataatcaaaccgttaaccgtgtcgatccacatcattgtctggctaaaacggctgaaagcacgcggcagcagagagtgcagcacttcgtctttcagcgaatctttttcggttttcttcagcttacgcgcctgttccgcttccagtttggcgattttcgcttccagcgcctgtttaatcaccggagacgggaggattttttcttctttgcgcgcgcagataacaatttgaccattggcaacgtgcgttaacgcatcgctgtgcgatcccatcggaggaacccagcccatcttcgccatgtcctggctgccgcatggggtaaatgccatcgaggctagctgtttttccatctcttctgcacgcagcgaaatctcgcggctaagacggtaaaccattaaatttttgaaccacagcatgataatttccacggccttgtcgttaaatttagcgggcatgataacgaattgtcggcggccttgcattgccaatccggttgtccgtctctacgctattgatattgaaaaaaataaggagagtaccgtgcgtataggtatcgatttaggcggcaccaaaactgaagtgattgcactgggcgatgcaggggagcagttgtaccgccatcgtctgcccacgccgcgtgatgattaccggcagactattgaaacgatcgccacgttggttgatatggcggagcaggcgacggggcagcgcggaacggtaggtatgggcattcctggctcaatttcgccttacaccggtgtggtgaagaatgccaattcaacctggctcaacggtcagccattcgataaagacttaagcgcgaggttgcagcgggaagtgcggctggcaaatgacgctaactgtctggcggtttcagaagcagtagatggcgcggcagcgggagcgcagacggtatttgccgtgattatcggcacgggatgcggcgcgggcgtggcattcaatgggcgggcgcatatcggcggcaatggcacggcaggtgagtggggacacaatccgctaccgtggatggacgaagacgaactgcgttatcgcgaggaagtcccttgttattgcggtaaacaaggttgtattgaaacctttatttcgggcacgggattcgcgatggattatcgtcgtttgagcggacatgcgctgaaaggcagtgaaattatccgcctggttgaagaaagcgatccggtagcggaactggcattgcgtcgctacgagctgcggctggcaaaatcgctggcacatgtcgtgaatattctcgatccggatgtgattgtcctggggggcgggatgagcaatgtagaccgtttatatcaaacggttgggcagttgattaaacaatttgtcttcggcggcgaatgtgaaacgccggtgcgtaaggcgaagcacggtgattccagcggcgtacgcggcgctgcgtggttatggccacaagagtaaaaaacgtaggcaattggcgcatcatgcctgatgcgacgcttgccgcgtcttatcaggcctacaaaaggtgccagaaccgtaggccggataaggcgttcacgccgcatccggcaataagtgctccgatgcctgatgcgacgcttgccgcgtcttatcaggcctgcaaaatgtgccagaaccgcgtagggcggataaggcgttcacgccgcatccggcaataagtaatgagcaccgagactataacctaccccagtggtttcgccagcaccggagtatccgccgcttgctggcgcttatagcgaccatacagcagcaacgacgacatcgcagcaaacgaaagcagggcggcaggcagcgccacgtaattatatgccagccccagcgtcagcatcatacctccgcaatatgcgccgacggcgctaccgaggttaaacgctatttgcccacctgcggcacctaataactctccgcctttggcgttttgtagtaacaatatttgtagcggtgctgaaagggcaaataatcccgcgcaacaaataaaagcaaaaataagcgacgttgttttcatgccgccgcagaaaaagagcatcagcagtgccagtacaattataaagtcagtcactgctgcaatgcgcagtggtgaataacgtcctgaaatcctgccacttagcatatttcccagcaccatccctagcccaactaacatcataataaaggtcatcgccgtttccgaaaaaccggaaataaacatcatgtatggctttacgtagctgaaccaggcaaacacacctgcgttgccaaacatcgtggcggcgaaaattaaccacggggccgggctgcgcaaaaagtgaaattgttcgcgcagatttcctttcgcctcgtcgcgaatatctggcacccaaaaatagaccgatgccatcaccgcaatattaaaaacagcgatcaataaaaaggtgtaacgccagctaaattcctgacttaaatacgttcccagcggaatgcccagcaaattggcgactgtcatcccggaaaccatccccgccacggcggcggtgacttttccgggtttgataatttttgataacacgatcgctccgacgccaaaaaatgcgccatgcggaaagccggataccagccgaccaatggcgagcatcaggtaagacgaagagagcgtgaacatggcgttgccaatgacgcacaacgccaccagaaacaacaagatatgtttgagtgagtagcggctggaaaagagtgcgatgattggcgcaccgaccaccacccccagtgcataatacgagatcatatgcccggcggcaggaatcgaaattcctacgttatgcgccagctccgtgagcacgcccataatgccaaattcggccatccccaaaccaaacgtgcccagagccaaagataaaatgacttttttcataccaccatcacaaccaccagaacggctaccaatcaccgtagccaataaagtgatagcttgcaggataacgaccagcaaggccaagagataattcgcccctctgtattcattatcctgctgaatagttatttcactgcaaacgtactttccagtttgctgtagcccaggccgttgatctttttcactttgatctgcaccggaatacgctctttcatcgcttctacgtggctaatcacaccgatggttttgccactggcgttcagggcatccagcgcatcaagggcggtatccagcgtttcgctatccagcgtgccaaaaccttcatcaaggaacagcgagtcaatacgtgttttatggctgaccagatccgaaagcgccagcgccagcgccagactaacgaggaaactttcgccgccggaaagggtacgggtatcgcgtaccgcatctgcctgccaggtatcaacaacctcgacttccagcgcctcgctggctttgcgctgtaacagatagcgcccgtgcagccgggtaagttgctgattagcgagatggactaaattatccagcgtcagcccctgggcaaacttgcggaatttatcgccctctttggaacctattagcgaattcagatatccccagtcctcaacctgctgcgtcatttgagcaatttgctgcattaaggtttgttgttgctgacggttatctgcatcctgcttcagctgctggcgaatctcgccttgactcgtggtgttttcacgcaacttttggtgagtttgcgctaactcttgctgaatctgctccaccgtcacagtgagagccaacccgtcgtcaggtcggtgttgttgatgctgtgccagcgtttctgctgtctgagtgaccagagtttgcgcctgacggcgctggttttccagattctgcttgagctgttccagctgcgttagtgtttgttcatccattagcgccgcaaggaacgcctgctgatcgtcaaagacgctggcctgtagcgcggtgtcaaactgcgcctgggctttttgcagactttgcgccgccagaacatcctgttgctgtaacgtctgctgctggctgtgtaatgcgagacattgttcatgtacctgccgccagttttccaataccacagtttcttcgcagtgcgggagttcatcactttgcggcaacgtttccagaatcggcgtcagctgctgaatacggttttgcagcgcggttaattcgttctggcgttgctgccagctctgcgcttcttgctgacgtgtcgccaaccagctctcttcttcatcttcctgtggcaatgtcagtgcataacccgtcaatgtcgttaaaagtagttgctggcgttgttcaatttgctgttgatactggataatttgctgattatgcgcggcaatctgcccttgtaattcatgccgttggctgagtaaccgcagctggcgttcgtgctcatcttgtgcatccagccacggttgaatatcgtccagtggctgcaaggtgatattgaggctggccgtgacggcttgccattgttgagtaagtgcttgctcatcttgtcggaggctttgcgcttcgttttcatcacgctgaagctgctttgttatggcgtccagttgcccacgtagcgtcgcaccttcttcaccgagctttttaacttcgttttccagcgccagtaatcgagactgattaacgccaggctccagcgcctgatacgcctcgaccgccgggtggctggtggaaccacaaagtgggcaaggctgacccgcctgtaactgtgcacgttgagcttccagcgttttgatgcgcgcttcctgctcgcaaatggttttcacatcggcaagttgctgcgtcttttctttataacgctggcgcatttcgttaagtgcggcgttacgttgcgtctgttcttgcgtgacattctggatagcgacctgtaactgcgccagacgtttttgttggggaacaatctgtccatgcagcgcgaccaggtgctgacgcagtgggcgttgctcagcatgttgcgccagggcggtagcaacttcatcggcggttaacgtcaacgtgatcgccgcaagcgcattaagtttttgctcagcatgggttaactgttgctgccattgccgcagatgctcgcgatcgctggtttgttgggagaactgcgcacgccaacccgccggttcgttgttccactgacggaagcggtcgtgttcctgtaaccaggtattcaggctttgttgctgctgctgtaattctgctgactgcttcgccgcgtggtggcgaatgctcgcgcgaagcgccattgtgctctgtaagcgagtatttacttcttcaatctgctggcgaatatgcgccagcgccgcgctgtgttctgcgatgcgttcccagtgtggacgaagatttcgtgccggttgtgccagactaagcgccgccagttgaggttgcgctttttcttcttcggctaacgcctgttgcaaggcctgctgacggcggctggcttcttgctgcaattcgtcctgacgcgttaaccagtttagcgattgttgttcttgctgctgcgcggtaattaactgtttttcttcgtcagtaagtacctgcaaactcgctgtcagcgattgcacttgttccggcgtgagcaacgtgacgccgctggcctgcgcttgcagcttctccagctctgtgcgggccgatttgtgctgctcaaaaaccatcgccgagatttgcccgtagatttcagtgccggttaactcctcgagcaattccgcgcgttctttgggtttggcattcaggaaggcagcaaattgcccctgcgaaagcagcatcgaacgggtgaagcgcccgtaatccagcccggttaacgtcgctgtcagttccagcttatctttcactttgtcggcgagaattttgccgtcggcgcagcgcgccagctctacgcgtggcacctgcaaattaccgtcgggttggttacgcgcccgattctggctccagaatgcacggtacgcttcacctttcacttcaaactccacctccgccagacattcggcggtatcgcgggtcatgagatcattttgcgattgtgaaacgttagagagacgcggagtttcgtgatacagcgccagacaaatggcgtccagcagggtggttttccccgcacctgttgggccggtaatagcaaacagcccgttgctggcgaacggctcgcgggtgaaatcaatcttccattcgccttttaatgagttcaggtttttcaggcgcaggctgagaattttcatgcttcgtgttctccggcgagggtatgcaacgtcgtggtgaaaagatgctgcagacgttgctgctgcgattcatccagttcttccagtgccagacggcgattgaacacctcttcgacgctgagttcgctgagggtttcacgctgttggctggctaacacacgctcgcgctgttcacgactccgacgtaccagcaatacttcgacaggcaatgattcggttaatgcctggattttgcgctgaatatcatgcagatactcatcagtagtgatttcgatatccagccagacaggtggctcctgcgatacatcgcgccactgttccagctgtgcggtaatcgacgccagatcgcctttcagcactgccatgggttgcgttaccggtacgttcaggttttccacgctctctaatttgccgtttgaaaatgtcaccagatggacatatttactcttaccgcattcatcaaaactcagtggaatgggggagccgcaatagcgaacatgttccatgccgccaataatctgtgcgcggtgaatatgcccgagcgcgatgtagtcggctggtggaaagttttgtgccggaaacgcgtccagcgtgccaatataaatgtcacgcacggcgtcacttttactggcccccacggtcgttaaatgtcccgtggcgatgatgggcagaggctgatcgccgcgcagtttgcaggcatcggcatagtgttgttggtaataatcggtaatcgctgccagtaaatgctgctgtttttcaataccgttaagccccgcctggctggtaataatgtcacgcggacgtaaaaacggaatggggcacagcactgcgcctggcgtcccgtcgcgacgaggcaagatttgcggcgcatgtccggcgctggcgaccacggtagtattgaggaacgccatgatatcgcgcgattcattcagcgtggcgaccgagtcatggtttcctgccagtaccaccagatgacagccagtttgctgtaaattgacaacaaaacggttgtataacgtgcgggcgtaactgggcggcgagccggtatcgaaaacatcaccggcaacaataatcgcatccacctgatgggtttgtgctgtctccagcagccagtcaagaaaagcctgatgttcagcttcgcggcttttactgtagaagttctggccgagatgccagtctgaggtgtgaaggatgcgcataacggttccctggcgaaaaagcatgggcgcgattatacccaaacagatgtgccatttgcttttttctgcgccacggaaatcaataacctgaagatatgtgcgacgagcttttcataaatctgtcataaatctgacgcataatgacgtcgcattaatgatcgcaacctatttattacaacagggcaaatcatggcgagacgtattctggtcgtagaagatgaagctccaattcgcgaaatggtctgcttcgtgctcgaacaaaatggctttcagccggtcgaagcggaagattatgacagtgctgtgaatcaactgaatgaaccctggccggatttaattctcctcgactggatgttacctggcggctccggtatccagttcatcaaacacctcaagcgcgagtcgatgacccgggatattccagtggtgatgttgaccgccagaggggaagaagaagatcgcgtgcgcggccttgaaaccggcgcggatgactatatcaccaagccgttttcgccgaaggagctggtggcgcgaatcaaagcggtaatgcgccgtatttcgccaatggcggtggaagaggtgattgagatgcagggattaagtctcgacccgacatctcaccgagtgatggcgggcgaagagccgctggagatggggccgacagaatttaaactgctgcacttttttatgacgcatcctgagcgcgtgtacagccgcgagcagctgttaaaccacgtctggggaactaacgtgtatgtggaagaccgcacggtcgatgtccacattcgtcgcctgcgtaaagcactggagcccggcgggcatgaccgcatggtgcagaccgtgcgcggtacaggatatcgtttttcaacccgcttttaacgccttgctcatcggacgcagagcagggcttatgatttcttaactggagtatcttacgtgctggaacggctgtcgtggaaaaggctggtgctggagctgctactttgctgcctcccggctttcatcctgggtgcattttttggttacctgccctggtttttgctggcatcggtaacaggactgcttatctggcatttctggaatttattgcgcctttcatggtggctgtgggtggatcgcagtatgaccccgccaccggggcgtggtagctgggaaccgctactatacggcttacaccagatgcagctgcgaaataaaaaacgccgccgtgaactgggcaatctgattaaacgctttcgtagcggcgcggagtcgctgcccgacgcggtggtgctgaccacggaagagggcggtattttctggtgtaacggtctggcgcaacaaattcttggtttgcgctggccggaagataacgggcagaacatccttaacctactgcgttacccggagtttacgcaatatctgaaaacgcgtgatttttctcgcccgctcaatctggtgctcaacaccgggcggcatctggaaattcgcgtcatgccttatacccacaaacagttgctgatggtggcgcgtgatgtcacgcaaatgcatcaactggaaggggcgcggcgtaacttttttgccaacgtgagccatgagttacgtacgccattgaccgtgttacagggttacctggagatgatgaatgagcagccgctggaaggcgcggtacgcgaaaaagcgttgcacaccatgcgcgagcagacccagcggatggaaggactggtgaagcaattgctgacgctgtcgaaaatagaagccgcaccgacgcatttgctcaatgaaaaggttgatgtgccgatgatgctgcgcgttgttgagcgcgaggctcagactctgagtcagaaaaaacagacatttacctttgagatagataacggcctcaaggtgtctggcaacgaagatcagctacgcagtgcgatttcgaacctggtctataacgccgtgaatcatacgccggaaggcacgcatatcaccgtacgctggcagcgagtgccgcacggtgccgaatttagcgttgaagataacggaccgggcattgcaccggagcatattccgcgcctgaccgagcgtttttatcgcgttgataaagcgcgttcccggcaaaccggcggtagcggattagggttagcgatcgtgaaacatgctgtgaatcatcacgaaagtcgcctgaatattgagagtacagtaggaaaaggaacacgtttcagttttgttatcccggaacgtttaattgccaaaaacagcgattaatccgcctttgtcatcttttattgccataagccagtcgatgctggcttattttctttgcagtcaaaatacgggcgttagattttacaacgattggtgattttttgttcgcatgattagccatgtctttttcacggaaatagtgttttatactggttggtgatttcttatcgctatatacctctggtttttagatccctccttgctttaaaacgttataagcgtttaaattgcgcttcaggtgctgtcatactgactgcattaacgcggtaaatcgaaaaactattcttcgccgcgcctggttgggagtatttcccgctaaaattgtttaaatataccgctgtatcatccccagggattggcacaaaaatttaacgttacaacaccacatccacaggcagtatgatttatgacccatcaattaagatcgcgcgatatcatcgctctgggctttatgacatttgcgttgttcgtcggcgcaggtaacattattttccctccaatggtcggcttacaggcaggcgaacacgtctggactgcggcattcggcttcctcattactgccgttggcctgccggtattaacggtagtggcgctggcaaaagttggcggcggtgttgacagcctcagcacgccaatcggtaaagtcgctggcgtactgctggcaacggtttgttacctggcggtggggccgcttttcgctacgccgcgtacagctaccgtttcctttgaagtggggattgcgccgctgacgggtgattccgcgctgccgctgtttatctacagcctggtctatttcgctatcgttattctggtttcgctctatccgggcaagctgctggataccgtgggcaacttccttgcgccgctgaaaattatcgcgctggtcatcctgtctgttgccgctattgtctggccggcgggttctatcagcacggcgactgaggcttatcaaaacgctgcgttttctaacggcttcgttaacggctatctgaccatggatacgctgggcgcaatggtgtttggtatcgttattgttaacgcggcgcgttctcgtggcgttaccgaagcgcgtctgctgacccgttataccgtctgggctggcctgatggcgggtgttggtctgactctgctgtacctggcgctgttccgtctggggtcagacagcgcgtcgctggtcgatcagtctgcaaacggcgctgctattctgcatgcttacgttcagcacacctttggcggcggcggtagcttcctgctggcggcgttaatcttcatcgcctgcctggtaacggcagttggcctgacctgtgcttgtgcagaattctttgcccagtacgtaccgctctcttatcgtacgctggtgtttatcctcggcggcttctcgatggtggtttctaacctcggcttaagccagctgatccagatctccgtaccggtgctgaccgctatttatccgccgtgtatcgcactggttgtattaagttttacacgctcatggtggcataattcgtcccgcgtgattgctccgccgatgtttatcagcctgctttttggtattctcgacgggatcaaagcatctgcattcagcgatatcttaccgtcctgggcgcagcgtttaccgctggccgaacaaggtctggcgtggttaatgccaacagtggtgatggtggttctggccattatctgggatcgcgcggcaggtcgtcaggtgacctccagcgctcactaaatcactgaacatttgttttaaccacggggctgcgatgccccgtggttttttattgtgttgatgggttaggaattgatggaaagtaagaacaagctaaagcgtgggctaagtacccgccacatacgctttatggcactgggttcagcaattggcaccgggctgttttacggttcggcagacgccatcaaaatggccggtccgagcgtgttgttggcctatattatcggtggtatcgcggcgtatatcattatgcgtgcgctgggggaaatgtcggtacataacccggccgccagctctttctcgcgttatgcgcaggaaaacctcggcccgctggcaggttacattaccggctggacctactgctttgaaatccttattgtcgccatcgccgatgtgaccgcttttggtatctatatgggtgtctggttcccgacggtgccgcactggatttgggtactgagcgtggtgctgatcatttgcgccgtaaacctgatgagcgtgaaggtattcggtgagctggaattctggttctcgttctttaaagtcgccaccatcatcatcatgattgtcgccggtttcggcatcatcatctgggggattggcaacggcgggcaaccgaccggtattcataacctgtggagcaacggcggcttcttcagtaacggctggcttggcatggtaatgtcgttgcaaatggtgatgtttgcttacggtgggatcgaaattatcgggattaccgccggtgaagcgaaagatcctgagaaatcgataccgcgtgcgattaactccgtgccgatgcgtattctggtgttctacgtcggtacgctgttcgtcattatgtctatctacccgtggaatcaggttggcactgccggtagcccgttcgtgctgacgttccagcatatgggcattacctttgccgccagcattcttaactttgttgtgctgactgcttcgctgtcggcaattaacagtgatgtatttggcgtaggccgtatgctccacggtatggcagagcagggcagcgcgccgaaaattttcagcaaaacgtcgcgtcgcggtattccgtgggttacggtgctggtgatgactaccgcgctgctgtttgcggtgtatctgaactacatcatgccggaaaacgtcttcctggtgatcgcttcgctggcaaccttcgccacggtgtgggtgtggattatgatcctgctgtcgcaaattgccttccgtcgccgtttgccgccagaagaagttaaggcgctgaaatttaaagtgccgggtggggtagcaacgaccatcggcgggctgattttcctgctctttattatcgggttgattggttatcacccggatacgcgtatctcgctgtatgtcggtttcgcgtggattgttgtgctgttgattggctggatgtttaaacgccgccacgatcgtcagctggctgaaaaccagtaatccttgcgttctgtaagccggttcaggaggaaatcctgatccggctattccgaaagttatccgcccccgtcctcctcccccaaatatccttcagatgatgagtgatcctgcattaggctatggcaaggtgatcagattttcatcacaggggaattatgatgttaaatgcatggcacctgccggtgcccccatttgttaaacaaagcaaagatcaactgctcattacactgtggctgacgggcgaagacccaccgcagcgcattatgctgcgtacagaacacgataacgaagaaatgtcagtaccgatgcataagcagcgcagtcagccgcagcctggcgtcaccgcatggcgtgcggcgattgatctctccagcggacaaccccggcggcgttacagtttcaaactgctgtggcacgatcgccagcgttggtttacaccgcagggcttcagccgaatgccgccggcacgactggagcagtttgccgtcgatgtaccggatatcggcccacaatgggctgcggatcagattttttatcagatcttccctgatcgttttgcgcgtagtcttcctcgtgaagctgaacaggatcatgtctattaccatcatgcagccggacaagagatcatcttgcgtgactgggatgaaccggtcacggcgcaggcgggcggatcaacgttctatggcggcgatctggacgggataagcgaaaaactgccgtatctgaaaaagcttggcgtgacagcgctgtatctcaatccggtgtttaaagctcccagcgtacataaatacgataccgaggattatcgccatgtcgatccgcagtttggcggtgatggggcgttgctgcgtttgcgacacaatacgcagcagctgggaatgcggctggtgctggacggcgtgtttaaccacagtggcgattcccatgcctggtttgacaggcataatcgtggcacgggtggtgcttgtcacaaccccgaatcgccctggcgcgactggtactcgtttagtgatgatggcacggcgctcgactggcttggctatgccagcttgccgaagctggattatcagtcggaaagtctggtgaatgaaatttatcgcggggaagacagtattgtccgccactggctgaaagcgccgtggaatatggacggctggcggctggatgtggtgcatatgctgggggaggcgggtggggcgcgcaataatatgcagcacgttgccgggatcaccgaagcggcgaaagaaacccagccggaagcgtatattgtcggcgaacattttggcgatgcacggcaatggttacaggccgatgtggaagatgccgccatgaactatcgtggcttcacattcccgttgtggggatttcttgccaataccgatatctcttacgatccgcagcaaattgatgcccaaacctgtatggcctggatggataattaccgcgcagggctttctcatcaacaacaattacgtatgtttaatcagctcgacagccacgatactgcgcgatttaaaacgctgctcggtcgggatattgcgcgcctgccgctggcggtggtctggctgttcacctggcctggtgtaccgtgcatttattacggtgatgaagtaggactggatggcaaaaacgatccgttttgccgtaaaccgttcccctggcaggtggaaaagcaggatacggcgttattcgcgctgtaccagcgaatgattgcgctgcgtaagaaaagtcaggcgctacgtcatggcggctgtcaggtgctgtatgcggaagataacgtggtggtatttgtccgcgtgctgaatcagcaacgtgtactggtggcaatcaaccgtggcgaggcctgtgaagtggtgctacccgcgtcaccgtttctcaatgccgtgcaatggcaatgcaaagaagggcatgggcaactgactgacgggattctggctttgcctgccatttcggctacggtatggatgaactaacgttttataacgccttgcgtgacgcctgcgccatcatccgcggataaaactgccagaagcgggtttcgagggcgtcataatgagcgtctaaatcgtaccaggagtcacgcagggcatccagacgtgggcggcggcttgccatgccgtttaacacgttctggatgaaatccatatcgcgatagcgcaccagccactgctctgaccacaagtaattgttcagattgataaaacgtggcggtgagtccggcaaaatcgtcatcacttgctcgcgggcataacagacaaattcctgtagcggaaagtccggcgacagctgcgaccagtggcgggaaagaaagtgatcccacatgacatccagcgtaataggcgcaacgcggcgcgtttcactacgaaaccactcccgtgcttcgcggacttccggcagattgtcagtcaatacgtcgatacgtcgatgcatatgaatgccagccacgacgtcgggcggaaaactttcttcaggatttccgcgtacgaaatcagccagtaaattgccggaaagcgagctttccgcgagatgggctaaatgcaggtgagctaaaaaattcatcgattatattctatccaaaagggggtaaaggttgcagggagagcgccccggcactagactacccgcctcttattttagtctgagtcagtgtcatgcgcgttaccgatttctcctttgaattgcccgaatccctgattgcccactatcccatgcctgaacgcagtagctgtcgtttactgtcgctggacgggccgacgggcgcgctgacgcacggtactttcaccgatttacttgataagctcaaccccggcgatcttctggtttttaataatacccgcgtgatcccggcgcgcctgtttgggcgtaaagccagcggcggcaagattgaagtgctggttgaacggatgctcgacgacaaacgcattcttgcgcatattcgcgcctcgaaagcgccaaaacctggcgcagaactgctgctgggcgatgacgaaagtattaacgcaacaatgaccgcgcgccacggcgcactgtttgaagtcgaatttaatgatgaacgctcggtgctggatattctcaacagcatcggccatatgccgctgccgccgtatatcgaccgtccggacgaagacgctgaccgcgaactttatcaaaccgtttatagcgaaaaaccgggcgcggttgcagccccgaccgcaggtctgcattttgacgagcctttgctggaaaaattgcgcgccaaaggcgtggagatggcgtttgtgacgttgcacgttggtgcgggcaccttccagccggtgcgcgtcgacaccattgaagatcacatcatgcactcggaatacgctgaagtaccgcaggatgtggtagacgcggtactggcggcgaaagcgcgcggtaaccgggtgattgcggttggcaccacttcagtacgttcgctggaaagcgcggctcaggcagcgaaaaacgatctcattgaaccgttcttcgacgatacccaaatctttatctatccgggcttccagtacaaagtggtcgatgcgctggtgacgaacttccacttgccagagtcgacgctgattatgctggtttcggcctttgccggttatcaacacaccatgaacgcctataaagcagcggtagaagagaaatatcgcttttttagttacggtgatgcgatgtttatcacgtacaatccgcaggcaattaatgagcgcgtcggggagtaattccgcggcgctggtttaaaacgttggactgtttttctgacgtagtggagaaaaaatgaaatttgaactggacaccaccgacggtcgcgcacgccgtggccgcctggtctttgatcgtggcgtagtggaaacgccttgttttatgcctgttggcacctacggcaccgtaaaagggatgacgccggaagaagttgaagccactggcgcgcaaattatcctcggcaacaccttccacctgtggctgcgcccgggccaggaaatcatgaaactgcacggcgatctgcacgattttatgcagtggaaggggccgatcctcaccgactccggcggcttccaggtcttcagccttggcgatattcgtaaaatcaccgaacagggcgtgcacttccgtaacccgatcaacggcgatccgattttcctcgatcctgaaaaatcaatggagattcagtacgatcttggttcggatatcgtcatgatctttgatgagtgtacgccgtatcctgctgactgggattacgcaaaacgctccatggagatgtctctgcgttgggcgaagcgtagccgtgagcgttttgacagtctcggaaacaaaaatgcgctgtttggtatcatccagggcagcgtttacgaagatttacgtgatatttctgttaaaggtctggtagatatcggttttgatggctacgctgtcggcggtctggctgtgggtgagccgaaagcagatatgcaccgcattctggagcatgtatgcccgcaaattccggcagacaaaccgcgttacctgatgggcgttggtaaaccagaagacctggttgaaggcgtacgtcgtggtatcgatatgtttgactgcgtaatgccaacccgcaacgcccgaaatggtcatttgttcgtgaccgatggcgtggtgaaaatccgcaatgcgaagtataagagcgatactggcccactcgatcctgagtgtgattgctacacctgtcgcaattattcacgcgcttacttgcatcatcttgaccgttgcaacgaaatattaggcgcgcgactcaacaccattcataaccttcgttactaccagcgtttgatggcgggtttacgcaaggctattgaagagggtaaattagagagcttcgtaactgatttttaccagcgtcaggggcgagaagtaccacctttgaacgttgattaatattaataatgagggaaatttaatgagcttttttatttctgatgcggtagcggcaacgggtgcaccggcgcaaggtagcccgatgtctttgattttgatgctggtggtattcggtctgattttctatttcatgatcctgcgtccacagcagaagcgcaccaaagaacacaaaaagctgatggactccattgccaaaggtgatgaagttctgacgaacggtggcctggttggtcgcgtaaccaaagtagcggaaaacggctacattgctatcgcgctgaatgacaccactgaagtagttattaaacgtgacttcgtagctgccgtcctgccgaaaggcaccatgaaggcgctgtaattaaaatttttccctaagggaattgccgtgttaaaccgttatcctttgtggaagtacgtcatgctgatcgtggtgattgtcatcggtctgctgtatgcgcttcccaacctgtttggtgaggatccggctgttcagatcactggtgcgcgcggagtcgccgccagtgagcaaacgctgatccaggtccagaaaacgttacaagaagaaaaaataactgctaagtctgtggcactggaagagggcgctattcttgcgcgcttcgactccactgacacccagttgcgcgctcgtgaagcattaatgggcgttatgggtgacaaatacgtcgtggcgcttaaccttgccccggcaacgccgcgctggctggcagctattcacgctgagccgatgaagctcggccttgacctgcgtggcggcgttcacttcctgatggaagtggatatggacaccgcgcttggcaaactccaggaacaaaatatcgatagcctacgcagtgacctgcgcgaaaagggcatcccgtataccactgttcgtaaagaaaacaactacggcctgagcatcactttccgcgatgctaaagctcgtgatgaagccattgcgtatctgagcaagcgccatccggacctggtgattagcagccagggcagcaaccagctgcgtgcggtaatgagcgatgctcgtctgagtgaagcgcgtgaatatgcggtgcagcagaacattaatatcctgcgtaaccgtgtaaaccaacttggcgtggcggagccggtggttcagcgtcagggtgctgaccgtatcgttgttgaactgccaggtattcaggacactgcgcgtgcgaaagagattctgggtgcgacggcaacgctggaattccgtctggtaaacaccaacgttgaccaggccgctgcggcatccggtcgcgtaccgggcgactctgaagtgaaacagacccgcgaaggtcagccagttgtgctgtacaaacgcgtaattctgaccggtgaccatatcaccgactccacttccagccaggacgaatacaaccaaccgcaggttaacatctcgctcgatagcgctggtggtaacatcatgtctaacttcactaaggacaacatcggcaaaccgatggcaaccctgtttgtggagtacaaagacagcggtaagaaagatgcaaatggtcgtgcggttctggtgaaacaggaagaggtgattaacatcgccaacatccagtctcgtctgggtaacagcttccgtatcaccggcatcaacaacccgaacgaagcccgtcagctgtcactgctgctgcgtgccggtgcgttgatcgcgccgattcagattgttgaagaacgtaccattggcccaaccctgggtatgcagaacattgaacaggggctggaggcttgccttgccggtctgctggtttctattctgttcatgatcatcttctataagaagtttggtctgattgcgaccagtgctctgattgccaacttgatcttaatcgtcggcattatgtcgctgttgccaggcgcaacgctgagtatgccaggtatcgcgggtatcgtcttaacccttgcggtggcggtcgatgcgaacgtactgatcaacgaacgtattaaagaagagttgagcaacggacgtactgttcaacaggcaattgatgaaggttatcgtggcgcattcagttctatcttcgatgcgaacatcaccacgctgattaaagtcatcatcctgtacgcagtgggtaccggggcaattaaagggttcgcgattactaccggtatcggtgtggcgacgtcgatgtttaccgcgattgtcggtacgcgtgccatcgtaaacctgctatatggcggcaagcgcgtcaagaagctgtcaatctgaggagtgcgatgtggcacaggaatatactgttgaacaactaaaccacggccgtaaagtctatgactttatgcgctgggactactgggctttcggcatctctggtctgctgttaatcgctgctatcgttattatgggcgtgcgcggctttaactgggggctggatttcaccggtggtacggttattgaaattacgctcgaaaaaccggctgaaattgacgtaatgcgtgatgcattgcaaaaagccggttttgaagagccgatgctgcaaaactttggtagcagccatgacatcatggtccgtatgccgcctgctgaaggcgaaaccggcggtcaggtgttgggcagccaggttctgaaggtgattaacgaatccaccaatcagaatgcagcagtgaagcgtattgagttcgtcggtccgagcgtgggggcagaccttgcgcaaaccggtgcgatggcgttgatggcagcgctgctgtctatcctcgtgtacgtaggtttccgctttgagtggcgactggcggcaggggtggttattgcgctggcgcacgacgttatcattacgctgggtattttgtcgttattccatatcgagattgacctgaccattgtggcatcgttgatgtcggttatcggttactcgcttaacgacagtatcgtggtatcggaccgtattcgtgaaaacttccgcaagatccgtcgcggtacgccttacgaaatctttaacgtgtccttgacccagacgctgcaccgtaccttgatcacatccggtactaccttgatggttatcctgatgctgtacctcttcggtggtccggtactggaaggcttctcgctgaccatgcttatcggtgtttccatcggtactgcatcttccatctatgtggcatctgcgttggctctgaaactgggtatgaagcgcgaacacatgttgcagcagaaagtggaaaaagaaggggcggatcagccgtcaattctgccgtaatcaagttcccgttgatgttgaaaatcccggtcagaagatcgggattttttttgatgtatggagattgcgaaaatccccgcatcttgggaaactgcgcgtaaccctacatttcatccaggtaacttttcatggctatcatcccaaaaaactatgcgcggttagaaagcggctatcgcgaaaaagcattaaaaatctatccgtgggtctgcggtcgctgttcccgcgagtttgtttattccaacctgcgtgaacttaccgttcaccacattgatcacgaccataccaataacccggaagatggcagtaactgggaattgttgtgtctctattgccacgatcatgagcattcgaaatataccgaagcggatcagtatggtacgaccgttatcgcaggggaagatgcgcagaaagatgtcggtgaagcgaagtacaacccattcgctgacctgaaagcgatgatgaacaagaagaagtgattaaaacgtaaaattgcctgatgcgctacgcttatcaggcctacgttatttcagcaatatattgaatttacgtgcttttgttggccggacaaagcgtttacgccgcatccggcatgaacaaagcacacgttgttaacaatcagaaatgccgggaataaatcccggcattttcataatcagaagttgtaacctactaccaggtaaccaccccagccggtagagcgaacgttgaagttgccgttgccgaagttcagttctgcatcgtcgttccactgaccaccgtcgtgccagtaacgagctacgacagagtagtgccagtgatcgtagttcagagccagaatatggctggaagcgatagagttattagtacgggtcttaataccgttgattgcgttaccgctgtcatcccctaaatcggaaccccagtcgaagttggtgaagccgatgtagctcagctgaccgccccacagatcggtaatcggcacaaagtatttaattttgaaacggtaaccgtcccactcgttttcgttcgctgcgccatagttctgccactggtatttcgcatagacgttcatggacaggctcatcggcaggccagtgtcgatatcggtacccagacccatgtaccaggtgctctggcgaccatctttattacgacccatgtcgtaaatgtagttgttcgcgaagtaccactctttgaacggaccgaagctaaggtcagtattggtcagcttgtcgatggagaaacgtggttcgatttccataaacagcggagaaccgtggttccagatacctttagcatcggagttaccgccgaagaataccggcgcatccgcataaccatagaagtcgaaccagtcttttttagcgaatgcttcgtactcaaggtaggtatcgttgcggatctgcggtccgaaacgggtgtgatagcttccgacaacgttaacgctctggtgccaccagtcggaaagatactgcggtttgtcgttttcagctgcgttgacagtaaaagacgaagagagcgccagtaccgcaccggctgccagtaatgtttttttcatatgtatgccactgtttgaaaatcccttgcgggagtgaaaaaggcgcaaattgcgtttctaaatatttcgtatacagaggagcctattataaaaatcattgctcacaaaaatatgtttcgtttcacagttctatcatttacgtaatcgattgcgttcacgtttacacacattcgggcggggattgtactgactttcgcccttgttgcaaacttttactatcaatccaggtgatgtaagcagagtaacaaaatgacggggaaagatgttgcgggacgcacaaaatcgtcccgaaatacgtttactgcataacaggttgaatgtcgtggatacgtacaaagcctaactgatccacagaaatcccctttaactgtaacggaatatcaacatcgctgggggcgaggacgctggcaggggcattaatcaattgattctgcacattgatttcctgaaagttgtctattgttccctgaatttgcccatattcaacagttccgctgaatgcgggcaagggatcattcgactcaccctgaatacgtagtgtaagggtggtgccatctgcatcaggcgtaatattcaccagcgacatacgtaaagtaccgatctggctttccagtcttgccggtgttttcgctccaggcagaaggtaaaccccactgctggattttgcattcagcctgttttgctgagtgattttgactgtttcttgattgagttgcgtcatctcctggttcagcgtgctgacgctgtgtttcatctgtcgcacttcactttgctgcacacaggcgctaaggctgaacaggcttcccagcaggagcagtcgaaaaacgttagtattcataggtcgtccctttctcgtcgcaattagcctaatggtagagggtaaaagcagcgaaagcatcgatcctttatctcaaaagcgttgcgcctttgttgtatcgtcagttcagggtaaaatagatttccgttaaccacctggtcaggacgccgtatgcattgcccattctgtttcgccgtggacactaaggtaattgactctcgtctcgtgggcgagggttcatccgtacgccgccgtcggcagtgtctggtgtgtaatgaacgtttcaccacctttgaagtggcggagctggttatgccgcgtgttgtaaaaagcaacgacgtgcgtgaaccgtttaatgaagagaaattgcgtagcggaatgctgcgggcgctggaaaaacgtccggtgagttccgatgacgtcgaaatggcaatcaatcatattaaatcgcagctgcgcgccaccggtgagcgcgaagtgccgagcaagatgattggcaatctggtgatggagcaattgaaaaagctcgataaagtcgcctatatccgttttgcctctgtctaccgcagtttcgaagatatcaaagaatttggcgaagagatcgcgcgcctggaggactaagccgtgcaggacgagtattacatggcgcgggcgctaaagctggcgcaacgaggacgttttaccacgcatcccaacccgaatgtcgggtgcgtcattgtcaaagatggcgaaattgtcggtgaaggttaccaccaacgtgcgggtgaaccacatgccgaagtacacgcgttgcgtatggcgggtgaaaaagccaaaggtgcgaccgcctatgtcacactcgaaccctgtagccatcatggtcgtacgccaccgtgctgtgacgcactcatcgccgctggcgtagcgcgcgtggttgcctcgatgcaagatcctaacccgcaggtcgctgggcgtggactttaccgtctgcaacaggctggcattgacgtcagccacggcctgatgatgagtgaagccgagcaattgaataaaggctttctcaagcggatgcgcaccggctttccttatattcagttaaaacttggcgcatcgcttgatggtcgcacggcgatggcgagcggcgaaagccagtggatcacttcgccccaggcgcggcgtgatgtacaactactgcgcgcgcaaagtcatgccattttaaccagcagcgccacggtgctggcggatgatcctgccttaacggtgcgttggtctgaactggatgaacaaactcaggcgctctatccgcaacaaaatctccgtcagccgatacgtattgtgattgatagccaaaatcgcgtgacgccggtacatcgcattgtgcagcagcccggcgaaacctggttcgcgcgtacgcaggaagattctcgtgagtggccggaaacggtgcgtaccttgctgattccagagcataaaggtcatctggatctggttgtactgatgatgcaactgggtaaacagcaaattaacagcatctgggtggaagcggggccaacgctcgctggcgcattgctgcaggcgggtttagtcgatgagctgattgtctatatcgcacctaaactattaggcagcgacgcccgcggattatgcacgctgccagggcttgagaaattagccgacgccccccaatttaaattcaaagagatacgtcatgtaggcccggatgtttgcctgcatttagtgggtgcatgatctcccggctcgaaagggaagcagcgcacgaaatattatgctaaaatccgcccccctgcggggccatactcgaacccgaaggaagaaaatgaacattattgaagctaacgttgctaccccggacgctcgcgtcgccatcaccatcgcgcgtttcaacaactttatcaatgacagcctgctggaaggtgcaattgacgcactgaaacgtatcggtcaggtaaaagatgaaaacattaccgttgtttgggtgcctggtgcctatgagctgccgctggcggcgggtgcactggctaaaaccggtaaatacgacgcggtgattgcgctgggtacggttattcgtggtggcactgcccactttgaatatgtcgctggtggtgcaagcaacggcctggcgcatgttgcccaggacagcgaaattccggttgcttttggggttctgaccactgaaagcattgaacaagcgatcgaacgtgctggcaccaaagctggcaacaaaggtgcagaagctgcactgaccgcgcttgaaatgattaatgtattgaaagccatcaaggcctgaaattagtaaggggaaatccgtgaaacctgctgctcgtcgccgcgctcgtgagtgtgccgtccaggcgctctactcctggcagttgtcccagaacgacatcgctgatgttgaataccagttcctggctgaacaggatgtaaaagacgttgacgtcctgtacttccgtgagctgctggccggggtggcgactaataccgcatacctcgacggactgatgaagccatacctgtcccgcctgctggaagaactgggacaggtagaaaaagcagtactgcgcattgcgctgtacgaactgtctaaacgtagcgatgtgccatacaaagtggccattaacgaagcgatcgaactggcgaaatcgttcggcgcagaagacagccataagttcgtcaacggcgtactcgataaagcagcacctgtgattcgccctaacaaaaagtgatatccaggccggtagattcacggaagaccgttccatgatcgccggccttttcttttttacctgctgaggcataacgtatggcatgtggcgagttctccctgattgcccgttattttgaccgtgtaagaagttctcgtcttgatgtcgaactgggcatcggcgacgattgcgcacttctcaatatccccgagaaacagaccctggcgatcagcactgatacgctggtggcgggtaaccatttcctccctgatatcgatcctgctgatctggcttataaagcactggcggtgaacctaagcgatctggcagcgatgggggccgatccggcctggctgacgctggcattaaccttaccggacgtagacgaagcgtggcttgagtccttcagcgacagtttgtttgatcttctcaattattacgatatgcaactcattggcggcgataccacgcgtgggccattatcaatgacgttgggtatccacggctttgttccgatgggacgagccttaacgcgctctggggcgaaaccgggtgactggatctatgtgaccggtacaccgggcgatagcgccgccgggctggcgattttgcaaaaccgtttgcaggttgccgatgctaaagatgcggactacttgatcaaacgtcatctccgtccatcgccgcgtattttacaggggcaggcactgcgcgatctggcaaattcagccatcgatctctctgacggtttgatttccgatctcgggcatatcgtgaaagccagcgactgcggcgcacgtattgacctggcattgctgccgttttctgatgcgctttctcgccatgttgaaccggaacaggcgctgcgctgggcgctctctggcggtgaagattacgagttgtgtttcactgtgccggaactgaaccgtggcgcgctggatgtggctctcggacacctgggcgtaccgtttacctgtatcgggcaaatgaccgccgatatcgaagggctttgttttattcgtgacggcgaacctgttacattagactggaaaggatatgaccattttgccacgccataaagatgtcgcgaaaagtcgcctgaagatgagtaatccgtggcatctacttgctgtcggattcggaagtggattaagcccgatcgttcctgggacgatgggctcgctggcagcgattccgttctggtatctgatgacctttttgccctggcagctctactcgctggtggtgatgctggggatctgtatcggcgtctatctttgtcatcaaacggcgaaagacatgggtgtgcacgatcatggcagcattgtctgggacgaatttattggtatgtggatcacgctcatggcgctgccgaccaatgactggcagtgggttgccgccgggtttgtgattttccgtattctggatatgtggaagccgtggccgatccgctggtttgatcgcaatgtgcatggcggcatggggatcatgatcgacgatattgtcgccggggtgatttccgcaggcatcctgtattttatcggtcatcactggccgctgggtattctgtcgtagttgtgcaccgatgcctgatgtgacgcttgtcacgtctcatcaggcctggactcttatttaaatcctacgacaggatgcggtttatacggcgtttccagttcggcaatctgttccggcttcaaagtgatatccaccgcgttcaatagctcatcaagctgttcttcgcgcgaagttccgataatcggtgcggcaatgcccggtttactcaacaaccaggccagcgcaacttgtgctcgtgtcgcccccagttcttcactgacgcctgttaaccgctctgcgatctgcgcgtcattttcatcgctttctttatagagatttttccccacctcatcagacaccagtcgtgcggtagtttctccccacggacgcgtcagacggccccttgccagcgggctccatggaattaccgccacgccctcctgataacacagtggtagcatctcgcgctcttcttcacgataaatcagattgtagtgatcctgcatactgacaaactgcgcccagccgtgctgtttttggagttccagtgcctgagcaaactgcgaagcgtgcattgatgacgcgccgatataacgcgctttcccggcttttaccacgtcgttgagggcttccagcgtctcttcgatcggcgtgttgtaatcccagcgatgaatttgcaggatatcgacataatccatgccgagacgtcgcaggctgtcgtcgatagagcgcaaaatttgcgcacgggataatccttccggtaaatcaccaacgcgatggaacactttggtcgcaacgaccacgtcttcacgacgggcgaaatcccgcagtgcgcgaccgacgatctcttcgctgctgccgtcagaataactgttggcggtatcaaagaaatttatgccgccttccagtgcacgtttaattatgggacggctgctttcttccggcagtgtccatgcgtgattaccgcgatctggctcgccaaaggtcatacagccgaggcaaagtcgggaaacgcgaaggtcggtttttcctaaggggttgtattgcatgctgccactcctgctatactcgtcatacttcaagttgcatgtgctgcggctgcattcgttcaccccagtcacttacttatgtaagctcctggggcttcactcgtttgccgccttcctgcaactcgaattatttagagtctatgaataatttcttaagcatagcaggagtggagtagggattatgccagccaggccttgattttggcttccataccagcggcatcgaggccgagttcggcgcgcatttcttcctgagttccttgcggaataaagaagtccggcaggccaatgttcagcacgggtactggtttacgatgggccatcagcacttcgttcacgccgctgcctgcgccgcccataatggcgttttcttctacggtgaccagcgcttcatggctggcggccatttccagaattaacgcttcatcaagcggtttcacaaaacgcatatcgaccagcgtggcgttcagcgattcggcgactttcgccgcttctggcatcagcgtaccaaagttaaggatcgccagtttctcgccacgacgcttcacaatgcctttgccaattggtagtttttccagcggcgtcagttccacgccgaccgcgttgccacgcgggtagcgcaccgctgacgggccatcgttatagtgatagccggtatagagcatctggcgacattcgttttcatcgctcggggtcataatgaccatttccggtatgcagcgcaggtaagagagatcaaaagcaccctgatgggtttgaccgtcagcaccaacaatgcccgcgcggtcgatggcgaacaggaccggaagcttttgaatcgccacgtcatgcagcacctgatcataggcgcgttgcaggaaagtggagtaaatcgcgacaatgggtttgtacccaccaatcgccagacccgcagcaaaggtcaccgcgtgttgctcggcaattgccacgtcgaagtagcgatccgggaatttacgtgaaaactcgaccatgccggaaccttcacgcatcgccggagtaatcgccatcagcttgttgtctttcgctgccgtttcgcacaaccagtcgccaaagatttttgaatagctcggcaaaccgccgctacttttcggcaaacaaccgctggagggatcaaatttaggcacggcgtggaaagtgatcgggtctttttctgccggttcataaccacgaccttttttggtcatgatatgcaggaactgcgggcctttcaggtcgcgcatgttctttagcgtggtgataagccccagcacatcgtgaccgtccaccgggccgatgtagttaaagcccagctcttcaaacaacgtgccaggcactaccatgcctttaatatgttcttcggtgcgtttgagcagctctttaattggcggcacgccagagaaaacttttttcccgccttcgcgcagtgaagagtaaagcttaccggaaagcagctgtgccagatggttgttgagcgcgccgacattttcggaaatcgacatttcattgtcgttgagaatcaccagcatatcaggacggatatcgcccgcgtgattcatcgcttcaaacgccatgcctgcggtaatcgcgccatcgccaatgacacagacggtgcggcgatttttgccttctttttcggcagcaaccgcaataccaattccggcactgatggaggttgatgaatgcccgacgcttaatacgtcatattcgctttcgccgcgccacgggaacgggtgcagaccgcctttctgacggatggtgccgattttgtcgcggcgtccggtcaaaattttatgcggataagcctgatgccccacatcccaaatcaattggtcaaacggggtgttgtagacatagtgcagcgccacggtcagttcgaccgtgcccagcccggaggcgaagtgcccgctggaacggctcacgctgtcgagtaaatagcggcgcagttcgtcgcagagtttcggtaaactctctttcggcaacagtcgtaactcctgggtggagtcgaccagtgccagggtcgggtatttggcaatatcaaaactcatcaggggcctattaatacttattgtttatttattacgctggatgatgtagtccgctagcgcttccagtgccgaggtatcgagtgactgttcagccagttgtttcagcgactgacgggcatcgtcgatcagatcccgggctttcttccgggcttgctcaagacccagaagtgcagggtaggtacttttaccaagttgctggtcggcaccctggcgttttcccaacgttgcagtatctcccaccacatccaggatgtcatcctgaacctggaaggcaaggccgatgctctctgcatacttgtcgagtaccggcagagcacgacgtcctttatctccggcgcttaatgcaccaaggcgaacggcggcgcgaatcaatgcgccggttttatgacgatgaatacgctcaagcgcgtccagaggtacgtgtttgccttccgcgtctaaatctaatgcctgaccaccgcacattccggcaataccactggcgctcgccagttcagaaatcatcgaaattctgtcgcggtccgacacttccggcatatcggcatcgcttaaaatcgagaacgccagcgtttgtaaagcgtcgccagcgagaatcgcgtttgcttcgccaaacttcacatggcaggttggcaaaccgcgacgcagatcgtcatcatccattgccggtaaatcatcatgaattaatgagtaagcgtggatacactcaacggcggcagcgggtgcgtccagcgtgtttgtgctaacgccgaacatatgaccggtggcataaaccaggaaaggtcgcaggcgcttaccacctaataatgcgccatactgcatggtttcgaccacgggagtgttctgaaagggcagtggggcgataaaacggctcagcgcctggttggcctgcttaacgcaggcttcgagttgctgcggaaagtccattactcattgtccggtgtaaaaggggttagagaggcgtcttcattgtcagacagcagaatttgtacgcgctgttcggcttgttgtaatttggcctgcccctgacgtgccagctgcacgccgcgttcgaactcgttcagcgcctcttccagcggcaggtcgccactttccagacgggttacaatctgttccagctcgctcagcgccttttcaaagctggcgggcgcctcatttttcttcggcataatgaatgtctgactctcaatatttttcgccccgtcatggtaacggactcagggcaaatagcaaataacgcgcaatggtaaggtgatgtgcacagcaaagcgatgttagtggtatacttccgcgcctggatgcagccgcaggtgtgggctgctgtatttttccctatacaagtcgcttaaggcttgccaacgaaccattgccgccatgaagtttatcattaaattgttcccggaaatcaccatcaaaagccaatctgtgcgcttgcgctttataaaaatccttaccgggaacattcgtaacgttttaaagcactatgatgagacgctcgctgtcgtccgccactgggataacatcgaagttcgcgcaaaagatgaaaaccagcgtctggctattcgcgacgctctgacccgtattccgggtatccaccatattctcgaagtcgaagacgtgccgtttaccgacatgcacgatattttcgagaaagcgttggttcagtatcgcgatcagctggaaggcaaaaccttctgcgtacgcgtgaagcgccgtggcaaacatgattttagctcgattgatgtggaacgttacgtcggcggcggtttaaatcagcatattgaatccgcgcgcgtgaagctgaccaatccggatgtgactgtccatctggaagtggaagacgatcgtctcctgctgattaaaggccgctacgaaggtattggcggtttcccgatcggcacccaggaagatgtgctgtcgctcatttccggtggtttcgactccggtgtttccagttatatgttgatgcgtcgcggctgccgcgtgcattactgcttctttaacctcggcggcgcggcgcatgaaattggcgtgcgtcaggtggcgcattatctgtggaaccgctttggcagctcccaccgcgtgcgttttgtcgctattaatttcgaaccggtcgtcggggaaattctcgagaaaatcgacgacggtcagatgggcgttatcctcaaacgtatgatggtgcgtgccgcatctaaagtggctgaacgttacggcgtacaggcgctggtcaccggcgaagcgctcggccaggtgtccagccagacgctgaccaacctgcgcctgattgataacgtctccgacacgctgatcctgcgtccgctgatctcttacgacaaagagcacatcatcaacctggcccgccagattggcaccgaagactttgctcgcacgatgccggaatattgtggtgtgatctccaaaagcccgacggtgaaagcagttaaatcgaagattgaagcggaagaagagaagttcgacttcagcattctcgataaagtggttgaggaagcgaataacgttgatatccgcgaaatcgcccagcagaccgagcaggaagtggtggaagtggaaaccgtcaatggcttcggcccgaacgacgtgatcctcgatatccgttctatcgatgaacaggaagataagccactgaaagtcgaagggattgatgtggtttctctgccgttctataaactgagcaccaaatttggcgatctcgaccagaacaaaacctggctgctgtggtgtgagcgcggggtgatgagccgtctgcaggcgctctatctgcgcgagcagggctttaacaatgtgaaggtatatcgcccgtaatttgtggtttttacgtcgcatctggtcagatgcgacgtttgccgcatccgacactactcgtaataattataaatccctgccgccatcaccagttgtgatgccacttcatgggctttttcacgcccaaccaacaggtcgataattttcagaccaaagtcgatagctgtacccggcccctggctggtcagcaattttacccgtgcatcccagacgacgcgcttgtccagccattgttcggcgggaattttgtctttcagcgtcgggaagccggtcatattaccaatcgggaagatatcgtgcggcaccagcacggtggctggcgcggcgcaaatagccgcgacgatacgcccggaacggtggaactgtttaacggtttcaaccagcagagtgctatcgcgaaaacactccgcgcctttaatgccaccaggcagcacgatcacgtcatattcgccatcagccacttcgaccagcggcgcatccgccagcagcttcacgccgcgcgagcaggtaatcgccaggttaccatcgctggcgacgctggcagtggtgactttgataccgccgcgaaccagcagatcgatagtggtgacggcttcagtctcttcactaccaggggcgaggcaaaccagtgccgatgcgctcatattcactctcctttctttttaccatttcaaacaggcgggtgttttccggtacggcaatcccatgcgcgcgggcgcggcgtaagagaaaaccattgatatagtcgatttcagtgtggcgcagcgcgcggatatcctgcaacatcgacgagatattttccgctgtggcatcaatcacctgcatcacgtaatcacgcaaatcttctgctgaagtatgatgcccttcgcgttcgatcaccgccgcgacttcttcgcatatctgcataatttcttgcggatgatgacgtaattcaccgttcgggcaattccagatggcagtcagtggattaatcacgcagttgactgccagcttgcgccacagctcggcgcgaatattgttatgccaggcaacgtcaggcaacacggtttgcaaaatatccgccagataactgtaatccccgtcctgttgccgtgccgggccaatatgcgtgataccgtttgccacatgaataatgacattgccgtcgcggcgggctgcatgggtggtggtgcccatcagtaatggctgctgaatgttttgcaactcttcgatggtgcccatgccgttgtgaattaacagtattggcgtagttacaggcagtgtggacgcgaggcttttgacggcatcggaaacctgccatgctttcagcgtcaccaggagcagatcgctggtggcgagaaaatcgggatcgttggcggtcagcgattcgttaaatatcgaaccatctgtctcaaccagattcacgctacaataaggttgcggtacgcgcagccagccctgaacttcatgaccctgtttgcaaagtgctgtaagccataattgccctaaggcaccgcatcccaatacggtaattttcattgttcctcctcacccgcaaccactccgggtgttcaataaggctatcccttaattgtgcatgctgttgcgactatgcacaattaagggatacgtcctggtgcaggactgtcggttatttaactttgcgggtattatgcttcgcatcaaaaatgaagggagaggaaaagatgccatctttcgatattgtctctgaagttgatcttcaggaagcacgtaacgcggtcgataacgcgagccgcgaagtggagtcccgttttgacttccgtaacgttgaagcctcatttgagctgaacgacgccagcaaaaccatcaaagtgttgagcgagtccgatttccaggtcaatcagttgctggatattctgcgtgccaagctgctgaagcgcggcattgaaggcagttcgctggatgtaccggagaatatcgttcatagcggtaaaacctggtttgtggaagcgaaactgaaacagggcattgagagcgcgacccagaagaaaatcgtcaagatgatcaaagacagcaaactgaaagtgcaggcgcaaattcagggcgatgaaatccgcgtaacgggcaaatctcgtgatgatttgcaggctgtcatggcgatggtacgtggtggcgatctcggtcagccgttccagttcaaaaacttccgcgattaatcgcgactatgtgcgttttgttcatgtcagatgcggcatgaacgcctgattcggcctacaaaggtttgtaattcagaaactttgtaggcctgataagcgtagcgcagcaggcaattcgccgcgttttttatgcctgacgaattgcctgttctatctcaaagcgattcgtcactttgctgtcgattttcacataagctgaatgttcttcttctgcaatcaacacttctttgatgccttcagtttctagcaaacgcacttttaacgcctcgtttgcggcaatgttcgccgggatttcaatgcgcaaactgctgacatacggcggttctttcatggtactggcgactgtcagccacactgcggccagcattgcgccagcgagaaataccccctgaccgtcaaacatgccgttaatccagccgcccagcgaaccgccaatcgccacgccaagaaactggctggtggagtaaacacccatcgccgtacctttgtaacctgctggcgactctttactgataagtgagggcaggagggcttccatcaaattaaacgccacaaagaaaagctgcacgccgaccaccagttgccagaactgcgtttgcgcgttccacaacacaatttccgcaaccacgatcaacccgacgcagaagacaaagacttgcttcattttgcgcttaacttcagcgtagataatgaaaggcacgaccgagccaaaggcgattagcattgtcgccagatagaccttccagtgttcagccgccgggaaccctgcatcagccagttgtccgggcagggcaacaaacgtcgacatcagcaaaatatgcagacacataatgccaaagttgagtttcagcagccgcggttccgccagcactttactgaaactgcctttcaccattccggactcacgattaagtacgtgagtgctactgttgggcacaacccaaatggtcaacgcaatgccggtcgttgccagaatagcgatcatccagaacagcgcgtgcagcccaagtttgtgagtgatgatcgggccaagcaccatcgcaatggcaaaggtaatgccaaagctcacgccgataaacgccatcgctttggtgcggttttgttcgcgcgtgagatcggaaagcagcgccataacggcggcggcaattgctccagagccttgtagcgcccggcccagaataattccccagatggagtcggaaagcgcagcgataacgctaccggcggcaaacaccgccagcccaccgacaattaatggtttgcgaccaatgcggtcggaaagcaggccaaacggaatctgaaaaacggcctgagtcagaccataaataccaatggcaataccgattaatgcttcgctggcaccttgcagagccatgccgtacgtggtcagaaccggcagaaccataaacatgcccagcatgcgcaacgagaatacggtccctaaaccccaggtcgcgcgcctctcacctggcgtcattttataatcgttcattaccacctctgttttaaattcgcgactagtgtaaagcggcaaacgaatggggtaaacatgcggattttttagtaaatatttcgagagggatatgtttctaatgctaagaaaaaaggtgccgtagcacctttttaatagagaggttttgttaccacacagcagccagcagcgtatgcgagtccggtaccataaaatcaacggacatcatcaccgagagggcagtgatggcgatgatagagaagccgaacagcttgcgcgcccagattctgtcatcagcaactttataaccgcgcagagccatacctaaccaccagacgctaaccgccgcggcgaccaccagatatttatacccagcgtaaccgccaagagagagcatcagcgtggcaacggcaaaggcgatgatatacagcgtgatgtgattcttcgccaccgaaatgccttttaccactggcaataccggaatgtttgccgcctggtaatccttaaagcggaaaatggcgatggcataggagtgaggcatctgccacaggctgaagatagccagcaggatcgctgcgccgctatcgaactcaccggttaccgcacagtagccgatcaccggcggcgcagcgccggagagcgaaccaatcaacgtgccgtagacagagtggcgtttcatgtacaggctataaacgccgacataaaccacaaagcccatcacccccagccagcaggccagcggattcgcgccaaaccacagcagcataaagccagcaatacccagcaacgtggcgtacaccagcgagacagcaggagagatcaggcctttcaccagcacccgattcttcgtcctttccatctttctgtcgatatccctgtcgatgtagttgttaaacacacaacccgacgccacaaccagtgacaccccaaccagcgtgtagataaacaggggataatcaatgctgccctttgaggccagcaggaatcccccaatcaccgagatcaggttgccaaagatgatgcctggtttcgttacttgcaggtattgcttaaacatcataaccgccgctcttagtgcatcatcatgttgtagttgaggttccacataatccagatggagcctacaaccaggatagcgatgattagcacggtgaagacaaacgccgtcatgttccagccttcatctgatttggtattcatgtgcaggaagcacaccagatgcaccagaacctgtaccactgccattgccaggattgttcccagaattacggccggagaggcagctcctgtcatcaccatccagaacggaatcaccgtcagaatgatcgacaggataaagcctgtcatgtaggtttttacgctgccatgggacgcgccgctgtgatcggtagaatgactcattacatcgcccccatcagataaacaacagtgaacacacagatccaaaccacatccaggaagtgccagaacaggctcaggcacatgatgcgggtacggttagtgctggtcaggccgcgacgggcgatttgcaccatcagcaccgccatccagataagaccagaagtgacgtgcagaccgtgcgtgccgaccagcgcaaagaacgctgacaggaagccgctgcgatccggacccatgccgttaacaatcaggtgatggaattcatagatttccatcccgataaatccggcaccaaacaaccaggtcaacgccagccaggagataacctggcttttgttgtttttgtacatggcgatagccgccatgccgtaggtgatggagctgaacaacagcaagaaagtttcaaccagaacgaacggcagttcgaaaatgtccttacctgtcgggccgcctgcggtgccgttcaccagaacggcataggtagcaaacaagatagagaacagaatgcagtcgctcatcaggtagatccaaaatccgaagattttggttccgcctgcatcgtggtgcccgtgttcgtgcgcgtgggcagtcgcgtgcgtcaaagtatcagttgccatttttcagccctgccttagtaatctcatcgaaatgctggttttccagtttttcgatttctgccaccggcacgtagtaatccacgtcctcgtcgaagcttttcacgatccaggtgatgatcatgcctgcgaagccaacaatcgccagccaccagatatgccagatcatggcgaaaccgaagatggtggagaaagctgcaatgacgatacctgcaccgctgtttttcggcatatgaatttcttcatagtggtcaggctttttatacgcttcgcctttctctttcatttcccagaatgcatcacgttcgtgaacgtgcggcactacggcaaagttatagaacggaggcggggaagaggttgcccactccagcgtacggccaccccacgggtcgccagtcaggtcacggttctggtcgcggtcgcgaatagaaacgtacatctgaataacgaggcagagaatacccagcgcaatcagtactgcaccgctggctgcaatcatcagcatggtgtggaactgcgggtcaatctgctggctcaaacgacgggtcatgcccatgaagcccagcgcatacagtggcataaaggcaacgaagaagccgatgatccagaaccagaacgcgcgtttaccccaggtttcgttcagtttgaaaccgaacgctttaggccaccagtaggtcatccctgcgaagcagccgaagaccacgccgccgatgatcacgttatggaagtgcgcaatcaggaacaggctgttatgcagaacgaagtccgcgcccggtacggccagcagcacgccagtcatcccgcccaccgagaaggtgacgataaaaccgatggtccacagcatcgcagaatggaacacgatgcggccctgatacatggtgaacagccagttgaagatcttcaccccggtcgggatggcgataatcattgtggtgataccaaagaaggcgtttacgttcgcgcccgcacccatcgtaaagaagtggtgcagccaaacgatgaacgacagcacggtgatacagacggttgcccataccagcgaggtataaccaaacagacgtttacgcgagaaggttgccgcaatttcggagaacacaccgaaaacaggcaggatcaggatgtaaacttccgggtggccccaggcccaaatcaggttgatgtacatcatcatgttgccacccatatcgttggtaaagaaatgggtgcccagatagcgatccagggtcaacaacgcgacggtaaccgtcagaattgggaaggaagcaataatcagtacgttcgcgcacagtgatgcccaggtaaatactggcatcttgaacatggtcatgcccggtgcgcgcatcttcagaatggtaacgaagaagttgataccggtaagcgtcgtacctataccggatagctggagactccatatccagtaatcgacaccgactcccggactgtactctattcccgatagcggtggataggccagccagccggtctgcgcaaattcgcccacgccgagagaaacgttaaccagaatcacaccaacaacggtaaaccagaagcttaagttgttgaggaacgggaacgcaacgtcacgcgcgccgatctgcagcggaaccaccaggttcatcagaccgataacgaaaggcatcgccacgaagaagatcataatcacgccgtgcgcggtaaagatctgatcgtagtggtgaggtggcaggaagcccgcttcgcccgccgaggcaagagcctgctggctacgcatcataatggcgtcagcaaaaccacgcagcaacatcacaatcgccacgatgatatacatgataccgaggcgtttatggtcgacggaggtcagccactctttccacaggtaggtccacttaccgaagtaagtgatcaggccaacgagcgccagacctcccaaaataatgccagcgatcgtaaccatgacgataggttcatggaacgggactgcatcaagtgataattttccgaacatctttattcttcctcaacccctttaatgggcggattccgcgtggctcatgtccatgccttccataccttcgtgtgcgctgtgctcaccttctggctgggtcatgtccatgctcttaccgtgagccataaacttgttaattacatcggcaaacaagtctggtttcacgttggagaaatattccacctggttgtattcgctaggcgcggccagtttttcgaacgcagccatgtcagacatggtgttcggcgactgcttcgcttttgcgacccactggtcgaatgcggcgcgatccggtgttgcaatagctttgaacttcatgcctgagaagcccgggccgctgtagctggcggagataccgtcataagtgccgggttcgttggcgatcagatgcaggcgagtctgcataccggccatggcataaatctggctacccagacgcggaatgaagaaggagttcatcacggagttggaggtcactttgaagtacaccggagtgttcgccgggaaagcgatttcattcacggtagcaatgccctgttccgggtagatgaagaaccatttccagtccatggaaaccacttcgatggtaatgggcttctcgtcgtgtgccagcggcttgctaggctcaagagcgtgagtggttttccaggtcagtactgcaaggaagatgatgattaagataggtaccgtccagaccacagcttccactttattggagtgtgaccagttcgggctgtacttagcatctttattgctcgcacggtacttccaggcgaaaccaacagccatcaagattgcgggaataacgacaatcaacatcaggccaaatgccgtcagtatcagtgaacgttgctccagaccaatctgtcctttgggatctaacagcgcagaattacagccactgagcaatacagtgcctgcaaataatgacaaccatcccaaacttttattgtatttcctgagtctcatttaacgacctcaattccacgggatctggtggcgtttaaagtgtgtgggcattttacgggaaggttacattactgtaaacatgattaaattcctgttacttggatttggctgccaggtcacatatgttgcaaaacatatcaggttgattttaagaagctgttgcaaaagggcgttataacaaaaggggagtgctgaaggagtctgggcgggcaattggtataaccaatgtgaaataaaacaattatttaacaaataattatcattagagtgacaactgggtgatgagaaaataaagactcattagctgaatcgtgtaagaaaaatagaatttataaatggcgccaataatttccaaacgctaagccgcacaaaagaacaaatattaataagcgatactgatgtttatttagccgtaataattacggcgagtgattactacagctaaataatatttacagattacgtcagatgcgtttttcgtagcgccagataatccagcaaaccaccaagcacgacgccagaaagggcgactaaaaccccgacttccagcagagcaggcaggaaagagaagtgcgtcaaatccagcgcgtccatcgtcaatagcagtaaccacacggccaacaggctgacgcccgccgccagtgtccacatggcaaaggcataacctgccggatatgcggtacgggagataaagttgtcatttactcgtgtatattcaagcgtctggcggcaaaccagcagcaaaataagccctggtacggcagcggcgacggagaatagatagaatgtcgaccagccgtgtgcttcaacaaaccaacccgccacggggccgacataaactcgccctacagcagaaagcgctgagagcagggcaaattgagtagcggaaaatgacttattacatagcgtcattaacagcgcgacaaaggctgatgtgcccatcccgccacagaggttttcgaaaaagacggctgcgcccatgctgtagagatgcttatcagtaatcgacagcagccagtaaccggcgttagacgcaccttgtaaaatgccgaaaatcagcagtgcccggaacagtgacaggcgctgcatcaaaatcccaccgtacaatgcgccaacaatggtcgctagtaagccaagcgttttgttaaccacgcctacttcacccgcatcaaacccgacgccgcgaatcaaaaacgtggttgtcaggctcatggcgaatgcgtcgcccagcttatacagcacgataagaagcaaaataagccaggcattattgcgaccaaagaaatctcgcagaggtgcaacaaccgcttgttccagcgttttgggcacaggaatggtgtcggttggttctggtgcaagcaacgtcgcgataatacaggggatcaacagtgccgccattaaccagtacatgccctgccagcccagccatttatctgccagccacagggctaggccgccggaaaccagcatccctaaacggtaacccagcacgctgattgccgcgcccgcaccacgttcttctgccggaagcacatcggttttccacgcatcgaagactatatcctgggaagcagagcaaaaagcgatcaccactgccagcgccgccatccagcggagttgggtgcctggttcgagaaaacccatcgccgcaatggcgactaataacaggatttgcgtggcgagcagccaaccgcgccgccgcccaaaaaatggaggcgtgtagcggtccatcagcggtgaccagaggaatttaaaaacgtaagcctggcctaccagagagaagaaaccaatggttttgagatcgatattctcgaccgtcatccaggcctgtaaggtaccggatgtcagggcgagcggtagcccggaagcaaaacccaggatcagcaatatggctgaacgcggctgttgaaaaatacgtaaatattgactggacatgggcgtctacaggcccggcttgcaccgggccagagggcagaaattaacgcgcgttctgcttgatgaattcgtggatgctggtgtcctgagacatatcagcgatggtatcggtcagcacactgttaaccgcatcggcgatatttttgttggaggcctggaacgcaccttcaacgttgtagctggcacgatagtttttggtcattttgttgccattctgcgcggtagcgatgatggcgatatccgctttggtcgcgatgttgtagcgcacgttgccctgggacacgtcagcatacagttggctaacgatgatttgcagattaaccgggccattcggaccaaccatgtaaccacgcgcggtcatctgtttttccagcacttcttgcagcaggaaacgcagatcgcgggaggcggtcagggtaacgatttgattatcgcgggtgacttttgccagcgcctgatcggtacgctgatcggcaccattaatgcttacggtgacgcccatcaggcttggatcctgctgtggcagtgtaatcgtcggggaaacttcaatagttgttggcggttttgcgcatcctgcaagcataaacagagcaactaacgggaagaggatttttttgaacatgttcgggctctcagagactcttaagcgtgtttggtaaaaattcccgccatcataacattgccaacggcgaggggaagtgggtaaggcatgtaaattcatcatgttgacgaaataatcgcccctggtaaaagaaacactgatgcgaggcctgtgtttcaatctttaaatcagtaaacttcatacgcttgacggaaaaaccaggacgaaacctaaatatttgttgttaagctgcaatggaaacggtaaaagcggctagtatttaaagggatggatgacatctcagcgttgtcggaggagatatttcatgatgatacgtgagcggatagaagaaaaattaagggcggcgttccaacccgtattcctcgaagtagtggatgaaagctatcgtcacaatgtcccagccggctctgaaagccattttaaagttgtgctggtcagcgatcgttttacgggtgaacgttttctgaatcgtcatcgaatgatttacagtactttagcggaggaactctctactaccgttcatgcgctggctctgcatacttacactattaaggagtgggaagggttgcaggacaccgtctttgcctctcctccctgtcgtggagcaggaagcatcgcgtaaaaacgcatttgcaactgtcggcgcttttccagtatgttgctaaagattttatgaaaaacggcctgcgggccgttttgttttgtctggattttgcgctttttgcccagcattcagacgaaaattgcccgggaattgtgaaaaaatacgcgacagcgcgcaataaccgttctcgactcataaaagtgatgccgctataatgccgcgtcctatttgaatgctttcgggatgattctggtaacagggaatgtgattgattataagaacatcccggttccgcgaagccaacaacctgtgcttgcggggtaagagttgaccgagcactgtgattttttgaggtaacaagatgcaagtttcagttgaaaccactcaaggccttggccgccgtgtaacgattactatcgctgctgacagcatcgagaccgctgttaaaagcgagctggtcaacgttgcgaaaaaagtacgtattgacggcttccgcaaaggcaaagtgccaatgaatatcgttgctcagcgttatggcgcgtctgtacgccaggacgttctgggtgacctgatgagccgtaacttcattgacgccatcattaaagaaaaaatcaatccggctggcgcaccgacttatgttccgggcgaatacaagctgggtgaagacttcacttactctgtagagtttgaagtttatccggaagttgaactgcagggtctggaagcgatcgaagttgaaaaaccgatcgttgaagtgaccgacgctgacgttgacggcatgctggatactctgcgtaaacagcaggcgacctggaaagaaaaagacggcgctgttgaagcagaagaccgcgtaaccatcgacttcaccggttctgtagacggcgaagagttcgaaggcggtaaagcgtctgatttcgtactggcgatgggccagggtcgtatgatcccgggctttgaagacggtatcaaaggccacaaagctggcgaagagttcaccatcgacgtgaccttcccggaagaataccacgcagaaaacctgaaaggtaaagcagcgaaattcgctatcaacctgaagaaagttgaagagcgtgaactgccggaactgactgcagaattcatcaaacgtttcggcgttgaagatggttccgtagaaggtctgcgcgctgaagtgcgtaaaaacatggagcgcgagctgaagagcgccatccgtaaccgcgttaagtctcaggcgatcgaaggtctggtaaaagctaacgacatcgacgtaccggctgcgctgatcgacagcgaaatcgacgttctgcgtcgccaggctgcacagcgtttcggtggcaacgaaaaacaagctctggaactgccgcgcgaactgttcgaagaacaggctaaacgccgcgtagttgttggcctgctgctgggcgaagttatccgcaccaacgagctgaaagctgacgaagagcgcgtgaaaggcctgatcgaagagatggcttctgcgtacgaagatccgaaagaagttatcgagttctacagcaaaaacaaagaactgatggacaacatgcgcaatgttgctctggaagaacaggctgttgaagctgtactggcgaaagcgaaagtgactgaaaaagaaaccactttcaacgagctgatgaaccagcaggcgtaatttacgcagcataacgcgctaaattcgcacaaaggcccgtcaccgccaggtggtgggcttttttttgtcatgaattttgcatggaaccgtgcgaaaagcctctttcggtgttagcgtaacaacaaaagattgttatgcttgaaatatggtgatgccgtacccataacacagggactagctgataatccgtccataaggttacaatcggtacagcaggttttttcaattttatccaggagacggaaatgtcatacagcggcgaacgagataactttgcaccccatatggcgctggtgccgatggtcattgaacagacctcacgcggtgagcgctcttttgatatctattctcgtctacttaaggaacgcgtcatttttctgactggccaggttgaagaccacatggctaacctgattgtggcgcagatgctgttcctggaagcggaaaacccagaaaaagatatctatctgtacattaactccccaggcggggtgatcactgccgggatgtctatctatgacaccatgcagtttatcaagcctgatgtcagcaccatctgtatgggccaggcggcctcgatgggcgctttcttgctgaccgcaggggcaaaaggtaaacgtttttgcctgccgaattcgcgcgtgatgattcaccaaccgttgggcggctaccagggccaggcgaccgatatcgaaattcatgcccgtgaaattctgaaagttaaagggcgcatgaatgaacttatggcgcttcatacgggtcaatcattagaacagattgaacgtgataccgagcgcgatcgcttcctttccgcccctgaagcggtggaatacggtctggtcgattcgattctgacccatcgtaattgatgccagaggcgcaactgtgccgctatacttatccagggcggcacaacgctgtaagcggcttgcgcctgagaatggcatttgcgtcgtcgtgtgcggcacaaagaacaaagaagaggttttgacccatgacagataaacgcaaagatggctcaggcaaattgctgtattgctctttttgcggcaaaagccagcatgaagtgcgcaagctgattgccggtccatccgtgtatatctgcgacgaatgtgttgatttatgtaacgacatcattcgcgaagagattaaagaagttgcaccgcatcgtgaacgcagtgcgctaccgacgccgcatgaaattcgcaaccacctggacgattacgttatcggccaggaacaggcgaaaaaagtgctggcggtcgcggtatacaaccattacaaacgtctgcgcaacggcgataccagcaatggcgtcgagttgggcaaaagtaacattctgctgatcggtccgaccggttccggtaaaacgctgctggctgaaacgctggcgcgcctgctggatgttccgttcaccatggccgacgcgactacactgaccgaagccggttatgtgggtgaagacgttgaaaacatcattcagaagctgttgcagaaatgcgactacgatgtccagaaagcacagcgtggtattgtctacatcgatgaaatcgacaagatttctcgtaagtcagacaacccgtccattacccgagacgtttccggtgaaggcgtacagcaggcactgttgaaactgatcgaaggtacggtagctgctgttccaccgcaaggtgggcgtaaacatccgcagcaggaattcttgcaggttgatacctctaagatcctgtttatttgtggcggtgcgtttgccggtctggataaagtgatttcccaccgtgtagaaaccggctccggcattggttttggcgcgacggtaaaagcgaagtccgacaaagcaagcgaaggcgagctgctggcgcaggttgaaccggaagatctgatcaagtttggtcttatccctgagtttattggtcgtctgccggttgtcgcaacgttgaatgaactgagcgaagaagctctgattcagatcctcaaagagccgaaaaacgccctgaccaagcagtatcaggcgctgtttaatctggaaggcgtggatctggaattccgtgacgaggcgctggatgctatcgctaagaaagcgatggcgcgtaaaaccggtgcccgtggcctgcgttccatcgtagaagccgcactgctcgataccatgtacgatctgccgtccatggaagacgtcgaaaaagtggttatcgacgagtcggtaattgatggtcaaagcaaaccgttgctgatttatggcaagccggaagcgcaacaggcatctggtgaataattaaccattcccatacaattagttaaccaaaaaggggggattttatctcccctttaatttttcctctattctcggcgttgaatgtgggggaaacatccccatatactgacgtacatgttaatagatggcgtgaagcacagtcgtgtcatctgattacctggcggaaattaaactaagagagagctctatgaatcctgagcgttctgaacgcattgaaatccccgtattgccgctgcgcgatgtggtggtttatccgcacatggtcatccccttatttgtcgggcgggaaaaatctatccgttgtctggaagcggcgatggaccatgataaaaaaattatgctggtcgcgcagaaagaagcttcaacggatgagccgggtgtaaacgatcttttcaccgtcgggaccgtggcctctatattgcagatgctgaaactgcctgacggcaccgtcaaagtgctggtcgaggggttacagcgcgcgcgtatttctgcgctctctgacaatggcgaacacttttctgcgaaggcggagtatctggagtcgccgaccattgatgagcgggaacaggaagtgctggtgcgtactgcaatcagccagttcgaaggctacatcaagctgaacaaaaaaatcccaccagaagtgctgacgtcgctgaatagcatcgacgatccggcgcgtctggcggataccattgctgcacatatgccgctgaaactggctgacaaacagtctgttctggagatgtccgacgttaacgaacgtctggaatatctgatggcaatgatggaatcggaaatcgatctgctgcaggttgagaaacgcattcgcaaccgcgttaaaaagcagatggagaaatcccagcgtgagtactatctgaacgagcaaatgaaagctattcagaaagaactcggtgaaatggacgacgcgccggacgaaaacgaagccctgaagcgcaaaatcgacgcggcgaagatgccgaaagaggcaaaagagaaagcggaagcagagttgcagaagctgaaaatgatgtctccgatgtcggcagaagcgaccgtagtgcgtggttatatcgactggatggtacaggtgccgtggaatgcgcgtagcaaggtcaaaaaagacctgcgtcaggcgcaggaaatccttgataccgaccattatggtctggagcgcgtgaaagatcgaatccttgagtatcttgcggttcaaagccgtgtcaacaaaatcaagggaccgatcctctgcctggtagggccgccgggggtaggtaaaacctctcttggtcagtccattgccaaagccaccgggcgtaaatatgtccgtatggcgctgggcggcgtgcgtgatgaagcggaaatccgtggtcaccgccgtacttacatcggttctatgccgggtaaactgatccagaaaatggcgaaagtgggcgtgaaaaacccgctgttcctgctcgatgagatcgacaaaatgtcttctgacatgcgtggcgatccggcctctgcactgcttgaagtgctggatccagagcagaacgtagcgttcagcgaccactacctggaagtggattacgatctcagcgacgtgatgtttgtcgcgacgtcgaactccatgaacattccggcaccgctgctggatcgtatggaagtgattcgcctctccggttataccgaagatgaaaaactgaacatcgccaaacgtcacctgctgccgaagcagattgaacgtaatgcactgaaaaaaggtgagctgaccgtcgacgatagcgccattatcggcattattcgttactacacccgtgaggcgggcgtgcgtggtctggagcgtgaaatctccaaactgtgtcgcaaagcggttaagcagttactgctcgataagtcattaaaacatatcgaaattaacggcgataacctgcatgactatctcggtgttcagcgtttcgactatggtcgcgcggataacgaaaaccgtgtcggtcaggtaaccggtctggcgtggacggaagtgggcggtgacttgctgaccattgaaaccgcatgtgttccgggtaaaggcaaactgacctataccggttcgctcggcgaagtgatgcaggagtccattcaggcggcgttaacggtggttcgtgcgcgtgcggaaaaactggggatcaaccctgatttttacgaaaaacgtgacatccacgtccacgtaccggaaggtgcgacgccgaaagatggtccgagtgccggtattgctatgtgcaccgcgctggtttcttgcctgaccggtaacccggttcgtgccgatgtggcaatgaccggtgagatcactctgcgtggtcaggtactgccgatcggtggtttgaaagaaaaactcctggcagcgcatcgcggcgggattaaaacagtgctaattccgttcgaaaataaacgcgatctggaagagattcctgacaacgtaattgccgatctggacattcatcctgtgaagcgcattgaggaagttctgactctggcgctgcaaaatgaaccgtctggtatgcaggttgtgactgcaaaatagtgacctcgcgcaaaatgcactaataaaaacagggctggcaggctaattcgggcttgccagcctttttttgtctcgctaagttagatggcggatcgggcttgcccttattaaggggtgttgtaaggggatggctggcctgatataactgctgcgcgttcgtaccttgaaggattcaagtgcgatataaattataaagaggaagagaagagtgaataaatctcaattgatcgacaagattgctgcaggggctgatatctctaaagctgcggctggccgtgcgttagatgctattattgcttccgtaactgaatctctgaaagaaggggatgatgtagcactggtaggttttggtacttttgccgttaaagagcgtgctgcccgtactggccgcaacccgcagaccggtaaagagatcaccatcgctgctgctaaagtaccgagcttccgtgcaggtaaagcactgaaagacgcggtaaactaagcgttgtccccagtggggatgtgacgaagttcaagggcgcatctactgatgtgccttttttatttgtattcggtgactttctgcgtcttgtgggctgacaattgcccccgtttcttgtcacaataggcctttgcgcgcatcgatacgttgcgtgaggtacacagtcatctacagcggagtgttgttacaccatgatggacagcttacgcacggctgcaaacagtctcgtgctcaagattattttcggtatcattatcgtgtcgttcatattgaccggcgtgagtggttacctgattggcggaggcaataactacgccgcaaaagtgaatgaccaggaaatcagccgtgggcaattcgagaacgccttcaacagcgagcgtaatcgcatgcagcaacagctgggcgatcaatactccgagctggcagcgaacgaaggctatatgaaaaccctgcgtcaacaggtgctgaatcgtctgatcgacgaggcgctgctggatcagtacgcacgtgagctgaaactgggtatcagcgatgagcaggttaaacaggcgattttcgcgaccccagccttccaggttgacggcaaatttgataacagccgctataacggtatcctcaaccagatggggatgaccgccgatcagtacgcccaggcgctgcgtaaccagctcactacccaacagctgattaacggcgttgccggtaccgattttatgctgaaaggtgaaaccgacgagctggcggcactggtcgcgcaacaacgcgtggtgcgtgaggcgactatcgatgttaacgcgctggcggcgaagcagcctgtgaccgaacaggagattgccagctactacgaacaaaacaaaaacaatttcatgacgccggaacaattccgcgtgagttacatcaagctggatgccgcaacgatgcagcaaccggttagcgatgcggatatccagagctactacgaccagcatcaggatcaattcacccagccgcagcgtacccgctacagcatcatccagaccaaaactgaagatgaagcgaaagcggtacttgatgagctgaataaaggcggtgattttgctgcattagccaaagaaaaatctgccgatattatctctgctcgtaacggcggcgatatgggttggttagaagatgccactatcccggacgaactgaaaaatgctggtctgaaagaaaaaggccaactgtctggtgtcatcaaatcttcggtcggtttcctgattgtacgtctggacgacattcagccagcgaaagtgaaatcgttagacgaagtacgtgacgacattgcggcgaaagtgaaacacgaaaaagccctcgatgcgtactacgcgctgcagcagaaagtgagcgatgcggcaagcaacgacaccgagtctctggccggtgcagagcaagctgccggcgttaaagccactcagacgggttggttcagcaaagataacctgccggaagagttgaacttcaagccggttgccgacgctatctttaacggcggtctggtaggtgaaaacggcgcgccgggcatcaactctgacatcatcaccgtagacggcgaccgcgcattcgtgctgcgcatcagcgagcacaaaccggaagcggtgaaaccgttggcagatgttcaggaacaagttaaggcattggttcagcacaacaaagctgaacaacaggcgaaagtggatgctgagaaactgctggttgatttgaaagccggcaaaggtgcggaagctatgcaggctgccggtctgaaatttggcgagccgaaaaccttaagccgttccggtcgtgacccgattagccaggcggcgtttgcactgccactgccagcgaaagacaaaccgagctacggtatggcgaccgatatgcaaggtaatgtggttctgctggcgctggatgaagtgaaacaaggttcaatgccggaagatcagaaaaaagcgatggtgcagggtatcacccagaacaacgcacaaatcgtctttgaagctctgatgagtaacctgcgtaaagaggcgaaaatcaaaattggcgatgcgctggaacagcaataatcctgaagccgcctcgcaaaaaaatgcgttgcagctgtaacaagaaaaggtcgctttcgcggccttttccatttctgaacattgccatttgtttactgttttcactgccgttaaggtgattccactgttaacaaacaaggagaaaacagtatgaaacacggaattaaagcactgctcattaccctgtccctggcctgtgccggaatgtctcatagcgcgctggcggcagcttctgtggcgaaaccgacggcggtagaaaccaaagcggaagctcctgcagcacaaagtaaagcagcagtaccggcgaaagccagtgacgaagaaggcacccgggtcagcattaataatgccagcgcggaagagctagcccgcgcgatgaatggcgttggcctgaagaaagcgcaggcgattgtcagttatcgcgaagagtacggtccgtttaaaactgtggaggatctaaagcaggtgccggggatgggcaattcgctggtggaacgtaatctggcggtattaaccctgtaattaatttgcatagtggcaattttttgccagactgaagaggtcataccagttatgacctctgtacttataacaacaacgtaaggttattgcgctatgcaaacacaaatcaaagttcgtggatatcatctcgacgtttaccagcacgtcaacaacgcccgctaccttgaatttctcgaagaagcccgctgggatgggttggaaaatagcgacagttttcagtggatgacggcccataacatcgccttcgtcgtggtcaatatcaatattaactatcgtcgcccagcggtattaagtgacctgttaactattaccagtcagttgcagcaattaaacggtaaaagcggcatcttaagccaggtcattacactggagccggaagggcaggtggtagcggatgcgcttattacgtttgtttgtattgatcttaaaacgcagaaagcattagctctggaaggggaattgcgcgaaaagctggagcagatggttaagtaaacgttttgtggtgccggatgctcaagccgcatccggcgacacccggaataattacctcaacccggttttctgcttcatcgctgccatcaccgtcggtttatcggccagataatgattcaaaccgttggcgcgtaaattacatgccgcacaatgaccgcaaccgtcgcctttaaagccgttatagcaggtcaacgtttcgttacggactaaatccagtttgccgtaataatctgccagcgcccaggtttccgctttatcaatccacatcagcggcgtttcaaaacgaatatctttcgccatgcccaaactgacggcatggtttagtgctttcacaaactcatcgcggcaatccgggtagccggagaaatccgtttcgcagacgccagtaattacggcttctgcttttacctgatacgcatatattgccgccagcgtcaggaacaaaatattacgccctgggacaaacgtattcgggataccatcggcttcaggttcataatcaggcaccggaatgctgtcacgcgtcaggctactgaccgccagctcgttgagcagggtgacatccagcaccttatgcgcgcgtgcccccagtttcagcgccagttcgcgtgccacgtcgatttctgcgcgatgccgctgaccgtaatcgaacgtcacgcaatggacttcatcatattgttgtaatgcctgcaccagacaggtggtggaatcctgacctccactgaacacaacgacagcacgtttcatagataatcctgcttgaacaataaaagcgttatggtaacgcctgcgattaacccggaccagctattcattgcgatggcgcgggaagccaggcttcggtaaattcaaaccagccgcgcggtgtcagtcgcacaccgttcacgccgggaggggcactaatgcgatagtgatagttgaacagcggcgtcagcgtcgcatctgtcattaactggctaaaaaccgctttcagggcattaaatcggttttcttcatcaggcattatttgcacggcatccagtgtcgattgtagatgtgcgtatgctggagcgtcgaaaacatgtggccacagcggatcgcagcgcagccattgctccagagtatattccggtgcttcgccaattaatctgtcgcccatcatgaggtctgcgtgtgcctgtagggtcgtgtcgtcccagttttttgcgttatgaaaaataattgtgagttcacagccttccgctgccagtgtcgcctgtaggcgttctgccatggtatgaagttctatcggtaggtgataaaccagcgtcaaggttttcggtagtttgacttcatccggtacctgccaatgcggaatagtccagcctggcagtaatgcatgactggcggtgatcaggttttctccgacttctaacgtttgtaataaaccggattgatgaataatggagatcacttttcgcgcctgccagagggagagtcggggacttttgcgcaacgtcaaatagcaaaaacctaaactgatgccgctactgacctggctgacccgttgcagctcctccggtttgccgatggtgatttgcacgggatgccgacaactggttcccaaatctttttcgaaaagcggcggagttatccagtactcaaccgctttaagcagcggatgacgtaaatggtaataatcatggctttccaggcgcaccagctctgctgtgaattgtgttaagcgaaaaggacccgtgccgatcagtgggaattgcggatgcgccagatggctgcaatagctcgccagccggtgcgcaagccagtaatcagggcgatgtaaaaagaaggtcagacactgcggatgggtgacttcaatacgcttcacgctaataaataattgatccagtgctggcagttgtaacagcatcaataatcgctggtgtaagtgtgaggcttttactgcatcgccgttatgccagtgtagggttgaacgaagataaaagtcccagcgtaacccgtcagtagaggtttcccagtgatgcgctaaatcgccaatcgggcgctgagtattattatcgaagcgggtcaggccggaaaatatctgcccggcgagatgctgctcggcacggccgggcaaaaagcctggttgtagcggttcgagcgggcgatagtagggaatacgcaacgtgggtgtatcgttttgccattgtccgcccataaacggctgtaacagagtgcgcagctcacctggggccagttgcgccagctccagcacatcttgctgctttccggtttccagtgcctgttccatcatcgcattgcgtagcgattccggcgtgaccagaaagcgtaattgtccgcgctttccgcgtcctgactgcgcctgccactccagccatcccgcctcctgtgcctgacgcaacagcgtacgaacatggcgttcgctgcaaaaacagcgttcggccagttcgctgacggtgacggtttgcggctttccggcggaaggttgccacagacgttgatactggttaagacggttgagcaatcgcatataaacccggaacaatattatttaactattcactattacttccgtatatatcaggtgatactcaatcaccattaaccgtgtcacagagtggagaaagaaatggctcgtctggcagcatttgatatggatggcactttattgatgcccgaccatcatttaggtgagaaaaccctctctactttggcgcgactgcgtgaacgcgacattaccctcacttttgccacggggcgtcatgcgctggagatgcagcatattctcggggcgctatcgctggatgcgtatttgattaccggcaacggaacgcgcgtgcattctctggaaggtgaacttttacatcgtgatgatttacctgcggatgtcgcggagctggtgctgtatcagcaatgggatacccgagccagcatgcatatcttcaatgacgacggttggtttaccgggaaagagatccctgcgttgttgcaggcatttgtctatagcggttttcgttatcagataatcgatgtcaaaaaaatgccactcggcagcgtcaccaagatctgcttctgtggcgatcacgacgatcttacacgcttgcagatccagctatacgaagcattaggcgagcgtgcacatttgtgtttttccgccacggattgcctcgaagtgctgccggtgggctgcaataaaggcgctgcattgacggtgctgacccaacatttaggtttatcgttgcgcgattgcatggcctttggtgatgcgatgaacgatcgcgaaatgttagtcagcgtcggtagcggatttattatgggcaatgcgatgccgcaactgcgcgcggagctcccgcatttaccggtgattggacattgccgaaatcaggctgtctctcactatttgacgcactggctggactatccacatctaccttattcccccgaataacgagatcccttccagcaccgggcaattgcccggttttttttgcgttgaatttgtcattttgtgccgtggtgtttaaaccgcacagaataaattgtcgtgatttcacctttaaaataaaattaaaagagaaaaaaattctctgtggaagggctatgttagataaaattgaccgtaagctgctggccttactgcagcaggattgcaccctctctttgcaggcactggctgaagccgttaatctgacaaccaccccttgctggaagcgcctgaaacggctggaggacgacggtatccttatcggcaaagtcgccctgctggatccggaaaaaataggcctcggcctgaccgcttttgtgctgataaaaacgcaacatcacagcagcgaatggtattgccgctttgtcacggtggttaccgaaatgccagaagtgctggggttctggcgcatggctggtgaatacgattatctgatgcgcgtccaggttgccgacatgaaacgctacgacgagttttataagcgtctggtaaacagcgtgccggggctgtcggacgtcacttccagcttcgcgatggaacagattaaatacaccacttctttacccatcgaataaatatccagaatcaggtcaggacacaacgcgtgcgattatttgctcaattaagctggtatttccgtcgggaatggcgtcgctatctcggggctgtcgccttgcttgtcattatcgcgatgctgcaactggttccgccaaaagtggttggtattgttgtcgatggcgtgacagaacaacactttactaccgggcagatcctgatgtggatcgccaccatggtgctgattgccgttgtggtttatctcctgcgttacgtctggcgggtattgctgtttggtgcgtcttatcaactggctgttgaactgcgtgaagattattaccgtcagctaagccggcagcatcctgagttttacctgcgtcatcgcaccggtgacctcatggctcgtgcgaccaatgacgtcgatcgcgtcgtgtttgccgccggagaaggggtgctgacgctggtggattcactggtgatgggctgcgctgtgttgattatgatgtctacgcaaattagctggcagttgaccttattttccctgttgccgatgccagtgatggcgatcatgattaagcgcaacggcgatgctttgcatgaacgctttaagctggcacaggcggcgttttccagtcttaatgaccgcacccaggaaagcctcaccagtatccgcatgatcaaagcctttggtctggaagatcgccagtcggcgttatttgccgcggatgccgaagataccggcaaaaaaaacatgcgggtggcgcgtattgatgctcgtttcgacccgaccatctatatcgcgattggtatggcgaacttgctggcgattggcggcggtagttggatggtggtgcagggcagtttaacgctgggccagctcaccagttttatgatgtatttaggtctgatgatttggccaatgctggcgctggcatggatgtttaacattgtggaacgtggtagtgctgcgtacagccgtattcgcgcgatgctggcggaagcgccggtggtgaacgatggtagcgaacccgtgccggaagggcgtggcgaactggatgtaaatattcaccagttcacgtatccgcagactgaccatcctgcgctggaaaacgtcaatttcgccctgaaacccggtcagatgctgggtatctgcgggccgactggttccggcaaaagtaccctgttgtcgctcattcagcgtcatttcgacgtcagcgagggggatattcgctttcatgatattcctctgacgaagttacaactcgatagctggcgtagccgcctggcggtagttagccagacgccattccttttttctgacactgtggcgaataacatcgcgctgggttgcccgaatgccacccagcaagagattgagcatgtcgcgcggttagccagcgtacatgacgatattttgcgtctaccgcaaggttacgatacagaggtgggcgagcgcggtgtgatgctttccggcgggcaaaaacagcgtatctccattgctcgtgcgttattagtcaacgcggaaatcctcatccttgatgatgcgctttcggcggtggacggacgcactgagcaccagatcctgcataacctgcgtcagtgggggcagggaagaacggtaatcatcagtgcccatcgcctttctgcactgacggaagccagtgaaattattgtgatgcagcacggacatatcgcccagcgtggcaatcatgatgtgctggcacaacaaagcggctggtatcgcgatatgtatcgctatcaacaactggaggcggcgctcgacgacgctccggaaaatcgcgaggaggccgtcgatgcgtagttttagccaactgtggccgactctcaagcgcctgttagcgtacggttcgccgtggcgtaaaccgctggggattgcggtcctgatgatgtgggttgcggcggcggcagaagtcagtgggccgctgcttatcagctattttatcgacaatatggtagcgaaaaataacctgccgttgaaagtggttgcagggctggctgcggcgtatgttgggctgcaactgtttgccgccgggctacattacgcgcagtcgctgctgtttaatcgggcggcagtaggcgtagtgcaacagttgcgtaccgacgtgatggatgctgcgttacgccagccattaagcgagtttgatacccaacccgtcgggcaggtgatttcccgcgtcactaatgacactgaagtgatccgcgatctctacgttaccgtagtggcaactgtcctgcgcagtgccgcgctggtgggcgcgatgctggtggcgatgttcagcctcgactggcgaatggcactggtggcgataatgattttcccggtggtgctggtggtaatggtgatataccagcgttacagcacgccgattgtccgtcgtgtgcgcgcctatttggcggatatcaacgacggctttaacgaaatcatcaatggcatgagcgttatccagcagtttcgtcagcaggcgcgatttggcgaacgtatgggggaggccagtcgttcacactatatggcgaggatgcaaaccctgcgcctcgacggttttctgctgcgtccgctgctgagtctgttttcatcgctcattctttgtggcttgttgatgctgtttggcttctccgccagcggcaccattgaagtgggcgtgctgtatgcgtttatcagctatcttgggcgacttaacgaaccattaatcgaactgaccacgcaacaggcgatgctgcaacaggctgttgttgctggtgagcgcgtgtttgaactgatggacggaccgcgccagcaatatggcaatgatgatcgcccgttacagagtggcaccatcgaagtcgataacgtgtcatttgcttatcgcgatgacaatctggtgctaaagaacattaatctctctgtgccttcgcgcaattttgtggcgctggtcgggcataccggcagtggcaaaagcaccctcgccagtttattgatgggctattacccgctaacggaaggtgagattcgccttgatggtcgtccattaagttcgctaagtcacagcgcgctgcgccagggcgtggcaatggtgcagcaagatccggtggtgctggcggataccttcctcgccaacgtgacgctggggcgggatatctccgaagaacgcgtctggcaggcgctggaaaccgtgcaactggcggagctggcgcgtagcatgagcgacggtatttacacgccgctgggcgagcaggggaataatctctcagttgggcaaaagcaactgctggcactggcgcgcgtgctggtcgagacgccgcaaatcctgatccttgatgaggcaaccgccagcattgactccggtactgaacaggcgattcaacatgctctggcggcggtgcgtgaacataccacgctggtagtgattgctcaccgcttatcgaccattgttgatgccgacaccattctggtgcttcatcgtgggcaagccgtggagcagggcactcaccagcaactgctggcggcccagggacgctactggcagatgtatcaactgcaacttgcgggcgaagagctggcagccagcgtgcgtgaagaggaatcattgagcgcctgaatagcgcaatatttcatcgttggtgcaaaaatgtaacgcactgtgcactgtcatagtgcgttttcattttcaaacttcttaacttcctgctctctttctcgtttttcatttctggcacaccgcttgcaataccttcttcgtgtagcagaaccattaccgaattctgaccggaggggatctatgaagctggtgaccgtgataatcaaaccattcaagctggaagacgttcgtgaagcgttatcttccattggtattcagggcctgaccgtcaccgaagtgaaaggtttcgggcgtcagaaagggcatgccgagctgtaccggggggcggaatacagcgtcaatttcctgccaaaagtaaaaattgatgtggcgattgctgatgaccaactcgatgaagtgatcgatatcgtcagtaaggcggcttacaccggaaaaattggcgacggcaaaatcttcgtcgctgaattgcaacgcgtcattcgtattcgtaccggcgaagccgacgaagcggcgctgtaatctctggcacacagcaacaggaacgaaaaatgaagatagcgacgataaaaactgggcttgcttcactggcgatgcttccgggactggtaatggctgcacctgcggtggccgataaagccgacaatgcgtttatgatgatttgtactgcgctggtgctgtttatgactattccggggattgccctgttttacggtgggttgattcgcggcaaaaacgtgctgtcgatgctgacgcaggtgacggtgacatttgcactggtctgtattctctgggtggtttacggttactcgctggcgtttggtgagggcaacaacttcttcggcaacattaactggttgatgctgaaaaacatcgaactgacggcggtgatgggcagcatttatcagtatatccacgtggcgtttcagggatcgtttgcctgcattaccgtcggcttgatagttggggcgctggcggaacgaatccgcttctcagctgtgttgattttcgtggtggtatggctgacgctctcttacattccgattgcgcatatggtgtggggcggtggtttgctggcttctcacggtgcgctggatttcgcgggtggcaccgtggtgcacattaacgccgcaatcgccggtctggtgggcgcgtatctgataggaaaacgcgtgggcttcggtaaagaggcgtttaaaccgcacaacctgccgatggtcttcaccgggactgccattctctatatcggttggtttggctttaacgccgggtcagcgggcacggcgaatgaaatcgcggcactggcatttgtgaatactgtggtcgcaacggcggcggcaattcttggctggatcttcggtgaatgggcgctgcgtggtaagccttcactgctgggggcgtgttctggcgcgattgccggtctggtcggcgtgacgccagcctgcggctacattggggttggcggcgcgttgattatcggcgtggtagctggtctggcgggcttgtggggcgttaccatgctcaaacgcttgctgcgggtggatgatccctgcgatgtcttcggtgtgcacggcgtttgtggcattgtcggctgtatcatgaccgggatttttgccgccagctcgctgggcggcgtgggcttcgctgaaggtgtgacgatgggccatcagttgctggtacagctggaaagcatcgccattacgatcgtctggtccggtgttgtggcatttatcggctacaaattggcggatctgacggttggtctgcgtgtaccggaagagcaggagcgagaagggctggatgtcaacagccacggcgagaatgcctataacgcgtaacaagcactgcaaaaaacagccggacggttttcacctccggctatttttttaattgtgattacgcatcaccccttcctgaacggtcgaggcaaccagtacgccgtcttgggtataaaactcaccgcgcacaaagccacgtgcgctggacgccgaggtgctctccacgctatacagcagccattcattcaaattaaacgggcgatggaaccacatggaatggtcaatggtggcaatctgaatccccggttcgagaaaaccgatgccgtgcggctgtagagctaccggcaggaagttaagatcagaagcgtaaccgagcagatactgatgaacgcgcaggtcatccggcacgctaccatttgcgcggatccacacctgacgatgtggttctgcgacgtgacctttcagtgggttatgaaactccaccggacggacttccagcggacgatcgcagatgaatttatctttcagcactggcggcagcaggtgcgccagcgattgggcgatttgcgtttccgaagggaggccatcaggcgctggcgcggacggcattgttttttgatgttcgaaacccgcttctggtgcctggaaagaggcagtcatataaaaaatcggtttgccgttttgaatagcagcaacccggcgggcgctgaagctgttaccgtcacgcagcgtttcgacatcataaataatcggcttcttactatcgccagggcgaagaaagtagctgtgaaacgaatgtaccagccgctcttcagggacggtctcttttgcagcatacaaggcctgacccacgacctggccgccaaacacctggcgtaaacctaaatcttcactctggccgcgaaagagtccttcctcaattttttccagatttaacaatgtcagtaaattttttagcgcctgactcatataactctccagtaacaaagctgccgcagcaagccaaagtgagttgagtataacgcaaatttgctactggtccgatgggtgcaatggtctgaattacgggctaattacaggcagaaatgcgtgatgtgtgccacacttgttgacgttactattttgttaaccactcttccggcgaggaaagttagcccgctggtgcattgataataaggagaaatgaatgaaactcgtgcacatggccagtggtttagcggttgcgattgcgttggcggcttgcgcagataaaagcgcggatattcagacgccagcaccggctgcaaatacgtctatttcagcaacacaacaaccagctatccagcaaccgaatgtctccggtaccgtctggatccgtcagaaagtcgcactgccgcctgatgctgtgctgaccgtgacactttctgacgcgtcgttagccgatgcaccgtcaaaagtgctggcgcagaaagcggtgcgtactgaaggtaaacagtcaccattcagctttgttctgtcatttaacccggcagatgttcagccgaacgcgcgtattctgttgagtgcggcgattaccgtgaatgacaaactggtatttatcaccgataccgttcagccggtgatcaaccagggcggaactaaagccgacctgacattggtgccggtacagcaaaccgccgtgccggttcaggccagcggtggcgcaacgactaccgtaccttcgacttcaccaactcaggtgaatccgtcttcggcagttccagctcctacgcaatattaagcgacgttaaccctctccgcccggagagggttagtagttccagcgataacgctgcaagtcgatttgcccgcttcccgataccatcacaccttctgccagtaatgcctgtcgctgacgctgtaaatccggtccggttagcgaaattgtgccgtggcgattaaccacccggtgccagggtaaggtgctgccttcagggagacgctttaacacaccgcccacctggcgcgcggcgcggggcgatcccgccagtttcgccacatcaccgtaagtggtgacatagccttcgggaatagcggcgacgatttgccagacgcgttggggaaatgaatcttctttttccatcttttcttcctgaggtaatttttcagcataatctggaaaaacgcccgagtgaagtcgcattgcgcaagaaaccagcatctggcacgcgatgggttgcaattagccggggcagcagtgataatgcgcctgcgcgttggttctcaacgctctcaatgggggctctgttggttctcccgcaacgctactctgtttaccaggtcaggtccggaaggaagcagccaaggcagatgacgcgtgtgccgggatgtagctggcagggcccccacccatttctgcctcccaccgtttcgtcaaaaaatcccaacatggctaaactttaaccacaactgacgtcgcaagaattgtctggctgcgcagtacgcttcggaggtatgtctgatgaagtatgttgatggttttgtggttgccgttcctgccgataaaaaggatgcctatcgggaaatggccgctaaggctgcgccattgtttaaagagtttggcgcgcttcgtattgtcgaatgctgggccagcgatgtaccggatggcaaagtgaccgattttcgtatggcggtgaaagcggaagagaatgaagaggttgtctttagctggattgaatacccttcaaaagaggtccgcgacgctgctaatcaaaagatgatgtcggacccacggatgaaagagttcggcgagtccatgccgtttgacggcaagcgaatgatctatggcggattcgagtcaatcatcgacgaataggtagcgtgacgggctgtgcggcgtgccgtcagcccaaaaattcacaaatgttgctcggcccagcgtaagaaatcttctttcggtaatgccttgctgtagagccagccctgaccgtagtgcacgccatgctggcgtaaccactcttcttgtttactggtttcgattccctccgctaccattttcagtttcagtgtttttgccatttcgatgatatgcggcgtgacatttttatattccagcgcatcaacgaaagatttatcgatcttcagaatgtcgacatccagatcctgtaaataacttaaacttgaataccccgtaccaaaatcatcaagataaatttcatggcccgcctcccggtagcgagaaattatcggggcgctggttttcggatcggcaaactcgcgttcagtgagttcaagcgcgatctgtctgggattaacctgatagtgattgatcatgtcacgcagcaattgcgggattttttccgaggtgagcacgggggattcaagattgatcgaaatatgctgctgtggatgctgacgcagccagtcgcccatatcttcaaagacgcttcttataatcagtagcgtcaatggctcagaaaggcccgtttgctgtgccagcggaataaaactatctggtgacaaccaactaccgtctgtctgcggccagcgcgccagtgcctcagcaccgacaattttgccattggctaaggagacaatcggctgatagtgcacgcaaatatcacgattttcgatagcatcctgcagccgatgatgcggtgactgaatacggcgcaaaatacgcagcacaaacatcgctgccagcaggccaatcaccaacccgagcggtaaccaaataaagacttgccgatgccagcctttctgcaacattttcgttgaagcccatgtgatgatcgaaatattcatctccggtaagggcaggatatcgtaaatgattccattattttcgatatgctcaccgggtgttttttgtagcctggtaataattccctgagcaatttcatcgctgctggttatgacaacgttatgggcattgccaataatggcggcatcaatttgccatgagctatagggaatgacatcaataaaggaagcggggtcgatcatgacgacataatgtgccgttcccatggcgaccatgtaacggataatgcctaaatcgttatgcgatgttaaccagacacgataaccatctttcgaaattttacctggctcggggaaggtatcgggcggactttcatgctccagagacgaacactggggaacgttgttatcgatataagccacttcctgaatatagcgataactgtaagatacccgacgcatttccatgagatgggcttcgctacaggcagcgccttgccatctttccagctcctgcagcgcatctttcccttgtgtcgccaccttattggctcgaatagcgacgcgggaggaataggtatccagctcttcaataaacgatgtttctacctgctgatgggccagccagatgcttaagccgacaggcagcaatactgaaagaatcagtactcccgaaataaggccgaccagatgtcgtgttctcaccagcatatccttattaacacagtgtagggaaagtatatctgattgtggaaaaaggctggctggagataaggaggtagagctggtatttcatgaagtgatgggtggaaacgatcattgtcatttgaccaggcgcagagctttacgcctggtatgtaaccctaacttaagatgttgattcggcgcgagcgagggtaaaaatatcgtaaaaagacagttcacctttacggacgatcattttttgcagttgttccttatgaacatccgcgacacgcggagagttcaagatggcttcaaccagcgcggcaggtacaaagcgcgtgttgtaccattcgccgttatagcaaacgcggaaatccagcacgtcgatatcttcatagcggtagcgtgggtagacatcgaaaaagaagaaaccattaagcaggataaataatacaaccagtagccagacagagcctgacagcgtttcggactgcaacatcaccgccagggtggcaaaaaaagcaacgtacataccgataaacagccccggatgtttacggataaaactgatactaaagcggggtttgttgtcgcgtttttcgcgggtattcagagactcaatcgtttcggtcagcaggcgttgtatttcggtcatcgtttgccttcgtggtatctgcaactttccagggaacaccctattttaacgtgggaatagtagaggggaagtaacagatctaccacaattttgcataacagttgcgaaaaaccgattacaattttttaattattctggctggattaccgcccacgacaacgttgtccgggacatcttttgtgacaactgcacctgaggctaccacgacgttatcaccaatggtcacaccagggttaatgaccgcgcgtccgccaatccagacgttattaccgatggtgacgggtttccccagttcagcaccgctattacgtgctacagggtcgatgggatgtgttgccgtgtagatatgaacgcctggtgccaacatacagttatcaccgatgcgaatagggcagacatcaagcatcacgcaatcgaagttggcgaaaaaattattaccgagaaaaatgttatagccatagtcacagcgaaacgttggctcaatataagcctctgtcacctgaccgaatagatcagcgagaatttgctggcgtaatgtgtgctcttccgccagggaatgattgtatcggtgaataagctgacgagcgcgcaggcgatcgcgagataacgtctcatctgccgagcgatacaactcaccagcaatcatcttttctttttctgtgctcattactgacctccggttgctgaaaatgcggcaacacagtaagacgaaaagtcagtgaagagaacgttcccattacatctgtgtgataaagatcacatagggtatgtcttcatggcgaaaaagtataaaattcttaataaacagccggttatagctccgaaagcgaattatttattagcgaataaatttccatactgaggaagggatcttgtcgtacagtttattcatggtcaattcggcgaggcggtgatctgcggctgagtaaaataccgccagttcattatctgataattcgtatttatttttctcgataacacgctccagcgtgtcaattgtctggcaacgacgtaaacgcattaaataatcggttttcgttaaaggtttttcggacatacttctacctatggttgtaataattctaacaagataaactcgcaggattctctttcgtcgcattgacaaaacaacggaatagtcgattacctgacttccgccatttctgaagatcctgcatattaataccataactactgaacaacataaaggtgtcatccagatattcgtcgatctgctcaatgagcttattgtcttcattatacttaattttgtaattaagtgcgaaggtcgcaatatgctcaatcagttcattcaactggaggttgatcgccgaggttgggtcgtttacccagccatgattgctttcttcaaggtttgcaaggcagtcatgatacagggtttcacagagaaacttaagctgtgcgatatcatgtcttttgggtgagtattcatccataacgcgtccccttcttagcggttgaactaacggacacctttcgggatggaaaaaacttactgacctggacttgccctctcgtttgttagcttaactataagccactctttgcaggttttcatcgcattattacgaaaaattacaattaggaaggaagcgggacaggactcactttttcatactagcactaacccgcagcaggtaaaagcagtttgctcgaactattcataacatttcaggattatcgccagatgaaattggtgacactaataccaggattgctctgaatatgacgtaataaccgaggaatgaataaagaattaccgcaaataattaagaatagcctctaaatgattatggattattaaatctattagcgctacttaatataaattaactaacaatcagtattttttatgaattttatccgtggttaatactggttttcgtatgagatcctgagttggtggttcaattactccttaatgttcgtaggttatgcataaaaaaggccgcttacgcggccttagtgattacacgttgtatcaatgatgatcgacagtatggctgtgctcgatatcttcattcttgcggctaaagcggcggcgaaccaccacaaagaataccggaacgaagaagattgccagtaccgttgcggtcaccatcccgcccattacaccggtacctactgcgttctgcgcgccggaaccagcaccagtactgataaccagcggcataacgccgaggataaacgccagcgaggtcatcaggatcggacgtaaacgcatccgcaccgcatcaagcgtcgcttcaatcagacctttaccttctttatccatcaagtctttggcgaattcgacgataaggatcgcgttcttcgccgacaacccaatggttgtgagcaggcctacctggaagtaaacgtcattggtcaggccacggaaggtggcagccagcaacgcaccgataacccccagcggaacgaccagcataacggagaacggaatcgaccagctctcgtacagcgccgccagacacaggaacacgacaatcaacgaaatcgcgtacagtgaaggtgcctggttgccggagagacgttcctgataggacatccccgtccagtcatagccaacaccggtaggcagtttgctcgccagttgttccatcagctccattgcttcaccggtacttttacccggtgccgcctggcctaagatttccatggatggcaggccgttgtaacgttccagacgcggcgaaccgtactcccaacgagaagaggagaacgccgagaatggcaccatctgaccatcagcagcacgaacataccagtcgccgatatcatccggcagcatacggtatttcgcttctgacatgacataaactttcttcacacgaccgcggtcgataaagtcgttcacatagctgccgccccatgcagcgcccagagtggtgttaatgtcgttgatagaaacacccagcgcctgcgctttttcctggtcgatatcaatcttaaactgcggggtatcttccagaccgtttggacgtacgctggtcaacatatcagggtgcttcgctgcttctgcaagcaactggttacgcgcctgagtcagtttttcgtgaccaaggccagcctggtcaatcagctcaaagtcaaagccggttgcagtacccagttccacgattgcgggcaggttaaaggcgaaaaccatcgcatctttgatttgcgagaaagcgcgtgttgcacgcatggtaatcgcttcaactttgttttcttcgcccggacgatcggcccagtccttcaaggaaacgaacgcaataccggtattctgaccacgtcccgcaaagccgaagccgttaacggcgaacaccgactcaacgttgttcttttctttggtcagatagtaatgcgttacctcattgagcactttctgtgtacgttcctgcgttgcacctgctggcagctgaaccatggtcataaacacgccctggtcctcatctggcaagaaggagcttggcagacgcacgaacagataggccatgccgaccacgatgatcagatacagcaccaggtaacgccccgtactgcgcagaataccgcctacgctgtcggtgtagtggtgcgtgctcttctcgaacatgcggttaaaccagccgaagaagccttttttaccttccccgtgatcgcctttggcaatcggtttcagcatggtggcacaaagagctggagtcaggatcaacgccaccagtaccgacagcgccattgctgaaacaatggtaatagagaactgacgatagatagcaccagtagaaccgccaaagaaggccatcggtacgaataccgccgacagtaccatcgcgataccgaccagagcgccctgaatctgccccatcgacttacgggtagcttcttttggcggcaaaccttcttccgccataacacgctcaacgttttctaccacaacgatggcgtcatccaccaacaggccgatggcgagcaccatcccgaacattgttagcgtgtttatcgagaagccaaaggcggcaaggacggcaaaggtcccgagcaataccaccggtacggcaatggtcggaatcaacgtcgcgcggaagttctgcaggaacagatacataaccaggaacacgaggatgatcgcttcgaccagcgttttaaccacttcgtgaatagagattttcacgaacggcgtggtgtcgtatgggtaaacaattttcagacccgacgggaagaacggttccatcttcgccagttcagcacggattgccgcagcggtatccagcgcgtttgcaccggtcgccagcttgatccccagaccggaagccggttggccgttaaactctgcgatgatgtcgtagttctcaccacccagctcaatcttcgcgacgtcacgcagcagcacgcgggaaccatcctgattcactttcagcaggattttgccgaactcttcagtagaggtcagacgcgtctgagcaataatagaggcgttaagctgttggcctttcaccggcggcgtaccaccgagctgacccgccgcaacctgggcgttctgcgctttgatggcggtaatgacatcaaccggcgttagctggaatttgttcagctcattcgggttcatccagatacgcatcgcgtactgtgaaccgaacaactgaacatcacccacgcccgacgtacggctgatggcatctttcatattcgccgccacgtagtcggagatatcctcctgcgtcatggtgccatcggtgttgataacgccgacaaccatcaggaagctgctggatgatttctcaacgctcaccccttgctgctgaacttcttgcggcagcaacggcatcgccagctgcagtttgttctgcacctgaacctgcgcgatatccgcatcagtaccagactcaaaggtcagggtgatctgcacggtacccgtggagtcactgttagaggacatgtacatcaggttatcgataccgttcatattctgttcgataacctgtgtcaccgtgtcctgcactgttttcgcatcagcgccggggtaggaggcggagatcgttactgccggcggtgcaatcgtaggatattgcgccaccggcagtttgaggatcgccagcccccctgccaacatgatgataatggcgatcacccacgcaaaaatcgggcgatcgataaagaaattaggcatgtcttaacggctcctgtttaagttaagacttggactgttcaggctgagcaccgcttgcggcttgctggttattatcagcggtaacttcttgtgcttttacctggacaccaggacgcactttctgcagcccacttattactacgcgatcgcctgctttcagaccttctgtcaccagccacttatcgccaatagcctggcttgcaacgatcggacgggtttccactttgtcatccgcgccaactaccagtacggtggcatcgccacgcggcgtacgggttacgccctgttgcgggactaaaatagcgtttggattaagcccttcttccagacgtgcgcgcacgaacatacccggcagcagagtgtgatccgggttcgggaagatagcgcgtagggtgatagacccagtggtctgatcaacggtaacgtcagagaattccagcgtaccgtcctgcgggaacttaatgccgtcactggtgatcagtgacactttggctttgccgttctcttgtttcagcgtgccattcgccagttcctgtttcaggcgcaggaagtcgttgctggactgggtcacatcaacgtagatcggatcaagttgctgcacggttgccagcgcagtcgcctgaccgttctgtaccaatgcgccttccgtcacgttcgacttaccaatgcgaccgctaatcggagaggtgactttggtgtaagccagattgatccgcgcagtttcaacggcagctttcgccgcagttaccgcagcattcgcctgttgcgcatcagccagagcctgatcgtactcttgcttactgatgtactgagtaccgagcagtttctgataacgattcaccgtcaattgcgcgatattggctgcagcctgggctttcgccagatcacctttcgcactgtcgtatgtcgcctgataggtcgcaggatcaatctgatagagagagacacctgcttcgatgtcgctaccttctttgaaattacgcttcaggataatcccgctaacttgaggacgaacttctgcgatccggtaggcactggtgcgacccggaagctcggttgtgatctgcagaggttcagttttgactgttactacgccaacggcgggcatctgctggccaccttgttgggcctgtttgtcgtcacatcctgttagggctaagctgcctgagagcatcagaacgaccgccagaggcgtaaaccctctgtttttgttcatatgtaaacctcgagtgtccgatttcaaattggtcaatggtcaaaagttaataaacccattgctgcgtttatattatcgtcgtgctatggtacatacattcacaaatgtatgtaaatctaacgcctgtaaattcacgaacatatggcacgaaaaaccaaacaagaagcgcaagaaacgcgccaacacatcctcgatgtggctctacgtcttttctcacagcagggggtatcatccacctcgctgggcgagattgcaaaagcagctggcgttacgcgcggtgcaatctactggcattttaaagacaagtcggatttgttcagtgagatctgggaactgtcagaatccaatattggtgaactagagcttgagtatcaggcaaaattccctggcgatccactctcagtattaagagagatattaattcatgttcttgaatccacggtgacagaagaacggcgtcgattattgatggagattatattccacaaatgcgaatttgtcggagaaatggctgttgtgcaacaggcacaacgtaatctctgtctggaaagttatgaccgtatagaacaaacgttaaaacattgtattgaagcgaaaatgttgcctgcggatttaatgacgcgtcgcgcagcaattattatgcgcggctatatttccggcctgatggaaaactggctctttgccccgcaatcttttgatcttaaaaaagaagcccgcgattacgttgccatcttactggagatgtatctcctgtgccccacgcttcgtaatcctgccactaacgaataaccctgaatctgactccaggatttttcctggacattttcgtcgttgctattctggttcactgcgtcgtgatattcttgcggtttgactttttcaggtcgttcttcaggttcagaaaccttcattcatcatgactatgttccagtattacaaacgatcacggcattttgttttttcagcatttattgcttttgtttttgtcttgttatgccagaacacggcgtttgcgcgggcgtcatcgaatggtgatctgccgacaaaagcggacctgcaggcgcaacttgactcactaaataaacaaaaagatctttctgctcaggacaaactggtgcagcaggatctgacagatacattagccaccctcgataaaatcgatcgcataaaagaagagacagttcagctacggcaaaaagtcgctgaagcgccggaaaaaatgcgccaggcgaccgcggcgttaacagcacttagcgatgtcgataacgacgaagaaacgcgcaaaattctgagcacgctgtcgttgcgccagctggaaactcgcgttgcccaggcgctggacgatttgcaaaacgcacaaaacgatctggcgtcttataacagccagctggtttcgttacagacgcagcccgaacgcgtgcaaaatgcgatgtataacgcttcgcagcagctgcaacaaattcgcagtcgtctggatgggactgatgtcggcgagacagccttacgtcccagccagaaagtgttaatgcaggcccagcaggcgttgctgaatgcggagattgaccagcagcgtaaaagcctggaagggaacaccgtcttgcaggataccttgcaaaagcaacgtgattacgtgacggcgaacagcgctcgtctggagcaccagttacaactgttgcaagaagcggtaaacagcaagcgcctgactttaaccgaaaaaacggcgcaggaagccgtctccccggatgaagccgcgcgtattcaggctaatccgctggtgaagcaggaactggaaattaaccagcagttaagtcagcgtctgattaccgcgactgaaaacggtaatcagttgatgcagcaaaacattaaagtcaaaaactggctggagcgggcgctgcaatcggaacgcaatattaaagagcagattgccgtcctgaagggcagcctgctgttgtctcgtatcctttaccagcaacaacaaacgctgccctcggcggatgaactggaaaacatgaccaaccgcatcgcggatttgcgtctcgaacagtttgaagttaaccagcagcgtgatgcactcttccagagcgatgcgttcgtcaacaaactggaagaaggtcacaccaacgaagtcaacagcgaagttcacgatgcgttattgcaagtggttgatatgcgtcgcgaattgctggatcaactcaacaaacagttgggtaaccagctgatgatggccattaacctgcaaatcaaccagcagcagttaatgagtgtgtcgaaaaacctgaaatccatcctgactcagcaaatcttttgggtgaacagtaaccgtccaatggactgggactggatcaaagcgttcccgcaaagcctgaaagatgaatttaagtcgatgaaaatcacggtgaactggcaaaaagcctggcccgccgtttttatcgctttcctcgctggtttgccgctgctgttgattgccgggctgatccactggcgtctgggctggctgaaagcgtatcaacaaaaactggcttccgctgtgggttccctgcgtaacgacagccagctcaacacaccaaaagcgatccttatcgacctgatccgtgcgctgccggtgtgcctgattattctcgcggttggcctgattctgttgaccatgcagctcaacatcagcgaactgctatggtcgttcagcaaaaaactggcgatattctggctggtgtttggcctgtgctggaaggtactggagaaaaacggcgttgccgtacgtcacttcggcatgccggaacagcagaccagccactggcgtcggcaaattgtccgcatcagtctcgcattgctgcctatccatttctggtctgtggtggcagaactttccccgctgcatctgatggatgatgtgctggggcaagcgatgattttcttcaacctgctgctgattgccttcctggtatggccgatgtgccgcgaaagctggcgtgataaagagtcgcacaccatgcgactggtcaccattaccgtgctgtcgataatcccgattgcgctgatggtgctgactgctacaggctacttctacactacgctgcgtctggcaggacgctggattgaaaccgtttatctggtgatcatctggaacctgctgtaccagacggtactgcgtggcttaagcgtagcggcgcggcgtatcgcctggcgtcgtgcgctggcgcgtcggcagaatctggtgaaagagggcgcagaaggtgctgaaccgccggaagaacccaccattgcactggagcaagttaaccagcagacgctgcgtattaccatgttgctgatgtttgcgctgttcggtgtcatgttctgggcaatttggtccgatttgatcaccgtgttcagctatctcgacagcatcacgctctggcattacaacggcactgaagctggcgctgcggtggtgaaaaacgtcaccatgggcagtctgttgtttgcgattatcgcctcaatggtggcctgggcgttgattcgcaacctgcctggtttactggaagtgctggtgctctcgcgactgaatatgcgccagggcgcgtcgtatgccattactaccatccttaactacatcattattgctgttggtgcgatgacggtgttcggatcgctgggcgtctcttgggataaactccagtggctggccgcagcattatccgtaggtcttggttttggtttacaagaaattttcggtaacttcgtctccggtttgatcattctattcgaacgtccggtgcgtattggcgatacggtaaccattggtagcttctcggggacggtaagtaagatccgtattcgtgcgacaacgattaccgatttcgatcgcaaagaagtgatcatcccgaacaaagcgtttgttaccgagcgtctgatcaactggtcgttgactgacactactacgcgtctggtgatccgtctcggcgtggcctatggctccgatctggaaaaagtgcgtaaagtgttactgaaggcggcgactgagcacccaagggtgatgcacgaaccaatgccggaagtcttctttacggcatttggtgccagcacgttggatcatgagctgcgtctgtatgtgcgtgaactgcgtgaccgtagtcgtactgtcgatgagctgaaccgtactatcgatcagctgtgccgtgaaaacgacatcaacattgcctttaaccagcttgaagtgcatctgcacaacgagaagggcgatgaggtgacggaagtaaaacgcgactacaaaggcgatgacccgacgccagcggtagggtaaaaacgaaagggggcaacatttagttgccccgagattgctaacaaagtgcgcgttgttcatgccggatgcggcgtgaccgccttatccggcctacgaaaccgcaagaattcaatatattgcaggagcggtgtaggcctgataagcgtagcgcatcaggcagttttgcgtttgcccgcaaccttaggggacatttagcgaccccatttatttctcacttttccgcctcatcatcgcgcgttaatttcttttcataatcacgctttacaatatccagcgcgcgcagcacggtactggcagggatctgattttcctccagcagcacaatcaaatcgacagccagtttgacatcgtcaggggcattttccagtgacatattctctccattgctagcgggttaaacgcgctaacctgttttcgattttttccagcgcatggcggcagcgtgccaggcgcgcttcataggcttccacttcacgatgcagcgtttgctgttccacgagatcggtcacccgcgccagacgggctctgcgttcggcaaccatctcacgtagccgccgctcaaaatcctgatgctgaatacgtttacgctgccagcgggcaattttcggtggtgcactgtcccactcgcgcaatgaccaggcggaggcttcacgcgcgatggcttccagttgtgccgccagatgttccgccagccaggccacttgcggcagctgttgctgctcaactgcatgacgaagcgcagccagattatcgcccgcctcgtcgagacaagcctgtagtgttgtcgcacgagtctgaaaaagatgcctgtcgaaacgagcacttagcgtggcgaactgtgacaccggggcacaacgctgacgcagcgtagcgagctgtccttccagtttttccagcagcagggcggttttcacgataagacctcaatgaaaatgataattgttatgctaaagtagccactctgtaagctgacaacactcaatatgcaacgaatcattttaatcatcattggctggctggcggtagtgctgggtacgctgggcgtggtattaccggtattaccgacgacgccgtttatcctgctggcggcctggtgctttgcccgttcttccccgcgctttcacgcctggttgctgtaccgctcatggtttggcagctatctacgtttctggcagaaacatcatgcgatgccgcgcggcgtcaaaccgcgggcgattttgcttattttgctcacgtttgccatttctctgtggttcgtccagatgccatgggtgcgcatcatgttgctggtaattctcgcctgtttgcttttctatatgtggcgaattccggtgattgatgaaaagcaagaaaagcactgaagcacaacaatcgcagttgcaattattgcgtacagccagtacattctggcgttttcgagcacaggcgcaggcggtcaaaggttaaacaactgttacttttgatacgtttaaaacgcgccgtgagtaccaccgtaacaagcaggcatacacttatgaccgcgactgcacagcagcttgagtatctcaaaaatagcatcaaaagcattcaggactacccaaaacccggcattcttttccgcgatgtcaccagcttactggaagacccgaaagcttacgctctcagcatcgacttgctggttgagcgttacaaaaatgcgggcattaccaaagttgtcggcaccgaagcgcgtggcttcttgtttggcgctccggtagctctgggtctgggcgttggctttgtaccggtccgtaaaccgggcaaactgccgcgtgaaaccatcagtgaaacttacgacctggaatacggcaccgatcagctggagatccacgttgatgccatcaaaccgggcgacaaagttctggtggtggacgacctgctggcaaccggcggcactatcgaagcgaccgttaaactgatccgtcgtctgggtggtgaagtggctgacgctgcgttcattatcaacctgttcgatctcggcggcgaacagcgtctcgaaaaacagggcattaccagctacagccttgtcccgttcccgggccattaattatcgccagtcttgtgctgcccacgctacggacagcacaagatgtgcattcagcctcgccgttctgacggggctgtgttagcattaccccttcgtgaatccaccttccagcgtttcagagcctgccaatgagttatcaggtcttagcccgaaaatggcgcccacaaacctttgctgacgtcgtcggccaggaacatgtgctgaccgcactggcgaacggcttgtcgttagggcgtattcatcatgcttatcttttttccggcacccgtggcgtcggaaaaacctctatcgcccgactgctggcgaaggggctaaactgcgaaaccggcattaccgcgacgccgtgcggcgtgtgcgataactgtcgtgaaatcgagcaggggcgctttgtcgatctgattgaaatcgacgccgcctcgcgcaccaaagttgaagatacccgcgacctgctggataacgtccagtacgctccggcgcgtggtcgtttcaaagtttatctgatcgacgaagtgcatatgctgtcgcgccacagctttaacgcactgttaaaaacccttgaagagccgccggagcacgttaagtttctgctggcgacgaccgatccacagaaattgccggtgacgattttgtcacgctgtctgcaatttcatctcaaggcgctggatgtcgagcaaattcgccatcagcttgagcacatcctcaacgaagaacatatcgctcacgagccgcgggcgctgcaattgctggcacgcgccgctgaaggcagcctgcgagatgccttaagtctgaccgaccaggcgattgccagcggtgacggccaggtttcaacccaggcggtcagtgcgatgctgggtacgcttgacgacgatcaggcgctgtcgctggttgaagcgatggtcgaggccaacggcgagcgcgtaatggcgctgattaatgaagccgctgcccgtggtatcgagtgggaagcgttgctggtggaaatgctcggcctgttgcatcgtattgcgatggtacaactttcgcctgctgcacttggcaacgacatggccgccatcgagctgcggatgcgtgaactggcgcgcaccataccgccgacggatattcagctttactatcagacgctgttgattggtcgcaaagaattaccgtatgcgccggaccgtcgcatgggcgttgagatgacgctgctgcgcgcgctggcattccatccgcgtatgccgctgcctgagccagaagtgccacgacagtcctttgcacccgtcgcgccaacggcagtaatgacgccaacccaggtgccgccgcaaccgcaatcagcgccgcagcaggcaccgactgtaccgctcccggaaaccaccagccaggtgctggcggcgcgccagcagttgcagcgcgtgcagggagcaaccaaagcaaaaaagagtgaaccggcagccgctacccgcgcgcggccggtgaataacgctgcgctggaaagactggcttcggtcaccgatcgcgttcaggcgcgtccggtgccatcggcgctggaaaaagcgccagccaaaaaagaagcgtatcgctggaaggcgaccactccggtgatgcagcaaaaagaagtggtcgccacgccgaaggcgctgaaaaaagcgctggaacatgaaaaaacgccggaactggcggcgaagctagcggcagaagccattgagcgcgacccgtgggcggcacaggtgagccaactttcgctaccaaaactggtcgaacaggtggcgttaaatgcctggaaagaggagagcgacaacgcagtatgtctgcatttgcgctcctctcagcggcatttgaacaaccgcggtgcacagcaaaaactggctgaagcgttgagcatgttaaaaggttcaacggttgaactgactatcgttgaagatgataatcccgcggtgcgtacgccgctggagtggcgtcaggcgatatacgaagaaaaacttgcgcaggcgcgcgagtccattattgcggataataatattcagaccctgcgtcggttcttcgatgcggagctggatgaagaaagtatccgccccatttgatcgtaagcacagcttacgttcgtcatccttaacgtgattgagagagaaacctatgtttggtaaaggcggtctgggtaacctgatgaagcaagcccagcagatgcaagaaaaaatgcagaaaatgcaggaagagatcgcgcagctggaagtcaccggcgaatctggcgcaggtctggtaaaagtgaccatcaacggtgcacacaactgccgtcgcgtagagatcgacccgagcctgctggaagacgacaaagagatgctggaagacctggtggctgcagcattcaacgacgcagcacgtcgtattgaagaaacgcagaaagaaaaaatggcctctgtatcctccggaatgcagctgccgcctggctttaagatgccgttctgatgcaaaccagcccgctgttaacacagcttatggaagcactgcgctgtctgccgggcgttggcccgaagtcggcgcagcgtatggcgttcacgctgcttcagcgcgatcgtagcggcgggatgcgtctggcgcaggcgctcacccgggcgatgtcggaaatcggccactgcgccgattgccgcactttcaccgaacaggaagtctgtaacatctgttcgaatccgcgtcgtcaggaaaacggtcaaatctgcgtggtggagagtccggcggacatctacgccattgagcagacggggcagttttcaggtcgttattttgtgttgatggggcatctgtcaccgctggacggcatcggtccggatgatatcgggcttgatcgtctggaacagcgtctggcagaggaaaaaatcactgaagtgatcctcgccaccaaccccacggttgaaggtgaagctaccgctaactacattgccgagctttgcgcgcaatatgacgtggaagccagccgaatcgctcatggcgttccggttggcggcgagctggaaatggtcgacggcaccacgttgtcacactcccttgccgggcgtcataagattcgtttttaagcaaacgagagcaggatcacctgctctcgcttgaaattattctcccttgtccccatctctcccacatcctgtttttaaccttaaaatggcattattgaggtagacctacatgaaaggacaagaaactcgtggttttcagtcagaagtgaaacagcttctgcacctgatgatccattctctctattccaataaagaaatcttcctgcgtgagcttatctctaacgcctccgatgcggcggacaagctgcgtttccgtgcgctctctaacccggacctgtacgaaggtgatggcgaactacgcgttcgtgtctctttcgataaagacaagcgtacgctgaccatctccgataacggcgtggggatgacccgcgacgaagtgattgaccatctggggactatcgctaaatccggtaccaaatcattcctcgaatccctgggttctgaccaggcgaaagacagccagctgatcggtcagtttggtgttggtttctactctgcgtttatcgtggccgacaaagtgaccgtgcgtactcgcgcggcaggcgaaaaaccagaaaatggcgtcttctgggaatcggctggcgaaggtgaatacaccgttgccgacatcaccaaagaagatcgtggtactgaaatcaccctgcatctgcgtgaaggcgaagacgagttcctcgatgactggcgcgtgcgttccatcatcagcaaatactccgaccatatcgcgctgccggtagagatcgaaaaacgcgaagagaaagacggcgaaaccgttatctcctgggagaaaatcaacaaagcgcaggcgctgtggactcgtaacaagtcggaaatcaccgatgaagagtacaaagagttctacaaacacatcgcccacgactttaatgatccgctgacctggagccacaaccgtgttgaaggtaagcaggagtacaccagcctgctgtacatcccgtcccaggctccgtgggatatgtggaaccgcgatcataaacacggcctgaaactgtatgttcagcgtgtgttcatcatggacgacgcagaacagttcatgccgaactatctgcgcttcgtgcgtggtctgattgactccagcgatctgccgctgaacgtttcccgtgaaatcctccaggacagcacggtaacgcgtaacctgcgcaatgcgctgaccaagcgtgtgctgcaaatgctggaaaaactggcgaaagacgacgcggaaaaataccagaccttctggcaacagtttggcctggtactgaaagaaggtccggcggaagatttcgctaaccaggaagcgatcgccaaactgctgcgttttgcttctacccataccgattcttctgcgcagaccgtatctctggaagactacgtttcccgcatgaaagaagggcaggagaaaatctactacatcaccgcagacagctatgcggcagcgaagagcagcccgcacctggaactgctgcgtaagaaaggcatcgaagttctgctgctttccgaccgcatcgatgagtggatgatgaactatctgactgagttcgacggtaaaccgttccagtcggtgtctaaagttgacgagtcgcttgaaaaactggctgacgaagttgatgagagcgcgaaagaagcggagaaagcactgactccgttcatcgaccgtgtgaaagccctgctcggcgagcgcgtgaaagatgtccgtctgactcaccgtctgaccgatacgccagcgatcgtttcgaccgacgcggacgaaatgagcactcagatggcgaaactgttcgctgcggcgggccagaaagtgccagaagtgaaatacatcttcgaactgaacccggatcacgtactggtgaaacgtgcggcagatactgaagatgaagcgaagttcagcgagtgggtagaactgctgctggatcaggcgctgctggcagaacgcggcacgctggaagatccgaacctgtttattcgtcgtatgaaccagctgctggtttcctgatgtaatgccggatgaccttcgtgtcatccggcatttttcttttcatcatctgcactttccgcaaattatctcgccattaaccgtttcagccccaggtgcctttcttgaggcaatcgcctgttggtggtatcgtttatcgctttttcaaaaaattcgacacattttaaggggattttcgcaatgcgtatcattctgcttggcgctccgggcgcggggaaagggactcaggctcagttcatcatggagaaatatggtattccgcaaatctccactggcgatatgctgcgtgctgcggtcaaatctggctccgagctgggtaaacaagcaaaagacattatggatgctggcaaactggtcaccgacgaactggtgatcgcgctggttaaagagcgcattgctcaggaagactgccgtaatggtttcctgttggacggcttcccgcgtaccattccgcaggcagacgcgatgaaagaagcgggcatcaatgttgattacgttctggaattcgacgtaccggacgaactgatcgttgaccgtatcgtcggtcgccgcgttcatgcgccgtctggtcgtgtttatcacgttaaattcaatccgccgaaagtagaaggcaaagacgacgttaccggtgaagaactgactacccgtaaagatgatcaggaagagaccgtacgtaaacgtctggttgaataccatcagatgacagcaccgctgatcggctactactccaaagaagcagaagcgggtaataccaaatacgcgaaagttgacggcaccaagccggttgctgaagttcgcgctgatctggaaaaaatcctcggctaattcgaaagcgcgcacggacagtcccctcgccccctcggggagagggttagggtgaggggaacaggcccgcacaagcaaacttatcagcaatctcaggccggatattcattcggccttttacaaaaacctcaatctgcgctattcctttttctgatttgacctctcacagcaattagttcttcttcctcacttttccgctacaattatcaacaagttgaatcgataagaggcggtaatgcgtcagactaaaaccggtatcctgctggcaaacctgggtacgcccgatgcccccacacctgaagcggtaaaacgctatctgaaacaatttttaagcgacagacgcgtggttgatacctcacggttgttatggtggccattgctgcgcggcgtgattttgccgctgcgctcgccgcgtgtggcgaagctgtatgcctctgtctggatggaaggtggctcgccgctgatggtttacagccgccagcaacagcaggcgctggcacaacgtttaccggagatgcccgtagcgctgggaatgagctacggctcgccatcactggaaagcgccgtagatgaactcctggcagagcatgtagatcatattgtggtgctgccgctttatccgcaattctcctgttctacggtcggtgcggtatgggatgaactggcacgcattctggcgcgcaaacgtagcattccggggatatcgtttatacgtgattacgccgataaccacgattacattaatgcactggcgaacagcgtacgcgcttcttttgccaaacatggcgaaccggatctgctactgctctcttatcatggcattccccagcgttatgcagatgaaggcgatgattacccgcaacgttgccgcacaacgactcgtgaactggcttccgcattggggatggcaccggaaaaagtgatgatgacctttcagtcgcgctttggtcgggaaccctggctgatgccttataccgacgaaacgctgaaaatgctcggagaaaaaggcgtaggtcatattcaggtgatgtgcccgggctttgctgcggattgtctggagacgctggaagagattgccgagcaaaaccgtgaggtcttcctcggtgccggcgggaaaaaatatgaatatattccggcgcttaatgccacgccggaacatatcgaaatgatggctaatcttgttgccgcgtatcgctaaagctgagcggtaaagaactgagcgccgtcgcgaagagcctcgtcggcggttttcatcatccgtgaataatgcaaaaaggcgtgcagcgtgcctgggtagagtttgaactcacagggctgctgatgcgccgctaacgtctggtaaagcagacggctgtcatccagcagcggatcgaactccgccccggcaataaaacagggcggaacttcgcgagtgagatcattattaaacagacagtaatacggcgactcgcggtccgcgtcgttgcttaaatatgcctcttcgtacatctgcaaatcctgttgcgttaagccatcccagacaccgcccaacagacgacgagtcacggaatcccgtaatccgtaaagcccataccacagcaaaacgcccgcaactttaccgcaatcgatctgtttatcacgcaaccacaacgcactggcgagcgccagcatggcacctgcggaatcaccggcaaagccaatgcgggacatattgatttgataatcctccgcctgctggtggaaataacaacaagcagccacaatttcctctatcgcttgcggaaaacgcgcttcaggtgaaagggtgtaatcaataccaatcaccgtacattggctgtagcttgccagcaggcgcatgatgcgatcgtgggtatcgagattgccgagaataaaaccgcctccatgcaaataaaatagcgtcgctgggctatctggctgcggacaaaagagacgtgtttccacctgcccatattttgttggaaccatgtaagctctggttgccatttctggagcgcccgcattccagaatcggcgctcaagcgtgtaatactgtcgttgctcagcaatcgttcccgttgcgggccagggcggtaaatccggctgaagagtattcacaacggtcttcatttcagcagaaataaggtccagaacaggtagtttgttttccggcttcatacaaaaactcctttcaaattacgtcattgtaaggaaccactgccatgaaaatgcgatcccgcctgctgatattgaaactggctgcgtctcgcgcgctcccgtcagattgtgttaacattcgccgctcagttaaccacccgtaaaaacaaccatgaaatttcccggtaaacgtaaatccaaacattacttccccgtaaacgcacgcgatccgctgcttcagcaattccagccagaaaacgaaaccagcgctgcctgggtagtgggtatcgatcaaacgctggtcgatattgaagcgaaagtggatgatgaatttattgagcgttatggattaagcgccgggcattcactggtgattgaggatgatgtagccgaagcgctttatcaggaactaaaacagaaaaacctgattacccatcagtttgcgggtggcaccattggtaacaccatgcacaactactcggtgctcgcggacgaccgttcggtgctgctgggcgtcatgtgcagcaatattgaaattggcagttatgcctatcgttacctgtgtaacacttccagccgtaccgatcttaactatctacaaggcgtggatggcccgattggtcgttgctttacgctgattggcgagtccggggaacgtacctttgctatcagtccaggccacatgaaccagctgcgggctgaaagcattccggaagatgtgattgccggagcctcggcactggttctcacctcatatctggtgcgttgcaagccgggtgaacccatgccggaagcaaccatgaaagccattgagtacgcgaagaaatataacgtaccggtggtgctgacgctgggcaccaagtttgtcattgccgagaatccgcagtggtggcagcaattcctcaaagatcacgtctctatccttgcgatgaacgaagatgaagccgaagcgttgaccggagaaagcgatccgttgttggcatctgacaaggcgctggactgggtagatctggtgctgtgcaccgccgggccaatcggcttgtatatggcgggctttaccgaagacgaagcgaaacgtaaaacccagcatccgctgctgccgggcgctatagcggaattcaaccagtatgagtttagccgcgccatgcgccacaaggattgccagaatccgctgcgtgtatattcgcacattgcgccgtacatgggcgggccggaaaaaatcatgaacactaatggagcgggggatggcgcattggcagcgttgctgcatgacattaccgccaacagctaccatcgtagcaacgtaccaaactccagcaaacataaattcacctggttaacttattcatcgttagcgcaggtgtgtaaatatgctaaccgtgtgagctatcaggtactgaaccagcattcacctcgtttaacgcgcggcttgccggagcgtgaagacagcctggaagagtcttactgggatcgttaagttatcgtcggttcgtaggccagataaggcgttcacgccgcatctggcatttggctctcgatgcctgatgcgacgctggcgcgtcttatcatgcctacatatttttcatattttacatccggcaaccaccgtttaccccgtcaccacctcacccgccggtggcgtttccagcagttccagcatggtacgggcgatttcacgctcgcccatcactacctgattcgcaccacgttcggtgatatacgccacttcatcgtcataatgggcgcgggcaataatctcaatatccggatttttcgcgcgggcagatgccacaatctcacccgcttcataaccgttgggaatcgtcaggatcagccattttgcacattccagatgcgccagttgcataatttcttcgttcgccgcattgcccaatactgcgcggaccccgcgctctcgcagctcatcaacacgggttcgtgacgtctcaatcaccaccagcggaatatcagaggcgagcaatttctcccccagcaggctgcctacacgaccgtaacccaccagtagcgcatggttgcaaatatccactgggatctgcttctcttcttcgattgcctcttccagcgtctgctcttccagcgtttcggtcttcgccagatatttctccagtagtgcgaacagtaccgggttgagcataatcgacaggatcgcccctgccagtaccaggttttgtccggcctgcggcagtaaattcaatgccattcccagtcccgccaggataaacgcgaactcaccaatctgcgccaggctggcggcgatggttaatgccgtacgttgggagtgaccaaacagtcgcaccaggaaaaatgcggctaacgacttaccaaacagaataatcgccagcgtcgccagcactgccagcggttgctgaatcagaattaacggatcaaacaacatcccgacggagacaaaaaacagcaccgcaaacgcgtcgcgcaatggcagcgtatcgtgggcggcacggtgactcagttcagactcgttcagtaccatcccggcaaagaacgcaccgagtgcaaaggagacatcaaacagctctaccgcaccaaaggcaacccctaacgccagcgccagcaccgacagggtaaacagctcgcgagaaccggttgccgcgctgcgtgccataatccacggcaccagacggcgacctaccagcatcataatggcgataaatgcgatcactttgccgatggtgatccccatatcgactgcaagagtggcaaagcccacatcgccctgttccatcattcctgccactgcgggcagcaacaccagcgtcagaaccattaccaggtcttccacaatcaaccaaccgatggcgatttgcccacgctgactgtcaattaattgccgttcttcaagtgcgcgcagtaacaccacggtactggcggtggaaagacataaaccgaacacgataccggtcattaacgaccagcccagcacggcagagagcgccatacccagcagcgtcgccacggctatctgggcgatcgcaccgggaatggcgatggcctttaccgccatcaaatccttcagcgaaaagtgcaaaccgacgccaaacatcaacagaatgacgcccagttcagccagttccggggcaagcttggtatcggcaacaaagcccggagtgaatggtcctgccagcacacccgctaacagatatcccaccagaggagaaatacgtagtttattggccagcatgccgaggataaaggcgagcacaaggccgccaacaatggtggtgataagcggggtggcgtgatgcattccgtctccttttcctggtggttattgtccatttttggccgggaaaaccaaaattacaggtaatagtttatgacaatttcattgatgatgttcatgaataattattgaattttgcagaaaaatggaattagctgcaaaaaaagcacggatcggaaaacagaaggcggtttaacagaggaaaggcttatggcgactgtaaaacgatgcagccaaagtttgcctttggctgcaatgaaatcagtctttatgccggttatcaggcaggaatatggtcaacatccccaatagtggcaggaaagcacagattttatagactaactcgatgctggtgtgatcggcgataagccccagaactgccgctcccagacctcccatgccaaaagcaaaaccgaaaaagagtccagaaaccataccgatacgtcctggaagcagctcctgagcgtagaccagaatggcagagaatgccgaagcgaggataaatccaataatcaccgttaaaacccccgtccagtgcaggctggcgtagggtaaaatcagcgtaaacggcgcaacgccgaggatagagccccaaatcacatatttccgcccaattttatcccctacaggcccgccgatcaccgtacctgccgcaacggcaaacaggaaggcaaacagatgaagctgagcattctggatagataatccgaatttttgcatcagataaaaggtgtaatagctgctgatgctcgccatatagaaatatttcgagaaaatgaggattaacagaatgctgaccgccagtacaactttattgcgcggcagtggattgataatcgtcgctttgggttttcctttattcattcggtgctgtgccgagtaccaacggctgatttgcgccaacaccacgatcgccagcagtgccgcaagcacaaaccaggcaacgttgcctttgccataaggcgcgataatcaccgccgccagcaagggtcccagggaactgccaaagttgccgccgacctgaaagatagattgcgccaggccatgccgcccgccggaagccatacgggccacgcgagaagattccggatgaaagaccgatgaaccggtaccgaccagcgccgccgccagcagaactgcgccaaaactgcccgccagcgcaagcagcaccagaccgcttaaggtaaagcacatgccaattggcaacgaccatggcatcggatatttatcggtccagtagccgaccactggttgcagtagcgaagaggcgagctggaaggtgagggttatcatgccaatctgcataaatgtcagagaaaattctgactgaagcagcggataaatcgccagaatcagcgattggatcatgtcgttcagcagatgtgagaggctgatagcacctaaaataccaaacgatgttcgggccttggtcgttgacgcagccgcgcccgccacaggctggggttgttcactcattgccataggaaagtcactttttcagggttgcgatgtaaagaatgatcttatttgtgattattaccagactaacatacctgtatgcgtcgtctgaaggaagtctcaacgccgaatacagaatttctaatctggatgcagatttatcttcaccggacgcagacttgtctatgatgtcgcgtcatactatttttcaacacgttgaaatcaggtcagggagagaagtatgaaattattgcagcggggcgtggcgttagcgctgttaaccacatttacactggcgagtgaaactgctctggcgtatgagcaggataaaacctacaaaattacagttctgcataccaatgatcatcatgggcatttttggcgcaatgaatatggcgaatatggtctggcggcgcaaaaaacgctggtggatggtatccgcaaagaggttgcggctgaaggcggtagcgtgctgctactttccggtggcgacattaacactggcgtgcccgagtctgacttacaggatgccgaacctgattttcgcggtatgaatctggtgggctatgacgcgatggcgatcggtaatcatgaatttgataatccgctcaccgtattacgccagcaggaaaagtgggccaagttcccgttgctttccgcgaatatctaccagaaaagtactggcgagcgcctgtttaaaccgtgggcgctgtttaagcgtcaggatctgaaaattgccgttattgggctgacaaccgatgacacagcaaaaattggtaacccggaatacttcactgatatcgaatttcgtaagcccgccgatgaagcgaagctggtgattcaggagctgcaacagacagaaaagccagacattattatcgcggcgacccatatggggcattacgataatggtgagcacggctctaacgcaccgggcgatgtggagatggcacgcgcgctgcctgccggatcgctggcgatgatcgtcggtggtcactcgcaagatccggtctgcatggcggcagaaaacaaaaaacaggtcgattacgtgccgggtacgccatgcaaaccagatcaacaaaacggcatctggattgtgcaggcgcatgagtggggcaaatacgtgggacgggctgattttgagtttcgtaatggcgaaatgaaaatggttaactaccagctgattccggtgaacctgaagaagaaagtgacctgggaagacgggaaaagcgagcgcgtgctttacactcctgaaatcgctgaaaaccagcaaatgatctcgctgttatcaccgttccagaacaaaggcaaagcgcagctggaagtgaaaataggcgaaaccaatggtcgtctggaaggcgatcgtgacaaagtgcgttttgtacagaccaatatggggcggttgattctggcagcccaaatggatcgcactggtgccgactttgcggtgatgagcggaggcggaattcgtgattctatcgaagcaggcgatatcagctataaaaacgtgctgaaagtgcagccattcggcaatgtggtggtgtatgccgacatgaccggtaaagaggtgattgattacctgaccgccgtcgcgcagatgaagccagattcaggtgcctacccgcaatttgccaacgttagctttgtggcgaaagacggcaaactgaacgaccttaaaatcaaaggcgaaccggtcgatccggcgaaaacttaccgtatggcgacattaaacttcaatgccaccggcggtgatggatatccgcgccttgataacaaaccgggctatgtgaataccggctttattgatgccgaagtgctgaaagcgtatatccagaaaagctcgccgctggatgtgagtgtttatgaaccgaaaggtgaggtgagctggcagtaatccgaaagtgccggatgtttgcatccggcacaatgcttaatcgcggcgggcgatatcagcaaatttggcatcgaggatctttgccagatcgcctgccgccagttcgatatccagtccgcgcttgccgccggaaacataaatagtggcaaattcttgtgcgggggcgtcgataatcgttggcagacgttttttctgccccagtgggctaatccccccaaccaggtatcccgtcgaacgctgcgcgaccatcggatcggccatctcaactttcttggcacccagcgcttttgctacttttttaagatccagttgacctgcgaccggcgtaacggccacggcaaggtgtttcatatcaccgttcactgccaccagcagcgttttgtagacctgatccggattcaaacctaattttttgacgacttcatcgccaaaattggtttcagccggatcgtgctcgtaggtatggatttgaaacgaaatcttgtttttttcgagtaatttaactgcgggtgtcatggtaattttcctgccttaaacaaaaaaacgaagcaagcatacgcctgatggcggtccaaaaaaaagagtcatcttgcctaagagtattggcaggatggtgagattgagcgacaatcgagttacaccgtcgcttaaagtgacggcataataataaaaaaatgaaattcctctttgacgggccaatagcgatattggccatttttttagcgcaacatttgcggcaaattcccttctccatacaggtgtagtgcaccgaccgcgaccacatatcgccccggcggcatggcgcgtaatttatcccgccaggcgagatttcgctgatgcatcagcacatcgtacagcgactgactgaacgtattgggcagcgttatatcattattttgcggcggtgcattcagccaccagctcatcatttgttgcagcaaccgtgcgttggtatgccagtgggtcagcgtatcgtccagcagcgccagtcctttgtcagggagctggagcaacatggcaatctggttttcagccccttccagttcaatcacgggtttatgttgttgcttcgccgcctgcaatagctggtaatcgataccgtattctgcccgcagccccagtttttgtgcctgcgtcgcctgaagaaccatcgcgatttgccacagcggttgggtagaaaagagtgagggagaaatgcccatctcctggctaatgtgctgcaggttttggagttgctcctcgctaatgcgctcttccagcgcctcgcaggcaggcaaattagcaaaaggcgtatcgctggtggaaacatccgcctcgacgatcagcgcatcggcgtttttgagctttttgagcaaacgggtgggcaggggagccatatcgtggctacccatatgaatactgccaatcagatgaaaatggcgattgccggggagggtgatatcgatggcaggccaggtgtaatgattaccgcgcagcgcggcccaaagcgtttttacccggtacaacagatccatacgacctccctttgtgaaatatcatgctagcgcgcggtgagggatggcgcaaatggagttggagacttgtttaatgtgtttgtatgattcagtatgttcttgcatcgctattcacaaggaagcaacagttaaaaaccatgaaacaggcaacaagaaaaccgacgacacccggagatattcttctctatgaatatctggaaccgctcgatttgaaaatcaatgagttagcagagttgctgcatgttcatcgtaatagcgtcagtgcactgatcaataacaatcgtaaactcactactgagatggcatttcgtctggcgaaagtttttgataccacagtcgatttttggctaaacctccaggcggcggttgatctttgggaagttgaaaacaacatgcgcacccaggaagaattgggacggattgaaacagtggctgaatatttggcacgccgtgaagagcgtgcaaaaaaggtcgcgtaaggccaaaacatcgcttcatctcgtaggccggataaggcgttcacgccgcatccggcatccgagcaccattgcctgatgcgacgcttacccgtcttatcaggcctacaaacttgtgcctgaaccgtaggccggataaggcgtttacgccgcatccggcatccgagcaccattgcctgatgcgacgcttacgcgtcttatcaggcctacaaacctgtgcctgaaccgtaggccggataaggcgtttacgccgcatccggcagtcatgcgtcgatgccaaatgcgccaccctaaagcagcgcatccgcaatgatgtacttattccttcggtttaaaccgcagcaaccggttggcgttactcactacggtaatcgacgagagcgccattgccgctccggcaactaccgggttaagcagtgttccagtgaacggccacaaaataccggcggcgaccggaataccgatactgttgtagataaacgcaccgagcaggttctgcttcatgttgtgcagcgttgcgcgggaaatagcgagcgcatccgcaacgcccatcaggctatggcgcatcagggtaatcgccgcggtttcaatggcaacatcactgccgccacccatcgcaatgccgacatccgcctgagccagcgctggcgcgtcgttaatgccgtcgcccaccattgccacctgacgtccttcactttgcagatgtttgatcgcttcggctttaccgtccggcagcaccccggcgatcacctcatcaatccctgcttctttggcgatcgcattggcggtggttgggttatccccggtcaacatcaccagacgatatcccgctttatgcaggcgttgcagcgccgccacgctatcactacgcaacggatcgcgtactgccagcagggctaccgctttcccgtcaaccgccagcagcacaggcgttgccccttgcgatgcctgagcagtaatctccgcttcgatagctttggtaccaacctgttgctcatttaacagcgcctgattgcccagcaataacgcatgaccttcagcttcaccgctcacgcccagcccgcgcaatgtgcggaaaccgttgacctgcggtagctgcatatcacctgctttatcgaggatcgctcgtgccagcggatggctggaaccttgctccagtgccgccgccagacgcaatgcctgcgcttcatcaacatcagcaaatgttttcactgcgacaacctgcggcttcccttcagtcagcgtcccggttttatcgaacactacagtgtcgagtgtactggcgcgttgcagcgcgtcagcgtcccgcaccagcacgccaaactcagccgcccgcccgacgccggaaataatcgacatcggcgtcgccagccccagcgcacacggacaggcaataatcagtaccgtggtggcaatcaccagggtatagacaatctgcggtgccggaccaaagaaataccagattgccgcactgacaagcgcaataaccaccactaccggcacaaatacggctgagattttatccgccagctgaccgatttctggcttgctgctctgggcctggcgcaccatgcgaatgattcgtgacagcgtagtatggctgccaaccgcactggcacgaaacagcacactgccgtcctgtaccactgtcccggcatggacgctatcgccttcgcctttttgctgcgggattggttcgcccgtcagcatcgcttcatccagccatgcttcgccctgggtaatctcgccatctaccggcacgcgatcgccggtcgtcaggcgcagcaacatacctggctgcacttctgccagaggcacgcttttttcaccttcgtcagtaaccaggcgtgccgtcggcggggttaaatcgagtaacttttccagcgccttagaagaacgctggcgtgcgcgcgcttccagcatatggccgagattgatcagaccgataatcatcgcgctggcttcgtaataaagatgtcgcgcttccatcgggaaccactgcggccacaggttgacgctcatcgaatagagccacgccacgccagtacccagcgccaccagcgtatccatcgtcgccgcaccgttcagcaggcttttccatgcactgcggtaaaaatggccgccggcgaaaaccatcactgccagggttatcaggccgataaccaaccacaggctgcggttgtcagcggtgaccatcatgttatcgccgatcatcccccagaccatcaccgggatacccaccgccagtgcgacaattgcctgccagcggaagcgcttcatcgtagcgacggcggtttcttgctggcgctcgcggcgtttagcgtcatcttcaatcgcttccgcgccgtagcccgctttttccaccgcctgcactaaatcttgtggggaggcactgcccatcaccagcgcagtacgctccgccaggtttacccgtgcctgagtgacgcccggtacgctttgcagcgcattttgtacgcgggtgacacagctggcgcagctcatgccgctcagcagcaactgctggctgtcatcgtcatcggcggtcgctgccggaagcgcctcagaaaccgctgtcagtgcttccgacgggattgatgactccgccagcggtttagcctttgggtggcttacagatgcgtcataacccgcttgtttgatggtttcgatcagctgttctgcactggcagtcccggtaacgtgcgcttcagtgatagacacatccgcctgctcaacatccggacgctgttcaagactttctttcacgcgtttaacgcagtgaccgcaggacaggccgtccagggtcaggtcgatagtttgtgacataaaacactcctttaagacagttttgactggctgtgataaaggttaaaccttccagcaaggggaaggtcaagaaattaataaaccaggcgggtaaaagtccgtaaagattaaaaaatcggctcgatttgcatcaggattagacatttatctctttgttttcctgtagttaagttgcgggtgctaagttaaatcaggatgcctgaaaatcggcaccggggtgaggaattacctcccgcatctataaaaaggagttaacaaaagatgttagatgcaaacaaattacagcaggcagtggatcaggcttacacccaatttcactcacttaacggcggacaaaatgccgattacattccctttctggcgaatgtaccaggtcaactggcggcagtggctatcgtgacctgcgatggcaacgtctatagtgcgggtgacagtgattaccgctttgcactggaatccatctcgaaagtctgtacgttagcccttgcgttagaagatgtcggcccgcaggcggtacaggacaaaattggcgctgacccgaccggattgccctttaactcagttatcgccttagagttgcatggcggcaaaccgctttcgccactggtaaatgctggcgctattgccaccaccagcctgattaacgctgaaaatgttgaacaacgctggcagcgaattttacatatccaacagcaactggctggcgagcaggtagcgctctctgacgaagtcaaccagtcggaacaaacaaccaacttccataaccgggccatagcctggctgctgtactccgccggatatctctattgtgatgcaatggaagcctgtgacgtgtatacccgtcagtgctccacgctcctcaatactattgaactggcaacgcttggcgcgacgctggcggcaggtggtgtgaatccgttgacgcataaacgcgttcttcaggccgacaacgtgccgtacattctggccgaaatgatgatggaagggctgtatggtcgctccggtgactgggcgtatcgtgttggtttaccgggcaaaagcggtgtaggtggcggtattctggcggtcgtccctggagtgatgggaattgccgcgttctcaccaccgctggacgaagatggcaacagtgttcgcggtcaaaaaatggtggcatcggtcgctaagcaactcggctataacgtgtttaagggctgatcatgatgaacacggaaggtaataacggtaacaaacctctcggtctatggaacgtcgtttccatcggcattggggcaatggtgggggcggggatcttcgcgctgctggggcaggctgcattgctaatggaagcctcgacctgggtcgcctttgcttttggcggtattgtggcgatgttttccggttatgcctatgcgcgtctgggggcgagctatcccagcaatggcggcattatcgacttctttcgtcgcggattaggcaacggcgtcttttcgctggcgctctcgttactgtacctgttgacgctggcggtgagcatcgccatggtcgcccgtgcttttggcgcttatgccgtgcagtttttgcatgaaggcagccaggaggagcaccttattttgctctacgcgttggggatcattgcggtgatgacgcttttcaactccttaagcaaccatgcggtagggcggctggaagtgatcctcgtcggcattaaaatgatgatcctgttattgctgattattgccggtgtctggtcgctgcaaccggcgcatatttccgtctctgcgccccccagctccggtgcgttcttctcctgtattgggataactttccttgcctatgcgggctttggcatgatggcgaacgcggcggataaagtgaaagatccgcaggtcattatgccacgggcgtttctggtggcgattggcgttaccacgttgctttatatctcgctggcactggttttgcttagcgatgtatcggcattagagttagaaaaatatgccgataccgccgtagcgcaggctgcttctccgctgctcgggcatgtgggttatgtgatcgtcgtcatcggcgctttactggcgacggcttcagccattaacgcgaacctgttcgccgtgtttaacatcatggacaacatgggcagcgaacgcgaactgccgaagctaatgaataaatccctgtggcggcagagtacctggggcaacattattgtcgtggtgttgattatgctgatgacggcggcactgaatttaggctcactcgccagcgttgccagcgccacctttttgatttgctacctggcggtgtttgtggtggcgatccgcctgcgtcatgatattcacgcctcgttgccgattcttatcgttggtacgttggtgatgttgttggtgatcgttggctttatctacagtctgtggtcccagggtagccgtgcgttgatatggattattggctcactcttactcagccttattgtggcaatggtcatgaagcgcaataaaaccgtataacatctctctgtgcgcagtacttcctgtattattgtggtggcggtcgatattcgcactggcaaaaaaacgtgcttgaatatctgttgaaaccctttaacaaagcacaggaggcgttgcgcgaacgatgaacatcagcgatgtagcaaaaattaccggcctgaccagcaaagccattcgcttctatgaagagaaggggctggtgacgccgccgatgcgcagcgaaaacggttatcgcacctacacgcagcagcatctcaacgaactgaccttactgcgccaggcacggcaggtgggctttaacctggaagagagcggcgagctggtgaatctgtttaacgacccgcagcggcacagcgccgacgtcaaacggcgcacgctggagaaggtggcggagatcgaacgacacattgaggagctgcaatccatgcgcgaccagctgctggcactggcgaatgcctgccctggcgatgacagcgccgactgcccgattatcgaaaatctctccggctgctgtcatcatcgggcagggtgattaagacgagacggctcggatatgtagggttatcccttctatcgcaatgacttcaacatgcgtacctgcaccgagatcctcgctggcgctgacaggccatgaactgtcaccgacgcgcatatgaccgcgcccgttgaccagcggagattccagcacaaaacgtcggccaatcagctgctgcccgcgctggtttaaatgactatcgctgtgcttttgttcgcgcacccgccgcgacaaccatttccaccacagccaggcggcgagcagcgtcaggatggcaaacattaccccttgccactcccaacccagcggcaccagccagaccaccaggccggtaatcaccgctgccacgccgctccacaacaaataaccatttccgcccagcatctcggctgccagcagcaaaccgccgagactgagccagaaaatatgtggatgaacgaccattaactccatcatggctgagtccgtttgttggcgctgtctttcaccagctcggcaatcccggcaatcgaccccatcaggctgctggcctctaatggcatcatcactactttgctgttactggaggaaccgatctgctgtaacgcttcggtgtatttctgcgctacgaagtagttcaccgcctgaatatcaccggaggcgatagcttcagacaccattttggtggcgcgggcttctgcttcggcggaacgttcacgcgcttcagcctgtaaaaacgccgactgacgttcgccttccgctttcaggatttgcgactgtttttcaccttcggctttgaggatttccgcctgacggatcccttccgcttcaagaatgtaagcgcgtttggtacgttccgctttcatctgcgcgttcattgaagagataagctctgccggtgggcgcacgtcgcgaatttcaatacgggtgactttaatcccccacgggttggtggcttcatcgacaatacgcagcaggcgtgagttgatgctgtcgcgctgagagagcatttcgtcaagttccattgaacccagcacggtacggatgttagtcatggtcaggttgatgatcgccagctccagattgctgacttcataagccgcgcgcggcgcgtcaatcacctgaataaagcacacggcgtcgatggtaacgttggcgttatctttcgagataacttcctgggaagggatatcgagcacttgctccatcatattgatcttgcgaccaatgcgatccataaacggcaccaccagactgagccccggctgtaacgttttggtatagcgaccaaagcgttctactgtccactgatagccctgcggtacgattttgacacccgcgccgacaatgaccagcgcgacaaaaatgagaatcgggataaagataagcatcggaaaaacctcctgttgtaccgtccataatcagcaaaattgctgcttgattaaacaaattatacctgattactgaaagagagttcccccttattcctgcgaaggataaactgtttttagtaaaaatcagaaaaagggaacagcgatgcaggaaaatagtcctttgcttcagctacaaaacgtaggatatctggcgggtgatgcgaagattcttaataacatcaatttttcgctgcgtgctggcgaatttaagttaattaccggtccttctggttgtggcaaaagtacgctgctaaaaatagttgcttcattgatcagcccaaccagcggaacgttactgtttgaaggtgaggatgtcagcacactaaagccagaaatctaccgccaacaagtctcttactgcgcccagacaccgacgctgtttggcgatacggtatacgataatctgatctttccctggcagatccgtaaccggcagcctgacccagccatttttctcgattttctcgaacgcttcgccttgccggacagcattttgacgaagaatatcgccgagctatctggtggtgaaaaacaacgcatctcattgattcgtaacctgcaatttatgccgaaggttttattgctggatgaaataaccagtgcgctggatgaaagtaataaacataacgtcaatgagatgatccatcgttatgtgcgcgagcaaaatattgccgtgctgtgggtgacacacgataaagacgaaattaatcatgcggataaagtgattacactgcaaccgcatgccggagaaatgcaggaagcacgctatgaactcgcataatattactaacgaatcattagcactggcattaatgctggtggtggtggcaatcttaattagccataaagaaaaactggcgctggagaaagatattctctggagcgtcgggcgagcgataattcagctgattattgtcggctatgtgctgaagtatattttcagcgtggatgatgccagcctgacattattgatggtgttatttatctgctttaatgcggcgtggaacgcgcaaaaacgcagtaaatatattgctaaagcttttatctcatcgtttattgccattacggtcggggcgggaattaccctggcggtgctgattctctcagggtcgattgaatttatcccgatgcaggtgatccctatcgccgggatgattgccggtaacgccatggtagcggtggggttgtgttacaacaatttagggcaacgggtcattagcgaacagcaacagattcaggagaaactgagtcttggtgcgacgccgaagcaggcttcagcgatattgattcgcgacagtattcgcgcggctttaattccgacggtcgattcagcaaaaacggttggcttagtgagtttaccaggaatgatgtccgggctgatatttgccgggattgatccggtgaaggcgattaaatatcagattatggtgacctttatgctgctctcaaccgccagcttgtcgaccattattgcctgctatttaacctatcgtaagttttataattcgcgccaccagttggtggtgacgcaattgaagaagaaatgatgcgatgccggatgcgcagcatcgcatccggcgttgtggttcatgtgccgatcaacggaatatcaatacaacaatgcatacagctggcggcgatacttcgacgccagtgcatcacccgtacccagcgcagcgaggatctcctggaacgttttacgcgtctgaccgtctgcggcggtgagatctttacgcagatgcccgaacagcaactccagcgcctcttcattgcgcccaacctgatgcagttgcagcgccagttgcgtcgccagtgcggcatcttctggattctccgccacctgctgttgcaactgttgaatttccggcgtatcagccgcctgcttcagcagttcgatttgcgccaccagcccctggtagcgggtgtcctgatcctgcaacggaatggttttcagcaccgcttccgcatcttcagaacggttcagcgcaatcagcgtttctgccagcagcaggccgatctccccgttctgattcgacaactgccaggcgtctttcagcaatggcagggcatcggtgtaattgctttcctgcatcagttgcatcgcctgctgcgctttcagctcttcttcgcgcggcagcactttatccagcagggcgcggatcgcctcttccggttgcggcccctggaagccatctaccggttgcccgttctggaacagatacacggtcggaatcgcacgcagaccaaactgcgcggcaatcatctgctccgcgtcgcagtccagcttcgccagaataaattgcccgttgtactgcgccgcgaggctttccagaattggggttaactgcaaacagtgctggctacgttcagaccaaaaatagaacagcaccggagtggtcatcgactgttcaagaacctgttgcaggttagattcgttaatgttgacaatattttctacggacatggagtcgctctctgttgtcgatattttctttgacatgggggcttaagcgcgcgcttcaactcacccctgcaatattttgtccatcacgcgccccggcagcaggcgcttaagcaccattaccgcccaggtcaccagcgtcaccggatagcgcatcttcggcttctcgctaataaaagcatggcgtactttgtccaccaccgcttccggtcccaacgtaaagcgggcggcgatgccgggattttcgactggtttatcactttgcgtctggttgacgttgtcggtgaagcgagtacgaatgggaccgggttcgatcaggctgactttaattccgctgtggcgcagctccatgcgcagtgcatctgaccacgcctccagcgcatatttactggccgcgtaagcgccacgacccggcgtggagattaatcccatcaccgatgatgtcatcacaatacgcccttcaccgtgcggtaacatcgcgggtaacaggcgcatggtgagctggtgtgcgccgaaaaagttggcggaaaactgctgttccatctgcgcacggctgatggtggaaagggggccatacatgccgaatccggcattgttaaagatcccatacagacaattatcggtcagggcgatcacctcgtcggctgcgcgatcaacactttctggtgaatccagatcgatcaacacgccggtaaatcccatgctgttcatgcgctcaacatcatccggtttccggcaacctgccagcacatgaaaaccctggcgttttaattcgagcgcgctttccaggccaattccactggaacatccggtaattaagaccgatttttgcataactttacctgtcaggatctccgttgctttatgagtcatgatttactaaaggctgcaactgcttcgccatccagtcggcaataaacggctgggcgtcgcggttgggatgaataccgtcatcctgcatccattgtggcttgaggtagacctcttccataaaaaagggcagcagcggaacatcaaactctttggcgagtttggggtaaatggcgctaaaggcttcattataacggcgaccatagtttgcaggcagacgtatttgcattaacaatggttcagcgttggcggctttgacatcctgcaaaatctggcgcagcgtttgctcggtttgctgtggctgaaaaccacgcaaaccgtcattgccgcccagttcaaccagcacccaacgcggctgatgctgtttcagcagagccggaaggcgcgccagtccttgttgcgaggtgtcgccgctgatgctggcattaactaccgacgttttactctgccacttatcattcaacaaggcaggccaggccgcgctggcagacattcgatacccggcgctcaggctatcacccagaatcaataacgtgtccgctgcggcggcacggaaggttaacaggaccaggaacaggaagggcaaatgccagcggaaaacattgttgaagttcatcatcttaagaagtccgtcggtcagggggagcatgaactctccatcctcaccggagttgagctggttgtcaaacgtggcgagaccatcgcactggtgggcgagtcgggatcgggtaagtcaaccttgctggcgatcctcgccgggcttgatgacggcagcagtggcgaagtgagtctggtgggacaaccgctacataatatggacgaagaagcgcgggcaaagttgcgcgcgaagcacgtcggctttgtttttcagtcatttatgttaattcctacccttaacgcgctggaaaacgtcgagcttccggctctgctgcgcggtgagagtagcgcggaaagtcgtaacggggcgaaagcgttgctcgaacagttagggctgggtaaacgtctggatcatcttccggcacagctttccggcggtgaacagcaacgagtggcgctggcacgagcctttaatggtcgacctgatgtgctgtttgccgacgaacccaccggcaaccttgaccgccagacgggcgataaaattgccgacctgctgttttccctcaaccgtgaacatggcaccacgttgattatggtgacccacgacctgcaactggcggcacgctgcgaccgctgcttacggctggtgaacgggcagttgcaggaggaagcatgattgcacgttggttctggcgcgaatggcgttcgccgtcgctattaattgtctggctggcgctaagcctggcggtggcctgcgtgctggcgctgggcaatatcagcgatcgcatggagaagggcttaagccagcaaagccgtgagtttatggcgggcgatcgggcgttgcgcagttcacgcgaagtgccgcaagcgtggctggaggaagcgcaaaagcgcggcctgaaagtcggcaagcagctgactttcgccacaatgacctttgcaggcgacacaccgcagctggcgaacgtcaaagcggtggatgatatctacccgatgtatggcgatctgcaaactaatccccctggcctgaaaccgcaggcgggcagcgtattgctggccccacgcctgatggcactgcttaacctgaaaacgggcgacaccattgacgtgggcgatgccaccttgcggattgccggagaagtgattcaggaaccggattccggttttaaccccttccagatggctccgcgtctgatgatgaatctggcggatgtcgataaaaccggagccgtgcagccggggagtcgggtcacctggcgttataaattcggcggcaacgagaaccagctcgacggctatgagaaatggttgttacctcagcttaaacccgaacaacgctggtacggtctggaacaggacgaaggcgcgctggggcgatcgatggaacgctcgcaacagttcctgctgctttcggcgcttctgaccttgctgctggcagtggcagcggtggcggtagcgatgaatcattactgtcgcagtcgctacgatctggtggcgatcctcaaaacgctgggggcagggcgagcgcaactgcgtaagctaatcgtcggtcagtggttgatggtgctgacgctttcagccgttaccggtggggccataggcctgttgttcgaaaacgtgttgatggtgctgctcaagcccgttctgcctgctgcactaccgccagccagcctctggccgtggctgtgggcgcttggcaccatgacggtcatctcgctgctggtggggctacgaccatatcgcttgttgctggcaacgcagcctttacgcgtattacgtaatgatgtggtagcgaacgtctggccgctgaagttttatctgccgattgtcagtgtggtggttgtgctgctgctcgccggattaatgggtggcagcatgctgctttgggcggtgctggcgggcgcggtagtactggctttgctgtgcggtgtgctgggctggatgctgctgaatgtacttcgccgcatgacgctgaaatcgctgcctctgcgcctggcggttagccgcctgttacgtcagccgtggtcaacgttaagtcagctttcggcattttcgctctcctttatgctgctggcactgctgctggtgttgcgtggcgatctgctcgaccgctggcagcagcagctacctccagaaagcccgaactactttttaattaacatcgccacagaacaggtagcaccgctaaaagcgttcctcgcggaacatcagatagtcccggaatcgttttatccggtggtgcgggcgcggctgacggcgattaacgataagccgacagaaggtaatgaagatgaggcgcttaaccgcgaactcaatcttacctggcaaaatacgcggcccgatcataatccgattgtcgccggtaactggccgccaaaagccgatgaagtgtcgatggaagaggggctggcgaaacgcttaaacgttgccctcggtgataccgtgacttttatgggcgatacccaggagttccgcgctaaagtgaccagcctgcgcaaagtggactgggaaagtctgcggcctaatttctattttattttccctgaaggggcattagacgggcaaccgcagagctggcttaccagtttccgctgggagaatggcaacggcatgttgacacaactcaaccgccagttcccgaccattagcctgttagatattggcgcgattttaaaacaggtcggtcaggtgctggagcaggtaagtcgggcgctggaagtgatggtggtactggtcaccgcctgcggtatgttgctgttgctggcacaggtgcaggtgggaatgcgtcagcgtcatcaggagctggtggtgtggcgcacactcggtgcggggaaaaaactgctgcgtaccacgttgtggtgtgagttcgccatgcttgggtttgtttccggcctggtggccgcaattggtgcggaaacggcgctggcagtgttgcaggcgaaagtgtttgattttccgtgggagccagactggcgattgtggattgttctgccgtgcagcggagcgctgctgctgtcgcttttcggcggctggctgggtgcgcgactggttaagggtaaggcgctgttcaggcagtttgcggggtgatgagagtaaataaggggcgttctggttgaatggaacgccttgtttaaattaattctacaatatgtttcattgatgatgttattgaattggtgatttcctatctttctattgctgatattaatctgaatcggtggagtttattgattttaaatatagccctacaaaaataactcagactaataaaatcataaatcatatgcgttgaatggatattatccatatagtgaatttgttgatgatgaattcatctgtgctaaaaatgttagtttaataaaatattgaaagtgacctgtaataacagttgttgttgattgagaacaaataagtttatgtgaaaaatatataaatacattagctggtcttgtgtgtcattttatttttttttgttgctaacacagggatatgaacaataactaaaagggcactttatatgagcggaaaaccagcggcgcgtcagggagatatgactcagtatggcggtcccattgtccagggttcggcaggtgtaagaattggcgcgcccaccggcgtggcgtgctcggtgtgtccgggcgggatgacttcgggcaacccggtaaatccgctgctgggggcgaaggtgctgcccggcgagacggaccttgcgctgcccggcccgctgccgttcattctctcccgcacctacagcagctaccggacgaagacgcctgcaccggtgggcgttttcggccccggctggaaagcgccttctgatatccgcttacagctacgtgatgacggactgatactcaacgacaacggcgggcggagcattcactttgagccgctgctgccgggggaggcggtgtacagccgcagtgagtcaatgtggctggtgcgcggtggtaaggcagcacagccggacggccatacgctggcgcggctgtggggggcgctgccgccggatatccggttaagcccgcatctttacctggcgaccaacagcgcacaggggccgtggtggatactggggtggtctgagcgggtgccgggtgctgaggacgtactgccagcgccgctgccgccgtaccgggtgcttaccgggatggcggaccgcttcgggcggacgctgacgtaccggcgtgaggccgccggtgacctggccggggaaatcaccggcgtgacggacggtgccgggcgggagttccgtctggtgctgaccacgcaggcgcagcgtgcggaagaggcccgcacctcttcgctatcttcttctgacagttcccgccctctctcagcctcagcgttccccgacacactgcccggtaccgaatacggccccgacaggggtatccgcctttcggcggtgtggctgatgcacgacccggcatacccggagagcctgcccgctgcgccactggtgcggtacacgtatacggaagccggtgaactgctggcggtatatgaccgcagcaatacgcaggtgcgcgctttcacgtatgacgcgcagcacccgggccggatggtggcgcaccgttacgcgggaaggccggagatgcgctaccgctacgacgatacggggcgggtggtggagcaactgaacccggcagggttaagctaccgctatctttatgagcaggaccgcatcaccgtcaccgacagcctgaaccggcgtgaggtgctgcatacagaaggcggggccgggctgaaacgggtggtgaaaaaagaactggcggacggcagcgtcacgcgcagcgggtatgacgcggcaggaaggctcacggcgcagacggacgcggcgggacggaggacagagtacggtctgaatgtggtgtccggcgatatcacggacatcaccacaccggacgggcgggagacgaaattttactataacgacgggaaccagctgacggcggtggtgtccccggacgggctggagagccgccgggaatatgatgaaccgggcaggctggtatcggagacatcgcgcagcggggagacagtacgctaccgctacgatgacgcgcacagtgagttaccggcgacgacaacggatgcgacgggcagcacccggcagatgacctggagccgctacgggcagttgctggcgttcaccgactgctcgggctaccagacccgttatgaatacgaccgcttcggccagatgacggcggtccaccgcgaggaaggcatcagcctttaccgccgctatgacaaccgtggccggttaacctcggtgaaagacgcacagggccgtgaaacgcggtatgaatacaacgccgcaggcgacctgactgccgttatcaccccggacggcaaccggagcgagacacagtacgatgcgtggggaaaggcggtcagcaccacgcagggcgggctgacgcgcagtatggagtacgatgctgccggacgtgtcatcagcctgaccaacgagaacggcagccacagcgtcttcagttacgatgcgctggaccggctggtacagcagggcggctttgacgggcggacgcaacgttatcattatgacctgaccggaaaactcacacagagtgaggatgagggacttgtcatcctctggtactacgatgaatcggaccgtatcactcaccgcacggtgaacggcgaaccggcagagcagtggcagtatgatggccacggctggctgacagacatcagccacctgagcgaaggccaccgtgttgccgtccactatggctatgacgataaaggccgcctgaccggcgaatgccagacggtggagaacccggagacgggggaactgctgtggcagcatgagacgaaacacgcatacaacgagcaggggctggcaaaccgcgtcacgccggacagcctgccgccggtggagtggctgacgtatggcagcggttacctggcgggaatgaagctgggcgggacgccgctggtcgagtatacgcgggacaggctgcaccgtgagacggtgcgcagcttcggcagcatggcaggcagtaatgccgcatacgaactgaccagcacatacacccccgcaggccagttacagagccagcacctgaacagcctggtatatgaccgtgactacgggtggagtgacaacggcgacctggtgcgcatcagcggcccgcgacagacgcgggaatacggctacagcgccacgggcaggctggagagtgtgcgcaccctcgcaccagacctggacatccgcatcccgtatgccacggacccggcgggcaaccggctgccggacccggagctgcacccggacagtacactcacagtgtggccggataaccgcatcgcggaggatgcgcactatgtctaccgccacgatgaatacggcaggctgacggagaagacggaccgcatcccggcgggtgtgatacggacggacgacgagcggacccaccactaccactacgacagccagcaccgcctggtgttctacacgcggatacagcatggcgagccactggtcgagagccgctacctctacgacccgctgggacggcgaatggcaaaacgggtctggcggcgggagcgtgacctgacggggtggatgtcgctgtcgcgtaaaccggaggtgacgtggtatggctgggacggagacaggctgacgacggtgcagactgacaccacacgtatccagacggtatacgagccgggaagcttcacgccgctcatccgggtcgagacagagaacggcgagcgggaaaaagcgcagcggcgcagcctggcagagacgctccagcaggaagggagtgagaacggccacggcgtggtgttcccggctgaactggtgcggctgctggacaggctggaggaagaaatccgggcagaccgcgtgagcagtgaaagccgggcgtggcttgcgcagtgcgggctgacggtggagcaactggccagacaggtggagccggaatacacaccggcgcgaaaagctcatctttatcactgcgaccaccggggactgccgctggcgcttatcagcgaagacggcaatacggcgtggagcgcggaatatgatgaatggggcaaccagcttaatgaggagaacccgcatcatgtgtatcagccgtaccgtctgccagggcagcagcatgatgaggaatcagggctgtactataaccgtcaccggtactacgatccgttgcaggggcggtatattactcaggacccgatggggttgaaagggggatggaatttatatcagtatcctttaaatccactacaacaaattgaccctatgggattattgcagacttgggatgatgccagatctggagcatgtacggggggagtttgtggtgttctttcacgtataataggaccaagtaaatttgatagtactgcagatgctgcgttagatgctttgaaagaaacgcagaatagatctctatgtaatgatatggaatactctggtattgtctgtaaagatactaatggaaaatattttgcatctaaggcagaaactgataatttaagaaaggagtcatatcctctgaaaagaaaatgtcccacaggtacagatagagttgctgcttatcatactcacggtgcagatagtcatggcgattatgttgatgaatttttttcaagtagcgataaaaatcttgtaagaagtaaagataataatcttgaagcattttatctcgcaacacctgatggacgatttgaggcgcttaataataaaggagaatatatttttatcagaaatagtgtcccgggattgagttcagtatgcataccgtatcatgattaattttagtgcttttattagtggggcctataaggagattcaatgaaatatagttcaatattttcgatgctttcattttttatactatttgcctgtaatgagacagctgtttacggttctgatgaaaacattatttttatgaggtatgtggaaaaattacatttagataaatactctgttaaaaatacggtaaaaactgaaacaatggcgatacaattagctgaaatatatgttaggtatcgctatggcgaacggattgcagaagaagaaaaaccatatttaattacggaactaccagatagttgggttgttgagggagcaaagttaccttatgaagttgcgggtggtgtatttattatagaaattaataagaaaaatggatgtgttttgaatttcctacatagtaaataatgctggcgctgatggatgcggatggaaacattgcgtggagcggggagtatgatgagtggggcaaccagctgaatgaagagaacccgcatcacctgcaccagccgtaccggctgccggggcagcagtatgataaggagtcggggctgtactacaaccggaaccggtactacgatccgttgcaggggcggtatatcactcaggacccgatagggctggaggggggatggagtctgtatgcgtatccgctgaatccggtgaatggtattgatccattagggttaagtcccgcagatgtagcgctaataagaagaaaagatcaactaaaccatcaaagagcatgggatatattatctgatacttatgaagatatgaagagattaaatttaggtgggactgatcaatttttccattgtatggcattttgtcgagtgtctaaattaaatgacgctggtgttagccgatcggcgaaagggctgggttatgaaaaagagattagagattacgggttaaatctgttcggtatgtacggcagaaaagtaaagctatcccattctgaaatgattgaagataataaaaaagacttggctgtaaatgaccatgggttgacatgtccatcaacaacagattgctcagatagatgtagtgattatattaatccagagcataaaaaaacgataaaggctttacaagatgctggctatctcaagtaatctatcaaagatgataatatttatttttgctattataatcattgttgttttatgcgtaattacttatctttatttatacaaagatgaatctcttgtaagtaaacattacataaactatatggcaataccagaaaatgatggagtttttacatggctcccagatttttttccgcacgtagcggtggatatatcaatatacacaaatgtagaagatgattatttttttcttatttttccctaacaaatgatgatgggggtaggtttaagaaaacattgacagtgagggccagggaacaagtggcgaaaatcgtatcaaagaatgatccagatacaaaaaaagtgtggtgtaaatatggtaagataccagggcaaggggatggtgtaaaccttttttttgttggtgaaattaatgttacgcattattttataacaaatattggagctggattgcctgatgcttgtgcagagtaattgcttgaattaagagtctatcccatatcgaagtcgtcaacttcgtagtgaggaaaagtaaaattcctgactgagaaaagacatgtcggctattgtgtaaagccatatagctcagacgatgaatatctactcgtattcagttgtttattgagggtgagttccgaccctgaaacaacaaataaaatgaacagtcagagagtttacatagaattgcactggtcttttacgatatctgacattgtgtaatacatattcagccatgcattaattaaaatgttacgtgtttaatgtgagtccctatctgaaaataaataatccttccggattaaaataaattcttgccgggaaagaaagaggaaataaaccattagcggaaaaccagcggcacgccagggtgacatgccccagtacggcggcccgatagtccagggttcagcgggggtactgatagtcgcgccgactgcatcgagaactccatacaactttttacggaacgtcacctgataaaatttgttcagtatcgtcttttgagattctcaaggttatggagtaaccagacagaacggacaccactgtcggagataaaaaccccctgtttacgcagctcgttgctggcccggtgctgaccatgtgtcgggaaagcgacggcgtaatcaacaacagcctgttcagttgcctcatcggtacggttcttaaggttaggagcgcggcgactacgattaatctgcgcatccacaccgccttcagcgaccagttcgcggtaacgataaaacgtatcacgcgaaacgcccatgattttacaggcttttgatacgttgctgagttcttcagccagattgagcaaaccggctttgtgtttgatgacgggattggcagtatgaagcatgagagttacctcttgttttggataaggattcgacactcatatcaaaaccggtaactctcaacctttcaaggccatgtgtcagatcaagtcgcgactaatacaaatacgtccctcattaccgcgccttaacccattccgccacttccgcccactcaccgcgaaagacaactttttccgcttttttctcaagctgatagcgatacatcgggtcgtaatattcttcaagtaacggcaccagccaggccagatgaccgtcggtgctgccggtggtgagttgcgttgtcagtgctgcatccagccttgcagccagttcgttatagcgctgtagccccagccgacgcttaatcgccgaaagtccgtgatgcaggtattcgcaatactcctgccagccctgttcgtcgccgtacgcgtgggtaaaatcatgatgcatacgcaagaaatactcttcgttcaggcgctcaagacggatctcaaacggatcttctaccaccgcaatcgccgcctgagtcattcgctcgcgcaggcattccggcaggtgattcgaaccgatcatccggctttcgtcttccagcacccacaggcgcaaattctgacgggcgtcggtttttagcatttcggcagccagcaggttttcaaaactcgcctggctaagttgtggttgtaacgtgcgaccaaacgccgaaccgcgatgacgcgccaacccttccagatcaacaccgttcggctgttgctgcactaacagcgttttaccgctgccggtacaaccgccaatcagcactatcggtttttgtgccagttcaatagtcgcctgaatcgcggtctggcgcagtgccttataaccgccttccaccagcggataatcaatccccgctgcatgcaaccagctttgcacaatatgtgagcgctgaccgccacgggcgcagcagagaataccttgcggattttgcaggcacgctgcccgccaggcgtccatgcgctgctgacgaatttcacccgccaccagtttatgtcccagcgccagcgctgcgtctgagccttgctgtttatagcaggtgccaacggcggcgcgttcatcgttattcattaacggcagattgatagcggcgggcattgcgccgtgctcaaactcgataggggcgcgaacatcaataatgggcgtatcagcaatcagcagggcacgatagtcctgttccgtgtgtctctcttgcatagttaaaagtgaacctcaaatcagcttgcgcgctattttacgcgccaacgcgcaaggaaacttgatttttaactgcgtgggttgccgaaaatttctaaaaatccgctgatttccggcctgcgctgggtaaacaaggtcacaatatcttctaccgctttgccgctgccaaatttgcgccatgccagactcaatggcgaaggagggcgcatcgttgggattacccggctgaccagttgttgattatcgatcattgactggcaaagcgattttggcaaaaaaccaatgccaacgcccgccagatgggcggcgattttcgtttccatatcgggaacaataatctctttttgccctggcaatcgccaggcgacgcgtttggttaaggtgcgggcgctgtcttcaatattgaccgccggaaagcgccgcaactgcgcttctgttagcggctcttcaacgttcgccagcggatgatccgccgccatgacaaagcgccattgcaccgatcctaagggatcaagactaaaggtatttgccagcgcctcagttcccgtgacgccgatagccagcgaaaaaccttcgtacaatagcgagtcccagacgcccatatagatttgtcgggagatgtgaaactgggtaaaggggtaacgctcattcagccacgccagcaactgggcgacggcctgggggttgtagagcaggttgttgatgacaatattcacctggcgttccacgccatcattcacctgttgcagctcgcttggcatactttccagccagctcagccagtctctggcctgggaaagtagatgctcgccagccgctgtcaacgtcacgctgcgagtcgtacggaaaaacagcgctactccggtattctcttccagaagtttaatgcgataactgatcgtcgccgtggttttacataatcgttctgccgcttttgaaaaacttcctgtttcagcaaccgcaatgaaagtccgcaaggtttctggatcgaacatcttcaggtatccccttttaaatccgcaagttgcgtgattttcttatcctctgatttatcagtatttttacatgataaccctgttcaatttgtggactaaatctagttttggaaaaatattccaacttttgtattgatgttgttctcttaaggttttagattgcctgttattgaaaccaagctgaccggtcggcggtggttgaacggaattatgttacaaggacaaaaagatgaaacttcaggtattaccgttaagtcaggaagcctttagtgcttatggcgacgtaatcgaaacgcagcaacgggattttttccatattaacaatggcctggtggagcgttaccacgatttggcgctggttgagattcttgagcaagactgtacgcttatcagcattaaccgcgcgcaaccggcgaatctgccgctgaccattcacgaactcgaacgtcatccgctgggtactcaggcctttatcccgatgaaaggtgaggtgtttgtggtggtcgtggcgttaggtgacgacaaaccagacctgtcaacgctgcgggcgtttatcaccaacggcgaacagggagtgaattaccatcgtaacgtctggcatcacccacttttcgcctggcagcgcgtcaccgattttctgaccatcgatcgcggcggcagtgacaactgtgatgttgaaagtattcctgaacaggaactctgttttgcgtgacgcctgcaaccgacttgcataagataaactaattgttcattgtttatgctcacttgtaggtcggagttaacgtaggtatgacggaagttagacggcgcggcaggccaggacaggcggagcctgtggcacagaagggcgcacaggcgttagagcggggaattgcgattctgcaatatttggaaaaaagtgggggaagttcgtcggttagcgatatttctctcaatctggatttgccgctctccacgacctttcgcttgctgaaggttttacaggcagcggattttgtctatcaggacagtcaattaggctggtggcatataggattaggtgtctttaacgtcggtgcggcgtacatccataaccgcgatgtcctctccgtcgccgggccgtttatgcgccgcctgatgttactttccggcgaaacggtcaatgtcgcgatccgtaacggcaatgaagcggtattaattggtcagttagagtgtaaatcgatggtcaggatgtgtgcgccactgggcagtcgtctgccactgcatgcttccggtgcgggcaaagcgctgctttatccgctggcggaagaggagttgatgagcatcattctgcaaaccggtttgcagcagtttacgccaactacgcttgtggatatgcccaccttgctgaaggacctggaacaagcgcgtgaactgggctataccgtagataaagaagagcatgttgtaggtctgaattgcatagcttcagcaatttacgatgatgtcggtagtgttgttgccgctatctccatctccgggccttcatcaagactgacagaagatcgttttgtcagtcagggtgagctggtcagagacaccgcccgcgatatcagcacggcgttgggactgaaagcacatccataatgtctgtcgcatcccgctctgcggagcgggtttttttgacaaaatttgaaagttggaaaaattttccaataaatagaggtaggaataaaatggcaaaaatgagagccgttgacgcggcaatgtatgtgctggagaaagaaggtatcactaccgccttcggtgttccgggagctgcaatcaatccgttctactcagcgatgcgtaagcacggcggtattcgtcacattctggcgcgtcatgtggaaggtgcttcgcacatggcggaaggttatacccgcgcaacggcagggaatatcggcgtatgtctggggacttccggtcctgcgggcacggacatgatcaccgcgctctattccgcttctgctgattccattcctattctgtgcattaccggccaggcaccgcgcgcccgtctgcataaagaagattttcaggccgtagatattgaagcaattgctaaaccggtcagcaaaatggcggttacagttcgtgaagcggcgctggtgcctcgcgtgctgcaacaggcatttcacctgatgcgttctggtcgtccgggtccggtactggtggatttaccgttcgacgttcaggttgcggaaatcgagtttgatcctgacatgtacgaaccgctgccggtctacaaacctgctgccagccgtatgcagatcgaaaaagctgtagaaatgttaatccaggccgaacgtccggtgattgttgccgggggcggggtaattaatgctgacgcagctgcactgttacaacagtttgctgaactgaccagcgttccggtgatcccaacgctaatgggctggggctgtatcccggacgatcatgaactgatggccgggatggtgggtctgcaaaccgcgcatcgttacggtaacgcaacgctgctggcgtctgacatggtgtttggtatcggtaaccgttttgctaaccgtcataccggctcggtagagaaatacaccgaagggcgcaaaatcgttcatattgatattgagccgacgcaaattggtcgcgtgctgtgtccggatctcggtattgtctctgatgctaaagcggcgctgacactgctggttgaagtggcgcaggagatgcaaaaagcgggtcgtctgccgtgtcgtaaagaatgggtcgccgactgccagcagcgtaaacgcactttgctgcgcaaaacccacttcgacaacgtgccggtgaaaccgcagcgcgtgtatgaagagatgaacaaagcctttggtcgcgatgtttgttatgtcaccaccattggtctgtcacaaatcgctgcggcacaaatgctgcatgtctttaaagaccgccactggatcaactgtggtcaggctggtccgttaggctggacgattccggctgcgctaggggtttgtgccgctgatccgaaacgcaatgtggtggcgatttctggcgactttgacttccagttcctgattgaagagttagctgttggcgcgcagttcaacattccgtacatccatgtgctggtcaacaacgcttatctggggctgattcgtcagtcacaacgcgcttttgacatggactactgcgtgcaactcgctttcgagaatatcaactccagtgaagtgaatggctacggtgttgaccacgtaaaagtagcggaaggtttaggttgtaaagctattcgggtcttcaaaccggaagatattgcgccagcctttgaacaggcgaaagccttaatggcgcaatatcgggtaccggtagtcgtggaagttattctcgagcgtgtgaccaatatttcgatgggcagcgaactggataacgtcatggaatttgaagatatcgccgataacgcagcggacgcaccgactgaaacctgcttcatgcactatgaataagggagataaataatgttacgtttctctgctaatttatcgatgttatttggagaatatgattttctcgcccgttttgagaaagctgcgcagtgtggttttcgcggcgttgaatttatgtttccttatgactacgacattgaagaattaaaacatgtgctggcgagtaataaactcgaacatacgctgcacaatttaccggcgggtgactgggcggcgggggagcgcggtattgcctgtattcctggccgtgaagaagagtttcgggatggcgtagcagcagcgattcgttatgcccgtgcgctgggtaataaaaaaattaactgtctggtcggtaaaacgccggctggtttcagcagtgaacagattcacgcaacgcttgtagaaaacctgcgttatgccgcgaatatgctgatgaaagaagatattttattactgattgaacctattaaccattttgatattcctggtttccatctcaccggaactcggcaggcgctgaaattgattgatgatgttggttgctgcaatttgaaaattcagtatgacatttatcatatgcagcggatggaaggtgaattaaccaacaccatgactcagtgggctgataaaattggtcacctgcaaattgccgataatccgcatcgcggcgaaccgggaaccggagaaattaattatgattatctctttaaggtaatcgaaaattctgactacaacggttgggttgggtgtgaatataaaccccaaaccaccacggaagccggtttacgctggatggatccgtaccgttaaaacgtaacgctattcagacaatgcttttttaggccgctaagttggcaggggatcgtgttgtctgaattcaggaaaagcgaaatttaaaagaggttaattatgaaactgggatttattggcttaggcattatgggtacaccgatggccattaatctggcgcgtgccggtcatcaattacatgtcacgaccattggaccggttgctgatgaattactgtcactgggtgccgtcagtgttgaaactgctcgccaggtaacggaagcatcggacatcatttttattatggtgccggacacacctcaggttgaagaagttctgttcggtgaaaatggttgtaccaaagcctcgctgaagggcaaaaccattgttgatatgagctccatttccccgattgaaactaagcgtttcgctcgtcaggtgaatgaactgggcggcgattatctcgatgcgccagtctccggcggtgaaatcggtgcgcgtgaagggacgttgtcgattatggttggcggtgatgaagcggtatttgaacgtgttaaaccgctgtttgaactgctcggtaaaaatatcaccctcgtgggcggtaacggcgatggtcaaacctgcaaagtggcaaatcagattatcgtggcgctcaatattgaagcggtttctgaagccctgctatttgcttcaaaagccggtgcggacccggtacgtgtgcgccaggcgctgatgggcggctttgcttcctcacgtattctggaagttcatggcgagcgtatgattaaacgcacctttaatccgggcttcaaaatcgctctgcaccagaaagatctcaacctggcactgcaaagtgcgaaagcacttgcgctgaacctgccaaacactgcgacctgccaggagttatttaatacctgtgcggcaaacggtggcagccagttggatcactctgcgttagtgcaggcgctggaattaatggctaaccataaactggcctgatacccgcaataaaaatggccgatatcagaaaatgaatcggccagcaatattaaaaaagaaagcagccaaagatgttgcttcagtattaaaaataatatttttattttatttgttcctcatagctagattaaaacaacgttattcgatacgtgaaattaagagggatttatggaacatcagagaaaactattccagcaacgcggctatagcgaagatctattgccgaaaacgcaaagccagcggacctggaaaacatttaactattttaccttatggatgggttcggttcataacgttcccaattatgtgatggtcggcggcttttttattctcggcttgtctacctttagtattatgctggcaattatcctcagcgcctttttcattgccgcggtaatggtattaaacggtgctgcgggcagtaaatacggtgtgccttttgccatgatcctgcgtgcttcttacggtgtacgtggtgcactgtttcccggattattaaggggcggaattgccgccatcatgtggtttggtttgcaatgttacgcggggtcactggcctgcttgattctgattggcaaaatctggccgggatttttaactctcggtggtgatttcactctgttaggcctttctctaccgggcttaattactttcttaatcttctggctggtcaacgttggtataggttttggcggtggcaaagttttaaataaattcactgccattcttaacccgtgcatctatatcgttttcggcggtatggcgatttgggcgatttcactggtcgggatcggtccaatctttgactacattccgagcggtattcagaaagcagaaaacggtggcttcctgttcctggtggtgattaacgcggtagttgcggtctgggcggcaccggcggtgagcgcatccgactttacgcaaaacgcccactcgtttcgtgagcaggcgctggggcaaacgctgggtttagttgtggcctatattctgtttgcggtcgccggggtatgtattattgccggagccagtattcactacggcgctgatacctggaacgtgctggatattgttcagcgttgggacagcctgttcgcctcgttctttgcggtactggttattctgatgacaactatctccactaacgcgaccggtaatattattccagccggttatcagattgccgccattgcaccgacaaaactgacctataaaaacggcgtactgattgccagtattatcagcttgctgatctgcccgtggaaattaatggaaaatcaggacagcatttatcttttcctcgatattatcggcggaatgcttggtccggtaattggtgtcatgatggcgcattattttgtggtgatgcgcggacaaattaatcttgatgaactgtataccgcacctggcgattataaatattacgataacggttttaacctcactgcgttttcagtaactctggtggccgttattttatctcttggcggtaagtttattcactttatggaaccgttatcgcgtgtttcatggtttgtcggcgtcatcgtcgcctttgcggcctacgccttattaaagaaacgtacaacagcagaaaaaacaggagagcaaaaaaccataggttaattaatcccgatattgaacattgagttaaaaaccaatctgtattttacaaggagtttgttatgtcttttgatttaatcattaaaaacggcaccgttattttagaaaacgaagctcgcgttgtagatatcgccgttaaaggcggaaaaattgctgctatcggtcaggatctgggcgatgcaaaagaagttatggatgcgtctggtctggtggtttcgccgggcatggttgatgcgcacacccatatttctgaaccgggtcgtagccactgggaaggttatgaaaccggtactcgcgcagcggcaaaaggtggtatcaccaccatgatcgaaatgccgctcaaccagctgcctgcaacggttgaccgcgcttcaattgaactgaagttcgatgccgctaaaggcaagctgactattgatgcggcacaactcggtggcctggtgtcttacaacatcgaccgtctgcatgagctggatgaagtgggcgttgtcggcttcaaatgcttcgttgcgacctgtggcgatcgcggtatcgacaacgacttccgtgatgtaaacgactggcagttcttcaaaggtgcgcagaagctgggcgaactgggtcagccggtgctggtgcactgcgaaaacgcgctgatttgtgacgaactgggcgaagaagcgaagcgtgaaggtcgcgtaaccgctcatgactatgtggcttcgcgtccggtatttaccgaagtggaagcaattcgccgcgtactgtatctggcgaaagttgctggttgccgtctgcacgtttgccacgtcagcagcccggaaggtgttgaggaagtgactcgtgcacgtcaggaaggtcaggacgttacttgtgaatcctgcccgcattactttgtactggataccgatcagttcgaagaaatcggtactctggcgaagtgttcaccgccgatccgcgatctggaaaaccagaaaggcatgtgggaaaaactgtttaacggtgaaatcgactgcctggtttccgaccactctccatgcccgccggaaatgaaagccggtaacatcatgaaagcatggggcggtatcgccggtctgcaaagctgcatggacgtgatgttcgatgaagcggtacagaaacgcggtatgtctctgccaatgttcggcaaattaatggcgactaacgcagcagatattttcggtctgcagcaaaaaggccgtatcgccccaggaaaagatgccgacttcgtcttcattcagccgaatagcagctatgttcttaccaatgacgatctggaatatcgccacaaagtcagcccgtatgttggccgtaccattggcgcgcgtatcacgaaaaccatcttacgtggtgatgtgatttacgacattgaacagggcttccctgttgcgccgaaaggtcaatttatccttaaacatcagcagtaatctggcccctgcaatgcccgtccttgcggcgggcattctccggttaaggtgtgtttatgttcaattttgcagtcagccgcgaaagcctgttatcaggatttcagtggtttttctttattttttgcaacacggttgtggttcctcctacgctactttctgcttttcagttgccgcaaagtagcctgcttacgctcacgcaatatgcttttcttgctaccgcactggcctgcttcgctcaggcgttttgcggtcatcgtcgcgctattatggaagggccaggtggcctgtggtggggaaccatccttactatcacccttggtgaagcatcgcgcgggacaccgatcaacgatatcgccaccagcctggcagtggggattgcactctccggcgtgctgacgatgttgattggttttagcggattaggccatcgcctggcacggttatttacgccgtcggtgatggtcttgtttatgttgatgctgggcgcgcagctgaccactatctttttcaaaggtatgctcgggctgccgtttggcatagccgacccgaattttaaaattcagttaccgccgttcgcgctctcggtggcggtgatgtgcctggtactggcgatgattatcttcctgccgcaacgttttgcccgttatggcctgctggtcggcaccataaccggctggttgttgtggtacttttgctttccttcttcgcactcgctctccggtgagttgcactggcagtggttcccgctcggcagtggcggtgctttgtcgccgggaattattctgacggcggtgattacaggtctggtaaatatcagcaatacctacggtgcgattcggggcacggatgttttttatccgcagcagggcgcagggaatacgcgttatcgtcgtagctttgtggcgaccggatttatgacgctgataaccgtaccgctggcggtaattccattttcaccgtttgtttcatccattggtttattaacccagactggcgattacacgcggcgttcgtttatttatggcagcgttatttgcctgctggtggcgctggttcctgcactcacgcgactgttttgcagtatccctttacccgtgagtagtgcggtcatgctggtttcttatctgcctttactcttttccgcgctggtgtttagccagcaaataacgtttaccgctcgcaatatttatcgactcgcattgccgttatttgtcggcatatttttaatggcattaccgcctgtgtatctgcaagaccttccattaacgcttcgtcctctgctcagtaacggcttattggtcgggattttactggctgttcttatggataaccttattccgtgggaacgcatcgaataatttgttgaaaaaggattgataatgaagattgtcattgcgccagactcttttaaagagagcttaagtgcagaaaaatgttgtcaggcaattaaagccgggttttcgaccctctttcccgatgcgaactatatctgtttgccgatagcggatggcggcgaagggacggtggatgcgatggtcgccgcgacgggcggcaacatcgtgacgcttgaagtctgcgggccgatgggcgaaaaagtgaatgctttttatggccttaccggcgacgggaaaacggcggtgattgagatggcggcagcaagtggcctgatgctggtcgcgcctgaaaagcgtaatccgttgctggcctccagttttggtacgggggagttaattcgtcatgcgctggataacgacattcgccatattattctcggcattggcggcagtgcgacggtcgacggcggtatgggcatggcgcaggcgctcggtgtgcgtttccttgatgccgacggtcaggcgctggcggcaaacggtggtaatttagcgcgcgtggcaagcattgagatggatgaatgcgatccgcgtctggcgaattgccatattgaagtagcatgtgacgttgataacccgctggtaggggcacgcggcgcggcggcggtgtttggcccgcaaaaaggggcaacgccggagatggtcgaagaacttgaacaggggctgcaaaattacgcccgtgttttacaacagcaaactgaaattaatgtctgccagatggcgggcggcggcgctgcgggcggtatgggtattgcggcggcggtatttctcaatgcggatattaaaccgggcattgaaattgtgttgaatgcggtcaatcttgcgcaggcagtgcagggcgcagcactggtgattaccggggaagggcgcatcgactcgcaaacggcaggcggtaaagcgccgctgggtgtggcgtcggtggcgaagcagtttaatgtaccggtgattgggattgctggcgtattgggtgatggcgtggaagtggtgcaccagtacggcattgacgcggtattcagcattttgcctcgtctggcacctttagccgaagtgctcgccagcggtgaaaccaatctcttcaacagcgcgcgaaatattgcctgcgccattaaaataggtcagggaattaaaaactaacccttacctttaaagcggatgcgatttatatcgcataagagtgcagtactcatgccggatgcggcatgagtaccatatccttcctgaaaatcgcgcaaattctatatattgcagagatcatgtaggcctgataagcgaagcgcatcaggcaatgttacaaaaaaagccacggtataaaccgtggcaaaatccaacatagctaaaaataatcaggcgagtggtatgacttaaatctctacgtcgcggttacaatctttcgagtaaatatagctgaacgcttcaccacgccctacaccataaccagcctgtaaagaataagcgcccataaagatgtaatcgccttttttcaccgggatccagttattgtcgaggttataaaccccctgaccggaaagaatataggcaccgtgttcctgaacgtgtgtttcgatataaccgtggctggcacctggtgcaaaagagaggatatgcatgttcatatcaaaacctaactctttgggcagaaaatccagcagaataacatcgtccatgccttcataatgaatgcgttccagttcgctggcattgccagaaaccagccacggtgcatagccttctaccggaacatagcggcgcttatataaaaagatttggctgtcttcggcctgggcgttaacaaacgtcattaaggagcctggcgggcaataaagatagccaccttcgcttaaggcaaatgttttgccttcggctttggcagtgatatttccagagatcacatacaggaacgtttcaatgccttcgccaccgaagccctgttggttgccaccgttttgatgcagtgtgaccagataatcaacaaaagaggcacccagctttggcgtggagaggattgtcgcgtcacaattttcaaagcccggaataatattttttaccagaccatccggggttaacagtgcgaaattaccgtgtttaacaatcgcacggttagccagtaaatcttcgcggtaaccggtgacgttatttaaatatcccatttatgactccttatttctgccaggcaagttgataaagcatgagtgccaacgttttgaccccttcggcaaggtcggtaatattggtgcgttccgccgggttatggctgatcccgttgatgctggggataaaaatcatgcaggttggtacgcgaggcgcgaaaatttgcgcgtcgtgcccggcaccactgtgcatcacccggtaattcagtttttctctttcacacaattctgtcagggtggcgaccagctccttattcatcggcacgggttcttcgtccatccataaatcgatatcaataccaatgtccatttcatcgcaaatcgcccgcatgtcgttttctaactgttgggtgaaatcgcgcagcacggcagcgtcggtatgacgacaatcaatggtgaacgtggttttacccggcaccacatttaccgtattcgggcgcggctctactttgccaaaggtcagaaccagcggatcgcccatccttttcgctttttcgaccgactgatggcaaatgcgactgaaagcgtaaactgtatcacgacgataacccatcggcgtggtgcctgcatggtttgattcgccgttcagcgttaccgtataacgacgctgcccgacaattgcattcaccacgccaattgattgcccattactttccagcacacagccctgttcaatatgcagttcaacaaaggctttaatatcctgacgcggagttagtggggcgttcggaagagtaaatccgcaagccttcatcgcatcgacaaaactatttcctttggcatcacagatattccgcacgtcgtcaggattcgccagcccaaaaatatttttactgccccagaagacatacgggaagcggctgccttcttcttctgccatcgccaccacttcgaccgtacgtagcggcgcgccgtattgcgttttcagccagtcaattgccagccacgccgccagcgcgccgaattgcccgtcaaggttaccgccgttaaccacggtatcgatatgcgaaccgctcagaaccacttcctgtggatattcggtgccattcaggcgaccgtataaattccccacttcatcgaaacgtgtttccagcccgcttgctgccattctttttttaaattgctgctgggtttccagccattccggcgaataaagtaaacgggtcatcccacccgctgggtcagcgccaaaagaggaaagccagggcagcgtttcttctatagcttgacggaaatgtgtaatcataagaaagtcctgtctcaataattattgcgcaaagggatttttcgtttcgtatgacgtgttataaagcgcgtcggaaattaaatactggtaaatatcatcaacaatttcgatgccttcgacggcggctttgcgttgtttaatatcctgatcctgtccgggataataaacctgattaaaaccgggcgcgggggtaatggcatttaattcgcgcatggtctggctaagatgttgacggaataattcgctggaggagaaaaagttcggattaataactatatgtaattgccccaaattacgccctgcgtgtaaatcgtcatacatcgaactaacctgtcgcccgaacggtaagccgagtaagacgcctgagaggacgtcaatcatcatcatcaggccatacccttttggcccggcggcggggagcagagcatgtaccgcgaacggatcggttgttggtacaccgtttttatcgaccgcccaggtatccgggatagacatattacgcgagcgggcgtcgagcacttttccccatgcctgtacggtagtcgccatatcaaaggtaaggatctcgtcgccttctcccggcgcggcaaaggccagggggttagtaccgtagtaaatttccgcgccgccaaacggcaccaccattggatcggactggcacatcgaaatgccaatgaatccggcgcgggctgcctgctgcacaaaataagagattgcgccgctgtgacccatccggctgataccgaccaccgcaacgccattttgctgggcggttttgatggcatgttccatacccattttcgccgcgacctgtccggcggcattgtcggcatgtaaaattgccgagcacggcccggtttcctcaagacgaaactccggttcgcggttggtgccgccttttgaaatgcgttccgcgtagtattccacgcgcaccgcgccatgagagtggatccctctggcatcggcgtaaaccaatacttcagccacggttgcagcgtgctcacgttttaacccagcctggcagagtttattctcaattagctggtggagtgtttcccgactgattttcatctgtcttcctttttaacgacggtgtgaagcatgactgcaattaacatacagggaaaatatctggattatgtgatccagacaggcaaaaaaatatagttagaatttatttgataatccgctcacttttaacctgatttttaaaacaacaacgcttattaaaaaataatgagtaatagcctggtggttatttgaattcttttgttaataattcctgtgtgatattcatcaccttatttactcgttgtcatcgataccgtaatcgccacattaacactgctcgtgcaattgccatgggtgcaatttttaaggagttgttatgatccacgcctttattaaaaaagggtgttttcaggattcggtcagtttaatgattatttcacgaaaactcagcgaatcagaaaatgttgatgatgtttccgtaatgatgggtacgcccgccaataaagcgttattagataccacaggtttctggcatgacgattttaataacgccacgccgaacgatatttgcgtggcaattcgtagcgaagcggcggatgcggggatcgcgcaggcgattatgcagcagcttgaagaggcgctaaaacaactggcgcaggggtcaggcagcagccaggcgttgacgcaggtgcgtcgctgggacagtgcctgtcagaaattacccgatgccaatctggcgctgatttcagtggctggcgagtatgcggcggagctggcaaaccaggcgctggatcgcaacctcaacgtgatgatgttctccgataacgtcacgctggaagatgaaatccaacttaaaacccgcgcgcgggaaaaaggcttgctggtgatggggccggactgcggtacgtcgatgattgccggcacaccgctggcttttgctaacgtgatgccggaaggcaatattggcgtcattggcgcttccggtaccgggattcaggagctgtgttcgcagattgcgctggcaggggagggaattactcacgcgattggccttggcgggcgcgacctcagccgtgaagtgggcggcatcagtgcgctaacagcgctggaaatgctcagtgcagacgagaaaagcgaagtgctggcatttgtttcaaaaccacctgccgaagctgtgcgtctgaaaattgttaatgccatgaaagcaaccggcaaaccgacggtggcgctgtttttaggttataccccggcggtggcccgcgacgagaatgtctggtttgcctcctcgctggatgaggccgcacgcctggcttgcctgctttcacgcgtcacggcgcgacgtaacgcaatagcgcctgtcagcagcggatttatttgcggtttgtataccggcggtacgctggctgccgaagcggcgggattacttgccggacaccttggcgtggaagccgacgatacccatcaacatggcatgatgctggacgccgatagccaccagattattgacctcggcgatgatttctacaccgtcgggcgtccccatccgatgatcgacccaaccttacgcaaccagttaattgccgatctcggcgctaaaccgcaagtgcgcgtgttgctgcttgatgtcgtgattggcttcggtgcgaccgccgatcctgccgcctcgctggtgagcgcctggcaaaaagcctgtgccgcgcgtttagataatcaaccactgtatgccattgccacggtgacaggcactgaacgtgacccgcaatgccgctcgcagcaaatcgccacgctggaagatgcggggattgcggtcgtgagttcgctaccggaagccaccttgctggcggcagcgttaattcatccgctctcgcctgccgcacagcaacacacaccgtcattactggaaaacgtcgccgtgattaacatcggattacgcagctttgcgctggagctacaaagcgccagcaaaccggttgtgcattaccaatggtcgccagtcgccggtggcaataaaaaactggctcgtttattagaacgtttgcaataaggggttcccatgtttacatcagtggcgcaagccaatgctgcggttatcgaacaaattcgtcgcgctcgtccacactggctggatgtgcaaccggcttcttcacttatcagcgaactaaacgagggcaaaacactgcttcacgccgggccgccaatgcgctggcaggagatgaccggacccatgaaaggggcgtgcgtgggcgcatgtctgttcgaaggttgggcgaaagatgaagcgcaggcgctggcaatactggagcagggggaagtgaacttcattccttgtcaccatgtgaatgccgtcgggccaatgggcggtattacttctgccagtatgccgatgctggtggttgagaacgtgaccgacggcaaccgggcgtactgcaacctcaacgaaggtatcggcaaagtgatgcgttttggcgcttacggcgaagatgtcctgactcgccatcgctggatgcgcgatgtgttaatgccagtattaagcgcggcgctggggcgcatggagcgcggtatcgatctcacggcgatgatggcgcagggcattacgatgggcgatgagttccatcaacgcaatattgcttcctctgcactgttaatgcgtgcgctggccccacaaattgctcgcctcgatcatgataaacagcacatcgccgaagtgatggatttcctcagcgtgaccgatcagttcttcctcaacctcgcgatggcttactgcaaggcggcgatggatgctggcgcgatgatccgcgcaggcagcatcgtcacggcaatgacccgcaacggcaatatgttcgggattcgggtaagcgggctgggcgaacgctggtttactgcgcctgtaaacactccgcaaggtctgtttttcaccggcttctcgcaggagcaggcgaacccggatatgggcgatagcgcgattaccgaaacctttggtatcggaggtgcggcaatgatcgcagcgcctggcgtaacgcgctttgtcggtgcgggtggcatggaagcggcaagagcggtatctgaagagatggcggaaatttaccttgaacgcaatatgcagttgcagatcccaagctgggattttcagggcgcgtgcctggggctggacattcgtcgcgtggtagaaaccggcattacgccactcatcaataccggtatcgcccataaagaggcggggatcgggcagattggcgcaggcaccgtgcgggcaccgctggcgtgctttgaacaggcgctggaagcactggctgaaagcatgggtattggttgaggaacgcgcaatgacgatcatccatcctctgcttgccagtagtagcgcaccgaattatcgccagtcctggcggttagcgggagtgtggcggcgggcgattaacctgatgacggaaagcggcgaactgttaacgttgcatcgtcagggtagtggtttcggccccggaggatgggtgcttcgccgtgcgcaattcgatgcgttatgcggtggattatgcggcaatgaacgaccacaggttgtggctcaagggattcgcctcgggcgtttcacggttaaacagccacagcgttattgtttgctgcgtattacgccgcctgcgcatcctcaaccacttgcagctgcatggatgcaacgcgcggaggaaaccgggcttttcgggccactggcgttggcggcaagcgatccgctgcctgctgagttacgccagtttcgtcactgttttcaggccgcgctcaatggcgttaagaccgactggcggcactggctgggtaaaggccccggattaacgccgagtcatgatgacacgctgagcggaatgctgctggcggcctggtattatggcgctttagatgcgcgctccggtcgtccgttttttgcctgttccgacaatctgcaactcgttaccacagcggtgagcgtcagttatttacgttatgccgcgcaaggatatttcgcctcgccactcctgcactttgttcatgctctgagttgcccgaaacgtaccgctgttgcgattgattcgctgctggcgctggggcatacgtcaggggcagatacgctgctggggttctggcttggccaacaattattacaaggaaaaccatgaaaacactggttgtggctcttgggggcaacgccttactccagcgcggtgaggcgctgacggcagaaaatcaatatcgcaatatcgccagtgctgtacccgcgctggcacgcctggcccgttcttatcggttggcgattgttcacggcaacgggccgcaggtggggctgctggcattgcagaatctggcgtggaaagaggtagaaccgtatccgctggatgtgctggttgcggaaagccaggggatgattggctatatgctggcgcagagtttgagcgcacagccgcagatgccgcccgtgacgacggtgctgacgcgcattgaggtttcgcctgatgatccggcgtttttgcagccagagaaatttattggtccggtttatcagccagaagaacaagaggcactggaagcggcttacggctggcagatgaaacgtgatggtaaatatttgcgccgggtggtggcgtctccgcaaccgcgtaaaattctcgacagcgaagccatcgagttgttgctcaaagaggggcatgtggtgatttgcagtggcggcggcggtgtgcctgtgacggatgacggagcagggagtgaagcagtgattgataaagatctcgccgctgcgttgctcgccgagcagattaatgcagatggactggtgatcctcaccgatgctgatgcggtatatgaaaactggggaacgccgcagcaacgtgccattcgccatgccacaccggatgagttagcgccatttgccaaagccgatggttcgatggggccgaatgtaacggcggtgagtggttatgtcagaagccgtggtaaacccgcgtggattggggcgttatcgcgaattgaagagacgctggcgggcgaagcggggacctgtatttcgctgtagtcgtaggcattagacatttgtgcctgatgcgacgcttgacgcgtcttatcaggcctacaaccggtgccgcatccggcaattggtgcacaatgcctgatgcgatgcttgacgcatcttatcaggcctacaatgggtaccggatcggtaggccggataaggcgtttacgccgcatccggcaagaatagagcaccagttaaccgaacttactctgcgcccaaatcacgccgctggcatattccggcggcagcagcgggattaaggcttccagcgtcgcagtcagacgcgatgtgtcgctgtcggtcaaattcagatgccccactttacgccccggacggacttctttgtcgtaccagtgcagatgcaccagcggcagtttcagccagtcataattcacatcgctaccaatcagattgatcatcaccgacggattattcaccactggttgcggtaacggcagatcggtaatcgcccgcagatgcagctcaaactggctgatgctggcaccgttttgtgtccagtgaccgctgttatgcacacgcggtgccagttcgttgatcaacagaccttgcggggtgacaaaacactccatcgccatcacgcccacatagcccagctcctgcataatcgccgacagcatctcttcggcttgcgcctgctgctgtgcgttggcctgcggaaaagcgacgctggtgcgcaaaataccgtcctgatgcaggttatgcgtcagcggataaaacacggtgctgccatcaaagccgcgcgcgccaaccagcgacacttcaccagagaagttaatgccctgctcgacaatacattcgccgtaacactctgccggtaactgttcggtttcatttgcgcgtaaacgccattgaccgcgaccgtcataaccaccagtgcgacgcttaacaatcgccagctcacctaaacgatcaaacaccgcaggccactcgctgcgttcggcaagtaactgccacggtgcagtcggcaggtggagcttatcgaaaagctgcttctgagtcagacggtcagcaataatcgggaacacatcgcggttcacaaaggccggatggcgcgccagctcgcgggttaatgcggtttccggccagcgttctatctcagcggtaatcacgctttgttgaaaaggcaccgccgccggttcagcgtccagcccgactggccagacagcaatgcctaacggttcgcctgcctgacgcagcatacggcctaactgcccgttaccgaggacgcaaacctgtttcatgccgcacctcgcgggtccgggttttccagcacttcgtcggtctgggctttgcgccagtcattcagacgctggtgcagttctttatcatgagtcgcaagaatttgtgctgccagtaacgccgcgtttgccgcgccagctttaccaatcgccagcgtacccaccggaatgccgcgcggcatttgtacgatggagtagaggctatcgacaccgctcagtgcggcgctctgtactggcacgcccagcaccggcaccagcgttttggcggcaatcatgcctggcagatgcgctgcgccgcctgcgcccgcaataatcacctgataaccgttctcttcggcgctttcggcgaagctgaacagtttatcgggggtgcggtgagcagaaaccacttcaacgtggtgcgggacattcaggatttcgaagatttcggcggcgaactgcatggtagcccagtcgcttttggaccccatcacgatggcgacacgcgccggattattgcgggaagacatgcgtcttaaaactcctgtggtgcacaactctcggctttagagggcacagagaatagcacggaaagagagcaaggaaaacggttgcgtggctgtgaaatcagcaaagttgcgggttttttaaaacggaaaatgaatcagctcaacgtcatccgccgtgactttcaccattgaaccttccgtatgccaggcacccagtaccacgcgaaaagcaggttgctgattggcgataagttcatgcaccgccgggcgatgggtatgcccgtggatcagccattgcacctgatgtttttccatcgcactgaccaccgcgttttggttaacgtccatgatcgccagcgatttactgctgttggcttctttgctgttcgcgcgcattcgcgcggcaatgcgtttgcgcacaaacaacggcagggcgaggaatagcgtctgcagccagggtttgtggaccttggcgcgaaaagcctgataacccgcgtcatcggtgcacagcgtgtcgccatgcataatcaacacccggcgaccataaagttcgagcaccttttcttccggcaataacgtcatgccactttcacgggcaaagcgtttgccgagcagaaaatcacggttgccatgaatgaaataacagggaacgccggaatcggacaccgctttgatcgccgccgccatcttgcgatggagtgggttgggatcgtcgtcgccaatccatgcttcaaacagatcgccaagaatatacagcgcgtcggccttgcgggcttcccccgctaaaaaacgcagaaaaccggcggtgatcgccggttcttccacgcagagatgaagatctgcaataaagagtgtcgccacgattactcgctaacggtcacgctttcaatgataacgtcttcttttggcacgtcctggtgcataccgctacgaccggttgcaacacctttgattttgtctaccacgtccatgccgtcaaccacttcagcaaacacgcagtagccccaaccttgcaggctttcgccagagaagttcaggaagtcgttatcaaccacgttgatgaagaactgtgcagttgcagagtgcggagcctgagtacgtgccattgccagcgtaccacgggtatttttcaggccgttgttggcttcgtttttgatcggttctttggtggctttttgtttcatgcccggttcaaaaccgccgccctgaatcataaagccgttgataacacggtggaaaatggtgttgttgtaaaaaccttcgcggcagtagtccaggaagtttttaactgtttcaggtgctttatcgtcaaaagttttgatgacaatatcgccgtgattggtgtggaaagtaaccatttttgcatcctgttccgtttgattggtgcttcaacccagttcgggtcatatatagggtggtgttatagcataaccgcacgatcggatcatcacgcaatgtatgctgattcgcgcgggaaatatgggtattatacgcaactcaattacccacacatgtctaaacggaatcttcgatgctaaaaatcttcaatactctgacacgccaaaaagaggaatttaagcctattcacgccggggaagtcggcatgtacgtgtgtggaatcaccgtttacgatctctgtcatatcggtcacgggcgtacctttgttgcttttgacgtggttgcgcgctatctgcgtttcctcggctataaactgaagtatgtgcgcaacattaccgatatcgacgacaaaatcatcaaacgcgccaatgaaaatggcgaaagctttgtggcgatggtggatcgcatgatcgccgaaatgcacaaagattttgatgctttgaacattctgcgcccggatatggagccgcgcgcgacgcaccatatcgcagaaattattgaactcactgaacaactgatcgccaaaggtcacgcttatgtggcggacaacggcgacgtgatgttcgacgtcccgaccgatccaacttatggcgtgctgtcgcgtcaggatctcgaccagctgcaggcaggcgcgcgcgttgacgtggtcgacgacaaacgcaacccaatggacttcgttctgtggaagatgtcgaaagagggcgaaccgagctggccgtctccgtggggcgcgggtcgtcctggctggcacattgaatgttcggcaatgaactgcaagcagctgggtaaccactttgatatccacggcggcggttcagacctgatgttcccgcaccacgaaaacgaaatcgcgcagtccacctgtgcccatgatggtcagtatgtgaactactggatgcactcggggatggtgatggttgaccgcgagaagatgtccaaatcgctgggtaacttctttaccgtgcgcgatgtgctgaaatactacgacgcggaaaccgtgcgttacttcctgatgtcgggccactatcgcagccagttgaactacagcgaagagaacctgaagcaggcgcgtgcggcgctggagcgtctctacactgcgctgcgcggcacagataaaaccgttgcgcctgccggtggcgaagcgtttgaagcgcgctttattgaagcgatggacgacgatttcaacaccccggaagcctattccgtactgtttgatatggcgcgtgaagtaaaccgtctgaaagcagaagatatggcagcggcgaatgcaatggcatctcacctgcgtaaactttccgctgtattgggcctgctggagcaagaaccggaagcgttcctgcaaagcggcgcgcaggcagacgacagcgaagtggctgagattgaagcgttaattcaacagcgtctggatgcccgtaaagcgaaagactgggcggcggcggatgcggcgcgtgatcgtcttaacgagatggggatcgtgctggaagatggcccgcaagggaccacctggcgtcgtaagtaattgcgctattgccggatgcgagttttcgcatccggttatcgtctgcgccaccacaacattcccatcagtagcatccccggcaaccacacccacatcaattcagaaataatcacctgatgcccgtacggcgtggtgtaacgagacaatgcaaacggcgcgacttttatcacctgccagggagcgaaaaagcgttcatctgaccacggccacagccagccaacgcctttaccgccagtggttaccgaatccagcaagctgtgcgatagcaacgagacggttaaaaacagccagcagcgaatcagcccagccctgaaccatcggcgtccaataaacacacataacagcgggacaacaaacgcaaacaccagcgaatgggtaaacccgcgatgaccaaaaacattgccgtaagcaacgccaaatttaaacgacaatacgtcggcgtcgggcagcatcgccaggatgattccggcaaataacagacgcggagggatgactttcgaacccaaccctaaaccaatgcataggggaacggcggcgtgcgtaataacggttggcatgatggtcgcttcggcaaaatgtcgatgctatcagcatggatgaacggggcgtagagggcaaaagtctgaaaagagaaccggcctgttgatacaggccgggaaagggatcaggcaacaacctgtacgctgtgacctgcaaaactcactgtctgaccggcgacgattttgcagcgtttgcgcgtttcaaccgcaccgtcgactttcacctggccttcggcaatcgcgattttcgcctgcgcgccgctttcgctccagccttccagtttcagcaagtcgcacagctcaacgtgcggatgtttacctaaagaaaatgtcgccatgttactcatcctgtggatcatgatattcaacgcacgcctgtagcgtgttttcaatcagcgtggcaaccgtcatcgggccaacgccgccgggaacaggcgtaatgtatgaggcgcgtttagccgcgtcttcaaacacgacgtcgcccacaactttgccattttccagacggttgatgccgacatcaatcacaattgcgccttctttgatccagtcaccgggaataaagcctggcttgccaacggcaacgatcaatagatcggcattttctacgtgatgacgcagatttttagtgaagcggtgagtcactgtagtggtgcaacctgccagcagcagttccatgctcatcgggcggccaacgatattcgatgcgccaatcaccacggcgttgaggccgaaggtatcaatgttgtaacgctcaagcagcgtgacgataccgcgcggggtgcagggacgcagacgcggcgcgcgctggcacagacgaccgacgttgtaaggatggaaaccgtccacgtctttgtccggatgaatacgttccagcactttgacgttatcaatacccgccggtaacggcagttgaaccagaatgccatcgatggtgttgtcggcattcagcgtatcgataagctccagcagctccgcttcgctggtggtttccgggaggtcataagagcgggagacgaacccgacttcttcacaagccttgcgtttgcttgcgacataaatttgcgatgcagggttactacccaccagcacaacggccagtcctggtgcccgcagtccggctgcaatacgcgcctgaactttttgagcaacttcagagcgcacctgctgcgcaatcgttttaccgtcaataatctttgctgccatcagagagaggattccatctgttacgtagatcgaaggggatgcgcctattttgtcagaagcggggcgcgctgtcaggtttcgtttcagatttatcgcgtgaagcgacctcttgcgaaggtgaggcgcaccgtcgctgagactgaaagcttcatttttcgtccatgatggcgttgtaaatctggaactgatttatttccttgtctaaggattaagataatttaagaaatacctgacaatataaaaagaattttcagcctggtaatttaccgcttcaggtctatatttgtgttgaatatattttgcgcggaagtattcatctaacggggctctctattttttagaatagagtgcatattttcaattaagacattcttagaggataaaaaggaatttactactatcagtgtcttaaataaagtaatcggttatatacggatgtggagtcgataaatgagattgaaggaatatatatgaaattaagatttatttcgtctgcgctggctgccgcactattcgccgctacgggtagttatgctgccgttgtagatggcggtacaattcactttgaaggcgaactggtgaatgctgcctgttcagtgaatactgactcggcagaccaggttgtcacactcggtcaatatcgtaccgatattttcaatgctgttggtaatacctctgcattaattccattcaccattcagttgaacgactgcgatcctgttgttgccgctaatgctgccgttgcattttctggtcaggctgatgcaatcaatgataatttattggccattgcatccagtaccaatacaacaacagcaacgggtgtcggtattgaaatacttgataatacatccgcaattctcaaacctgatgggaatagcttctcaaccaaccagaacttgatccccgggaccaacgttcttcatttttctgcacgttataaaggcaccggtacaagtgcatcagcagggcaagcaaatgctgacgcgacttttattatgagatatgaataatcaaaaccacgttgttttgaattatatatcacgtcttataacaaagtaatgtaccggttgtctgaagcggtatggtggcaatgtaaatcgaaatcatgttcactttgtatcatgccgctttattaaatgaaaagggaatgatgtgttgtaagaaaccaaagcaatcatttctttatattccttatttttgccgtcaggaatacacaaggcgtattaactatgatgactaaaataaagttattgatgctcattatattttatttaatcatttcggccagcgcccatgctgccggagggatcgcattaggtgccacgcgtattatttatcccgctgatgctaaacagactgcggtatggattagaaatagccataccaatgagcgctttctggtcaattcgtggattgaaaacagcagcggtgtaaaagaaaagtcattcatcattacaccgccactgtttgttagtgaacccaaaagcgaaaatactttgcgtattatttacaccggtccaccgctggcagcagatcgtgagtctctgttctggatgaatgttaagacgatcccttcggtagataaaaatgcattgaacggcaggaatgttttgcaactggcgattttatcgcgcatgaaattatttctccgtccaattcaattacaagaattacccgcagaagcgccggacacactcaagttttcgcgatccggtaactatatcaatgttcataatccatcacctttttatgtcaccctggttaacttacaagtgggcagccaaaagttggggaatgctatggctgcacccagagttaattcacaaattcccttaccctcaggagtgcagggaaagctgaaatttcagaccgttaatgattatggttcagtaactccggtcagagaagtgaacttaaactaaccgaatcatctgacaatatcagagctaattatgaaaatacccactactacggatattccgcagaggtatacctggtgtctggccggaatttgttattcatctcttgccattttaccctcctttttaagctatgcggaaagttatttcaacccggcatttttattagagaatggcacatccgttgctgatttatcgcgctttgagagaggtaatcatcaacctgcgggcgtgtatcgggtggatctctggcgtaatgatgagttcattggttcgcaggatatcgtatttgaatcgacaacagaaaatacaggtgataaatcaggtgggttaatgccctgttttaaccaggtacttcttgaacgaattggccttaatagcagtgcatttcccgagttagcccagcagcaaaacaataaatgcatcaatttactgaaagctgtacctgatgccacaattaactttgattttgcagcgatgcgcctgaacatcactattcctcagatagcgttgttgagtagcgctcacggttacattccgcctgaagagtgggatgaaggtattcctgctttactcctgaattataatttcaccggtaacagaggtaatggtaacgatagctatttttttagtgagctcagcgggattaatattggcccgtggcgtttacgcaacaatggttcctggaactattttcgcggaaatggatatcattcagaacagtggaataatattggcacctgggtacagcgcgccattattccgctgaaaagtgaactggtaatgggagacggcaatacaggaagtgatattttcgatggcgttggatttcgtggtgtacggctttattcttctgataatatgtatcctgatagccagcaagggtttgccccaacggtacgtgggattgcccgtacggcggcccagctaacgattcggcaaaatggttttattatctatcaaagctatgtttcccccggcgcttttgaaattacagatttgcacccgacatcttcaaatggcgatctggacgtcaccatcgacgagcgcgatggcaatcagcagaattacacaattccgtattcaacagtgccaattttacaacgcgaagggcgtttcaaatttgacctgacggcgggcgattttcgtagcggtaatagtcagcaatcatcgcctttcttttttcagggtacggcactcggcggtttaccacaggaatttactgcctacggcgggacgcaattatctgccaattacaccgcctttttattagggctggggcgcaatctcgggaactggggcgcagtgtcgctggatgtaacgcatgcgcgcagtcagttagccgacgccagtcgtcatgagggggattctattcgcttcctctatgcgaaatcgatgaacaccttcggcaccaattttcagttaatgggttaccgctattcgacacaaggtttttatacccttgatgatgttgcgtatcgtcgaatggaggggtacgaatatgattacgacggtgagcatcgcgatgaaccgataatcgtgaattaccacaatttacgctttagccgtaaagaccgtttgcagttaaatgtttcacaatcacttaatgactttggctcgctttatatttctggtacccatcaaaaatactggaatacttcggattcagatacgtggtatcaggtggggtataccagcagctgggttggcatcagttattcgctctcattttcgtggaatgaatctgtagggatccccgataacgaacgtattgtcggacttaatgtttcagtgcctttcaatgttttgaccaaacgtcgctacacccgggaaaatgcgctcgaccgcgcttatgcctcctttaacgccaaccgtaacagcaacgggcaaaatagctggctggcaggtgtaggtgggaccttactggaaggccacaacctgagttatcacgtaagccagggtgatacctcgaataatgggtacacgggcagcgccacggcaaactggcaggccgcttacggtacgctggggggcgggtataactacgaccgcgatcaacatgacgttaactggcagctgtctggcggtgtggtcgggcatgaaaatggcataacgctgagccagcctttaggggataccaatgttttgattaaagcgcctggcgcaggcggtgtacgcattgaaaatcaaactggcattttaaccgactggcgcggctatgcggtgatgctgtatgccacggtttatcggtataaccgtatcgcgcttgataccaatacgatggggaattccatcgatgttgaaaaaaatattagcagcgttgtgccgacgcaaggcgcgttggttcgtgccaattttgatacccgcataggcgtgcgggcgctcattaccgttacccagggcggaaaaccggtgccgtttggatcactggtacgggaaaacagtaccggaataaccagtatggtgggtgatgacgggcaagtttatttaagtggtgcgccattgtctggtgaattactggttcagtggggagacggcgcgaactcacgctgcattgcgcactatgtattgccgaagcaaagcttacagcaagccgtcactgttatttcggcagtttgcacacatcctggctcataaaggaaattatcaataagataatctgcagattattattggcgatggcatgtttgtgtctggcaaacatatcctgggctactgtttgtgcaaatagtactggcgtagcagaagatgaacactatgatctctcaaatatctttaatagcaccaataaccagccagggcagattgttgttttaccggaaaaatccggctgggtaggtgtctcagcaatttgtccacccggtacgctggtgaattatacataccgtagttatgtcaccaactttattgttcaggaaactatcgataattataaatatatgcaattacatgattatctattaggtgcgatgagtctggttgatagtgtgatggatattcagttccccccgcaaaattatattcggatgggaacagatcctaacgtttcgcaaaaccttccattcggggtgatggattctcgtttaatatttcgtttaaaggttattcgtccctttattaacatggtggagatccccagacaggtgatgtttaccgtgtatgtgacatcaacgccttacgatccgttggttacacctgtttataccattagttttggtggccgggttgaagtaccgcaaaactgcgaattaaatgccgggcagattgttgaatttgattttggtgatatcggcgcatcgttatttagtgcggcagggccgggtaatcgacctgctggtgtcatgccgcaaaccaagagcattgcggtcaaatgtacgaatgttgctgcgcaggcttatttaacaatgcgtctggaagccagtgccgtttctggtcaggcgatggtgtcggacaatcaggatttaggttttattgtcgccgatcagaacgatacgccgatcacgcctaacgatctcaatagcgttattcctttccgtctggatgcagctgcggcagccaatgtcacacttcgcgcctggcctatcagtattaccggtcaaaaaccgaccgaagggccgtttagcgcgctggggtatttacgcgtcgattatcaatgaggtacggagaatgagaagagtactctttagctgtttctgcgggctactgtggagttccagtggatgggcagttgaccctttaggaacgattaatatcaatttgcacggtaacgttgttgatttctcctgtaccgtaaacacagcggatattgataagacggtagatttaggcagatggcctacgacacaactactgaacgctggcgataccacggcactcgtcccttttagcctgcggctggagggatgtcctccgggttcagttgcgattttatttacgggaacgccggcatccgataccaacctgctggctctggatgatcccgcaatggcacaaaccgtcgccatcgaattacgtaatagcgatcgctcccggctcgcactgggggaggcgagcccgactgaggaagtagatgcaaatggcaatgtcacactaaacttttttgccaattatcgagcgttagccagcggtgttcggccaggtgtggcgaaagcggatgcgatatttatgatcaattataattaatattatattaattcgtataatttggcgtagtcgataagctctacaattgaatgcaaacctagcttgccataaatattagatttatgcgcactaactgttttattgctaagtaataacttatcggcaatttctttattagataatccgctaaccagataacgtaatatggtcacttcacgattagatagcacagtgaccgttgaactattcgtactacatttattgctttttatatagttaagcgtttcgctgggaaaaaacgtgtatccggagaggatcatctgaacggcatgaaaaatatcattctgatcattgcatttactgacaaaaccgttagcaccagcttgtatcgctctgccagcataaaagcattctgatttcgatgataaaaataacactttcactgtgctctggatttgtttgatccttttcaggaaggtaaaaccgtctgttccgggcaagtctatatccataatgattaaatcaacaggacgggttcggagataatcgatggttatgcgataatcatccgttttcaggacaatctgcaattcactgtttttttgcaacagaacttcaatagacattctgatgataggatgagtatccataatgatcaccgacgttggtttcatagttaccagtctcataggagcggacaattttccgttaggtcgggaaattgtactttgatacatgaaaatacgggttttcttgattcagacgcgcagcggtgtgcgtttgtttgccgctatagcgaaataaatcagaaaatcagacgcggtcgttcacttgttcagcaaccagatcaaaagccattgactcagcaagggttgaccgtataattcacgcgattacaccgcattgcggtatcaacgcgcccttagctcagttggatagagcaacgaccttctaagtcgtgggccgcaggttcgaatcctgcagggcgcgccattacaattcaatcagttacgccttctttatatcctccataatttcagagtgggacatatttgggacattatcaccaaaaatgtcgtctattttcctcgcatgctctgtcaaatgattaggcgcaaggtgagcatacctacgaaccatttctatggactcccatccgcccatttcctgaagcactgataatgggacgcctgactgaatcagccagcttgcccaggtgtgtctgaggtcatggaaacggaaatcttcaattcctgcacgacgacaagctgatagccatgatgtcttgctgtcgatgcgcatcttcctgaccgcaggcgttgatgttccatctgctcgcttagccgccttggtatgtacaaacacccatttgtgatgcttgcctatttgatcacgcaacactttacaggcggtatcgttcagcgccacaccaatggcgcggtttgatttgctctcttctggattcacccaggcaactcgtcgctgcatgtcgatttgttgccattccagatttatgatgttcgactttctcagaccagttgccagcgcaaacttgacgacagatttcagtggttcggggcactcatcaataaggcgttttgcttcctccttttccagccatctgactcgcttgtttctgaccgctggtatcttgatgacaggcgctttttccagccacttccagtcgcgttctgcagcacggagaatggcctttatcatggcaagatgctttgcctttgtctgagttgatactggctttggttcataaacaggcagttctttacctttcctgatggcggcctgaactttctgtttccatatttctttcgtctttctgttatgcattctgcttacagcagagtaaatctttgcctccgagatatctttaagccttataccctcaaaatgttcaagccagaactcaatccggcttttatctgaatcgagagattttttatcagctttttcctcaagccatcttaggcaggcctcttcaaaagtgacatcaggtaaatcccctagcttttctactcgccagagttctgcttttcgcttgtcgtgcaactcctgagcttgccgtttgtcctttgtgccaagagattccttaattcgtttcccgcccgggagcgaatacgaggcataccatatttcatttctgcggaagagtgacattttctttcctctgttatgccatcacccgcgctcacctggacagtatgcagcggagactgaagcgccgcaatgcaggcttgccgtgttgtgaggtacccggatattatcgtgaggatgcgtcatcgccattgctccccaaatacaaaaccaatttcagccagtgcctcgtccattttttcgatgaactccggcaccatctcgtcaaaactcgccatgtacttttcattccgctcaatcacgacataatgcaggccttcacgcttcatgcgcgggtcatagttggcaaagtaccaggcatcttttcgcgtcacccacatgctgtactgcacctgggccatgtaagccgattttattgcctcgaaaccaccgagccggaatttcatgaaatcccgggaggtacgagtattgccggaagcgtggcctgtatccggatgcagagtcttatccgtggaaatcgaacgcgcattactggttggttaccaacttgtaccagaacatgcgggccaatgcgctggctgacgcggaattacggcgcaaggctgccgatgaactgacctgtatgacagcgcgaattaaccgtggtgagacgatacctgaaccagtaaaacaacttcctgttatgggcggtagacctctaaatcgtgcacaggctctggcgaagatcgcagaaattaaagctaagttcggactgaaaggagcaagtgtatgacgggcaaagaggcaattattcattacctggggacgcataagagcttctgtgcacaggacgttgccgcggtaacaggcgcaaccgtaatctgatcttacccagcaatagtggacacgcggctaagtgagtaaactctcagtcagaggtgactcacatgacaaaaacagtatcaaccagtaaaaaaccccgtaaacagcattcgcctgaatttcgcagtgaagccctgaagcttgctgaacgcatcggtgttactgccgcagcccgtgaactcagcctgtatgaatcacaactctacaactggcgcagtaaacagcaaaatcagcagacgtcttctgaacgtgaactggagatgtctaccgagattgcacgtctcaaacgccagctggcagaacgggatgaagagctggctatcctccaaaaggccgcgacatacttcgcgaagcgcctgaaatgaagtatgtctttattgaaaaacatcaggctgagttcagcatcaaagcaatgtgccgcgtgctccgggtggcccgcagcggctggtatacgtggtgtcagcggcggacaaggataagcacgcgtcagcagttccgccaacactgcgacagcgttgtcctcgcggcttttacccggtcaaaacagcgttacggtgccccacgcctgacggatgaactgcgtgctcagggttacccctttaacgtaaaaaccgtggcggcaagcctgcgccgtcagggactgagggcaaaggcctcccggaagttcagcccggtcagctaccgcgcacacggcctgcctgtgtcagaaaatctgttggagcaggatttttacgccagtggcccgaaccagaagtgggcaggagacatcacgtacttacgtacagatgaaggctggctgtatctggcagtggtcattgacctgtggtcacgtgccgttattggctggtcaatgtcgccacgcatgacggcgcaactggcctgcgatgccctgcagatggcgctgtggcggcgtaagaggccccggaacgttatcgttcacacggaccgtggaggccagtactgttcagcagattatcaggcgcaactgaagcggcataatctgcgtggaagtatgagcgcaaaaggttgctgctacgataatgcctgcgtggaaagcttctttcattcgctgaaagtggaatgtatccatggagaacactttatcagccgggaaataatgcgggcaacggtgtttaattatatcgaatgtgattacaatcggtggcggcggcacagttggtgtggcggcctcagtccggaacaatttgaaaacaagaacctcgcttaggcctgtgtccatattacgtgggtaggatcaaccagcataaatcaggctgcggctaaaatggcgcgggcaggaatcctggtcgttgatggtaaggtctggcgaacggtgtattaccggttcgctaccagagaagaatgggaaggaaaggtgagcacgaatctgatttttaaggagtgtcgccagagtgccgcgatgaaacgggtattgagggtatataaaagaacatcaatgggaacacaatgatgaaacaggtgagttgagttcaaactgtagtacaattctctccagtttgaacaggaaagaatatgctatgaacccttatatttatcttggtggtgcaatacttgcagaggtcattggtacaaccttaatgaagttttcagaaggttttacacggttatggccatctgttggtacaattatttgttattgtgcatcattctggttattagctcagacgctggcttatattcctacagggattgcttatgctatctggtcaggagtcggtattgtcctgattagcttactgtcatggggatttttcggccaacggctggacctgccagccattataggcatgatgttgatttgtgccggtgtgttgattattaatttattgtcacgaagcacaccacattaaaataatttgtttctaaacgactaaaatatggaggctcttatatttatatgagcctcgttttatgctttttgttaatgtctttattttttatgtattcttttgtgctttcaagattatggcgtaagaaaattgcaatacgattattgttgtatattcaagataatgtgaccttaattgtctttttaaataaaaaataaacaaaaattatatcccaccactaaggtttataaaagcatacgttagcaggtgtcaccatgaaaaaagccatagcatatatgcgattttcatcaccaggtcagatgtctggcgactcattaaaccgacagagaagacttattgctgaatggttaaaggtaaatagtgattattatcttgataccataacatatgaagatttaggattaagtgcattcaaaggaaagcatgcacaatcaggagctttttcggaatttttagatgctatagagcatggttatatattgccaggaactacattgttagttgaaagtctggacagactttcaagagaaaaagtcggtgaagcgattgaacgtctgaaattgattttgaatcacggtattgatgttataactctttgcgacaatacagtctataatattgactctttgaatgagccatattcattaataaaagccatacttatagcacaaagggcaaatgaagaaagcgagataaagtcaagtcgggttaaattatcatggaagaaaaaacggcaggatgcactggaatcaggtacgattatgacggcgtcttgtccgagatggctctccttagatgacaaaagaacggcttttgttccagaccccgacagggtgaaaactattgagctaatttttaaactcaggatggaaaggcgctcattgaatgcaatagccaagtatttaaatgatcatgctgtaaagaatttctcaggaaaagaaagtgcatggggaccttctgtaattgaaaaattattagcgaataaagctctgataggtatttgcgtaccttcatatcgtgcaagagggaaagggataagtgaaatcgctggctattatcccagagtcatatcagatgatttgttttacgctgtacaggaaattcggttggcaccttttggtattagcaatagtagcaagaatcctatgctaataaatctacttcgaacagttatgaagtgtgaggcttgtggtaataccatgattgttcatgcggtatctggaagtttgcatggctattatgtttgtccgatgagaagattacatcgatgtgacaggccatcaataaaaagagatttggttgattataatatcattaatgaattgctttttaattgtagcaaaattcaaccagttgaaaacaagaaagatgctaatgaaactttagagttaaaaattattgagcttcagatgaaaattaataatttaatcgttgcattgtctgtcgcgcctgaagttaccgctatagcagagaaaataagactattagataaggaattacgaagggcttcggtatcattgaaaactttgaagagtaaaggtgtaaattcattcagtgatttttatgctattgacttaaccagtaaaaatggacgagagttatgccgtacacttgcctataaaacattcgaaaaaatcataattaatacggataataaaacctgtgatatctattttatgaatggcattgtttttaaacactatcctttaatgaaagtaatatccgcccagcaggcgataagtgctctcaaatatatggttgatggtgagatttatttctaaataatgatctcggattttaagttatgctatggtgataaagtgcaagacagaattaattatctttgacgaaacttaatgggtaattactttgtttgctcccacaagcgagttttgtacggctgtattggggtagtaaatgagctatacaatcttaatcatttgttaggtgagaactcttggtcgcagattcaaatactgaaaatacgtgacaaattattatgagcaaaatggtgtatgtcacgtattttgaatggtaggttaaaaaataacaccgactttcgtaggtgttactaataataaagcagagtttttagatagtatcaatgtgctttgtgtatattgtggcaaataattgggttgggggtacaattgtgattgcttttgcatgaacattgcgcctttatgcataatgagataaaggaatatcaaataaaataacgataggtcataacaaagaggtttttatgaaaacacttatcgtttcaactgtattggcattcataacattttctgcgcaggctgcagcatttcaggtcactagtaatgaaataaaaacaggagagcaacttacaacgtctcatgtcttttctggatttgggtgtgaaggtggtaatacatcgccctcattaacctggtctggtgttcctgaaggtaccaaaagctttgccgtaactgtatatgatccagatgcacctacaggcagtggttggtggcattggactgttgttaatattccagcaacagtaacatatttgcccgttgatgcagggagacgtgatggaacaaaactgccgactggtgctgttcaaggccgaaatgattttggctatgctgggtttggtggcgcatgtcctcctaaaggagataaaccacatcattaccagtttaaagtatgggctctaaaaactgaaaagattcctgtagattctaactccagcggagcgttagttggttatatgcttaatgctaataaaatcgcaaccgctgagataacaccagtttatgagataaagtagggtgagagtatgctggcaagaggtaagactaacttaaagatcgaagaaatacggatgcataaacatcatgagattcatagggttaagcctcttatgccagctttgtgtcgtatccgtcagggaaagaaagttatcaattgggagacgcatactttaactgttgataataatcaaataatattatttccttgtggttatgaattttatattgagaattatcctgaagcagggctttatcttgcagaaatgctttacttacccattgatttaattgagagtttccaaaaactttatacggtaactgatcaaatacgtaacaaaacaagtttctttttacctcagaatcctgagttaatatattgttgggagcaactaaaaacatctgtttcccgaggcttctcaactaaaattcaggagcacttagcaatgggcgttctactttcgttaggagtgaatcatgttaatcatttacttttatcatatagtaaacaatcattgataagtcgttgttataacctgctgctatccgaacccggcacaaaatggacagcaaacaaggttgctcgatatctctacatttctgtttctacattacatcgccgtctagcaagcgagggggtaagtttccaaagtatactggacgatgtgaggttaaataatgcgttgtctgctatacaaacgacggtaaaacctataagcgagattgccagagaaaatggttataagtgtccttctcgttttactgaaagatttcataatcgttttaatataacaccaagagagataagaaaagcttccagagagtaaaagtgttttaagaaggagcaattctatcgattttgattttgggaaatcaacacggcataattatgtcaccggagcctgaacaactccggtgacttctgcgctaaacggggacgtttatgcgcacatacaatccaaactctcttctcccttcacagatgcagaaatgcacctgcaattctttgcatctagcgtttgacctctgcggaggggaagcgtgaacctctcacaagacggcatcaaattacatcgcggcaacttcaccgctatcggtcggcagatccagccttatctggaggagggcaaatgctttcgcatggtgcttaaaccgtggcgtgagaaacgcagtctttcccagaatgcactcagccacatgtggtacagcgaaatcagtgaatacctcatcagcaggggtaaaacgttcgccactccagcttgggtaaaagatgctctcaaacacacatatctcggttatgaaaccaaagacctggttgatgtcgtaaccggtgatatcaccactatccagtcgttacgccatacctccgatcttgataccggagagatgtatgtcttcctgtgtaaggttgaagcctgggcgatgaatattggttgccacctgactattccacagagctgcgagttccagctgctgcgcgacaagcaggaggcgtaatggctacaccgcttattcgtgtcatgaacggacacatctacagagtaccaaatcgtcgtaagcgtaaacctgagctgaagccatccgaaataccaacactgctcggatataccgccagcttggttgataaaaaatggttgcgactggcagcaaggaggagtcatggctgatttgagaaaagcagcgcgtggtcgggaatgccaggtaagaatccctggcgtatgtaatggcaaccctgaaacgtctgtactggcacatatccggctgactggattgtgcggcaccggtacgaaaccgccagacctgattgccaccattgcatgttctgcctgccacgacgaaatcgaccgccgcacgcattttgttgacgctggatatgcaaaagaatgcgcgctggaaggtatggcgagaacacaggttatctggctgaaagagggggttattaaggcgtgaatacctacagcatcacattaccctggcctccgagcaataatcgctattaccgccataatcgcgggcgcacgcacgtcagcgcagaggggcaggcataccgcgataacgtcgcccgaatcattaaaaacgcaatgctggatatcggcctggctatgcctgtgaaaatccgcattgagtgccacatgccggatcgccgtcgccgtgacctggataatctgcaaaaagccgcttttgacgcactcactaaagcaggtttctggctggatgatgctcaggtcgttgattaccgcgttgtgaagatgcctgttaccaaaggtgggaggctggaactgaccatcaccgaaatggggaatgaatgatgtttgagtttaatatggcagaacttcttcgccaccgctgggggcgtctgcgcttatatcgtttccccggttctgttttgaccgattaccgaatactgaagaattacgccaaaaccctgacaggagcaggagtatgaagtcagagataacaatcaactaatactgttttgttgatttttgcttgtaattggcgttctggtctgatttttgtggagtaagttgatgcgtgatattcagatggttcttgagcgttggggagcgtgggcggctaataatcatgaagatgtgacctggtcgtccattgccgccggttttaagggattaattacttcaaaagtaaaatctcgcccgcaatgttgtgacgatgacgcgatgatcatttgcgggtgcatggcccgtctgaaaaagaacaacagcgatttgcacgatttattagtagattattatgtagtcggtatgacattcatgtcactggcaggtaagcattgctgctctgatggttatatcgggaaaaggttacagaaggctgagggcataattgaagggatgttaatggcattagatatccggttagagatggatatcgttgttaataactctaattaatatgccaattgtttactaaaaattattaaaaatggggcgttgagacgcccccaaaaataaagggtaatatataacagaaggtttatatagttagaagcaaggttgtgcttctaaaggaagtggcttgagggagccacttatatgttggggaggcaacgcctcccgcaacatatctttttcgtaatcagattagaactggtaaaccagacctacagcaacgatgtcatcagtgcttacaccgagtgctttagggaaggtgcgaataagcggggaaattcttctcggctgactcagtcatttcatttcttcatgtttgagccgattttttctcccgtaaatgccttgaatcagcctatttagaccgtttcttcgccatttaaggcgttatccccagtttttagtgagatctctcccactgacgtatcatttggtccgcccgaaacaggttggccagcgtgaataacatcgccagttggttatcgtttttcagcaaccccttgtatctggctttcacgaagccgaactgtcgcttgatgatgcgaaatgggtgctccaccctggcccggatgctggctttcatgtattcgatgttgatggccgttttgttcttgcgtggatgctgtttcaaggttcttaccttgccggggcgctcggcgatcagccagtccacatccacctcggccagctcctcgcgctgtggcgccccttggtagccggcatcggctgagacaaattgctcctctccatgcagcagattacccagctgattgaggtcatgctcgttggccgcggtggtgaccaggctgtgggtcaggccactcttggcatcgacaccaatgtgggccttcatgccaaagtgccactgattgcctttcttggtctgatgcatctccggatcgcgttgctgctctttgttcttggtcgagctgggtgcctcaatgatggtggcatcgaccaaggtgccttgagtcatcatgacgcctgcttcggccagccagcgattgatggtcttgaacaattggcgggccagttgatgctgctccagcaggtggcggaaattcatgatggtggtgcggtccggcaaggcgctatccagggataaccgggcaaacagacgcatggaggcgatttcgtacagagcatcttccatcgcgccatcgctcaggttgtaccaatgctgcatgcagtgaatgcgtagcatggtttccagcggataaggtcgccggccattaccagccttggggtaaaacggctcgatgacttccaccatgttttgccatggcagaatctgctccatgcgggacaagaaaatctcttttctggtctgacggcgcttactgctgaattcactgtcggcgaaggtaagttgatgactcatgatgaaccctgttctatggctccagatgacaaacatgatctcatatcagggacttgttcgcaccttccttagtgaagtcatttttgtcaagcaggttgattttgtaatcaacgaaagtagacatatttttgttgaagtaataggttgcacctacatcaacatatttgactaagtcctgatcgccccatactccaagatccttacctttagattgcaggtaagcaacggacggacgcagaccgaaatcgaactgatattgtgcaacagcttcgaagttttgggctttattagcaacgaagtgatcagcaaatacagtcatattctgggtttcagaataggtagtggccaggtaaatgttgttagcgtcatatttcagacctgcggcccaaacttctgcatttttaccggaagcaaatacttcaggaagaactttccctgcattaacttgagtgtcggtacgatcagatttcgcataagttgcaccgataccgaatccttcgtattcataggtagcagagaaaccgaagccatcaccgttaccttcagtgtagttatcgaaatcgctacgatcgtttttgccttggtactgagcagcaaagttcagaccatcaaccagaccaaagaagtcgttgttacgataggttgcaacaccagttgcacgttgagtcatgaacacgtcggtttgagtccaagtgtcaccaccgaattctggcaggacgtcagtccacgcaccgatgtcgtatgctacaccgtagttacggccgtaatcgatggagccgtagtcaccgaatttcaggccagcgaaggcaagacgggttttatctttggaggaaccttgagattcagcgcggttgcctttgaattcatattcccactgaccgaaaccagtcagttgatcgttgatttgggtttcacctttgaagccaagacgggcataagtagtatcaccatcatctgcatcattagaggagaagtagtgcttagcattaactttcccgtacagatccagcttgttactgtctttattataaatttcagctgcctgagcagacatcgccattagtactgatgcagctacagcagaaattgccactgttaattttttcatcgtgagccctttttttgaactattattaaaaaatgatgtcactgcgcgataaatattcatctaatcaatgtgattatttcaagatgtaagttttggtttctcgtttgatttgtgaagtagatctctatttttatctgaacttttttctatcgaatcctattcatggctcttggctgaataaaaataaatctattagccaatttatattaacggctgttatttataagtgctctataatttgaaggttcaatttaaaccggctaaaaataacactggaaattattttttggttatttgttgagatttgcttatgtatttgtagtggtgttttcaatactcggtagcattctctcaaatatcatttagtggtttacgtacgtaaaaaattggttatgctgttaagagtggttacttcgtcacacagcttaaacccgccgtcgagcgggtttttccattttttgagtctcgatattagctgataacccaatacctgagttattcactgactccgagtctgttacgtttcgtagtattccctcaatttacacccgctttgtctgcgaggtggggttatgaaatccatggataagttaacaacgggtgtcgcctatggcacctcagcaggtagtgccgggtactggtttttacagctgctagataaagtcactccctcacagtgggcagcaataggtgtgctgggtagcctggtatttggcctgctgacgtacctgacaaacctttatttcaagattaaagaagataagcgcaaggctgcgagaggtgaataatgcctccatcattacgaaaagccgttgctgctgctattggtggcggagcaattgctatagcatcagtgttaatcactggcccaagtggtaacgatggtctggaaggtgtcagctacataccatacaaagatattgttggtgtatggactgtatgtcacggacacaccggaaaagacatcatgctcggtaaaacgtataccaaagcagaatgcaaagcactcttgaataaagaccttgccactgtcgccagacaaattaacccgtatatcaaagtcgatataccggaaacaacgcgcggcgctctttactcattcgtttacaacgtgggtgctggcaattttagaacatcgacgcttcttcgcaaaataaaccagggcgatatcaaaggcgcatgtgatcagctgcgtcgctggacatacgctggcggtaagcaatggaaaggcctgatgactcgtcgtgagattgagcgtgaagtctgtttgtgggggcaacagtgagcagagtaaccgcgattatatccgctctgattatctgcatcatcgtcagcctgtcatgggcggtcaatcattaccgtgataacgcaatcgcctacaaagtccagcgcgacaaaaatgccagagaactgaagctagcgaacgcggcaattactgacatgcagatgcgtcagcgtgatgttgctgcgctcgatgcaaaatacacgaaggagttagctgatgcgaaagctgaaaatgatgctctgcgtgatgatgttgccgctggtcgtcgtcggttgcacatcaaagcagtctgtcagtcagtgcgtgaagccaccacggcctccggcgtggataatgcagcctccccccgactggcagacaccgctgaacgggattatttcaccctcagagagaggctgatcactatgcaaaaacaactggaaggaacccagaagtatattaatgagcagtgcagatagagctgaccatatcgatgggcaactcatgcaattattttgagcaatacacacgcgcttccagcggagtataaatgcctaaagtaataaaaccgagcaatccatttacgaatgtttgctgggtttctgttttaacaacattttctgcgccgccacaaattttagctgcatcgacagttttcttctgcccaattccagaaacgaagaaatgatgggtgatggtttcctttggtgctactgctgtctgtttgttttgaacagtaaatgtctgttgagcacatcctgtaataagcagggccagcgcagtagcgagtagcatttttttcatggtgttattcccgatgctttttgaagttcgcagaatcgtatgtgtagaaaattaaacaaaccctaaacaatgagttgaaatttcatattgttaatatttattaatgtatgccaggtgcgatgaatcgtcattgtattcccggattaactatgtccacagccctgacggggaacttctctgcgggagtgtccgggaataattaaaaacgatgcacacagggtttagcgcgtacatgtattgtattatgccaacaccccggtgctgacacggaagaaaccggacgttatgatttagcgtggaaagatttgtgtagtgttctgaatgctctcagtaaatagtaatgaattatcaaaggtatagtaatatcttttatgttcgtggatatttgtaatccatcggaaaactcctgctttagcaagattttccctgtattgctgaaatgtgatttctcttgatttcaacctatcataggacgtttctataagatgcgtatttcttgagaatttaacatttacaacctttttaagtccttttattaacacggtgttatcgttttctaacacaatgtgaatattatctgtggctagatagtaaatataatgtgagacattgtgacgttttagttcagaataaaacaattcacagtttaaatcttttcgcacttgatcgaatatttctttaaaaatggcaacctgagccattggtaaaaccttccatgtgatacgagggcgcgtagtttgcattatcgtttttatcgcttcaatctggtctgacctctttgtgttttgttgatgatttatgtcaaatattaggaatgttttcaattaatagtattggttgcgtaacaaagtgcggtcctgctggcattctggagggaaatacaaccgacagatgtatgtaaggccaacgtgctcaaaccttcatacagaaagatttgaagtaatattttaaccgctagatgaagagcaagcgcatggagcgacaaaatgaataaagaacaatctgctgatgatccctccgtggatctgattcgtgtaaaaaatatgcttaatagcaccatttctatgagttaccctgatgttgtaattgcatgtatagaacataaggtgtctctggaagcattcagggcaattgaggcagcgttggtgaagcacgataataatatgaaggattattccctggtggttgactgatcaccataactgctaatcattcaaactacttaacctgtgacagagccaacacgcagtctgtcactgtcaggaaagtggtaaaactgcaactcaattactgcaatgccctcgtaattaagtgaatttacaatatcgtcctgttcggagggaagaacgcgggatgttcattcttcatcacttttaattgatgtatatgctctcttttctgacgttagcctccgacggcaggcttcaatgacccaggctgagaaattcccggaccctttttgctcaagagcgatgttaatttgttcaatcatttggttaggaaagcggatgttgcgggttgttgttctgcgggttctgttcttagttgacatgaggttgccccgtattcagtgtcgctgatttgtattgtctgaagttgtttttacgttaagttgatgcagatcaattaatacgatacctgcgtcataattgattatttgacgtggtttgatggcgtagatgcacgttgtgacatgtagatgataattattatcattttgtgggtcctttccggcgatccgacaggttacggggcggcgacctcgcgggttttcgctatttatgaaaattttccggtttaaggtgtttccgttcttcttcgtcgtaacttaatgtatttatttaaaataccccctgaaaagaaaggaaacgacaggtgctgaaagcgagctttttggcctctgtcgtttcctttctctgtttttgtccgtggaatgtgcaatggaagtcaacaaaaagcagctggctgacattttcggtgcgagtatccgtaccattcagaactggcaggaacagggaatgcccgttctgcgaggcggtggcaagggtaatgaggtgctttatgactctgccgccgtcataaaatggtatgccgaaagggatgctgaaattgagaacgaaaagctgcgccgggaggttgaagaactgctgcaggccagcgagacagatctccagccagggactattgagtacgaacgccatcgacttacgcgtgcgcaggccgatgcacaggagctgaaaaatgccagagactccgctgaagtggtggaaaccgcattctgtactttcgtgctgtcgcggatcgcaggtgaaattgccagtattctcgacgggatccccctgtcggtgcagcggcgttttccggaactggaaaaccgacatgttgatttcctgaaacgggatatcatcaaagccatgaacaaagcagccgcgctggatgaactgataccggggttgctgagtgaatatatcgaacagtcaggttaacaggctgcggcattttgtccgcgccgggcttcgctcactgttcaggccggagccacagaccgccgttgaatgggcggatgctaattactatctcccgaaagaatccgcataccaggaagggcgctgggaaacactgccctttcagcgggccatcatgaatgcgatgggcagcgactacatccgtgaggtgaatgtggtgaagtctgcccgtgtcggttattccaaaatgctgctgggtgtttatgcctactttatagagcataagcagcgcaacacccttattccagctggcttcgtggctgttttcaacagtgatgagtcatcgtggcatctcgttgaagatcatcggggtaaaacggtttatgacgtagcgtcaggggacgcgttatttatttctgaactcggtccgttaccggaaaatgttacctggttatcgccggaaggggagtttcagaagtggaacggtacagcctgggtgaaagatgcagaagcagaaaaactgttccggattcgggaggcggaagaaacaaaaaacagcctgatgcaggtagccagtgagcatattgcgccacttcaggatgctgtagatctggaaatcgcaacggaggaagaaacctcattgctggaagcctggaaaaaatatcgggtgttgctgaaccgtgttgatacatcaactgcacctgatattgagtggcctacgaaccctgtcagggagtaatcattgggattatgccgcagcacgtcttaagcaagaacatgctgcggttggatgctatttttttcctgaagcggaaaacattactacagtaccttgaaccttggttttaacattctcgaaatgctctgagagtatatgtgttaagccttcttcggaatcttttgtgtttgaaaagatgcctttctgattgtaaatgcgcatcagtttttgaccgaagctattgtgcacaactccatcgccaagaattgtggctccgtatagagttccatcgtcagttaaggcctgcgccgcattgcgtattacacagctttttgtagatatatttccaggcaggcagtgaagaaggtaagacatggaaatggaatcaaattgaccatgtaacgccgcgggataaggttcaaaaacatcatggctaattttatgtttaatttttgattccccagcccttgtagatgccgcgttcaggctagcttcgttcaaatccattaaagatatcagactactctcaggtacgtgagtaaggtaaaacccagttccaacaccaatatccagatggttgttacctaaatgttccagaaagtgtggaagaaggtgttcctttgtaggacatccccatgcaagccgatttgatactcccaaaacccaccagtcataaagctttagggtaagtggtgtgtaaattctagccccatcatctgtgtttttttattaatttcaccatgttatagttttatttgtgaattaaatcaattatggcaatgaattacaaggggttaaatgctgccgcagcatagcgatattgaaatagcctggtatgcttcaatacagcaggagccgaatggctggaagaccgtcaccacacagttctacatccaggaattcagtgagtatattgcgccactgcaggatgctgtagatctggaaatcgcaacggaggaagaaagatcgttgctggaagcctgaaaaaagtatcgggtgctgctaaaccgtgtggacacttccgtagcaccagatatcgagtggcttattcaaccataataaacagtatgtatatcataggttattaattgtgagttttttcggtgtgttatttgtttgtttgatgttatgcttttgcgccccaaaaggttgtttagatgtattttatcaattgattttcaatatcgtttaataaagaaaaattaagcaagctggatgttggttttttgttaattgaatggttctaataatgtttttttactgttgttgaatgtgacttgataagaaatgcaagtaaaaatgatactctttttattttaaattcaaacggttgacatatatatagcaagaggtttcaggtgcgttgtagtgagtttatgttaataaaaagcatagtaagcgttgaaaaatgtaactttgaaataagttagaataaaaaacaacatacatataataatttaatcttaaatgaaatttattaaaatttgcaaactataattttgtgtataaaaatataaatgcacatcatcctgattatgattgtgtatttaattggttgttatttgactactatcaacttgttttaattttatgataggtgcaagatggattatgtttgctccgtagttttcatctgtcaatcatttgatttaattataaacaggagagttatctcgttcaaaaaaaattcattgtttattgtaagcgacaaaattagaagggagttaccagtatgcccctctaaactaagaattgttgatatagataagaaaacatgtttatccttttttatcgacgtgaataatgagctgcctggcaaatttactcttgataagaatggctatattgctgaagaggaacctccattatcgcttgttttttctctgtttgaagggattaaaatagcagactcacactccctttggttaaaagaaagactatgtatatccttacttgccatgttcaaaaaacgcgaaagtgtaaattcatttatactaacaaatataaatacatttacctgtaaaattactggaataatcagttttaatattgagcggcaatggcatttaaaagatattgcggaattgatttatacgagtgaaagtttaataaaaaaaagattaagggatgaaggaacgtcatttactgaaatattgagagatactaggatgaggtatgcaaaaaaactcataacttcaaactcttattctatcaatgtcgtagcccagaaatgtggctataacagtacttcatatttcatatgtgcatttaaagattattatggtgtcacgccatctcattattttgagaaaataatcggcgtcacagatggaataaacaaaacaattgactgataatgtttattacaagttgtctacatgttaattataatattatacagcgttttttttgatgtgatattctggaaccattaatttgtaattgggttgctgtcgcctattttatacatactataattgatggttttctatgtgatttagttaataaccttctgggtttattttaagggttaattgttacattgaaatggctagttattccccggggcgattttcacctcggggaaattttagttggcgttcttaaaatgtgtacttaagaccagcagtagtgatgaagttatagttttctatacctgctccatttttgctgtagtctgaagtgttattattgtgatcataaagtgaagtattaccttttttattcgtaacccgattccatgcgccttcaacataaacttttgcgttaggtgtgacgtaataacctgcattgactgcaacagaatagtaattttggtctttgaccttactgcgataagtgattctttttcccgggtcatagtgttcatcgttatcagatgattccacccagccgctgtatttaaatgtgccaccgagttcaaaatcttcataacgataacttccagtcaagccaatgtagggcattttaaaacgttgtttgtagccgattgctctttctccattcgggaaggagccgatatcatctctgaatccctcctcagaactgtagatataggaaccacctctggctgtaaagctataacggctttcctgatatccggccatgagtcccaggcggtaattgggttcgttgaggagccagcctttgatattcagatcaaattcgttggcataattgagttgtgtatcagggtgtctactttcatccgtccaggttccggggttactggaatccatccagtcctgatcgaccatattgccacctcggctgccgagagttgtccagccagcagccccgatagatatctggggcatcaaatcccaattaattgcacctttaataattgcagcgttattgaatttccagtcgagttgactgacttttcggcctccttcttcggctagataaacacgctcttttgtttttccgctcagagttccaagactaatgtccgcatttatgttgtcaggagtaaacgataaagtctcggtagaagcaaaagagctgatcgcaataggggttgtcaggactattcccagaagtttcgcccgcataaaagttctccattcaatcgttttaatgattgaatatgtattttttatatctaacttaatgagtcaattacatattgctccactgtttatattttgtttagtattgaatgattatcacaatgcgctatctgtttttggtttaattatctgttattgtttcatatttcggttttactgtgtggtttttttatgcttttgtggtgcttttatctatttaagtgccatgcctttagaggcatataagcgaaaatagcatgaggtttatcctcaattactatgttttttagtacaaaaaagagggacaaaactgagacacataaggcctcgcaatggcttgcaaggctttacatgttttgaggtagtgggacgtgtgagcgcagagatggcgcggtaagttgttgacttaaaatgtcgttctaggaacttctaagtcgtgggccgcaggttcgaatcctgcagggcgcgccatttcttcctcatttatgcccgtcttatccgtttccgctttgcccttcaccacatcactttttgtcgctgtttggcgagataattcaacggtgtcaggccgtaaaacgccttaaaaacagagataaagtacgacgtgctgctatagccacataattgcgccacctgagtgatatttttgttatccatcaataacatctgtacggcgtaacgcatacgacactctgtgacaatctggctatagctggtattttcgttttttaatttctttttgagcaggctggggcttaaacatagcgaactggcgacaattcgcagattccagtaatgctgaatatcgctttgaataatgcggcagacgctgtcgcggacgctgctgcgtaagatatacatcagtagggcaataaaccgcgattgctcaagaaagttagacaatacggtaaaaagcaatgcgcgcgtcaactccgcttcgcagggtctgctgggttgctgcttgctgtggttggcggctagccggaacacttccggtgtacggctatgacaagcgataaccggggttgccagccgcgaccagggctttacacaggttaagttcttatttaaaaacaacagataatcgttgatgatgttacggttgatgtgggtgattaatacgtgatttaacgttgagagttcaatgacgttattgttgcacgcgaaggcggccaggtagtttttcggaagggtaaacgtagcatggttattgacgcttacctctacctctttttcggtcaggatcaccacgcaaggttcactgctgctcaattgcatttcgcactcctcagatatcagaaactccgctcaaaggatctatgcttcctgcatgagtgatcggcccgttcgccgataacgatcttctttctttagcacgctttttagcaattaatcttgatggaattctgatgagagcgaaagaggtaagccaggtcgtacccgacttacctggaggagatttaatactcgagaatgccgtgcgcgacgggcaaatagcgcagagagaaatagagagtgtctttaccgcaagaggaacgtttcgctaacagcgaggcaatttctgcgtccggtttcggtttcgctgtaaaggttttgcctttgccggcgacaaaaagttcataaacaacgccgctggcaggggcgggactttggcaatcggcgctggcctgtaaataacgttcacgctgttcagcggtcagtttatccacgccgctgccatcctgtacccagacattaacgccggttgctttaacgtgttccagcagttggcgatagccatcgggcgacatgtttccggcgaaaaaactactgatataaaccggttttgctgaaacatcgctaatcagccgctgcgcgttgtttaaccatgttagcaaaggctgacgggcggcttcgctgcgccagttcaggtcgtcaatttccgcgctgatgtaccagccatccggcgttatgccaggcgcggcgctccataatctggcttgctggagatcggcagccagcaggcgattaagatagctttccagcgctgcggacgactgtttctggtgcataaaaaattccggatcggcgttcagcccgacaataagcttcagaccagcctgttgcgcagctgcggcccgcttaaacaataacgtgcgctgttctggctgggtaaatgcatcgccgtaacgggtccattgcaaaacaagggtatcgaagccttgcaaacgtaactgactcatcagcccctgccactgggtatcggtaacctgactatctcggttttgtggttgccagataatacctttcatcgcaaaggaaaaagggctgaccaaaagcagtgtcagcaatacgaaaatgaacttacgcatttaccagtgcactccaatggtgagaaacgcgttgttgcgctctccgttacgttgattaatcgccttaaaggtatgttgatactcgacgccgagactgactttgtgcggccaggcgtcgtagtgcgtctcgccggtccagatattccagcggaccccgactccgccaagctgcgcgccctgagtgcctttatcacgatagccgttgtcctgaacgtgagcgtaaggctcaatagtctgtccgttagctaccttctgatgccagctgacgcgataatctgccgtccacgcctgaatatcctggcggatatattgcgccgcatcgaggtacaggttttgggcaaaccagcctgaaccgttcgggtgccattcgtcgctgtatttgccgccattaaagaatgaggcgctggcgcgcagcatggtatcggatgcgccattttggccgttcagcggcaactgctgttcgacggcgatgaaaaagatctgatcgcgcagcggcttccagcgcagaccggtgccggacatcggatttttcaccggcatcatcaccccgttttctccggtatcggcaaagacgcggctataaactgagagcaggtcgccttccagcagcatattgcgtccgatgcggtactcggcttccagttgtccgtagctacgatagcttttccctggcgctgcgccgccgacattattgttagcggtactcattgcgccggaacgcaagccgatggaagaatcgaaactgaacgtccagcggcgaccgacctcctcatgcaaacggcggaaattgaagcgttgttgattttgttctggggtcagtggggttatcagcgcctgattatcaatgtcatcaatcaccagccgggcgtagtgctgcgtcgcaggcatgtcatccagacgctggttcacgtaggccagttgtcggatcagtgccggatcgtccggaagccctttatgcgccggttcgagcatttcccgcgactgtgcgatatcaccgctatcccacaaggcgtaaccaagcgctgcctgggtgttgctattattcggttccagttccagcgcggcgcgcaaatcactcaccgcggccgggacattatgacgttggcgataaattgtcgcccgcgcaacgtaagcgttggcagaaggcgcaatattgattgagcgcgtgagatcgttcagtgcgagttccggctgaccaggaatgtaacgttgcgcatgcagccaccagtagagggcattgcttcccagtccacgtttttctgcctgttgtagccagcgatcgcgagccgcaccatttcctgccgcctgggcggtattggcagcagcaagcagatcctcattgctcatgtcgtgaagactgattttctgccaggccgccagtgcggtggcgtagtcctcaacctgatacgcctgataggctaccgcacgatgttgccaggcgctcggttgtcgttgttcggcctgaagccatgcatacaacgccacaccgggtagcgtgtcccgataacactttgccagacggttccaggcggcggcatcgtaggaaggcgacatatcgcccagcaagcgaactattgccgggcaattatctgcaatacccggcaactgactttgccactgacgttgctccgccagcggtaagggtttcgataaaatcgccaccttcgccggcgttgccaggtaaggatgactttccagcagagacgccagtcgcgccattaaagtctggctgacacgcgcatcgccctggaaaggatagcgttgcagcaataaatcggcagcttcgcgtgactgctcgttctgcatcagttgccaggttagttgatccaggcgggtaagatttgccggttcttgctgatacagcaatcgtgccagacgcagagcttcagccttgttacgggtcgccacgctgacagcataacgctcctcaagcatttcattggcggggagggtggcgagcagtttttgcgctgcgtcgtactgaccttcttttaacagcaccggtagcgtcgcgccaacaacatactggcggttgtcggcaaactgtaccgtataattcgccaacgcctgaacggggttagcgctgtatttagataacagatagagccaacttttctcttgtgcgtccgtggtaaatagtggcttattttcaatgagataatgctggaggcgtgctttttcgccacgataagccagcgcggtcgcgtaagtaatatatgactgaggatcggtgaagatcccctgtgattgcagtgccaggatccgatcgtccagctgcccggcaagaagcacgtcaaaccactgacggcgttctgccgcgcttaatgtgttctgctggcgtgcttcattgtatagcgtatctgcctgggaccattgtttcaggtagattgcccgttgcagcagatcggttcgcagcgtttttccttccggcgatgcagcaaacgtcgcatcgttcagttgcgctctggcgacaggtaactgtgccagccgcagggcattctgcccgacttcactgcgacaacgcagggtcggcgcagcatcgcacgctttttgctgggcaagcagttcttcaactgtcgtaacgcttttcacttcaaccggaatagccgccagactgcgctcaagtcgggcatctcctgggtgacgtttcagttgatcctcaagcaacagccgcgcccggtcatcatgaccaaaatggcgataggcttccgcaaggtataaagtcagcggaatattatccggcacctgctggtgtatatattcaaattcgcggatggcggttgcttcgtcgttatttttctgtgccttcagcgctttatcgagacggggataaataacaaaatggcgataatcgctcagccccagctcttctgcgctggtgccgatattgtctgcgagtgcgctggtactcaataaagacgtcagcagtaaaccagaccatccgatgacgcgattaaggttattctccttcattttcggactccagttgcgcaacctgttctgtgtttaaacctgctttgagtaatagtgattgcatcgaaacttgtaattcgcgttgaattgtcaggacgcgatccaacgtttcctggctgataacgccttcggtgaccaaaaacttgccgagcggcagagaactgcgttcatggcgcaataacaacacgttaattgctgaacgattaatatgaccgagcgtggtcagtatttcggcgaacaggaactgatgcggcacatattgccgccagatttcaccggcctgctgttccgtgagccactgatgctgaaccgcattgtacaacattgcccgcggatcgtgaccgcgtcggcgtgcataccagtgacgtaaccctgtgacaatttgtccccgcagaacaatgacgtaacgcactttgcgtccgactttacgcgtcagggccgccagcgaaaccgggtcaataccatcttcactgccgacaattaactcgtcattttccagacgcagcggcagtaccgcataatgcagcgccacggaggccggcatttcggcaatcagcgaggaagggatctgccaggcatcgatggattcccacgccacgccgttttgctctgccagcgcctgtgccagctgctcggcgctaatcagcccctgcatcagcattgaaccgcccaggcgtagaccttcgacgcgattacgcagtgctgtatcgagttgttcttcagtgatgacctgattttccagcagaatttgacctaacgggcgcaacgagcgggtatcgccagtcacgctggggaagtcatgcgttgttttatcccacgccacgcgacgtggatcgccgtgttgaagtacctgttttagcgcgcgccagttggccatgaagttaatcaggttgccccagaaaagacgcaggacggaaagcagcccctgcgtcaggccgtagtagccagtaacgaaaatcacccgctgcacgatgcggttaaccatcaaaccaaagtttagccacagcagggtcattaaccatgcgctgccgctgaaaatagaaaggaaatgccaggcatcgggccacaaactttcatacgccagcaacagcaaaagctggatcatcaccagcatcgcgaggaagctgacaaagttactgattgcccctttgcggtcgcgccagagaaagtagttcagcgtcaggctggaggtccatttatgggttttaaagccttggaaaacaatgccgatgatccagcgggatttttgtcgaaccgcagtcgaaaaggtatcggggaaatattcgcgcacgcagatcatgtttgatgtccgcgcgtgctgtaaaaatttacgctgctcgcgttctttggcttcgtccaccaccggaaaacggacaaaaatttccgtcatacctttttctttcaggcggaagccaatgtcgtaatcttcagtaagactctgcacgtcgaaagcaataccgtcaccgtcagctaacagtgcggtcacggcgcggcggctgaaacaggtgccgacgcctgcgctgggcacttgtccggcgagggcttcacgcaccggaacatctttgccatgcagctctgaaaactcatcaatgtaagtcatgctggtgaagtgcgtccattcgcgttcgaacggatacaccgggatctgaatcagatctttacgctcgaccagatagttgaacagacgcaattccatcggtgaaatcacatcttcggcgtcatgcagaataaaaccagcaaaagcgaaattggcgctacgctcaaattgggtgatggcgtccagcacgttgttcagacagtcggctttgctggtggggccaggacgcgcgcagactaccttatgcacattcgggaagcgagcgcacacttcgtcaacatcacgctgagtatcggggtcgttggggtaggtgccaacaaagatatgatagttttcgtagtcgagcgtggtcgccgccagctcggccatattgccgatgacgcccgtttcattccacgccggaaccataatcgctaacggtttttcatctggtttatacagttcgcggtaactcattcgcgggtagcggcgataaacactcaacttgcgtttaatgcggcgtacccagtagacgacatcaataaaaaaatcgtccagcccgctgatgaacatgatgaccgctaacgttatcgcgattacttttaagccgtagagccaggtagcaaaaacatcaagaagccagtccacacaaaaaccttacattaacgctggttatgtttagggtggcgtatattaaggttttttatgaattgtgacagctttttaccattaataggtatgactattgcggcacgttatttttacactggttataaaagttgccgtttgctgaaggattaagcgggtaatgtgataacaaaccttgtcccccgcgcatccgacgttaccgcaaccgtgcctttatgcgcgacaacaatcgatttcactatcgccaggccaataccgctaccttcaccttttcgctggcgggaggggtcaacgcgatagaaacggtcaaacaatcgcggtaagtgctcgggcgcaatgggcgtaccggggttttcgacgataacttgcaccaggtgatcgaccgtctgacagcgcactacaattgtctctccggttggcgtataacgcagggcgttcgaaagcaggttgcttagcgcccgacgcagcatcagcggatcgcccgcgacctgacacttgtcgccaacaaaccgcaactccacgccgcgatcttccgctaacgcctcgaaaaaatcgaacactttgccgacttcatccgccaggttgagcattttcttttcggggattagctggttgttatcggcctgagcgagaaacagcatatcgctgaccattttcgccattcgcgtcagctcttcgagattagagtagagcacatcttccagctccttctggctgcgcgactggctgagggcgatttcggtttgcgttatgagattcgtaattggtgtgcgaatttcgtgagcgatatccgctgagaaattggactggcgggtaaagacatcctcaatacgctcgatcatatggttgaacgacagtaccagctgttccagctcaatgggcacggtctgcgggtcgaggcgaacgtcgagatctttcgaggtaatattctggatttgacggctgacgctgcggatcggcgcgtgacctttatgtaccgccaacagtacgataaagacgatcaggatgctgattaccgatgcggtcataataagtttattcatcaaatcatttatgtaatgaagatgaaaatcgatcgaaagcgcgatgtagagcgtataaatcggtttgccgtccaccaacgggccaaccggcaagttaatcatccgccagttgctgtgttccatatgcccgtgaccgtggcctggcatcatcatcgtcgggccggaaaggagatacacctcgccaccctgagcgtctttatcgggtatggcgtcacgcgtaaactcgcggatatccggcgcaccgggggagtgatacaccgttttaccctgactatctgccagggaaatcaacacattggaataaccactgacgatatcttccagcgtcattaagcgtcgggcttgcgtttcgtcagggtgatttagtacccgttcaagggtggcgctaatctcttttaaatcattaatatcctgctcggcaaaatgaacttttactgagtggatcatgatccatgcaaaggcgaaaaacgccgcgatggtggccaggctgataaaaaaggtcaggcgggttgccagcgaaaacgggcgctgaaatggcttactgaccatccggcacctcaagcatgtaacccacgccgcgcacggtctgaattagcttcggctcaaagtcgttgtcgattttgccgcgcagccgcttcaccgccacatcaatagcattggtatcgctgtcaaaattcatgtcccatacctgcgaggcgataagcgagcggggcagcacttcgccctgatggcgaaggaagaactccagcagagtaaactctttactggtcaaagtgatgcgcgtgccgctgcgggtgactttgcggctgacgagatcgaccatcaaatcggcaacctgaaactgactttcgataatcaccgccgccccgcgccgcagtaatgtgcgcacccgcgccagcagttcagcaaaagcgaatggcttcaccaggtagtcatctgcccccaactccagccccttgacgcgatgttcaatggtgccaagcgcggtaagcaacagaatcggcatccctttattggcggagcgtaacatgcgcacgatatcccagccgttcacgtccggcagcataatatcgaggattatcagatcataatcaccggtcatcgccagatggtagccattcagcccgttgtcggccaaatcgaccacaaaaccggcttcggttaaccctttggtcaagtattctccggttttcttttcatcttcgacaatcaacagtttcatatttcctccgcatgttgcccgggcaattctagagtagcgggatcagatggcaatcgcttattggcaaaatgacaattttgtcatttttctgtcaccggaaaatcagagcctggcgagtaaagttggcggcataaaatcaccagaaattatgagcctatgtctccttgtaaacttctgccattttgtgtggcccttgcgctaaccggttgttcactggcaccggattatcagcgtccggcaatgcccgtgccgcagcagttctcactcagccagaacggcctggttaacgcagcagataactatcagaacgcgggctggcgcaccttttttgttgataatcaggtgaagacgctgattagcgaggcgctggtgaataatcgggatttgcgcatggcgacgctgaaagtgcaggaggcacgggcgcaatatcgtctgaccgatgccgaccgctacccacagctcaatggcgagggcagcggcagctggagcggtaatcttaaagggaataccgccacgacacgggagttttcgaccggccttaacgccagctttgacctcgattttttcggtcgcttaaagaacatgagcgaagccgagcgacaaaattatttagccactgaggaagctcagcgcgcggtgcatattctgctggtttctaatgtcgcgcaaagctatttcaatcagcaactggcgtatgcgcaattgcaaatagccgaagaaacgctgcgtaattatcagcagtcatatgcgtttgtcgaaaaacaactgttgacaggtagcagtaatgttctggcgctggaacaggctcgcggggtgatagaaagtacccgcagcgacatcgctaaacgtcagggggaactggcgcaggcgaataatgcattgcaactgttgctgggaagctacggcaagctgccgcaagcgcagacagtaaacagcgacagcctgcaaagcgttaaattaccggcgggattgtcgtcgcaaatcttattgcagcgcccggatattatggaagctgaacacgcgttaatggcggctaatgccaatattggcgctgcacgcgcggcattttttccgtctataagcctgaccagcggaatatcgaccgccagtagcgatctatcgtcattatttaacgccagcagcgggatgtggaattttatacccaaaattgagatccccatttttaatgccggacgcaaccaggccaatctggatatcgccgaaattcgccagcagcagtcggtggtgaattatgaacagaaaatccagaacgcctttaaagaagtggcagatgcgctggcattacgtcaaagcctgaacgatcaaattagcgcccagcagcgttatctggcatcgctgcaaattactttgcaacgggcgcgggcattatatcagcacggcgcagtaagttatctggaagtgctggatgccgagcgttctttatttgcaacccgacaaactttacttgatctgaattatgcccgtcaggttaacgaaatttctttgtataccgcacttggtggcggttgacagcaatatactcgtcatacttcaagttgcatgtgctgcgtctgcgttcgctcaccccagtcacttacttatgtaagctcctggggattcactcgcttgtcgccttcctgcaactcgaattatttagagtatgacttttaactccaggagagaataaatgaaaaaagcactgcaagtcgcaatgttcagtctgtttaccgttattggctttaatgcccaggctaacgaacatcatcatgaaaccatgagcgaagcacaaccacaggttattagcgccactggcgtggtaaagggtatcgatctggaaagcaaaaaaatcaccatccatcacgatccgattgctgccgtgaactggccggagatgaccatgcgctttaccatcaccccgcagacgaaaatgagtgaaattaaaaccggcgacaaagtggcgtttaattttgtccagcagggcaacctttctttattacaggatattaaagtcagccagtaacccaggtttaatgagatgaaaaaaatcgcgcttattatcggcagcatgatcgcgggcggtattatttctgcggcaggttttacctgggttgcaaaggcggaaccgcctgcagaaaaaacgtcgaccgcagaacgtaaaatcttattctggtacgacccaatgtatcccaatacgcggttcgataaaccaggtaaatcgccgtttatggatatggatctggtgccgaaatatgccgatgaagagagttctgcgtctggtgtgcgcattgacccgactcagacgcagaatctgggggtgaaaacggctaccgtcacgcgcggaccgctgacttttgcccagagtttcccggcgaatgtcagttacaacgagtatcagtatgccattgtgcaggctcgcgctgccgggtttatcgacaaggtgtatccgcttaccgtgggcgataaagtacaaaagggcacaccgcttctcgacctgaccattcctgactgggtggaagcgcagagtgagtatttactgctgcgcgaaaccggcggtacggcgacccagactgaaggcattcttgagcggctgcgactggcgggaatgccggaggcggatattcgccgcctgatcgccacgcaaaaaatccagactcgctttacgctcaaagcgcccattgatggcgtgatcaccgcgtttgatctgcgcgcgggaatgaatatcgccaaagataacgtggtagcgaaaattcagggtatggacccggtgtgggtcactgctgcgatcccggagtctatcgcctggctggtgaaagatgcctcgcagtttaccctcaccgttccggcgcgaccggataaaacactcaccatccgcaaatggacgctgctacctggcgtggatgccgcgacccgcacgctgcagctgcgtctggaagtcgacaacgccgacgaggcgctaaaaccgggcatgaacgcctggttgcaactcaacaccgccagcgaaccgatgctgctcattccgtcacaagcgctgattgataccggcagcgaacagcgggtgattaccgttgatgccgacgggcgctttgtaccgaaacgcgttgctgttttccaggcatcgcaaggcgtcaccgcattacgctctggtctggcggaaggtgaaaaggtggtttccagcggcctgttcctgattgattccgaagccaatatttctggcgcactggagcggatgcgctctgaaagtgctacccatgcgcattgagggaataaccaatgattgaatggattattcgtcgctcggtggcgaaccgttttttggtgctgatgggcgcgttgtttctgagcatctggggcacctggaccatcattaatacgccagtggatgcgctgccggatctctccgatgtgcaggttattattaaaaccagctatcccggtcaggcaccacaaatcgttgaaaatcaggtgacttatccgctaaccaccaccatgttgtcggtgcctggcgcgaagactgtgcgcggtttctcacagtttggcgactcttatgtgtatgtcattttcgaagatggcaccgatccgtactgggcgcgttcgcgggtgctggagtacctcaaccaggtacagggtaagctgcctgcgggagtcagcgccgagctggggccagatgccacgggtgttggctggatctatgaatatgcactggtggatcgcagcggtaagcacgatctggccgatttacgctcattacaggactggtttctcaaatatgagctgaaaaccatccctgacgttgcggaagtggcgtcggtgggcggtgtggtgaaagagtatcaggtggttatcgatccccagcgcctggcgcagtatggcatcagtctcgccgaagtaaaaagcgcgctggatgcttcaaaccaggaagcgggcggttcgtcgatcgaactggcggaagcggaatatatggtgcgcgccagcggctatctgcaaacgctcgacgactttaatcacatcgttttaaaagccagtgaaaatggcgtgcccgtttatctgcgcgatgttgcgaaggtccagattggcccggagatgcgccggggcattgccgaactaaacggcgaaggcgaagtggcgggcggggtggtgatcctgcgatccggcaaaaacgcccgagaagtgatcgccgccgtgaaggacaaactggaaacgctgaaaagtagtctgccggaaggcgtggagatagttacaacatacgatcgcagccagctcattgaccgcgccatcgacaacctcagcggcaagttgctggaagagtttattgtggtggcggtagtctgtgcgctgtttctctggcatgtgcgctcggcgctggtggcgattatttcgttgccgctggggttgtgtattgcttttattgtcatgcacttccagggactgaatgccaatattatgtcgttgggtggcattgcgattgccgtcggggcgatggtcgatgctgctatcgtcatgatcgagaatgcgcataaacggctggaagagtggcagcaccagcatcctgacgccacgctggataataaaacgcgctggcaggtgatcaccgatgcgtctgttgaagtggggccggcgctatttatcagtctgctgattatcacgttgtcgtttatcccgatcttcaccctggaagggcaggaagggcgtctgtttggcccgttggcgttcaccaaaacgtatgcgatggcgggtgcggcgctgctggcgatcgtagtgatcccgatcctgatgggctactggatccgtggcaaaattccgccggaaagcagtaacccgctcaatcgctttttgattcgtgtttatcatccgctgttgctgaaagtactgcactggccgaaaaccacgctgctggtggcggcgctttcggtgctgacggttctctggccgctcaataaagttggcggggaatttttaccgcagatcaatgaaggcgacttgttgtatatgccatcgacgctgccggggatttccgcagcagaggcggcgagtatgctgcaaaaaaccgacaagctaattatgagcgtacctgaagtggcgcgggtatttggcaaaaccgggaaagcggaaaccgccaccgattctgctccgctggagatggtagaaacgaccatccagcttaagccgcaggagcagtggcggccaggcatgacgatggacaaaatcattgaggaactggataacaccgtgcggctgccggggctggcgaatctgtgggtgccgccaattcgtaaccgtatcgatatgctctcaaccggcattaaaagccccatcggcattaaagtttccggcactgtgctggcggatatcgacgcgatggctgagcaaattgaagaagtagcgcgaacggtgccaggcgtagcttctgcgcttgccgagcggctggaaggtgggcgctatatcaacgttgagattaaccgtgaaaaagccgcacgttacggtatgacggtggcggatgtgcagttgtttgtgacttctgcggtgggcggggcgatggttggcgaaacggtggaagggattgcccgttatccaattaatctgcgttatccgcaaagctggcgcgatagtccgcaggcactgcgccagctgccgatcctgacgccgatgaagcagcaaatcaccctggcagacgtggccgacattaaagtctctaccggaccgtcgatgctgaaaaccgagaatgcgcgcccgacgagctggatttatatcgatgcccgcgatcgtgacatggtgtcggtggttcacgatttgcaaaaagcgatagctgaaaaagtgcagttaaaaccgggcaccagcgtggcattctccgggcagttcgagctactggagcgcgccaaccataagcttaaactcatggtgccgatgacgttgatgattatcttcgtgctgttgtatctggcgttccgtcgggtgggcgaagcgttgctgattatcagcagcgtaccgtttgcgctggtgggcggcatctggttgctgtggtggatgggctttcatctttccgtggcgacgggcactggctttatcgccctcgccggggtcgccgccgaatttggcgtggtgatgctgatgtatttacgtcacgccatagaggccgtgccgtcgttgaataatccacaaacattcagcgagcagaagctggatgaggcgttatatcacggcgcggtcctgcgcgtgcgcccgaaagcgatgacggtggcggtgattatcgccggtctgctgccgattctgtggggaacgggggctggttcagaggtgatgagccggattgccgcgccgatgattggcggcatgatcaccgcacctttgctgtcgctgtttattatcccggcggcgtataagctgatgtggctgcaccgacatcgggtacggaaataaaagcaggataccccgtttaaccgtgtggattgtgtcttgcgacgatgggcactaaatgttaaaaggtgcccctcaacaaaaaagacacacaggggaaaggcgtgaaaaacgcgtcaaccgtatcggaagatactgcgtcgaatcaagagccgacgcttcatcgcggattacataaccgtcatattcaactgattgcgttgggtggcgcaattggtactggtctgtttcttggcattggcccggcgattcagatggcgggtccggctgtattgctgggctacggcgtcgccgggatcatcgctttcctgattatgcgccagcttggcgaaatggtggttgaggagccggtatccggttcatttgcccactttgcctataaatactggggaccgtttgcgggcttcctctctggctggaactactgggtaatgttcgtgctggtgggaatggcagagctgaccgctgcgggcatctatatgcagtactggttcccggatgttccaacgtggatttgggctgccgccttctttattatcatcaacgccgttaacctggtgaacgtgcgcttatatggcgaaaccgagttctggtttgcgttgattaaagtgctggcaatcatcggtatgatcggctttggcctgtggctgctgttttctggtcacggcggcgagaaagccagtatcgacaacctctggcgctacggtggtttcttcgccaccggctggaatgggctgattttgtcgctggcggtaattatgttctccttcggcggtctggagctgattgggattactgccgctgaagcgcgcgatccggaaaaaagcattccaaaagcggtaaatcaggtggtgtatcgcatcctgctgttttacatcggttcactggtggttttactggcgctctatccgtgggtggaagtgaaatccaacagtagcccgtttgtgatgattttccataatctcgacagcaacgtggtagcttctgcgctgaacttcgtcattctggtagcatcgctgtcagtgtataacagcggggtttactctaacagccgcatgctgtttggcctttctgtgcagggtaatgcgccgaagtttttgactcgcgtcagccgtcgcggtgtgccgattaactcgctgatgctttccggagcgatcacttcgctggtggtgttaatcaactatctgctgccgcaaaaagcgtttggtctgctgatggcgctggtggtagcaacgctgctgttgaactggattatgatctgtctggcgcatctgcgttttcgtgcagcgatgcgacgtcaggggcgtgaaacacagtttaaggcgctgctctatccgttcggcaactatctctgcattgccttcctcggcatgattttgctgctgatgtgcacgatggatgatatgcgcttgtcagcgatcctgctgccggtgtggattgtattcctgtttatggcatttaaaacgctgcgtcggaaataaggcattcacgctacatccgacaaaacgatgtcaaccatccgaaaccgctctcatccattcgatgagagcggtttttttaattactgcttaaatgcacccgccagagagcgaatatcattgccggttggcgactgatgaagtcgcagaccaaactcttcgacaatcgcaaatatgtgatcgaatatatcagcctgaatgctttcatattccagccacaccacggtgttagtaaacgcgtagatctcgagcggtaaaccgttatcacctggagccagttggcgtaccattaaggtcatatctttacgaatccgcggatggttacgcagatattcgttcagataggcacgaaaggttccaatattggtcattcggcgcagatttaataccgactccgtagaaccttgctggcgattccactcattaatttcctgatggcggctggttaaataaggctttaacaaatgcgctttattcagacgttgcatttcgtcttcatcaagaaaacgaatactggtgacatcaatactgatactgcgcttaatacgtcgcccgccagatgctgacatcccgctccagtttttaaaggagtcagaaaccagagaccaggtgggaatagtggtaatggtattgtcccagttacgcactttgacggtggttaacccaatatcgatcaccgcgccatccgcgccgtatttcggcatctccagccagtcgcccagtttcagcatatcgttcgcggaaagctgaatacctgccaccagaccaagaatcggatctttaaataccaacatcagcacggcagccattgcaccaagaccgctgatcagaatcgctggcgactgaccaatcagcagcgagatcatcaaaatgccgaccagaatcgcgccgatcagtttaatcccctgaaatatccctttcagcggtaactgagatgctgccgggaatttctgcgccagattcaaaataacatccagcaacgagaagactgaaagcagcgcatacatcatgatccacaactgcgcgcaggtagtcagaatatctgccgcttcggtgcctttttgcagccagaataccgcctgaatattgacgataatcccctgcagggtaaaagctaaacggtggaagagtttattctgggtaatgatttgcaaccaaagccgtgaactggcgatggcacgtttttcgaaggtccgcagtaccacccaatgcaaaataatatgcaccacgacggcggtcagaaaaataataccgaaaatcatcaccatcgaggtggtgtgatcgatctcaatacccgctaaatcttcaacctgggatattaaatcctgcataacgtctcctttatacaacagcagcctatgatgacggctgaaacagggttatgcaaatcaggagaatctgagaggaaatagccgggcagatgcccggcaagagagaattacacttcggttaaggtgatgttttgcggcagacgagatttcggcagcgtagcgttaaaatcttcaacgctgtgatgacctaccggaacaaccaccagactggtgtagcctttctctttcagaccaaattctgcatcgaggatggcggcgtcaaaaccttcgatgggtaccgcgtccagacccagagccgccacgccgagcaggaagttaccgacgttgagataaacctgttttgccatccactctgcatcatcatgcagatctttacggtgcatatcagcgaagaacttgcgacctttatcgttcgcggctttcgcttccggcgtggcaaagcggccatcggcatcttcctggtcaacaaccagcttcagccagacatcgtccatcgcggtttttgcacagaacaccacgacgtgcgaggcatcaagcattttacgctcgttgaacacgtaattaccggcagcggatttggcaacacgcgctttaccttcttccgtgctggcaacaataaaatgccacggctgggagttggtgctggatgggctgtattgcagtagcgttttgatctgctcggcctgttccggggtaagttttttgctggcatcaaatgccttagtggaatgacgctttaaggcgacagaaatgatatccataaagactccatgtgaaagtaattttgcgtgccagcagattacaaggttcaacgagaaatggtaagcgagaaaaatgcgctatagatttccgctttagcctggacgcactcttttttgatcgcgtttagccagaccatcaaccaccagattccacgaatcgttgatcagatcgcgaagtaacgcttcggagatttcttcgccgggatacactgaaatccagtgctttttattcatgtgataccctggcttaatgcttgggtatatttgctgatttaacagggatttttgtggatcggacttcagattgataaaggggacgccgcgtagctccgacgacagcataaaaatcttgccgccaattttaaaaacatcgaactccgggccaaaaggccagcaaagctcgacaaagggtaactcaagggccaggcgtttcgccgtttcgtgcagtgattgcttatccataaacgttcctttaggcgaaggagaataagcaaagtatgccgcgaagtacggcgataatcgacgtttaatccgccagcgagaaccagcgtcgccagataaagcgcagaacaaaatactcaatagcgcccagcactaaaaaccacagacaaaacaataaagtgtaaagctgactaagatccatcagatggaacatggtcaccagtttttgtgccagcgccagccccagtgcgggggcgggcagcagcaggcaagagaggaaagccatcagcaaaatgcctgctgcggtggtcaaggtttctaaagggtgtttcataacattgttaaatgtaagttaaaacaccattgtcagggatattcttctgtaaggcaattcccggcttagtcaccggcccagatctcacaatgctttttcaccagcccaatcagcgagccgccatcggcgacgaaatcgcgcattagctgcgcttcattcagaccgctgacgacctggcgatgcagggcctcaatcgcgctcgatgcaccaattttatgtgcggaaggggcgattttttccagcaatcgcaaggtatcttccgttagcggtcgacgatctccagtgtgcggatcggtgatgacgccttcaagcccatagcgacaggcctggaaacggttgaatttatacagcaggtaatctttttcctgatgtttaaacgggcgttccgtcagtaaccagtgggcggtagcctgaattaatcccgccatatttactgcgtggctaagggttaacggggtatccatcacccgaacctccaccgtgccaaaatgaggactggggcgaatatcccagtgcagatctttaatgctgtcgatcatcgtggtgtaactcagacagcgaaacagggcttcaaattgttgccagttactgacccacggcatcgggccattatcaggaaaggcggaaaaaatattcggtcgtgaggaggcaaaacgcgtatccgttccctgcatatatggcgacgcggcggaaagggcgataaagtgcggcacaaatcgtgacaagccgtgcagcaaataaatggcgtcatcgccactggcgcagccaacatggacatgctgaccaaaaacggtcgcctgctgaatgagataaccaaagttttccagcgtgcgttgatagcgttcgttatcgcatacctcctgacgctgccatttctgaaacgggtgcgtgccaccgccgcaaatttccagatgatggtctgtggctgcctgcaatacgactttctgcatcgctgaaaactgcccggcagcctggttgatatcacggcaaacatccgtcgccagctccagcatactttcggtgatatcgtgctttacctctccggccgtgatcttatttttaaccgcgtcaatcagcattgaagagtcctggcttaagtcatagcccggcggattaaccacctgcatttccagttcaataccgagggtaaaaggttcagaaacatgaaaatcgggtaatggcataggtttctcttatgttggcgttttctattcagtatagaagtcggagcggctgggcgagatgcggaagttctggaatgtttcttttttttggtgatggtgaactgatggtgcctgaagcaatttggctacttttgcaatgtgacaagttatggcagtgctgactggtggcgaagaattttgacgattgagtcatgcagaaaaaaacgggttcagcttcagttgattaaatgaggagtgagaagtccgaaacaggactcactgtataaataaacagctattttgttgaggaagggtaagataacggcgggtgcctgaagctttccggtttcaggtttactctgaggtctggaaagatgaagccccaggagatatttctatcaaccctggggctgccactccaaacccgaacaatttggatggtagtcccttcttcgcatggaggcaatataaacatgctgacgaaatatgcccttgcggcagtcatagtgctgtgtttaacggtgctgggatttacgcttctggtcggagactcgctgtgtgagtttacggtgaaggaacgtaatattgagtttaaggctgttctcgcttacgaaccgaagaagtagccgttgtgcggggagtaatcccataagcgctaacttaagggttgtggtattacgcctgatatgatttaacgtgccgatgaattactctcacgataactggtcagcaattctggcccatattggtaagcccgaagaactggatacttcggcacgtaatgccggggctctaacccgccgccgcgaaattcgtgatgctgcaactctgctacgtctggggctggcttacggccccggggggatgtcattacgtgaagtcactgcatgggctcagctccatgacgttgcaacattatctgacgtggctctcctgaagcggctgcggaatgccgccgactggtttggcatacttgccgcacaaacacttgctgtacgcgccgcagttacgggttgtacaagcggaaagagattgcgtcttgtcgatggaacagcaatcagtgcgcccgggggcggcagcgctgaatggcgactacatatgggatatgatcctcatacctgtcagttcactgattttgagctaaccgacagcagagacgctgaacggctggaccgatttgcgcaaacggcagacgagatacgcattgctgaccggggattcggttcgcgtcccgaatgtatccgctcacttgcttttggagaagctgattatatcgtccgggttcactggcgaggattgcgctggttaactgcagaaggaatgcgctttgacatgatgggttttctgcgcgggctggattgcggtaagaacggtgaaaccactgtaatgataggcaattcaggtaataaaaaagccggagctccctttccggcacgtctcattgccgtatcacttcctcccgaaaaagcattaatcagtaaaacccgactgctcagcgagaatcgtcgaaaaggacgagtagttcaggcggaaacgctggaagcagcgggccatgtgctattgctaacatcattaccggaagatgaatattcagcagagcaagtggctgattgttaccgtctgcgatggcaaattgaactggcttttaagcggctcaaaagtttgctgcacctggatgctttgcgtgcaaaggaacctgaactcgcgaaagcgtggatatttgctaatctactcgccgcatttttaattgacgacataatccagccatcgctggatttcccccccagaagtgccggatccgaaaagaagaactaactcgttgtggagaataacaaaaatggtcatctggagcttacaggtggccattcgtgggacagtatccctgacagcctacaaaacgcaattgaagaacgcgaggcatcgtcttaacgaggcaccgaggcgtcgcattcttcagatggttcaacccttaagttagcgcttatgggagtaatccccgcatatccggttgtcaggtcaggatggtaaggcacctgctttacactttcgcccgtggtcagtgatggctgcgggcgaatcgtaccagatgttgtcaattaatcgtgttggcacagcgttatgactatcttttcttttatctgccagtgcacagcaaacatctcattctcacgatgaatgatgacctgctgtttattccagctaattatctgatagtccagaaaacctgcatcagtttggatctcacttgccttaaatgcgctctctttggcggaaaatgccagtgtcagcgccagagaaaaggctaaaccgcagtctgcgagtcgctcgtgttccgctggtgtaataatgttgtctgtcaattctcttgcggtttgtacagaaaaaatttcttctatatcaatgccaatcggttgacgagataccacggctaatgccgtagtcccacagtggctaatactgccgtatacctccgcaggccagacaggttggcgtagctcgccgattgcgggcacacatttatagccatattcccgcaaagcataaacagcagcgatccgtccggctaaatgctctgttttacgtttacgtccagcgtgttgcagttgtgcgtagtgcggcagccagagtaaatcctgctcacaaaaattcgccggatcgaactcaacaaaatgcagcgtatgtccggcaaaggggagggaggtatgcgtagttttcatatcgaccatattcgagactgatgacaaacgcaaaactgcctgatgcgctacgcttatcaggcctacatggtcctgcaatatattgaattggcaagatttttgtaggccggataaggcgttcacgccgcatccggcatgaacgacgcgcactttgtcaacaatctgacgttagcatcagaagtgggtgtttacgctcatataccacgtacgtcccggctcgttataggtatacgccccggcaccggcgatatagttggcccctgccaaatcgcccgtggtctgggcattacccgcacgccacaaacgtttgtcgaacagattgtccacgccgccggtcagactgacattcttcgtcacatcccaggtcgcgctcaggccaacaatgctgtaaggactaatttctttggtttccggtccaaccgctggctgacctttatagttgtacttcttcggctgctgcttgccgtaccaggtgaaggtcgtttgcatcgacaaatcttcccgtgcctgccagctcagcgttgagttcaacgtatactccgggatgatcgacaaacggtcgcccgtggttttgttttcactcttcagcatataagtgatgttattggtccacatcaccgtttcgctaaccggtacgtttaacgatccttccagaccttcaaccaccgctttcggcacgttatcccactgatagagatcggtgccgactgcgttttgccctacagccacatagcccgcttcaatcttattgcgataatcgttacggaaccaggtgacgcccgccagccacccgtcgcgtttgaactccagaccaatctctttgttgatgctggtttctgctttcaggtcatcgttaccttgcagatagcagccgcccgcgctggcatagcaaccctgacctttactgtagagaatgtagttcgggttagtctggtacaggctcggcgctttataagcacgggcgatgcccattttcagcgtgaagtcatcgcctaaaccttgcgatatgttcagcgccgggctccagttattgccgacaatactgtgatgatcgaaacgcagccccggcgttacgatggtgctgtcagtcagctccatgttgttttcggcaaacagcgagaaaatttctgcttttgaatacgggctacggtcggtggtactcacgccatcaatagcgccaccggtattcgttccggtcagtgcctgggtgttggaacttaagtccttcatccgttgctgattccactccgtacccagcgtcagcgtctggttaacgaggaaatcaatcggcaggttaacttcgctgtgcagcatcacgtcatcaagatcgatatcgacgaaatcctgtgtcgctttttcgttaaatttcccttcggtaccgcccgccagaccttccggaatacgcgagttacgggtgtgttcgtactgcacccagttgctggtggtcacgccgttatcccagccaccgttccaggtcagcgcgtagttctggcgatacagacggttggtttcatcgccatatttcgagcgggtataggaatcggagttggtattctgggtgtcgcccgcatacaggttaccctggcggctgtaacctgcttccagttccagcgattgcaatggcgcgaaatcccagcgcaccacgccattaatatctttgttgattaccccttcgcgcccggctggtaacgtcgtggcatacgttccggcacgcgcggactgatggccctggttgatatcccacgcgtcagcctgggttttgtcgaggttgccatacaaacggaagctgaattcgtcgcccagcggaccggtcaggctaaagttagtgcgtttggtggcaccttcctctttatgttctggcgcattgaaatatgcgtcccaggagccgtgccactcgccgctgccttttttggtaatgatgttaaccacgccgcccgccgcgccgttgccataacgcgcagctgccggaccacgcagaacttcaatacgttcaatcatttcaggtggcacccaggaagtatcaccacgggtatcgcgctcgccacgccagccctgacgcaccgagttacggctgcttaccggcttgccgtcaatcaaaatcagcgtgttttccggacccataccgcgaatatcaatctgtcggttattcccacgctgaccactggtggagttaccggtcaggttaacgcctggcatggtacggatgatcttcgacacatcgcgggcaaccgggtttttgcggatttcatctgcggtgatggtcgaaacgccaggcgcctgtaagttctgctcggcggcggtaacgacaatagtatcgtcatgtgaaacaggagtatcggtcggctcttgtgcctgcgctaccccataaatccccagattgaccaacaaggccagggaatgaatcttcttgttcattgttttattcctgcatttttgccacgaattgcaactgtcgggcatggtcgtcatcaacacgacgcatcccgctaccgcgaaaacctttgatcctgaaagacacgcagtgcagttggttaattaatgtccgcgcttcccacggcgcgccattacgctattgcaaatgcaaatagttatcaataatattatcaatatatttctgcaatcaatgaaaaattgcacagtaaacatggggttatggtgtgacggcgttaaaagtaggaagtgagagctggtggcagtcgaaacatggcccggaatggcagcgtctgaatgacgaaatgtttgaggtcactttctggtggcgtgatccccaaggttctgaagaatactcgacgataaagcgcgtatgggtctacatcactggtgtgaccgatcaccatcagaacagccagccccagtcgatgcagcgaattgcaggcactaacgtctggcagtggacgacacaactcaatgccaactggcgcggcagctactgctttattcccaccgaacgcgatgacattttttctgtaccatcccccgatcgcctcgaattgcgcgaaggctggcgaaaactattaccccaggcgatagccgatccgctgaacctacaaagctggaaaggcgggcgagggcacgctgtttctgcactcgaaatgccgcaagcgcctctgcaaccgggatgggattgtccgcaagcgccagaaatacctgccaaagaaattatctggaaaagtgaacggttgaaaaagtcacggcgtgtatggatttttaccaccggcgatgcaacagcagaagaacgcccgctggcagttttgctcgatggcgaattttgggcgcaaagtatgcccgtctggccagtgctgacttcgctgacccatcgtcagcaacttcctcccgccgtgtatgtgttgatcgacgctatcgacaccacgcaccgcgcccacgaactgccgtgtaatgcggatttctggctcgcagtacagcaagagttattacccctggtgaaagctattgccccttttagcgatcgtgccgatcgcaccgtggttgccgggcagagttttggtgggctttccgcgctgtatgccggactgcactggcctgaacgctttggctgtgtattaagccagtcaggatcgtactggtggccgcatcggggcgggcagcaagagggcgtgttacttgaaaagctaaaagctggtgaagttagcgccgaaggtctgcgcattgtgctggaagcgggtattcgcgagccgatgatcatgcgggccaatcaggcgctgtatgcgcaattacaccccataaaagaatccattttctggcgtcaggttgacggcggacatgatgcgctttgttggcgcggtggcttgatgcaggggctaatcgacctctggcaaccacttttccatgacaggagttgaatatggcattcagtaatcccttcgatgatccgcagggagcgttttacatattgcgcaatgcgcaggggcaattcagtctgtggccgcaacaatgcgtcttaccggcaggctgggacattgtgtgtcagccgcagtcacaggcgtcctgccagcagtggctggaagcccactggcgtactctgacaccgacgaattttacccagttgcaggaggcacaatgagccagcatttacctttggtcgccgcacagcccggcatctggatggcagaaaaactgtcagaattaccctccgcctggagcgtggcgcattacgttgagttaaccggagaggttgattcgccattactggcccgcgcggtggttgccggactagcgcaagcagatacgctgcggatgcgttttacggaagataacggcgaagtctggcagtgggtcgatgatgcgctgacgttcgaactgccagaaattatcgacctacgaaccaacattgatccgcacggtactgcgcaggcattaatgcaggcggatttgcaacaagatctgcgcgtcgatagcggtaaaccactggtctttcatcagctgatacaggtggcggataaccgctggtactggtatcagcgttatcaccatttgctggtcgatggctttagtttcccggccattacccgccagatcgccaatatttactgcacatggctgcgtggcgaaccaacgcctgcttcgccatttacgcctttcgctgatgtagtggaagagtaccagcaataccgcgaaagcgaagcctggcagcgtgatgcggcattctgggcagaacagcgtcgtcaactgccgccgcccgcgtcactttctccggcacctttaccggggcgcagcgcctcggcagatattctgcgcctgaaactggaatttaccgacggggaattccgccagctggctacgcaactttcaggtgtgcagcgtaccgatttagcccttgcgctggcagccttgtggctggggcgattgtgcaatcgtatggactacgccgccggatttatctttatgcgtcgactgggctcggcggcgctgacggctaccggacccgtgctcaacgttttgccgttgggtattcacattgcggcgcaagaaacgctgccggaactggcaacccgactggcagcacaactgaaaaaaatgcgtcgtcatcaacgttacgatgccgaacaaattgtccgtgacagcgggcgagcggcaggtgatgaaccgctgtttggtccggtactcaatatcaaggtatttgattaccaactggatattcctgatgttcaggcgcaaacccataccctggcaaccggtccggttaatgaccttgaactggccctgttcccggatgtacacggtgatttgagtattgagatcctcgccaataaacagcgttacgatgagccaacgttaatccagcatgctgaacgcctgaaaatgctgattgcccagttcgccgcggatccggcgctgttgtgcggcgatgtcgatattatgctgccaggtgagtatgcgcagctggcgcagctcaacgccactcaggttgagattccagaaaccacgcttagcgcgctggtggcagaacaagcggcaaaaacaccggatgctccggcgctggcagatgcgcgttacctgttcagctatcgggaaatgcgcgagcaggtggtggcgctggcgaatctgctgcgtgagcgcggcgttaaaccaggggacagcgtggcggtggcactaccgcgctcggtctttttgaccctggcactccatgcgatagttgaagctggagcggcctggctaccgctggataccggctatccggacgatcgcctgaaaatgatgctggaagatgcgcgtccgtcgctgttaattaccaccgacgatcaactgccgcgctttagcgatgttcccaatttaacaagcctttgctataacgccccgcttacaccgcagggcagtgcgccgctgcaactttcacaaccgcatcacacggcttatatcatctttacctctggctccaccggcaggccgaaaggggtaatggtcgggcagacggctatcgtcaaccgcctgctttggatgcaaaatcattatccgcttacaggcgaagatgtcgttgcccaaaaaacgccgtgcagttttgatgtctcggtgtgggagtttttctggccgtttatcgcaggggcaaaactggtgatggctgaaccggaagcgcaccgcgacccgctcgctatgcagcaattctttgccgaatatggcgtaacgaccacgcactttgtgccgtcgatgctggcggcatttgttgcctcgctgacgccgcaaaccgctcgccagagttgcgcgacgttgaaacaggttttctgtagtggtgaggccttaccggctgatttatgccgcgaatggcaacagttaactggcgcgccgttgcataatctatatggcccgacggaagcggcggtagatgtcagctggtatccggcttttggcgaggaactggcacaggtgcgcggcagcagtgtgccgattggttatccggtatggaatacgggtctgcgtattcttgatgcgatgatgcatccggtgccgccgggtgtggcgggtgatctctatctcactggcattcaactggcgcagggctatctcggacgccccgatctgaccgccagccgctttattgccgatccttttgccccaggtgaacggatgtaccgtaccggagacgttgcccgctggctggataacggcgcggtggagtacctcgggcgcagtgatgatcagctaaaaattcgcgggcagcgtatcgaactgggcgaaatcgatcgcgtgatgcaggcgctgccggatgtcgaacaagccgttacccacgcctgtgtgattaaccaggcggctgccaccggtggtgatgcgcgtcaattggtgggctatctggtgtcgcaatcgggcctgccgttggataccagcgcattgcaggcgcagcttcgtgaaacattgccaccacatatggtaccggtggttctgctgcaacttccacagttaccacttagcgccaacggcaagctggatcgcaaagccttaccgttgcctgaactgaaggcacaagcgccagggcgtgcgccgaaagcgggcagtgaaacgattatcgccgcggcattctcgtcgttgctggggtgtgacgtgcaggatgccgatgctgatttcttcgcgcttggcggtcattcgctactggcaatgaaactggcagcgcagttaagtcggcaggttgcccgccaggtgacgccggggcaagtgatggtcgcgtcaactgtcgccaaactggcaacgattattgatgctgaagaagacagcacccggcgtatgggattcgaaaccattctgccgttgcgtgaaggtaatggcccgacgctgttttgtttccatcctgcgtccggttttgcctggcagttcagcgtgctctcgcgttatctcgatccacaatggtcgattatcggcattcagtcaccgcgccccaatggccccatgcagacggcggcaaacctggatgaagtctgcgaagcgcatctggcaacgttacttgaacaacaaccgcatggcccttattacctgctggggtattcccttggcggtacgctggcgcagggtattgcggcgcgactgcgtgcccgtggcgaacaggtggcatttcttggcttgctggatacctggccgccagaaacgcaaaactggcaggaaaaagaagctaatggtctggacccggaagtgctggcggagattaaccgcgaacgcgaggccttcctggcagcacagcagggaagtacttcaacggagttgtttaccaccattgaaggcaactacgctgatgctgtgcgcctgctgacgactgctcatagcgtaccgtttgacggtaaagcgacgctgtttgttgctgaacgcacacttcaggaaggtatgagtcccgaacgcgcctggtcgccgtggatagcggagctggatatctatcgtcaggattgtgcgcatgtggatattatctctccagggacgtttgaaaaaattgggccgattattcgcgcaacgctaaacaggtaaattaatattatttataaacccataattacagaaaataattatgggttttttatttgtttgatttataggtttgatgaatatttctcttaaatagagtgaatgttgcattcagtggaaggaatttacaaacttcagcttcggataattatcaccaactggtaaagtgagcgccgtggagatttccccctattggactcattttcaggttataccccatgtcatcactgaatattaaacagggaagtgacgctcattttcccgattatcctctggcgtcgcccagtaataatgaaattgatttacttaatctaatctcagttttatggcgggccaaaaaaacggtcatggcggtcgtttttgcgtttgcctgcgcaggcttgctgatctctttcatcctgccgcaaaaatggaccagcgcggcggttgtcacgcctccagaacctgttcagtggcaagagttggagaaatcattcactaagcttcgtgtgctggatctggatatcaaaattgatcgtacagaagcatttaacctgtttatcaagaagtttcagtcggttagcttgctggaagagtacctgcgttcatcaccttatgtgatggaccaattaaaagaggcgaaaatcgacgaactggatttgcatcgcgcaattgtcgcattgagcgaaaaaatgaaagcggttgatgacaatgccagtaagaaaaaagatgaaccgtcactgtatacctcctggacgctaagttttaccgcgccaaccagtgaagaggcgcagaccgttttgagcgggtatatcgattatatctctacgttggtggtgaaagagtcgctagaaaacgtccgtaataaactggagatcaaaacccagtttgaaaaagaaaaactggctcaggatcgcattaaaacgaaaaatcaacttgatgcaaacattcagcgcctcaattattcactcgacattgccaacgcggcaggaattaaaaagcccgtttacagtaatggtcaggccgttaaagatgaccccgatttttctatttctctcggtgcagacggtattgaacgcaaactggaaatagaaaaagcggtcactgacgttgcggaactgaacggtgaattacgtaatcggcagtatcttgtcgagcaattaacaaaagcacatgtcaacgatgtgaattttacgccgtttaaatatcagttaagcccgtcattgccagtgaaaaaagacggtccgggtaaggcgattattgtgatcctttccgcgttgatcggcgggatggtggcttgtggtggcgtgctgttgcgctatgcgatggcatccagaaaacaggatgccatgatggcagaccacttagtttaactatttgcggttgaaggtgccgttcgtccgagcggcaccacaagcggcgttccggcaactggatcgtcaatgatcatgcagcgcagaccataaatgcgctcaatcagttcagcagtgacaatctccttcggcgctccctgagcaacaattttcccttcccgcaatgcaatcaaatggctggcgtaacgacaggcctgattaagatcgtgcagcaccgccgccagggtatagcctttttcgcggttcagttcgcttaacaactccagcaaatcaatctgatgactgatatccagccaggtcgtgggttcgtcgagcagcataattgccgtttcctgggccagcaccatcgcgatccacgctcgctggcgttgtccgccagaaagggtatccacgctttgatctgccagatgagttattcccgtggcctgcattgctttcgttaccgcttcttcatcctctttgcgccagcgggtaaacagcggttgatgcggataacgtccacgcgccaccagctcctgcacggtgatatcgcccggcgtggtagcattttgcgccaacagaccaatccggcgtgcaacctctttactggcgtaatgttgaatgtgctcgccatccagccagacatgcccatgagcaggcgtcatcaggcggcttaaggtacgcagtaacgtggatttaccgcagccatttggcccgataattgccgtgaagtgaccatcaggtatttctacagtcagattttccgcaacggtatatttgccatatcccagggttaactgttcgccgcgcaaacgggctactgattcggtcattttttgcgagactcctgaattaacaagacgataaggtaaataccgccgaggctgacggtaacgacgccaaccggaagttgatacggcataaacagttgttgggcgcagagatcggccgccagcagtaacagcgccccgcatagcgccgcctgggttagcccccagcgagcggtgccgctaatgcgtcgggcaatgtgcggtgcgactaaagcaataaaggaaatcggcccggcaagcgctgttgccgcagcggtaagcaccactgcaaccagcatcattaacagacgcgaacgttcgacgctgacgcccagcgcacacgcggtatcatcgcccatttccagcaagcgcatccggcgtaccagtaaggcggcggcaatgagcatcaatataatgatgggtgcggaaggcgaggtttttgcccacgtcaggccgttgagcgatccggcattccacaaacctgctgttagcgccgtttctaaagacgctttcagcaacagccaggtattaaaggccaccagcatggcgcgaacgccgataccgataataatcaaccgaaaggtgtcgatgccgttgcgccaggcgagcagccagaccagcagcgaagtgacaatgccgcccaccattgctgacagcgcgatagccgtcaggtcctgaccaaacagcaccatcgccaccagcacgccgctccacgccccggtgttaaagcccattacgtcagggctgccgagcgggttacgcatcagcgactgaaaaatcgcgccactgacgcccagtgctgcgccaatcaacagcgccatcagcacgcgtggtaaacgccattcggtgaccaccatcgtcatactgcgcggcgcatcgcccatcagcgcggcgaatacctgcgaggtttccagcgtgacggcaccgctgcgtaatccccagatacctgcaaccacacaggcggaaaccagcagcaaacaggtgatgagtaatcggcgagagacgtaaatcatgcaccacctcgcgttttacgtcgcacgaggaagatcagcaccggtgcaccaataaacgcactgaccacagaaacgcgcagttcgccgggcacaatcacccgcccgatgatatcggcaaacagcagcagggcaggggtagcaagtagcgtgacgggcagcgaccagcgatgatcggcacccaccagccaacgcgccatatgcggcatcatcaggccaataaaggcaatcgggccaactattgccgtcgcactaccacaaagcacggtaatcgccagcagaccaatcaactgtgtgcgcgccacgcgactgcccagcgccgtcgcggtgtcgctgccgaggctcaaactgttcagcgcgcgactcagtaatagcgcagttgctccggcgatcagcaccgggatcagcaccacttttaaggtatgtagattgcgaatatccagcgaaccggcttgccagaaacgcaactgatcgtagacgtcaggattaagcagggcgatgccgctggtcagtccttccagcaccgccgccagcgccacgcccgccagggttaaacgcaccggacttaactgcccgccgccctgactgccggtaaaggcaacaatcaatgaggccaccagcgccccggcgaaggccatcgccagttgttcctgcgcggaagagtaaccaaacagcgccgcacccagcacaatggcaaagctggctccggcgttcacgccaagcaagccggggtcggcaagtgggtttcgggtgagggtttgcattaacgccccggcaaggccaagcgcgccgcctgccagtaaaccggcaagggtacgcggcagccgcgcgtcgagcacgatggtgcagtcggcgctctggcaggtgccggagaaggcctccagcactacggaagcggggagtgattttgccccaatgagcaggcttaatgccgtcgcgataatcagtaataacagcaatccgggcacggcaatggcgcgtgtcacggcaacagaaccagacatacgaacttccatgataatgaaattaattatcgttatcgatcttatttggatatgttagcatgtgcagcctaagaataggtatttaaaatatttgatggcaaggcattgtaatgaataaacaatcctggctgcttaacctcagcctgttgaaaacgcacccggcgtttcgcgcagtattcctcgctcgtttcatctcaattgtgtctctgggtttgctcggcgtcgcggtgccggtgcagatccagatgatgacacattccacctggcaggtggggctttcggtgacgctgaccggcggcgcgatgtttgttggcctgatggtcggcggtgtgctggcggatcgctatgagcgcaaaaaagtgattttgctggcgcgcggcacctgtggcattggcttcattggactgtgccttaatgcactgctgccggagccgtcattgctggcaatctatttacttggtttatgggatggttttttcgcatcgcttggcgttacggcgctattggcggcgacaccagcactggtagggcgtgaaaacttaatgcaggccggggcgatcaccatgttgaccgtgcgtctggggtcggtgatttcgcccatgattggcggtttattgctggcgaccggtggcgtagcctggaactacgggctggcggcggcgggcacgtttattaccttgctaccgttgttaagccttccggcgttgccaccgccaccgcagccgcgtgagcatccgttgaaatcattactggcaggatttcgttttctgcttgccagcccgctggtgggcgggattgcgctgctgggtggtttattgacgatggcgagcgcggtgcgggtactgtatccggcgctggctgacaactggcagatgtcagcggcacagattggttttctctacgcggcgatcccgctcggcgcggctattggtgcgttaaccagcgggaagctggcacatagtgcgcgaccagggttattgatgctgctctccacgctgggatcgttcctcgccattggtctgtttggcctgatgccgatgtggattttaggcgtggtttgtctggcgctgttcggctggttgagtgcggtcagctcgttgctgcaatacacaatgctgcaaacgcaaaccccggaagcgatgttagggcggattaacggtttgtggacggcgcagaacgtgacgggcgatgccataggcgcggcgctgctgggtggtttgggcgcgatgatgacaccggttgcttccgcaagcgcgagcggttttggtttgttgattatcggcgtgttgttattgctggtgctggtggagttgcgacattttcgccagacgccgccgcaggtgacagcgtccgacagttaatgcttaaaacagcgccttaagcctatccagcacttgcatggcgctgtagtaatccagacggaacgtctcggttcccagcgcataaacctgcttgttttgtactgcaggcaggtgcgcgagcagcggattagcataaatagcatcggcatctttctgatcaccggcgaacaggaatagtgactcgccatttaaccctgcagccagattttccccaccaagctgaatgatgtcatggcgtttaccctgactttggctggcatttaaccctgcgggtaacttcgccagcgtaaagccgagttgttccagcatctgcccttgtgctgattctggcgtccagagattggcactgtgtgcagcggcagtatagacaatggcagtgaccggctgcggcggtaatttgatttgctctttcgccgccgccagttgcttatcaaactgcgcaatccgctctgccgcttgtttctcatgcccggtaatttcgccaagttgcgttaacagcgactgccagcttttgtcgtcgtaattgatgattaatgtcggggcgatggtggaaagctgatcatacagtgccagcgccgaatccccgccggttgcgctaattaaaatcagatccggcatttgcgcggcaacggcttcggcgctcggttcgccgatatagagccgttgcagtttgcgttctttcgccaccttgctccactggcgtaaaaagccctggtcatccgcgacgcggttattcggcgtggtcgcgccgctggcgatcaccggagcatcaatcgccagcagtgagccggtcagggtgacgctggtggaaacaatacgctgcggctggctttccagtgtatgtgtgccacggctgtcagtaatctgacgcggccagtcagcggcctgaactgcggctattcctgaaagcaaaagtcctgttaatagaagggcgttgcggtagagcggggcgagtctcacaaatcagcttcctgttattaataaggttaagggcgtaatgacaaattcgacaaagcgcacaatccgtcccctcgcccctttggggagagggttagggtgaggggaacagccagcactggtgcgaacattaaccctcaccccagccctcaccctggaagggagagggggcagaacggcgcaggacatcacattgcgcttatgcgaatccatcaataatgcttctcattttcattgtaaccacaaccagatgcaaccccgagttgcagattgcgttacctcaagagttgacatagtgcgcgtttgcttttaggttagcgaccgaaaatataaatgataatcattattaaagcctttatcattttgtggaggatgatatggatacgtcactggctgaggaagtacagcagaccatggcaacacttgcgcccaatcgctttttctttatgtcgccgtaccgcagttttacgacgtcaggatgtttcgcccgcttcgatgaaccggctgtgaacggggattcgcccgacagtcccttccagcaaaaactcgccgcgctgtttgccgatgccaaagcgcagggcatcaaaaatccggtgatggtcggggcgattcccttcgatccacgtcagccttcgtcgctgtatattcctgaatcctggcagtcgttctcccgtcaggaaaaacaagcttccgcacgccgtttcacccgcagccagtcgctgaatgtggtggaacgccaggcaattccggagcaaaccacgtttgaacagatggttgcccgcgccgccgcacttaccgccacgccgcaggtcgacaaagtggtgttgtcacggttgattgatatcaccactgacgccgccattgatagtggcgtattgctggaacggttgattgcgcaaaacccggttagttacaacttccatgttccgctggctgatggtggcgtcctgctgggggccagcccggaactgctgctacgtaaagacggcgagcgttttagctccattccgttagccggttccgcgcgtcgtcagccggatgaagtgctcgatcgcgaagcaggtaatcgtctgctggcgtcagaaaaagatcgccatgaacatgaactggtgactcaggcgatgaaagaggtactgcgcgaacgcagtagtgagttacacgttccttcttctccacagctgatcaccacgccgacgctgtggcatctcgcaactccctttgaaggtaaagcgaattcgcaagaaaacgcactgactctggcctgtctgctgcatccgacccccgcgctgagcggtttcccgcatcaggccgcgacccaggttattgctgaactggaaccgttcgaccgcgaactgtttggcggcattgtgggttggtgtgacagcgaaggtaacggcgaatgggtggtgaccatccgctgcgcgaagctgcgggaaaatcaggtgcgtctgtttgccggagcggggattgtgcctgcgtcgtcaccgttgggtgagtggcgcgaaacaggcgtcaaactttctaccatgttgaacgtttttggattgcattaaggagcgaggatgagcattccattcacccgctggccggaagagtttgcccgtcgctatcgggaaaaaggctactggcaggatttgccgctgaccgacattctgacgcgacatgctgcgagtgacagcatcgcggttatcgacggcgagcgacagttgagttatcgggagctgaatcaggcggcggataacctcgcgtgtagtttacgccgtcagggcattaaacctggtgaaaccgcgctggtacaactgggtaacgtcgctgaattgtatattacctttttcgcgctgctgaaactgggcgttgcgccggtgctggcgttgttcagccatcagcgtagtgaactgaacgcctatgccagccagattgaacccgcattgctgattgccgatcgccaacatgcgctgtttagcggggatgatttcctcaatactttcgtcacagaacattcctccattcgcgtggtgcaactgctcaacgacagcggtgagcataacttgcaggatgcgattaaccatccggctgaggattttactgccacgccatcacctgctgatgaagtggcctatttccagctttccggtggcaccaccggcacaccgaaactgatcccgcgcactcataacgactactactacagcgtgcgtcgtagcgtcgagatttgtcagttcacacaacagacacgctacctgtgcgcgatcccggcggctcataactacgccatgagttcgccaggatcgctgggcgtctttcttgccggaggaacggttgttctggcggccgatcccagcgccacgctctgtttcccattgattgaaaaacatcaggttaacgttaccgcgctggtgccacccgcagtcagcctgtggttgcaggcgctgatcgaaggcgaaagccgggcgcagcttgcctcgctgaaactgttacaggtcggcggcgcacgtctttctgccacccttgcggcgcgtattcccgctgagattggctgtcagttgcagcaggtgtttggcatggcggaagggctggtgaactacacccgacttgatgatagcgcggagaaaattatccatacccagggttacccaatgtgtccggatgacgaagtatgggttgccgatgccgaaggaaatccactgccgcaaggggaagtcggacgcctgatgacgcgcgggccgtacaccttccgcggctattacaaaagtccacagcacaatgccagcgcctttgatgccaacggtttttactgttccggcgatctgatctctattgatccagagggttacatcaccgtgcaggggcgcgagaaagatcagattaaccgtggcggcgagaagatcgctgccgaagagatcgaaaacctgctgctgcgccacccggcggtgatctacgccgcactggtgagcatggaagatgagctgatgggcgaaaaaagctgcgcttatctggtggtaaaagagccgctgcgcgcggtgcaggtgcgtcgtttcctgcgtgaacagggtattgccgaatttaaattaccggatcgcgtggagtgtgtggattcacttccgctgacggcggtcgggaaagtcgataaaaaacaattacgtcagtggctggcgtcacgcgcatcagcctgaaggagagaacacgatggctattccaaaattacaggcttacgcactgccggagtctcacgatattccgcagaataaagttgactgggcctttgaaccgcaacgtgccgcgttgttaatccatgatatgcaggactattttgtcagcttctggggcgagaactgcccgatgatggagcaggtgatcgcgaatattgctgcgctgcgcgactactgcaaacagcacaatatcccggtttattacaccgcccagccgaaagagcagagcgatgaagatcgggcgctgttgaatgatatgtgggggccgggcctgacccgctcgccggaacagcaaaaggtggtggatcgcctgacgccagatgccgacgacacggtgctggtgaagtggcgctacagcgcgtttcatcgttctccgctggagcaaatgctgaaagagagtggacgtaaccagctgattattaccggggtatatgcccacattggctgtatgaccaccgcaaccgacgcatttatgcgcgatattaaaccgtttatggtggcggatgcgctggccgatttcagccgtgacgagcatttgatgtcgctgaaatatgtggccggacgttctggccgggtggtgatgactgaagaattactgccagcacctatccccgccagcaaagcggcgctgcgtgaggtgatcctgccgttgctggacgagtccgatgaaccgttcgatgacgacaacctgatcgactacggtctggattcggtgcgcatgatggcgctggcggcgcgctggcgcaaagtgcatggtgatatcgactttgtcatgctggcgaaaaacccgaccatcgacgcctggtggaagctactctcccgcgaggtgaaataatggatttcagcggtaaaaatgtctgggtaaccggcgcaggtaaaggtatcggctacgccacggcgctggcgtttgttgaggcgggagcgaaagttacaggttttgatcaagcgttcactcaggagcaatatccctttgcgaccgaagtgatggatgttgccgacgctgcgcaggtcgcgcaagtgtgtcagcgactgttagctgaaacggagcgactggacgcgctggtcaatgcggcgggaattttacgcatgggcgcgaccgatcagctcagtaaagaggactggcagcagacttttgcggttaacgtcggcggtgcgtttaacctgttccagcaaaccatgaaccagtttcgccgtcagcggggcggggcgattgtcactgtggcgtccgacgccgcgcacacgccgcgtattggcatgagtgcttatggcgcatcgaaagcggcgctgaaaagcctggcgttgagcgtcgggctggaactggcgggtagcggcgtgcgctgtaatgtggtttcgcctggctccaccgacaccgatatgcaacgcacgctgtgggtgagcgatgacgccgaagaacagcgtattcgcggctttggcgagcagtttaaactcggcattccgctggggaaaatcgcccgtccacaagagatcgccaacacgattttgttcctcgcctctgacctcgccagccatattaccctacaggatattgtggtcgatggcggctcaacgctgggggcataagcatgatctggaaacgccatttaacgctcgacgaactgaacgccaccagcgataacacaatggtggcgcatctgggaattgtgtatacccgtctgggcgatgatgtgctggaagccgaaatgccggttgatacccgtactcatcagccgttcggtttactacatggcggcgcgtcggcggcgctggcggaaacgctgggatcgatggccggatttatgatgacccgcgacggacagtgtgtggtaggcacagaacttaatgcaacacaccatcgcccggtgtctgagggaaaggtacgcggcgtctgccagccgctgcatcttggtcggcaaaatcagagctgggaaatcgtcgttttcgatgaacaggggcggcgttgctgcacttgtcggctgggtacggcagttttgggatgaacccgacagaattagatgagattgcaggaaaactcggttaacggagtgatcgagttaacattgttaagttaaatattggtttcaactccgatttacatggttgctgtgttgttaaattgtacaaagatgttatagaaacaaaatgtaacatctctatggacacgcacacggataacaactatgaacaaatcagggaaatacctcgtctggacagtgctctctgtaatgggagcatttgctctgggatacattgctttaaatcgtggggaacagatcaacgcgctgtggattgtggtggcgtcggtctgtatctatctgatcgcttaccgtttttatgggctgtatatcgccaaaaatgtgctggcggttgacccgacgcgtatgacgccagcggtgcgccataacgacgggctggactatgtgccgacggacaagaaagtgctgttcggtcaccattttgcggccattgccggagcaggtccgctggtggggccggtactggcggcgcaaatgggctacctgccggggatgatctggctgctcgctggggtggttctcgccggtgcggtgcaggatttcatggtgctgtttgtttctacgcgccgtgacggtcgctcgctgggtgagctggtcaaagaagagatggggccaaccgccggggtgattgcgctggtggcctgctttatgatcatggtcattatccttgcagtgctggcgatgatcgtggtgaaagccctgactcatagcccgtggggaacatataccgttgcgttcaccattccgctggcgctgtttatggggatctacctgcgctatctgcgtccggggcgtattggcgaagtgtcggtcatcggtctggtattcctgattttcgccattatctctggcggctgggtggcagaaagtccgacctgggcaccgtactttgactttaccggcgtgcagttgacctggatgctggtgggttacggttttgtggcggcggtgctgccggtgtggttactgctggccccgcgtgactacctctctaccttcctgaaaatcgggactatcgtcggtctggcggtaggcattttgattatgcgcccgacgctgaccatgcctgcgctgaccaaatttgtcgatggcactggcccggtatggaccggtaacctgttcccgttcctgtttatcaccatcgcctgtggcgcggtgtctggcttccatgcgctgatctcttctgggaccacgccgaagatgctggcgaacgaagggcaggcgtgctttatcggctacggtgggatgttaatggaatccttcgtggcgattatggcgctggtttccgcctgtatcatcgatccgggcgtgtattttgccatgaacagcccgatggcggtgctggctccggcagggacggcggatgtggtcgcttctgccgcgcaggtggtgagtagctggggctttagcattacaccagatacgctaaaccagattgccagcgaagtgggtgaacagtcgatcatttcccgtgcgggcggtgcgccgacgctggcggtggggatggcctacattctgcacggcgcgctgggcggcatgatggatgtggcgttctggtatcacttcgccattttgtttgaagcactgtttattctgacggcggtggatgcaggtacgcgtgctgcgcgctttatgttgcaggatctgctgggcgtggtgtctcctggcctgaagcggaccgattcactgcctgctaacctgctggcaacagcgctgtgcgtactggcgtggggctacttcctccatcagggcgtggtcgatccgctgggcggcattaacactctgtggccgctgtttggtattgccaaccagatgctggcagggatggcgctgatgctctgtgccgtggtgttgttcaagatgaaacgtcaacgttacgcctgggtggcgctggtaccaacggcctggctgctgatttgtaccctgaccgcaggctggcagaaagcgtttagcccggatgcgaaagtcggcttcctggccattgctaataagttccaggcaatgatcgacagcggcaatattccgtcgcagtatactgagtcacagctggcgcaactggtgttcaacaaccgtctggatgccgggttaaccatcttctttatggtggtcgtggtggttctggcactgttctcgattaagacggcacttgcggcattgaaagatccgaagccaacggcgaaagaaacgccgtatgaaccaatgccggaaaatgtcgaggagatcgtggcgcaggcaaaaggcgcacactaaagtcagagtgagggggggatgttggcgaatgttggcttagtgcccagggttccctctcaccctaaccctctccccggtggggcgaggggactgaccgagcgcgttgatagcatttgtaggccggataaggcgttcacgccgcatccggcactctttcagcaacatggttagcggaggccaagatgtttgattcactggcaaaagccggaaaatatttaggtcaggcggcgaagctgatgattggtatgcctgattacgacaactatgtcgaacatatgcgggttaaccatcccgatcaaacgccgatgacctacgaagagtttttccgtgagcggcaggacgcgcgctacggtggaaaaggcggcgcgcgctgctgctaaatttgtacgtcaggctttaaacgattccacttttttgaacgctgcacgcaacgtatctggtgtcagcgtgactggcaggtaatgaatggactccaccggacgcagggtgtgggcaatcactttgtcgatctccgcctgattattgatatccacttccagctccgccagtgtagtcggcagatgaaaacgctgatacgctccagttaattgcgccagcacatcatcctgacccagcaaggcgctttgcaccagaattccgtaggcgactttggtgccgtggagaaacttctcggtttgcggcagcacggtcagaccgttatgcacggcatgagctgccgccacacgcgtaaaacgatcgcccagaccaccaaccatcccaccaccagcaataatagcatccaccacatcgcaaaatgattgcgttaactgttgattttgctgatcgctcagcgcctgttcgctactgtttaacaagacgtcgcgaatggcttgcgcattattgatccccagtcgcacggttagcggcaacgtttctggttgcggagccagcaccaccgcttcataccatttcgccagcgtgtcaccgatccccgccagcagatattgttgcggtgcattgaggataatctccggttccaccagcaccataaaattggcgtcgtcgaaaatctcataatgcagcgcctgtccggcatcattataccagacggagagcggtgtccaggcggcgcaggtggcggcgatcgtcggaacggcaacaaacggcagaccgagacggcgggcgagggctttcgcggtgtcgagcagtgcaccgccaccgacgccaatcaccacgctgcggtcgtcaccggactcagccgccagttgttgtacatcgctttcgctgcaatgaccgcgaaacaaaatatgctttgcccctggcagtccaaacgctggcggaagtttggtttgcgccgcagcaatggcgcgtttgccgtagatccacaccgcgcgagaaagttgttcatcagtgaaaaaatcgtgcaggtgattgaaacttcctggatgtgaaaagtagttagccgggccgacgaccacgcggataggattgtgaggcatgttgtgttgtccttattgttttatttagacatctaaacgtcttgattgccaaatactagcatcgtgttatagtgccttcaacacgcaacttcgtcaggtacaataaaaatgacaaataaccctctgattccacaaagcaaacttccacaacttggcaccactattttcacccagatgagcgcgctggcgcagcaacaccaggcgattaacctgtcgcaaggctttcctgattttgatggtccgcgctatttacaggagcggctggcgcaccacgttgcacagggggcaaaccaatacgcgcccatgaccggcgtgcaggccttgcgcgaggcgattgctcagaaaacggaacgtttgtatggctatcaaccagatgccgatagcgatatcaccgtaacggcaggggcgacggaagcgttatacgcggcgattaccgcactggtgcgcaatggcgatgaagtgatttgttttgatcccagctatgacagttacgcccccgccatcgcgctttctgggggaatagtgaagcgtatggcactgcaaccaccgcattttcgcgttgactggcaggaatttgccgcattattaagcgagcgcaccagactggtgatcctcaacactccgcataaccccagtgcaactgtctggcagcaggctgatttcgccgctttgtggcaggcgatcgccgggcacgagatttttgtcattagcgatgaagtctacgagcacatcaacttttcacaacagggccatgccagtgtgctggcgcatccgcagctgcgtgagcgggcagtggcggtttcttcatttggcaagacctatcatatgaccggctggaaagtgggttattgtgttgcgccagcgcccatcagcgccgaaattcgcaaggtacatcagtatctgaccttttcggtgaataccccggcacagctggcgcttgctgatatgctacgtgcagaacctgagcattatcttgcgttaccggacttttatcgccagaagcgcgatattctggtgaatgctttaaatgaaagccggctggagattttaccgtgtgaaggtacatactttttgctggtggattacagcgcggtttctaccctggatgatgttgagttttgccagtggctgacgcaggagcacggcgtagcggcgattccgctgtcggtgttttgcgccgatcccttcccacataaactgattcgtctctgttttgccaagaaggaatcgacgttgctggcagcagctgaacgcctgcgccagctttagctatttaaccgtccaggcgcgggaatattgacggtcggcaaacaactcttgcaggccgttaatttgcttcaggcgcagcacttcgtcgctgtccattcccagctctttgccaattttattatcgtcccatcccaactggctaagttcacggacgatttccgacatggcggtgatttgatggcgtccacgagcgcgattatgacgaatagtcgcggcgatgcgttgattacgcgtaccttccagacaggtcaccggcaaataaccttttaagcgtaattttaatgatgatgagcctttaccaatttcatggcggtgaaaaccatccacgatttccatggcatttttatccgtatgtgtgaccacaatgggttgggtaaaaccatctatttcaatggatttttgcagcagttttttttcgggtggtgccacgttgtttgggttgtaatcattaggcataagttggctgtttttaacccacagaacgcaatccactggctcttcacgaaaggggctaacctgatggatcgccatgcggatttcattaatcgctttgatgcgatcatcttccggcaagctggcgagaaattgcgttaaatcctgcgttaatcgttgttgcatagtatcccccattcctgacgttttccttttatccgttcgttataacgctgatagttcttcgattttgtggggctaaatgataatgcccgacaccagtaatcgttattgagtaaaactttgcatatccgccgccaggaggggatatctttcgcgccaatgtccccttgctgggtttgtggaacctcgatgccttttttctgataccagtgcaaataaatggcgattttattgcggtaatgctcagctgttttttccggcatgctattgagcagcaataatgcatattcttgccagtctaaatgttctggcttgaggattttccgatgcccatagaaatgattgtcatgtccggcgtaaatgccgccactttttaccccgctgactcgtgcgcacatagcagcccagcgatccggttcgataacgtgatagagccataatccttgtcgttgctccgggccaaaaggttcgcaaattcgcatatgacgcagaggaacgcctgcctgatacattaggttatacagtgggttgcagagactttgatgatttgcataccaggtccagatatcagccactttccagtcgtaaatggggtaaatgtaccagctatgaccgcctggtgcggccgtagtccagggtttatcgtcggcaaaacgttgtttatttaaactggcgatggcgacaaaacggttgtaggactcatccgcacggatgccgatcatcatcgccgccggacgtttttgtgaaaaccattcggcaaactcacgtacaaattgttcgaaggtcatgcctggctggtaaaagcagaaaaagtcagggtcggttatcgcatcttggggaggttgacgtacccattcgacatcaggttcccagcactgccattcgggttggtattgtgaaagggaattttgcgtcgtaagcgggagcgcaacccagtaaaactcttcgatgacatcggtgtacaactcgcgcagggactgaacatagttaatggtgcaagagaattgcgcctcccagtcgataaacaaaacgcagatttttttgcccatttgtcgggcaagttcggctgtcagatgcagcattaaaccagagtctttgccgccagaaaatgagacacaaacgcggggtagggtgttgagtgtccaggtaatacgctctcgtgcagcttccagaatattgagcggaagaggaattttataaatagacatctgaagacgctctctgaacgttacagggtgatcagtgagataagtctgttaattataaagtaaacactgtaaagcagagtgttttatttttcattcgcgctgtgaataaatagatgaaagttatagtagctgtctgtagttatatatcaaaaactctcatttagacggtcaataaatcgggagaacaccaaattatttaaagaagatttattataggaaatgtaaagctttattgaaggtaacggatgttctagttttatctcttttaagttaagaaagtcacggtaggaattataaagttcataggggactattcccagtaaatctgtaactgcaatgctattaatgattgtcagcaaagaggaaccacgaaatgagattttgcgattcataaatctctcgtctatttccatttgaatatcatcaacccctgctgatttagatattaattgggtgaactcttctgccataatttgttcataagtgctattgtcagtaattcgtggatgcctattactacaaattagagtattgcgaatcgtatgcaatggcatgcaaatgacggaacggctgatcactggcatttgggtgatcaccagatcggctttgcggtgaaccaacagttcttcagcattctctgctgacatgaggatatcatggcactcaatctcgacagaggaatcttgccgtaggcagcggatcagcatactattattagagcaagaaatgagctgagggccgtagataataaagtttttctttagttcggacttattgactatattaattgtttgttcaaggcctctgagatttttctcaagatggtgatgcagatttaaccctgttgtcgtcggcgcgataccttttcctgagcgaatgaataaagggtcattaaattgcgcacgtaagcgttgtaacgactggctcacggctgatggggtgatatatagtgattcagcagctttgctaatgcttaaatgctggtaaatacactcaaatatgacaagaagatttaagtcgaactttttcaagtcgtagagattggccatacactactccggttatatttttcttccatgatatattcacttaatcaatgttttttgcgtatatatttttattgattatgtttttttgcttaactcaggattaagtttttctaaaatagcacagccacttagggcagagcgagcaattcatgcttttttaggatggttgaaaagcagggatatagttcaaccatccatgaattaccttttatttattccccataatgatattaagcgttttctgatcgggcaaccccacggcctgttgtagcgtattttccttactcatgtaatagatagccggcgtgacatttgcccccagatcgtccatcagtttctcattgtcacttaacactttcatttgctctgtacttacgtttgcaggcacgtttagcttaagcttgccaccagaggcttcatattgttgccaggtttttgcgggatctttggaggcaagaattgccgctgctgtcgccgggctttctggcttgataaccccaaccaacaatgttcttaattgcactttgccagaatctacccacgggcgcgcctgctgccagaactgtttacaatatgggcagaacggatcggcgaagacgtagacaatgaccggcgcatcttttttaccgtcgaggagccagtgggattgttccatccgttgccacatttcgcgtccggctggtgcgtaaatttctttttcgataagtgtgttactcaggttttcacctttctcgttgtacatgtaaccagagatagcgtgcttaccatctggagtcaggtagatggtgacgcccatatcctgatactttccgagataacctttcattcctccgggggcatcgaatgttttgatgattgtaatgccctgtttttcaatcgcttttactggagcaggaagttcctctgcgaaggcgattgcaggaagcagagccagtaaaagtatcttttttaacattaatttgtccttttcagtcagtgcaaaagtcgagtaaaaggcataacctatcactgtcataggtaagagcttagatcaggtgattgccctttgtttatgagggtgttgtaatccatgtcgttgttgcatttgtaagggcaacacctcagcctgcaggcaggcactgaagataccaaagggtagttcagattacacggtcacctggaaagggggccattttactttttatcgccgctggcggtgcaaagttcacaaagttgtcttacgaaggttgtaaggtaaaacttatcgatttgataatggaaacgcattagccgaatcggcaaaaattggttaccttacatctcatcgaaaacacggaggaagtatagatgtccttgattaacaccaaaattaaaccttttaaaaaccaggcattcaaaaacggcgaattcatcgaaatcaccgaaaaagataccgaaggccgctggagcgtcttcttcttctacccggctgactttactttcgtatgcccgaccgaactgggtgacgttgctgaccactacgaagaactgcagaaactgggcgtagacgtatacgcagtatctaccgatactcacttcacccacaaagcatggcacagcagctctgaaaccatcgctaaaatcaaatatgcgatgatcggcgacccgactggcgccctgacccgtaacttcgacaacatgcgtgaagatgaaggtctggctgaccgtgcgaccttcgttgttgacccgcagggtatcatccaggcaatcgaagttaccgctgaaggcattggccgtgacgcgtctgacctgctgcgtaaaatcaaagcagcacagtacgtagcttctcacccaggtgaagtttgcccggctaaatggaaagaaggtgaagcaactctggctccgtctctggacctggttggtaaaatctaaatttccttcgtctttcacgccatagcggcgttggcgtcgcccgctcaccccggtcacttacttgtgtaagctcccggggattcacaggctagccgccttgctctgacgcgaaatacttcggaaattcacctaattcttcgggtgctgcggcacccgattttcttccccgcaccatgatgcaagctgcatccaggtagccgcagaggccgcttgcatgatgatgtttaaagcccaggagataaacatgctcgacacaaatatgaaaactcaactcaaggcttaccttgagaaattgaccaagcctgttgagttaattgccacgctggatgacagcgctaaatcggcagaaatcaaggaactgttggctgaaatcgcagaactgtcagacaaagtcacctttaaagaagataacagcttgccggtgcgtaagccgtctttcctgatcaccaacccaggttccaaccaggggccacgttttgcaggctccccgctgggccacgagttcacctcgctggtactggcgttgctgtggaccggtggtcatccgtcgaaagaagcgcagtctctgctggagcagattcgccatattgacggtgattttgaattcgaaacctattactcgctctcttgccacaactgcccggacgtggtgcaggcgctgaacctgatgagcgtactgaacccgcgcatcaagcacactgcaattgacggcggcaccttccagaacgaaatcaccgatcgcaacgtgatgggcgttccggcagtgttcgtaaacgggaaagagtttggtcagggccgcatgacgttgactgaaatcgttgccaaaattgatactggcgcggaaaaacgtgcggcagaagagctgaacaagcgtgatgcttatgacgtattaatcgtcggttccggcccggcgggtgcagcggcagcaatttactccgcacgtaaaggcatccgtaccggtctgatgggcgaacgttttggtggtcagatcctcgataccgttgatatcgaaaactacatttctgtaccgaagactgaagggcagaagctggcaggcgcactgaaagttcacgttgatgaatacgacgttgatgtgatcgacagccagagcgccagcaaactgatcccagcagcagttgaaggtggtctgcatcagattgaaacagcttctggcgcggtactgaaagcacgcagcattatcgtggcgaccggtgcaaaatggcgcaacatgaacgttccgggcgaagatcagtatcgcaccaaaggcgtgacctactgcccgcactgcgacggcccgctgtttaaaggtaaacgcgtagcggttatcggcggcggtaactccggcgtggaagcggcaattgacctggcgggtatcgttgagcacgtaacgctgctggaatttgcgccagaaatgaaagccgaccaggttctgcaggacaaactgcgcagcctgaaaaacgtcgacattattctgaatgcgcaaaccacggaagtgaaaggcgacggcagcaaagtcgttggtctggaatatcgagatcgtgtcagcggcgatattcacaacatcgaactggccggtattttcgtccagattggtctgctgccgaacaccaactggctcgaaggcgcagtcgaacgtaaccgcatgggcgagattatcattgatgcgaaatgcgaaaccaacgtgaaaggcgtgttcgcagcgggtgactgtacgacggttccgtacaagcagatcatcatcgccactggcgaaggtgccaaagcctctctgagtgcttttgactacctgattcgcaccaaaactgcataagaagaagtaagattcacctgcaattgcttagccgccggggtcaaacctggcggcttttttatggcattaaaaagccccgccgggatggctccgggcagggcgggatacttattctggcaattaacgcacaaccagcaccggcagattggcgtggcggatcacgctcgaggcgttagaacctaacagatgggtcgaaatcgatgggttgcgagaaccaataactacaacatcagcccccagttcttctgccaactcattgacttcatcccgcacgctaccaaaacggacatgttgtttaatgcgggaaggatcgatggtgaagtggctgaccatcgtttgcagacgttcttgtgcttcatgttgcagatgctcttcaaaacgacgcacatcagcggcaaaacggtgcaggctcaggctggctgacccgggtagtacgtgaagtagatgaataactccgtcatcctgggcgaggaattcagcgtggcgaacagctttgtcgctcaattccatttcaaatacatcaactggcataatgattgtcttatacataaccctttctccctgttaatcatgaacaaatcattcgccatgattataatatttatccctgatatttgtctggttctttttccttacgaactgtttctgtgatgaatatattctcactgaacaccaggaattctcccaaaacctgtggtaccgcccgttttcccgctgtgatagctacccttaaagactgactcttttttgaactgtctctggaggttgcatgaaagcattgacttatcacggcccacatcacgttcaggtagaaaatgttcccgatccgggcgttgaacaggcagatgatattattctgcgtattacggcaacggcgatctgtggctctgacctccatctttatcgaggcaaaatacctcaggttaaacatggcgatatttttggtcatgaatttatgggggaagtagttgaaaccggaaaggacgtaaaaaatttgcaaaaaggcgaccgagtggtaattccgttcgtcattgcttgtggcgactgttttttctgtcgattgcaacaatatgccgcctgcgaaaataccaatgcgggtaaaggcgctgcgctcaataaaaaacagataccagctccagcggcattgtttggttatagtcacctgtatggcggcgttcctggtgggcaggcggaatatgtccgcgtccctaaagggaatgtggggccgtttaaagtaccgcctttgctttcagatgataaagcgcttttcctttctgatattctgccaacggcatggcaggcagcaaaaaatgcgcagatccaacaaggttcaagcgttgcagtctatggtgctggtcctgtgggattgttgacaatcgcctgtgcacggttgctcggtgcggaacagatttttgttgttgatcatcatccctaccgcttgcatttcgccgccgaccgctacggcgcgatcccgattaattttgatgaagacagcgatccggcacagtcaattattgaacaaacggcaggtcaccggggcgtggatgcagtaatagacgccgtcggttttgaagcgaaaggcagcaccacggaaacggtgctgactaacctgaaactggagggcagcagcggtaaagcgttgcgtcagtgtattgcggcggtcaggcgtggcggcattgttagcgtaccgggcgtctacgctggatttattcacggtttcctgtttggcgacgcctttgataaagggttgtcgtttaaaatgggacagacccacgttcacgcatggctgggagaattattaccgttaattgagaaaggattactgaaaccagaagaaattgttacccactatatgccgtttgaagaggccgcccggggatatgagattttcgaaaaacgtgaagaggagtgccgtaaggtgattctggtacccggtgcacaaagcgcagaggcggcgcagaaggcggtttcaggtctggtgaatgcgatgccggggggaacaatatgatcgtcaggagtggttttcgaggtaaaggacagccatgacgataatcgccgccataatcagaaatcctatcaggatgtaaaatgcttctgccatggttattcccacaaacgaaacggaataattttgcagcaaaagtgaacagtgagaaccaggaaaaattgctgattttgcgtaaagaggatgcgagtgcatcctctgggcaaagcgagttatcgcttgtgcagatgggattaaagcaggtagtcgccagcagcttctggctggtattcgagttccagcacttcaaggtgggttgcaacgccgcccggaagttcccagtgaatggaatcgccaacgcgcagccccagcagtgcggcacctaccggagccataacggaaagctgagtattgctatcggtcatttttgccggatacaccagcgtgcgcacacgcacttcgccatcgctaagattgcggaatttaacccggctgttcattgtcaccacgtcgtgtggcatctcttctggcgaacacatttgggcgcgatccaactctgcgtttaacgcgtcggcgattggcaaaccagcataggcgggttgctccagcagaatatcgatgcgttcggcatccaggtcgttaatgatgatagttggtctggacatttttactccatgtcgtcggtgctgcgagtgtcgcagataaacatacccaaaagaaaaccctcaccgtcaggcggcgagggtttaactcacatgatgatactgactgttgctcactctttgaagtgatttgcgtcacattcagggaattcctcaatgcagcgcattatgtataaatcttaatcgccttggtttatggaagacgaattagcgtgttttgtaaatcagatgattaataacccgctttatcaatcacaaaggttttgccacagttacctgggtgaggttgtggcaagaatgagtttgcagaaagcggagcgttgatggcgtcagctttgatcgagatctgaatttcagtcaaatacgcagggttaccctggcacgttagcttaactgctttcacgttctcttttccccagcttttggcaaaggcggcgtcaaagtcacggcggctcactgttttaccgtaattatccgcaaggaattttccggcttcgctctctttaatttcttgattcaggcgtaccatcgtaccgaagtatgcgtccggatcaaaaccaaagcaggcaccgtgtttggcatattcgtagcgttccaggcaggaacgtccgccagctcctggcatgacttcacttagtttagcggccgtttccagtgataatccggtttccggcgatgaacacattcggctggcgcgcgcttctggtagattcgggattgggcgagtagcgcaaccgaagcgcatccagcggcgttcatcaacaccacgggcagcaaccgatttaggcaatcctggccacagaccatgtacggtcagaaaatcagctttgttggtcgtttcggtttgcaggcgacattcatctcgttcgttacgatttcgatcgtgttgactctggcaaaatccggtttgccaggagagggccaggacatagcgatcaaaatcgccatactgttttgcctgcaacgctaaggcgttggcagaagagaagggaagcagagaaaccgcgagcaacgcggcgttacgccagaatgctttcataatgggtgtggaactcatacatacactgaatactatctattaaatcataaaaaagcccgccaggtgggcttacctggcgggcgtgatgatttattcagcgtttggcgaacgtattagttccacatggcgagaatcggccagccaaccaacagcaacatagagatgtaaatcaccccgaagattgcgccaagacgccagtaatcttttgatttcacatagccacagccgtaaataatcaccccaggaccggttgcatacggcgtcagacagcccatgataccgatagacagcaccagcaggatacacagttgttccattggtacgcccggaatacctttaccgacggccagaataaccggcagcatggttgcggtgtgcgcagacaggctggcaaacaggtagtgtgcaaagtagaacaccagaaccagtacaatcaccgttgcgtttggtgagaatccttccaggtgcgtactcatggtaccggcgaaccagtcaataaaaccagaacgagtcaggccgttagccatcacaaccagagttgccaggttgaccagtgtgttccatgcgctgttatagcgggtaatgtctttccaaggcacaacgtgcagggccagcattagcgaaactgccagcagaccaaccgcagtagcattaatgacttcactgccaaatacccacaaacctaagctgagcaatacaaggccaatcagtgtccactctctgcgtgtcagcgcacccatggttttcagttcatcacccgcccaggttgccacttcttcactgtgtgtgatttccggtttgtacagcacgtaggaaagccacggcgcaatgataagcaagataaccccaaccggcaggaagcagaggaaccactgcaaccagctaatctggataccggcaattttgctgacgaactccagacccagcacgtttggtgccgcaccggtgacaaacatggacgaactcagactggtactaatgaccatcatccacatcaaatagccgccaatacgacgcgcggacggatcgttcgggaatgatttaaacaacggcggcaggtttttaatgaccggaaaaaccgtacccccggtacgcgcggtgttggaaggtgtaaacggtgccagcagaatgtcgataatgacaatcgcataacccaacgtcagcgtgcgtttgcccatgaatttcaccaggaaaagggcaatgcgacgacctaacccggaaacttcataccctaatgcaaaaataaatgcgccaaataccagccataccgtggtgctggaaaaaccagccaggccccatttcagcgcctgtttttgcgcattaaacgctgggtcagctaattctttggcatcaaagagcaggtaattactgccaataacgcaaatagtaaccgcaataaaactgatcgctgttgccggaattggctcgaggatcatgccgacaatcattgccacaaacacagcgaagtaatgccatgcctgcggcggcataccgtcggggacagggataagaaacatgacacccatcaccaccagtggggccaatagtttccatatattatcttttgctaaagacatacgggttctccgaaaattaatatttccaaatttatcaagtgcttaaataattaaatctgtgctaaaaaccaggtaaggatcagtaggtcagcactgccgcctggactgagatttcgttcgatacactccctgtcgaactgccggagataatcgagatcggcgggggttcgaatgccccctttttgcaataatgtttgcgcctcgcgctgtagccagcgcaggcccccctcgccaccgcgcgatgcaacgttggtatcgccgttgatcgccatcagtaggagcaaggtatcgagcaatgccagttcaggatctaacccctgatccagcagagtgaggtaatgcggcaaggcgtgattgatcaccagtggataacccgcttcggcttcaccgcgtgcgccggtaaggccaagctgttggtacaaccgttgacctgccgtcagttgtgaattattggtacgcagttcgcgatcggtcaggccacggcagaaacttgccgccgtagaacaaacggttgttggcgttaccggttggttgagttgaagcaaacggccaattgccgcacatagcagccctaaagaaaaaatgctgcctttatgcgtgtttacgcccgcagtggcgcggaacatatcaccttcgcaagccataccaattgggcgtaatccgtggagtaccgcttctggtgccatttccgcactacaggcaccaaattcaatgaaacggggtagccagccctgaatcgccagcgcgctgcggtggaaatcttccagcgccatatctttgtgcgcaccgcagttaatgcgatccacgaggcctggtttcggtgacagattgacttcagtcagcatggcgcgccagcccagcagggcgtactcatcgattaatgacgtcgcaagctttgtggttttagttgacgttgcaggcatcgacatcgttcagcagtgcctccatgcggttgagtaaatcggtcagttgatgggtttttccacgcgcgcagacggctgcgctttgttcgcacaacaggcagcggcgaggcggcagtgaatagtcgcggcgggagagaatttcgccttcgggcgtcaggacatcgatatcccataaccgcccgagaggatgactatgttcaagctcaatggtggcgagcttgaggtcgcgagccggggcggcaatgctcaacatgccctccggcccgctggcggaaaccagtgcagcctgctcctgaatttgccagccctgttttgcggctaaggcacgcaaggctgtcacgccatgattaaaaattcggcgtgtgacctcgctgtctttaatcggcccaggcgcaaccacggtaaaggagaccagtggaacaggatggcgcttgagccagacgtgttgccgtgcttgcctttcatcccggctgacgagcagctcgggaattgataccgcatggtggctggcgagttcaggaagcaggtgcatggcttattccttcacctgatgcacaacatcgatcaccgagccatcgcggtaacgcacaacggcaacgacgcggtctgtgaattcaatcggctgtggttcaccggtcagcagacgcgcacgttcgcgcagccactcaatggaaaccactttaatgcccgcttcctgcagacgttctgccagttccggacgtgccgggttaactgcgataccgtggtctgtgaccagaatatcgacactggagcctggggtgatgcaggtcagtacgttatccaccagagtcggaatacgaccgcgtaccagcggcgcgacgatgatggaaagcgcagaggcaatcgcggtatcgcagtgaccaccggaagcaccacgcagtacgccgtcagagccggtcagcacgttaacgttgaactgggtgtcaatttccagcgcgctcagtaccaccacgtcgagacgatcaaccgatgcgcctttcgaaccccagttagcgtactggttggcgctgatttcgatgtgattggggttacgggccagcgattgcgcagcatggctgtcaaagctctgcacatccagcagtttgcggatcagacctttttcgtgcaggtcaaccatcgtcgcggtaataccgccaagggcgaagtcggcgcgaatatcgcggctacgcattttgtcttccaggaaacgggttaccgccagcgatgcgccgccggtgccggtttgcatggagaaaccttctttgaagtagccagagttgacaatcacatccgcagcgctacgggcaataagcagttcgcgcgggttagtggtcatacgggtcgcgccagcgccgatttttgcagcatcgccaacgcggtcaactttgacgatcaaatcaacctgatcttgctcaatgcttgccggattatgcggataaggcagcagttcttcggtaagcatcacgacctgttttgcgttgtcggcatcaactattgcatagccgagggagccgcagcaggctttaccggtgtagccgttggcattaccgaattcatcacaggacgggacgccgaggaaagccacgtcgatattcagttcgccgctctgtaccagatgcacacgaccgccgtgagagtggatctgcaccggttctgccagcagaccacgggagatctcttccgccagtggaccacgcaggccggaggtataaatgcgggtaaccacgccctggcgaatgtgttctaccagcggcgcatggcaatcactcagggagctggacgccagggtcaggtttttaaagcccatcttcgcgatgacgtccatcaccatattgacggtcaggtcaccgccacggaaagcgtgatggaaggaaaccgtcatgccgtcctgtaaaccagagcgacgaatcgcttcttccaggttggcgcacagtttgcgatcgcgcgctttttcagcctggtaggtttgctttggcgagttctggaaagcggcaagatcgcattcagcgcgacgattccaggccgctacccgttcttgtcgttgagattgttcaattttctgcgtcattttgattgccttattcttcgcggatgccggaaagttctgcacgggagagcaccagacgggcgcgatcgataaccggaccgtccaccatcttgccgttcagggaaaccacgccgaggccttcgcgagcggcggcttcagcggcttctacgacgcggcgggcgtgatccacttctttctgggtcggtgcgtagaggttgtgcagcagatcaatctgacgcgggttgatcagcgatttgccgtcaaagcccagctgtttgatgtgggcggcttcttgcagaaatccggcttcgttgttagcgtcggaatagacggtatcgaacgcctgaatacccgcagagcgcgcggcctgcaaaatggaacagcgtgcgaacagcagttcagttccttccggggagcgttctgtacgcaggttgcgcacatagtcttctgcaccgagggcgataccgatcaaacgctcggaagcgtgagcgatttccactgcgcgggtaatccccagcggagattcaatcgccgccagcaggccggtgctgccgggttcacgaccacaggctttttcgatacgcaggatctctttttcaatatccagaacatcctgagcggtatcggttttcggcagacgcacaacgtccgcaccaccgcgaacgacggcttccaggtcgttaacaccccattcggaatccagcgcgttgacacgcacaatggtttcaatatcgcgatacagcggatgttgcagcgcgtggtaaaccatgcggcgggcggtgtctttttcacgcaatgctacggagtcttcgaggtcaaacatcagggcatcagccgggtagatgaaggagttgctgaccatcgcggcattggcaccaggcacaaacaacatgctgcggcgggtgcgagttttacgttgttgcagcgaagcggaaatcattggcaatcctcccatggcagagccgggataccgctggcgcgtgccagcagggcttccagtcgtgcacgtaaaatgcagtccagtgcgcctttgtcatcgacattcagctgtacgccgcgcacgttgtagcgggcgagaacgtccagaatggtggtgcgaattgcatcgccaaactgtttctcaacgctgctattgatttgcaggtcgatatcctgcgtatcgagtggggcgatgcgtatcatcacatccccagactcaagggtgcctgcaacggcgggctggtttattttcatttttcacctgtttctcatgcgggggtcttttgacgagctgccgcgtcctggcgggagtgctcaagcaggttctgcaaataatgcagcgtgactgcagggaccagcggcgcgatagccgtgagatcgtttttcgccagcagttgacgtacccgggaagcggatatcggcatctcctggtaacgcagccgctcaatttcaaccagttcgatgggcggtgcggagatagtcggcgtttccagccagtagcgcatatcctggttgtactgggcggtaacgcgacaaaagggttcagtaccgacaaagcggtgagttacacccagcgcgggagcgaggtactgacggaaaatcttcagatcaatttcggtgtaacaatggttaatgacgctctgttctttaatgaagtagcaagggaacgtagcgcgggagatgatgtattcggagccacgatgcacagtcaggcgtggaatatcggcggtgccttttaacaccaaatccagccggtcttcataggggaagcgtgaagaatcttctttgactaaaaacagatgcaaccagtcgcactgtgccgcagcctgttgaatcagataacggtgaccattcgtaaagggattggcgttcatcacaatgcagccaatcttgttccctggatgacgaaattttttcagcgattcggcatagcgtttcagtcgcgtggcgctgttttccatcagcaccatcacgccgggtacgctggtcagcgtggaaaaaccgcactggcggaacagcgcctcgtattcggttttggtataaataaacagatgcgtgctgtgccgctcataggcgaggtttatcaattcagtggctaatgtcagcgccagtccttcaccgcggacggattcactgatagcaacgcatttaataatatttccggcaattccaccgcacgcgataagcttttcatcgcgggttacggtaataaatacttcgactgtggtgtcaacgctcaaatcattttcatgcaggaattgggcgatttccgccatttttttattttctgaacgttttacgcgggtgaaaatatcattgccgaacataataaatagtatcctgaaggtgcatgttgttatcgatttgcaacgaatgttgttcaatgttgcaaactgataaccttttattttcacttgggagaaagggggtgatcgaggtatatctttttctcctttcgctatacatcctaaggagtatttcggcgtgaaattttgatttatttcacatagagttagtggttttttatttatttaatgattttaagttttttaattaatgtaattacgaaatgactcgcaggtttaagtgatttaattgatttaatgaataaaatttgccacgatcataattaatatctatgtattttgattcaacattttaattacatccgtcaaagaggctcgggacaacccgcaaggaaaacaatgttgcagcttaacgagaataaacagtttgcatttttccaaagactggcatttccgctgcgtatctttttgctgattctggtgttctcaatatttgtcattgcagccctggcgcaatattttacggccagttttgaggactatttaacgcttcatgtacgcgacatggcaatgaatcaggcgaaaattattgcctccaatgacagtgtcatctctgcggtgaaaacgcgtgactacaaacggctggcgaccatcgctaacaaattacaaagagataccgattttgattatgtggtgattggggaccggcactcgatccgcctttaccatcctaatccggagaaaattggttatcctatgcagttcaccaaacagggcgcgctggagaaaggggagagctacttcattaccgggaaagggtcaatggggatggcgatgcgcgccaaaacgccaatctttgatgacgatggaaaagtcatcggcgtggtgtcgattggctacctggtgagtaaaatcgatagctggcgggctgagtttttattaccgatggcaggtgtgtttgtcgtgctgttagggattctgatgttgctgtcgtggttcctggccgcgcatatccgtcggcagatgatgggcatggagccaaagcaaatcgcacgcgtggtccgtcagcaagaggcgctgtttagttcggtttatgaagggctgattgcggtggatccgcatggttacattaccgccatcaatcgtaacgcaagaaagatgctggggctgagttcccccggacggcaatggttgggtaaacccattgttgaagtggtcaggcccgccgatttctttaccgaacagattgatgaaaaacgtcaggatgtggtggcgaactttaacggtctgagcgttattgccaaccgggaagctattcgttcaggtgatgatttgctgggggccattatcagctttcgtagtaaagacgaaatttccaccctcaatgcgcaactgacgcaaataaaacaatacgttgagagccttcgtacattgcgacacgagcatctcaattggatgtcgacgctcaatggtctgttgcagatgaaagagtatgatcgcgtgctggcgatggtgcagggggagtctcaggcccagcaacagcttattgacagcctgcgcgaggcgtttgccgatcgccaggtggcggggctgctttttggtaaagtgcagcgcgcccgggaactggggctaaaaatgatcattgtccccggtagccagctttcgcaactgccgccaggactggatagcaccgagtttgcagccattgtgggcaatttacttgataacgccttcgaagccagcctgcgtagcgatgaaggaaacaagatcgttgaattattcctcagcgatgaaggcgatgatgtggtgattgaagtcgccgatcagggctgcggcgttccagagtctctacgagacaaaatatttgagcagggggtcagtacgcgtgctgacgagcccggtgaacatggcattgggttgtacttgattgccagctacgtaacgcgctgcggtggtgttatcactctcgaagataatgatccctgcggtaccttattttcaatctatattccgaaagtgaaacctaatgacagctccattaaccctattgatcgttgaggacgaaacgccgctggcagagatgcatgcggaatatattcgtcacattcccggattcagtcagatattactggcgggaaatctggcgcaggcccgaatgatgatcgagcgttttaagccggggctaatcttgctcgataactatcttcctgacggtagagggattaatttactgcatgaactggtgcaggcgcattatcccggcgacgtggtgtttaccactgcagccagcgatatggaaacggtgtctgaagccgtacgttgtggtgtatttgattatctcattaagcccattgcctatgaacggctggggcaaacgctaacccgtttccgccagcgtaaacatatgctggaaagtattgatagcgccagccagaagcaaattgatgagatgtttaatgcttatgctcgcggtgaacctaaggacgagctaccgaccggcattgaccccttgacgctaaacgcggtgcgaaaactgtttaaagagcctggtgtgcaacatacggcagaaacggtggcgcaggcactgaccatcagccgcaccactgccaggcgttatcttgaatattgcgccagccgccatctgattattgctgaaattgttcacggcaaagttggcagaccacaacgcatataccacagtgggtgacatgataaagccggaggaaacttgcctccggcattactatttacttgcctgtgaccgctgctgccgttcctggcaccatcagctctgtagcaacgataacaatcaccaaaccaacaagcaccggtaccgaggtgcgttttacgacttcaaacggcgagatcttcgccatcccggcaaccgcaacgactacgccagaaacgggcgaaagggtacggccaaggtttgacgcctgcagcatcgggatagtcaaatacgccgggttaatgccggaagagtgcgccagtttcgggatcatctcaacaaacgcataaaacggcgcattgcctgaaccggtcgtgactgccgccagcattgtcagaatcaccaataccagcatcaggatgatactcgccgaaccaaacgaggtagcgatagaaatcagactttgaataaagccgatggtgctaagcccctgagcgaataccccagcggcaaccagcagcatcaccacgttagcaaacgcatctgccatcccgcgataagccacttccagaccagagaaaactttctgggtattaaagctgcggaggaactccagaatggaggcaatcagcatacaaatcaccagaatagtgatgatgtgtaattgcggaccccatttaccgtcaaaaatcagtacaccgatgatcggcgtgaacggcaaaatggcataaaacgcaggagcagtggtggtgatttcactgacatctaacatttcatgagagatgtgctcttttttatccagataacgttgccagaagaagtgggcgatcgccatgccgataattgcagcaattgagataggcagcgtcgttttgaaggcgaagtcaatcagcgacatttcggaagcttgcgccgccagcaccacatcccctgaagtcggtgcgagaataatcgccgccggggaggcacaaatggcagcagctgcgccacgactgataccaacgtttaccatcaccggaaatagggttgccatcagcaaaacacccagaccggttgcggaagagacggccagagacatcagacaggcgacaaaataggcggcaatcatcagcaggtaaggggagttaatatactgcaatggttttgacgccagcttgaccaccatatcattcgcgccgatatgggtcatgtaagcggcaaatccacacagcatcataatcatcatgccgaggtcgccgccgcggctcattagtaatattttaacgtattcaacgatatccgtggcgctgtagcctgttgaagcctggctggacggtaacactttgtgccccataatggcactgataatcagcaataacaggccaccgacaaataacacaccagtggcggaataccctttaatgatgtagcgagctacacccacaataaccacaaccccaataaggagctcaatgaatgtcagcataatttttcctgtctccaggccccaaagtaaataataaaaaattcctaaagcttaaggaaaaaatatgcccaataaattggcgatgaatgctgattaaaatcaagaaaaactgccattaagacattgaagttgctgtttttatacatagataacaaaacgcatatttagcggttggcaattatcacataataatgtgtgcaaattgatggtggattgatgcaaatttgttaattgcaatggtgttagctgcggctgtgcgctcaaaaaataatctaatatgagcataggttgacgatatatattatatacttcgttaagatgattgttgtatctcgttaaaaaataaaataatttttccttgattgcattttgtcatcaaaaaagacttggtttttcttttttgactattcccatcgcagaaaacgacgcatcatctttaatcgatgcgcggaaatatttaacttgaacaagcggaaataaatagagcagctattcagattattctttatgttgggtctattaaggttatgttaattgtagctttgctatgctagtagtagatttttgataaatgttttatggtcacaaatgaacgtgagtaaatatgtcgctatcttttcctttgtttttattcagttaatcagcgttggtaaagtttttgctaacgcagatgagtggatgacaacgtttagagaaaatattgcacaaacctggcaacagcctgaacattatgatttatatattcctgccatcacctggcatgcacgtttcgcttacgacaaagaaaaaaccgatcgctataacgagcgaccgtggggtggcggttttggcctgtcgcgttgggatgaaaaaggaaactggcatggcctgtatgccatggcatttaaggactcgtggaacaaatgggaaccgattgccggatacggatgggaaagtacctggcgaccgctggcggatgaaaattttcatttaggtctgggattcaccgctggcgtaacggcacgcgataactggaattacatccctctcccggttctactgccattggcctccgtgggttatggcccagtgacttttcagatgacctacattccgggtacctacaacaatggcaatgtgtactttgcctggatgcgctttcagttttgagacaaatgaagttttagtaacttctttaaaatcaatagctaaaataagtaacatcaaaaataacgcgacttttatcactttttagtaaagttacactggacaaagcgtaccacaattggtgtactggtaaccgacacagcatttgtgtctatttttcatgtaaaggtaattttgatgtctaagattaaaggtaacgttaagtggtttaatgagtccaaaggattcggtttcattactccggaagacggcagcaaagacgtgttcgtacacttctctgcaatccagactaatggttttaaaactcttgctgaaggtcagcgcgtagagttcgaaatcactaacggtgccaaaggcccttctgctgcaaacgtaatcgctctgtaagatacgtcagcaagaattcaaaacccgcttaatcagcgggttttttttggtctttagtgtgcggttgaggccgaaaacagccagaatgccagtgcggtcatggcaaaagaccccagaaggttgacgaaaacgttcagtaatgcccagccaaagcggccctcttgtaacaaaaacaccacttctgccgaaaatgttgagaaggttgttagaccgccacaaaatccggtggtgattaatactttccacactggatcaatgttcgtcatcctgctgaaccatgcgaatcctattcctatgatgaatgccccaatcaggtttgctgtcagcgtccccaacggaatcgcctgatgcagtgggttaaatcgcatacttaacagccatctcgccacgcttcccgtaccaccgccaataaaaactgctaaaagaagttgtaacactgcaaaatcctgctatttgatttgtatgagtgataagtgtaacgccgaataatcgtcgttggcgaattttacgactctgacaggaggtggcaatgctggttgccgcaggacagtttgctgttacatctgtgtgggaaaagaacgctgagatttgtgcctcgttgatggcgcaggcggcggaaaacgacgcatcgctgtttgccctgccggaagcattgctggcgcgcgatgatcatgatgcagatctatcggttaaatcagcacagctgctggaaggcgaattcctcggactttacggcgagaaagtaaacgtaacatgatgacgacaattctgacgattcatgttccttcaacgccggggcgcgcatggaatatgctggtggcacttcaggcaggaaacatcgtcgcccgttatgccaaactgcatctctatgatgcatttgccattcaggaatcacgccgtgttgatgctggtaatgaaatcgctccgttactggaggtggaagggatgaaggtcggtctgatgacctgttatgacttacgctttccagagctggcgctggcacaggcattacagggagctgaaatcctggtacttcctgccgcctgggttcgcgggccgctcaaagagcatcactggtcaacgttgcttgccgctcgtgcgctggataccacctgttatatggtggcggcgggggagtgcgggaacaaaaatatcggtcaaagccggattatagatccctttggcgtcaccattgcggcagcgtcagaaatgcctgcactcattatggcggaagtgacgcccgaacgtgtgcgtcaggtgcgcgcgcaactgcccgtcttaaacaaccgtcgctttgcgccgccgcaattattatgatgtttttttactcggcgcttgattcaccttgttacagattgctattgtgtgcgcgcgtcgaatgaccgttaatattctctggtttttaaggcgcgttctgttgccggttatatgtcaagaaggtatctatgggtgagattagtattaccaaactgctggtagttgcggcgctggtcgttctgctgtttgggactaagaagttacgtacgctgggcggagaccttggagcggccattaaagggttcaagaaggcgatgaatgatgacgatgctgcggcgaaaaaaggcgcagacgttgatcttcaggctgaaaagctctctcataaagagtgacgtggcgagcaggacgctccctcaatatcttgttcgatacaaaaaacccgcttcaaaaagcgggttttttatcagacagatgtaagtaattattacaggattacttaacttccatccctttcgcctgcaaatcggcgtggtaagaagagcggacaaacggaccgcatgcagcatgggtaaagcccatcgccagcgcttcggctttcatttcgtcgaactcatccgggctaacgtaacgttgaaccggcaggtgatggcggcttggctgcaaatattgccccagcgttaacatcgtcacaccatgacggcgcaggtcgcgcattacctcaataatttcttcattggtttcacccagtcccaccatcagaccagacttggtcgggatttccggatgcgcttctttaaagcgttccagcagcttcagcgaccagttgtaatctgcaccaggccgtacctgacggtaaatacgcggtacgttttccaggttatggttgaacacatctggtggcgttgcagtcagaatatccagagcacgatccatacgaccgcggaaatccggcaccagagtttcaattttgatttgcgggcttttttcccgaatggcagtaatgcaatccgcaaagtgctgggcaccgccatcgcgcaggtcatcacggtcaacggaggtgataaccacataacgcagcgccatatcggcaatggtctgcgccagtttcactggttcattggcatcaggagctaccgggcgaccgtgggcaacatcacagaacggacaacggcgggtacaaatagcgccgaggatcataaacgttgctgtgccgtggttgaagcattccgccaggttagggcaggaggcttcctcgcagacagaatgcaggccatttttgcgcattgcggctttgatgccctggatacgtgtagagtccgctggaagcttgattttcatccattccggcttgcgcagcagggcttcgcgctctgttgccacgtttttaaccgggataagggccatcttatcggcatcgcggtatttaacaccgcgttccatcacaatgggtttactcatagcgtgcgtgttccagttgcgaattacgaaggaaagcgtttcaattcaatagattgttgtaattatcaactatttttgaattaacgactggcagtatatcattgaaacggacctgaaagcagccaaagcggtcgcgaaaatgtaaaattgttgttggattgtgccattttatcgttctgcgctgtgatctggctgtaacaatactttttcaaaatgcattacggataacatctattactccgtgcaggatgggatcacgcaggctgaatttgttgtagtggatagagaaatctatttgctcctcatttaaggacggaaaaggcagtttttccagcggccagcagcggctaaacaggttataaaaacggctgggaataatcgctaacatgtcactgttggcaaccagtgcagcgattgtcaaaatgttgtagctggtgaaattgatttgccggtccggaaacatttcttgaactctctgccgcagaccgctgaaattttgctcttccggtaacagaagtacatgcgcagcgttgtcgatagtctctctgtcatcttctaaagagagtagtggatttccctcgcggcaaattaacaccatattgtcggtgaacagaacatgatgttgcaccgtacgattggtgcaaaacatgttatcgatgatgagatcggtttgaaactgactgagttggttttccgcgtcgctgatgggcgggttgcgcagtaaaagctgcggatagtgagttttaatcgcccgatagatgacaggaaggaccagtgctccgaccgagggagtggtcgcaatagttatcgttcgttgcttatcatagcttccttcgatatccagcgcgccaagaatggactcaaggccctgactgatatactcatgtagatgcatcgcaaatgcggtaggagtgacaccctggcctttgcgaataaacaatgggtcagggaatataacgcgcagtttctgaatagactgactgattgccgagggggtcagattaagcactttcgctgcattaacgatccctttatgtacatatacagcttcaaaaatagtcagaaggttaagatcaatatttcgtaaggttgtaaatatttgtggtttaccttctgacgactttctgcttaaacagggttcaatttgattattactatccacgcacttactccaattttattcatggaaaaataatatttaaaaaattacaataatcttatgtctaattggaacggaacgcttttgctcaccataatcaactatttcaataggttaatcaatggggtgagttacggagcaaggcgtggcaccgcatttctgcaagtgataaagaaaatatacaaacgcgaaggagatgtaaagcattagcagatattatgagtaatgacccagtgtaaattgggccattgatgtatggaattaagcggtaatatattcgaagtccggattgtttagtagcgctaaaatattttccagtaaacgtggagcaatattattagtcgtcgcttcgggtttccattgtgatattttagccatttccattccggcatacccacaaggattaatacgtaaaaatggtgaaagatccatattgacgtttaatgccagaccgtggaatgaacaaccgcgtcgaatacgtaaacccagtgagcaaattttcttttccccaacatagacacctggcgcgtcagcccgaggatgcgcttctatacccagttcagccagggtattcaccactgtttgctcaagcaaggtcaccagttcacgcacaccgagtttacggcgtttcaggttaagcaacacatacatcacctgttgccccggcccgtgataagtcacctgcccaccgcgatcgctctggatcaccggaatatcacccggcattaaaatgtgctccgcttttcctgcctgaccttgggtgaataccggatagtgctcgaccagccagatttcatcaagggtactatcatcgcgggtatcggtgaattcatgcatagcctgggagattggctcgtaaggctgaagaccgagctggcggacaagaattttatcctgatacaaaacggcatctccgtggagaatgagtaaaagtgggggaaaagtatatcacagcgaggagaggggagttacccgaccaggagccgggtaacggagaagcgagttacagaaccatgcggacaatatcgattttgcccagttcttcatacagtgtttcaacctgctcgatatgagtggcgttgatagtgatagataccgagtggtagttgcctttgctgcttggttttaccgttggggtgtagtcacctggcgcatggcgctgtaccacttcaaccacctgatcaaccagctcaggtaacgcctgccccataactttgtaagtaaaaggagtagggaattcaagcagttcgttaagtttggttttcatgtcagctccggcgtaacgtaattaaatagcaactcccgccagaaggcgggagttttttactgatgcttagtatatggggacggaaattacactttcaagtgtttaatttttaaccaaaccagtgatggaacattaatttaatgtaatcaatgattttgccgaagaagttaccttccgggatttcttgcaacacaaccagcgggcgttgctcgatcgttttgccatcaagctggaagttgatagttccgacgacctgattcttttgcagcggcgcatgcaattcactgctgttcagcacatagctggctttcagatctttcatgcgaccacgcggaatggtcaggtacacgtctttatcaacccctaacgaagcgcgatcagaatcaccaaaccaaaccggttcagaggcgaactctttacctactttcagtgggttaacggtttcaaagaaacggaagccccaggttagcagttttttactttcggcttcacggcctttaaaagtacgtccgcccattaccgcagaaatcaagcgcatctggccttcagtcgcagaagcaacaaggttgtaacctgctttgtcagtgtgtccggttttgatgccgtcgacattcaggctgttatcccataacaggccgttacggttcagctggcgaataccgttaaacgtaaattctttttctttatagatcgagtattcattcggtacgtcacggatcaatgcctggccgatcagcgccatatctcgcgcggagctgtactgaccatcagcatccagaccatgtaccgtctggaagtgggtatttttcaggcccagtgcgttaacgtagctgttcatcaagccaacaaaagcgtcctggctaccagcggcaaaatcggccatggcgacacaagcatcgttacccgattgcaggttaataccgcggatcagctgagaaaccggaacctgcatgcccggtttgaggaacatcagcgaagaacctttaaacaccgggttaccggtggcccatgcgtcgttgccgatagtgactaaatcagtttctttaaatttaccggctttcattgcctggccgataacgtaactggtcatcattttggtcaggctggcaggatcgcggcggacatctgcgttctgttcggcgagcactttgccggagttatagtcaatcaggatgtaggactccgcatcgatctgcggtacacccgggatcatagttttgatattcaggtcatcggcatgtgcagcagagataaaggctgtgcaaagagccgtggtgagcgccaggcgcttcatgatacgagcggaaaaaatggtattcatggtctgaactacgacatccgtgatggaattaaaaaagtgccctactatagcaaatgcactaccggcaggcatctgactttccgcgtgactttgttaacgtcatttacagaaattgacacatcagatgcctgctttacgctactgcgcggtagtaataaatgactgtaattgggcttcggtttgcaaacgttgctgcaaggtactggcttcggctttgctggcgaatgggccaagctggatccgccagaccgcgccattttgagttacgcgaccggggacgccgaacttctgtcccagttgctgttggtactgttgcgcacgagcctgatcgcttacggccccgacttgcaccataaagttgccgctggcgctttgcgagacggcttgcggtgtcaccattgcaggcgaggttgcaggcgttgtcgacggagctgtaacaacgggctgtggcgcaggcgtcggttcgctgccttccagtacaccaggcgctaaggtcgttggtgcgccgaggaaaccgctactggttaccggcgcgccggtcggatcttcgctttttagcgtcgaattactgaccggaagaatgtcaccctgcgggccagacactgaacttgttcccgcgccaccgcttaaatcgggaggtgcaggcagggcgtaagtctgtttggcgactgtggtacaagccataccaggaccagaaagcgaaccatcctgggcaacaataatcggatcgatacgaactttggtgttgtttgacgtgttaagacggtcagctgccgcgcgagaaagtgaaataacgcggtcgttgccgtaagggccgcgatcattaatgcgcaccacgatcattcgcccgttagccaggttagtgattctggcgtagctggggatcggaagcgttggatgggctgccgtcagctgtgtcggatcgaatgcttcgccagaggccgtcaggttactgccgggttcggcatcatagattgccgccagtcccgcctggctaaatcgagacggatcctgcacgattttgtagcttttaccgtcgcgctggtaatcctgatttgccgtcgcgttcagtggttcgaaacgcgggtccgccccgctaatttcaactatagggccgttacataccgcaggctgcggtacacttaccgtctgttgctgaccatcatcgcttgtacatgccgcgagcattcctgccgcgatgcagatcccgagccactgcttacgcattgcgcacctcttacacgcttttcgacaacattttcctgtgggtgtggattgacattacaatcccgaacccagccatcagcacaattagcgccgatcctccataactgaccagtgggagcggaacccctacaaccggcagaataccgcttaccataccaatatttacgaagacataaacgaataatatcagcattaagccgccagccatgacgcgaccaaaggtggtttgcgctctggcggctatccacagcccgcgcatgatcagcagaatgtagagagcgagcagaatcagaatgcccactaatcccagctcttccgccagtaccgcgaagataaagtcagtatggcgttcggggagaaattcaagctgtgactgagtgccgtgcagccagcctttgccgcgtaatccgccggagccaatagcaattttagactgaataatgtgatagcccgcgccgagtgggtctgattccgggtccaggagcatcattacgcgctggcgctggtaatcatgcatcaggaagaaccacagaatcggaatgaacgccgctaccagcactactgcgacgccaatcagacgccagctaaggccagagaggaacagtacaaacagaccggaaagcgcaacgaggattgatgttcccaggtcaggctgtgcagccaccagcagcgtgggcataaatatcagcaccagcgcgatgccagtgttcttcaacgatggcgggcaaacgtcgcggttgataaagcgcgcaaccatcagtggtacggctattttggcaatttccgacggctgaaaacgaacaataccgaggtccagccagcgttgagcacctttagagatggcaccgaaagcatctaccgccaccagcaaaataatacagatgatatagagatagggggcccagccttcataaacgcgtggaggaatttgcgccatcaccaccatgatgaccagacccatcgcgatttggccgattttacgctccatcatgccaatatcctgaccgctggcgctccagataaccagggcgctgtaaaccagcaatgccagtaagatcagcagcattgtgggatcgagatggactttatcccagaatgtttttttattcggattatccgtcatgattaatggtcctccgctgcggcaaccgctggattttccgcaggcagatcggtgttgttatcacccagcataatgtggtcgaggatctggcgcatcagtgtaccaaccgccggacccgcaccaccgttctccagaatcatggcgacagccacttgcggattgttgtatggcgcaaaggcggtcatcagtttgtggtcacgtaaacgctcggcaattttgtgcgcattataggtttcgttcgctttcagaccgaagacctgagcggtaccggatttcgccgcaattttgtacggtgcgctagcaaagtatttatgcgccgtaccgttagggcggttagcaacaccgtacataccgtctttcgccagctcccagtaaccggaatgaatatcgccgacgggcggttcatgcggctgtacccatggcacctgtttgccgtcttcggcggtgctcatcagcaaatgaggaaccttcacgataccgtcattaatcaggatcatcagtgccttactcatctggattggggtcgctgtccagtaaccctgaccgataccaaccggaatggtgtcaccctgataccacggttttttaaagcgtttctgtttccattcgcgggtaggcatgttgccggaacgttcttccgccaggtcgataccggtgtaatgaccataaccgaatttacccatccattcggagaggcgatcgatccccatatcgtaggccacctgatagaagaaggtatccgcagattcttccagcgatcttgtgacattcagacgcccgtggccccattttttccagtcacgataacgtttttccgaacctggcagttgccaccagcctgggtcaaacagcgtcgtattgcgcgtgatcaccccggcgctcaatgccgaaaccgccacatagggtttaactgtagacgcgggaggataaaccccctgtgtggcgcggttcaccagcggtgtattcggatcgttcaacaaggcggaataatctttgctggagataccgtcaacaaacaagtttgggtcataactaggcgtggaaaccagcgccagcaccccacctgtacgcggatcggtgactaccacagctgcgcggctacccgccagcagcgtttcaatatattgctggagtttgagatccagcgtcaggtaaatatcgtgtccggcttgcggtggtacttcttttaactggcgaataacacgcccacggttgttaacttcaacctcttcataaccggtctgaccgtgcagcacatcttcatagtaacgctcaatgcccagcttaccgatatcatgcgttgccgcatagttggccagtttgccgtcattattcaggcgttcgacgtctttatcgttgattttcgacacatagccgatgacgtgggtcaacgccgaaccgtaaggatagtaacgacgtttatagcctttaacttcgacacccggaaaacggtactgattgacggcaaagcgagctacttgtacttcggtcaggttagttttcaccggaatagaggtgaaacggtgtgaacgtgcgcgctcttttcggaatgcagcaatatcgtcatcggtcagatctaccacgctgcgcaaagcgtccagcgtttgctgcacgttatcgactttctccggcatcatttctatctggtagatagtgcggttgagggccagagggataccgttacgatcgtagataatgccgcggctgggcgcgataggcaccagcttaatgcggttttcattagagcgggtctggtagtcggtaaagcgaacaatttgcagattatacaggttggcgataagcacgccggtcagcagcaaaatccccaaaaaggcgaccagcgcccggcgcacaaacagcgcggactctgccgtatagtcgcgaaaagagttctgtagtttcatccgctgcgttttctactcaaagctcccttatcactcacggtgataaggatggttggtggtgatgctccacgcccggtacagactctctgcgaccagcacgcgaaccagcggatgggggagggtaagcgccgacagcgaccagctctgctcagccgccgctttacaggcaggcgacaacccttcaggcccgccaatcagtagactgacgtcgcgaccatccagcttccagcgttccagctcagcggctaactgcggcgtatcccagggcttgcctggaatatcgagggtgacaatgcggtttttgcctgcggccgccaacatctgctcaccctctttgtcgagtatgcgcttgatgtccgcattcttgccgcgttttccggccggaatttcaatcagctcgaagggcatatctttcggaaaacgacgcaggtactcggtaaaaccggtttgtacccagtccggcattttcgttcccacggcgacaagttgcagcttcacgcattaactccagagtttttccagttcatacaggcgacggctctcttcctgcatgacatggacaatcacatcgcccaaatccacgacaatccagtcggcgctgttttcaccttctacgccgagcggtaacaggcccgctgcgcgagactcctgcacaacgtggtcagcaatggacataacatgacggctggacgtacccgtacagatgatcatgcagtcggtgatgctggatttgccctgaacgtctaaggcgatgatgtcctgacctttgaggtcatcaattttgtcgataacaaaatcctggagtgctttaccctgcaagttttccccctgggtgaatcaaatagataaaaatggtctgtcagtatacctgaaccagaggcgatttcgggacaattgtcgccgaatcggctttcgaaagtgggctatcatcccaccccgcgccgcagattgcatcgccatttttgtaaaacaatttctacaaagtcgtgtctggcggaaaaagtctggctgcggagaatatcagcctgcccgggtctgtcaatggtcgttgcggcttacccgtaaaaaaacagaaaagtcatgcattctcgaccccgatggcacggctattgaggacgcgtagcgtcgcgaatttttggttgatatcaatggcgctccaacacccctggtcaacgcgaaaatgccacatagcttcggcaggcatgccaattaaacgggcgattaacagactcagtacaccctgatggctgacgactaaaatattctgatagtgctgaaattcactaagccttgcgataaagcgttccacacgttgcgaaaatgcctgaaatccttcaccgttcgtggggattgcatgctgccagtcattgcaccacgcgctatagttttcggcatcttcttgcatgaggtcgcgatgatgtcgcatctcccagtcgccaaaaaacatttcgttgagttcaggtatgatttgcacggggagctggcggtcactgagaaccagtcgcgcggtatgctgtgcccgttccagttcactgcataaaaccagatcaaaggaaacaccatgtagcagcgtatgcagattttgcgcttgctcaataccgcgcgcggtcaggggggtgggcgcatgaccgctgtaaagaccatcgatattcgcttgcgtttcaccatgacgaattaaccacagtcgcatcatgccctccgtaacgacaggtatcagcgatacaagccttgttggttaatgtaagtcagtaccggttccggcaataaatcctcacatgattcaccgttttgcaaacgttcgcggatgatggtcgccgagatgttaaaccacggcgtttcagccagataaattttaccggcaggctgaaggtgaagatcttccgggttatgtgtcaaatgatcttccagccattgctggtattgcggttgcgccatttcaagtgggtaacctggacgccgacagacgatcaaatgtgcattgtcgagtatcgtttcgtattcgtaccaggtcggaaaggtcagcagtgaatcctgaccaataataaacgccagcggcacgtccggtccttgttcctgccgccactctttcagtgtttgcgcagtgtaagagggggcattgcgctttagctcgcgttcatcaagagtaaataatggcttgtcggcaatcgccagttcaagcatgtgtttacgctgcacgctgttcgcttccggctggggacgatgcggaggaacattattagggatgattgtgacccgcgtcagaccaatcaaattcgccagcgtttccacgggttttagatgaccatagtgcaccggatcaaaggtgccgccaaacagagcctgtaaagatttcatatcaaccgtcgataaatacgtccgccaggggtttatggcacaacagaagagataacccttccagctctgcccacactgactgaccgtaatcttgtttgagggtgagttccgttcgtgtcaggagttgcacggcctgacgtaactgcgtctgacttaagcgatttaacgcctcgcccatcatgccccggcggttctgccatacccgatgcttatcaaacaacgcacgcagtggcgtatgggcagactggcgtttcaggttaaccagtaacaacagttcacgttgtaatgtgcgcaacaaaataaccggttcgctgccttccagacgcagttgctgaagaatatgcaatgcgcgcttactttttcccatcaacaaagcatcaacccaatgaaaaggggtgaaatgcgcggcatcattcaccgcctgttcaacgcgcggtaatgtcaatttgccgtctggccagagcagcgataaacgctccagtgcctgagccagcgccagcaggttaccttcataacagtagcagagcacctgatttgccgcgtcatccagttctaagttgagctgttttgcgcgcgcagcaacccagcggggaagctgagcctgctccggtgtctgacaggtcacctgcacgctgcgattcgcaagcgcagtaaaccaggcggcattttcttgcgctttgcttaatttattaccgcggacgatcaacagcaggtcgtcatgcagaagtccggtgagtgtgagaagttgctcattgatcgccgcattcggtccgttttctggtaacaacagcaatagcgtttgtcgactggcaaacagactcatagcctggcataacgaaaagatcgcattccagtcagtgttgggatcaatggaaaaagtgtggtgttcttcgaatccttgtgccgcagctacctgacgaacagcgtcctggctttcctgcaataacagaggatcgttaccaagtaaaagatacgccgcgcgcagcccttcattgagctgcgcgcggagttgttccgggtacaaccgaatcatcagttacccagcgtggtggagacgcgtgcaggcgttgccggagtatccgttgtggtcgacgtctgttcttcgtcggaacgaatatccgcagcacggatgcttggcagcttacgaatcagctgttcggcagcacggtcgtacatctcttttacgatcatgtcttgttcgttatctttcgctaacgccatttgcgggttatcgaagaacgaacggaagactttggcgctaatcgggtagatatcacggccggggatcaacacggtcgcattaaccgtcatgatcatctgatactctgctgtttgaccgttacggaataccgatgcggtatctttcgcgatgctcactttacccaaacgcaaggatggaacgtccttacgcgtggtttctttatcaagcaactcgacaccattcagacgtaactggttacgcaccgcacggcttaatggcccgttcggatcgcctgagtccaggatcatgaccttcatagtggaaggaacctgcgtggtatcacgcagatgccagccacacccggcggtgattaacaccgccagagataacaacaatgttgccagatatcgcacgcttcctcccgcgcttagccaacgaccagattgaggagtttacctggtacgtaaatcactttacgtacagtaacgccatcaagatattttgctaccagatgttcctggccagcacgttcgcgaacctgttcttccgttgcgtccaccggaacggtgattttggcacggactttaccgttaacctgcaccacgaccagcgtggagtcttccaccatcgctttttcgtcagcaaccggccacggcgcgttgtcgatatcgccttcgcctttcagttcctgccacagcgtgaagcagatgtgcggggtgaacgggttaagcatacggacaacggccagcagtgcttcctgcatcagagcgcgatcctgctcgccatcggttggtgctttcgccagtttgttcatcagctccataatcgccgcaattgcggtgttgaaggtctgacgacggccgatatcatcggtcactttagcgatcgttttatgcacatcgcgacgcagcgctttctgattttcagtcagcgcatcaacgttcagtgccgcaacatcaccttttgctgtgtgctcgtaaaccagtttccagacacgtttcaggaagcggttagccccttccacaccggattcctgccattcgagagtcatatcagccggagaagcaaacatcataaacagacgaacggtgtccgcgccgtaacgttcaaccatcacctgcgggtcgataccgttgttcttcgacttggacattttgctcatgccggtataaaccagttcatggcctgccgcatctttcgctttcacgatacggcctttctcgtcacgttcaacgatagcatcaaccggggaaacccagttacgttcgccgttttcgccaacatagtagaaggcatctgccagcaccataccctgacacagcaactgtttcgctggttcgtcagagttcaccatgcctgcatcacgcatcagtttgtggaagaagcggaagtagagcaggtgcataatggcgtgttcaataccaccaatgtagatatccaccggcagccagtagttagccgcttcggaatccagcataccttctttgtactgcgggcaagtgtagcgcgcatagtaccaggaggactccataaaggtgtcgaaagtgtcggtttcacgcagtgctggcataccgttaacggtagttttcgcccactccggatctgctttaatcgggctggtaatgccgtccattaccacatcttccggcaggatcaccggcagctggtcgtccggggtcggcattacggtaccgtcttccagcgtcaccatcggaatcggcgcgccccagtaacgctgacgggaaacaccccagtcgcgcaggcggtagttcactttacgctcgccaacgcccatcgcagtcagtttatcggcgatggcgttgaaggccgcttcatggtcaagaccgttgaactcgccagagttgaacagcacgcctttttcagtcagggcttgctgagaaagatctggctcagagccgtcagctgccaggataaccggtttgatgttcaggccgtatttagaggcaaactcgtagtcgcgctggtcgtgccccggtaccgccataactgcgcccgtgccgtactccatcaatacgaagtttgctgcccaaacgggaatttcttcgcccgttaatgggtgaaccgctttaaagccagtatcgacgccttttttctccatcgtcgccatttcagcttcggcaactttggtgttacggcattcgtcaataaaggccgccagttcaggattattttccgccgctttctgcgccagcggatgacccgcagctaccgccaggtaggtacaacccataaaggtgtccgggcgggtagtgtaaacggtcagcgtgttgtcatagtcgttaacgttgaaggtgatctccacgccttcggaacgaccgatccagttacgctgcatggttttaacggtgtctggccagtgatccagtttatccagatcgttgagcagctcgtcagcgtaagcagtgattttgataaaccactgcgggatctctttacgttcaactttggtatcgcagcgccagcagcagccgtcgataacttgttcgttcgccagtacggtctggtcgttcgggcaccagttgaccgcagaagtcttcttatataccaggccttttttatacagctcggtgaagaatttctgttcccaacggtagtattccggcgtacaggttgccagctcgcggctccagtcataaccaaagcccagcattttgagctggtttttcatatacgcgatgttgtcgtacgtccacggtgccggagcggtgttgtttttcaccgccgcgccttccgcaggcagaccaaacgcgtcccagccgatcggctgcaggacgtttttgcccagcatacgctggtagcgggcgatcacgtcaccgatggtgtagttacgtacgtggcccatgtgtagtcgaccagaaggatagggaagcatagacaggcagtaatacttctctttgctctcgtcttcggttacttcaaatgtgcgcttctcatcccaatgaagctgtactttggattctatctcttccgggcggtattgctcttgcatggcagccagtggtcctgttttcaatacggctacaaatgtagcgttgaggtggtttttcagatccgcatagcatagcccaaacgtccgcgtcaaaacagcctttcgcgcactcgacgttgaaatgatgcccggattattcatacattaatttacagagtttgtgggcgtattagcaaagcaaggaacaaagaacgtctattattatagtcagttaacgacccgggagatgaaacgatgaacaaggttgctcaatattaccgtgaactggttgcgtcactgagcgaacgcctgcgcaatggcgaacgtgatatcgacgcactggtggaacaggcgcgcgagcgcgtaataaaaacaggggagttaacgcgaaccgaggtcgatgagctgacgcgagctgtcagacgtgacctggaagagttcgccatgagctatgaagagagcctgaaagaagaatctgacagcgtctttatgcgggtgattaaagaaagcttgtggcaggagctggcagacatcaccgataaaacgcagcttgaatggcgcgaagttttccaggacctcaatcatcatggggtttatcacagcggagaagtggtcgggctgggaaatctggtctgcgagaaatgtcacttccatctcccgatctacacaccggaagtgctgacgctatgcccgaaatgtggtcatgaccagttccagagacgcccgtttgagccgtaatagtctgatttcgcacagcaataaagagaatatgggccgaatgaaattccccggcccttgtttttatctctacagtaaatcttcagtctcacgaatttcctgactgacatctctggttccggatgactgaactttacgatacaggtcgagagcctgtcggagatcgacaggtcttccttctccgtagtgatacataatggccaggttataccaggcagtggcgtcattgcattcagcggctttcgtaaaccattcaaaggcagcctgataatctttctcaacgccttgtccgtgtttatacatataaccgatgttgacgtaagcgccgacgctcccctgagcggcagccttcagataccagtacatcgcttgcttatagtcctggtccaccccttcgccagcgttataatcccatgcaatttgaaactgggcgtgccgattaccctgctgtgcgcttttcaaataccagaatgcggcgagtgtcttgttttgagcaacgccttttccgtcttcataaagatcggccagattgttttgcgcgtcactatggccttgtaatgcagcttgtttgtaccagaaaaatgccagcgcatagtcttttgcgactccgttgccatttctgtacatccacccaagattattttgcgcataagacattccgctctccgcggctatctgataccagacaaccgcttctttataattgggggcttctccacgatccagtgtccagccaagggcgttggaagcgaaagtatggccttgtagggcagcttttttcagccagaagatggcttgctcattatctttatgacggcttttatcctcggtatacttttgccctaaggaatactgtgcttcacaatgaccttgctcagcggccagcttcagccagtaaaaggctttttcgtcgtccggagaatcaattgcgctatcgcgattataataaaacccaacaatatattgagcctcgcaatcgcctttttcagcacgttcgataatctcatctattgataaattatcgcagcaacttgacgtgaaaatcattatcatttccttatggttgcagataaaacatattatatttttatgtgttccatttttgcgtaagccttattttatgcgtattatgtcgcgtcagaaaagtataaataaacgagcctcgcaatgcggctaatattcatttaatgaatatttaaggataaattatatggacatggagtcgcaaaaaatattgtttgcactttccactccgatggaaatacgcaatgaatgctgtttaccttcgcattcatcacccaaaatgtatttaggtacatgcttttttgacctttcttcctcatggggaattgatgaccgtgatgacctgctgcgcacaattcaccgaatgatcgataacggtcatgccgctcggttggcagggttttatcaccgctggtttcgttattcgccatgtgaatggcgtgactatcttgctgaactaaatgagcaaggtcaggcttatgcgcaatttgtcgccagcaccgccgaatgctgtggcgaagggggaatcaaagcctgggattatgtccggatgggttttttaagccgaatgggcgtacttaataactggttgagcgaagaagaaagtctatggatccagtcgcgcattcatctacgggctctacgttattatagtaactggcggcaatactttgccggttatacctttggtcggcaatattggcagtctcccgaagatgatcatctgcctttattacgcgaattcttagcgcgtaaagaatacgacgattccggcaatgatatgttttatcaattatttgccagtgatgatgcgtattaccctaccttgtcctggcaaccattggcttactattctgcatgcccggaaacgcttaaggatatgagcgacctatgaaaaattgctggaagatcctcgatatagaggaaacgactgacgtcgatattatccgccgcgcttatctggcgctgttaccgtcctttcatccagaaaccgatccgcagggttttaaacaacttcgtcaggcgtatgaggaggcgctacggattgcgcagtcgcctgctaaatctgtttggcaaccagaagaatatgaggtagcagaacatgaaattctgctcgcctttcgtgcgttacttgcctctgatagtgaacgttttctgccctccgcctggcagcgattcattcagcaattaaattattgctcgatggaggagattgatgaattacgctggtcgctgtgcacaatcgccatgaacactgcccatttatccttcgagtgcgtggtgttattagcagaaagattgcggtggttacaggaggaaaataccggggaaatagacgaagaagaactggaatcctttttatatgccattgcgaaggggaatgtttttaacttccagaccattctgcatctgcccgttgccgtgcaaaatgacaccatcgatttttaccaaatgttcgctcggatttggtcatcgcatccacaatggctgacattgtatttagcgcaacatcgcgcagtgattatccccgatgatgcaaaactgcacagaaatttactccgctggtatagcgcaggtcgcctggatatccccgaacttctggattacgcccagtcatggcgggaaactgaacctgataatgaagatgcgccttattatgaatacgcgcaacgcgtctattgtggagaaggcgaaagcctgttggcagaactttgtgactactggcgcgagtatccctccacccaggcggatgctttaatgttgcaatggtgccgtcagcatcgggtcgattattacccattactggtgatgatgattgaagcgcgtgatctggttaacgatcagggaaaaccgctactttatgtccccggcgacagcgcccgtacgcgttttcatttatacgaaatactcagcgatgaaaaactctctgcgctggggcgttcactggtcgagatggttttgcacaaaggacgtaagccgcggatctcactcacgcgtgatacagaacataccttatggccattatatctagttgccaaacaattagtgcaggcctgccaacctacagaagaatcattaatgccgattgtgagccgccttgatgcagaaaatcgttgtccactggaagcattaattattcgtcgattattaattcaggcggcgaattttaccgagaagcaaactgttgaaccggagccgcaaccgcagccaatgcccgttgacgatggtgggccaggctgtctgggcatcattaaaattattttctatatttttatctttgctggtttgatagggaaaatactccatctgttcgggtgacagtcgacgttaatgtgcgggaagcccggcaagtaatctttccgcatttttgtaatgttgtttggcggtcagttttaaccatttttgagattcataatggttaacattaatacctgagccatttctgtagatcaaacctaaagtatattgagcatgagcatacccttgttcagctgcttccttataccagagaattgctttacgggtgtcgggtttgacccccagacctttgaggtagatccaccccagtttactttgcgcgcgtggattttcctgttccgctgattgctcataccagtatctcgcctgtgtataatccagtggtttaccgtcgctaccatgaagataaaattctccaaggcgatattgcgacgttgagtgaccatgaatcgcggaaagctccgtggctgccgtggtgaatggaagactgcccggtgagcttaaataatcaaaggcataattcaccatggctttatcacgcaacgtcgttttcttgggttggctaatacaggtaattgctgcaactataaaaattgcgaatatatacattaattttttattcatgtgtgaatgcttcgattttctttttattttgaaagcgtcaagtttatactcatcaataataaaaaagtagtcagttaatgcacttaagggattattaacaaatgaataaggaagaacaatatcttctttttgcgctttctgcgcccatggaaatacttaatcagggttgcaaacccgcgcatgactcgccaaaaatgtatactgggataaaagaattcgagctctcatcatcctggggaataaataatcgtgatgatttaattcagactatttatcagatgactgatgatggtcatgccaatgatttagctggcttatatctgacatggcatcgctcttcccctgaagagtggaaagcattaattgctggtggctcggagagagggttgatttatacccaattcgttgcccaaaccgctatgtgctgtggggaagggggaatcaaagcctgggattatgttcgaatggggtttctgtcacgggtcggtgtgctcaacaagtggctgacggaagaagagagtttatggctgcaatcgcgcgtctatgtacgagctcaccattactatcacagctggatgcactatttttccgcctattcgttaggacgtctctactggcaatcttctcagtgcgaagacaacacttcgctacgcgaggcgctaaccctgtacaaatacgatagcgccgggagtcgtatgttcgaagagctggcagcgggaagcgatcgtttctatgccacgcttccctggcagccattaactgtccagtctgaatgcccggtaacgcttaaggatgtgagcgacctatgaaaacatgttggcaaatcctcgaaattgaaagcacgacgcaaatagacattatccgccaggcttatcttgctcgcttaccgttgtgtcatcccgaaaccgatccgcaagggtttaaagcattacgccaggcctatgaagaggccctgcgactggcggtaaatcctgtcgaggaagcagatgatgaagaaaaagatgctgccgctgaacatgaaatactacgtgcattcaggacattactggattcagaaagtgatcgttttcagccttccgcctggcagaaatttattcagcaattaaatacctggaacatggaggatgtcgatcaattacgctggccgctgtgtgcaatcgccatagaagcgcgatatctttcattaaattgtgcttctttgctggcagagcgtttgaactggcattcatttaatgacagcgaaggaatggatgaggaagaaagggaggcttttcttgaggccattcaggctggtgattgtttcgatttccttagccttctggaatatcccattgcgttgcagaaccagactgttgagtattacttcgcgctggaacgttgctgccgttaccatcctgactatgtcactgcgtttttggcgatggaaggtccgtggttaattcctgatgatgcaaagttacatcgcaaactgttgcgctggtacagctcggtgcaaacaggtatggcggaactcattcctgtcgctcaacagtggcaaacggaagaaccagaaagcgaagatgcccggtattacttgtgtgcacaacgtttgtactgcggcgagggggaaagcctgcttgccgatctctgcgcgtactgggaaagttacccatctacacaagctgataatttgttgttgcagtggagcaagcgtcattgcccggattatttcgcgttattagtgatggttatcgaagcgcggagcatggtagatgcgcaaggtcaaccgctgaaatatgttcctggtgagagcgcccggacgcggctgttatgggcggagattttacatagcggaaaattatcgccgttaggtcaatcgtttattgagtcgttattcttcaagcgcaaagcatgggcgtggtggaaatcgagagtcggtagcgagacagagcaagattcaccgttcctggatttgtatcgggtagcggaacaggtagtacttgaagcgtttccgaaacaagagatgctggcccgtcttaatacaaggctggaaggcggagatgctcatccattagaggccattgtcacccggatgcttttgacgaaagtgaaactcgagccggaggatgaagatgtcgatgagccaacacctgaaaatcatgaagaaaaaaatgatgagggtgaaaaaccacagagcattaccagcattatcaaaatcagtttaacggtgctggtgataggttatgctctcggcaaaatcgcgatgttgtttagctgacgatgtgttttttgcgccgatgccggatgcagcgtttacgccgcatccggcagccgtgtttatgggatctcaatggctaaataatcgctcgcccgccgccgaacttcatccacgcgggccatatcgtttgactgcaacgccgcatcaaaatcggtgatcacccggccgatctcttctcgctcgtcacccagcgcccgcgcccacaactcttccagtttggctttaaaggtgcgattgatgagcatatcgcgcggataaattttcaatgcggataaccgcgtccgactctcttcaatctgctgcgcgctcaatgttaccgggctgtggttaatcactctggacttaacgctgccgtcttccagaagcacgtcaacttcaagcaacccgttgatatcataactaaagcgaatatcaatcgactgataagccccggttttcttcaacggcacatcgaaggattccaccagaatgttgtttttaactttgtggttttctccctgatagacgttaaccgtaattgaatcctgttccgggtgcatggttgaataagtttctacacgcgacacgggcacagtggtgtttcgttcaataatcggcgagaaaatgccggaaacgccctggcggttaacttcaacgcccaacgagtaagggcaaatatcagtgaggattacctcttcaatatcttcactgcgtaagcggcaggcggcctggattgctgcgcccagcgcgacaatggtgctcggatcgtaactttgatacggtaatttgccaaacagacgcacggcgattcgctgcaccagcggcatttgtgacgcgccgccaaccagcaccagactgtcgatttgactcggcttcagacgcgcatcgcgcaacgcctgttcaatcggcactcgcaagcgattgagcagcggcaaccacaaatcttccagttcgttctcgtaaaattcgcattcccgcgtttcttcctgatactgccagcgaatgtgcaatggcgattgattgctacattttgccgcttccacacaggcgtacaaggctgccagttcactctcgttaagcgtggtcctggcgacatccgcgcgttttaaaacctcatcgaccagcatatgggtaaaatcttcgccaccaagaaagttgtcgccagcggaggcgtgaacttcaatcaccggcgtggcgtactcaagcaccgtaacgtcaaacgtgccgccaccgagatcaaacaccagcgaacgggtattttgttgggtatgcaggccatacgccatcgcagctgctgtgggttcattaattaagcgtaccgcatttaacccggctaactccgctgctaaacgggtatgcttgcgttgttcatcgctgaaataagccggaacggagatcaccacatctttaatcggacgttgcagaaattcttcggcatcttcttttaatgagcgtaataccaaagaggacagttctggcgcgttaaatgtgtcgctgcctaaccgccagttggtattactgcccattgcacgtttaaataacgctgccgttttatccggatgcgaagtacgccgtgatacagccggttttccgactaaaatatgattattttcatccatgctaattatggatggtgttaaatattcaccgaacttatttggaattaattgcgcggcaccgtctttccagacggcaattaaactattggtagtaccgagatcgataccaatggcgagttctgcattatccattgcatttatatcttgaaagaaaaagagataaacagattaagaccacccaggtaacgcgtggtgatcttaatcaatgacgtgtgttaagcgtaaaatttcagacgatcagccagtaaatcaacaaagccctgacgatcaacatcgaccattacggtggcattcggtttattgcctgtcagataataataatcaacaaccgtcataccctgggtatatttcccctgtgtttccacgccaacccagcgctcaacagaggtaaataactccggtttcaacagccaggcgatggtgcatgggtcatgcagtggtgcgccgacaaagccccatttttcgtctttatgatattcgaggaagaaatccagcagttcggcaacaatggttgaaacagggttaccaatcgcgcggaaacgctcggtgtcttcaacgtggatttgtgctttatgagtaacatccagaccggccatcaccaccgggatccctgactggaagacaatttctgccgcttccgggtcaacgtaaatattaaattcagccgcaggcgtccagttacccagccccatagcgccacccataatcacgatacgggcaattttgctatgcagttccggatggctattgagcagcaaggcaacgttagtttgcggtccggtagacacaatggtgacaggttccgcactttcacgcagcgttttcgccatcagctctaccgccgtacagttttgcggtgcgaatgtcggttccggtaatgccgggccgtcgagaccgctttcgccgtgcacattgtccgcgataatcaactcacgcattaacggttttaccgcgccgcctgctaccggaatatcggtgcgattaagcaaggtcagcatacgcagaacattgcgtaaggttttttctggtgtctggtttccggcggaagacgtaattgctttgacatcaagctctggtgaggcgagggcgagaactattgcgatagcgtcgtcatgacctgggtcgcaatctaacagaattggcagtgccattgttgctccttgttgtgtgcttctttgcgacaagggtaacgccaggatgtaacagatacgaggggcgaaacgataaagcgtgagatggcgcgcaattgggtatgcgcgccagagtgattaatgcaggattttcgcgaggaagtcttttgcgcggtccgatttcggatcatcgaagaaagcgtctttcggcgagtcttcgacaattttaccctcgtccataaagatcacccgattcgccactttacgggcaaagcccatttcgtgggtcaccaccatcatggtcattccttcgttcgccagttccaccatcacgtccagtacttcgttgatcatctccggatccagcgccgatgtcggttcgtcaaacagcatcgcaataggatccatacacaacgcgcgagcgattgccacacgctgctgctgaccgccggaaagctgcgccggaaacttattggcgtgagcagaaagcccgacacgctccagcagtttcagggctttttcacgagccggcgctttatcgcgtttaagcactttcacctgcgccagggtcaggttttcgataatcgacagatgagggaacagctcgaaatgctggaataccatcccgacgcgggaacgcagctttgccagatcggttttcttgtcgttaaccacgataccatcgacggtgatttcaccttgctgcaccggttcgaggccgttgacggttttaatcagcgttgatttgccggaaccagacgggccgcaaaccaccaccacttcgccttttttcacttcggttgagcagtcggtcagcacctgaaagtgaccataccattttgaaacatttttcagggtaatcattatgctgtccttcttttcaagtagctgaccaacaacgacgcgctaagactaataacgaaataaacaaatccggcaaacaggatcatctcaacctgcgtaccatcacgctcaccaatggttgaggcggtacggaagaaatcggccagggataacacatacaccagtgaggtatcctggaacagtacgatgccctgagtgagcagcagcggcaccatcgcgcggaacgcctgcggcagaataatcagtttcatcgactgccagtgagtcattcccaacgccagcgcggcgctcgattgaccacgagaaatactttgaataccagcacggataatctctgaatagtaggccgcttcaaacatcgaaaacgccaccatcgccgaaattaaacggatatcattttttggcgataatcccagcacgttttgcagaaaacccggcacgatcaggtaaaaccacagcaaaaccataactaaaggaatcgagcggaatacgttaacgtaggctttggcaaaccacgccacgggcgcaaagctggataaacgcatcaccgccagcatcgtgccccacaaaataccaatcactaccgccgtgacggtgattttcagggtgatcaccagcccgtcgagcagatatggcagggaagggacaatggaactccagtcaaactcgtacattatttgccccccatgttgccaggcaggcgaactttacgttcaaccagcgtcatcaccagcatgataaaagcgttaatcaacacatacgccagcgtaatggcggtaaacgactcccaggcatgggctgagtaatcgagcaatttacccgcctgcgccgccatatccaccagaccgatagtcgaggcgatggcggagtttttcaccaggttcatcatctctgaggtcatcggcgggacgataacgcgataagcattaggcagcagtacgtatcgataagcctgcggtagcgtcaggcccatcgccagcgcggcatttttttgccctcgcggcagcgactgaatcgcggcgcgtacctgttcgcaaacacgggcggcggtaaacagccccaggcagagcatggatgaaaggaaaaactgaatattgggatccagctcggccttaaaccacatgccgattttctccggcagcagctccgggatcaccagataccaggtaaagaattgcacaatcaacggcacgttgcggaacagttcgacatacaacgtacccagaccagagagaaaacggtttggaacggtacgtaaaatgccgaaaaatgaaccgacgaggaaagcgataatccaggcgcagatcgacaaagcgatcgtcacctgaaaaccactccagatccaaccaagataggtggtgttgccgaacggggcttgttgtaaaaaaataccccagttccagtctatagacataaatctactccagaaaaaagagggtagcagcgttaactgctaccctcgaagattgttacccagcgtattgcggttttcaggcccgatggggaacgaccatcaggcgtatagtctgtccgtgctacgtaacaatcgagagggctggaatttccgcccctggttcttgtaattagttcagtgccttgtcattcggttctttgaacagtgctttcatttcgtctgacagttcgaaattcatgttcaggtttttcggcggaattggatttttgaaccacttatcaaaccatttttccgcttcaccggaggtctgcacctgagcgatggtgtcatccatcagctttttgaactgcggatcatctttacgcaacatacaaccgtaggcctcctgagactgcggcttgccgacgatttcccagttgtctggtttcttcgctttcgcacgttcaccggccagcagagcgtcatccatcataaaggcaacggcacgaccgctttccagggtgcggaaagagtcaccgtgatctttggcgctgatgatgcgcatattcattttttgctcttcattcagtttgttgagcaaaacttcagaggtagtgccggaagtgacgactacggctttgtctttcaggttggcaaaatctttgatatcgccaccctttttggtcaacaggcgcgtaccgaccacgaaaatagtgtcagagaaagccgcctgtttttggcgttcgacgttgttggtggtagaaccacattcaaaatcgaaagtgccgttttgcagcagtggaatacggttttgtgaggtaatcggaatcagttttacctgcaagtccggtttgttgagtttctttttcactgcttcaacaatggcgttggagtaatcctgcgagtaacccaccactttttgctgattgtcgtaataagagaaaggcactgaagattcacggtgaccgacgacaatcacaccgtttttggcgattttgtccagagtactgcccgctgccggggcggcgtcatctgcctgtgccagtcctgcggaaagcgccagggcgaggattgctgtggcaggtttacgtaattgcatatccaactcctttatcttctgcgttaagaacgcatggatacccgttgtgagtgtttgtgttgttatcgtctgcaactttattgtgcagtgttgtgcctgttagggaaggtgcgaataagcggggaaattcttctcggctgactcagtcatttcatttcttcatgtttgagccgattttttctcccgtaaatgccttgaatcagcctatttagaccgtttcttcgccatttaaggcgttatccccagtttttagtgagatctctcccactgacgtatcatttggtccgcccgaaacaggttggccagcgtgaataacatcgccagttggttatcgtttttcagcaaccccttgtatctggctttcacgaagccgaactgtcgcttgatgatgcgaaatgggtgctccaccctggcccggatgctggctttcatgtattcgatgttgatggccgttttgttcttgcgtggatgctgtttcaaggttcttaccttgccggggcgctcggcgatcagccagtccacatccacctcggccagctcctcgcgctgtggcgccccttggtagccggcatcggctgagacaaattgctcctctccatgcagcagattacccagctgattgaggtcatgctcgttggccgcggtggtgaccaggctgtgggtcaggccactcttggcatcgacaccaatgtgggccttcatgccaaagtgccactgattgcctttcttggtctgatgcatctccggatcgcgttgctgctctttgttcttggtcgagctgggtgcctcaatgatggtggcatcgaccaaggtgccttgagtcatcatgacgcctgcttcggccagccagcgattgatggtcttgaacaattggcgggccagttgatgctgctccagcaggtggcggaaattcatgatggtggtgcggtccggcaaggcgctatccagggataaccgggcaaacagacgcatggaggcgatttcgtacagagcatcttccatcgcgccatcgctcaggttgtaccaatgctgcatgcagtgaatgcgtagcatggtttccagcggataaggtcgccggccattaccagccttggggtaaaacggctcgatgacttccaccatgttttgccatggcagaatctgctccatgcgggacaagaaaatctcttttctggtctgacggcgcttactgctgaattcactgtcggcgaaggtaagttgatgactcatgatgaaccctgttctatggctccagatgacaaacatgatctcatatcagggacttgttcgcaccttccttaggtaacatttagtttggctaaatgtaaagatattgctgttttattgtttgtttttgcgagatgcgccgcaccattccgaagcaaaattcttaaaatgcactcttttagtgctaccgctggattactgtggtgcaactaggttgtactgatgctgtttcagggtttgccttgtataacaaagcaatagatgtgccaaagttggataggagaatattgttatccggataatgcactgatgccgcatccggtgagcgtgccgaaatatgggatgtattccggcacgataagaagggattatttacgtcgctgacgcagactcatcaacacagcagcaaaaccaaacaatgccgtcagcacccacagcggccagttgccggtacgtgcgtatggtgtgagtccggtggtcggcgtcacgttagtggttaacacctcgcgggtgaactgcgggatcatcgcctgaatctcaccctgcgggccaatcaccgccgtaatgccgttgttggtgctgcgcaacagtgggcgcgccagctccagcgcacgcattcgcgccatctggaagtgttgccatggaccaatagatttaccaaaccacgcatcgttggagatagtcagcagatagtcggtatccgggcggaagttatcgcgcacttgctcgccgagaatgatctcgtagcaaatagccgcagtaagctcaataccatttgccgacagcggcggctggatatatggcccacggctgaacgacgacatcggcagatcaaagaacggtgctaacggacgcagaatcgactccagcgggacaaactcgccaaacggcaccagatggtttttgttatagcgatcggctgattcgtagctgtacggcgcacctttacccagcgtgatgatggtgttgtaggtatcgtagcggttctgcttattgagacgcgcgtcgacaatcccggttaccagcgagctacctttatcacgcaactcaccgtccagtgctttgaggaacggttgctgattaatttccagatcggttatcgccgactccggccagataatcaacgatgatttgcccatcagcggtgccgttgcgttgtagtaaatcttcagcgtattaagaagctggccttcgtcccatttcagcgattgcggaatatcgccctgaaccatcgaaacctgaatggttttctccggttgtggggtaaaccactggatgtaacgcagcgggaagggaagggcaaacagcacgacggccaccaccagcggacgccagttgcgtttgaccaacgccagtgccagcaggccactaaccatcatcagcaggaagttaatggcttccacgcccattatcggtgccagcccttttaacgggccatcaatctggctatagccgaactgtaaccacgggaagccggtcagtacccaaccgcgcagaaactcggtcacttgccagagggcaggggcggcaatcgctacgcgcagccaggtggttttcggccacagacgcgacagcacgccagcaaacagtccggtatacagcgacaaatacgccgccagcagcaccaccaggaagatgttaaccgggccaggcattccgccaaaggtcgcgatgctgacatagacccagttaataccgctgccaaagaggccaaatccccagcaaaagccaatagcggcagactggagtggacggcggttaaaggtcaacgcctgaagccccatcagcgaaataatcgccgcaggccagacgtcgtaaggagagaaggccagcgttccgcaggcaccgaataataacgccagcagcaggcgaatgcgctggcgttcaattaatgaggcaaaagccatgtagttatctatccagtttcggttttattcatccagcttcggctggggtgagtcatccgggattttgacatgaacctgaataatacgccgactgtcggccatcgccactttgaactggtaaccgtcgatgtcgatagtttcgccacgcgccggaagatgcccaaatgcctgcatcaccagaccaccgatagtgtcgacttcttcatcgctaaagtgggtgccgaacgcttcgttgaagtcttcaatggaagccagtgcgcgtacggtccaggtatgacgactcagctgacggaagtcgatatcatcttcttcgtcatactcgtcttcaatctcaccaacaatcagttccaggatgtcttcaatggtcaccagaccggaaaccccaccgaattcgtcaataacgatcgccatgtggtaacgctgagagcgaaactctttcagcatccggtctacgcgcttactttcaggaacgacaaccgcctgacgtaacactttgtccatgctgaaggcttcagcatcgctgcgcataaacggcagcaagtctttcgccatcagaatcccttcaatgtgatctttgtcttcgctaatcaccgggaaacgtgagtgggcggactcgatgatgacatcaagacattcgtccagcgtctggttgcgtttcagggtaatcatctgggagcgggggatcatgatgtcgcgaacgcgttggtctgcgatgtccatcaccccttcgagcatatcgcgcgtatcttcgtcgataaggtcgttctgcccggaatcacggatcagcgccagcagttcgtcacggtttttcggttcaccgtggaaaagttggctgagtaacagggagaaaaatcccttcttgttgcttatcgtgtcactactgtgtgaattgtcgtcgctcatggcgtcgtatgggttctcatgttagttaatcaaaacgccgtcgttaatcaccaacggcggggacgtctgccagtcaaatgcctggcaaattattctttctcggcaatgtacggatcctcatagcccagagcaagcataatctctgtttcgagggcttccatttcttctgcttcgtcatcttcgatgtgatcgtaacctaacaaatgcagactgccgtgcaccaccatatgcgcccagtgcgcctccagtggtttgccttgctcctgagcttccttctcaaccacctgacggcagataaccagatcgcccagtagcgacatttccatgccaggcggcacttcaaacgggaaggagagcacgttggtcggcttatccttaccgcgataggtcagattcagactgtggctttcggcggtatcgaccacgcgaatcgtcacttccgattcttcctgaaactgcgggatcaccgcattcagccatgtctgaaactggctctcttccggtaacccggaattatcttcacatgccagttgtaaatcgaggatcacctgactcatttttgttcctgttcttcgcgcttgcgttctgctgccagcgccgcttttcgtttttgttcggcttcttcccaggcttcataggcgttaacgatacgcgccaccacagggtgacgaaccacgtcttcgctgtggaagaagttaaagctgatctcttcgacatcggccagcacttcgatggcgtgacgtaagcctgatttagtattacgcggcaggtcgatctgtgtgacgtcgccggtgataaccgcttttgagttaaaaccgatacgggtcaggaacatcttcatctgttcgatggtggtgttctggctctcatcgagaatgataaacgcgtcgttcagcgtacgaccacgcatataggccagcggtgcgacttcaataacgttgcgctcaatcagtttctcgactttctcaaagcccagcatttcaaacagcgcgtcgtacagcgggcgcagatacgggtctactttctggcttaaatcgccaggcaggaagcccagtttctcaccggcttctactgccggacgagtcagcagaatacggcgaatttcctgacgctccagggcatcaactgccgcagccactgccaggtaggttttacccgtacccgccgggccaacgccgaaggtaatgtcatggtcgagaatattggcgatgtactgcgcctggtttggcgtgcgcggcttaattacgccgcgtttggttttgatattgaccgctttgccgtactccggcacgctctccgcgctttgctccagtacccgcgcttctttaatcgcaaggtggatctgttccggttcgatatcctgaatctgaccgcgcatcggggcagtatcgacatacaggctacgcagaatgtctgccgcagcggtgacgcaaatcggacggccggtcagtttaaagtggttatcgcggcgattgatctcgatgccgagacggcgttcgagctgcttgatgttgtcatcaaacgggccgcacaggctcaacagacgcgcattgtctgctggctccagggtgatttcgcgagtgtctatgttcaaaccgttcctcttatctgtatgccgccggaagctgaacattcaccggcctataaggaaattattcacgccacaggaaaaaggcgcaagcattgcaataaagatggggataaagagagaaaaaacaaggcccaccggaacggcaggcctgagaattacggctgataataacccacgccaaggtcgttttctttgcgggtacgggcaatcactgattccggtgtttctgccacgcgcagacccatttcatcttcagtacgcaccactttaccgcgcagagagttcgggtagacgtcggtaatttctacatcgacgaatttaccgatcatatccggcgtgccttcgaagttgaccacgcggttattttccgtacgcccggaaagctccatgatgctcttacgcgatgtaccttctaccagaatacgctgggtggtgccgagcatccggcggctccacgccatcgcttgctgattaatgcgctcttgcagaatatacagacgctgcttcttctcttcttccggaacatcatcaaccatatcggcggctggtgtacccggacgtgcagagaagataaagctgtagctcatgtcgaaattgacgtcggcaatcagcttcatcgttttctcgaagtcttcggtggtttcgccagggaagccaacgatgaaatcagaactgatctgaatatctggacgcgccgcacgcagtttacggatgatcgctttgtactccagcgccgtatgggtacggcccatcaggttcagaatgcgatcggaaccgctctgtaccggcagatgcaggaagctcaccagctccggcgtgtcgcgatacacttcgatgatatcgtcggtgaattcgatcggatggctggtggtaaagcgaatacgatcgatcccgtcgatcgcagcaaccagacgcagcagatcggcaaacgatccggtggtgccgtcgtagttttcaccacgccaggcgttcacgttctgaccgagcaggttgacttcacgcacgccctgagccgcaagctgggcaatctcaaacagaatatcgtcggacggacggcttacctcttcaccacgggtgtaaggcaccacgcagtaggtgcaatatttattgcagccttccatgatggagacaaacgcggtcggcccttcggcgcgcggttccggtagacggtcaaacttctcgatttccgggaagctgatatctacaaccgggctgcggtcgccacgcacggagttgatcatctccggcagacggtgcagcgtttgcggcccaaaaataatatcgacatagtgggcgcgctggcgaatgtgctcgccttcttgcgatgccacgcagccaccgacgccgataatcaggtctggattcttctcttttaacagtttccagcgacccaactgatggaagactttttcctgagccttctcgcggattgagcaggtgttcagcagcagcacatccgcttcttccgccacgtcggtcagttgatagccgtgggtggcatccagcagatcggccatcttcgatgaatcgtactcgttcatctgacagccccaggttttaatatggagttttttggtcatcgacttgctcttgcgaaatagtagccaggaatgcagggcgcatagtgtaatgctttgctgccgttgtgaccagtatgagcgttatcagcccttaggggtaaaaatcctgtaaacttaaagcatattgctaacaggatgattgaccatgacaaatcaaccaacggaaattgccattgtcggcggaggaatggtcggcggcgcactggcgctggggctggcacagcacggatttgcggtaacggtgatcgagcacgcagaaccagcgccgtttgtcgctgatagccaaccggacgtgcggatctcggcgatcagcgcggcttcggtatcattgcttaaagggttaggggtctgggatgcagtacaggctatgcgttgccatccttaccgcagactggaaacgtgggagtgggaaacggcgcatgtggtgtttgacgccgctgaacttaagctaccgctgcttggctatatggtggaaaacactgtcctgcaacaggcgttgtggcaggcgctggaagcgcatccgaaagtaacgttacgtgtgccaggctcgctgattgcgctgcatcgccatgatgatcttcaggagctggagctgaaaggcggtgaagtgattcgcgcgaagctggtgattggtgccgacggcgcaaattcgcaggtgcggcagatggcgggaattggcgttcatgcatggcagtatgcgcagtcgtgcatgttgattagcgtccagtgcgagaacgatcccggcgacagcacctggcagcaatttactccggacggaccgcgtgcgtttctgccgttgtttgataactgggcatcgctggtgtggtatgactctccggcgcgtattcgccagttgcagaatatgaatatggcacagctccaggcggaaatcgcgaagcatttcccgtcgcgtctgggttacgttacaccgcttgccgctggtgcgtttccgctgacgcgtcgccatgcgttgcagtacgtgcagccagggcttgcgctggtgggcgatgccgcgcataccatccatccgctggcggggcagggagtgaatcttggttatcgtgatgtcgatgccctgattgatgttctggtcaacgcccgcagctacggcgaagcgtgggccagttatcctgtcctcaagcgttaccagatgcggcgcatggcggataacttcattatgcaaagcggtatggatctgttttatgccggattcagcaataatctgccaccactgcgttttatgcgtaatctcgggttaatggcggcggagcgtgctggcgtgttgaaacgtcaggcgctgaaatatgcgttagggttgtagccttacaacattgccggatgcgtgccaaccgtaggtcggataagacgcggcagcgtcgcatccgacattgaaggataagacgtgtcaacatcgcattcgacattgaatgaacgcagaaaagcaaaaagctcgccgaagcgagcttttttaatgtggctggggtacgaggattcgaacctcggaatgccggaatcagaatccggtgccttaccgcttggcgataccccaactgggtgcacttacaaggtaagcgtcttgaataaattggctggggtacgaggattcgaacctcggaatgccggaatcagaatccggtgccttaccgcttggcgataccccaacaaattggttttgaatttgccgaacatattcgatacattcagaatttggtggctacgacgggattcgaacctgtgaccccatcattatgagtgatgtgctctaaccaactgagctacgtagccagattgtttcttcgatggctggggtacctggattcgaaccagggaatgccggtatcaaaaaccggtgccttaccgcttggcgataccccaataaccgggcggtgaaccgcttactcgaagaagatggctggggtacctggattcgaaccagggaatgccggtatcaaaaaccggtgccttaccgcttggcgataccccatccgtacaacgctttctggtgaatggtgcgggaggcgagacttgaactcgcacaccttgcggcgccagaacctaaatctggtgcgtctaccaatttcgccactcccgcaaaaaaagatggtggctacgacgggattcgaacctgtgaccccatcattatgagtgatgtgctctaaccaactgagctacgtagccatcttttttttcgcgataccttatcggcgttgcggggcgcattatgcgtatagagccttgcagcgtcaacctctttttcaaggaaaattgctcgaaagtgactgtttggttaggttgcgaacagcgtggcgctatattcgtcaattattgtttactttgtgttttttcccaccctacagccattcttttgtcatacaggatgaaattcggaatttaacaatagtggtgggaaattaatctatgaaatactggcctacagtgatgagttgtcaaacagtgatgtggcaaacccggaacatttccttactgcatatcagaatcaacaagcacctcaataactgaaacagccccggatttcaccggggctgtttcgcatttcttacttatacgccgactggtgaacaccaaccgcgcgaccagacggatcgtccattttcttgaacgcttcatcccattcgatcgctttagcggaagaacaagcgacggaaggaccgcccggcacgcactcagcggcgctcggaagcgggaatagttcttcaaagatctcccgatacaagtacgcttctttagaggttggcgtgttgtacgggaagcggaagcgggcagtttccagttgctgatcagaaacctgctgcgcagccacttctttcagggtgtcgatccaactgtaaccgacgccatcggagaactgctctttctgccgccaggccacgcttgcaggcagatacgcttcaaaacattcacgcaggatgtgtttttccattttgccgttaccgcacattttatcctgtgggttaatacgcatcgccacatcaaggaattttttgtcgaggaacggaacgcgtgcttccacgccccaggctgacatcgctttgttggcacgcgcgcagtcatacatatgcagggccagcagtttacgcaccgtctcttcatgcagttctttggcattcggtgctttgtggaagtaaagataaccgccgaacacttcatcagaaccttcaccggacagcaccattttaatgcccatcgccttgatcttacgcgacattaaatacatcggtgttgaagcgcgaatagtggtcacatcataagtttcgatgtggtaaatcacgtcgcggatggcatccagaccttcctgtacagtgaagtgaatttcgtgatgcaccgtgcccagatggtttgccacttcctgggctgctttcagatccggtgaacccggcagacctacagcaaaggagtgtaactgcggccaccaggcttcagagcgttcctgatcttccacgcgacgggctgcgtatttcttggtgatagcggaaataattgaggaatccagaccaccagaaagcagcacaccgtaaggcacatcagacatcagatggcttttaactgaatcttccagtgcctgacgcagctcgtttttgtcggtcacgttatctttcaccgcatcgtagtcgaaccagtcgcgatgatagtaagaacggatttcgccgtcctggctccacaaatagctccccgccgggaactctttaatcgtgcggcaaactggcaccagcgctttcatttctgaggccacatacagctgaccgtgttcgtcataccccatatacagtgggatgatccccagatggtcgcgaccaatcaggtaggcatctttttcgctgtcgtacagtgcaaaggcaaacatgccctgcaagtcgtcgagaaattccggccctttttcctgatacagcgcgaggatcacttcacagtcagacccggtctggaactggtaacgatcgccatattcggcgcgcaatgcctggtggttgtagatttcaccgtttaccgccagtacgtgggttttttgttggttgtagagaggttgcgcccccgcgttaacgtcaacaattgacagacgttcgtgggcgagaatggcgttatcgctggcataaataccggaccagtccgggccacgatgacgcatcaggcgtgacagctcgagggctttcttacgcagctcaactgcgtctgttttgatatcgaatacgccaaaaattgaacacataaccttctccgttaacctggtatttgttgcttgttgtgtttgcttgtttaaaaaaatgccgcaaagcagcactgtgcgcaagcgatttggcggtgaaaaaataaaaaacgtaatggtgattgtcgattggtgaaaaaaggtctggtgtgaggatatatttattgatgaatcgataatttttagcgggttttattgaatgtttatattttacgggggccaaattgctgacaaagtgcgatttgttcatgccggatgcggcgtgaacgccttatccggcctacaaaagcatgaaaattcaatatattgcaggagctgcgtaggcctgataagcgtagcgcatcaggcagtttggcgtttgtcatcagagccaaccacgtccgcagacgtggttgctattcagataacgtcgatttcagcgactgacgggtaaatccagctggggcggaaaggcatactgtcgatatcgtcgagcgacgaaacaccagaaagcaccagaatcgtctccagacctgcctggaagccggccagaatatcggtacgcaggttatcgccgacaatcaccgtttcttccgaatgcgcctgcattttgtttaatgctgcgcggatgatccacgggctgggcttaccaacatagaacggtttgcgcccggagattttctcaatccctgcacacaacgcgccacaagcgggataaaaaccgcgcccgtgggtgtccggattggtggcgataaaacgtgcaccgttagcgacgaaataggctgctttatgcatcatgtcccagttgtaggaacgcgtttcgccaacaatcacgaaatcagggttcacatcggtaatagtgaaaccggctttgtacagttcatgaatcagtgcgccttcgcccaccacatacgctttcttgccttcctggcgacgcaggaaatcggcagtcgccatcgcagaggtataaaacacgctgtcaggtacatcgacacctgcggtggcaaagcggttcgccagatcttgcccagtctgcgaaggatagttggtcagcaacaccagcggcaggcctttatccataatcccgtgcaaaaattccgctgcacccggtacggcgacgttatcgtgcatcagcacgccgtcgatatcgcaaattacatttttaatggtcatggactacccagaatattgacaacaataagcgccactataaaagcacattaattttccagcaaatgctggagcaaaataccgttgagcatggcgcgttttaccagcgcaaaagcgccgattgccgagcggtgatccagctcagaacgtaccaccggcagattagtgcgaaacgccttcagcgcctgggtattaatgcagctttcaatagcagggagcagcactttatcggcttcggtgatttcaccggcaataacaattttttgcggattaaataagttgatagcaatggcgatggttttacccagatgacgaccgacatactcaattacttccgacgccagactatcgcctttgttcgcggctttgcagatagttttgatggtgcagtcgtccagcggcacgcggctctggtagccctgctttaacagattcaacacccgttgttcaatggcagcgttggcagcgatagtttccaggcagccaaagttgccgcagtggcagcgttcacccagcggttcgacctgaatatggccaatttcaccgacgttgccgttgcggccaataaaaatgcgcccgttagagataatcccggccccggttccgcgatggacacgcaccagaatggagtcttcgcaatcctgacttgcaccgaagtagtgctccgccagcgccagactacggatatcgtgaccaacgaaacaggtcactttaaaacgttcttccagagcttctaccagcccccagttttctacctgaatatgcggcatgtaatgaattttgccgctgtccgggtcaacaagccctggcaggatcaccgaaatcgcgatcagctcgcgcagtttgcgctggtagctatcaataaactgagcaatggcattcaacagggcatgttccagcgtttgctgggtacgttccggcagcgggtaatgttcttctgccagcactttgctgctgagatcaaacagagtgatggtggcgtcatgacgaccaagccgtacgccgattgcgtggaaattgcgggtttcggtgacgatggagatagcgcggcggcccccggtggaggcctgctgatcaacttctttgatcagcccgcgttcgataagctgacgcgtaattttggttacgctggcgggggcaagctggctttgctcggcaatctgaatccgcgagattggcccgtactggtcaatcaggcgataaaccgccgcgctgttaagctgttttacgagatcaacattacctatctgagcttgtccgcctggtgtcatactttctcttattgagttacgacctcgttaccgttaacgatggtcttggtgattttaaaatcaggtgtgaatgcagtcaggttggctactttacctgcggcgagtgtgccgagacgtttctcaacgccaatcgcacgcgccggatagagcgtcgccatacgtagcacttcatccagtgcgataccgcaatgttcgaccagattacgcacgccttcaatcatggttaaggatgaaccgcttaacgtaccgttctcatccacacaaagtccgttacggtagtatattgttttacccgcaaaaatgaactgttcaatgttggcacctgctggcgcggtggcgtcagtaaccagacacagtttgtcgcctttcagacgtttagcgttgcgaatgttggcgtaatcaacatgcaggccatcagcaataataccgcaataaatgtcagcttcgtcgaggatcgcgcccgccaggccaggttcacgaccggtaatatacggcatcgcgttgtacagatgggtggcaaaggtaatccccgcgcggaaaccggcttttgcttctttcaacgtcgcgttggagtgaccggcagaaaccacaatcccggcatttgccagtttgctgatgacttccgcaggaaccatttccggtgccagggtcactttggtaatgacgtcggcgttttcacacaggaaatcgaccagcgcggcatcaggcttacgcacaaaattcggattatgggtgcctttttttaccagattcagccacggaccttccagatgcagacctaacgcctgattcggatgttttgccaggtactcgcgcataacgcgcacgccctgtttcatcagctcatcgctggtggtgataagcgtcggcagatagttagtacagcctgatttctcattggctttctgcatgatttccagcgtttccacgctgaccgcttcagcggtgtcgttaaactgtacgccgccgcagccgtttaactgcacatcgataaaaccgggggagagaatggccccgttcagtgaacgttgttcgatctctggcggcagttccgctaccggacagacgcttttaatcaggccatcagcgataacaaccgcgtggtcatcaagaaattcgtggccggtaaagatccggccctgggttaatgcatacattctgacccccgattttaaaaaatattgccctgagcaaggagccagggcagggataacaattacagacctttgatattttctgcttctaattcattgaaatatcttaaagtcttaactttcagctccatggtggaaggttcatcgcacaccatgatcgctttcggatgcagttgcagacagctgatggtccacatatggttcacgcaaccttcaacggcggcctgcagcgccagtgctttctggctacccagcaccagaatcatcacttcttcggcatccagcagtgtaccaacaccgacagtcagggcatattttggcacctgattaacatcgttatcaaagaaacgagagtttgcgacgcgagtgtcatgagtcagggttttgatacgagtacgagaagccagagaagacgccggttcgttaaatgcaatatgaccgtcgttacctacaccgcccataaacagatgaatttttccgtaagaacggattttttcttcatactggcggcactcggcgtcgatatccggggcgttgccgttgagaaggttgatgttttctgctggaatatcaacgtgatcgaagaaattacggtgcataaagctgtagtagctttccggatgctctttcggcagaccgacatattcgtccatgttgaaggtgacaacgtgcttaaagctgacctggcctgctttatgcatttcgactaacgctttataggtggtcatcggcgtgccgccagtcggcaggcccagtacaaacggacgatcggcagtcggtttgaacgcattgatacgattgacgatatggcgagcagcccatttgccgacctgttcagcggtagtcagggggatcagtctcattattcacctcaataagtaaaatgtaagccgttggcggattaggcatctttaagcgtaacctggatttgcgcagacaggcgtcaatccgacctgattttttgaatgataaaataagttttctggtttagccagtaaaagggagtgataataacgatatttggtgacaaaactcacaaaagacacgcgtttaatttgcgatacgaattaaattttcacacactctgtagcagatgatctaacaatctgattacagaacatcggcagtacaatttgcagcaaaataaaaatacggcttgaaacgagccaaatagggttctcgtagggggaataagatgaatattttaggttttttccagcgactcggtagggcgttacagctccctatcgcggtgctgccggtggcggcactgttgctgcgattcggtcagccagatttacttaacgttgcgtttattgcccaggcgggcggtgcgatttttgataacctcgcattaatcttcgccatcggtgtggcatccagctggtcgaaagacagcgctggtgcggcggcgctggcgggtgcggtaggttactttgtgttaaccaaagcgatggtgaccatcaacccagaaattaacatgggtgtactggcgggtatcattaccggtctggttggtggcgcagcctataaccgttggtccgatattaaactgccggacttcctgagcttcttcggcggcaaacgctttgtgccgattgccaccggattcttctgcctggtgctggcggccatttttggttacgtctggccgccggtacagcacgctatccatgcaggcggcgagtggatcgtttctgcgggcgcgctgggttccggtatctttggtttcatcaaccgtctgctgatcccaaccggtctgcatcaggtactgaacaccatcgcctggttccagattggtgaattcaccaacgcggcgggtacggttttccacggtgacattaaccgcttctatgccggtgacggcaccgcggggatgttcatgtccggcttcttcccgatcatgatgttcggtctgccgggtgcggcgctggcgatgtacttcgcagcaccgaaagagcgtcgtccgatggttggcggtatgctgctttctgttgctgttactgcgttcctgaccggtgtgactgagccgctggaattcctgttcatgttccttgctccgctgctgtacctcctgcacgcactgctgaccggtatcagcctgtttgtggcaacgctgctgggtatccacgcgggcttctctttctctgcgggggctatcgactacgcgttgatgtataacctgccggccgccagccagaacgtctggatgctgctggtgatgggcgttatcttcttcgctatctacttcgtggtgttcagtttggttatccgcatgttcaacctgaaaacgccgggtcgtgaagataaagaagacgagatcgttactgaagaagccaacagcaacactgaagaaggtctgactcaactggcaaccaactatattgctgcggttggcggcactgacaacctgaaagcgattgacgcctgtatcacccgtctgcgccttacagtggctgactctgcccgcgttaacgatacgatgtgtaaacgtctgggtgcttctggggtagtgaaactgaacaaacagactattcaggtgattgttggcgcgaaagcagaatccatcggcgatgcgatgaagaaagtcgttgcccgtggtccggtagccgctgcgtcagctgaagcaactccggcaactgccgcgcctgtagcaaaaccgcaggctgtaccaaacgcggtatctatcgcggagctggtatcgccgattaccggtgatgtcgtggcactggatcaggttcctgacgaagcattcgccagcaaagcggtgggtgacggtgtggcggtgaaaccgacagataaaatcgtcgtatcaccagccgcagggacaatcgtgaaaatcttcaacaccaaccacgcgttctgcctggaaaccgaaaaaggcgcggagatcgtcgtccatatgggtatcgacaccgtagcgctggaaggtaaaggctttaaacgtctggtggaagagggtgcgcaggtaagcgcagggcaaccgattctggaaatggatctggattacctgaacgctaacgcccgctcgatgattagcccggtggtttgcagcaatatcgacgatttcagtggcttgatcattaaagctcagggccatattgtggcgggtcaaacaccgctgtatgaaatcaaaaagtaatctgctttatgcctgatgcgacgcttgagcgtcgcatccaacaatgacaagcggtggagatcttctctgccgctttttttttcatcaatcatccccataatccttgttagattatcaattttaaaaaactaacagttgtcagcctgtcccgcttataagatcatacgccgttatacgttgtttacgctttgaggaatccacgatgagtgaggcagaagcccgcccgactaactttatccgtcagatcatcgatgaagatctggccagtggtaagcacaccacagtacacacccgtttcccgccggagccgaatggctatctgcatattggccatgcgaaatctatctgcctgaacttcgggatcgcccaggactataaaggccagtgcaacctgcgtttcgacgacactaacccggtaaaagaagatatcgagtatgttgagtcgatcaaaaacgacgtagagtggttaggttttcactggtctggtaacgtccgttactcctccgattattttgatcagctccacgcctatgcgatcgaactgatcaataaaggcctggcgtacgttgatgaactgacgccggaacagatccgcgaataccgcggcaccctgacgcaaccgggtaaaaacagcccgtaccgcgaccgcagcgttgaagagaacctggcgctgttcgaaaaaatgcgtgccggtggttttgaagaaggtaaagcctgcctgcgtgcgaaaatcgacatggcttcaccgtttatcgtgatgcgcgatccggtgctgtaccgtattaaatttgctgaacaccaccagactggcaacaagtggtgcatctacccgatgtacgacttcacccactgcatcagcgatgccctggaaggtattacgcactctctgtgtacgcttgagttccaggacaaccgtcgtctgtacgactgggtactggacaacatcacgattcctgttcacccgcgccagtatgagttctcgcgcctgaatctggaatacaccgtgatgtccaagcgtaagttgaacctgctggtgaccgacaagcacgttgaaggctgggatgacccgcgtatgccgaccatttccggtctgcgtcgtcgtggttacactgcggcttctattcgtgagttctgcaaacgcatcggcgtgaccaagcaggacaacaccattgagatggcgtcgctggaatcctgcatccgtgaagatctcaacgaaaatgcgccgcgcgcaatggcggttatcgatccggtgaaactggttatcgaaaactatcagggcgaaggcgaaatggttaccatgccgaaccatccgaacaaaccggaaatgggcagccgtcaggtgccgtttagcggtgagatttggattgatcgcgccgatttccgcgaagaagctaacaagcagtacaaacgtctggtgctgggtaaagaagtgcgtctgcgtaatgcttatgtgattaaggcagaacgcgtcgagaaagatgccgaaggtaatatcaccaccatcttctgtacttatgacgccgataccttaagcaaagatccggcagatggtcgtaaagtcaaaggtgttattcactgggtgagcgcggcacatgcgctgccggttgaaatccgtttgtatgaccgtctgttcagcgtgcctaacccaggtgctgcggatgatttcctgtcggtgattaacccggaatcgctggtgatcaaacagggctttgctgaaccgtcgctgaaagatgcggttgcgggtaaagcattccagtttgagcgtgaaggttacttctgcctcgatagccgccattctacggcggaaaaaccggtatttaaccgcaccgttgggctgcgtgatacctgggcgaaagtaggcgagtaattttaagtttcgctatgccggatggggcgtttacgtcgcatccggcaaggaacagacaaacagtttcaaacgctaaattgcctgatgcgctacgcttatcaggcctacatgatctctgcaatatattgagtttgcgtgcttttgtaggccggataaggcgttcacgccgcatccggcaagaaacagcaaacaatccaaaacgccgcgttcagcggcgttttttctgcttttcttcgcgaattaattccgcttcgcaatttatccataaaataaatttaaaataacaaaacataattaaataaaatgtaaccgctttcatcttgctggaatttcacgcttttattcttctgcaagcctttcaaccgcaaacttaagccttgtaacaaaaatcatcaaaatatgtgcggttgctcatgttcttacattctggttacagaaagagattgataattcgcgtcgcgaaaaatagtctgttcctgtagtcagcgagacttttctcaacgctacttttttaatttttattttttcgctgttcacctttggtgcagcaatttatacgtcaaagaggattaacccatgcgtacgtttagtggcaaacgtagtacgctggcgctggctatcgccggtgttacagcaatgtcgggctttatggcaatgccggaggctcgcgccgaaggattcatcgacgattcaaccttaaccggcggtatctattactggcagcgtgaacgcgaccgtaaagatgttaccgacggcgacaaatacaaaaccaacctttctcactccacctggaatgccaacctcgattttcagtccggttatgctgctgatatgttcggccttgatattgctgcgtttacggcgattgaaatggcggaaaacggcgacagctcccacccgaacgaaatcgcgttttcaaaaagtaataaagcctatgacgaagactggtccggcgacaaaagcggtataagcctgtataaagctgcggccaaatttaaatacggtccggtttgggcgagggcaggttacattcagccaactggtcaaacgctgttagcgccgcactggagctttatgccaggtacttatcagggggcggaagccggggcgaattttgattacggcgatgctggtgcgttgagtttctcctacatgtggaccaacgaatacaaagcgccgtggcatctggaaatggatgagttttatcagaacgataaaaccaccaaagttgattatctgcactcctttggggcgaaatacgacttcaaaaataacttcgtactggaagcggcatttggtcaggcggaagggtatatcgatcaatattttgccaaagccagctacaaatttgatatcgccggtagcccgttaaccaccagctaccagttctacggtacccgagataaagttgacgatcgcagcgtcaacgacctttatgacggcaccgcctggctgcaagcgttgacctttggttaccgggcggctgacgtagtggatttgcgcctcgaaggcacctgggttaaggctgacggtcagcagggatacttcctgcaacgtatgactccaacctacgcttcctcaaacggtcgcctggatatctggtgggataaccgttctgacttcaacgccaacggcgaaaaagcggtcttcttcggtgcgatgtatgacctgaaaaactggaatcttccaggcttcgccatcggcgcttcctacgtttacgcatgggatgctaaacctgcgacctggcagagcaatccggatgcgtactacgacaaaaaccggactattgaagagtctgcctacagcctggatgcggtctataccattcaggacggtcgcgccaaaggcacgatgttcaaactgcatttcaccgaatacgacaaccactccgacatcccaagctggggcggtggttacggcaacatcttccaggatgagcgtgacgtgaaatttatggtaatcgcaccattcaccatcttctgatgcccgacgcggcaggttttgtgcctgccgcacgtttgaggaatttgctatgaaaaaactgattctcatcgccataatggcatcggggctggtagcttgtgcgcaatcaaccgcgccacaggaagacagtcgtctgaaagaggcatacagcgcctgtatcaacaccgcacaaggttcgccagaaaaaattgaagcctgccagagcgtgttaaacgtgctgaagaaagagaaacaacatcagcagtttgccgaccaggaaagtgtacgcgtactggattatcagcagtgtctgcgtgcaacgcaaaccggaaatgatcaggcggtgaaagccgattgtgataaagtctggcaggaaatacgcagtaataacaaataagtgagagctgtaactctcgcttttcttatttcccttgcataaaaaagccaacccgcaggttggcttttctcgttcaggctggcttatttgccttcgtgcgcatgttcatcttcgcggcaatcgccttcggcacagtgaccgtaaagatagagactgtggttagtcaggcgaatgccatgttttgcggcaatttcacgctgacgcgcttcgatggaatcatcactaaattcgataaccttgccgcagtcgaggcagatcaggtgatcgtggtgatgttgctgtgtcagttcaaatacggatttaccgccttcaaaattgtggcgggtgacgataccagcgtcgtcaaactggttcagtacgcgatataccgtagccagaccaatttcttcacccatatcgatcagacgtttgtataaatcttccgcactgacgtgatggttgtccggctcctgaagaacttccaggatttttaaacgaggaagcgttactttcaggccagctttctttagggcggtattgttatcagtcatgcggaatctgtcctgttactaagcggttcacttcattagaagaagtgacagaatttgctcttgagataatgcgtatcattatagaattgccacgcctaaatgaaaaccacaagtccctggcaaatattgttaataaaaacgtggcacagcttacatttacaacggcaaggccacttgaacaccgggacattgtacaggtacaacagcaaaagttacaaatttgtagcaattattttgattggcattatctattaatacggcgtagacatgagtctacgccgcatcacatcaggcattgagaatttcgtcgagatgcaactcttcagaaatctgtttaacccatttttctacacgttcagcggtcagttccggctgacggtcttcgtcgatagccagaccgacaaagtggtcgtcatctgccagaccttttgatgcttcgaaatgatagcccgcagttggccagtgaccaacgatggttgcaccgcgcggttcaatgatgtcgcggatggtgcccaatgcgtcgcagaaatattcggcgtaatcttcctggtcaccacaaccaaacagcgcaaccagtttgccgttgaaatcaatctcttcgagagtcgggaagaagtcatcccagtcacactgcgcttcgccgtaataccaggttgggatgcccagcagcagaatgtcataagcttccagatcttctttgctgctttttgcaatgtcatggacatcggcaacgtctttaccaagctgtttttgaatcatttttgcgatattttcggtattaccggtgtcgctgccgaaaaagatgccagtgatagccatgagtgaaataacctcttgaaacttattgaaatgggggtggaaaattgcccacggataaaggcaatcatagcagaacaggcagtcttgcggaatcagcaaacgagcaggactgcacactgtgctacatgaaagtggaaatttaaacgatgccctgactacgcagcgccgccagttgctgcattaacatctcttcgatcagttcgctacggctcatattgcgcgactccgccagctcgttcagcgcctcgacagcttccgcgttcagcttcagttcgacacgcttaaggccacgtactttgtcgcgttttagctggttgcgtttattaatacgcagctgttcatcgcgcgaaagcggattagttttcggtcgtcccggtcgacgctcgtgcgcgaacagatctaatgtcgtacggtccgtttgttctttggccatgatcttggtgacttcgggggaaacaatcagccaggcctctgcccggatggatagcgcgccataatacatcagcgcgatgagtcacgccaacgcccacgcgcggaaagcgacgcggacgctgggtttttaatcagttgcgttaatcattgagatagcgacggatagcgcgtaataccgcatccggtttttcagcatggacccagtgacccgcgcctgcaatcacatgcgcccgtgcctgtggaaattgagccagtaaatcatcacggtactgctcgctaacatacggagaattgccgccagggataaacagggcagggtgatcccatgccgggattttctcccaacctacaatatgcggatactgatcccacaataccggcacgttaaagcgccactccccgtcaacaaaagatttcagcagaaactgaatcaccccttcttcattaagatgctggcgcattattgctgctgcttgctggcgagtttgtgcgtccgattcactgaccgcgttgatagccgcaaaaatctcatcatgacggcgtacgtgatagtcgaccggcgcgatatcgatcgccaccagtttatcgatgcgatcggaggctagtgcagtaagtgccattaccgctttaccgcccatggagtgaccgataaatgttgctttgtcgatctgctgtgcatccagagtatcaacaagatcctgcgccatcgccgggtaattcattaccggatctctcggtgaaagaccgtggttacgcatatcaacctggatgatattgtgatcgtttaccagatcgcgagccagtacgccaaggttgtcgaggctgccaaacagaccgtggacaagaacgatgggagaattattgtgctggttttgtgcagtttgcgcgcggatattcaatttcatggcaaagttctttttttcgcgttgtcgggttagggtattatgttgaccattgtgccacagggctgcaacaaataaggtttattccgagtttttctgcaagccaggcttgacgctatccgctgccgggatttattcatatactcctggcgacttgtattcagctaagacactgcactggattaagatgaaaacgattgaagttgatgatgaactctacagctatattgccagccacactaagcatatcggcgagagcgcatccgacattttacggcgtatgttgaaattttccgccgcatcacagcctgctgctccggtgacgaaagaggttcgcgttgcgtcacctgctatcgtcgaagcgaagccggtcaaaacgattaaagacaaggttcgcgcaatgcgtgaacttctgctttcggatgaatacgcagagcaaaagcgagcggtcaatcgctttatgctgctgttgtctacactatattctcttgacgcccaggcgtttgccgaagcaacggaatcgttgcacggtcgtacacgcgtttactttgcggcagatgaacaaacgctgctgaaaaatggtaatcagaccaagccgaaacatgtgccaggcacgccgtattgggtgatcaccaacaccaacaccggccgtaaatgcagcatgatcgaacacatcatgcagtcgatgcaattcccggcggaattgattgagaaggtttgcggaactatctaaaacgttgcagacaaaggacaaagcaatggcaatccacaatcgtgcaggccaacctgcacaacagagtgatttgattaacgtcgcccaactgacggcgcaatattatgtactgaaaccagaagcagggaatgcggagcacgcggtgaaattcggtacttccggtcaccgtggcagtgcagcgcgccacagctttaacgagccgcacattctggcgatcgctcaggcaattgctgaagaacgtgcgaaaaacggcatcactggcccttgctatgtgggtaaagatactcacgccctgtccgaacctgcattcatttccgttctggaagtgctggcagcgaacggcgttgatgtcattgtgcaggaaaacaatggcttcaccccgacgcctgccgtttccaatgccatcctggttcacaataaaaaaggtggcccgctggcagacggtatcgtgattacaccgtcccataacccgccggaagatggtggaatcaaatacaatccgccaaatggtggcccggctgataccaacgtcactaaagtggtggaagacagggccaacgcactgctggccgatggcctgaaaggcgtgaagcgtatctccctcgacgaagcgatggcatccggtcatgtgaaagagcaggatctggtgcagccgttcgtggaaggtctggccgatatcgttgatatggccgcgattcagaaagcgggcctgacgctgggcgttgatccgctgggcggttccggtatcgaatactggaagcgtattggcgagtattacaacctcaacctgactatcgttaacgatcaggtcgatcaaaccttccgctttatgcaccttgataaagacggcgcgatccgtatggactgctcctccgagtgtgcgatggcgggcctgctggcactgcgtgataagttcgatctggcgtttgctaacgacccggattatgaccgtcacggtatcgtcactccggcaggtttgatgaatccgaaccactacctggcggtggcaatcaattacctgttccagcatcgtccgcagtggggcaaagatgttgccgtcggtaaaacgctggtttcatctgcgatgatcgaccgtgtggtcaacgacttgggccgtaaactggtagaagtcccggtaggtttcaaatggtttgtcgatggtctgttcgacggcagcttcggctttggcggcgaagagagtgcaggggcttccttcctgcgtttcgacggcacgccgtggtccaccgacaaagacggcatcatcatgtgtctgctggcggcggaaatcaccgctgtcaccggtaagaacccgcaggaacactacaacgaactggcaaaacgctttggtgcgccgagctacaaccgtttgcaggcagctgcgacttccgcacaaaaagcggcgctgtctaagctgtctccggaaatggtgagcgccagcaccctggcaggtgacccgatcaccgcgcgcctgactgctgctccgggcaacggtgcttctattggcggtctgaaagtgatgactgacaacggctggttcgccgcgcgtccgtcaggcacggaagacgcatataagatctactgcgaaagcttcctcggtgaagaacatcgcaagcagattgagaaagaagcggttgagattgttagcgaagttctgaaaaacgcgtaaacacatttaataaaaaaagggcggtcgcaagatcgcccttttttacgtatgacaaacacagaattgcctgatgcgctacgcttatcaggcctacgaggatggtgcaatatattgaatttaagcgattttgtaggccggataaggcgttcacgccgcatccggcaaaaacaacgaacactttgtcaacaaactgagtagctcaaggaaatcccaatgaagaccaacaggagtctggtcgtcatagtgtcactaattaccgccacattactgctgactgcatgcgcccaacctgaacaatcatcattagctggcgactggttactgacccctaaagataaaaccagaggattaacgggtagcattgcggtaaatattgcacctttccggtgtaagacaaattgccgtggtgataacttacctgataatacccgccgctggcagttgtcaggcgggaacgaaaaagaacttacttatcttcataatatgtcagcacaagaaaaggtcggtttaaatcccggttggcaatgctacacctcattttttatgcgggtttgccagggcaagcccggcactcgaccgatagtcaatgaggattatgtcagcgaaagcggattttttggctcgatgatgcatgtcgggattattgagttacgacgctgccagtcagaaaattgccagcaagaattgaaagcgataaatacacattaaaatagtgagtccgggaatgaaacccggacctgaacatgtcttattgcgtgaatgtttctttcatttgatactgcatttcccagagttcagtaagcgaaataacttttcttgttcttgcttcttcactttgtacccataagaaagggtagaacgtgaaggcttccgttgccgataattttattacgtcttctcgccattgctgccatcgtacattttcatagaaggtatctaaatcaccggataatgcccactgaagaaactcagaatatccaacttccagactttcccaattcagcgtatctggcgcaaaataataaacgcagccagtatcttccccaagatcgccaccattaagagcaaaaattacccctgcgacatcgtcagcgatgggtaaagcccgcacgcctgcgaattcagggcgttgtgtccaacttactggatctcgtggcaaccgggggtgaccagatcctgctatgcgtaactaaccattatcaatcagcagacctccggagccatagacaagcgcacccatcggtgattttgttgtcacctgtaattgataaagtgcggtttcggctaaatctttattaaccggtaagagttcggtatggtttgtggcgtcttttaaccagttctggattattggccaggctgaatcttcagtatttactaactgattcatttcacgcatcgctacttgctccttgtgtgctacggtgtcatttatgatgaggaattgtatggaacattttttaaatattaagttccttatatttgaataaaaaatgactttatccatacattgccacttttttcaaagcataaaccgatacccaataccggtttcagtaataaaatggcgaggccgggccggatcctgttccagtttttgtcgcagatgccccatataattacgcaaatagttgctgtgttcgatcgcgtttagaccctacatctgccggatgcggcataaataacgaactatttgccaacaaacagaaagggcgatcattcaatcgcccttttttactttgttttattaaccgtgtttatttttcagttcaaagcgtggtgataccagaccatacagtgtccaaccaaggaaggtcacgatggaaccgtacagcatggcttcttccccggatgagtacagcgcataaaagctatacatcgcgccaacaaaagcaacaaagtttgcaactttcgcttttgaggggggcacattagcgaccttctgaataatgactaatgccgccattgacagaatatacggaatgatattggtcaccacggccaggttaaccagcacgttgaactgactgtttagcgacgggctaatggtcatcagtgccaatccactctgaataatcacaatggtcaacattccctgcaccggtgcatccactttggttacacgggagaaaattttagggaagtagccttcatcagatgaagatttaaacacctgggcaatggtgaactgccagccaagtagcgaaccgcagcaggacatcaccatcagcgccataatgactttacccacttccggcgtgaacatctgcgcgaaggccagaccaaatggtgccgttgaatttgccagctccatatttggcacaatcccggcaatcacgttggtggagacgatataaatcaccgccgcacctaacgtaccgccgagtaccgcgattggcacattacgttccgggttttccactacatcagtattcgcacacgcagactccagaccaagaaaagcccacagcgtcatagcgatggaagaacctaccgcactgaagaacggtgcatgatgcggattccaggaatcaacgtacagcgtcgggctaaaccagaaccagccaataatgcacagaccgacgaccggaataatgaccccccacacggtaatgctactgatttgcccggtaatgcgcgcaccaccaaagttagccacggtacaaatccacagcaccccgatggtcgcaagaccaatctgcactggcgacaaactcgcgccgagcagttcggtgccgtaaccaaccgccgaaatagcaatcgcgacgttagcaatcagcagtgagacgccgtaggtatagttcgccataaagttaccggatttaccgaaagcatactcggcataaccgcccataccgcctgatttacggctgaacataccgcattttgcgaatgcccatgccagtgccattgagcctacggctgtcaccagccaggagataattgagattgtcccgacttcggcaagctttgtcggcagcatgatgataccggagcccatcatgttgaccatcgtcagtatggttaactgaacgacgcccattttgttcgatttagcctgactcataatttttcccctttcaacagggtgctttgcgcatcacgaggcttgatgacatagcaccaaacttgcttacgaccatcatgttcttcgatatagacaccctgcagctccggtgcaaaacctggcagcaggttgatcccttcttccagagcgctgaagtaacgcagaacagcaccaccccagatttcacccggaacaacacacagcacacccggaggataaggaagcgcaccttcggcagcgatacggccttctgcatccggcagacgaaccagttccacttcaccgcgtaaataggcgtagttggcttcttgcggattcatgctgacgcgtgggaagtgctccttacggaacatctctttttgcagttgtttcacgttgtggcgggcatacaaatcatgcatttcctgacacaactgacgcagggtataaccggcgtagcgctcttcatgctgtttgtagatggaaggtagcacttctgctaatggcgcgtcggactcaagcagtttttcgaagcgtaccagcagggcaacaagttgctgaagtttggccatatcttctgccggagtcagcaggaagaggatggagttaagatcgcatttttccggcactacgccattttcgcgcaggaagttagcaagaatcgtcgcgggtacaccgaacgcttcatattcgccgttacgtgcatcaatacctggggttgtcagcaacagtttgcatggatcgacaaagtattgattctctgcatagccttcaaaagaatgccagtgttcccctggtacaaactggaagaagcgcagatcaaccgcaatttgcgctgtttcatacgactgccagggtttaccatccaccagttcaggtacgaacggacgaatatgctgacagttatcgaggatcagtttgcgggcattaatgccatttaccacacaatccatccacatattacgaccgctgacaccttcatgcattttggcgttgatattcagtgcggcaaacagcggatagaacgggctggtggaggcgtgcatcataaaggcgttgttcatgcgtttgtgcggtacataacgctgttgccctttgatgtggctgtcttttttatgaatttgtgaagtctgagaaaaaccagcctgttgtttatgcacagattgcgtaaccagaatacccggatcgttctcattaagatccagcaacagcggcgaacagtccgccatcatcggaataaactgttcatagccgacccatgctgagtcaaacaggatgtagtcacacagatgaccaattttatccaccacttggcgggcgttataaatcgtaccgtcgtaggtgcctaactgaatcacagcgaggcggaaaggacgagcctcttttgcccgctgcggtgcgacttccgcgatcagctcacgcaggtaactttcttcaaaacagtgcgcatcaatgccaccgataaagccatacgggttacgtgccgtttccagataaaccggtgttgcaccagcctgtagcaacgctccgtggtggttagatttgtggttattgcgatcaaacagcaccagatcacccggtgttagcagggcgtttaaaaccactttgttagaagatgaagtgccatttaaaacgaagtaggttttatcggcattaaacacttttgccgcatgttgctgtgcaatgcatggcgcgccttcgtgaatcagcagatcgcccatcgctacgtcggcgttgcacaagtcggcacggaacagcgcctcaccaaagtattccacaaactgattccccgccggatggcgacggaaaaattcgccgccctgatgaccagggcaatcaaacgcgctgttaccttgattgacataatcgaccagtgcgcggaagaaaggtgggcgcagttgagtttcataatggctggcagcggtttctaactggcgaccataaaattctcgtcgcgattcgcaattctcaaagacacccgaaatacggggcaaatactctgcgggtacacgttcttgattttcagtagcaataaataccgggatgccataacccgtggcatcgatttcatcgagttttccgcatgtaacatcgttgagcgataaaactattgccgccacatcgatattacgactttcattaatgtagatacattctcgctgcgtggtaaaacagtccgggcaagaatcactaaccgcaatttttaattttgacatttttcatctctttattttaggtaatagcaggtcctcaatttctcgaatgagaaatcgatcgtgccggaaaaaagcaaagttaccccgctgataaataaatcaggtagattgcttttttcagaatgcagaaacccttaccagtcaggtggctgataatacaagggttaacagagaatgagcactgcggaatacaggcatatgcctgtaatacagagagtcaggaagacctgtacgctgaagtgcccttagtcggtagactaacgggcattgaagaagtgaaagtcgaagctattgcgatgagcaaacttcataatatgagttgtccgccttatatggggcatagtgcggctgttattttccatttaatttacctttcctgatgtgaatgaaggtgaagatattctatccaggaaatacggttgaactgtgaaggtgatcaataaaaaatgatcaatcttaatttatttaatgatgagctttttactcagtaatataaaatattgaattgttatttttgtgtgttgtttaagataaaaagccgtatttattattacggctttaattaataaaaggcaggctgtattaaaattaatattcaaagcataaaccgatagccaataccggtttcagtaatgaaatggcgtgggcgggcgggatcctgttccagtttttgtcgcagatgtcccatataaatacgcaaatagtgactgtgttcgaccgcgtttggcccccacacctggttaaggagctggcgctgggtgagtacttttccggcattgttgagcagcaccgccagcaggcggaactcaattggtgtgagatgcacctcttcctcaccccggtgaatcacgcgggcggctaaatcgacggtaacatcggaaaattttaccagcggatcgggcgcggtggtggcagagtggcggcgtaatgcgacgcgcagacgggcctgcaattcgccaatgccaaacggcttactcagataatcatccgctccggcatccagcgcggcgattttgtcgctctcttcgctgcgtgcggaaagcacaatcaccggcaccgcgctccactggcgcaggtcgcggataaactcaatcccatcaccatcgggcaggccgagatcgagaataatcaaatctggcttacgggttgccgcttccagcaagccgcgttgcagcgtttcggcctcaaagacgcgcatcccgtcgccctccagcgccgtgcgcagaaagcgacgaatagcctgttcatcttcaacaatcagaacgtttgtcacatatcctcatgaaattcttcaagttcaggggcagtttgctggggaagtgtaacacgaaaacaggcaccaccttccggtcggttgaacgcggtaatagtgcccccgtgtacatccactatcgcccgacaaattgccagtccaagccctacccccggtactgccgactctttattcccgcgagcaaacttatcaaatatcgtctgctcctggcctggcggaagaccggggccgttatcccagacatccagttgtagattttcgccctcaacgtgggcatcgataccaatttcggcctgcgcacccgcatatttcaccgcgttctccagcagattaatcagcacccgttcaaagagtggcccgtcaacgtggattaaggtcagcggttctggcagagaaagattgatgggcgacgataaacccggttccagcatttgcagcgcgctgccgactacttcttccagcgttaaccactctttcttcaaattaaagccgccggactgaattcgcgccatatccagtagattattcaccagtcgggtagtgttcagcacatgctgacggatctcgctggcctggcgggcgtggggtgatccttcgcttgccagatcgagcgttaagatttctgcctgaccaaacagcaccgtaagcggcgtgcgtaaatcatgcgaaagcgccgccagcagggcgttgcggatctgttcacgttcgcttgccatccgcgcctgttcttcgctggcggttagcgtcagccgctcaagggcattggcgactaacagcgtaaacgtctccagcaggcgctgctgttccgggatcatcaactggcgcagattccccggctccaccaccaccagcccgtaggttttctcgccgctttttagcggcaaaatctggtacggtacaccgggtaacgtgtcggtgcccgcgcccgcaggcaggcctttatcaaaactccactgcgcgatggcatcgtcccacggcgtcattccttgcggatgtgttaacggctgcaatttaccgttgtcatcgggcaacaacacctgactgcgggcatgaaacgtggaggcaataaattgttcgctggtggcagcgatatcctgcggactgcggcccaccgccagagctttcgacatttcatataagtgccgtgtgcgttgctcgcggtaacgggctacccgcgcctgataacgcacgccagcagtaaggttcccgatcaccagcccgacggttaacatcaccgcgaaggtcagcagatattgcacatcagagacggcgagcgtgccgcgtggggcgataaaaaagagatcgaaactcactacattaatgacggtggcaaccactgaaggccagcgtccataaaatagcgccaccaccaccacgccaagcagatacagcatcaccaggttggcggcatcaaacgccatcagccactgcatggcaattaaggtgataacggcgcataacgcggcggcaaccacgcatccctgaatttgtacacgccacttgtctttaaaagagcggttatccggcgcgttgttaatcgtgcgggcgggtggttcatcaagcgcgaccagcacctgatcgagatcgggggcgatgcgcgccagtcggtcagcaaacgtttcccgacgccaccagcggcgcgaggccgggcgaccgagaataatcttgccgagattatgttcacgggcataacgcactaccgctttctcttccgctggatcagaaagtgttgccgtctccgcgcccagttcctgcgccagacgtaaggcgctgagaattgcccgacgttttttttccggtaagcggtgcagggcaggggtttcaacatacaccgcgtgccagacgctacccagccgtgacgccagccgcgccgctgcgcggaccagtttttcgctgccggtgttatggccgatgcataaaaggatcgcgtcgcgcgtgtgccacactttctcttcgccaggatgcccccgccaggcgcgcatttgctcatcaacgcgatcggcagtacggcgcagtgccagttcgcgcagggcgatcagattacctttgcggaaaaaatgttcaatggcgcgctccgcctgcccggcaatatagactttgccttctttcagccgctggcgcagatcgtccgggggcaagtccaccagcaccacgtcgtcggcggcatcgaaaaaaggatcgggcacggtttcccgtacctgaattccggtgacgccgctgaccacatcattcagactttccagatgctgaacgttgacggtagtgaaaacatcaatgccagcttccagcagttcttcgatatcctgccagcgtttgggatgacgggaacctggcgcattactgtgcgccagttcgtccattaagatcagcgccgggcggcgggcgagggcggcatcgagatcaaactcgctgatatgccgcccacggtacgcctggcgttttaacggcagaacagccagcccttccagcatggcggcggtatcttttcgcccgtgggtttctaccacgccaaccacaatatccagcccttgcgcccgcagtcgctgggcttctgccagcatcgcccaggtcttcccgacgcctgcacaggcaccgaagaaaactttcagcttcccccgatgcggcgcggcagtttgttccagcagacgatcggggtcgggacgtaagggttcgttattcatcaagtttatccagcgccagattgagttcaacaatgttgacaaccggctggccgatatatttcaccagcggttgttggctgtattttgcgatcagttgcgtgagctgttcaacgctgagattacgcgctttcgccacgcgtgggatttgccaggccgccgcttgcggggtgatattattgtccagcccgcttgccgatgccgtcaccagttcaaccggaacgctcgcgctggcatccgggttagcggcccgtaatgcagcaacgcgtgcggctattagtttatccagctcagggttactgaccgccagattgctcccgccagaagcctgtggattatagggcatttctgccgttgccgacgggcgaccatgaaaatagccgttgccggtaaaattctgcccgattaatgccgaaccgcgcaccgtatcaccttcacgaatcaacgaaccattggcctgccagggaaaccaccattgccccagtacggtggtcagcagcgggtaaacgccgccagtaatcaataacagaaagataaatgttgataatgccggacgtaatccactcatggtaaacctcacaccagaccgcaaacggtcagcagtaaatcaatgactttgataccgataaacggcaccagcagcccacccagaccgtaaatccataagttacggcgcaacatggcagaagcggtaagcggtttataactcacgccttttaacgccaggggaatcaaaaagacgataatcaaggcgttgaaaatcaccgcactgaggattgcggagtcgggcgaatgcaggcacatgatgttcagcgcatttaactgcggatacgttgccgcgaatgccgccggaataatggcgaagtatttcgccacatcgttggcaatgctgaaggtggtcagcgagccacgggtcatcagcatctgtttgccaatgtgcaccacctcgatcaacttggtcgggttagagtcgagatcgaccatattgcccgcctctttcgccgcctgggtgccggagttcatcgccaccgcgacatctgcctgcgccagcgccggagcatcgttggtgccgtcgccggtcatcgctaccaaacgaccttccgcctgatactgacggatcaatgccagcttggcctccggtgtcgcttcggcgagaaaatcatcgacacccgcttccgcagcaatcgcggcggcagtcagacggttatcgccggtaatcatcaccgttttaatgcccattttgcgcagctgggcgaagcgctctttaataccgcctttgacgatatctttcagcgcaataacgcccagcacacgagaaccttccaccaccaccagcggcgtggctccctgacgcgcaacctgatcgactttttgatcaacatcggtagggaagtgaccaccgttagcctcaacatggcgacgaatggcatcgacagaacctttacggatcatgcggttgtcgatgttgatcccgctcatccggctttgcgcagtaaacggtacaaaggtggcatggagcgactgcacatcgcgctcgcgcaggttaaaacgctgcttggcgaggatcacaatactgcggccttccggcgtttcatcagccagcgaagccagttgtgcggcgtcagccagcgttttttcatccacgccctgcgcggggataaactccgacgcctgacggttaccgagtgtgatggtgccggttttatccagtagcagaacgtcaacgtcacctgccgcttcaactgcacgtccgctggtggcaatcacattcgcgcctagcatccggctcatcccggcgacgccgatcgctgacaacaggccgccaatagtggttgggatcagacagaccagcagcgccaccagtaccgttacgctgactgcattaccgccccacgcggaaaacggccacagcgtggcggttgccagtaaaaagacgatagtcagggcaatcagcagaatggtcagggcaatttcgttcggcgttttgcgtcgctgtgcgccttccaccatcgcgatcatccgatccagaaatgtctcgccggggttaacgctacactcaatcaccagccagtcagaaagaatacgcgtgccgccggtgacggaggcaaaatcgccgccggattcacggatcaccggtgccgattccccggtgatggcgctttcatcgaccgatgcacccccttcaataacttcaccatcgcaggggataatatcgccagcttctaccagtacgatatcgcctttacgaagttggtcggcaggaactttgtccgccgcagcgccatatttcggctcacgcagcttgcgggcaaaggcagtttttttcacccctttcagactgttggcctgcgctttactgcggccttctgccagcgcctcggcgaaattagcgaacagtacggtgatccacagccaaccgctaatggccgcgctaaacagcgcattgccgggcatcgcaccgcttgccatcgcgatgctaatacaggtggtcagcagactgccgatccagacgataaacatcaccggattgcgccattgcgcctgcgggtttaattttttcaccgcttctttcagcgcctgaacgacaagtgttggttcgaatagcgccagttgtttacgactcatattcagtgctcactcaatatcatcaggagagatattccgccaccggaccaagcgccagggcagggataaaggtcagtgcgccaaccagcaacacggtgccgattaacaggccaacaaacagcgggccgtgcgttggcagcgtgccggagctggcggcttggctctttttactcaccagcgaaccggcaattgccatcaccgggataatcaccccgaagcgaccgacaaacatgcagaacgccagtaaacagttccagaacggagagttggcgcttaatccggcaaaggcgctgccgttgttgttagcggcggatgacacggcgtacagcacttcgctaaaaccatgcgggccagggttgagcatggcgctacgtccggcgtcggtcatcatcgccaacgccgcgcccatcagcaccagcgtcggggtaaccagaattgccagtgcagtcagtttcatctcgcgtacgtcgatttttttacccagatattccggtgtacgaccaatcatcagcccggcaataaacaccgccagcaggacaaacagcatcatgccgtaaagaccagaaccgacaccgccgaacaccacttcaccaatttgcatcagccacatcggcaccatgccaccgagagcggtaaacgaatcatgcatcgcaatcaccgcgccacaggaagccgccgtcgtcacgaccgcaaacaggctactgaccagcacgccgaaacggctctctttaccttccatattgatgctgctgtccgtgcccagtgccagcagatgaggattaccctgaacttctgcccacatcaccacgcctacgcagatgacaaaaatcactgacatcgcccacagcaacatgcgcccctggcggcgatcgcccatcacttcaccaaaggcaaagcacagcgccgttgggatcaagaagatcgccagcatctgcacgaagttggtcagtgcggttgggttttcaaacggatgcgacgagttggcattaaagaagccaccgccgttagtaccgagcatcttgatcgcttcctgagaagctacaggccccatgggtaacagctgttgcgctccttcaacggtattcacagcctgataaggcagaaagttttgcagcgcaccttgttgaataaaaaacagtgcaatcaacaacgccacagggactagcacccataacgtgatgcgtagcagatcgacccaggcattcccgagcgtgctcatgctctggcgggtaaacgcacggatgagggcaaaaatcaccgcaatcccgctggcggcagaaagaaagttttgcaccgttaagcccgccatctggctgaaatagctcaacgtggtttcaccgctataagattgccagttggtattggtgacaaagctgacggcggtattcagcgccagatcccacgacagccctggcaactgctgtggattaagcggcagatagtgctgaccgagcaacataaaaaacagcaccgccagccccagcatgttcaggccgagaatggcacaaagatattgcttccagttcatctcacggtcagagacgccaagtgcgcgaaaaagtacgcgctcaacgcccgttgtaccgggaagaggaatgtcattaatcagccgcgccagcccgctgcctaaaggacgcgccagcaccattaacaccagtaaaaacgtggcgatcagtaagaacccttgcgcagccatcagaacgcctccgcattgatcagggcataaaccagataacccagtaataaaaacaccagcaatacgccggttatcacgcctgcactcacagtgcacctccagtggcctaaaagtgataccggaagggtagaattctggctgcaaagatttcgcaaaaatctgcgggcggggtgtaaaaaaagtataaaaatggcaaaagccatgatttaactaatgtttagtattaatttaacttttgtgtaacttaattacaggatgaatgtaaataaaccatcaataagcaaaaataagtggtcggatgagtagtaaaattacacaaaaggcggtactattttcatcagataaacaaattcatttttccggtgccattcaccgggtagatacaaaagggggagaaaagtatggaactctacagagaatatcctgcatggcttatctttttacgccgtacttatgcggttgcagcgggcgttctggcgctgcctttcatgcttttctggaaagaccgcgcccgcttttacagctacctgcatcgcgtctggtcgaaaaccagcgataaaccggtgtggatggatcaggccgaaaaggcaactggtgatttttattgattgctgagttttgaatacattgaaaaccgccagcggaaacgctggcggttttttgtatcaggaagatgttcagaggaatatttagacatcgttataccaatcgaaacatatattcatgaaatatatataaatattttcctaattgttcttatctgacagatatctcacttaaggctttcttataaatctgtagggtttcgcctgtcagcagacaaataacccgataaaacaaggatgagcagatgagcggaaaaccggcggcgcgtcagggcgacatgacgcagtatggcggtagcattgtccagggttcagccggggtacgcatcggtgcccccaccggcgtggcctgttcggtgtgccccggcggggtgacgtccggccatccggtcaatccgctgctcggtgcaaaggtccttcccggtgaaaccgacatcgccctgcccggcccgctgccgttcattctctcccgcacctacagcagttaccggacaaaaacgcccgcgccggtggggagcctcggccccggctggaaaatgcctgcggatatccgcttacagctgcgcgataacacactgatactcagtgataacggcggcagaagcctgtattttgagcacctgtttcccggtgaggacggttacagccgcagcgagtcactgtggctggtgcgcggcggcgtggcgaaactggatgaaggtcaccggctggccgcactctggcaggcgctgccggaagaactccgcttaagtccgcatcgttatctggcgacaaacagtccgcaggggccgtggtggctgctcggctggtgtgagcgggtgccggaagcggatgaggtgctgcctgcgccgctgccgccgtaccgggtactgaccgggctggtggaccgcttcgggcgcacacagacgttccaccgcgaagccgccggtgaattcagcggcgaaatcaccggcgtgacggatggtgccgggcgtcacttccggctggtactgaccacgcaggcgcagcgggcagaagaagcccggcagcaggccatttccggcgggacggaaccgtccgcttttcctgataccctgccgggttacaccgaatatggccgggacaacggcatccgtctgtctgccgtgtggctgacgcacgacccggaatacccggagaatttacctgccgcgccgctggtgcgctatggctggacgccccgcggcgaactggcggcggtgtatgaccgcagcaatacacaggtgcgcagctttacttacgatgataaataccggggccggatggtggcgcaccgtcacacgggccgaccggaaatctgttaccgttacgacagcgacgggcgggtgacagaacagctaaacccggcaggcttaagttacacgtatcagtatgagaaggaccgcatcaccatcaccgacagcctgaaccgccgtgaagtcctgcacacgcagggtgaaggcgggctgaagcgggtggtgaaaaaggaacacgcggacggcagcgtcacgcagagtcagtttgacgcggtgggcaggctcagggcacagacggatgccgcaggcaggacaacagaatacagtccggatgtggtgacgggcctcatcacgcgcatcaccacgccggatggcagggcatcggcgttttactataaccaccacagccagttaacgtcagccaccgggcctgacgggctggaaatacgccgggaatatgatgaatggggccgtctgattcaggaaactgcccctgacggcgatatcacccgctaccgttatgataatccacacagtgacttaccctgcgcaacggaagatgccaccggcagccggaaaaccatgacgtggagccgttacggtcagttgctgagcttcactgactgttccggttatgtaacccgctatgaccatgaccgttttggtcaggtgacggcggtgcaccgcgaggaagggctgagtcagtaccgcgcatacgacagccgtggacagttaattgccgtgaaagacacgcagggccatgaaacgcggtatgaatacaacgccgccggtgacctgaccaccgtcattgccccggacggcagcagaaacgggacacagtacgatgcgtggggaaaagccatctgtaccacgcagggcggtctgacgcgcagtatggaatacgatgctgccggacgggtcatccgcctgaccagtgaaaacggcagccacaccaccttccgttacgatgtactcgaccggctgatacaggaaaccggctttgacggccgcacacagcgttatcaccacgacctgaccggcaaacttatccgcagcgaggatgaggggctggtcacccactggcactatgacgaagcagaccgcctcacgcaccgcaccgtgaatggcgaaaccgcagagcggtggcagtatgacgaacgcggctggctgacagacatcagccatatcagcgaagggcaccgggtgacggtgcactatggttatgacagtaaaggccgcctcgccagtgaacacctgacggtgcatcatccgcagacgaatgaactgctctggcagcatgagaccagacatgcgtacaacgcacagggactggcgaaccgctgtataccggacagcctgcccgccgtggaatggctgacctacggcagcggctggctgtcaggcatgaaactcggcgacacaccgctggtggagtacacccgcgaccgcctgcaccgggaaacgctgcgcagcttcggccgttatgaactcaccaccgcttatacccctgccgggcagttacagagccagcacctgaacagcctgctgtctgaccgcgattacacctggaacgacaacggcgaactcatccgcatcagcagcccgcgccagacccggagttacagctacagcaccaccggcaggctgaccggcgttcacaccaccgcagcgaatctggatatccgcatcccgtataccacagacccggcaggtaaccgcctgcccgacccggagctgcacccggacagcgccctcagcatgtggccggataaccgtatcgcccgtgacgcgcactatctttaccggtatgaccgtcacggcaggctgacagagaaaaccgacctcatcccggaaggggttatccgcacggatgatgagcgcacccaccggtaccattacgacagtcagcaccggctggtgcactacacgcggacacaatatgcagagccgctggtcgaaagtcgctatctttacgacccgctgggccgcagggtggcaaaacgggtatggcggcgtgaacgggacctgacgggctggatgtcgctgtcacggaaaccgcaagtgacctggtacggctgggacggcgaccgcctgaccacgatacagaacgacagaacccgcatccagacgatttatcagccggggagcttcacgccactcatcagggttgaaaccgccaccggtgagctggcgaaaacgcagcgccgcagcctggcggatacccttcagcagtccggtggcgaagacggtggcagtgtggtgttcccgccggtgctggtgcagatgctcgaccggctggaaagtgaaatcctggctgaccgggtgagtgaggaaagccgccgctggctggcatcgtgcggcctgacggtggcgcagatgcaaagccagatggacccggtatacacgccggcgcgaaaaattcacctgtaccactgcgaccatcgcggcctgccgctggcccttatcagcacggaagggacaacagcgtggtacgcagaatacgatgaatggggtaacctgctgaatgaagagaacccgcatcagctgcagcagcttatccgcctgccggggcagcagtatgatgaggagtccggcctgtattacaaccgccaccgctattatgacccgctgcaggggcgatatatcactcaggatccgattgggctgaaagggggatggaatttttatcagtatccgttgaatccgatctcaaatatagatccattaggattagaaacactaaaatgcattaagccactgcattcaatgggcggaactggtgaaagaagcggtccagatatatgggggaatccgttctatcatcaatatctttgtgtcccagatggtaaaggggactatacttgtggtggccaagaccaacggggagaatcaaaaggagatggtctatgggggccaggtaaagcaagtaatgatacaaaagaagctgctggccgttgtgacctcgttgaaaccgataatagttgtgtggagaactgtttaaaagggaagtttaaagaggtaaggccgcgttattctgtattgcctgatatattcacacctataaatttagggctatttaaaaactgccaagactggtctaatgattctttagaaacatgtaagatgaagtgctccggaaataacattggacgttttattagatttgtattcaccggagtgatgtaatgaaatatattatttttttattcagagctatatggctggctttatcgcttttaatactattcttttccatgcatagactttcactattagactccactcgtgatgtgagcgagttaattagtctcatgtcttatggaatgatggtaatatgttttccaacaggcatagtattctttattgctctaatatttatagggactgtatcagacattattggcgtaaggattgatagtaagtatattatggcgataataatatggctttattttctgtcaggagggtatattcaatggtttgtattaagtaagcgcattataaacaaataaattaagttaattgctcttattattatatgtaacctgggcattgatatcccgtatgccacagacccggcaggtaaccgcctgcccgacccggagctgcacccggacagcaccctcagcatgtggccggataaccgtatcgcccgtgacgcgcactatctttaccggtatgaccgtcacggcaggctgacggagaaaaccgacctcatcccggaaggggttatccgcacggatgatgagcgcacccaccggtaccattacgacagtcagcaccggctggtgcactacacgcggacacaatatgcagagccgctggtcgaaagccgctatctttacgacccgctgggccgcagggtggcaaaacgggtgtggcgacgtgaacgggacctgacgggctggatgtcgctgtcacggaaaccgcaagtgacctggtacggctgggacggcgaccgcctgaccacgatacagaacgacagaacccgcatccagacgatttatcagccggggagcttcacgccactcatcagggttgaaaccgccaccggtgagctggcgaaaacgcagcgccgcagcctggcggatacccttcagcagtccggcggcgaagacggtggcagtgtggtgttcccgccggtgctggtgcagatgctcgaccggctggaaagtgaaatcctggctgaccgggtgagtgaggaaagccgccgctggctggcatcgtgcggcctgacggtggagcagatgcaaaaccagatggacccggtgtacacgccggcgcgaaaaatccacctgtaccactgcgaccatcgcggcctgccgctggcgcttgtcagcacggaaggggcaacagaatggtgcgcagaatacgatgaatggggcaacctgctgaatgaagagaacccgcatcagctgcagcagcttatccgcctgccggggcagcagtatgatgaggagtccggcctgtattacaaccgccaccgctattatgacccgctgcaggggaggtatatcactcaggatccgattgggctgaaggggggatggaatttttatcagtatccgctgaatccggttcagtatatagattcaatgggactggcatcaaaatatggacacttaaataatggcggatatggagcgagacccaacaaaccgcctacgcccgatccaagtaaattgccggacatagcgaaacaattaagactgccatatcctattgaccaggccagtagtgcgcctaatgttttcaaaacattcttcagagcattaagcccttacgactacacactgtattgcaggaagtgggtaaaaccaaatctgacttgtacgccacaggatgattcccagtatccagggatggatacaaagacagcaagtgattacctgccacagacaaattggccaacaactcaattaccaccaggatatacttgtgcagaaccctatttattcccagacattaataaacccgatgggccagcaacagcagggatagatgatttgggtgaaattttagctaagatgaaacagagaacatcgagaggaataagaaaatgaaaagagttttgttctttttgctgatgatatttgttagttttggtgttatagctgattgcgaaatacaagctaaagatcatgattgttttactattttcgctaagggtactattttttccgcgtttcctgtcttaaataataaagccatgtggagatggtatcagaatgaggacatcggtgagtattattggcaaacagaactgggtacatgtaaaaataataaattcacaccaagcggggcgagactcttaattcgcgtcgggtcactacgccttaatgaaaatcatgccatcaaaggaacgttgcaggagttgataaatacagcagaaaaaacggcgtttctcggcgatcggtttagaagttatataagagcgggtatctatcaaaaaaagagcagtgatccagttcagttgttggcagtccttgataattcaatcatggtaaaatattttaaagatgagaaaccaacttatgctcgaatgacagcacatctcccgaacaaaaatgagtcttacgaatgtttaataaagatacagcatgaactaattcgtagtgaagagaaataaaatctcttcctgagaaaacaaattaatcattgtgaaaaattatataactcatggaataggtgtttattttgcgttccatttgcagggaaagatcacgtaacgctacttttttgtactaaataattcgaattttaagttcaacaattgagatactacttattgtctaaagctgtttttcatagcttatacatgatcaaatactccttacataaataaggtgaacaaatggaacttaaaaaattgatggaacatatttctattacacccgattacagacaagcctggaaagtggtgcataaattgtcagatattctactgttgactatttgtgccgttatttctggtgcagaaggttgggaagatatagaggatttcggggaaacacatctcgattttttgaagcaatatggtgattttgaaaatggtattcctgttcacgataccattgccagagttgtatcccagggaaagatcacgtaacgctacttttttgtactaaataattcgcattttatgtttaaaaattgagatattccttattacctaaagctgtttttcatagcttatacatgatcaaatactccttacataaataaggtgaacaaatggaacttaaaaaattgatggaacatatttctattattcccgattacagataagcctggaaagtagagcataaattgtcaggcatcctactattgactatttttgccgttatttctggtgcagaaagttgggaagatatagaggatttcggggaaacacatctcgatttcttgaagcaatatggtgattttgaaaatggtattcctgttcacgatactattgccagagttgtatcctgtatcagtcctgcaaaatttcacgagtgctttattaactggatgcgtgattgccattcatcaaatgataaagacgtcattgcaattgatggaaaaacgctccggcactcttatgacaagagtcgccgcaggggagcgattcatgtcattagtgcgttctcaacaatgcacagtctggtcatcgggcagatcaagacggataagaaatccaatgagatcacagctatccctgaacttcttaacatgctggatattaaaggaaaaatcatcacaactgatgcgatgggttgccagaaagatattgcagagaagatacaaaaacagggaggtgattatttattcgctgtaaaaggaaaccaggggcggcttaataaagcctttgaggaaaaatttccgctgaaagaattaaataatccagagcatgacagttacgcaatgagtgaaaagagtcacggcagagaagaaatccgtcttcatattgtttgcgatgtccctgatgaacttattgatttcacgtttgaatggaaaggactgaagaaattatgcgtggcagtctcctttcggtcaataatagcagaacaaaagaaagagccagaaatgacggtcagatattatatcagttctgctgatttaaccgcagaaaagttcgccacagcaatccgaaaccactggcacgtggagaataagctgcactggcgtctggacgtggtaatgaatgaagacgactgcaaaataagaagaggaaacgccgcagaattattttcagggatacggcacatcgctattaatattttaacgaatgataaggtattcaaggcagggttaagacgtaagatgcgaaaagcagccatggatagaaactatctcgcgtcagtccttgcggggagcgggctttcgtaatctttccctgctttttgtactaaataattcgcattttatgtttaaaaattgagatattccttattacctgaagctgttttttattgcttatacatgatcaaatacttcttacataattaaggagaacaaaatggaacttaaaaaattgatggaacatatttctattatccccgattacagacaagcctggaaagtggaacataaattatcggatattctactgttgactatttgtgccgttatttctggtgcagaaggctgggaagatatagaggattttggggaaacacatcccgattttttgaagcaatatggtgattttgaaaatggtattcctgttcacgataccattgccagagttgtatcctgtatctgtcctgcgaaatttcatgagagctttattaactggatgcttgactaccattcttcagatgataaagacgtcatcgcaattgatggaaaaatacaccggcattcttatgacaagagtcgccgtaagggagcgattcatgtcattagtgcgttctcaacaatgcacagtctggtcatcggacagatcaagacggataagaaatccaatgagatcacagctatccctgaacttcttaacatgctggatattaaaggaaaaatcatcaaaaccgatgcgatgggttgccagaaagatattgcagagaagatacaaaaacagggaggtgattatttattcgctgtaaaaggaaaccaggggcggctaaataaagccttcgaggaaaaatttccgctgaaagaattaaataatcccaagcatgacagttacgcaattagtgaaaagagtcacggcagagaagaaacccgtcttcatattgtttgcgatgtccctgatgagcttattgatttcacgtttgaatagaaagggcagctatggttagaaactacctgacgtcagtccttgcggggagcaggctttcgtaaatttgtcctgctacaacaggattaacttcacaaatatcatttctcaacgtctacacttactcctgtaaaccgctcaggagcagtaatgaatctacaacgatttgatgacagcaccctaatccgtatctttgcccttcatgagttacatcgactgaaagaacatggcttaacgcgcggggcgcttctcgattatcacagccgctataaactcgtctttctggcgcattctcagccggagtaccgcaaacttggcccgttcgtggctgatattcaccagtggcaaaatctggatgactattacaaccagtaccgccaacgcgtagttgttttgctttctcaccccgccaacccgcgcgatcacaccaatgttttgatgcacgttcagggttattttcgcccgcatattgattccacagaacgccagcagctggctgcgcttatcgacagttatcgccgtggcgagcaaccacttcttgcgccgctgatgcgtatcaaacactatatggcgctttatcctgacgcctggctttcagggcagcgttatttcgaactttggccgcgtgtgattaacttgcgccattcaggagttttatgactacccatctggtctggtttcgccaggatttacgtctgcacgataatctcgcactggctgccgcctgccgcaattcgtctgcacgcgtgctggcgttgtatatcgctacaccacgccagtgggcgacgcataacatgtcgccgcgtcaggctgaacttatcaatgctcaactgaatgggctacaaatagcgcttgcggaaaaaggtattcctttattgttccgtgaagtggatgactttgtcgccagtgtcgaaatagttaaacaggtgtgcgcggaaaacagcgttacccacctgttttataactatcagtatgaagtgaatgagcgggcgcgggatgtggaagttgaaagagcgctgcgtaacgtggtgtgtgaaggatttgatgacagcgtgatcctgccgcctggcgcggtgatgaccggtaatcacgagatgtacaaagtctttacgccttttaagaatgcctggctgaaacggctgcgggaagggatgccggagtgcgtcgctgcgccaaaagttcgtagtagcggatcgatagagccctcgccatccattacgctgaattatcctcgtcagtctttcgatactgcgcattttccggtggaagaaaaagcggcgattgcgcaattacgccagttttgccagaacggtgccggagaatatgagcaacaacgagattttccggcagtggaaggcaccagccgtttgtcggccagcctggcaacgggcgggttatcgcctcgccagtgcttgcatcgcttgttggctgaacagccgcaggcgctggacggtggggccggtagtgtctggcttaatgagctgatctggcgcgagttttaccgtcacctgataacgtatcacccctcgttgtgtaaacatcgtccatttattgcctggacggatcgtgtacagtggcagagcaatcccgcacatttacaggcctggcaggaaggcaaaacgggatacccgattgttgatgccgctatgcgtcagcttaacagcactggctggatgcataacaggctacggatgattacagccagttttctggtgaaagatttattgatcgactggcgcgaaggcgagcgatatttcatgtcgcagctgattgatggtgatttggcagccaataacggtggctggcagtgggccgcttcaaccggaaccgatgcagcgccgtattttcgtattttcaacccgacaacccagggcgagaaatttgatcatgagggcgagtttatccgccagtggctaccggaactgcgcgatgtgccagggaaagtggtgcatgagccgtggaagtgggcgcagaaagcaggtgtgacgctggattatccgcaaccgatagtcgagcacaaagaagcgagagtacaaacgttggcagcgtatgaggcggcgcggaaggggaaataacagacgcgtcaggcaatcgagcccagatgccggatgcggcgtgaacgccttatccagcctacaaatttgtgcaaattcaataaattgcaggaaatacgtaggcctgataagacgcgtcaagcgtcgcatcaggcatcggtgctggcctattaagactccagcgccagcgcgcggtttctgaatttcagcgcctgatacagccaaatcatcagtaccagtcctacacacgccagtgcgccccaggtaatttgatcaaatacttcaatatatgcattgatggagtagttgatcgccccggaagcatcaaacgaagcctgcgatgtctgatcggcaatcacgcccgccagatagttcgcgatcgcgccagaaagcagcatgtagatgccggttaatacgccggtcacaccggggatttcaatgcgcgtaatttgcgacatggcaaccgggtcgataaacagttccgcaaagcccatcaccgccaggcctaataccatcagtggcagagaagagtgaccatacattgcggaccagcgggcgcttaaggtcagaatgcagaatccggcgctcatcaggccaaggccaagagcaaatttcccccagatgcgcacggtacgattacccgcgacactctcttttaccacccacgccaggaacacaccgcacagcataactgcgaaggcattaatcgactggaacatcgcggtcggaacggtataaccaaacatatcgcggttaacgaagcggtcgatataaaggctaatcgagctaccgccctgttgtgcgaaggcccagaacaacatactgaagaaggtgagcgtcacaatcagccccagctccttccgctgtttctggttttctgctttgcgataaatttttgccagtacacccaggccaataatagtcgcgacaattaaggcgtataccgaccactctttccagaacagtatggtaatcagtgcaggcgttgccaccagcagaaccagcagccatccccagttcggcaggagaaagtttgtcgcacgcagtacttttttgttaacgccgcgggtatgagtgaaatgacgattgccacataagaaaatgaccagacccgcgatcatgccaaccgccgccaggccaaagcccatcgcccagctgtactcttcctgggcgtaaccacaggcgataggtgcgataatagaccccacgttacccgccgcatacatcagcgagaaaccgccatcacgacgcggatcggttggctcatacagctcgccgagcagacagcttacgttagatttaaacaggccatagccgcagacgataatcgccagggacagatagaggaatgacggatggatctcactggcacccagcaccacatgaccgatcgccatcaacaacgcccccagcatcaccgccatgcgattgccgagaactttatccgccaaaaagccaccgaggattggcgtgacatacaccagcgaacagtaggcgctaaataactcgtaggcgtgagtatcgttgtattttagttgattggtgagatagagaatcagcagggcacgcatgccgtaaaagctaaaatattcccagatttgcagcgcaacgacatagtaaatagcgcgcggctgtgatgcgtgtttattcataataattccacaattgacggcaacgtcacgtaatagttgcgcggcgtgcttgtgtttccttaaagttaaaactttgatacagatctgattatttatgcaatatgctgtctgattgcataaatatacattagctgaagcgtgatgatataaacaatttgcgtcttttggcgtcgggtttgtttcttaatatgtcaaaagattggctatcgacgaactggcgaggtaacgctatgttaacggtgtagctatcagaatacggaaggcgcgaagatgaaaaacaccgaactggaacaactgattaacgaaaaactgaacagcgcggcgattagtgattacgcgccgaatggtttgcaggtggaaggcaaagagacggtgcaaaaaattgttaccggtgtcaccgccagccaggctttgctcgatgaggcagtgcgtctgggcgcggatgcggtcattgtgcatcatggctacttctggaaaggagagtctccggtcattcgcggaatgaagcgtaaccgtttaaaaacgttgctggcgaatgatatcaacctgtatggctggcatttgccgcttgacgcacatcctgagctgggcaataacgcacagctggcggcgttactggggatcacggtcatgggcgaaattgagccgttggtgccgtggggcgaactgaccatgcctgtgccgggactggagctggcttcctggattgaagcgcgtctgggacgtaagccgttatggtgtggcgataccggacctgaggtggtccagcgcgtcgcctggtgcacgggcggcgggcaaagttttatcgatagcgccgcgcgttttggcgtggatgcttttattactggcgaagtttctgaacagaccattcattcagcccgcgagcagggattgcatttttatgctgcaggtcaccatgccactgaacgtggtggtattcgcgcattgagcgagtggctgaatgaaaataccgatcttgatgtgacctttattgatattcctaatcctgcataacgaataatcagagggatcgaaagtgcaacgagcgcgttgttatctgataggtgaaacggcggtagtgctggaactggaaccgccggtgacgctggctagccagaaacggatctggcgactggcgcagcgtctggtggatatgccgaatgtggttgaagccattcccggcatgaacaatatcacggtgattttgcgtaatcctgagtcgctggcgctggatgccatagagcgtttgcaacgctggtgggaggagagcgaggcgctggagccggagtctcgctttattgaaattccggtggtttacggtggtgcaggcggaccggatttggcggtggtcgcggcgcattgcgggttgagcgaaaaacaggttgttgaattgcactcctccgtggaatacgtggtctggtttttaggttttcaaccgggcttcccgtatctcgggagtttgccggaacaactacacacgccacggcgcgctgaaccgcgcttactcgttccggcaggttctgtcgggatcggcgggccgcagactggtgtttatccgctggcaacgccgggtggctggcagttgattggtcatacctcactcagcctgtttgatccggcgcgtgacgaacccatcttattacgtccgggagacagcgtgcgctttgtaccgcagaaggagggagtatgctgaagattattcgtgcgggcatgtataccactgtgcaggatggcggtcgtcacggttttcgccagtcgggtatcagccactgcggcgcactggatatgcccgcgttacgcattgctaacctactggtgggtaatgacgccaatgcccccgcgctggagatcacgctcggtcagttaactgttgagttcgaaactgatgggtggtttgctctgacgggtgccggttgcgaagcgcggctggatgataatgccgtctggaccggctggcgattgccgatgaaagcaggccagcgtttaacgcttaaacgcccgcagcacgggatgcgcagttatctggcggtcgcgggtggtattgatgttccgccggtaatgggctcatgcagcaccgatctcaaagtggggattggcgggctggaaggccgtttactgaaggatggtgaccgactcccgattggcaaatcgaagcgtgattctatggaagcgcagggcgttaaacagctgctgtggggcaaccgcattcgcgccttgccggggccggaatatcatgagttcgatcgcgcctcgcaggatgcattctggcgttcgccctggcagcttagctcgcaaagtaaccgcatgggctatcgcttacaggggcaaattttaaaacgcaccaccgatcgcgaactgttatctcacggtttgttaccgggcgtggtgcaggtgccacataacgggcagccgattgtgttgatgaacgacgcacagaccaccggtggttacccgcgtattgcctgtatcattgaggctgatatgtaccatctggcgcaaattccgctcggtcagccgattcattttgtccagtgttcactggaagaggcactaaaagcacggcaagatcagcaacgttattttgaacaattagcgtggcggctgcacaatgaaaattgacctgaacgccgatctgggcgaaggctgcgccagcgacgcagagctattaacgctggtttcctctgccaatattgcctgtggatttcatgcaggcgatgcgcaaatcatgcaggcttgcgtgcgtgaagcaataaaaaatggtgtcgcgattggcgctcacccgagttttcccgacagggaaaattttggtcgcagcgccatgcagctgccgccagaaaccgtttacgcccagacgctgtatcaaattggcgcgctggcaacgattgcccgtgcgcaaggcggcgtaatgcgtcatgtcaaaccgcacggcatgttgtacaaccaggcggcgaaagaagcacaactggcagacgccatcgccagagcggtatacgcttgcgatccagcattgattctcgtcgggctggcgggaagcgagctgattcgtgcaggcaagcaatatggtctgacaacgcgcgaggaagtgtttgccgatcgcggttatcaggctgacggctcgctggtgccgcgaagccagtcaggcgcgttgattgaaaacgaagaacaggcgctggcgcaaacgctggagatggtgcaacacggcagagtcaaaagtatcaccggcgaatgggcaacggtcgcggcgcaaacggtctgcctgcatggcgacggcgagcacgcactggcgttcgcccgccgactacgctctgcatttgccgaaaaggggattgttgtcgcagcataaccccgattaataaagaatgaaaaaaggatatcaccatgcctgaaggcccggagatccgccgtgcagcggataacctggaggcggcgatcaaaggcaaaccactaactgatgtctggtttgccttcccgcagttaaaaccttatcaatcacaacttatcggtcaacacgttacccatgtggaaacgcgtggtaaggcgttgttaactcatttttccaacgacttaacgctctacagccataatcagctttacggcgtctggcgcgtggttgataccggcgaagagccgcagaccacgcgagtattgcgggtaaaactgcaaacggctgacaaaaccattctgctttatagcgcctcggatattgagatgttgaccccggaacaactgaccacgcatccgtttttacaacgcgttggtcccgatgtgctggatccgaatctgacgccggaggtggtgaaagaacgattattgtcgccgcgctttcgtaaccgtcagtttgctggattactgctcgatcaggcgtttctggctgggcttggcaattatttgcgggtggagatcctctggcaggttgggttgactggaaatcataaagcgaaagatctcaatgcggcgcaactggatgcactcgcacacgcgttactggagattcctcgattttcctacgctacgcgggggcaggtggatgagaataagcatcatggggcgctgtttcgctttaaggtttttcatcgagatggcgaaccgtgcgaacgttgtggcagcatcattgagaaaaccacgctgtcatctcgcccgttttactggtgccctggctgccagcactaggccgaccgcttcggcgcataggttgaaataaaccgcgcaatggcaggccctgtcagcaaaatactgaacaggcgtagggtttgcatcgccataatgagcgccatatcggcattgctccctgcggcgatgaccgccacggtatcaagcccgccggggctggtggcgaggtaggcagtcataaaatcaatgtgcataaaccgggtcagcccccacgccatacccgcacaaatagccagcagagcaaaaatcgacagcaggatttgcggtagcgggcgtagtgcccgcagtaagatttgtttatcgaaaccaagaccaatccgccagccaattgccatatacgccatcgccagcagccattccggtagttcgatggtgatgagctgaccagactggagcactgcgcccgccagcatcgggatgagcatcgtgccggaaggaagacgcagcaggcatcccactgtaccggcaacgaccgcgagcaaaatagtaagcaggagattaatgctcactggcgggaaccagacgatatgctggttaaccgcttcagcgttatcgcccagcatcatgcgggtgaccagaacagcggcccccgcgacgaacagcactcgcagatattgcataaacgccaccaggcgaatatctgcgccgtaatcttgcgccatagcgaccattgccgccgcgccgccaggagaggagccccaggcaccggtatttccaggcaatgagctatagcgcaccaataaccaacccacaatggcgctggaaagcagcgttaccagtaaaattgcaagcacgatcggccagttgacggccagggtggtgagaatcgaaccagtgaggttttgcgcaatcatgcagccaagaatggcctgggcggcgagaaaagcagagcggggaagttgcagagtaattccgcgcatactaaagatgatcccggcgatcatcggcccaagtaatagcgccgccgggagatgtaccgcgaggaaaccaatagaaaggagaagtgatagcacacataacattccccactgcaaaactggcatccttcgctccctcattattttctctttggtgtatcgatacagcataaagaaagctgggccaggaaaaaataacagcaatcaaggaaaaggggaaaatcagcaattttctgaaagagatgccctttccggcggcaaagggcatcatggtaaatcagttatagttaatcttaaaaagcaccactgtatcgaaggggccagcctcgatgggggtgcctggaatggacgaaagttcagccgtataggttttttcgtagaccaacatgtcactggtgaaatcggcgtattcagcatatttattgaaggtataaggcgaggcgttttcatccagtaaacgtagcttcagaccattaccaatcaacaatgctttatcttcttcaaccaacgtttcttcggtataaaaggaggaactgactttaaatccgtcggtgcattgatcgttttggctcttggtcgttttaatactgaacgttttcgacattgtgtggcgacgtatatccagcaaattaaatttaccaaaatcaatcacctgtgtttccggtgaaatggaaaaattgacgctgcaatccagcacgcgaatgttttccagaccagtaatatgatatttcaggttttgggcagtagggtcttcgttaacgctaccggcaccgtcaaattgcacgacgatatagtcgctaagcgtactttgataatcatgcggcggcatttctcgtattttgacgtataaccgcatgcgagcgagaaaggtacgcgacatatgaatattagcgggatcgcccgagcaaattttgttctgccatcccatcgcgatgatctgctcaggggtataaatatcaatgttcttactgtcgatacactggttagtgtcgatgcgactttttcccagactggcatcgtaatcgacaccgttgtatgtcacgccgagttgataataacgatcctgcacccccggataggggtttacccaggcgtagacatgctcgctttcaaagttgccgttggtattgttgtcacaatagacgggaattttaatatcgtcagattcccagatcttatcaccgggtttggcattgcctggtacagcaaacggttgaatcgcttctgatttttctactgcgccaccagatgtaccaaaatagcagttcagcgccattgcagacttcaacggcagaaataacaggcagatgacgagcaacaatcccttgccagcactcatttcgcctccactgcttgtaaacggcattgtccgctgcagttgagcgtcgtcatgcgtaatgcgccgtaatcatccatgtaaccgagataaaactggctgccgctataacttccggtgtttgtgttgaccgtactaaaaggtgcaaccatcacggttttgaagcctgggagaacgcctttttcatttctccccagataggcaatggtcagataatacgcggtaggatttttcagtgtcagttggttgccctgctggctgacctgtaactgcagttcgaccttttctcctgctttcttgcgtaatgcagccggtcgccagaacaatttaatacgactttgaatagcgacctgaagtatcgcatggtcgctgcttttatccggagcgggaggaatttcgcgcatattgtagaaaaatagcgtttcgcgatcgccaggtaattgtgtggttgaggcttgtttcacaacccgcacctgcgatgtcgctttcggttccagacgttgaatagggggcaaagcgaccagaagagcatcgcttttctcccctttttcattttctatccaggaataagcaagataaggcagtttgtcactttggttttcgatacgcaggctggtggctttgtcattggcgttaaacacaatgcgtgtgcgatcgggttgcaccgcagcattgcaacccaagctgatggttaacaacattaagggtaatcctttaataaatgtcattctcttttccttaattaatgacaaggtaaaatcaggcgtttggtcgtgtcttccagacgttctggcagatgaataatgcagctttgctcaccccagaccacggtaaacagttgattttcagcgacaccgcttaaccaggcatgtccttcctcgccaaccatacccacgctaatgccgctgtcatcctggcggatatccgcaccgaggggagggaactgaccgctggcgttgcgtatgatgacgttaacgtctttaccggaacgggaagccagtgatttgtaacctatcgcgccttcaatccatgtttccttgatgacgttttctgcaactgttacgccgtcgggtaagtcattcatgttcaccgccacggtggaaggctggtaactggaaatcaacggcaccaccgcaatgccaaaatggttggtgtagtcgagattgccctgaaccggaatatctgccacgccatcggtgctgaccatcaggcgtggttcattggtggagctgcggcgatgaaatgctgcaccatattgggttgcggtgaaagaaccgctccagctgctgctgacggaactgtaatcactggcggcataggtaccagaaatatcccactcacccgctgaactcaggtgctgatagttaccgctcacctgggctccattgtccggacgatcggattgcagtccggcagacatgccccagctattacgttcatccagcgtatcgttccacgacatgcggtgtatggtgctgtggctactgttttgcatgtcatagccaacccgaccaccgttaccgaaggggagcgaaatcgacagataaatctggttgtcgcgatctttatcttcgtagtgggtcgtattgaatgacgtcgaaatcgagatatctctccagtcaccaatatcaacattaaaacctgctgtgatgttggcggtcgtggaggcgtctgcattccaccaggtttgatgtagcaggttggcgtaaagattgaggtttagtggggtaatcggttggcccacggataagctgatcgtctgtttttcgtcctgcgcatcgctgtcgttgtatttgtgatccagatagttggcgtagctgtgaaaatgacgatctgagaagcgataagcggcgagcgaaatcgtgctgttggtggcatccacttgtttgctgtaattaaaacggtagcttaagccccgctcgtcctgctgagtatcaaaatggctactggcccaggtgacatcaaaggacagtgcgccaagccacagcatattttgcccgatacccattgcggcagaatggtagtcatcatcagaaatcagcaggccgccgtacagcgaggtgtttgagagcatcccccaggaaacttcattgctaaaaaaggtttcattttcagtttgatgtgacatggaaggccgtggctgacccgcggccaatttatagcgaacctgtccctggcgagtcaggaagggcgtcgatgctgccgaaacctggaaattgttcacccgaccatcttcttccgtcactttgacatccagcgtgccctgaacagactgattgaggtcatcaataataaacgggcctggcgggacttttttctggtaaatgacgcggcctgattgactgatcgtcaccgtggcattggtctgtgcaataccgctaatttgtggggcgtagccacgcagctcccacggtaacattcgatcgtcactcgccagtgccgcgccggtataagaaaaaccatcgaaaatattggaactgaaatcggtttcgccgagggttaacttagagcctaattgcggtaatggacgaaaaagataggtgcgcgatattccgcctgactggtcatggttatcttcgctatcggtcttattaagctggtaatcactgcgtaagcgccatgccccggcgttaattccggcggtaccgtaggcattcaggttagtgctgctgctgccgtcctgtgggcggtagctgctggcaaacaagttgtaatccatcaggacaccggcaacaccttctttccatgtagaggggggagcccagttttctgagtgccacgccagccaggcttgcggaatactaatattcagttgctgattggcttgatcgaaattgaagagcatttcaggtcgggaactgaaatcaatacaccgatctatctgtggcaaggactgacggatatctggttttaaaccaaatttatcgaccagtgaatcattgatgcatggaatggttttgtcaccctttttttgccagttaattttttgcccattactgattttgttgttattcaccgcaacgctaacaaaatattcaccgggagcaatgactcctttttcctttaataatgaaatatcaatgcggtcgcgcattgatttatcgagaacattcagattgaattcgaccgccattgcgcaaggcatcgccatgaccaggcaggatacaaaagagagtcgataaatattcacggtgtccatacctgataaatattttatgaaaggcggcgatgatgccgccaaaataatacttatttataatccagcacgtaggttgcgttagcggttacttcacctgccgtgacatcgactgcattatcaatttgttccatccaggcgaaaaagttcagcgtctgttctgatgagcttgcatccaggtcaagatctggcgcggctgaacctaatacgatgttaccgtcatttttgtccatcagtcgtacaccgaccccagttgcttcgcctgcactggtgttgctcaacaaaggcgtagcaccagttgtcttagccgtgctatcgaaggttacgccaactttggataccggcattccgctaccgttgtcagaagcaggcagatcacagttgatcaagcgaatgtcgacggccactttattgctatgatgctcccggtttatatgggttgtcgtgacttgtccaagatctatgtttttatcaatatcttctggatgaatttcacaaggtgcttcaataacctcccccttaaagtgaatttcgccagaaccttcatcagcagcataaacaggtgcagtgaacagcagagatacggccagtgcggccaatgttttttgtcctttaaacataacagagtcctttaaggatatagaataggggtatagctacgccagaatatcgtatttgattattgctagtttttagttttgcttaaaaatattgttagttttattaaatgcaaaactaaattattggtatcatgaatttgttgtatgatgaataaaatataggggggtatagatagacgtcattttcatagggttataaatgcgactaccatgaagtttttaattgaaagtattgggttgctgataatttgagctgttctattctttttaaatatctatataggtctgttaatggattttatttttacaattttttgtgtttaggcatataaaaatcaacccgccatatgaacggcgggttaaaatatttacaacttagcaatcaaccattaacgcttgatatcgcttttaaagtcgcgtttttcatatcctgtatacagctgacgcggacgggcaatcttcataccgtcactgtgcatttcgctccagtgggcgatccagccaacggtacgtgccattgcgaaaatgacggtgaacatggaagacggaatacccatcgctttcaggatgataccagagtagaaatcgacgttcgggtacagtttcttctcgataaagtacgggtcgttcagcgcgatgttttccagctccatagccacttccagcaggtcatccttcgtgcccagctctttcagcacttcatggcaggtttcacgcattacggtggcgcgcgggtcgtaatttttgtacacgcggtgaccgaagcccatcaggcggaaagaatcatttttgtctttcgcacgacgaacaaattccggaatgtgtttaacggagctgatttcttccagcattttcagcgccgcttcgttagcaccgccgtgcgcaggtccccacagtgaagcaatacctgctgcgatacaggcaaacgggttcgcacccgaagagccagcggtacgcacggtggaggtagaggcgttctgttcatggtcagcgtgcaggatcagaatacggtccatagcacgttccagaatcggattaacttcatacggttcgcacggcgtggagaacatcatattcaggaagttaccggcgtaggagagatcgttgcgcgggtaaacaaatggctgaccaatggaatacttgtaacacatcgcggccatggtcggcattttcgacagcaggcggaacgcggcaatttcacggtgacgaggattgttaacatccagcgagtcgtgatagaacgccgccagcgcgccggtaataccacacatgactgccattggatgcgagtcgcgacggaaagcatggaacagacgggtaatctgctcgtggatcatggtatgacgggtcaccgtagttttaaattcgtcatactgttcctgagtcggtttttcaccattcagcaggatgtaacaaacttccaggtagttagaatcggtcgccagctgatcgatcgggaaaccgcggtgcagcaaaataccttcatcaccatcaataaaagtaattttagattcgcaggatgcggttgaagtgaagcctgggtcaaaggtgaacacaccttttgaaccgagagtacggatatcaataacatcttgacccagcgtgcctttcagcacatccagttcaacagctgtatccccgttgagggtgagttttgcttttgtatcagccatttaaggtctccttagcgccttattgcgtaagactgccggaacttaaatttgccttcgcacatcaacctggctttacccgttttttatttggctcgccgctctgtgaaagaggggaaaacctgggtacagagctctgggcgcttgcaggtaaaggatccattgatgacgaataaatggcgaatcaagtacttagcaatccgaattattaaacttgtctaccactaataactgtcccgaatgaattggtcaatacttccacactgttacataagttaatcttaggtgaaataccgacttcataacttttacgcattatatgcttttcctggtaatgtttgtaacaactttgttgaatgattgtcaaattagatgattaaaaattaaataaatgttgttatcgtgacctggatcactgttcaggataaaacccgacaaactatatgtaggttaattgtaatgattttgtgaacagcctatactgccgccaggtctccggaacaccctgcaatcccgagccacccagcgttgtaacgtgtcgttttcgcatctggaagcagtgttttgcatgacgcgcagttatagaaaggacgctgtctgacccgcaagcagaccggaggaaggaaatcccgacgtctccaggtaacagaaagttaacctctgtgcccgtagtccccagggaataataagaacagcatgtgggcgttattcatgataagaaatgtgaaaaaacaaagacctgttaatctggacctacagaccatccggttccccatcacggcgatagcgtccattctccatcgcgtttccggtgtgatcacctttgttgcagtgggcatcctgctgtggcttctgggtaccagcctctcttcccctgaaggtttcgagcaagcttccgcgattatgggcagcttcttcgtcaaatttatcatgtggggcatccttaccgctctggcgtatcacgtcgtcgtaggtattcgccacatgatgatggattttggctatctggaagaaacattcgaagcgggtaaacgctccgccaaaatctcctttgttattactgtcgtgctttcacttctcgcaggagtcctcgtatggtaagcaacgcctccgcattaggacgcaatggcgtacatgatttcatcctcgttcgcgctaccgctatcgtcctgacgctctacatcatttatatggtcggttttttcgctaccagtggcgagctgacatatgaagtctggatcggtttcttcgcctctgcgttcaccaaagtgttcaccctgctggcgctgttttctatcttgatccatgcctggatcggcatgtggcaggtgttgaccgactacgttaaaccgctggctttgcgcctgatgctgcaactggtgattgtcgttgcactggtggtttacgtgatttatggattcgttgtggtgtggggtgtgtgatgaaattgccagtcagagaatttgatgcagttgtgattggtgccggtggcgcaggtatgcgcgcggcgctgcaaatttcccagagcggccagacctgtgcgctgctctctaaagtcttcccgacccgttcccataccgtttctgcgcaaggcggcattaccgttgcgctgggtaatacccatgaagataactgggaatggcatatgtacgacaccgtgaaagggtcggactatatcggtgaccaggacgcgattgaatatatgtgtaaaaccgggccggaagcgattctggaactcgaacacatgggcctgccgttctcgcgtctcgatgatggtcgtatctatcaacgtccgtttggcggtcagtcgaaaaacttcggcggcgagcaggcggcacgcactgcggcagcagctgaccgtaccggtcacgcactgttgcacacgctttatcagcagaacctgaaaaaccacaccaccattttctccgagtggtatgcgctggatctggtgaaaaaccaggatggcgcggtggtgggttgtaccgcactgtgcatcgaaaccggtgaagtggtttatttcaaagcccgcgctaccgtgctggcgactggcggagcagggcgtatttatcagtccaccaccaacgcccacattaacaccggcgacggtgtcggcatggctatccgtgccggcgtaccggtgcaggatatggaaatgtggcagttccacccgaccggcattgccggtgcgggcgtactggtcaccgaaggttgccgtggtgaaggcggttatctgctgaacaaacatggcgaacgttttatggagcgttatgcgccgaacgccaaagacctggcgggccgtgacgtggttgcgcgttccatcatgatcgaaatccgtgaaggtcgcggctgtgatggtccgtgggggccacacgcgaaactgaaactcgatcacctgggtaaagaagttctcgaatcccgtctgccgggtatcctggagctttcccgtaccttcgctcacgtcgatccggtgaaagagccgattccggttatcccaacctgtcactacatgatgggcggtattccgaccaaagttaccggtcaggcactgactgtgaatgagaaaggcgaagatgtggttgttccgggactgtttgccgttggtgaaatcgcttgtgtatcggtacacggcgctaaccgtctgggcggcaactcgctgctggacctggtggtctttggtcgcgcggcaggtctgcatctgcaagagtctatcgccgagcagggcgcactgcgcgatgccagcgagtctgatgttgaagcgtctctggatcgcctgaaccgctggaacaataatcgtaacggtgaagatccggtggcgatccgtaaagcgctgcaagaatgtatgcagcataacttctcggtcttccgtgaaggtgatgcgatggcgaaagggcttgagcagttgaaagtgatccgcgagcgtctgaaaaatgcccgtctggatgacacttccagcgagttcaacacccagcgcgttgagtgcctggaactggataacctgatggaaacggcgtatgcaacggctgtttctgccaacttccgtaccgaaagccgtggcgcgcatagccgcttcgacttcccggatcgtgatgatgaaaactggctgtgccactccctgtatctgccagagtcggaatccatgacgcgccgaagcgtcaacatggaaccgaaactgcgcccggcattcccgccgaagattcgtacttactaatgcggagacaggaaaatgagactcgagttttcaatttatcgctataacccggatgttgatgatgctccgcgtatgcaggattacaccctggaagcggatgaaggtcgcgacatgatgctgctggatgcgcttatccagctaaaagagaaagatcccagcctgtcgttccgccgctcctgccgtgaaggtgtgtgcggttccgacggtctgaacatgaacggcaagaatggtctggcctgtattaccccgatttcggcactcaaccagccgggcaagaagattgtgattcgcccgctgccaggtttaccggtgatccgcgatttggtggtagacatgggacaattctatgcgcaatatgagaaaattaagccttacctgttgaataatggacaaaatccgccagctcgcgagcatttacagatgccagagcagcgcgaaaaactcgacgggctgtatgaatgtattctctgcgcatgttgttcaacctcttgtccgtctttctggtggaatcccgataagtttatcggcccggcaggcttgttagcggcatatcgtttcctgattgatagccgtgataccgagactgacagccgcctcgacggtttgagtgatgcattcagcgtattccgctgtcacagcatcatgaactgcgtcagtgtatgtccgaaggggctgaacccgacgcgcgccatcggccatatcaagtcgatgttgttgcaacgtaatgcgtaaaccgtaggcctgataagacgcgcaagcgtcgcatcaggcaaccagtgccggatgcggcgtgaacgccttatccggcctacaagtcattacccgtaggcctgataagcgcagcgcatcaggcgtaacaaagaaatgcaggaaatctttaaaaactgcccctgacactaagacagtttttaaaggttccttcgcgagccactacgtagacaagagctcgcaagtgaaccccggcacgcacatcactgtgcgtggtagtatccacggcgaagtaagcataaaaaagatgcttaagggatcacgatgcagaacagcgctttgaaagcctggttggactcttcttacctctctggcgcaaaccagagctggatagaacagctctatgaagacttcttaaccgatcctgactcggttgacgctaactggcgttcgacgttccagcagttacctggtacgggagtcaaaccggatcaattccactctcaaacgcgtgaatatttccgccgcctggcgaaagacgcttcacgttactcttcaacgatctccgaccctgacaccaatgtgaagcaggttaaagtcctgcagctcattaacgcataccgcttccgtggtcaccagcatgcgaatctcgatccgctgggactgtggcagcaagataaagtggccgatctggatccgtctttccacgatctgaccgaagcagacttccaggagaccttcaacgtcggttcatttgccagcggcaaagaaaccatgaaactcggcgagctgctggaagccctcaagcaaacctactgcggcccgattggtgccgagtatatgcacattaccagcaccgaagaaaaacgctggatccaacagcgtatcgagtctggtcgcgcgactttcaatagcgaagagaaaaaacgcttcttaagcgaactgaccgccgctgaaggtcttgaacgttacctcggcgcaaaattccctggcgcaaaacgcttctcgctggaaggcggtgacgcgttaatcccgatgcttaaagagatgatccgccacgctggcaacagcggcacccgcgaagtggttctcgggatggcgcaccgtggtcgtctgaacgtgctggtgaacgtgctgggtaaaaaaccgcaagacttgttcgacgagttcgccggtaaacataaagaacacctcggcacgggtgacgtgaaataccacatgggcttctcgtctgacttccagaccgatggcggcctggtgcacctggcgctggcgtttaacccgtctcaccttgagattgtaagcccggtagttatcggttctgttcgtgcccgtctggacagacttgatgagccgagcagcaacaaagtgctgccaatcaccatccacggtgacgccgcagtgaccgggcagggcgtggttcaggaaaccctgaacatgtcgaaagcgcgtggttatgaagttggcggtacggtacgtatcgttatcaacaaccaggttggtttcaccacctctaatccgctggatgcccgttctacgccgtactgtactgatatcggtaagatggttcaggccccgattttccacgttaacgcggacgatccggaagccgttgcctttgtgacccgtctggcgctcgatttccgtaacacctttaaacgtgatgtcttcatcgacctggtgtgctaccgccgtcacggccacaacgaagccgacgagccgagcgcaacccagccgctgatgtatcagaaaatcaaaaaacatccgacaccgcgcaaaatctacgctgacaagctggagcaggaaaaagtggcgacgctggaagatgccaccgagatggttaacctgtaccgcgatgcgctggatgctggcgattgcgtagtggcagagtggcgtccgatgaacatgcactctttcacctggtcgccgtacctcaaccacgaatgggacgaagagtacccgaacaaagttgagatgaagcgcctgcaggagctggcgaaacgcatcagcacggtgccggaagcagttgaaatgcagtctcgcgttgccaagatttatggcgatcgccaggcgatggctgccggtgagaaactgttcgactggggcggtgcggaaaacctcgcttacgccacgctggttgatgaaggcattccggttcgcctgtcgggtgaagactccggtcgcggtaccttcttccaccgccacgcggtgatccacaaccagtctaacggttccacttacacgccgctgcaacatatccataacgggcagggcgcgttccgtgtctgggactccgtactgtctgaagaagcagtgctggcgtttgaatatggttatgccaccgcagaaccacgcactctgaccatctgggaagcgcagttcggtgacttcgccaacggtgcgcaggtggttatcgaccagttcatctcctctggcgaacagaaatggggccggatgtgtggtctggtgatgttgctgccgcacggttacgaagggcaggggccggagcactcctccgcgcgtctggaacgttatctgcaactttgtgctgagcaaaacatgcaggtttgcgtaccgtctaccccggcacaggtttaccacatgctgcgtcgtcaggcgctgcgcgggatgcgtcgtccgctggtcgtgatgtcgccgaaatccctgctgcgtcatccgctggcggtttccagcctcgaagaactggcgaacggcaccttcctgccagccatcggtgaaatcgacgagcttgatccgaagggcgtgaagcgcgtagtgatgtgttctggtaaggtttattacgacctgctggaacagcgtcgtaagaacaatcaacacgatgtcgccattgtgcgtatcgagcaactctacccgttcccgcataaagcgatgcaggaagtgttgcagcagtttgctcacgtcaaggattttgtctggtgccaggaagagccgctcaaccagggcgcatggtactgcagccagcatcatttccgtgaagtgattccgtttggggcttctctgcgttatgcaggccgcccggcctccgcctctccggcggtagggtatatgtccgttcaccagaaacagcaacaagatctggttaatgacgcgctgaacgtcgaataaataaaggatacacaatgagtagcgtagatattctggtccctgacctgcctgaatccgtagccgatgccaccgtcgcaacctggcataaaaaacccggcgacgcagtcgtacgtgatgaagtgctggtagaaatcgaaactgacaaagtggtactggaagtaccggcatcagcagacggcattctggatgcggttctggaagatgaaggtacaacggtaacgtctcgtcagatccttggtcgcctgcgtgaaggcaacagcgccggtaaagaaaccagcgccaaatctgaagagaaagcgtccactccggcgcaacgccagcaggcgtctctggaagagcaaaacaacgatgcgttaagcccggcgatccgtcgcctgctggctgaacacaatctcgacgccagcgccattaaaggcaccggtgtgggtggtcgtctgactcgtgaagatgtggaaaaacatctggcgaaagccccggcgaaagagtctgctccggcagcggctgctccggcggcgcaaccggctctggctgcacgtagtgaaaaacgtgtcccgatgactcgcctgcgtaagcgtgtggcagagcgtctgctggaagcgaaaaactccaccgccatgctgaccacgttcaacgaagtcaacatgaagccgattatggatctgcgtaagcagtacggtgaagcgtttgaaaaacgccacggcatccgtctgggctttatgtccttctacgtgaaagcggtggttgaagccctgaaacgttacccggaagtgaacgcttctatcgacggcgatgacgtggtttaccacaactatttcgacgtcagcatggcggtttctacgccgcgcggcctggtgacgccggttctgcgtgatgtcgataccctcggcatggcagacatcgagaagaaaatcaaagagctggcagtcaaaggccgtgacggcaagctgaccgttgaagatctgaccggtggtaacttcaccatcaccaacggtggtgtgttcggttccctgatgtctacgccgatcatcaacccgccgcagagcgcaattctgggtatgcacgctatcaaagatcgtccgatggcggtgaatggtcaggttgagatcctgccgatgatgtacctggcgctgtcctacgatcaccgtctgatcgatggtcgcgaatccgtgggcttcctggtaacgatcaaagagttgctggaagatccgacgcgtctgctgctggacgtgtagtagtttaagtttcacctgcactgtagaccggataaggcattatcgccttctccggcaattgaagcctgatgcgacgctgacgcgtcttatcaggcctacgggaccaccaatgtaggtcggataaggcgcaagcgccgcatccgacaagcgatgcctgatgtgacgtttaacgtgtcttatcaggcctacgggtgaccgacaatgcccggaagcgatacgaaatattcggtctacggtttaaaagataacgattactgaaggatggacagaacacatgaacttacatgaatatcaggcaaaacaactttttgcccgctatggcttaccagcaccggtgggttatgcctgtactactccgcgcgaagcagaagaagccgcttcaaaaatcggtgccggtccgtgggtagtgaaatgtcaggttcacgctggtggccgcggtaaagcgggcggtgtgaaagttgtaaacagcaaagaagacatccgtgcttttgcagaaaactggctgggcaagcgtctggtaacgtatcaaacagatgccaatggccaaccggttaaccagattctggttgaagcagcgaccgatatcgctaaagagctgtatctcggtgccgttgttgaccgtagttcccgtcgtgtggtctttatggcctccaccgaaggcggcgtggaaatcgaaaaagtggcggaagaaactccgcacctgatccataaagttgcgcttgatccgctgactggcccgatgccgtatcagggacgcgagctggcgttcaaactgggtctggaaggtaaactggttcagcagttcaccaaaatcttcatgggcctggcgaccattttcctggagcgcgacctggcgttgatcgaaatcaacccgctggtcatcaccaaacagggcgatctgatttgcctcgacggcaaactgggcgctgacggcaacgcactgttccgccagcctgatctgcgcgaaatgcgtgaccagtcgcaggaagatccgcgtgaagcacaggctgcacagtgggaactgaactacgttgcgctggacggtaacatcggttgtatggttaacggcgcaggtctggcgatgggtacgatggacatcgttaaactgcacggcggcgaaccggctaacttccttgacgttggcggcggcgcaaccaaagaacgtgtaaccgaagcgttcaaaatcatcctctctgacgacaaagtgaaagccgttctggttaacatcttcggcggtatcgttcgttgcgacctgatcgctgacggtatcatcggcgcggtagcagaagtgggtgttaacgtaccggtcgtggtacgtctggaaggtaacaacgccgaactcggcgcgaagaaactggctgacagcggcctgaatattattgcagcaaaaggtctgacggatgcagctcagcaggttgttgccgcagtggaggggaaataatgtccattttaatcgataaaaacaccaaggttatctgccagggctttaccggtagccaggggactttccactcagaacaggccattgcatacggcactaaaatggttggcggcgtaaccccaggtaaaggcggcaccacccacctcggcctgccggtgttcaacaccgtgcgtgaagccgttgctgccactggcgctaccgcttctgttatctacgtaccagcaccgttctgcaaagactccattctggaagccatcgacgcaggcatcaaactgattatcaccatcactgaaggcatcccgacgctggatatgctgaccgtgaaagtgaagctggatgaagcaggcgttcgtatgatcggcccgaactgcccaggcgttatcactccgggtgaatgcaaaatcggtatccagcctggtcacattcacaaaccgggtaaagtgggtatcgtttcccgttccggtacactgacctatgaagcggttaaacagaccacggattacggtttcggtcagtcgacctgtgtcggtatcggcggtgacccgatcccgggctctaactttatcgacattctcgaaatgttcgaaaaagatccgcagaccgaagcgatcgtgatgatcggtgagatcggcggtagcgctgaagaagaagcagctgcgtacatcaaagagcacgttaccaagccagttgtgggttacatcgctggtgtgactgcgccgaaaggcaaacgtatgggccacgcgggtgccatcattgccggtgggaaagggactgcggatgagaaattcgctgctctggaagccgcaggcgtgaaaaccgttcgcagcctggcggatatcggtgaagcactgaaaactgttctgaaataaatatctgtaataagaaatagccctcgccgcttccctctacaggaatggcgaagggctgtcggtttcgacatggttggccatcgtatgatggccttttttgtgcttatcgcgatgattttcgctgcgctatcagggtaaatttatagtcatcggtattaaaagcgttgcggctatattcaaacacccgaccatcaactaaatatccacgcgatactttttcaagaatcggctttgtctggctgatattaagcagacggctcatctcttcggttggcatcagaggaatgatttcctgttcgctacgatcgataaccattttcttcacttcttcgataaagtgatatttcgaattttccatgacctgccaggtgagatccgggaacaacgcaagcggcatccaggtttcttccagcgccattggcttttgcttgcgatagcgcacgcgcttcacatgccacacacgatcctgcggggtgatttgtagctgttgctgaagaaaatcgtcagccggaatcacttcgaatatcagaacttcactgtgtgtatcgacgtgacggtccgacagtttttcatcaaaactggttaactgaaaaatatcgtaattgacccgctcttctttgacgtaagtcccgctgccctgaatgctttcgaggatctgctgctcgactagctggcgcaaagcctgacgcaccgtaacccggctgacgccaaactctgtttgtagcgctgattcagtgggtaacgcatcgccaggtttaagctcgccacgcgcaatttgttcacgaatgcgatcggcaatctgccggtataagggcttgtgtcccatttttagtatctcattaatacgaatttaaccattatgcccgataaattcatcctgtaaataatacaaatacaatacaaataatttcaatcaagtgaaattgatcacataatggtattgttttatcgggcacactggcgcgactataaaaacgatcaagtgaggatcatgatgaatctgacgactctgacccaccgcgatgcgttgtgtctgaatgcgcgctttaccagccgtgaagaggccatccacgcgttgactcaacgtcttgctgctctggggaaaatttccagtactgagcaatttctggaagaagtgtatcgccgtgaaagccttggcccgaccgccttaggtgaagggttggctgtgccgcatggcaaaactgctgcggtaaaagaagcggcgtttgcggtcgccacactcagcgagccgcttcagtgggaaggcgttgatggcccggaagcagttgatttagtggtgctgctggcgattccccccaatgaagcgggtactacgcatatgcaactgctgacagcgctgaccacgcgccttgcggatgatgagattcgggcgcgtatacagtcggcgacgacgcctgatgagttgctctcggcgctggatgacaagggaggcacgcaaccttctgcctctttttccaacgcgccaactatcgtctgcgtaacggcctgtccggcgggtattgctcacacctatatggctgcggaatatctggaaaaagccggacgcaaactcggcgtaaatgtttacgttgaaaaacaaggcgctaacggcattgaagggcgtttaacggcggatcaactcaatagtgcaaccgcctgtatttttgcggctgaagtcgccatcaaggagagtgagcgttttaatggcattcccgcgctttcagtgcctgttgccgagccgattcgccatgcagaagcgttgatccaacaagcgcttaccctcaagcgtagcgatgagacgcgtaccgtacagcaagatacgcaaccggtgaaaagtgtcaaaacggagctgaaacaggcactgttgagcggaatctcttttgccgtaccgttgattgtcgcggggggcacggtgctggcggtcgcggtattactgtcgcaaatcttcgggctacaagatctgtttaatgaagaaaactcctggctgtggatgtaccgcaagctgggcggcgggctgctcggaattttgatggtaccggtgctcgcggcctataccgcctattctctggcagataaaccggcgttagcgccaggctttgcggctggacttgccgccaacatgatcggctccgggtttctcggcgcggtcgttggcggattgatagccggttacttgatgcgctgggtgaaaaatcacttgcgtcttagcagtaaattcaatggattcctgactttttatctctacccggtgctcggtacgttgggagcgggcagtctgatgctgtttgtggtgggggaacctgtcgcctggatcaataactcgcttaccgcctggctgaacggtctgtcaggaagtaacgcgctgttgctgggtgccattctcggttttatgtgttcctttgaccttggagggccagtgaataaagccgcttatgcattctgcctgggcgcaatggcgaacggcgtttacggcccgtatgccattttcgcctccgtcaaaatggtttcggcatttaccgtaaccgcttccacgatgctcgcaccgcgcctgtttaaagagtttgaaattgagaccgggaaatccacctggctgttagggctggcaggtattaccgaaggggcgatcccgatggcgattgaagatccgctgcgggttattggttcgtttgtgctgggctctatggtaacgggcgctattgtcggtgcgatgaatatcggcctttcgacacccggtgccggcattttctcgctctttttacttcatgataatggcgcgggcggtgttatggcggcaattggctggtttggcgcggcattggtgggggctgcaatctcgactgcaattctcctgatgtggcggcgtcacgcggttaagcatggcaactatctgactgatggcgtaatgccataaacaaaaaggaaacgacgatgaaagcagtatctcgcgttcacatcaccccgcatatgcactgggatcgagagtggtatttcaccaccgaagagtcacgtattctgctggtcaataatatggaagagatcctgtgccgactggaacaggacaacgaatacaaatattacgtactcgacgggcaaacggcgatcctcgaagattatttcgcggtgaaaccggaaaacaaagaccgtgtgaagaaacaggtagaagccggcaagttgattatcggcccctggtatacccagaccgataccacgattgtttctgcggaatccatcgtccgtaatctgatgtacggaatgcgtgactgcctcgcgtttggcgagccgatgaaaataggttatttaccagattcctttggcatgtccgggcaactgccgcatatctacaatggatttggcattacccgcaccatgttctggcgcggatgttcggagcgccacggtactgataaaaccgagtttttgtggcaaagcagtgacggtagcgaagtgacggcgcaggtgctgccgctgggctacgccatcggtaagtacttacctgccgacgaaaacggattacgtaaacgcctcgacagttattttgacgtgctggaaaaagcgtctgtaaccaaagagattttgctgccgaatgggcatgaccagatgccattgcagcaaaatatcttcgaagtgatggataagctacgtgagatctaccctcaacgtaagtttgtgatgagccgctttgaagaggtatttgagaagatcgaagcgcagcgagataatctggcaaccctgaaaggggaatttattgatggcaaatatatgcgcgtgcatcgcaccatcggttctacgcgtatggatatcaaaattgcccacgcgcgtattgaaaataagattgttaatctgctggaaccgctggcaacactggcctggacgttgggttttgaataccaccacggcttgctggagaaaatgtggaaagagatcttaaaaaatcatgcccacgacagtatcggctgctgctgtagtgacaaagttcatcgcgaaatcgtcgcccgcttcgaactggctgaagacatggcggataatctgattcgtttctacatgcgcaaaattgccgacaacatgccgcagagcgacgccgacaaactcgtcctgtttaacctgatgccctggccgcgtgaagaagttatcaacaccactgtgcggctgcgcgccagccagtttaatttgcgggacgatcgcggtcagcctgtaccgtattttattcgccatgcccgtgagatcgatccaggcctaatcgatcggcaaatagttcattacggtaattacgatccctttatggagtttgatatacagatcaaccagattgtcccttctatgggctatcgcacgctttatatcgaagcgaatcagcctggcaacgtaattgcggcaaaaagtgacgctgaagggatactggaaaatgctttctggcaaattgcgctcaatgaggatggttctctgcaactggtagataaagacagcggtgtgcgctatgaccgggtattgcaaattgaagaaagctctgatgatggtgatgaatatgactattcacccgcaaaagaagagtgggtaattaccgcagcgaacgcgaaaccgcaatgcgatattattcatgaagcctggcagagcagggctgttatccgctatgacatggcagtgccgctcaatttgtcagaacgcagcgcccggcaatccactggcagagtaggggtggtgttggttgtcactcttagtcataacagcaggcgtattgatgtggatatcaatcttgataaccaggctgacgatcatcgccttcgtgtcctggtccctacaccttttaacaccgacagtgttctggcagatacgcagtttggttcgctaacgcgccccgtgaacgacagtgcaatgaacaactggcagcaagaaggctggaaagaagcgccggttccggtatggaatatgctcaactatgttgccttacaggaagggcgtaacggcatggctgtctttagcgaagggttacgtgaatttgaagtcatcggtgaagagaagaaaacctttgccattacgttgctgcgtggcgtgggcttactgggcaaagaagatctgcttttaaggcctgggcggccttcgggaattaaaatgccagtcccggactcacaactacgtggtctgctttcttgtcgcctaagtttattgagttataccggtacgccaaccgccgctggtgtagctcagcaggcgcgagcatggctgactccagtacagtgttacaacaaaatcccatgggatgtgatgaagctcaacaaagccggattcaacgtgccggaaagttatagtttgttgaaaatgcccccagtgggatgcctgataagcgcacttaagaaagctgaagaccgacaagaagtgattttacggctgtttaatccggctgaatcagcaacctgtgatgcgactgttgctttcagtcgcgaggtgatttcttgctcagaaacgatgatggatgaacacattaccaccgaggaaaatcaaggttcaaatctatcggggccttttttacccggccagtcacggacgttcagttaccggcttgcctgaatagcaatcaaaccgaagccacatatgcgcggccagattgttgacaaagggcgctttgttcatgccggatacggcatgaacgctttattcggtctacaaaagcaggcaaattcaatatattgcagagatgatgtagacactggcaagcgtagcgcatcaggtaattttgcgtttatcttcactctcaagccacgtatatgtggctttatttttaacaaaataataaccctgggtgagttaattataatataattataagttaactaaatgttaatattggcggggtggatttatgcctttattagtaatcctgaaactctgcgtcgtattagccagtgaccaaaaaaagaattaaggtcaaccgtgctgtttttgcttcgtctctttttatctttaattgccaaccgaaactaatttcagccttataactcacacattttaaacataaatgtcactaaagttaccttattgaaacatgattaacataatttgtaggaattgatatttatcaatgtataagtcttggaaatgggcatcaaaaagagataaattgttctcgatcaaattggctgaaaggcggtaatttagctataaattgatcaccgtcgaaaaatgcaaatttgcttcaacaaaaacctgtttattgtaaggattttgcggcgtaatatatacgtgggatcaatttgagtttttattaacatgtttgcaacctttctttacgccgtttttgtgtgcattcacatggtatgatgaaagtgttcaaacaaatttctattggggcatgcgtgtgaccctttctaacggggttcactctcggagtcttcatgcgatgagcaaggagtcatgatgttagatatagtcgaactgtcgcgcttacagtttgccttgaccgcgatgtaccacttcctttttgtgccactgacgctcggtatggcgttcctgctggccattatggaaacggtctacgtcctctccggcaaacagatttataaagatatgaccaagttctggggcaagttgtttggtatcaacttcgctctgggtgtggctaccggtctgaccatggagttccagttcgggactaactggtcttactattcccactatgtaggggatatcttcggtgcgccgctggcaatcgaaggtctgatggccttcttcctcgaatccacctttgtaggtctgttcttcttcggttgggatcgtctgggtaaagttcagcatatgtgtgtcacctggctggtggcgctcggttcaaacctgtccgcactgtggattctggttgcgaacggctggatgcaaaacccaatcgcgtccgatttcaactttgaaactatgcgtatggagatggtgagcttctccgagctggtgcttaacccggttgctcaggtgaaattcgttcacactgtagcgtctggttatgtgactggcgcgatgttcatcctcggtatcagcgcatggtatatgctgaaaggtcgtgacttcgccttcgctaaacgctcctttgctatcgctgccagcttcggtatggctgctgttctgtctgttattgttctgggtgatgaatccggctacgaaatgggcgacgtgcagaaaaccaaactggctgctattgaagccgagtgggaaacgcaacctgcgcctgctgcctttactctgttcggcattcctgatcaggaagaggagacgaacaaatttgcgattcagatcccttacgcactgggcatcattgcaacgcgttccgtggataccccggttatcggcctgaaagagctgatggtgcagcatgaagaacgcattcgtaacgggatgaaggcgtactctctgctcgaacaactgcgttctggttctaccgaccaggcggttcgtgaccagttcaatagcatgaagaaagacctcggttacggtctgctgctgaaacgctatacgccaaacgtggctgatgcgactgaagcgcagattcaacaggcaaccaaagactccatcccgcgtgtagcgccgctgtactttgcgttccgtatcatggtggcgtgtggcttcctgcttctggcaatcatcgcgctctctttctggagtgtcatccgcaaccgcattggcgagaaaaaatggcttctgcgcgccgcgctgtacggtattccgctgccgtggattgctgtagaagcgggctggttcgtggctgaatatggccgccaaccgtgggctatcggtgaagtgctgccgacagctgtggcgaactcgtcactgaccgcaggcgatctcatcttctcaatggtgctgatttgcggcctgtataccctgttcctggtggcagaattgttcttaatgttcaagtttgcacgcctcggcccaagcagcctgaaaaccggtcgctatcactttgagcagtcttccacgactactcagccggcacgctaagacaggagtcgtcaaatgatcgattatgaagtattgcgttttatctggtggctgctggttggcgttctgctgattggttttgcagtcactgacggtttcgacatgggggtgggcatgctcacccgtttcctcggtcgtaacgacaccgagcgtcgaattatgattaactccattgcaccacactgggacggtaaccaggtttggctgatcaccgcgggcggcgcactctttgctgcctggccgatggtctatgccgctgcgttctccggcttctatgtggcgatgatcctcgtgctggcgtctttgttcttccgtccggtcggttttgactaccgctccaagattgaagaaacccgctggcgtaacatgtgggactggggcatcttcattggtagcttcgttccgccgctggtaattggtgtagcgttcggtaacctgttgcagggcgtaccgttcaacgttgatgaatatctgcgtctgtactacaccggtaacttcttccagttgcttaacccgttcggcctgctggcaggcgtggtgagcgtagggatgatcattactcagggcgcaacctatctgcaaatgcgtaccgtgggcgaactgcacctgcgtacccgtgcaacggctcaggtggctgcgctggtgacactggtctgtttcgcactggctggcgtatgggtgatgtacggtatcgatggttatgtcgtgaaatcgacaatggaccattacgcagcctctaacccactgaataaagaagtggttcgtgaagctggcgcatggctggttaacttcaacaacacgccaattctgtgggctattccggcactgggtgtggttctgccgctgctgaccatcctgactgcacgtatggataaagccgcgtgggcgtttgtgttctcctccctgacgctggcctgcatcatcctgacagccggtatcgcaatgttcccgtttgtgatgccgtccagcaccatgatgaacgcaagtctgacaatgtgggatgcaacttccagccagctgacgcttaacgtcatgacctgggttgcggtggttctggtaccgatcattctgctctacaccgcctggtgttactggaaaatgttcggtcgtatcaccaaagaagatattgaacgtaacacccactctctgtactaagtaaggagctaaaaatgtggtatttcgcatggattctgggaacgcttcttgcctgttcgtttggggtaatcaccgcgctggcgcttgaacacgtcgaatcaggcaaagccggtcaagaagacatctgatgagtaagattatcgcgactttgtatgcggtaatggacaagcgccccctgcgggcgctttccttcgtgatggcgcttctgttagcaggatgtatgttttgggacccatctcgttttgccgcgaagaccagtgaactggaaatctggcatggtttattgctgatgtgggccgtctgtgctggtgtgattcacggcgtgggctttcgtccgcagaaggttctttggcaagggattttttgcccattgcttgccgatattgttctcattgtcgggctgattttcttcttcttttaaatcagaattctctttaaaaaattatgggccgctccaggcccataaatttttacgctcccttaacttgccctcattcccaaacctcaatcgcgcgcgtatagtagcagcgtttaaaagctctaacttttgttgcattaccgggatgtaaagtgaatacaacgctgtttcgatggccggttcgcgtctactatgaagataccgatgccggtggtgtggtgtaccacgccagttacgtcgctttttatgaaagagcacgcacagagatgctgcgtcatcatcacttcagtcagcaggcgctgatggctgaacgcgttgcctttgtggtacgtaaaatgacggtggaatattacgcacctgcgcggctcgacgatatgctcgaaatacagactgaaataacatcaatgcgtggcacctctttggttttcacgcaacgtattgtcaacgccgagaatactttgctgaatgaagcagaggttctggttgtttgcgttgacccactcaaaatgaagcctcgtgcgcttcccaagtctattgtcgcggagtttaagcagtgactgacatgaatatccttgatttgttcctgaaggctagccttctggttaaacttatcatgttgattttgattggtttttcaatcgcatcttgggccattattatccagcggacccgtattcttaacgcagcggcgcgcgaagccgaagcgtttgaagataaattctggtctggaatcgaactctctcgcctctatcaagagagccaggggaaacgggataatctgactggttcggaacaaatcttttacagcgggttcaaagagtttgtgcgcctgcatcgtgccaatagccatgcgccggaagccgtagtggaaggggcgtcgcgtgctatgcgtatctccatgaaccgtgaacttgaaaatctggaaacgcacattccgttcctcggtacggttggctccatcagcccgtatattggtctgtttggtacggtctgggggatcatgcacgcctttatcgccctcggggcggtaaaacaagcaacactgcaaatggttgcgcccggtatcgcagaagcgttgattgcgactgcaattggtctgtttgccgctatcccggcagttatggcctacaaccgcctcaaccagcgcgtaaacaaactggaactgaattacgacaactttatggaagagtttaccgcgattctgcaccgccaggcgtttaccgttagcgagagcaacaaggggtaagccatggccagagcgcgtggacgaggtcgtcgcgatctcaagtccgaaatcaacattgtaccgttgctggacgtactgctggtgctgttgctgatctttatggcgacagcgcccatcatcacccagagcgtggaggtcgatctgccagacgctactgaatcacaggcggtgagcagtaacgataatccgccagtgattgttgaagtgtctggtattggtcagtacaccgtggtggttgagaaagatcgcctggagcgtttaccaccagagcaggtggtggcggaagtgtccagccgtttcaaggccaacccgaaaacggtctttctgatcggtggcgcaaaagatgtgccttacgatgaaataattaaagcactgaacttgttacatagtgcgggtgtgaaatcggttggtttaatgacgcagcctatctaaacatctgcgtttcccttgcttgaaagagagcgggtaacaggcgaacagtttttggaaaccgagagtgtcaaaggcaaccgaacaaaacgacaagctcaagcgggcgataattatttcagcagtgctgcatgtcatcttatttgcggcgctgatctggagttcgttcgatgagaatatagaagcttcagccggaggcggcggtggttcgtccatcgacgctgtcatggttgattcaggtgcggtagttgagcagtacaaacgcatgcaaagccaggaatcaagcgcgaagcgttctgatgaacagcgcaagatgaaggaacagcaggctgctgaagaactgcgtgagaaacaagcggctgaacaggaacgcctgaagcaacttgagaaagagcggttagcggctcaggagcagaaaaagcaggctgaagaagccgcaaaacaggccgagttaaagcagaagcaagctgaagaggcggcagcgaaagcggcggcagatgctaaagcgaaggccgaagcagatgctaaagctgcggaagaagcagcgaagaaagcggctgcagacgcaaagaaaaaagcagaagcagaagccgccaaagccgcagccgaagcgcagaaaaaagccgaggcagccgctgcggcactgaagaagaaagcggaagcggcagaagcagctgcagctgaagcaagaaagaaagcggcaactgaagctgctgaaaaagccaaagcagaagctgagaagaaagcggctgctgaaaaggctgcagctgataagaaagcggcagcagagaaagctgcagccgacaaaaaagcagcagaaaaagcggctgctgaaaaggcagcagctgataagaaagcagcggcagaaaaagccgccgcagacaaaaaagcggcagcggcaaaagctgcagctgaaaaagccgctgcagcaaaagcggccgcagaggcagatgatattttcggtgagctaagctctggtaagaatgcaccgaaaacggggggaggggcgaaagggaacaatgcttcgcctgccgggagtggtaatactaaaaacaatggcgcatcaggggccgatatcaataactatgccgggcagattaaatctgctatcgaaagtaagttctatgacgcatcgtcctatgcaggcaaaacctgtacgctgcgcataaaactggcacccgatggtatgttactggatatcaaacctgaaggtggcgatcccgcactttgtcaggctgcgttggcagcagctaaacttgcgaagatcccgaaaccaccaagccaggcagtatatgaagtgttcaaaaacgcgccattggacttcaaaccgtaatcgcgatgttgactgttcggacggtcaacatcaggcaccggttgccacggggttctggtagttttgtgtattttagtttgttaacattctgctaaattatcgtgggccatcggtccagataagggagatatgatgaagcaggcattacgagtagcatttggttttctcatactgtgggcatcagttctgcatgctgaagtccgcattgtgatcgacagcggtgtagattccggtcgtcctattggtgttgttcctttccagtgggcggggcctggtgcggcacctgaagatattggcggcatcgttgctgctgacttgcgtaacagcggtaaatttaatccgttagatcgcgctcgtctgccacagcagccgggtagtgcgcaggaagtacaaccagctgcatggtccgcactgggcattgacgctgtagttgtcggtcaggtcactccgaatccggatggttcttacaatgttgcttatcaacttgttgacactggcggcgcaccgggtactgtacttgctcagaactcgtacaaagtgaacaagcagtggctgcgttatgctggtcataccgccagtgatgaagtgtttgaaaaactgaccggcattaaaggtgcgttccgtactcgtattgcctacgttgttcagaccaacggcggtcagttcccgtatgaactgcgcgtatctgactatgacggttacaaccagtttgtcgttcaccgttcaccgcagccgctgatgtctccggcgtggtcaccagacggttctaaactggcttatgtgaccttcgaaagcggtcgttccgcgctggttattcagacgctggcaaatggcgctgtacgtcaggtggcttcattcccgcgtcacaacggtgcacctgcattctcgccagacggcagcaaactggcattcgccttgtcgaaaaccggtagtctgaacctgtacgtaatggatttggcttctggtcagatccgccaggtgactgatggtcgcagtaacaataccgaaccgacctggttcccggatagccagaacctggcatttacttctgaccaggccggtcgtccgcaggtttataaagtgaatatcaacggcggtgcgccacaacgtattacctgggaaggttcgcagaaccaggatgcggatgtcagcagcgacggtaaatttatggtaatggtcagctccaatggtgggcagcagcacattgccaaacaagatctggcaacgggaggcgtacaagttctgtcgtccacgttcctggatgaaacgccaagtctggcacctaacggcactatggtaatctacagctcttctcaggggatgggatccgtgctgaatttggtttctacagatgggcgtttcaaagcgcgtcttccggcaactgatggacaggtcaaattccctgcctggtcgccgtatctgtgataataattaattgaatagtaaaggaatcattgaaatgcaactgaacaaagtgctgaaagggctgatgattgctctgcctgttatggcaattgcggcatgttcttccaacaagaacgccagcaatgacggcagcgaaggcatgctgggtgccggcactggtatggatgcgaacggcggcaacggcaacatgtcttccgaagagcaggctcgtctgcaaatgcaacagctgcagcagaacaacatcgtttacttcgatctggacaagtacgatatccgttctgacttcgctcaaatgctggatgcacatgcaaacttcctgcgtagcaacccgtcttacaaagtcaccgtagaaggtcacgcggacgaacgtggtactccggaatacaacatctccctgggtgaacgtcgtgcgaacgccgttaagatgtacctgcagggtaaaggcgtttctgcagaccagatctccatcgtttcttacggtaaagaaaaacctgcagtactgggtcatgacgaagcggcatactccaaaaaccgtcgtgcggtactggtttactaagagaattgcatgagcagtaacttcagacatcaactattgagtctgtcgttactggttggtatagcggccccctgggccgcttttgctcaggcaccaatcagtagtgtcggctcaggctcggtcgaagaccgcgtcactcaacttgagcgtatttctaatgctcacagccagcttttaacccaactccagcaacaactttctgataatcaatccgatattgattccctgcgtggtcagattcaggaaaatcagtatcaactgaatcaggtcgtggagcggcaaaagcagatcctgttgcagatcgacagcctcagcagcggtggtgcagcggcgcaatcaaccagcggcgatcaaagcggtgcggcggcatcaacgacgccgacagctgatgctggtactgcgaatgctggcgcgccggtgaaaagcggtaatgcaaacacggattacaatgcagctattgcgctggtgcaggataaatcccgccaggatgacgcaatggtggcatttcagaatttcatcaaaaattaccctgattcaacttacctgccaaacgccaattattggctgggtcagttaaactacaacaagggtaaaaaagatgatgcggcgtactattttgcttcggtagtgaaaaactatccgaagtcaccaaaggctgcagatgcgatgtttaaagtcggcgtcatcatgcaggacaaaggtgacaccgcaaaagcgaaagccgtataccagcaggttatcagtaaataccctggtactgatggcgctaaacaggcacaaaaacgtctgaacgcgatgtaatgcataacacacgaccagaagtcgcattatttctggtcgtgtcgtgcgaatcataagcagttgagtgatctacatcgaaatttttgttgcgctcaagtctgaaatcagtaatatatgccgccgttgccacgggatatcaaacaaaccgaaagcaacgaaaaagtgggtcgttagctcagttggtagagcagttgacttttaatcaattggtcgcaggttcgaatcctgcacgacccaccaatcgctaaggtggaagcggtagtaaaacgtgaaggataacgttgcatgagcaacggcccgaagggcgagacgaagtcgagtcatcctgcacgacccaccactaacatagttagttgtagtatccagcgtagtatcgggtgattagctcagctgggagagcacctcccttacaaggagggggtcggcggttcgatcccgtcatcacccaccaccgggtcgttagctcagttggtagagcagttgacttttaatcaattggtcgcaggttcgaatcctgcacgacccaccagttttaacatcgaagacagatgttaagcgtgtaggataacgttgcgtcagcaacggcccgtagggcgagcgaagcgagtcatcctgcacgacccaccactaatgacggtgggttcggtggaagtagtttgtagtatccagcgcagtatcgggtgattagctcagctgggagagcacctcccttacaaggagggggtcggcggttcgatcccgtcatcacccaccactcgggtcgttagctcagttggtagagcagttgacttttaatcaattggtcgcaggttcgaatcctgcacgacccaccagttttaacatcaaactcagatgttaagcgtgaaggataacgttgcgccagcaacggcccgtagggcgagcgaagcgagtcatcctgcacgacccaccaatcttaaagattggccccgagtaaaaatctttcaggtaacacccgtatgggtcgttagctcagttggtagagcagttgacttttaatcaattggtcgcaggttcgaatcctgcacgacccaccaatttaaaggtggttactggtagagaacgtgaaggataacgttgcgttagcaacggcccgaagggcgagacgaagtcgagtcatcctgcacgacccaccatcctgaatgattaaggcagcataatcccgcaaggggtcgttagctcagttggtagagcagttgacttttaatcaattggtcgcaggttcgaatcctgcacgacccaccaatgtaaaaaagcgccctaaaggcgcttttttgctatctgcgatactcaaagattcgaacctgcagcaggtttgagttgagcgcagcgaaacaacggagccgctcgcggcgacggcccgaagggcgagcgaagcgagtcatcctgcacgacccaccaatgtaaaaaagcgccctaaaggcgcttttttgctattcaggcatcctcaatttcactttgtaaacctgatgacatcgtcagagcttactgtgcaagcaactctatgtcggtggaattaggcgtaaaatgacgcatcctgcacattaggcgtaattcgagtgacttttccccaccattcgactatcttgtttagcatataaaacaaattacaccgataacagcgaatattacgctaatgtcggttttaacgttaagcctgtaaaacgagatggtaagatgagcgtaatgtttgatccagacacggcgatttatcctttccccccgaagccgacgccgttaagcattgatgaaaaagcgtattaccgcgagaagataaaacgtctgctaaaagaacgtaatgcggtgatggttgcccactactataccgatcccgaaattcaacaactggcagaagaaaccggtggctgtatttctgattctctggaaatggcgcgcttcggtgcaaagcatcccgcttctactttgttagtcgctggggtgagatttatgggagaaaccgccaaaattctcagtccggaaaaaacaattctgatgccgacacttcaggctgaatgttcactggatctcggctgccctgttgaagaatttaacgcattttgcgatgcccatcccgatcgtactgtcgtcgtctacgccaacacttctgctgcggtaaaagcgcgcgcagattgggtggtaacttcaagcattgccgtcgaacttattgatcatcttgatagtttgggtgaaaaaatcatctgggcacccgacaaacatctggggcgttacgtgcaaaaacagacgggtggagacattctatgctggcagggtgcctgtattgtgcatgatgaatttaagactcaggcgttaacccgcttgcaagaagaatacccggatgctgccatactggtgcatccagaatcaccacaagctattgtcgatatggcggatgcggtcggttccaccagtcaactgatcgctgctgcgaaaacattgccacatcagaggcttattgtggcaaccgatcggggtattttctacaaaatgcagcaggcggtgccagataaagagttactggaagcaccaaccgcaggtgagggtgcaacctgccgcagctgcgcgcattgtccgtggatggccatgaatggccttcaggccatcgcagaggcattagaacaggaaggaagcaatcacgaggttcatgttgatgaaaggctgcgagagagggcgctggtgccgctcaatcgtatgctggattttgcggctacactacgtggataacgaataataaggcgtaacgttacgctttgggggaaagatggatttttttagtgtgcagaatatcctggtacatataccaataggggcaggcggttatgatctctcatggatcgaagcggtaggcacgatcgccgggttgctgtgtattggccttgccagtctggagaagatcagcaactacttctttggcctgatcaacgtcaccttgtttggcattattttctttcagattcagctgtatgccagcctgctattacaggtgtttttctttgccgcgaatatttacggttggtatgcgtggtcgcgacaaaccagtcagaacgaggcggagttgaaaattcgctggttgccattgccgaaggcactcagctggttggcggtttgcgttgtttcgattggtctgatgacggtatttatcaatccggtgtttgcatttttgacccgcgtggcagtcatgatcatgcaagcattaggattacaggttgtgatgcctgaactgcaaccggacgctttcccgttctgggattcatgcatgatggtgttatctatcgtggcaatgattctgatgacgcgtaagtatgtggaaaactggctgttgtgggtgattattaacgtgattagcgtcgttatttttgcacttcagggcgtttacgccatgtctctggagtacatcatcctgacctttattgcgctcaacggcagccggatgtggatcaacagcgcacgtgaaagaggctcacgcgcgctgtcccattaatggtgatgatgtgaatggccagacaccccttcattcaggtggcagtctggcccatgacaaggttgatattccatctgaatggtggcgtgctcaatctgatagtgatccatcaggtagtgttggatctgatccaacaaggcatcgtgatcgtgtggcgggatcacctgcacatgcaacgtcatcaccggcttctcgcctaccatccatacatgtacatggtgcacattgcggacttccgggatttcccggcacatacgacgcttcagttcagcgatatccagcgataccggtgcaccttcaagtaattcattcacgctatctttcaacagtcgccacgcgctacgcagaaccagaagcgacaccagtatcgagagaatggggtcagcaggtgtccagccagtccagataataatcaacgcggcaataatagccccaaccgaacccagcaggtccccgagcacatgcagtgccgctgctcgtacgttgaggtttttctcttcgctgccgtgatgaagtaaccagaaagaaagtatatttgccagcaacccagccacggcaattgccatcatcatgccgccctcgaccggacgcggcgtgcggaagcgttctatcgcctcccagacaatcaaaatggtaattaccacgagggctatggcattcacaaacgccgcgagcgtggtcagtcttagccaaccgaaagtgtggcgaatggtgggaggacgacgtgaaaattgcacggcgagtagggcgaaaagcagggcggcagtatcggtcaacatatgacccgcatcggccagcaatgccagagaaccagaaagaaaaccaccaacgacttctaccagcataaacccggcagtcacgccgaaagcatacaacaagcgacgagcattattatcttctggcaggtgtgaggacgtgtgtgagtgtgagtgcgccatgacgagtcatcccttaattattctcacttaactttatgacatcatactgcttttagaagtgaaaaattaaaagggagagactccgctctcccattattggctattttgcagggttactgcgtggtaccgtcggttttggtatcgacatcattattgatgccatcaccggtttgtacctttttattgatatccggacagcgaccatctttgcacatggtgttcttgtgctcttcatctttggtcattccgtcattgttcattgaagaaccatccgaatgcagcattgtgccgccagaaccggtatttaccccgttattgtcgacgttatttggcgcgacattttcacgggcgtcaggggctacctggcccgcatcagctgcggcgtttgcctggccgttattagtttgcgctccgctatcggcagccagtgcggcaccgctggcaaggcttagagtggcagtcagaaataatgtggccagttttgtcattttcataggatgctcctgttatggtcgttatgtcggataacctcttccaacagtgcatttgcaggtgaatataaggcattggtttaagatttcagccaggttatgaaacgcagcagagaatcttgaaataattaacaaacaaaggagttacagttagaaattgtaggagagatctcgtttttcgcgacaatctggcgtttttcttgctaattccaggattaatccgttcatagtgtaaaaccccgtttacacattctgacggaagatatagattggaagtattgcattcactaagataagtatggcaacactggaacagacatgaattatcagaacgacgatttacgcatcaaagaaatcaaagagttacttcctcctgtcgcattgctggaaaaattccccgctactgaaaatgccgcgaatacggttgcccatgcccgaaaagcgatccataagatcctgaaaggtaatgatgatcgcctgttggttgtgattggcccatgctcaattcatgatcctgtcgcggcaaaagagtatgccactcgcttgctggcgctgcgtgaagagctgaaagatgagctggaaatcgtaatgcgcgtctattttgaaaagccgcgtaccacggtgggctggaaagggctgattaacgatccgcatatggataatagcttccagatcaacgacggtctgcgtatagcccgtaaattgctgcttgatattaacgacagcggtctgccagcggcaggtgagtttctcgatatgatcaccccacaatatctcgctgacctgatgagctggggcgcaattggcgcacgtaccaccgaatcgcaggtgcaccgcgaactggcatcagggctttcttgtccggtcggcttcaaaaatggcaccgacggtacgattaaagtggctatcgatgccattaatgccgccggtgcgccgcactgcttcctgtccgtaacgaaatgggggcattcggcgattgtgaataccagcggtaacggcgattgccatatcattctgcgcggcggtaaagagcctaactacagcgcgaagcacgttgctgaagtgaaagaagggctgaacaaagcaggcctgccagcacaggtgatgatcgatttcagccatgctaactcgtccaaacaattcaaaaagcagatggatgtttgtgctgacgtttgccagcagattgccggtggcgaaaaggccattattggcgtgatggtggaaagccatctggtggaaggcaatcagagcctcgagagcggggagccgctggcctacggtaagagcatcaccgatgcctgcatcggctgggaagataccgatgctctgttacgtcaactggcgaatgcagtaaaagcgcgtcgcgggtaaggtttaattgtcggatgcgccgtcagagtggcgtatccgatgaatcaccacaggcctgataagtcgcgcagcgtcgcatcaggcaatgtgctccattgttagcaacaaaaaagccgactcacttgcagtcggctttctcattttaaacgaatgacgtttacttcgctttaccctggtttgcaaccgccgctgctttcgctgcgatctcgtcagcattacccagataatagcgtttcagcggtttgaaattctcgtcgaactcatacaccagcggcacgccagtcgggatattaagctcaagaatctcttcttcgctcatgttatcaagatatttcaccagcgcacgtaaagagttaccgtgtgcagcgatgatcacgcgctcaccgctcttcatacgcggcagaatagtttcattccagtaagggatcacgcggtcaatggtcagcgccaggctttccgtcagcggcagttctttctcgctcagtttcgcgtaacgcggatcgtgacccggataacgctcatcatctttagtcagttccggcggagtcactgcaaaaccacgacgccactgtttcacctgctcgtcgccatacttttcagcagtttccgctttgttcagaccctgcaacgcaccgtagtgacgttcgttcagtttccaggatttctcaacgggcagccatgcctgatccagttcgtccagcacattccacagggtatggatagcgcgtttcagcacagaagtgtaagcaaagtcaaagctgtaaccttcctctttcagcagcttacctgctgcttttgcttcgcttacgcctttctcagacagatccacgtcgtaccaaccggtgaaacggttttctttgttccactgactttcgccatgacgaaccagaaccagcttagttacagccatatacttactcctcaaatcatcttttaatgataataattctcattatattgccgcgacgaagcaacagcaatgcttacgcataaccatagcgaaaatagtggcgcagtgtaaggttgttgtgaatattgagttgcaaatatgtcggtgtttgctggtgatttgaacaatatgagataaagccctcatgacgagggcgtaacattactcagcaataaactgatattccgtcaggctggaatactcttcgccaggacgcaggaagcagtccggttgcggccattcagggtggttcgggctgtccggtagaaactcgctttccagagccagcccttgccagtcggcgtaaggttcggttccccgcgacggtgtgccgccgaggaagttgccggagtagaattgcagagccggagcggtggtgtagaccttcagctgcaatttttcatctgctgaccagacatgcgccgccactttcttgccatcgcctttggcctgtaacaagaatgcgtgatcgtaacctttcactttgcgctgatcgtcgtcggcaagaaactcactggcgatgattttggcgctgcggaaatcaaaagacgttccggcgacagatttcaggccgtcgtgcggaatgccgccttcatcaaccggcagatattcgtccgccagaatctgcaacttgtgattgcgcacgtcagactgctcgccgtcaagattgaaatagacgtgattagtcatattcaccgggcaaggtttatcaactgtggcgcgataagtaatggagatacggttatcgtcggtcagacgatattgcaccgtcgcgccgagattacccgggaagccctgatcaccatcatctgaactcagggcaaacagcacctgacgatcgttctggttcacaatctgccagcgacgtttgtcgaacccttccggcccgccgtgcagctggttaacgccctgacttggcgaaagcgtcacggtttcaccgtcaaaggtataacggctattggcgatacggttggcataacgaccaatagaggcccccagaaacgcggcctgatcctgatagcattccgggctggcacagccgagcagcgcctcgcggacgctgccatcggaaagcggaatacgggcggaaagtaaagtcgcaccccagtccatcagcgtgactaccatccctgcgttgttacgcaaagttaacagtcggtacggctgaccatcgggtgccagtgcgggagtttcgttcagcactgtcctgctccttgtgatggtttacaaacgtaaaaagtctctttaatacctgtttttgcttcatattgttcagcgacagcttgctgtacggcaggcaccagctcttccgggatcagcgcgacgatacagccgccaaatccgccgccggtcatgcgtacgccacctttgtcgccaatcacagctttgacgatttctaccagagtgtcaatttgcggcacggtgatttcgaaatcatcgcgcatagaggcatgagactccgccatcaactcgcccatacgtttcaggtcgccttgctccagcgcgctggcagcttcaacggtgcgggcgttttcagtcagtatatgacgcacgcgttttgccacgatcgggtccagttcatgcgcaacagcgttgaactcttcaatggtgacatcacgcagggctggctgctggaagaaacgcgcaccggtttcgcactgttcacgacgggtgttgtattcgctgccaaccagggtacgtttgaagttactgttgatgatgacgacagccacacctttgggcatggaaactgctttggtccccagtgagcggcaatcgatcagcaaggcatgatctttcttgccgagcgcggaaattagctgatccatgatcccgcagttacagcctacaaactggttttctgcttcctgaccgttaagcgcgatttgtgcgccgtccagcggcagatgataaagctgctgcaatacggttccgaccgcgacttccagtgaagcggaagaacttaacccggcaccctgcggcacattgccgctgatcaccatgtccacgccgccgaagctgttgttacgcagttgcagatgtttcaccacgccacgaacgtagttagcccattgatagttttcatgtgcgacaatgggcgcatcgagggaaaactcgtcgagctgattttcataatcggctgccatcacgcgaactttacggtcatcgcgtggtgcacaactgatcacggtttgataatcaatcgcgcagggcagaacgaaaccgtcgttgtagtcggtgtgttcaccaatcaaattcacgcggccaggcgcctgaatggtgtgagtggcagggtagccaaatgcgttggcaaacagagattgtgttttttctttcagactcatttcttacactccggattcgcgaaaatggatatcgctgactgcgcgcaaacgctctgctgcctgttctgcggtcaggtctcgctgggtctctgccagcatttcataaccaaccataaatttacgtacggtggcggagcgcagcagaggcggataaaagtgcgcgtgcagctgccagtgttgattctcttcgccattaaatggcgcgccgtgccagcccatagagtaggggaaggagcactggaagaggttgtcataacgactggtcagctttttcaacgccagcgccagatcgctgcgctgggcgtcggtcaaatcggtgatccgtaaaacgtgggctttgggcagcagtagcgtttcgaacggccaggcagcccagtaaggcacgacggctaaccagtgttcggtttcgacaacggtacggctaccgtctgccagctcgcgctgaacataatccaccagcattggtgatttctgttcggcaaaatattctttttgcaggcggtcttcgcgctcagcttcgttaggcaggaagctatttgcccaaatctgaccgtgcggatgcgggttagagcagcccatcgccgcgcctttgttttcaaaaacctgcacccatgggtacgttttccccagttctgcggtttgctcctgccaggttttgacgatttccgtcaatgctgcaacgctgagctctggcagcgttttactgtgatccggtgaaaagcagatcacccggctggtgccgcgcgcgctctggcaacgcatcagcggatcgtgactttctggcgcatctggcgtgtcagacatcaaagccgcaaagtcattagtgaaaacgtaagtcccggtgtaatcggggtttttatcgcctgtcacccgcacattacctgcgcagaggaagcaatctggatcgtgcgcaggtaacacctgtttggctggcgtttcctgcgccccctgccaggggcgcttagcgcggtgcggtgaaaccagaatccattgcccggtgagcgggttgtagcggcgatgtggatgatcaacgggattaaattgcgtcatggtcgttccttaatcgggatatccctgtggatggcgtgactgccagtgccaggtgtcctgcgccatttcatcgagtgtgcgcgttacgcgccagttcagttcacggtcggctttgctggcgtccgcccagtaggccggaaggtcgccctcgcgacgcggtgcaaaatgataattaaccggtttgccgcaggctttgctgaaggcattaaccacgtccagcacgctgttgcctacgccagcgccgaggttgtagatgtgtacgcctggcttgttcgccagtttttccatcgccacgacgtgaccgtccgccagatccattacgtggatgtaatcgcgtacgccagtaccatcttcggtcggataatcgttaccaaaaatcgccagcgagtcgcgacggcctacagcaacctgggcgatgtatggcatcaggttattcggaatgccttgcggatcttcgcccatatcgcccgacggatgcgcgccaaccgggttgaagtagcgcagcagggcaatgctccagtccggctgggctttttgcagatcggtgaggatctgttccaccatcagcttgcttttgccgtaagggctttgcggtgtgccggtcgggaagctttcaacgtatggaattttgggctgatcgccataaacggtggcggaggagctaaaaataaagtttttgacgttagcggcgcgcatggcgctaatcaggcgcagagtgccgttgacattgttgtcgtaatattccagcggtttttgtaccgattcgcccacggctttcagcccggcgaagtggatcacggtgtcgatagcgtgatcgtgcaggatctcggtcatcaacgcttcgttacgaatatcgccttcaacaaacgttggatgtttgccgcctaaacgctcgataacaggcagtacgctgcgcttactgttacagaggttatcaagaatgatgacatcatgaccgttttgcagtaattgcacacaggtatgacttccaatgtaaccgctaccaccggtaaccagaactctcataattcgctccattaggcttatggtatgaaataaccatagcataacaaagatgcgaaaagtgtgacatggaataaattagtggaatcgtttacacaagaatttagccgttttttatgcgcgattaagtgattataaaacagagggtttatgaatgattgcgctttttatctgaaaaaagacgcggtttcatgcctgcatgcgtcgaaccgttggccggagagggtgctaaggccgcctccggcaaggtcagcactaccgactcaatatatttttgtcagcacatagcgatagagtccaccgtccggcacgaactcaagacgatgggtaatacaggcaggcgcatcttcagcgtggtgcgaaacaaacaacaattgcgtttcaccttcgctaatcagcacatcaacaaaacggcggataagctggcgattcagcggatcaagcccctgtagtggttcatcgagaataagcaacgtcggatgtttcaccagtgcgcggacaatcagcgccagacgctgctgtccccaggaaagactatggaacggagcgtcagccgtgcgtttatcaatgccgagaatatccagccactgctgcaccagtttttgctggcgatccgaaacggcctgataaatgccaatcgaatcaaaatagccagaaagaatcacattacgcacggtagtgctgacccggtaatccagatgcaaactactgctgacgtaaccgatatgctttttgatatcccagatggtttcgccgctgccgcgacgtcgtccgaaaagcgtcaaatcgttgctgtaaccttgcggatgatcgccagtaaccaggcttaataacgtcgattttcctgcaccatttggcccgacaatttgccagtgttcgcctggattcacctgccagctaaggttattaagaatggggcgatcgttataagaaaccacgccattgttcagcacaatgcgcggttcgttggcgggtaaggcgtgacgtgctgaaggttcatccggctccggcagttgcacaccttcaagctgttcactatgcgccagttgcgcgacgagtgcttgttggagcagttcctctttagcgccagtttccgctaacgtgcaatccgccagcacgccagcaaactggacaaactccgggatctcatcgaagcgattgagcaccagtaccagagtaataccggactgatgtaacgaggcgagtcgctcagccagctgctgacgtgaggcaacatccaggccatcgaacggctcatcaagaatcaacaagtcaggctccgacatcagcgcctgacacagcagggtttttcgcgtctcgccagtggaaaggtatttaaagcgtcggtcgaggagggcggtaataccgaactgctgcgccagttgcatgcaacgcggtgcatcctttacttcatcctgaatgatctcagccgtagtgcgtccggtgtcatcttcgccagggccgagcatatcggtgttattccgctgccattcgtcgctgacgagtttttgcaattgctcgaaggagagacgagtgatgtgggaaaactggctttgccgttcacctttcaaaagcggaagttcccccgccagcgcgcgggccagggccgatttcccgcttccattcgaaccgacaaacgcccaactatcacccgcgtttaacgttagctgaggcaattgcagcgtttttgtgtcgctaagacgaaacgtgccttgcaaaatttgcaacgatgacattttatatcccactttgtgcagcgattactgacagggatacgtgtttcataacaaattgtcaacacgcttagcacagcgtggcgataatcacgctgtcggcattaaagtaggccgtgacattctgtccttgctgaagagaagtcgcttcatttaccggcactgtggcgcacagtgtttgcccgtcgggtagcgccattaatacttcgcactgctctgcgccgcgctcaatatgactaataatacccggtaattggttgtcagcgttttgcgcgaccgcctcgtcctgagtaatacctacccacggcgcttttagcaatatcaacacttctttgccttcatccagccccagacgcgcgccgctttgtgcggtaattgcgactttcaggcgtgtttttccgtcagccagtaagacatcaacatgctgttgaacgtcatcatgatcgcgggcggtgatggtaccgaaccactggttacgggcgctggtttgcagtgaaaaacgtgagatcgcggccagcaggctgttcagcggcagggcgtcatcgtcacttaacacatcaaaggctttttgctggatttgcgccagtaagtcatagagctgaatcagtcgctgaccatagcgggtcagtactgcgccgccgccacctttaccgcctgttgcgcgctcgaccagaatatgctcacttaactgattcatctcgttaatggcatcccaggcgcttttatagctaataccggcatctttcgctccctggctaatggaaccggaaagcgcaatgtgttttagtagcgaaatgcggcgcgggtcggcgaataatttttgttggagcttaagggtgagaaggatttcggcctgcataacaatgtcctggcaaaagtcttattgtgacggaaaacgaacgccacgcaaagctgaccgcacaaaaggggagtgcttttctgtgcttagcggttagaatagtctcatgactatatctggagttgaccatgttagagttattaaaaagtctggtattcgccgtaatcatggtacctgtcgtgatggccatcatcctgggtctgatttacggtcttggtgaagtattcaacatcttttctggtgttggtaaaaaagaccagcccggacaaaatcattgattccctgaatgcccgcttagtcgggcattttctttttctcaacttcctgcttttcctgccgatattttttcttatctacctcacaaaggttagcaataactgctgggaaaattccgagttagtcgttatattgtcgcctacataacgttacattaaggggttaccaatggctcgtaaatggttgaacttgtttgccggggcggcactctctttcgctgttgctggcaatgcactggcagatgaagggaaaatcacggtgttcgccgccgcatcactgactaacgcaatgcaggacattgctacgcagtttaaaaaagagaaaggcgtggatgtggtttcttctttcgcttcgtcatctactctcgcccgtcagattgaagcgggtgcgcctgcggatctgtttatttctgccgatcagaaatggatggattatgcggttgataaaaaagcgatcgatacagctacgcgtcagacactgctcggcaatagcctggtcgttgtagcaccgaaagccagcgtgcagaaagatttcaccatcgacagcaaaaccaactggacttcactgctgaatggcggtcgcctggcggttggcgatccggaacatgttcccgctggcatttatgcaaaagaagcactgcaaaaactgggcgcatgggatacgctctctccgaaactggccccagcggaagatgttcgtggggcgctggcgctggtcgaacgtaacgaagcgcctctgggcattgtctacggttctgacgcagttgccagcaaaggggtaaaagtggttgccaccttcccggaagattcacataaaaaagtggaatatccggttgctgttgtggaagggcataacaatgcgacagtgaaagcattttatgattatctgaagggaccgcaggcagcggaaatctttaaacgttacggatttacaatcaagtaatgatactgaccgatccagaatggcaggcagttttattaagcctgaaagtttcttccctggctgtgctgtttagcctgccgtttgggatcttttttgcctggttactggtgcgttgcacgtttccgggcaaagctctgctcgacagcgtactgcatctaccgctggtgttaccgcccgtggtcgtcggttacttattattagtttcgatgggacggcgcggatttatcggtgaacgtctgtatgactggtttggtattaccttcgcctttagctggcgcggcgcggttctcgctgccgccgtcatgtcgtttccgctgatggtgcgggcaattcgtctggcgctggaaggggttgatgtcaaactggaacaggccgcaagaacactgggggccgggcgctggcgcgttttctttactatcacgttaccgctgaccttaccgggaattattgttggtacggtactggcttttgctcgttctctcggtgagtttggtgcaaccatcacctttgtgtcgaacattcctggtgaaacgcgaaccattccttctgccatgtataccctgatccagacccccggcggggaaagtggagcggcgagactgtgcattatttctattgcgctggcgatgatctccctgttgatttcagaatggctggccagaatcagccgtgaacgggcggggcgctaatcatgctggaactgaatttttcccagacgttgggcaaccattgcctgactattaatgaaacgctgcccgccaatggcatcactgctatctttggcgtctccggtgccggaaaaacttcgctgattaacgccatcagtggactgacgcgcccgcaaaaagggcggattgtcctcaatgggcgggtactaaatgatgccgaaaaaggtatctgcctgacgccggaaaagcgtcgcgttggctatgtttttcaggatgcgcggctgttcccgcattacaaagtgcgtggcaatctgcgctacggcatgtcgaaaagtatggtcgatcagttcgataagctggtggcgcttttaggcattgaaccgttgcttgaccgtttaccaggcagcctgtccggaggcgaaaaacagcgcgtggcgattggtcgggctttgctgacagcaccggaattgctgttgctggatgaaccgctggcgtcactggatattccgcgtaaacgcgaactgttgccttatctgcaacggctgacacgggaaatcaacattccgatgttgtatgtcagccattcgctggatgagatcctccatctggcagacagagtgatggtactggaaaacggtcaggtgaaagcctttggcgcgctggaggaagtgtggggcagtagcgtgatgaatccgtggctgccgaaagagcaacaaagtagcattctgaaagtgacggtgcttgagcatcatccgcattacgcgatgaccgcgctggcgctgggcgatcagcatttgtgggtcaataagctggacgaaccgctgcaagctgcgctacgtatccgcattcaggcttccgatgtttctctggttttacaaccgccgcagcaaaccagcattcgtaacgtattgcgggcaaaagttgttaatagttatgacgacaacggccaggtggaagtggaactggaagtcggcggtaaaacgctgtgggcgcgtatcagcccgtgggccagggatgaactggcgatcaaacctggcctgtggctgtacgcgcaaattaaaagtgtgtcgataaccgcctgattaaatcaggtggctataaatgaactgggcaatgctgtcggtggtgttatcaccaatcacaatgttggcgcgcgcttttaccgcgtcatcggcgttgcccatcgccacgcctgtaccagcggcttccagcatactgatatcattaaagttatcgccgaatgccacgacgttttccatcgaccaaccttgcgcctcaacccatttcgtcaaacgtttacctttgctgttgccgccgcgtgcaatatcaacctgatcgtgccaggaccattcacactccagtcccagttcatgttcgacatgcttaccaaaatgctgcaattgcggcaggtcatcgtgcgtcagggcgaacttccatacggcgttaacttgttgcgccgtttcagccagagaagcgacttgtgtgaaagtcggacgctgttccggcggcagggtttgcgcccagttagatgtgcgaatgacatgcccggtcgggtgctcatagaccattgcatcatcgacatacatcagaccgtgaatgtggtgttcattcagcatctcaatgagttgcagggctttaataacgggcattgggtccgcttccagcacggtttttgcatgataatcatacaaataggtgccattacagcaaatagcaggtgtatccagcgccagcgcctgataaaaaggatgaatagcgacgtgatggcgacctgtgacgatgattaattgatagcctgcttcgcgagcgcgggccagggcttctatcgatgaaggaagcagggtctttttcggggtcaataaggtgccgtctaagtcgagagcaatcacgcgtgtggtcatggcgtattccagattaaggttaagaattttcgtctgcgcgaatggtacaccgataccactatcggacaaaattctgcgttttaattcagcattcaccgccaaaagcgactaattttagctgttacagtcagttgctaaatgcaaaggagcattcatgaagcaaacagtttatatcgccagccctgagagccagcaaattcacgtctggaatctgaatcatgaaggcgcactgacgctgacacaggttgtcgatgtgccggggcaggtgcagccgatggtggtcagcccggacaaacgttatctctatgttggtgttcgccctgagtttcgcgtcctggcgtatcgtatcgccccggacgatggcgcactgacctttgccgcagagtctgcgctgccgggtagtccgacgcatatttccaccgatcaccaggggcagtttgtctttgtaggttcttacaatgcgggtaacgtgagcgtaacgcgtctggaagatggcctgccagtgggcgtcgtcgatgtggtcgaggggctggacggttgccattccgccaatatctcaccggacaaccgtacgctgtgggttccggcattaaagcaggatcgcatttgcctgtttacggtcagcgatgatggtcatctcgtggcgcaggaccctgcggaagtgaccaccgttgaaggggccggcccgcgtcatatggtattccatccaaacgaacaatatgcgtattgcgtcaatgagttaaacagctcagtggatgtctgggaactgaaagatccgcacggtaatatcgaatgtgtccagacgctggatatgatgccggaaaacttctccgacacccgttgggcggctgatattcatatcaccccggatggtcgccatttatacgcctgcgaccgtaccgccagcctgattaccgttttcagcgtttcggaagatggcagcgtgttgagtaaagaaggcttccagccaacggaaacccagccgcgcggcttcaatgttgatcacagcggcaagtatctgattgccgccgggcaaaaatctcaccacatctcggtatacgaaattgttggcgagcaggggctactgcatgaaaaaggccgctatgcggtcgggcagggaccaatgtgggtggtggttaacgcacactaaccgctgatttacccggcgcagtctctcctgcgccggtgtattaacctatctcctgtaacgcgtgtctctggcgttcgacgatattggtccacaaattgtctttatcgtcagtccataaattaatcagcaaggcaaaaaagcgttctgctgctggagaaagtacggcatctttacggcgaattattcccaatgttcgacgtataacgggttccaccaatgggataccaataatcgaagaatagggcgcatgaggcattgccaggccaggaagcgccgaaatccccagtcccgcctccaccagtcctaatgacgtcgaaagatgacgcacttcgtaaaaccagtccagcttccagggcttgtcggccagctgttgttctatcaacagtcggttgccgctggaggagcgtacgccaatcattttgtaacccactaactcctgccattctacaagctgctttttggccaatggatggtcacgccgacaggccagcacgaacggctcgttgaccagtggggtaaaatcaatggatgaatttgtgacgttgttcatgtttatgccaaagtctgattcgttacacagcaccgattccatgcaattattcgtgccttgttccagaatccgcactttaatattgggatacagctcattaaatttaccgattgccagcggtaaaaaataaaatactgcggtcggaatacacgctaacgtcaccataccacgatgataagcattcatatcacgaatattaaaaagcgtttcatcgaatttctttattaattcccgcgcctccgggagcaacctttttcctgcttttgttaacgtaaccttgcgagttgtacgctcaaatagttgaacatgtaaatcttcctccatcttttttattcttcgcgttaatgcaggttgcgtaatattgagtaatttagcggcattgttaaacgaactggactctgccagtatgacaaatgccttcatacttgataattcatgcttcattattactccggaaaatggaagcgacgattttgggtggctggccgttaaaaattttaactgcatttagccaacttaaattaatgaaaaaatgttattaatcgttgagctaaagtcattagagatgctttgcccttaatgtaaccatatcgcaataagttatgtttttaaattgagggcattattatgaaaaaaataccctgcgtgatgatgcgaggtggaacctcgaggggcgcgttcctgttagcggaacatttacccgaagatcaaacgcagcgcgataaaatattgatggcaattatgggttccggtaacgatctggaaattgacggtattggcggcggtaatccactgaccagtaaagtcgccattattagccgttccagcgatccgcgtgctgatgtcgattatctgtttgcgcaggtaatcgttcatgagcaacgtgtcgataccacgcctaactgcggcaatatgctgtctggtgttggggcattcgccattgaaaatggtttgattgcagcgacttcgccagttactcgcgtacgtatccgcaacgtcaatacgggtacgttcatcgaagctgatgtgcaaacgccaaatggtgttgtcgagtacgagggtagcgccagaattgacggcgtaccgggtactgccgcaccggttgcgctcactttcctgaatgccgctggaaccaaaaccggaaaagttttcccgactgataatcagattgattattttgacgatgtcccggtgacctgtatcgatatggcgatgccagtcgtcattattccggctgaatatctgggaaaaacaggttatgaattaccggcggaactggatgccgacaaagcattattagcccgcattgaatctatccgtctacaagcgggtaaagcaatgggcttaggtgatgtcagtaatatggttatccctaaacctgtgcttatttctccagcgcagaaaggcggggcaattaatgtgcgttattttatgccgcattcttgccatcgcgcgctggcgataaccggtgctattgctatttccagtagttgtgcattggaaggcaccgtcacccgacaaatcgtcccttctgtaggatacggcaatatcaatattgaacaccccagtggtgcgctcgacgttcatttaagtaatgaaggtcaggatgccacgacgttacgcgcatctgttattcggacgaccagaaaaatattttccggtgaagtttatcttccctgaaaaaattcgttgtcaggataaggacaatcaataaaggacttctgtatgagtcatacagaaagaacaggattttaaatgaataagaaatcgttatggaagctaattctgatattagcgatcccatgtattattggttttatgccagctccggcaggattaagcgaactggcgtgggtgctttttggtatttacctggcggccattgtggggctggttatcaagcctttcccggaacctgtcgtactgttaattgccgttgctgcctcaatggtggtggtcggtaacttatccgacggtgcgtttaaaaccaccgccgtattaagcggttactcttcaggtaccacctggctggtgttctcggcgtttaccttaagcgccgcatttgtgaccaccggtttaggtaaacgtattgcctatctgctgattggtaaaatcggtaacaccacgctgggtctgggttacgttacggtattcctcgatctggtactggctccggcaacaccgtctaacaccgcgcgtgcgggcggcattgtgttaccgatcatcaacagcgtggcggtggctttggggtccgaaccggaaaaaagtccgcgtcgtgtcggacattacctgatgatgtccatttacatggtcaccaaaaccaccagctatatgttctttaccgcaatggcggggaacattctggcgctgaaaatgatcaacgacattctgcacctgcaaattagctggggtggatgggcgctggcagccggattgccgggcatcattatgctgctggtcaccccgctggtgatttacaccatgtatccaccagaaattaagaaggtggataacaaaaccatcgctaaagcgggccttgccgaactaggaccgatgaaaatccgcgaaaaaatgctgctcggtgtctttgtgctggcgctgctgggctggattttcagtaagtctctgggggttgatgaatccaccgtggcaatcgttgttatggcaaccatgctgctgctgggtatcgttacctgggaagacgtggttaaaaataaaggcggctggaataccttaatctggtacggcggtattatcggcttaagctccttattatcgaaagttaaattcttcgaatggttagctgaagtctttaaaaataacctggcatttgatggtcacggtaacgttgctttcttcgttattattttcctcagcattatcgtgcgttatttcttcgcttccggtagtgcctatatcgttgctatgttaccggtatttgccatgctggcgaacgtctccggcgcaccgttaatgttaaccgcgctggcactgttgttctccaactcctatggcggcatggttactcactatggcggcgcggcaggtccggtcatctttggcgtgggttataacgatattaaatcctggtggttggtcggtgcggtactgacgatattaaccttcctggtgcatatcaccctcggcgtgtggtggtggaatatgctgatcggctggaacatgctgtaaatattctcgtcatacttcaagttgcatgtgctgcgtctgcgttcgctcaccccagtcacttacttatgtaagctcctggggattcactcgcttgtcgccttcctgcaactcgaattatttagagtatatccatttattatctttctgcgcacttcacggtgcgcagatatctggagcatttgatgatcaagttatctgaaaaaggcgtgtttctcgccagtaataacgaaataattgccgaagaacatttcaccggcgaaattaaaaaagaagaagccaaaaaaggcactattgcctggtctattctctcttcgcataatacgtccggaaatatggataaacttaaaattaagtttgattcattagcctctcacgatattacctttgttggtattgtacagaccgctaaagcgtccggtatggaacgtttcccgctgccgtatgtgctgaccaactgccataactcactctgcgccgtcggcggcactattaacggtgatgaccatgtttttggtttatcggcggcccagcgttatggcggtatttttgtgcctccgcatattgcggtcatccatcaatatatgcgtgagatgatggcaggcggcggcaaaatgatcctcgggtcagacagccacacccgttacggtgcattagggacaatggcagtcggtgagggcggcggtgagttggtaaaacagctgcttaatgacacctgggatatcgactatccgggcgtggttgcggtgcatctgaccggaaaacctgcgccgtatgtggggccacaggatgtggcgctggctatcattggcgcggtgttcaaaaacggttacgtcaaaaacaaagtcatggagttcgttggaccgggcgttagcgcgctctctaccgatttccgtaacagcgttgacgtgatgaccactgaaacgacctgtttaagttctgtctggcaaaccgatgaagaagtccataactggctggcgctgcacggtcgcggccaggattactgccagcttaaccctcaaccgatggcgtactacgatggctgcatcagcgttgatttaagcgccatcaaaccaatgattgcgctgccgttccacccgagcaacgtgtatgaaatcgacacactgaaccagaacctgaccgacattctgcgtgagattgaaattgagtccgaacgcgtggcgcacggtaaagccaaactctcgctgctggataaagtggaaaatggtcgcctgaaagtgcagcaggggattatcgcgggctgttctggcggtaactacgaaaacgtcatcgcggcggcgaatgcactgcgcggtcaatcctgtggcaatgacaccttctcgctggcagtttacccgtcatcacagccggtgtttatggatctcgccaaaaaaggtgtggtagcagatttgattggcgcaggcgcaatcatcagaaccgcgttctgcggcccatgctttggcgcgggcgatacgccaatcaacaacggtttgagtattcgccacaccacgcgtaacttcccgaaccgcgaaggctctaagccagctaatgggcagatgtcagcggtggcgttgatggacgctcgttctatcgctgcgactgcggcaaacggtggctatttaacctctgccagcgaacttgattgctgggacaacgtgccggagtacgccttcgatgtaacgccgtataaaaaccgtgtttatcagggctttgtgaaaggggcaactcagcaaccgctgatttacgggccgaacattaaagactggccggaattgggtgcgctgactgacaatatcgtcctgaaagtgtgctcgaagatcctcgacgaagtgaccaccaccgacgaactgattccttccggtgaaacctcttcttatcgttcaaatccgattggtctggcggagtttaccctgtctcgccgcgatcccggttatgttagcagaagtaaagcgactgctgagctggaaaatcagcgtctggcggggaatgtcagcgagctgacagaggtgtttgcgcgcattaagcagattgctggtcaggagcatattgatccgctgcaaactgaaattggcagcatggtctatgcggtgaaaccaggcgatggttctgcgcgtgaacaggcggcgagctgccagcgtgtgattggcggtctggcgaatattgccgaggagtacgcgactaaacgctatcgttctaacgtcatcaactgggggatgttaccgctgcaaatggcggaagtaccaacctttgaagtgggggattacatttacatccctggcattaaagcggcgctggataatccgggtacgacgtttaaaggttatgtgatccatgaagatgcgccggtaacggaaattacgctctatatggaaagtctgactgctgaagagcgcgagattatcaaggcgggtagtttgattaacttcaataaaaaccgtcagatgtaaaaagcgccatgtgaatgtaggtcgcattcggcacttattgtcggatgcgatgcttgcgcatcttatccgacctacgaatcgcatcgaatctgtaggccagataaggcattttcgcagcatccggcacttattgtcggatgcgatgcttgcgcatcttatccgacctacaaatcgcatcgaaccgtaggccggataaggcgtttacgccgcatccggcaaatagttaattgctcttacttcttcgcctctgcaaccactttactacccacgccgcggttattgtattcccacatgcggttgtagttagtgtcattcagattgcgctgtatttcgtcgttatcatctacgctgccggtattacccgcaaacggacgattagagatcaccgcatcggcccacggtttagccgtgttaaaaccttcgttgatggcgctatcacggatcaccacctgaccgttggtattggcatcaacatccagcgagcggcccagttgcgccacaccatcaccgaaagcattgaaacggctgtttacggcgaggaaaccgtagtaaatgttggacagcgtagccggtgcaaacacatacgcttcttgctgagtacgtgagttcaccacgcggaattcggtgttatcgaacaccactgcgccgcgaccagaaacgatatccacatccccttcaatgtagctgttggtcaccagcgtacgcggctgacgattcgtttccagacggttctgcacaccgctgttggtgacaaagaaggtgttctgacgaccgagaatgttaacgttgttaatctgtacctggtcaccatcagtacgcagtgccaccgccggatggttacctgcatctacgctatcgcccagcgtgttttcgatggtcagattttgcagttgcaggccattgttttgtgaccagaagaccgcagagcagagaacaccgatactgtcgctgcgtttgctctggcagctatcgtacatataccacgctggtttacctggcatatatttgccgcgcgggttgacgtcgtgacgccagtcggcagggctcatgccaccatcaagggaaagcccaatcttcacatcaatcggtttttcacctgtaccgtacagagtaattccacccggagcggcagggacatataccgttccctgatactcaccaggcatcacggcaatatactggcgcttgttggtacgcttgataattgccgcatctaccgccgcctgaatcgtggtatgcgttacaccttgagtgcccgccgggccgacaacaaagtcaggttgcgcaggcagggtaatcggggaaggattccacgctgcagcacctggtgtcagggatgcaaaatagtgttgagcatcgaaattctgcgcttcttttgccgacagaatcgggcgagaagaggtaccaggcgcggtttgatcagaaggacgttgatcgggcggggttgagctacaggcggtcagcgtcacgccaaaagccaatgccagcgccagacgggaaactgaaaatgtgttcacaggttgctccgggctatgaaatagaaaaatgaatccgttgaagcctgcttttttatactaacttgagcgaaacgggaaggtaaaaagacaaaaagttgtttttaatacctttaagtgataccagatggcattgcgccatctggcagagtgattaactaaacatcgcagtaatcgaggcgcttgccagagagtggaaatgaacgttaaacccgaccatcgcgccgctggcaccttcatcgacatcaatacgttctatatccagcgcgtgaacggtaaaaatgtagcgatgagtttcgcctttcggcggtgctgcgccatcgtacccggttttaccaaagtcggtacgcgtctgcaaaacgccgtctggcattgctaccagaccagagccaaacccttgcggtaatacgcgggtatcagcgggtaagttaacaactacccagtgccaccagccggagccggttggcgcatccgggtcgtagcaggtgacaacaaaacttttcgttcccgcaggaacatcatcccacgccagatgcggtgaaatattatcgccatcgtaacccatgccgttaaagacatgacgatgcggcaatttatcgccatcgcgcagatcgttactgatgagtttcatgaaccctcctttcttgtttgcagaaagtgtagccagaaaccctcacgcggacttctcgttattggcaaaaaaatgtttcatcctgtaccgcgcggttaaccgctgcggtcagacgctgcaactgttgcgggagaataatatagggcggcatcaggtaaatcagtttgccaaaaggccggatccagacaccctgttcgacaaagaatttttgcagcgccgccatattcaccggatgagtggtttcgaccacgccaatggcccccagtacgcgcacatcggcaaccatttcggcatcacgggcgggggcaagttgctcgcgcagctgtacttcaatatccgccacctgttgctgccagtcgccagattcgagaatcgccaggctggcgtttgctgccgcgcaggccagcggattgcccataaaagttggcccatgcataaagcaaccggcttcaccgttactgatggtttctgcaacctcgcgcgtggtgagtgtggcggaaagggtcattgtgccgccggttaaggctttaccgaggcacaaaatgtccggcgcgatttctgcatgttcacaggcaaacagtttcccggtacgaccaaatccagtggcgatctcgtcggcaatcagcaagataccttcgcgatcgcatattttgcggattcgttttaaccattccggatggtacatgcgcatcccgcctgcgccctggacaatcggctcaatgatcaccgccgcgatttcatgacgatgcgccgccatcaggcgggcaaagcccaccatatcgcgctcatcccattcgccatccatgcggctttgcggggcgggagcaaacaggttttctggcaggtagcctttccacagactgtgcattgagttatccggatcgcacaccgacatcgcgccaaaggtatcgccatgataaccattgcggaaggtcagaaaacgctggcgcgcttcgcctttggcttgccagtactgcaacgccattttcatcgccacttccaccgctacggaaccggagtccgcgagaaaaacgcactccagcggttgcggcgtcatcgccaccagtttgcggcacagctcaatggctggcgcatgggtgataccgccaaacatcacatgcgacatggcatcaatttgcgacttcatcgccgcattaagctgcgggtgattgtagccgtggatcgccgcccaccaggacgacataccgtcaaccaggcgtctgccgtcagacaaaatcagctcgcaaccttcggcgctcaccaccggataaaccggcagaggggaggtcatggatgtgtatgggtgccagatatggcgttggtcaaaggcaagatcgtccgttgtcataatcgacttgtaaaccaaattgaaaagatttaggtttacaagtctacaccgaattaacaacaaaaaacacgttttggagaagccccatggctcaccgcccacgctggacattgtcgcaagtcacagaattatttgaaaaaccgttgctggatctgctgtttgaagcgcagcaggtgcatcgccagcatttcgatcctcgtcaggtgcaggtcagcacgttgctgtcgattaagaccggagcttgtccggaagattgcaaatactgcccgcaaagctcgcgctacaaaaccgggctggaagccgagcggttgatggaagttgaacaggtgctggagtcggcgcgcaaagcgaaagcggcaggatcgacgcgcttctgtatgggcgcggcgtggaagaatccccacgaacgcgatatgccgtacctggaacaaatggtgcagggggtaaaagcgatggggctggaggcgtgtatgacgctgggcacgttgagtgaatctcaggcgcagcgcctcgcgaacgccgggctggattactacaaccacaacctggacacctcgccggagttttacggcaatatcatcaccacacgcacttatcaggaacgcctcgatacgctggaaaaagtgcgcgatgccgggatcaaagtctgttctggcggcattgtgggcttaggcgaaacggtaaaagatcgcgccggattattgctgcaactggcaaacctgccgacgccgccggaaagcgtgccaatcaacatgctggtgaaggtgaaaggcacgccgcttgccgataacgatgatgtcgatgcctttgattttattcgcaccattgcggtcgcgcggatcatgatgccaacctcttacgtgcgcctttctgccggacgcgagcagatgaacgaacagactcaggcgatgtgctttatggcaggcgcaaactcgattttctacggttgcaaactgctgaccacgccgaatccggaagaagataaagacctgcaactgttccgcaaactggggctaaatccgcagcaaactgccgtgctggcaggggataacgaacaacagcaacgtcttgaacaggcgctgatgaccccggacaccgacgaatattacaacgcggcagcattatgagctggcaggagaaaatcaacgcggcgctcgatgcgcggcgtgctgccgatgccctgcgtcgccgttatccggtggcgcaaggagccggacgctggctggtggcggatgatcgccagtatctgaacttttccagtaacgattatttaggtttaagccatcatccgcaaattatccgtgcctggcagcagggggcggagcaatttggcatcggtagcggcggctccggtcacgtcagcggttatagcgtggtgcatcaggcactggaagaagagctggccgagtggcttggctattcgcgggcactgctgtttatctctggtttcgccgctaatcaggcagttattgccgcgatgatggcgaaagaggaccgtattgctgccgaccggcttagccatgcctcattgctggaagctgccagtttaagcccgtcgcagcttcgccgttttgctcataacgatgtcactcatttggcgcgattgcttgcttccccctgtccggggcagcaaatggtggtgacagaaggcgtgttcagcatggacggcgatagtgcgccactggcggaaatccagcaggtaacgcaacagcacaatggctggttgatggtcgatgatgcccacggcacgggcgttatcggggagcaggggcgcggcagctgctggctgcaaaaggtaaaaccagaattgctggtagtgacttttggcaaaggatttggcgtcagcggggcagcggtgctttgctccagtacggtggcggattatctgctgcaattcgcccgccaccttatctacagcaccagtatgccgcccgctcaggcgcaggcattacgtgcgtcgctggcggtcattcgcagtgatgagggtgatgcacggcgcgaaaaactggcggcactcattacgcgttttcgtgccggagtacaggatttgccgtttacgcttgctgattcatgcagcgccatccagccattgattgtcggtgataacagccgtgcgttacaactggcagaaaaactgcgtcagcaaggctgctgggtcacggcgattcgcccgccaaccgtacccgctggtactgcgcgactgcgcttaacgctaaccgctgcgcatgaaatgcaggatatcgaccgtctgctggaggtgctgcatggcaacggttaataaacaagccattgcagcggcatttggtcgggcagccgcacactatgagcaacatgcagatctacagcgccagagtgctgacgccttactggcaatgcttccacagcgtaaatacacccacgtactggacgcgggttgtggacctggctggatgagccgccactggcgggaacgtcacgcgcaggtgacggccttagatctctcgccgccaatgcttgttcaggcacgccagaaggatgccgcagaccattatctggcgggagatatcgaatccctgccgttagcgactgcgacgttcgatcttgcatggagcaatctcgcagtgcagtggtgcggtaatttatccacggcactccgcgagctgtatcgggtggtgcgccccaaaggcgtggtcgcgtttaccacgctggtgcagggatcgttacccgaactgcatcaggcgtggcaggcggtggacgagcgtccgcatgctaatcgctttttaccgccagatgaaatcgaacagtcgctgaacggcgtgcattatcaacatcatattcagcccatcacgctgtggtttgatgatgcgctcagtgccatgcgttcgctgaaaggcatcggtgccacgcatcttcatgaagggcgcgacccgcgaatattaacgcgttcgcagttgcagcgattgcaactggcctggccgcaacagcaggggcgatatcctctgacgtatcatctttttttgggagtgattgctcgtgagtaaacgttattttgtcaccggaacggataccgaagtggggaaaactgtcgccagttgtgcacttttacaagccgcaaaggcagcaggctaccggacggcaggttataaaccggtcgcctctggcagcgaaaagaccccggaaggtttacgcaatagcgacgcgctggcgttacagcgcaacagcagcctgcagctggattacgcaacagtaaatccttacaccttcgcagaacccacttcgccgcacatcatcagcgcgcaagagggcagaccgatagaatcattggtaatgagcgccggattacgcgcgcttgaacaacaggctgactgggtgttagtggaaggtgctggcggctggtttacgccgctttctgacactttcacttttgcagattgggtaacacaggaacaactgccggtgatactggtagttggtgtgaaactcggctgtattaatcacgcgatgttgactgcacaggtaatacaacacgccggactgactctggcgggttgggtggcgaacgatgttacgcctccgggaaaacgtcacgctgaatatatgaccacgctcacccgcatgattcccgcgccgctgctgggagagatcccctggcttgcagaaaatccagaaaatgcggcaaccggaaagtacataaaccttgccttgttgtagccattctgtatttggttaaattgcgagcgagatcgcgtcttcgattgactgcaatttaaccaattaaattctaaaataatcacgaaaaaaattttacttccgcctcatgcggcgaatgtgggaattgcccaggcggcgggggataggggctggagacagttatccactattcctgtggataaccatgtgtattagagttagaaaacacgaggcaagcgagagaatacgcggcttgcacgcgaattggcgttaaagacggctcaaagaaatatcttttattttttaactggttagataaatgcaatggcagtcactgaacaggcatctcttgccataaaactgtcatcactcatcttgacaaatgttaaaaaagccgttgctttggggataacccggtaaggccggagttttatctcgccacagagtaaattttgctcatgattgacagcggagtttacgctgtatcagaaatattatggtgatgaactgtttttttatccagtataatttgttggcataattaagtacgacgagtaaaattacatacctgcccgcccaactccttcaggtagcgactcatgagtaaaccgttcaaactgaattccgcttttaaaccttctggcgatcagccagaggcgattcgacgtctcgaagaggggctggaagatggcctggcgcaccagacgttacttggcgtgactggctcagggaaaaccttcaccattgccaatgtcattgctgaccttcagcgcccaaccatggtacttgcgcccaacaaaacgctggcggcccagctgtatggcgaaatgaaagagttcttcccggaaaacgcggtggaatatttcgtttcctactacgactactatcagccggaagcctatgtaccgagttccgacactttcattgagaaagatgcctcggttaacgaacatattgagcagatgcgtttgtccgccaccaaagcgatgctggagcggcgtgatgtggttgtggtggcgtctgtttccgcgatttatggtctgggcgatcctgatttatatctcaagatgatgctccatctcacggtcggtatgattatcgatcagcgcgcgattctgcgccgactggcggagctgcaatacgctcgtaatgatcaagcattccagcgtggtactttccgcgttcgtggcgaggtgatagatatcttcccggcagaatcggatgacattgcacttcgcgtggaactgtttgacgaggaagtggaacgattgtcgttatttgacccgctgaccgggcagattgtttccactattccacgttttaccatctacccgaaaacgcactacgtcacaccgcgcgagcgcatcgtacaggcgatggaggagatcaaagaagagctggccgccagacgcaaagtgctgttggaaaacaacaaactgctggaagagcagcggctgacccagcgtacccagtttgatctggagatgatgaacgagctgggctactgttcggggattgaaaactactcgcgcttcctctccggtcgtggaccgggtgagccaccgccgacgctgtttgattacctgcctgccgatgggctgctggtcgtcgatgaatctcacgtcaccattccacaaattggcggcatgtatcgcggtgaccgggcgcgtaaagagacactggtggagtacggcttccgcctgccatcagcgctggataaccgtccgcttaagtttgaagagttcgaagcattagcgccgcaaaccatctatgtttcggcgacgccgggtaattacgagctggaaaaatccggcggcgatgtggtggatcaggtggtgcgtccaaccggattgcttgacccgattatcgaagtgcggccggtggcgacacaggttgatgatcttctttcggagattcgtcagcgagcggcaattaacgaacgcgtactggtcaccacactgaccaagcggatggcggaagatcttaccgaatatctcgaagaacatggcgagcgcgtgcgttatcttcactcagatatcgacaccgtcgaacgtatggagattatccgcgacttgcgtctgggtgagttcgacgtgctggtagggatcaacttactgcgcgaaggtctggatatgccggaagtgtcgctggtggcgatcctcgacgctgacaaagaaggcttcctgcgttccgaacgttcgttgatccagaccattggtcgtgcggcacgtaacgttaacggtaaagcgattctctacggcgataagatcaccccatcaatggcgaaagcgattggcgaaaccgaacgtcgccgtgagaaacagcagaagtacaacgaggaacacggaattacgccgcaaggcttgaacaagaaagtggtcgatatcctggcgctggggcagaacattgccaaaaccaaagcgaagggcagaggaaaatcgcgcccgattgttgagccggataatgtgccgatggatatgtcgcctaaagcgttgcagcagaaaatccatgagctggaagggttgatgatgcaacacgcgcagaatctggagttcgaagaagcggcgcaaattcgtgaccagttgcatcagctgcgtgagctgtttatcgcggcatcgtaacaggatagcgaagaagactgatgacaaacggaaaacagcctgatgcgctacgcttatcaggcctacattttctccgcaatatattgaatttgcgcggtttgtaggccggataaggcgttcacgccgcatccggcataaacaacgcgcactttgtcttcaataggaagccggaattttccttcggatttccgttaacctaaagcctgtaacgccttttccagcgcgttatgtaacaactggcggtcatgacgatacggaatatcgctggcctccagtacctcctggatcacaatccgctctttcaccgccgagacatccacttttggcccgacgatgaccgcatcaatgacctttttaccaacatactgctccataattgccagcttgctttccagcttcaaattagccgcaggtaaactcaactcacgccccagattgccgatataaaccatcggcgctggcgtgcggcgtaatgcctgggcgatttccttcagcagcagaattggcatcaggctggtataaaaactgccaggcccaataatgatgagatccgcttcattgatagcgtgaaccgcctcacgcgttgcgggtacattaggcgttaacaataactcttgaatcggcgtagttaactggtcgatattgacctcgccgtaaacttcatgcccctgatcgtcaatcgccatcagatcaacaggatgctctgacattggaatcaaatgcgtatccactttcagcagattacgaattaaattgatggcttccagaggccgcacgctaaggtgatccagcgcctttaacatcaagtttccgagattatgaccggaaagttcgccattgccaccaaaacggtattcaaacatcgcggaggcgacgctcggttccgttatcagctggttgaggcagttgcgcatatcgccccaggcaatgccgccttctgaacggcgaatacgccccgtcgagccaccattatcggtggtggtgacgatacccgttaaacgagaacccaaagacgaaagtgatgagagaacgcgtcccagtccatgccctccgccgagagcaacgacacgatcaagatcagccagcgtacgattgcgcatatagtttcctggagtcagattatccgcgctacagtagcgcaaattgcggggaaacagcaattaacctgccaatattgaggatacaaactattttcttctacctctaaaggacgatgcacgctatgcctccctgatgatgtatatcaaagtaaaaccgccattttcccttattctgtagcgaaatagcacgatcatgacgctatatacatgattacatagcgaaagtgtggatggtaaaaatctcatttacacgctagtatcggcataaccactaaacactctagcctctgcacctgggtcaactgatacggtgctttggccgtgacaatgctcgtaaagattgccaccagggcgaaggaagaaatgacttcgcctcccgtatctggaaaggtgtacatggcttcacaactgactgatgcatttgcgcgtaagttttactacttgcgcctgtcgattaccgatgtgtgtaactttcgttgcacctactgcctgccggatggctacaaaccgagcggcgtcaccaataaaggctttcttaccgtcgatgaaattcgccgggttacgcgcgccttcgccagactgggcaccgaaaaagtgcgcctgacaggaggagagccgtctttacgccgcgactttaccgatatcatcgccgctgtgcgggaaaacgacgctatccgccagattgcggtcacaaccaatggttaccgtctggaacgcgatgtggcgagctggcgcgatgcgggacttactggcattaacgtcagtgtcgacagtctggacgcccgccagtttcacgctattaccgggcaggataaattcaaccaggtcatggcagggattgatgctgcatttgaggccggttttgagaaggtcaaagtcaataccgtgctgatgcgtgatgttaatcatcaccagctcgacacctttctgaactggatccagcatcgccctatccagctgcgtttcatcgaactgatggaaacgggcgagggcagcgagctcttccgtaagcatcacatctctggtcaggttctgcgtgacgagctactgcgtcgcggctggatccaccaattacgtcaacgcagcgacggtcccgcgcaagtcttttgccatccagattacgccggagagattggccttatcatgccgtatgaaaaagacttctgcgccacttgcaaccgcctgcgcgtttcctccattggtaaactccatctctgcctgtttggtgaaggcggcgttaacctgcgcgatctgctggaagacgatacccagcaacaggcgctggaagcgcgtatttcagcggcgctgcgggagaagaaacagacccatttcctgcatcaaaacaacaccggtattacgcaaaacttatcgtacattggcggctaaaacgtcaaaaggagagatcagatgagtcaggtaagcactgaatttatcccgacccgtattgctattcttacggtttctaatcgtcgcggtgaagaagacgatacctccggtcactatctgcgcgattcggcgcaagaagcgggccatcacgttgtcgataaagccattgtgaaagaaaaccgctacgctattcgcgctcaggtatctgcgtggatcgccagcgacgatgtacaagtggtattgattacgggtggtactggcctgacggaaggtgatcaggctcccgaagcattgctgccgttgttcgaccgtgaagttgaaggttttggtgaagtgttccggatgttgtcgtttgaagagattggcacttccacgttgcaatctcgtgcggtagcgggcgtcgccaacaaaacgctgattttcgccatgccgggttcgaccaaagcgtgccgtaccgcatgggaaaatatcatcgcgccgcagctggatgcccgtacgcgtccgtgtaatttccatccacatttgaagaaataagtatgtcgcaactgacccatatcaacgccgctggcgaagcgcacatggtggatgtctccgccaaagcggaaaccgtgcgtgaagcgcgggcggaagcctttgtcaccatgcgcagcgagacgctggcgatgattattgatggtcgccaccacaaaggcgacgtatttgccactgcgcgtattgccggtattcaggcggcaaaacgcacctgggatctgatcccgctctgtcatccgctgatgctcagcaaagttgaagtcaatttacaggccgagccggagcacaatcgggtgcgtatagaaaccttatgccgcctgaccgggaaaaccggtgtcgaaatggaagcattaaccgcggcctccgtggcggcgctgaccatttatgacatgtgcaaagcggtgcaaaaagatatggtgattggtccggtacgtttgctggcgaagagcggcggcaagtcgggtgactttaaggtggaagcggatgattaaagttctttttttcgcccaggtgcgcgagttggtgggaacagatgcaaccgaagtggctgcggatttcccaactgttgaagcgttacgccagcacatggctgcgcagagcgatcgctgggcgctggcgctggaagatggcaaattactggctgccgtcaaccagacgctggtgagttttgaccatccgctgactgacggcgacgaagtagctttcttcccgccggtaaccggaggttaagatggcagaaaccaaaattgttgttggtccgcagccgttcagcgtaggagaagagtacccgtggctggcggagcgtgacgaagacggtgcggtagtcacctttactggtaaggtgcgcaaccataacctgggcgacagcgtcaacgcattaaccctcgaacactatccggggatgactgaaaaagcactggcagaaattgttgatgaagcgcgtaaccgctggccgctggggcgcgtcactgtgattcaccgcatcggggaattatggccgggcgatgaaatcgtttttgtcggtgtcaccagtgcgcatcgcagcagtgcgtttgaagccgggcagtttattatggattatctcaaaacccgcgcaccgttctggaagcgcgaagccacgccggaaggcgaccgctgggttgaagctcgggagagcgatcagcaggcggcaaaacgctggtagttttttgttagccggataaggcaccgctgcgtccggcaatttcaccgctcagtacatacgtttacgctgcgtcgatgcacagcctcatcattttgcagtatccttaagatattccttatatcttcaggagatcgtcatggacagattcccacgttctgattcaatcgtacaaccccgggctggcttgcaaacttatatggctcaagtctatggctggatgaccgttggcttgttgctgaccgcatttgttgcctggtatgcggctaattccgcggccgtgatggagctgttgttcactaaccgtgtctttttaatcggtctgatcatcgcgcaattagcattggttattgtgttatcagcgatgattcaaaagctgagcgcaggtgtaacgacgatgctctttatgctttattcggcgctgacgggtcttacgctttccagtatattcattgtctataccgctgcttctatcgccagtactttcgtcgttactgccgggatgttcggcgcaatgagcctgtacggttacaccacgaagcgcgatttaagtggctttggcaatatgctgtttatggcgttaatcggcattgtgctggcatcgctggtcaacttctggttgaaaagcgaagcattgatgtgggcagttacctacatcggcgtgattgtctttgtcggattgacggcgtatgacacgcagaaactgaaaaatatgggtgagcagattgatacccgcgacacgtcgaacctgcgcaaatattccattcttggcgcgttaaccttgtatctggacttcatcaacctgttcctgatgttgttgcggatcttcggcaaccgccgttaattctttttcaccatcactatcccggccatgtgtcgggatttttttcttactaaaaacgacacttaacaagtaccaggtataaaatatgccttatggacgagcggaagcgttttctgtatccataaatgcaaaagtattttgtatgcgtggttttaaatttattgatggtgaatattaatattttttctaaggataactaaaagaatggaatcatactcgcaaaacagcaataaattagattttcagcacgaggccaggatattaaacggtatatggctcattaccgctttaggtttggtggcaaccgcaggactagcctggggagctaagtatatcgaaattacggcaaccaaatatgattcaccaccaatgtatgtcgccatagggttattattactttgtatgtatggcttaagtaaggatatcaacaagataaatgccgccatcgcgggcgtaatatatctgtttttactctctttggtggcgattgtcgttgcaagtttagttcctgtatatgccattatcatcgtgttcagcactgcgggcgcgatgtttttaatcagtatgctggccggtttattatttaatgttgatcctggttctcaccgttttatcattatgatgacgttgacagggttggccctggtaatcatcgtgaatgcggcattaatgagtgaacggcccatttggataataagttgcttaatgattgtgttatggtcaggcattatctcgcatggacgaaataagctccttgaattggcggggaaatgccatagtgaagagttgtggagtccggttcgttgcgcttttacaggtgcattaacactctattactattttatcggcttctttgggatacttgccgcgatagctataacgcttgtctggcaaaggcatacgcgtttttttcattagccgtaaatgcacatactaaagaacttaactaaacttcacatcgccgcttcatttttcgcccgtagcttcttcgcctggctttccagcaacaggtaacagatcagcgccagcagcagtgggataaagtaatacagcacacggtaagcgagtagggcggcgataattgtacctttggaggtatgctccccagccagtagtgcgataaacaccgcttccagcacaccgatccccgccggaatatgcacgatgacgccagcaatactactaaccagtaacacgcccagtacaaagaaatagttcacgctttgaccaagtaacagccagataatcgcccccattaccatccagttaacgctggaaatcagcatctgagcgagggcgaatttccatgaaggcagcaccagcttttgccctttgatggtcatatggcggtgcttcgcgaaagcgcaaaaccacaaataaaccgcgataatcatcagtaagccaatgccgagaatacgcagcgtagtttgatcgacataccagtgatccggcaactccaccacgcctgcggtaaagataatccctgccagtaaaatgtagcccagccagttggtggtaatactgagcgagaaaatccgcgtaatagtgctaccgggcaaccccagacgagagtacaaacgatagcgcataccaatgccgccgacccaggtactgagcgtcaggttgaaggcgtagcagataaacgacaccagcatcacctggcgcttcgccagtttgtgaccgcagtaaaagcgggcgagcaggtcatagcagccgtaaatcagatagctgacgaccaccagcccgaccgcactaagcagcgcaacgcgattgtagtcgcggatgaccttccagacctcttcccagtccacttttttggcgtagaccaccagcaacacaatcaccgcgataaaaaacagccaggtgaggatcttctttgctaagcgccagcgcgggtgtgatttactcatcagggttttacccccgtgttttcagtttctacccgatcctgcgtttccattgtcggttgtgcgggcggatcaacctgcgccagacgtggcgtgtgtgccggaagccagccaaccagcgccgggaagtggcgtaaaaagtggaacgccagcacgcttttggtcaggttccaccaggtgcgtttgggcagcatggtttcatccacctgctgacaatctgcggcaataatgccgttcagattatcgcgcagcgtctggttaaaatgacgatcgtggatgatgacatttgcttcgagattcagtgacaaactgagcggatcgagattactggaccctactgtcgcccagtgatcgtccatcaatgccactttgccgtggagcgggcggcggcggtactcaaaaacctgaacgccgcctttaaccagatagttatacagcaagcgcgcaccgactctgacaatcggcatatccggttcgccctgaatgatcagtttgatccgcaccccgcgccgtgccgctttacgcaaggcgtgtaaaaatcgatagccggggaagaagtaggcgttggcgataatcacttcccgccgcgcctgagtgagcattttcaaataatggcgttcaatatcatcgcgatgttcttcgttatcgcgccagaccagcaatacctgcgcttctcccggctggcggttctcttccgctttgtgatgacgtcgccaccagcgtcgtgccgcgctctgtccaggcaggttttccagctcaaactggagaatatcttcgacaatcggcccttcaaggcgtaccgcgtaatcctgtttagcctctggaccgtagctggacatatgctcggcggagtaattcagcccgccaataaaggctatacgcgcgtcgatcaccacaattttgcgatgcatccggcgaaacacattggtgcgcataccaaaaaggcgagggcggggatcgtagtagcggaacactacgccagctgccgtcagttcattgacaaactcatcgctgagatccggcgaaccgtagccatccagcaagacttccgctttaaccccgcgttgcgctgctgccagtagtgccgcatgcagttgtttgccgacgtcatcctcaaaccagataaacgtttcaagaatgatgcgttcttgtgcctcgccaatcgccttaaacaccgcgggataatattgctcgccgttttccagcaactggatcttattgccttcgcgccagctacatttcataaatgaatctccgcacttaaaggggcatgatcagaaaggtgtcgccatgtccgcagcggcaacgcggttggcgcgctggcgctggcatttttgacgtagatcctgtccagtcgtagtagaggaaattgcaccggaaacgtgcgcgccgggcgtccgtgggcgcgggtaaaaatctcatccagtccggcctgcacttttaacggatgattagctttttgccgccagtcattgaaatcacccgccaccaataccggttcgccgtccggtagctcattcacccattcggcgagcatcgcaagctgcgcctgacggtgcgcctcacgcaggcccagatgtacgcacatcacatgaatcgcttttccggtcatcggcggcacaatgcggcagtagagcacgccgcgcttttccgcaccatcgaccgaaacatcgcgattctcataatgttcaatgggataacgcgacagtacggcgttgccgtgatgcccttccgggtatacggcattgcgaccgtaggcaaaatcgctccacatagtgtcggcgagaaactcgtagtgcgaggtatcgggccagttttccacatgcagcggatgaacttcgtgcgcgcccatcacttcctgcaggcaaacaatatcggcgctgacggtacgcacggcgtcgcgaagttccggcaaaatgaagcgtcggttaaacgcggtaaagcctttgtgaatattgatggtgagcaccttgaacgaaaattgttgtgtttgatcgggcataattttcctgtctttgcctcttatctcattgaaatagtgtagtcggcgtcacaaaaaggtgcggtcttacggaattttccgtaaagttcggtactctgagtaagtagagataaattcttcaggagagaagccatgaagtggcaacaacgtgttcgtgtcgcaacgggtctaagttgctggcagattatgttgcatttactggtagtggcgctgctggtggtgggctggatgagtaagactctggttcacgtcggcgtgggattatgcgcactgtattgtgtcacggtagtgatgatgctggtgtttcagcgccaccccgagcaacgctggcgtgaggtggcagacgtgctggaagagctgaccacgacctggtattttggcgcagcgctgattgtgctgtggctgttgtcccgcgttctggaaaacaactttttgctggcaattgcagggctggcaatccttgccggcccggcggtagtgtctttgctggcgaaagataagaagttacatcaccttacgtctaaacatcgcgtacgccgctgaccctgtcgtggccgttatcaccagtagcggccacaaactattccacacaatatccagactcgcatccttcaaataaatctgcttggtaatgtccgtaaagtggcgaatagggttaatccacgtcaggttttgcagccataccggcatgttttccaccggagaaacgtaaccggaaaggagaatggcgggcatcataaagacaaacacgccgataaacgcctgctgttgtgttgaacagagtgatgaaatcaacagaccgaatcccaccagcgataaaccataaatcaccatcgtaaagtagaacagcgccagcgatccggcgaaggggatttgatacgcccagataccaatcgccagcacaatggtggcctggaaggtggcgacaattaacgccggtacggctttgccgatgaagatctgccaggtggtgagcggcgaaaccagtagctgatcgagcgtaccttgttcacgttcgcgggcgacggaaagtgaagtgacgatcattacgccgatagtggtgatcatggcgatcagtgacggcaccacaaaccatttgtagtcgagattcgggttataccagttgcgtaccaccagctcgctgttgttaggtttcggttttccttccagcagctcctgctgataatttttgacgatctgttgcaggtagttggcggcaatttgcgcactgttggagttacgcccgtcgaggatcaactgcaaaggcgcggtctggaaggtatccagtttgcgcgagaagtcagccgggaaacgcaccagtagtaacgccttttgtgtgtcgatggttgggcggatctcctgtgggcttttcagcagcagcacatgagtaaaggcgctggcgcgggcaaaacgttgggtcagctccaccgaatgctcgccgttatcttcatcgtagatggcgatggtggcgttagtcacttccagcgtggcggcgaacgggaacaggatcacctgaattagcacgggtaaaatcagaatcgcgcgggtttgcggttcgcgcagcaacgactgcaactctttgcggattaacgtccataagcgatgaaacatgctcttctccctaatccagccgacgtttggttttcagccacgtcaggccgataaacatcaccgccgaagcgatcaaaaacagcacgtttaccaccagcaccactggaatattcccggcgaggaacaggctttgcagggtgctgacgaaataacgagcgggaataatgtacgtcaccgcgcggatcaccgcgggcatactgtcgatctgaaaaataaagccggaaagcataatcgacggcagaaaagcggcgttcagggcgacctgagcggcattgaactggttgcgggtaatcgtggaaatcagcagccccatccccagggtactgagtaaaaacaggctggagataaaaaacagaatcagcagcgacccgcgatacggcacgccgagaataaacactgacaccagcatacacagcaacatcgccagcatcccgagaaagtaataagggatcagcttacacagcagcagttccgtgcgggtaatctccgtagagagcagagcctccatggtgccgcgttcccattctcgcgccaccaccagcgaggtgagaatcgcgccgatgaccgtcatgataatggtcaccgcaccggggataatgaagtgctggctaatcgccgccgggttaaaccagtagcgggtttgtacatcaataagcggttcaaaagtctgcccgttgtcctccgctcgctgcatttgccagatctgccagatcccttcgacatacccctgtacaaagttagcggtattcggctcactgccgtcggtgatcacctgaatcggtgcggtggcgttggcgcgctccatctgttccgcaaaatccaccggaataaccaccagaccgcgaattttccccgcctgcattttggcgatcagttcctgacggttatcgctgatggtggcgtcgatgtagggcgaaccggtcatggtgtgggtgaaatccagcgccgcttcgctacgctgttccagtaaaatcccgacccgcagcttgctggagtcgaggttaatgccgtaaccaaaaataaacagcagtagcagcgggatcactaccgcaatcagccagctactcggatcgcgaacgatctgccgcgtctctttaacgcacagcgcccgtacgcgacgccaggacaggatcgggttactcattgctatgctccttatcccagtcgtggatcaactgaataaaggcttgctccatggtgggatcgggttgctcatcgttagccgactgtgctttcaaatcgtccggcgtgccgctggcgattaatttcccgcggtacaccaggccgatgcggtcgcaatattccgcttcatccataaagtgggtggtgaccatcaccgtgacgcctttctctaccatgctgttgatgtgcagccaaaattcacggcgggtgagggggtcaacgccggaagtcggttcgtcgagaaacagaatgtccggttcatgcatcagcgaacaggccagcgccagccgctgtttaaaacctaatggcagttcatcggtggcgtgggaggcgatacttttcaggccgaacgcctcgctcatgcgggagattttttcgttctgcgcccgaccgcgtaagccatacacaccagagaaaaagcgtaaattctgttcgaccgtcaggttaccgtagagcgaaaatttttgcgccatatagccgagatgctggcgcgctttaccggaactctctttcagatccatccccagcaccagcgcctggccggaagtcggcaccagcaaaccgcacatcatcttaaaggtggtcgatttacccgcgccgtttggccccagcaaaccaaaaatctccccacgtttaacggcaaagttgacgtgatcggtggcggcaaaatccccaaatttcttggtcagttctttcgcttcgatcaccgtctcgccgggtgtgccttctaccgtatgtaatattgcgcccagcggcgattccgaggttccggcaccgcccagcaaatcaataaacgcatcttcaaaacgcggcgtagtttcgttgatgttgatttccggcatcccgtcggcatggcgaatatcgtctggtgtggcctcttttttgaggatcagacgtaccgatttcccctgaatcatgccgtcgctgacctgcggcagtttcaaggcgcgttgcaacagtttgcggttgccctcgtgtggactggtcatcagaaagctgcgtccggccatggtttgtgtcagggcttttggttctccctgatacagcaactcgccttcgttcatcagtaacacgtcacggcactgctcggcttcgtcgagatacgaggtactccagaggattaacatcccttcgcccgccagctcatgcaccatctgccacagttcgcgccgtgagatagggtcaacgccgacgccgggttcatcgagcagcaacactttcggttcgcccaccagggtacaggccagaccgagtttttgtttcatcccaccggagagcttgcccgccaggcgtccggtaaacggcccaagagacgtaaactccagcaggcgagcaaaagtttgcttacgtgcctcgccggtgacgctgcgcaaatccgcgtacagattgaggttctccatcaccgtgagatcttcatacagaccaaatttctgcggcatataaccgagcacggcgtgcagcgcgccgtcgtttttgatcggatcaaagccaatcaccgtggcactgccgctgtcgggtttcagtaatcccgccaacatccgcatcagcgtggttttacctgcaccgtccggccccaccaaccccgtcacataaccggcgtgaatggtacaatcgagcggcgcgacggcgggcttgtccatgcccggaaagcgtttttccaggccgttcagcgtgataacggcatcattcatgtcctgcctcgtcaccgaattgtaccgtcactggcattccctggcgtaacgcatcatcggcgtcggtcaccacaatacgcaggcgatagacgaggtcggtacgcagatccggcgtttcgacggttttcggggtaaattcagcagtcggcgaaacgaaaccaatctgcccgtgatacggcttgtccgggcgaccatcggtataaagcagcactttgcgccccggctgggcctggtcaagattacgttcatcaacataagcgcgcacccacaccggacgcgttagtgaaacggtaaacaccgtgccaccttcattgaggaccgtgcctggctccaccgcgcgcgttaacagcgtgccatcagacggggctatcaacgttgagtcctgtaaattcaactccgcctgcgccagttgcgcctgcgcctgttcgaggctggctttcgcctgagcgatgtcctgttcacggttaccggaacggtactgacgcaatttatcctgtgctgatttcagcgttgcctgcgcctggtcgcgcgaggagcgggcattttccaggtcatttgccgaaatagtgcggcttttccacaacccttgctggcggttatagaagttctgcgcatagtcataggcggcttgcgcctgtttcaccgctgcggcggcctgagcgatttcttcattgcgatacccggcaagcatcaggtcatactgcgcctgtgccaccgaaacacccgctttcgcctgcatcagggcaatctcatacggcttgtgatccagttcgcccagcacctggcccgctttgatagcatcaccttcgtccaccgccagcgattcaacgcgccccccaacacggaaactaagatttaccgtacgaatatccacgttgccatacagcgtcaggccgttatcctggcggctttgataccaccagtagcctccggcaaccacggcggcaagtaccactaccgccaatccgatcacgacaggttttttcatcactacaaactcctttgcgataatccttgcaaaatcaggtcgatatgacaggtcaccgtctggttgatcagttcggtcttttcttcatcgaacgcggtccagccggtacgtaacagaattgtttctttgccaagacggaacgccagaatctcaccaatcaacgcatgggtatgaaggatcatgcgggtgtcattggcgtcgcagccggtccaggcggcaatcaggcgtgtcaggtggctgtgtagcggactaatcacctgttcgtgcaccaggtggtaggctgccgtgggagagagctgctcacgggagataaacttgctgaggttgacggtgtcatcctgggtgagcagcttaatcatgttcctgcaggcgcgaaggatcagttcacggatggcagcccgatcaggctgtggttgcgcgaacaagcgttcggcttcctcggcatgcggacggaactgctcgccaataaaatcggcaatccactgggcgcaggcgaggtacaaatcttctttcgaaccgaagtagtaggtgatggcagcgatattctgcccggcctgggcggctatctcgcgagtggtggcgttcattccatattcaccaaactgcgccagtgcggcagcaatcagctgttttttcgcctgttcacccttgattgtcatggcaggattattcatcgcacagtccattcttaatcaaatgattgattaagattatgactccataggggagttgtccagtatggctaagaattttagcaacgccagtcacagggataatttatgcgctgcgtcacaaaaactgctacactccgctccctcatgacattgtggtttttgtcattttccttttcagtatctccctgaaaactacaccggtaacggtcggggcggttcggagtagttatgtctttcgattctttgggtttaagccctgatatcctgcgcgccgttgccgagcagggttaccgtgaacccacccctattcagcagcaggcgatccctgcggtgctggaaggccgcgacctgatggctagcgcccagaccggcaccggcaaaacagcgggctttacgctgccgctgttgcaacacctgatcactcgccagccgcacgccaaagggcgtcgtccggtacgtgcgctcattcttaccccgacccgtgaactggcggcgcagattggcgaaaacgtccgtgattacagcaaatacctgaacattcgttcgctggtggtgtttggtggtgtgagtattaacccgcagatgatgaaactgcgtggcggcgttgatgtgctggtggcaaccccgggacgtttgctggacctggaacatcagaatgcagtgaagctggatcaggttgaaatcctcgtcctcgatgaagctgaccgcatgctcgacatgggctttatccacgatatccgtcgcgtgttaacaaaactacctgcgaagcgccagaacctgttattctccgcgaccttctctgacgatattaaagccctggcggaaaaactgttgcacaacccgctggaaatcgaagtggcacgccgcaataccgcgtctgatcaggtgacccagcacgttcactttgtcgataagaaacgcaaacgcgaattgctgtcgcacatgattgggaaagggaactggcagcaggtgctggtgtttacccgtaccaaacacggcgctaaccatctggctgaacagctcaataaagatggcatccgtagtgcggcgatccacggcaataaatcgcaaggtgcgcgtactcgtgcgctggctgattttaaatcgggcgatattcgtgtactggtggcaactgacatcgctgcgcgcggcctggatattgaagagctgccgcacgtcgtcaactatgaactgccaaacgtacctgaagattatgtccaccgtatcgggcgtaccggtcgtgcggctgctaccggtgaagcgttgtcgctggtgtgtgttgatgaacacaaactgctgcgtgatatcgaaaaactgctgaaaaaagagatcccgcgcattgcgattccgggctatgagccggacccgtcaatcaaagccgaaccgatccagaacggtcgccagcaacgtggcggcggcggtcgtgggcaaggtggtggtcgcggtcaacagcaaccacgccgtggggaaggtggcgcaaaatctgcaagcgcgaaacctgcagaaaaaccgtctcgccgcctcggcgatgccaaaccggcaggcgaacaacaacgtcgccgccgtccgcgtaaacctgccgctgcgcagtaatcttttatgccgggctatgcccggcatcaggctgatgaacaaacgcaaaactgcctgatgcgctacgcttatcaggcctacgtgaactctgcaatatattgaatttgcatgcttttgtaggccggataaggcgtttacgccgcatccggcatttcacaacaagcacttgtcagcaatttgagaacacgggaaaaaatttatctgttttaccgcccataagccaccgagacgttacttctctatagccaattgttcgcgcaactccattaaaaggtagcccagtcgattcttgcccttaccatgaccaccgtctccccagtaagcatcgttttccgtatgctcaaccagttttgcgggcgcggttgccagcaagagcgcacgcagttctgcatgctgttcgaatttagcgcgaagtgcttttcgcatcacctgttctttgaccgactcccagtttttacgcagaggcttagaacgatcgcgccccatgcgtgcggcgaccataggggaagaaacccgacggatctcttcgcggtatttttcatcaaggaatttttgtgcctgaaaatagtgttctgaggtaggccaggttttcccgtcaaccttgatgggccaggcggcaaagttagaaaaatcaccgtagtcatcgctggtgctgtagaaatttatgatggtgtcttgcatgacgtgttggatcctttgtgctcgaacgggcattaaaccgcattatgttggtggttattgcgagccgctttccagaaacagaaaaaccattacccctgaaaaccgaaaaatgccacaatattggctgtttatacagtatttcaggttttctcatggcattaaccgccgcgcttaaagcgcaaattgccgcctggtataaggcgcttcaggaacagatccccgactttattccccgtgcgccgcagcggcagatgattgcggacgtcgccaaaacgctggccggagaagaagggcgacatctggcgattgaagcccccaccggcgttgggaaaacgctctcttatttgattcccggcatcgccattgcccgcgaagagcaaaaaacgctggtggtgagtaccgccaacgtggcattgcaggatcagatttacagcaaagatttaccgctgctgaaaaagatcattcccgatcttaaattcactgccgcttttgggcgtgggcgctacgtttgtccgcgtaatctgacggcgctcgccagtactgaacccacgcaacaggatctgctggcgtttcttgacgacgaactgacgccgaacaatcaggaagagcaaaaacgttgtgcgaagctgaagggcgatctcgatacttataaatgggatggtctgcgcgatcatactgatatcgctatagatgacgatctctggcgtcgtttaagtaccgacaaagccagctgcctcaaccgcaattgttactactatcgtgaatgcccgttttttgtcgctcgtcgggagattcaggaagcggaagtggtggtggcaaaccatgcgctggtgatggcggcgatggaaagcgaagcggtattgcctgacccgaaaaatttactgctggtgctggacgaaggccatcacctgccggatgtggcgcgggatgcgcttgagatgagcgccgaaatcaccgcgccgtggtatcggctacagctggacttgttcacgaaactggtcgctacctgcatggagcagtttcgcccgaagaccatcccaccgctggcgatccctgaacgtttgaatgcgcattgtgaagagttgtatgagcttatcgcctcgttaaacaacattctcaatctctacatgcctgccgggcaggaggcagagcaccgttttgcgatgggcgaactgccagatgaagtgctggagatctgccagcggctggcaaaactcaccgagatgctgcgtggcctggcggagttatttcttaacgatttaagtgagaaaaccggcagccatgacattgtacgtctgcatcggttgattttgcagatgaaccgcgcgttggggatgttcgaggcgcaaagcaaactctggcggctggcttcgctggcgcaatcttccggtgcaccggtgaccaaatgggcgacgcgggaagagcgcgaagggcagctacacctctggtttcactgcgtgggaatacgtgtcagcgatcagctggaaaggctgctgtggcgcagtattccgcacattattgtcacctccgcaaccttgcgttcgctgaacagtttttcgcgtttgcaggagatgagtggtctgaaagagaaagcgggcgaccgttttgtggcgctggattccccctttaaccactgcgaacagggcaaaattgttattccccggatgcgcgttgagccttccatcgacaacgaagagcagcatattgccgaaatggcggcctttttccgtaagcaggtggagagcaaaaaacatctcggtatgttggtactgtttgccagcggacgggcgatgcagcgctttctcgactatgtgacggatttacgtctgatgttgctggttcagggcgatcagccgcgttaccgtttagttgaactgcaccgcaaacgcgtcgccaacggtgagcgcagcgtgctggtgggcttacagtcatttgccgaagggcttgatttgaaaggtgatctgctcagccaggtgcatatccacaaaatcgcttttccgcccatcgacagcccggtggtgatcaccgaaggggaatggctgaaaagcctcaaccgctatccgtttgaggtgcaaagcctgccgagcgcctcgtttaacctgattcagcaggttgggcgactgattcgaagccacggttgctggggcgaagtggttatctacgacaaacgcttgctgaccaaaaattatggcaagcgactactggatgcattaccggtatttccgatagagcaaccggaagtccctgaaggtatagttaaaaagaaagaaaaaacgaaatccccacgccgtcggcggcgttaatgatgtgagtcaggtaaggagtcgtaaatggactatcgcaaaatcattaaagagatcgggcgcgggaaaaaccacgcgcgcgatttagaccgggatactgcgcgcggtctgtatgctcatatgctcaatggtgaagtccctgaccttgagttgggcggcgtattgattgcgctgcgtatcaaaggagaaggggaagcagagatgctcggcttttacgaagccatgcaaaatcacaccatcaagctgacgccgccagcaggcaagccgatgccgattgtcatccccagttacaacggcgcgcgtaaacaggccaacctgacgccgttgttggcgattctcctgcacaaactcggttttcctgtggtggttcacggggttagcgaagatccaacccgcgtgctgactgaaaccatttttgaattgatgggtattacgccaacgttgcacggcgggcaggcgcaggcgaagctcgacgaacatcaaccggtgtttatgccagtcggcgcgttttgcccgccgctggaaaaacaactggcgatgcgctggcggatgggcgtgcgtaacagtgcacataccctggcgaaactggcgacgccatttgccgaaggtgaggcgctgcgtctttccagcgtttcgcatccggaatacattggacgcgtcgcgaagttctttagcgatatcggcgggcgggcgctactaatgcatggtactgaaggtgaagtgtatgctaatccgcagcgctgcccgcagatcaatctcattgaccgtgaagggatgcgggtgctgtatgaaaaacaggacactgctggtagcgagttactgccacaagcaaaagatccggaaaccacggcgcagtggattgagcgttgccttgctggcagcgaaccgattcccgaatcgctgaaaatccagatggcttgctgcctggtggctacgggtgaagcggcaactatcagcgacggcctggcgcgcgttaatcaggcattttaattcttttctcagccggatgagccatgtcatccggcttttaccccaccgcaatatgaaattcctgcatctttattgaccttcccacgcccggcgtgcagcataaaaatacaacaaacacataacataaacaggagttaaccatggaaagtggtcatcgctttgatgctcagacgctgcacagttttattcaggctgtatttcgtcagatgggtagcgaggaacaagaagcgaaattagttgccgatcatttaatcgcggcaaacctggcagggcatgattcacatggtattggcatgatcccaagctatgtacgctcctggagtcaggggcacctgcaaattaaccatcatgccaaaaccgttaaagaggcgggggcggcggtcacgctcgatggcgatcgcgcatttggtcaggtcgcggcacatgaagcgatggcgctggggattgagaaagcgcatcagcacggtattgccgccgtggcgctacataactcgcatcatatcggccgtatcggttactgggcggagcagtgtgcagcggcggggtttgtctctatccactttgttagcgtggtcggtattccaatggtcgcgccgttccacggtcgcgacagccgctttggcaccaatccgttctgtgtggttttccctcgtaaagataatttcccgctgttgcttgattacgccaccagcgccattgcatttggcaaaacccgcgtcgcctggcataaaggcgtccccgtgccgccaggttgcctgattgacgttaacggcgtgccgacgaccaatccggcggtaatgcaggagtcgccgttgggttcgctgttgacctttgccgaacataaaggctacgcccttgcagcgatgtgtgaaattcttggcggggcgctttccggcggtaaaacgacgcatcaggaaacgttacaaaccagtcccgatgccattcttaactgcatgaccactatcatcatcaacccggaactcttcggcgcgccggattgtaacgcgcagaccgaagcctttgccgagtgggtgaaagcctcgccgcatgatgatgataagccgattttgctaccgggcgagtgggaagtgaacacgcgtcgcgaacggcagaagcaggggattccactggatgcgggaagctggcaggccatttgtgatgcagcgcggcagattggtatgccggaagagacgttgcaggctttctgtcagcagttagccagctaaaaaaaagcccgtccagtggcggacgggcaaacaagggtaacataggatcaatgagggttagagcatatgcgtctgtcggcaaacagacagggaaatacttgtgctggacgtagcgtaaacgcctgatccgtccaacggttcggattttgtaggcctgataagacgcggtagcgtcgcatcaggcatctgttgccggatgcggcgtaaacgccttatccgtcctacgaattacttataaattaccgcagtaccgcttaatttattgttgttggtggcggaagtgatgctgtatccactggcaccggctgccgcggctttctcagccagtttcgcttccagggcatcgagggtggatgcgccatcggcagaaaccacgccgattttattcatgttctgtgcctgggatgccgttaccggttccgccgcgaacacgccaaatgacagagttgaaagagccatagcagcaacaacagtattgatagttttcataattaatctctcgcaggtgatttttgtataagtgacgttgtttcgtcgatgtgatgagtatcacgtttttttacgagagataaaatcgaagagaattgaccgccttgttcaaataaattgattgatatctaacctactgataaaccatttatttgttgtacttatgaacttgttttataccgcgtggcagtcacagcagcgttaaaggcacggaatgacacgcaaaatacaaattatactcgctatgcatctcgccagttgtagttaacgtaactggctgtctttcgaacctctgcgattatatcctgtataagctggtttttgtaaatctttctcctgctgacaatgaatacataagcgcacgccaggaatggcttcccgacgggcctgcgggatgggggcaccgcactcttcacattcatccaggctttcgccgcgcggaatttcaccccgagcgcgggcaatcgcatcttcaattgtactgttgatctgttcgttgacggcgtcatcgttagcccaaccggatgccatatcgacctccccatatcaatacttgtacagttaagtgtagctaatccagggacgaactcgggcagttcaagcatcagatctccgaccattcccgcagcagattatgataaagattaagcagcgacaggatctcttcactttcgccgtagcggcttttcagcgactgaatattgttgtccagttcaaacagcatggcgcgctttttatcatcgcggatcatcgactggatccacataaatgatgccactcgtacgccgcgggttacgggtgtcacgcaatgcaggctgctggagggatacaacacgagatcgcctgccgggagttttacccgatgttgtccgaaggtgtcattaacgaccagttcgccgccgtcgtagctttgtggatcgcttaaaaacagcgtggcagaaaggtcagtacgcatccagccgttttgtggatggctgcgtactgcgccatccacatggaaaccataggtttcattgttctgatagcgattaaacagcggcgtggaaagggtacgcggcaaggccgcggcaaagaataaagcatgttggttaaccgcgttcagcacctcattttgcagggcggcgtataacgtgctgcgggtgtcgacctgttgattgttcttaacttgcgcaccttgtgcgccggtggtgacgcgtccatccacccattcggcttgttccagttgttcgcgaaaacgagcgacgtcctgtggcgataacacgccgggaatgtggtacatcatacaatttctccaaaaagtggggcctgcgccccacatctgaatcagaaatgcatattggctgtgagcaagaaggttcttggctcgcccgggtgataacggtagccgctcttgttgattgaggcgacgtaatcggtatcaaacaggttgtaaacgtttagctggaagtcgagattgcgattaactcgataccccagtttggcatcggcgacccagtaaccttcggtaaacgctggcgttcccaccgcgccgtctgaacctttatgcatactgccgatatagcgtgcgcccgcgccaacagagatatcgtcggttgcctgatattggctccataaggtgaaggcgtgctccggggtatacggcagcgatgaggaaccatcctgggcaacatctttgccgtttttgatggttgctttttgctgggtatagccgccaatcacctgccacgcgggagtgatattcccggccacggatatctcatagccttcgacgcgtttcttaccgtattgcgagtaagttccgtcatcattttgctcaacttcattttcgatatcagtgcggaacagcgcggcggtgagcaacagacgtttatccagaacctgccatttggtgccaatctcgctggtgttggctttttgcggtttaaaatcggtgcggttggcactgttaccgctgccagactgcgcaagggcgaagttgttgccgcccggaggctgctgggaaacggcatagttaatatagacattgccgttttccgtcaggtgatacagcgccccggctttccagttcatcagattgcccgacttggcggtgtcgacggtggtgaccggagaaccttttgccacaccagttgggcaggtgatggcaccgcgtccgctgccgccgcaggcggtggcactgtcatattcagtatgataattatccagacggatcccgccgttcagctcaaaatcacgggtgatttgcagcgtatcaaaggcgtaaattgcgaaggtatccgtctgaccattggcgtttgcgccgttgcgcgtcaggccgccgggatgaatgctgctgtcaggatgataaatatttaccgcgggtaacgtcaccggattaacgccgtagttagtctgcgtttcacgggtaaattccacgccggtactgacatcatgaccgatagaaccggtatagaacgtcgaggtcaggttggtctggttggtgagaattttattactcacatctttggtattcgccgtgcgtgaccaggtccagctattcacatcgctggtgggctgagtaatattcgacgccccgcccataatcgccgtcatcaggtaatcctgctttacgcgcgaccaacgggtagtattgcgaatggtggtgttatcgttgatgtcgtgctcaaaacgcatggtggcggtgtcggtggtcgaatcgtcgtaatcggaatccgtgccgtaaaagttatgagtatcaacttttccggaatgattcagggccgccgttcccgcagatggggcagaatagcccggcaaaccgatggtcggaatgccgccgtctggcgtgttgtgctgggtgacatgcagataattaagatacaaacgattcgctgtaccaaggccaaaagcgacagaaggggcgacgccgtaacgctcatttttgactttgtcgcgtccggcatcgtgcgttttttcgcccattacattcaggcgcaccgcggtggtatcaccaatgacctgattgacgtccagcgtgccgcggcggaaccaggcgctgccaatactggcggaggcgtcaatgccggaatcattgcgcggctgcttgctgatcatattgatcgagcctgtcggtgcgctgcgcccgtagtcggtgccggacggccctttaatcacttcgacctgctcggtattgaaggtgtcgcgcgagacgctgccgatatcgcgaatgccatcaatataaatactgttagaggtatcggcaccacgcatataaatggcgtcgccagtggtggagttaccgttctcacccgcaaaaaacgcacccacgccggggacgtttttgagcgcgtcggtaaggttggttgcgccctgatctttaatcacttgttcagaaattaccgtcatcgtgcgggtagtatccgctaccggacgcgagaatttcggatcggcagattgttgtggcgcataaagcgaaggcgttgatgcttcgacaaccagcgtgtcatccgcgttagtttgcccttcggcggcgagtgcctgagccacaggcgtgatgccaatacaaagaccggcaaagaacgtgagcgaatgaaattgtctggcagggaaattgcgattgttttccattttgcaggtgactttttcttatatgttgaaattttcactgccacgagaaagcctctctgcggatgcgatgccactgttaatcccgtgatagtgctcgtgaaagtgataataattttgataagcattatcacttggagcgattttctatcacccattgcgcgaaaaagaaatacatttatttacattgagttcatatttgatgttttttgattacaaaacagacgaaaactgcatccagaggcgaatgcagttacgttggtggggttatttgtagatggttgcagtaccgaacatctggtcatttccgcctgcggaattaatgacataacctttcgcgccttgttcgcgcgctttttctgccagtttatcctccagatcgcttaggtttgatgcgccagttgccgaaacggtaccggcgggccgtagctgaccgctgtccaggttactcatcggttgcgcggcataagccgtgagagagattccgctcaggacggtggcaatcagtagtgtgaggcactttttcataatgacatcctcataaatacaacgggtagtgcctgataagtgtaggtcgcctgcgcgatgcaaatgacgcaaaaaattgacagagatgtgcttattttttgaacgatatatttttacaaaataagacaaatcaatgacatgcataatgctgatttttatgatgaattgccataaaccatagccatgttaaggttttggggaatgataaacgcagccagatatttaccctgtcgcgttatgcgggtatcttacgccgctgcttaaaggagaatgctatgtccgcccagaaaccggggttgcatccgcgcaaccgtcatcacagccgctacgatctcgccacgctttgtcaggtcaatcctgaactcaggcaattcctcacgcttacacccgccggggagcaaagcgtagactttgccaatccgctggcggtgaaggcgctcaataaggcgttgctggcccatttttacgccgtagcgaactgggatatccccgacggttttctctgcccaccagtaccgggccgggcggattatattcatcaccttgccgatttactggcagaagcaagcggaacaattccagcgaatgccagcattctggatatcggcgttggtgcgaactgtatttatccgctgattggcgtacatgaatatggctggcgttttaccggtagtgaaaccagcagccaggcgttaagcagtgcgcaggcgattatcagttctaatccggggcttaaccgcgccattcgtctgcgtcggcaaaaagagagtggggcgatttttaacggcatcatccataaaaacgagcaatacgacgcgaccttgtgtaacccgccattccacgattccgccgctgcggcacgggcaggtagtgagcgtaaacgccgtaacctggggctgaacaaagacgatgcactgaactttggcggccagcaacaggagttgtggtgtgaaggcggtgaagtcacctttatcaaaaagatgattgaagagagcaaaggcttcgcgaagcaggtgatgtggtttacatcactggtatctcgtggtgaaaacttaccgccgttgtatcgtgccctgacggacgtgggcgcggtgaaggtggttaaaaaagagatggcccaggggcaaaagcagagtcgctttattgcctggacctttatgaacgacgagcagcgccgccgttttgtcaatcgccagcgttaaagcgttggttcccccggcggtaacggttcagccggggtcgcgcccggagcaggcagcacctgataagtctgcactggcgcgcgaacgcccgccaggtcgaaatgttttttcacctggctgtcgagggcaaagcgtaccgtccactgtttgagtggcagcgtggtgaacgaaacacgcagtgtaaacgcggtattgcttaagccgacaatcccggcaaaattcggttcaccaataatcagcccgcgaatttcttcgttttccattaattccgctaccgcatctttcagtgcctgattggctttatcagcatcttcatggcgatcaacatcataatttgccaccaccgaaccaatgccgcggacaaagttagcaaaggtggttatcgaagaccacggaatgatgtgatacgccccggtatcctgtcgtacgcccacggagcgaatcgacatccgttccactgtgccggtcaacggcccgatagtcaccaaatctccagtgttcatgccgttttcaaactgaataaataccccggtgataatatctttcaccagcgtttgcgaaccaaacgagatagccagacctaatgccccggcacctgccagcaatggcgcgatattgacgccgatttccgacaacacaatcatgatggtgatggtactgataatcaccgccagcgcgttacgaaacagcgtaagcagggtacgcgtgcgggcgctgggtagcgggcggccatgaatatccgaagccagccggttttcgatcaaactggcgagcaccgtccagccaaccgccgagaagaaaagaatgagtgcgatacggatcaggatatctacggttttctgccccgcgccgttttgcagccagttccagaaatcgaacaatccccatgcgctcaacagcaacattaccgccacgcagactgtcagaatacgcgccgttttcagcgccgccgacagccagccattcaaccgtttttgcagctccggatagttacgctgagtatgtggcgagagagtgatggttttcgccagccagcgggaaaacataccggaaacaaacgctgcgataccaataatcgccaggctgcgcaccgttgcacccatcataaatttcaggctgttgcccggatcgaacaacgaaaagaaaaacagcacgataaaataggcgcttgccagccagtgccacaccagcgcaaaggcgcggataaacaggctgaaaaaggccagcgaatgctccgcgaagttgagcaaatgctgggtaatctcttttttattacgaaagatcaggtacaacgcccagacggtcatgcacagcataatgatgacgttcgccagcgcacctatctgtacattcacctgattagagataatcggcacggccacaatcaggccataacctatcaaactgcttaaccagctcaggcgacgactccagtaacgggcgctctcgtcctgaatcgtgaacgggcgcagctccgccacgtttgggcaaaaaatcaggcgtagtacggctttgaaaaattcaatgagggcaaaggcgttgagaaacaaactttgttggaaagcgatggtgcgactgcctgcattcaggttgtcgcttaatacctggccgacaaataatgtcagggccagtaacagcaggtcgataataaacgccccgataatcatcgccggaagctgcaaccagttgctgcgctcacgatttttttgccgcgcccactgacccattttgcgatacagcggcagtgcgcacaggcgaatcagccagtaaaaaccaaacactaataccgctaacattgaaaaatgggtcagcgcattgctgaaggtttgtggattaaacggcttatgcggggagccggtgatattgcgataaagttgcccgaagcgggcggaaagggcttcaccataatggcggctgacttcggtgaccttttgcagcacggtttgctcttcgaccagcgtcggcggcactatttttggtaccggttcagcagggggcgtagcggcaacggtgcgcaactggtcgatcaactctttacgcgaggtgtcattatccagcacatccgccagtgcgccataggccgcttttttttgttcgatatccggttccggggccggttcagtcgttgagtccgttgtcgttgtggttgtaacgccgggtatggataccgcgtgggcaggtgcgcccagcaggcagaagaggatgaacaggatccaccgcatgactcctccagtgagaaaatagagcaaaaagataagtatagatgctggaggaggggcgattttaaatgagaggaatctggtgtgcctccctttcgggtgaaagggaggaagggatattaagcaggttgctgacaacgtgcgggcttttttgccggatgcggcgtgaacgccttatccgtcctacaagttcatgcaattttaataagttgccagatatcctgtaggcctgataagcgtagcgcatcaggcaatgtgtcttattaagagacgtgctgcaaaaattcctgcaagcgctggctcggcgggttcttgatcaacacctgcggattgccatcttccgcaatccggcctttgtcgataaagatcagccgcgaagctactttctcggcaaaaccgatttcgtgggtcacgatcaccatcgtcatcccttcttcagccagatcctgcataaccttcagcacttcatggcgcagttccgggtcaagagcggaagtcggttcatcaaacagcatcattttcggcttcaccgccagcgcgcgggcaatcgccacacgctgctgttgaccaccagaaagttcggaagggtagtgatgtgcacgttctgccagaccgactttcgccagcagctcacgtgccagtttttccgcctcttctttgttcgcgccacgcacgcgtagcgggccaaacatgacgttttccagcgctgtcagatgcgggaagaggtaaaactgctggaacaccatacctgcttcctggcgaatcaggcgctcgtcaactttcggatcgttaaccttcaggccatcgacaatcagatcgccggaggtgatttcttccagtttgttgatgcagcgcagcagggtcgatttaccggaaccggacggcccgataatcaccacgacttcgccctgggcaatgttcaaatcgatattgtgcagcacctgggttgggccaaagtgcttggagacgtttttaaattcaatcacaggattttcatccttctttccagacgacgcagaataaagctcagcaccagggtaataatcagatagaacaccgccacggcgctccagatctcaagggcgcggaagttaccggcaataatttcttgcccctgacgggtcagttccgccacgccgatcacaataaacagcgaggtgtctttaatgctgatgatccactggttacccagcggcggcagcatacgacgcagtgccagcggtaaaatgacgtagcgaatggtttcccaacgtgaaagaccgagcgccagtcctgcttcacgaaaacctttgtggatagacagcaccgcaccacgcgtgatttccgcaatatacgcgccggagttgatcatgatggtgaccaccgccgcagtaaatgggtcgatgcgtaagtcgttaaacgccatcggcagggcgaaataaataaacatcacctggacgacgataggtgtgccgcggatcacttcaataaagaccagcgcgacgtggttggctatccaacctccgaaggtgcgtgcaaaacctgccagcaatccgattaccagaccgcctgccagaccgaggaccgaaatccacagggtcattttggcaccttcaatcagaagcggaatggcaggccagatggcactccagtcaaactgcatatgttgttcctgttaccgtggtgtaaataatcaaattcagggtaattaatggccccggagcgggtttgcgcccctcaccctaatcctctccccataggggagagggaactgccagtgcgttttacaggtgtagcgttattatttcggttcagtaccgaaccattttttgtagatttcgttgtaagttccgttctcgcgcagggttttcaacgcgccgttgactttgtcacgcagctcgtcgctacctttcgggaacgcaataccgtattgctgcgcttccagagagtcacctaccgctttgaactgaccgttaccggcggttttgatgaagtacagaatgtttggcgtatcgtgcagaacggcgtctgcgcggttggtgcccagttccatataggcgttatcgatgttcgggaactgacgcagatctttagttttgatgtttgctttcgcgtaatcaacggagccagtaccgctcttcacagcaaccactttcccgtcgagatctttcacgcttttcacatcgttattgttagctttcaccatcactaacaggccgcttttgtagtagccgtcagagaaatcgatcgcttttttacgctcgtcggtgatggtaatgcccgccagcgccagatcgacgtttttggtttgcagtgccggaatgatcccactgaaatccatcggcttcagttcgtaatccagcttcagctctttagcgatggcagcccacagatcaacgtcaaagcccacatatttatcgccctgtttaaattcaaacggaacgaaggcggtatccgtcgcgacaactaattttttatccgcggcatgagaagaaaccgcaaaagccagggtcagtgcagccagtgaaacttttaatacagacttcatagcatttccttttttctatccacgggacgatcccctgcgtgacattcacatatatgaaaaaatcgtgccagttttgcaactccttgatttttcgagatgcggcaaaaacgtgatgcacgatttatagggcaataccctgaagatgcaccattctggggcaccaatctggtgcgctaaaattgtgcactcaacacagtgattatttagcgtaaaacctgatgaaaaaacaatctttatgtaacgattgtgtgatgatgtggatacaaaaaatttacttaatcagctggagatagcagatggatgcactaaataagtgcgttgaggtgggctgcaaaacaaaacggcctcctgtcaggaagccgcttttatcgggtactaaagttctgcaccatcagcgatggatttattcgatgttagactcgataaaccacaggaatttatccaggtcgcgagacgcggcggtcaggatatctgcggtgtcgtcatctttcgcttcgccaatcgctttgcgtacgtcattagcgacgattgcgtaacggtcagccagttctttcaggtgatcctgaacgttgtggatgtccagcgggtaacttttcagcggggttttgctgttgataacttgagtggtccccagagctacaccgcccagctgcactgcacgttctgccatggtatccagatgatcgatcagtgcggtgcggaagccatccagcatttcatgtacggcaatgaagttagcgccgcgcatgttccagtgcgcttgtttggtaatcaaagaaagatcaataaactggataacctggcgattcagcaactctactgttgcttttttctcgctgtcggagacatcgttgcgggtataaagcagattggtcgcttttgatttaactaatttagcggtactcataatttcatatcctcttgatgttatgtcccagtaattaacgagattaagtatagcaccggctatgtgttccgctattctggctgttcctatcacactaatagtggtaacaagcgtgaaaaacaaaactaataaagattcaatgagttagatatattgataagaacaattcttatttatctgctcgccaggaattttcggaataaatatgcttttgcataattcgatatataaagacggtgtagaggaaaagtagcgagaaattctgcatggttatgcataaccatgcagaaatgtaaatttaattaatgtctaattcttttattttgctctctttgcgtactgtcagcgtagaccccattgaagcggcgatgatagcgccgagcgccagtagctgtatgggtgtcagtgtttctccgaggaaaatcatcccggaaacggcagccagcgccggttccatgctcatcagcgtaccaaatgtccgtgttggcaaacgggtgagggcaatcatttccagcgaataaggcagagcggtcgagagaatagcgacagccagacccaatggaataaccgaccagtgccagagtgcttcaccagcctgaagcgctccaattggcacgaaaattaacgctgcaatcaacgaaccaattgccaccgtcgcagggccatgttccgctcctgcgcgttgcccacttaaaatgtaaatagcccaacaagccccggcccccagtgccagcgcacagccggttaaatcgacatgggaaacgtcttgccccagcggtagcaggaaccacagaccaagaaccgccagcacaacccagacgaaatctaccgggcgacgagaagagaacagcgccaccgccagtggtccggtgaactccagcgccaccgcaatacccagcggtactgtctgaatagaaagataaaaaagataattcatcccacccagcgaaacgccgtaaaacaacagcggtaaccgttgctctttggcaaagcgcagtcgccatggcttaaagaacgcgatgaggatcagcgttcctaatgccagacgcagcgcagtgacacccggtgcgcccaccagaggaaaaagtgacttagctaacgaggctccaccctgaatagacgccatggcaacgagcaatatgactattggtaaccagaccggcattttacgtaatgaaccaggcatcctttctcccacaaatatctagacttaagtaaagcgtggagtgtactggatatacccaatgctggttgagcatttgttgaaaaaattttcccccgttttgactaaaatgcgccaggattgatggaatcattagtctggtgattaggaataatctggatgaatgacagggaaaacatgcgtaatacttacgcagttctctgaaaaagtgatttaaatttagatggatagcggtgtatggaaacgttctgttacatgaaatggcccgttagacatcacaaatcgcgaagagtttcccattaatttttgatatatttaaaacttaggacttatttgaatcacatttgaggtggttatgaaaaaaattgcatgtctttcagcactggccgcagttctggctttcaccgcaggtacttccgtagctgcgacttctactgtaactggcggttacgcacagagcgacgctcagggccaaatgaacaaaatgggcggtttcaacctgaaataccgctatgaagaagacaacagcccgctgggtgtgatcggttctttcacttacaccgagaaaagccgtactgcaagctctggtgactacaacaaaaaccagtactacggcatcactgctggtccggcttaccgcattaacgactgggcaagcatctacggtgtagtgggtgtgggttatggtaaattccagaccactgaatacccgacctacaaacacgacaccagcgactacggtttctcctacggtgcgggtctgcagttcaacccgatggaaaacgttgctctggacttctcttacgagcagagccgtattcgtagcgttgacgtaggcacctggattgccggtgttggttaccgcttctaatcactttggtgatataaaaaatccgcctctcggggcggatttttgtttttaaggtttcgggtcgaaaatatcggttccgagatggttgtaatccaccttctgtaactggaagttggtgatgtatatcggcccggctttcttctcagatataaacgggtatttgatgttaatttccttcgctttaatccccgtccactgggagaaaaagcctaagaagtcattggctgagcggcgggctttaatcacacgatgcgctttatcgtcgctggaaatgaccataaaaggcacctggaaattttgctgatatttatcatcatgggcaaggtattgcacgtctttaccgcgctctttaaaggccagaccgtggtcagaaaagtaaaccagcgagaagctgctgccgctgttgcgtaactgatcgtacagcttgcgcagtaaatcgtccgtttgcgtcatggtatagagatagcacgacgtttctttcgattgcacaaaggtttcgtattttccttgtgtcctgtcgcaggcctgcggatgtgagcccatcagatgtagaacaatcagctgcggttgcgagtgctcttgcgccagcacttgagcggtcatatccagtaacgcttcgtctttggtgtttttatctgcttcaaaattaccttctttcaggaagtacacttcatctgctcgtttggcgatgctggcgatagcggtatcgtattcgccgatttgaccctggttggaaaaccaccaggtctggaagcccgcgcgatttgccagggtgacaaagttatcctgaaactgtggtttgccatcgacaacgcgattgagcgttaagccaagcgatttctgcgtggagccactggcggcaatgtagtcagcaaatatcaaaccgttaacgctgctggcaaacggggtattgtcccagtgaccgccaaaggcaccgagggcatcgcgacgcgcgctttcaccgatcaccaccacataggtctgatacttcggcttaacggcagtgaccgtccaggtatctttcattccggaaagttttgccatccgttcttgctcttcaatcacctcgttattattgacgatgacatccttagcaaaacgaaataccggatagccagtatctttcagtttaaatacgccaccccaggccaggttttgcacgggagcaacaaaaaatgtcgccacactgaataccagacacaggctgtcgaaggtattccagcgcgctttttcattctctttttttcgcctgattgctattacgccgagcgcaaaaataaataagccgaccaggtagctgtaccacggaaaaatcgtcaggatttcggtcgactcttccatattggtggagtgcaatgccagcaatgtattgaaattaggcgcgccgtaggcctgagcaaaagggaaataacaagccgccaccagcgaactgacaccgaccagaactttttgtacgcgaggcaatgttcgccatagcaaaagcaaaatagccgtaaacgcagcggtgtagagcaaactgaaggggtaacctaagccgaggttaattaatagcgactgtaaaaagtagaacgcagtccacgggctaaatacccggctacgggtaacaagcgattctttgagggttaaattcatatgccactatcgtaacaaacgccatgtgcttaccctggcgtcaagggtcaatacctgcaagagtgcgtgaagagtggaaaggggtccgcatccgcgagccgcaatatacgcagggctgcaagaagatagagcgagccgccgttcaggtcaactactgacgaacaaatcttttgcgaaggggattgcaaatccgacaaaaagtggggtttttcagaccaaaacgcgttatgcctgcatgaaagcaggagtgaagcggcgtaccgcgacgccgctatttatcggaaggtttatcttgctgcggtttgttgttgaccatatcgcacaacatagagagcagcattaaccgtactttaaagggagaatgactaaacacgcgcatacacctcttgaactcattcataagacctcctgacttgctaatcccgtcgatccttgagggatgattgcattacatacagatatagcacaggctatattatatagctattgctaaaacgttaattttttgtaccttcgcaactctggtttacaatgtgcgcacgaaatgagaacgctatgtatgcgtcaccataatgaggaagcacaatgagtcgtcgcgcaggtacgccaacagcaaaaaaagtgacgcagttagtgaacgtggaagagcacgttgaagggttccgccaggtcagagaggcgcatcggcgcgagcttattgatgattacgttgagctgatttctgacttgatcagggaagtgggggaagctcgtcaggtggacatggctgctcgtctgggagtttcgcaaccgacggtggctaaaatgcttaagcggctggcaaccatggggctgattgaaatgatcccctggcgtggcgtgtttttaacggcagaaggagagaagctggcgcaggaaagccgcgagcgacatcagatagtcgaaaatttcttgttggtgttgggcgtcagtccggaaatcgcccgtcgcgacgcggaaggcatggagcaccatgttagtgaagagacgctcgacgcttttcgtttgtttacccagaaacacggtgccaaatgagcctgccttttttacgcacgctgcaaggcgatcgtttttttcagttattaattcttgttggtatcggattaagctttttcgtgccctttgcaccgaaatcctggcctgctgctatcgactggcacaccatcatcaccttaagcggcctgatgctgctgaccaaaggtgtggagttaagcggttattttgatgtgctggggcgcaaaatggtgcgccgctttgctacggagcgtcggctggcgatgtttatggtgctggcggcggcgctgctttctacctttctgaccaacgatgtcgcgctgtttattgttgttccgctgactatcacgctaaaaagactgtgtgagatcccggttaatcggctgattatttttgaggcgctggcagtcaacgctggttcgctactgacgccaattggcaacccgcaaaatattcttatctggggacgttctggtctttcgtttgccggatttattgcccaaatggcaccgctggctggcgcaatgatgctgacgctcctgctcctgtgctggtgttgtttccctggaaaggcgatgcaataccatacgggggtgcaaacaccggagtggaaaccgcggctggtgtggagttgtctggggctgtatatcgtctttctgacggcgctggagttcaaacaagagctgtggggactggtgattgtggcggcaggctttgcgctgctggcacgtcgcgtggtgctcagtgtggactggacgctgctgctggtgtttatggcgatgtttatcgacgtccatttactgacccagcttccagcgttgcaaggcgtgttgggtaacgtgagtcatctatctgaacccgggttatggttaacggcaatcggtttatcgcaggtgatcagtaacgtgccgagtaccatattgttgctgaactatgtgccgccgtctttattactggtatgggcggtaaacgtaggtggctttgggttattacccggatcgctggcaaatttgattgcgctacgtatggcgaacgatcgccgcatctggtggcgtttccatctctattcaataccgatgctgttgtgggcggcgttggtgggatatgttttgttagttatactcccggccaactagggtctggcaaataaaaaaggcggattatgagtccgccttttgctttaagttttgaagattaattcagacgaaccggcatcccggagcggtttttaatcgcttcatcaagaacaacctggtcaacatctggctgaccggtcactgtctgcacgctcttcgtcagggtaattggcacaatttcctgaccttcaaactgggcttcggtggtagacagcgggttatggacttcaatataacggctgccgtctggctcggtggtcgcttttaccggctcatcaataaactgtacgcgggtaccgaccggtactttctcgaacaggaatttgatgtcttcgttacgcagacgcacacaaccatgacttacacgcaggccgataccgaagttggcgttggtgccatggatagcatacaggcgaccgatatagagtgcatacagccccatcgggttatccggacctgccggaacgacagccggaagcggttcgcccgcagcgcggtactctgcgtgcattttggcggtcggcgtccaggtcgggcctgcttttttacgctcaactttggtggtccagttgataggcgtatctttgcctaactgaccaatgccgatcggcagcacgataacggtgttggtccctttcggatagtaataaagacgcatctcagcactgttaatgacgatgccttcatgaacggtatccggcaggatcagctgctgcggaatgttcagtacagtaccgcctttcggcaggaaggtatccacacccgggttcgcttccatcatattggaaagccccatctggtactcggcggcaaaatactccagcggctgagtgttaccttcaggaatggtgatcacctgattctgaccaaccaggcgactcccgtcggttggcagaggataagttaccgcagaggcggtactgcaaaagccgacaacagcgaaggccgctgcgaataatgttttcaatttcatattcatgttaagcgagattttgtgcctggcaggccattgggttgagaatattagagtattggaagcgcattataagttcattccagctcacagtgaaatcagatgtgtacgaaatcacattttttgcctttggcttgagtgtagaccttaagcgaggagcaggatcttctttcagacttatggcataatgcgcggtttgtcatatctcttttcaggatacgcctgtgttagtttccagtaacgtcaccatgcagttcggcagtaagccgttgtttgaaaacatttccgtcaaatttggcggcggcaaccgttacggcctgattggcgcgaacggtagtggtaaatccacctttatgaagatcctcggcggcgaccttgagccgacgctgggtaacgtttccctcgatcccaacgagcgcattggtaaactgcgtcaggatcagtttgcctttgaagagttcactgtgctggatacggtgatcatggggcataaagagttgtgggaagtgaagcaggagcgcgaccgcatctatgctttgccggaaatgagtgaagaagacggctataaagtggccgatctggaagttaaatacggcgaaatggacggttactctgcggaagctcgcgccggtgaactgttgcttggcgtgggaattccagtggaacagcactacggcccgatgagtgaagttgctcctggctggaagctgcgtgtgcttctggcgcaggcgctgtttgctgatccggatattctcctgctcgacgaaccgaccaacaacctcgacatcgacaccattcgctggctggaacaggtgctgaacgagcgtgacagcaccatgatcatcatctcgcacgaccgtcacttccttaacatggtctgtacccacatggcggatctggattacggcgagctgcgcgtttatccgggtaactacgatgagtacatgacggcggcgacccaggcgcgtgaacgtctgctggccgataacgccaagaagaaagcgcagattgctgagttgcaatctttcgttagccgctttagcgccaacgcctcgaaatctcgccaggcaacttcgcgcgcgcgccagattgataaaatcaaactggaagaggtgaaagcctccagccgtcagaacccgttcatccgttttgaacaggataagaaactgttccgtaacgcgctggaagtggaaggtctgaccaaagggtttgataacggtccgctgtttaaaaatctcaacctgctgctggaagtgggtgaaaaactggcggtactgggtaccaacggcgtcggtaaatcaacgctgctgaaaacgctggtgggcgatctgcaaccggacagcggcaccgtaaaatggtctgagaacgcgcgcattggttactatgctcaggaccacgaatatgagtttgaaaatgatctgaccgtgttcgaatggatgagccagtggaagcaggaaggcgatgacgagcaggcggtacgcagtattctcggtcgtttgctgttcagccaggacgacatcaaaaagccagctaaagtgctttccggtggggaaaaagggcggatgctgtttggtaagttaatgatgcagaagccgaacattctgatcatggacgaaccgaccaaccacctggatatggaatccattgagtcgctgaacatggcactggaactgtatcagggcacgctgatctttgtttcacacgaccgtgagttcgtaagctccctggcgacccgcattctggaaatcaccccggaacgcgtgatcgactttagcggtaattacgaagattacctgcgtagtaaagggatcgagtaagtgattatccgtcaccccgatactgtcggggtgacggcggctgatgacaaatgcaaaatagcctgatgcgctacgcttatcaggcctacgcagtacctgcaatatattgaatctgcaggactttgtaggccggataaggcgttaacgccgcatcaggcattaacaaagcgcatttgtcagcaatctgagtaacgtcgaatcgattttcttaatcccacatcaattcacttccattaattctcaaacatccatgcccaacgctcgcttaccgtgaatgttgaggtcggcaagcgtaaagcgtccttcccagtttgtttcatagtcctcgcgcgggaagtcgcccggcgatgcgcctttttccagtgcggccttcaccttgtgcgcgtaggcaagatttttctcgcacatcggtgccgcaggaatgtacatcacgttgccccaaccttgttgattttcaacgggggcaacggaatggatgacgtcgcagtgccaccagacggagtctccggcttcgagttttggaatgctggttaacgcctcaatcaacagtggatgccattgctctgataccggcaatactcttccgggcgctacgccgcacagttcatcctccggcacatcatcaagcagcggacgtaacagtacgtacgccatagcttcaggaatgggcacgacgtgcagcagcccctgaccaggcagcatatcagagagcgctgtccagccctggaatgtccgaaacacggaacatttggtggtgttgtccaccgtgtactcttcaacttccgtacgatgtgccgcatgccagggatcatattgcgccagattgccattaaagacgttggcgaaaacgcgctgatacgctggaagcagccagcgttccagtgccccggagtcggtatgcgctccaagacctttggaggtcgttccgggcggacggcggcggatacggtcagggtagatgacgctcacatccgggttaaaccattgctttccatcactttcaaatgtccacagacgattgagaaacgactgcgcattcgccatttcttcactctggcgggcctgcatttgcgcctgcgaccagtagatggggtaaatctcgggacgtgaagcgctgagcgtcccgaagaaattatcgccggggcctttgtagacctcgtcaaagcggttgcggtccagatagtccagcatcgactgatcccagcctagcgcttgttcgcgggggaaatggccttttatcaccgcacaaccgcgacgtttaatctgttcgcgctgctctgcagtaacatgacctgctttgatatcggcataagacagcaccggccagacggcatcgccctgtgctttgagtgcgttgatttcagccactcgcgtggcaatgtcatcgcttagctgattaaagatctgctggacgtcgccaagctgcgcccgcagcgcgtgcttcatctgacggatagctgctttgtgatcggcaggcaatgtgtcgctggtaaaagtagaagccataaccacctctcattaactttcattcgaaaccattctgatttgcatgtgacaatataagttataaataagttaatgcaagtttaatgatttgatgtgatgtacaggatgtaaaaagaagggaaaaccggagcgcacggctccggtagagaggtcagctgttaaaaggggatgtgttatccagcaccgcctgaatcacattcagcgcgccttcatgattattatcatcggtagcgtaacgggcgatttgtttaatgttttccgcagcattgcccatcgcaaaggaataacgcgccattttcagcatctccgcatcgttaccgctgtcgccaatcgctaccacattttgcggtgacagatcccagcgtttcagtaaccgcgaaataccgtttgctttatgtagaccgggaataatcaggtcgataaagccaaaaccactggtaacgggtttcataatgccatcgagcgctacgtgcagtttgtcgatcactaacgggatttgttcatccggcaggttgagcgaaaacttgaacagtacgtcgtcaatctcctgataatcttttacaggtttcaggcgatggtagtgttttgccatcagtgcgacaaatgcttcgggggcattttcgctgacatatgcactttgcagaccgcaggcgacaaaattgagttgcttatcttttagcaactcgccaataacaatccgcgattcatgtcgggtcagttcgccgtggaacaactgcttgccatgttcgtaaaccagtgcgccgttttccgcgacaaaagagatctcatcctttagctcaggaaagaatgaaataagctggtaatactgattaccgctggcaacaacgaacttaatgccgcgctttttcagttcctgatattgcgccataaaacgtggttggttgtacgttttggcgtcgttaagaaaagtaccgtccatgtctgtgacgataacttttacgctcataggtgtgctcctggctcgaaaatgaaaccgtaacagtgtaataacaatgtgacgcagagcacaaattatatttcgaatgaaagtaaggatgaaattgatgatgtgaatgatttagcccggcgacgacgccgccgggccgaggagattacagcatatgttcagtacgggcgatgatatcgtcctgagcgtctggagagagcgcggtgaagaacgcggaatagcccgcgacacgcactaccagatcgcgatactgatcgggatgttttttcgcatccagcagcgtttcgcgggaaacgatgttgtactgaatatgccagcctttatgcacttcaaagaaggtacgcagcaggatcatcagtttctgcttgtcagattcgttctccagcgttgccggattcagtttctggttgagcaacacgccgccgagaatcgctgccgtaggcagtttacccactgagccaatgaccgcagtagggccaagatggtcagtaccggaggccgggcttgcgccttctgccagcggggtgtgggctttacgcccgtccggtgttgccatagtctgcgcgccaaacggtacgttagcggagattgatgacgtacccgcgtaatagttgccgccaaccggaccacgaccgtagcgcggattatggtactgtttcagttcgtcgatataggtctgataagcgcgagccagcagcgtatcgacagtatcatcgtcgttgccgtacttcggcgcaccgttaatcagccgctgacgcagctgctcgtgagtcaggccgtcgaagtcatctgccagtgcggcagcaagctgttgctgaccaatcgcaccttgttcaaacaccagtttcttcactgccgccaggctgttgccgaggttggcaatgccgacctgcaggccagaaacccagtcatatttcgcgccgccttgcttgatacttttcgctcgctcaatacagtcatccaccagcgccgagcagagaatatcgtgcacgttctcttccagcatggtgtcgacgacatattcgatttcgattgatttgcgggtgtagtaacggatttgcgtatcccacgcgtccatcacttcatcgaagttgttgaagttacctgccgacaacgctttttcttgtggcaggaacactttgccgctggtggcatcatgcccgccttccagcgccgccagcatcacgcgggcgaagttgataaagctcatgccggtacagcgatagccccatttgccaccgacggcggtttctatacaaccaatcgctgcgtagtcataagcgtcctgcggttcaataccgagtttaataaattccgggatcacgatttcgtcgttgttgaacgccggcatcccgaagccgcaacggatcacctgtacgcaggcgtcgaggaaatcgttgctcattcctgcatggtaacgcacgctgaggttaggctgagtggaacgcaggcgaccgcaggattcgaggatcgcgtaagagagtggattcaccgcgtccattggttgaccatcaaccagattttgcccgccaatagtgacgttctgatacagcggacttcccgcagaggcttttgagtgtgagccggagcggatcttgttcacttccagcagtttcagccagcagctatgcagcatctcgatggcgtgttcgcgatccagcgtctggttgagttcaacgtcgcggcgatagtacgggtagagatactggtccatacgaccaaacgatactgagtgaccgttagattcgatctgcaaaatcaactggatgaagtaacacagttgcagcgcctgccagaaagtctgcggcggctggtgggcgataagatcgcagttttctgccatcgccagcagttcatcgcgacggctttcgcgggtttcggtcgcggccatttcacgcgccagggcagcgaaacgttcaatgtgttcactgactgccaccagcacgatatcaatcgctttcaggaattgctcaccgtgtaaatcttccagcaccgtcaggttgatgcgcgagcgacgttccgctacttcctcgcgcagaccatcaagccctttttccagcagcagcgggaaattcaccgccaggtgcgcatcgccggaggtcatattgccttccgctttaatgattccggtcgccagcagacctttttgctcatcggtaaacatgccgtagcagcgatcctgtacggtctgaccgcgccaccacgggcacacttcatgcagaacgcgtttgttctcttcgctcaccgcaaagccagcaccgggacgatctgccagatcatcaatctctttttcgatccacgagacagtatattccgggaagatcggcgcggcgcgaacttcgcttgcctggttgccaatgatcaactcatcgtgtttgatccagatggtgcgattcgccaggtgatgcgccagtgccagcgcgcgacgtaccgggatcggcttatcgagatgttgttgatacatctcggtatagtgctgcgcgcgctcggtacagactggcggtttcacaatatgcaccagcgcatttttgtgcgctttaatgcggtcgctgagcgtgtccagtttcagtgtggtcatggttgttatcctcgtaaggtcgcggttaaccctttctggcaggcatactgctgggcaaagtcgagcagttctggcgcatcaagcggtttttccggggcgtcatagggcagattaagtaagtgatatttgttgatgcccagcgtgtggtagggcagaaaatgaatttcgccaacgtgcagctcgtcggcggcaaaatcggtaatggcttttacagaggtttcgtcggcattaaagccctgaatcagcggcacgcggataatgatttttttgcccgctgcggcgagttttttcaggttatccagcactctggcggcgttaccgtcggtccactgtttaaacggcgcgtcggcaacgtgttttaaatcggcaagaaacagatcgatatagggcagagaaggggcgatatatttccacggcacatgcagacaggtttctaccgcagtatgaatgcctgcctcgtggctggcttgcagtagcgccatcgccatttccggctgcataaagggctcaccacccgaaagcgttaaaccgccgccgctgcgatcgtaaaacggtttatcgcgcagaacggtcgtcatgatctcctcaacgcttttcacttcaccacacacggttaatgcctgtgtcggacagcagtcggttaacgccgtcagatgctccggggttaacttttcccgatgaataagcaaaccattcagcgcgcgctcaatcacttccggcgcggccttagcgcacagctcgcagccttccagacacagtcgtgcgtcatacagcagatcctgcgtgcgggcgcggctttccgggttctgacaccagcggcagcccagcgaacagcctttaagaaatacgaccgtgcggataccggggccatcatgggtcgagtagcgctgaatattgaaaatcatagttgcctctctatttcgttcaagcattaaaatactttcgaatgaaagttagattgatgtgcgtcaactgttcagagagttttcccgtgatagtctacattcagacaaaaagtacattttgaggatggttatggaactgtatctggatacttcagacgttgttgcggtgaaggcgctgtcacgtatttttccgctggcgggtgtgaccactaacccaagcattatcgccgcgggtaaaaaaccgctggatgttgtgcttccgcaacttcatgaagcgatgggcggtcaggggcgtctgtttgcccaggtaatggctaccactgccgaagggatggttaatgacgcgcttaagctgcgttctattattgcggatatcgtggtgaaagttccggtgaccgccgaggggctggcagctattaagatgttaaaagcggaagggattccgacgctgggaaccgcggtatatggcgcagcacaagggctgctgtcggcgctggcaggtgcggaatatgttgcgccttacgttaatcgtattgatgctcagggcggtagcggcattcagactgtgaccgacttacaccagttattgaaaatgcatgcgccgcaggcgaaagtgctggcagcgagtttcaaaaccccgcgtcaggcgctggactgcttactggcaggatgtgaatcaattactctgccactggatgtggcacaacagatgattagctatccggcggttgatgccgctgtggcgaagtttgagcaggactggcagggagcgtttggcagaacgtcgatttaaccggacgttctgcatcctcataaattgctgatgacgtggcggagtgccgcgtcttatcaggcctggaggtggcaattactgcccacacacctcacaccccggattacgcatcagtttcatttcgcgaaactgacaggtcatcgcatcgtacatgacgattttcccgctggccggtttgccataacctgccagcattttgatcgcttccattgcctgcaacgaaccaattacgccgatcaacggtgccattacgcctgcttccacgcaggttaatgcattttcaccaaacaaacggctaaggcagcgatagcacggttcaccgtcctgataagtaaagacggtgatttgaccttccatacgaattgccgcgccggaaaccagcggtaccttcgcggcaaaacagcctgcgttcagttgattacgtaccgcaacgttatccgtacagtcgagcaccagatcgtgttcagcaatcaatgctgcaagttctgcgtcatccagcagtgcattgactggcgtaatcgcgatatgtgggttgatccgcgtcagggcgtcacgggcggattccaccttcggttgcccgaccgtggcatcactgtgcagtgtctggcgttgcagattcgagagcgaaaccgtgtcgaagtcgagcagcgtcaggttaccgacaccggcgcttgccagatactgcgaggctgcacagccgaggccgcccaggcccactatcagcacgcgagaatctttcagcgcctcctggccgtcaaaatcaaagccgcgcagaatgatttgccggttgtagcgcagcatctcctgatcgctgagttccgccattacaggcctccgaacaacgcgttaaacggttctacttccacccattcgcccacttccacattgccgcgatcgcgttccagcacgataaagcagttgccgaggctaaaggagctaaatatatgtgaaccctgatgtccggtggtcgtcacttccagttcgccatcggcgttgcgttgcagcacgccgcgctggaaatcaagacgtcctggcgtttttttcaggcgggacgctgtgcgtacgcgctggcgcgcgggcaggccgctggcggtgttaccgcttagttttgccagcaaaggctgtaccagttgatagaaggtcagcgtcgctgaaaccgggttgcccggcaggccgcagaaccagctattgctgagtttaccgaacgcgaacggtttacctggtttaatcgccagcttccagaaggcgatctcccccagctcttcaagaatcgttttggtgtaatccgcctcacccactgaaacaccgccggaactgatcaccacatccgcctggctgtcggcttcaataaatgcggcgcgcagggcatggggatcgtcgcggataatccctaagttaattacctcgcatcccaactgttctaacatcaggtgtacggcgagacggttggtatcgtagatttggccgtcgcccagcggctgaccgggcaactggagttcatcaccggtagaaaaaagcgctacacgcactttacgaatcaccggaacttcggcaatccccagtgaagcaattactggcagctctgcggtagtcaggcgagttcccgccgggaaaacaaccgcacctgcagagatatcttcaccgcgacggcgaatattttgcccgctacgcacttcagcagtaaaacgcacgccattgtccatttgttcagtctgctcctgcatcaccaccgcttcgcagccttccggcaccggcgcaccggtcataatacgaatgcaggtacccgcaggccattcaccatggtatggctgaccggcaaaggatttaccggcaacgggcagcggttgcccggaggcaatatcggctaaacgcaccgcgtagccgtccattgcggagttatcaaaccccggaacatcaagcggcgaaacgacatcgctcgccagaatacgaccaaaacactgtaccagtggcagcgtttcctgggcggtcagtggggtgacgcgagaaagcatctcattaagcgcggtgtcgagcgacatcaatccggtggtaaattccatgaaaacactcctgcggaggcaaaatcgaatttgcctattatgtcagaaaaacgccacagactgtatgccacctcgggcgtagcgctgggtcctgcctttacatgccatatccatctttctatattcaaaaattgaatgagtaattcataaaaattctgatatttatagcaaaagtggcgaaccacccttaatggacgaatactatgggcaaagcagtcattgcaattcatggtggcgcaggtgcaattagccgcgcgcagatgagtctgcaacaggaattacgctacatcgaggcgttgtctgccattgttgaaaccgggcagaaaatgctggaagcgggcgaaagtgcgctggatgtggtgacggaagcggtgcgtctgctggaagagtgtccactgtttaacgccggaattggcgctgtctttacgcgtgatgaaacccatgaactggacgcctgtgtgatggatggtaacaccctgaaagccggtgcggtggcgggcgttagtcatctgcgtaatccggttcttgccgcccggctggtgatggagcaaagcccgcatgtgatgatgattggcgaaggggcagaaaattttgcgtttgctcgtggcatggagcgcgtctcgccggagattttctccacgtctttgcgttatgaacaactactggcagcgcgcaaggaaggggcaaccgtcctcgaccatagcggtgcgccactggatgaaaaacagaaaatgggcaccgtgggggccgtggcgttggatttagacggcaatttggcggcagccacgtccacaggcggaatgaccaataaattacccggacgagttggcgatagtcccttagtgggtgccggatgctacgccaataacgccagtgtggcggtttcttgtaccggcacgggcgaagtcttcatccgcgcgctggcggcatatgacatcgccgcgttaatggattacggcggattaagtctcgcggaagcctgcgagcgggtagtaatggaaaaactccctgcgcttggcggtagcggtggcttaatcgctatcgaccatgaagggaatgtcgcgctaccgtttaacaccgaaggaatgtatcgcgcctggggctacgcaggcgatacgccaaccaccggtatctaccgtgaaaaaggggacaccgttgccacacagtgatgaacttgatgccggtaatgtgctggcggttgaaaatctgaatattgcctttatgcaggaccagcagaaaatagctgcggtccgcaatctctcttttagtctgcaacgcggtgagacgctggcaattgttggcgaatccggctccggtaagtcagtgactgcgttggcattgatgcgcctgttggaacaggcgggcggtttagtacagtgcgataaaatgctgttgcagcggcgcagtcgcgaagtgattgaacttagcgagcagaacgctgcacaaatgcgccatgttcgcggtgcggatatggcgatgatatttcaggagccgatgacatcgctgaacccggtatttactgtgggtgaacagattgccgaatcaattcgtctgcatcagaacgccagtcgtgaagaagcgatggtcgaggcgaagcggatgctggatcaggtacgcattcctgaggcacaaaccattctttcacgttatccgcatcaactctctggcgggatgcgccagcgagtgatgattgcgatggcgctgtcatgccgcccggcggtgctgattgccgatgagccaaccaccgcgctggatgtcactattcaggcgcagatcctgcaattaatcaaagtattgcaaaaagagatgtcgatgggcgttatctttatcactcacgatatgggcgtggtggcagagattgccgatcgggtactggtgatgtatcagggcgaggcggtggaaacgggtaccgtcgaacagatttttcatgcaccgcaacatccttacacccgtgcgctgttagctgctgttccgcaacttggtgcgatgaaagggttagattatccccgacgtttcccgttgatatcgcttgaacatccagcgaaacaggccccccccatcgagcagaaaacggtggtggatggcgaacctgttttacgagtgcgtaatcttgtcacccgtttccctttgcgcagcggtttgttgaatcgcgtaacgcgggaagtgcatgccgttgagaaagtcagttttgatctctggcctggcgaaacgctatcgctggtgggcgagtctggcagcggtaaatccactaccgggcgggcgttgctgcgcctggtcgaatcgcagggcggcgaaattatctttaacggtcagcgaatcgataccttgtcacccggcaaacttcaggcattacgccgggatattcagtttatttttcaggacccttacgcttcgctggacccacgtcagaccatcggtgattcgattatcgaaccgctgcgtgtacacggtttattgccaggtaaagacgcggctgcacgcgttgcgtggttgctggagcgcgtgggcctgttacctgaacatgcctggcgttacccgcatgagttttccggcggtcagcgccagcgcatctgcattgctcgcgcgttggcattgaatccaaaagtgatcattgccgacgaagccgtttcggcgctggatgtttctattcgcgggcagattatcaacttgttgctcgatctccagcgtgatttcggcattgcgtatctgtttatctcccacgatatggcggtggtagagcggattagtcatcgtgtggcggtgatgtatctcgggcaaattgttgaaattggtccacggcgcgcggtcttcgaaaacccgcagcatccttatacgcgtaaattactggcggcagttccggtcgctgaaccgtcccgacaacgaccgcagcgtgtactgctgtcggacgatcttcccagcaatattcatctgcgtggcgaagaggtggcagccgtctcgttgcaatgcgtcgggccggggcattacgtcgcacaaccacaatcagaatacgcattcatgcgtagataacattcaggcggagaataaaatggcaagagctgtacaccgtagtgggttagtggcgctgggcattgcgacagcgttgatggcatcttgtgcattcgctgccaaagatgtggtggtggcggtaggatcgaatttcaccacgctcgatccgtatgacgcaaatgacacgttatctcaggccgtagcgaaatcgttttaccaggggctgttcggtctggataaagagatgaaactgaaaaacgtgctggcggagagttataccgtttccgatgacggcattacttacaccgtgaaattgcgggaaggcattaaattccaggatggcaccgatttcaacgccgcggcggtgaaagcgaatctggaccgggccagcgatccggcgaatcatcttaaacgctataacctgtataagaatattgctaaaacggaagcgatcgatccgacaacggtaaagattaccctcaaacagccgttctcagcgtttattaatattcttgcccatccggcgaccgcgatgatttcaccggcagcgctggaaaaatatggcaaggagattggtttttatccggtgggaaccggaccgtatgaactggatacctggaatcagaccgattttgtgaaggtgaaaaaattcgcgggttactggcagccaggattgcccaaactggacagcataacctggcgtccggtggcggataacaacacccgcgcggcaatgctgcaaaccggtgaagcgcagtttgctttccccattccttacgagcaggccacactgctggagaaaaacaaaaatatcgagttgatggccagtccgtcaattatgcagcgttatatcagtatgaacgtgacgcaaaagccgttcgataacccgaaggtccgtgaggcgctgaattacgccattaaccgtccggcgctggtgaaagttgcctttgcgggctatgcaacgccagctactggtgtggtaccgccaagtatcgcctacgcgcaaagttataaaccgtggccttacgatccagtgaaagcgcgcgaattactgaaagaggcgggatatcccaacggtttcagtaccacgctgtggtcgtcacataaccacagcaccgcgcagaaagtgctgcaatttacccagcagcagttagcgcaggtcgggattaaagcccaggtgactgcgatggatgccggacagcgggcggcagaagttgaaggtaaagggcaaaaagagagcggcgtgcggatgttctacactggctggtcggcttcaaccggcgaagcggactgggcactatcgccgctgtttgcctcgcagaactggccaccgacgctgtttaataccgcgttttacagcaataaacaggtggatgacttcctggctcaggcactgaaaactaatgatccggcggaaaagacccgcttatataaggcggcgcaggatatcatctggcaagaatcgccgtggatcccgctggtggtagaaaaactggtgtcggcacacagtaaaaacctgaccggtttttggatcatgccagacaccggcttcagctttgaagacgcggatttgcaataagcaacgcagggagtggaatgcttaattacgttatcaaacgcttactggggttgattccgacgctgtttatcgtctcggtgctggtgtttttatttgtccatatgctgcccggcgatccggcgcgattgattgccgggcccgaagctgatgcgcaggttatagaactggtgcgtcagcagctggggttggatcagccgctgtatcaccagttctggcactatatcagcaatgctgtgcagggggattttggcctgtcgatggtgtcgcgtcgtccggttgccgatgagattgccagccgctttatgccaacgctgtggctgaccataaccagtatggtctgggcggttatatttggtatggcggcgggaattatcgccgccgtctggcgtaaccgttggccggatcgattgagtatgaccattgcggtgtcggggatctcgtttccggcatttgctctggggatgcttttaattcaggtattctccgttgaactgggctggctgcctaccgtgggagcagacagttggcagcactacattttaccctccctgacgctcggcgcggcagtggccgccgtgatggcgcgctttacccgcgcgtcgtttgtcgatgttttaagcgaagattatatgcgtaccgcgagggcgaaaggggtgagcgaaacctgggttgtcctcaaacacgggctacgtaacgcgatgatcccggtagtgaccatgatgggcttacagtttggctttttgctcggtggttccatcgttgtggagaaagttttcaactggccgggacttggacgcttactcgttgactccgtagaaatgcgtgattacccggtgattcaggcggaaattctgcttttctcgctggaatttattcttatcaacttagtggtggatgtgctttacgccgccattaacccggctatcaggtacaagtaaggatgcgactatttaactggcgacgtcaggcggtgttaaacgccatgccactggtcaaacctgaccaggtacgtacaccgtggcatgaattctggcgacgatttcgccgtcagcatatggcgatgaccgccgcattattcgttattttattgattgtggtggccatttttgcacgctggatcgctccctatgacgccgaaaattattttgattatgacaatctgaataacggaccttctttgcagcactggtttggcgtcgattcactggggcgtgacattttcagccgtgtcctggttggtgcgcaaatctcgctggcggcgggcgtgtttgccgtgtttatcggtgcggcgatcgggacgttgctgggcttgctcgctggatattatgaaggctggtgggatcggctgatcatgcgcatttgcgatgtgctgtttgccttcccgggtattttactggcgatcgctgttgttgcggtgttgggaagcggcattgctaacgtgattattgcagtcgccattttttccatccccgcgtttgcccgcctggtgcgcggcaacacgctggtgttgaaacagcaaacctttattgagtcagcacgcagtattggtgccagcgatatgaccgttttgttgcgtcatatcctgcctgggaccgtctcttctatcgtggtgtttttcaccatgcgcattggtacctcgattatctctgccgccagcctctcatttctcggcctcggtgcgcagccgccgacaccagagtggggagcaatgctcaatgaggctcgagcggatatggttatcgcgccgcatgtcgctgtttttccggccctggctatttttctgaccgtactggcgttcaatttgttgggcgatggtttacgcgatgcgctggatccgaaaattaaaggatagttacgtttgaatattgcttgaaagggtaatcacctcacaggaaattattgccctaagcaagtgttgtaactttctgctgattttgtagaatcgggtaatttggttaaaaagccgcagcaagggacaatttttgcagcggcacagcgttcagatagttattttgttaaatgtattaacatgctgagtttatacgaaaagataaagataaggctgataattttatttttattggcagcactgtcatttattggtctttttttcatcattaactatcaactggtatcggagcgcgcggtaaaacgtgccgatagccgctttgaacttattcagaaaaacgttggctatttctttaaagatattgaacgttcggccctgacattaaaggactcactgtatttattaaaaaatacagaggagattcaacgcgccgtgattcttaaaatggaaatgatgccatttttagactcggtgggactggtacttgatgataataaatattatcttttttcgcggagggcgaatgataaaatcgttgtttatcatcaggaacaagtaaatggaccgcttgtcgacgagtcagggcgggttatttttgccgattttaacccatcgaaacgaccgtggtcggtggcttcagatgactctaacaacagctggaatccggcatacaattgctttgatcgtccgggtaaaaaatgtatctcttttacgctacacatcaacggcaaagatcacgatttgttagcggtggataaaattcatgtcgatttaaactggcgatatctgaacgagtatcttgatcaaatcagcgctaatgatgaagttctatttttgaaacaaggccatgagatcattgccaagaatcaactcgctcgtgaaaaactgattatttataatagcgaaggtaattataatattattgattctgtcgatactgaatatatcgaaaaaacatcagcggtgccaaacaacgcattattcgaaatctatttttattatcctggcggtaatttattgaacgcatcagataaacttttttatctgccgtttgcgttcattattatcgtattgctggtggtttatttaatgaccactcgtgtgttccgtcggcaattttctgaaatgacagagctggttaatacgctggcgtttttgcctgactcaacggatcaaatcgaggctctgaaaattcgtgaaggcgatgcgaaagagattatcagcatcaaaaattcgatcgcggaaatgaaagatgccgaaattgaacggtcaaataaattgctctcactgatctcttacgatcaggaaagtggttttattaaaaatatggcgattattgagtctaacaataatcagtatctggctgtggggatcatcaaactgtgtggtctggaagccgtggaagcggtgtttggtgttgatgagcgcaataaaatcgtcaggaaattgtgtcagcgaattgccgagaaatatgcgcaatgctgcgatatcgtgacattcaatgccgatctctatttacttctgtgtcgggaaaatgtacagacatttacccgtaaaatagcgatggtaaacgattttgacagcagctttggctaccgcaatctgcgcatccataagtctgccatttgtgaacctttgcagggggaaaacgcctggagttacgcagaaaaactgaaactggcgatttccagtatccgtgaccatatgttctcagagtttattttctgtgatgacgcgaaactcaacgaaatagaagagaatatctggattgcgcgtaatattcgccatgcaatggaaattggcgaactattcctcgtctatcaaccgatcgttgatattaacacccgcgccattctgggcgcggaggcgttgtgccgttgggtgtctgcggagcgggggatcatttcaccgctgaagttcattaccattgctgaagatatcgggtttatcaatgagctgggttatcagattattaaaacggcaatgggtgaattcagacattttagtcagcgtgcgtcgctgaaggatgatttcttactgcatattaatgtttcgccctggcagttaaacgaaccacactttcatgagcgttttaccaccatcatgaaagaaaatggcctgaaggcgaacagcctctgtgttgagatcactgaaaccgtgatcgagcgaattaatgaacatttttatctcaatattgaacaactgcgtaaacaaggggtacggatatcgattgatgactttggcaccggtttgtcaaacctgaaacgtttttatgaaattaatccagacagcataaaggtggactcgcaattcaccggcgatattttcggtactgcgggaaaaattgtgcgcattattttcgacctggcacgctataaccggatcccggtgattgcggaaggcgtagagagcgaagacgttgcgcgcgaattaatcaaattaggatgtgttcaggctcaggggtatctgtaccagaaacccatgccattctccgcctgggataaaagtggaaaattagtaaaagagtagtttacgtatgtccagaatcaataagttcgtacttacagtcagtctgctgatttttatcatgatttcagcagttgcctgcgggatctacactcaaatggtaaaggaacgggtgtatagcctgaaacagtccgttattgatactgcttttgcggtggcaaatattgctgaatatcggcgtagcgtggcaattgatcttatcaacacgctaaatcccacggaggaacagctgttggttggtttgcgcacagcttacgccgactcggtttccccctcttatttgtacgatgtcggtccttatctgatttccagtgacgaatgtattcaggtaaaggagttcgagaaaaattattgtgcagatattatgcaggttgtgaagtatcgacatgtcaaaaatacagggtttatctcttttgacggtaaaaccttcgtctattacctctatccggtaactcacaatcgtagtctgatatttttgcttggtctggagcgtttttctttactgtcaaaatcgctggcgatggacagcgagaacctgatgttctctctatttaagaacggtaaaccggtgaccggtgatgaatataatgctaaaaacgccatcttcaccgtttcggaagcgatggagcacttcgcctatttgccgaccggattgtatgtatttgcgtataaaaaagatgtttatttgcgggtttgtacattgattattttctttgccgcattggtggcagtgatatcgggtgccagttgcctctatctggtacgcagagtgattaatcgtggtattgtggagaaagaagccatcattaataaccattttgaacgcgtactggatggcgggcttttcttttcggctgccgatgtcaaaaaactctacagtatgtataactcggcgttcctggacgacctgaccaaagcaatgggcagaaaatcctttgacgaagatttaaaagcgctgccggaaaaaggcggttatttgtgcctgtttgacgtcgataaattcaaaaacattaacgacaccttcggtcatttgctgggcgatgaagtgttgatgaaagtggtgaaaatccttaaatcacagatcccggtagataaaggtaaagtctaccgcttcggcggtgacgaatttgcggtgatttatacgggtggaacgctggaagagttgctatcgattctaaaagaaatcgttcatttccaggtgggaagcattaatttaagtaccagtatcggtgtagcacattcaaatgaatgtcctaccgtcgaacgcttgaaaatgctggcggatgagcggctgtataagagtaagaaaaacggcagggcacagattagctggcagtaatcattattcgcaggccggacaaatgattttgcccggcctgaattaattaaacccggctaccccacaaatcgtactcatcggcgtgctcgactttcacacgcaggatatcacccggcttaacgttggtttcaccattgagataaaccgcgccgtcgatttccggtgcatctgccatgctgcgaccaatcgcgccttcttcgtccacttcgtcgataatcaccagaatttcacggcccactttctcttgcaggcgctcggcggaaatctgctgctgcagctgcatgaaacggttccagcgttcttctttaacttcttccggaacctggtcaggcagggcattggcgtctgcaccttcaaccgggctgtatttaaagcagccaacgcgatccagacgcgcttctttcaggaagtcgagtagcatctggaaatcttcttctgtctcgccagggaagccgacaataaaggttgagcgtagggtcagttccgggcagatttcgcgccactgtttgatgcgcgccagttggcgatctacagaacccggacgcttcatcagtttgagaatgcgcgggctggcgtgctgcaacggaatgtccagatacggcaggattttgccttctgccatcagtgggatgacgtcgtccacatgcggataagggtaaacgtagtgcagacgtgtccagatccccagtttcgataactgttcgcacaggctgaccatgctggtttttaccggctcgccgttgtggaagccagtacgatgtttaacatcaacgccataggcggaagtatcctgcgagatcaccagaatctctttaacgcccgcatctaccagacgtttcgcttcacttaacacttcgccaatcggacggctcaccaggtcgccgcgcatagacggaataatgcagaaggtgcagcggtgattacagccttcagaaattttcagataggcataatgacgcggcgtcagtttcacaccttgttctggcaccaggctcaggaatgggttgtgtttcggttttggcacgtagtgatgaacgtgctccagaacctgctcatagctatgaggcccggtgatttccagcactttcgggtggacttcgcggatctgatcttcttttgcccccagacaaccggtcacaataaccttgccgttttcattcaacgcttcaccaatggcttccagtgattcttgtaccgcgctgtcaataaagccgcaggtgttgacgatcaccatgtccgcatcgtcatagctcggtaccacgtcataaccttcagtgcggagttcggtgagaatacgctctgaatcaacaaggtttttcggacagccaagggaaacaaagccgattttcggctggggagttactttgctcatagcttaaaaaatattcagttacaggaaaggtcagggcagggattctacagagttctggataaaatttgtatcgcaatctcattcgctggcggaggcgaaggaaatgtaaattttgttaattcggcgtgaagaattgatcctggacagcattttgctcaaaaaatagccatactatttaattgcaacaaggctgggaagaggaggatcgaagtatgttcgttgacagacagcgaatcgatctgctgaaccggttgatcgacgcacgcgttgacctcgccgcatacgtgcaactgaggaaggcaaaaggatacatgtccgtcagcgaaagcaatcatctacgagataacttttttaaactgaatcgcgaactgcacgataaatcgctgcggttgaatcttcatctggatcaggaagagtggagtgctcttcatcatgctgaagaagcattagcgacagccgcagtatgtttgatgagtgggcaccatgattgcccgactgttattaccgtcaacgccgataagcttgaaaattgtctgatgagcttaacgctgagtatccagagcctgcagaagcacgccatgcttgagaaggcctgaaaactaagggggagaaagcgtctcccccttcatgtttaagtttttgtaaaaatgaatttgttatctcctccactgactacgctttaagccagagtcaatccggaggcgttatgcatcgacaatcctttttccttgtgccccttatttgtctttcttccgctctctgggcggctcctgcaacggtaaatgtcgaagtactgcaagacaaactcgaccatccctgggcactggcctttttacccgataatcacggtatgttaatcactctgcgcggcggcgagttgcgtcactggcaagcaggaaaaggattatctgcgccgctttccggagttccggacgtttgggcgcacgggcagggcggcctgctggacgtggttttagcgcctgattttgctcagtctcgccgcatctggttaagttattccgaagttggcgatgatggcaaagccggaactgctgtgggttatggccgcttaagtgatgatctctcaaaagtgaccgacttccgcaccgtctttcgccagatgccaaaactgtctaccggcaaccattttggcgggcggctggtattcgacggtaaaggttatctttttattgctctgggcgaaaacaatcagcgcccgacggcgcaggatctggataaattacagggcaaactggtgcgtctgaccgaccagggcgaaatcccggatgataatccttttataaaggaatccggtgcgcgcgccgagatctggtcttatggcattcgtaatccgcaaggaatggcgatgaatccgtggagtaatgcactgtggctgaatgaacatggcccgcgcggtggtgatgaaattaatatcccgcaaaaaggcaaaaactacggctggccgctggcaacctggggaatcaactattcaggctttaagataccggaagcgaaaggggagatcgtcgccgggaccgagcaacctgttttttactggaaagattcgcccgctgtgagcggcatggccttctataacagcgataaattcccccagtggcagcaaaaattatttattggcgcgctgaaagataaagatgtcattgtgatgagcgtcaacggcgacaaagtgacagaagatggccgtattttaacggacagagggcagcgaattcgtgatgttcgcactggacccgacggttatttatacgttctcaccgacgagtccagtggggaattacttaaagttagcccacgcaattagctaacgggaatcatcaccactttgcgcactgcggggcgttcagtgagttgctgataccagcgttgcagatttggacgcggtgtccaggtcaggccaacgttaaacaaattgtagatgaacggtgcgatagcgatatcgcccacaccaaactcgtcgccagagaaccattttacttttgccagttccgcatcgagcagggcaaacagggcgtcgcactctttgcaactggcatcaatggcggcctgatcgcgctcttccggtggtgttctgactaatcccatcaggatcccgcgatgagcattactgagcgtctggtttgcccagtccatccatttttccgcttccgcacgacgtgccggtgagtcgatccacaggcgtttttgcccgtactgtgccgccagatagcggacaatggcgtttgattcccaaagaatgagatcactttcgtcgtcacgcaacaacggcaccagcccgttagggttcatcgccagaaaatcagcatcgtgatttatcccaaactcacggcccgcgagaatttgctcataaggtagttccagttcttcgagcgtcagcaatactttttttacgttagttgaattattccgaccccacagcgtaatcatactcaccccttttccgacaggcagccacaggctgaacaggactccgatggtgaagtaaagttaacttttaagcaacagctggcaaaaaaatgacaccagaagcagcgaagcggcaggatattgcataaactttaaaaactttaccaacttacggtttctttaagtttgtgtgtgcgttattaatcaccaaacttatcatacggcgatataacgtattttttttgaatggatactcgggtggcatttatgacgcaatactcctctctccttcgtggtcttgcagcgggttctgcatttttattcctttttgccccaacggcattcgcggcggaacaaaccgttgaagcgccgagcgtggatgcgcgtgcatggattttaatggattacgccagcggtaaagtgctggcagaaggcaatgcggatgagaaactggatcccgcgagcctgactaaaatcatgaccagctatgtggttgggcaggcgcttaaggccgataagattaaactcaccgatatggtgacggtcggtaaagatgcctgggcgacgggaaatccggcactgcgtggttcatcggtaatgttcctcaaaccgggcgatcaggtttcggtggcagacttgaacaaaggtgtgattatccagtccggtaatgacgcctgtattgcgctggctgattacgttgccgggagccaggagtcatttattggtctgatgaatggttatgccaaaaaactgggtctgaccaacactaccttccagacggtgcacggcctggatgcgccggggcagttcagcaccgcgcgcgatatggcattgctgggtaaagcattgatccacgatgtgccggaagagtacgccattcataaagagaaagagttcaccttcaacaaaattcgtcagcctaaccgtaaccgtctgctgtggagcagcaatctgaatgttgatggcatgaagacaggaaccacggcaggcgcgggatataatctggttgcttcggctacccagggcgatatgcgtttaatctccgtagtgttgggggcgaaaaccgaccgtatccgttttaatgagtctgagaaattattgacctggggtttccgcttctttgaaaccgtgacgccaattaaacctgatgccacctttgtgactcagcgcgtctggtttggtgataagagcgaagtgaatctcggggcaggtgaagcgggctcagtgaccataccgcgtgggcagctgaaaaacctgaaagcgagttatacgttaacggaaccgcagcttaccgcaccgctgaaaaaaggtcaggttgtcgggaccattgatttccagcttaacggtaaatccattgagcagcgtccgctgatcgtgatggaaaatgtggaagagggcggattctttggtcgggtgtgggatttcgtgatgatgaaattccatcagtggttcggcagctggttctcttaatcttctgataaccggatggcgcgaaacgtcatccggttatacgtcattaatacatcaacttaatgcgctgcgtctgcgcgtacttcacatactcatcttccgggcaacaatcgctcaccacaatatcaaagcgtttcaggtcacccatgcgcgccggacgcaccttgccaaatttactgtggtcgacaaccagcacatgcttttgcgccatcgacatggcccagtgttttaccggcaactcttcaagattaaaacaggtagcgcctttactgacatgcacgcccgccgcagaataaaaagcgatatccgggcaaaaattattcagcgtttgctgaaaatcgatgggtttgaaaatggcgttgctggcgtgaaattcaccaccgcaaagaaacgcgcggcaatggggtttctctttcagcgccagaaaggtatttagcgaataacaaacggcggtaaaagggatttcattatcaatcgcttcaataatccacggcgtggtggtgccacagtcaaaaaagagggtctgatcgggttctaccagcgtcgcagccagttttgccgcccggcgtttttcttccaccaggcgggatttttgatcgcttaacaggtaatggctggcactgcgcggttccagaacaatatagccgccgagcaaaacgacgggcgcactgtggttgttcagatcgcgacgaatcgtcatctccgaaaccccaagcagggcggcggcgtctttaagatgtaacttatcgctgcgttttaattcttgcagcagctgcccgatacgctcttcgcgacgtgtttccataatccctctgaatagttattgaagcgagccgctcaatactacactttttagcagagatcagtcacgcacccagcctttgcggatcggtaatgcaaaacagacgcgataccacgattgcagacgttgatagagtttatgccccatcgcttgccagataatctgggcactaaggcagccaatcatacctgccagcaatccaccgagcatatccagcggccagtggacgccaagataaacgcgcgaccaggcaatgacgacggccagcaccattaaaagtgagccggaccacaggcgatgccagcataaaaatgccagtgcaaaggtgaaaatcaccgtaccgtgatcgcttgggaatgagtcatccgccgcatgatgcaggaagttatagccgatattttcgacaaagggtcggtcgtgcggaaaaagatgtcccatcgtccaggacacaaacaggctgaccgccagcgcgatagcgatttttatcaccagttgccgttgtgctgtaagcccccacaaccaaagtaccacggccagcaacggcaccacggtaatcaaatctttagcaataaaaatcgccaacgagatcatccacggagccgagtctggcgtcgcgttaataagagagaatagagagagattcaaattttccagcataacttcccgacgcaaagtgattaaaagggagccaatacaggcaagtcgttgagaataaagtgcaggttaaactgggtaaagcggcatcgtcttatttccctcaagcggcctgtttacggtgggtgattgtaacgggcataggttaaataaaacttaaagaaagcgtagctatactcgtaataatgtaagaatgtgcttaaccgtggtttcagctacaaaattcgctttctcgttagctgcgcttttattaaactctgcgcgattattattggcgaagaaattgcatgcaaaataaattagcttccggtgccaggcttggacgtcaggcgttacttttccctctctgtctggtgctttacgaattttcaacctatatcggcaacgatatgattcaacccggtatgttggccgtggtggaacaatatcaggcgggcattgattgggttcctacttcgatgaccgcgtatctggcgggcgggatgtttttacaatggctgctggggccgctgtcggatcgtattggtcgccgtccggtgatgctggcgggagtggtgtggtttatcgtcacctgtctggcaatattgctggcgcaaaacattgaacaattcaccctgttgcgcttcttgcagggcataagcctctgtttcattggcgctgtgggatacgccgcaattcaggaatccttcgaagaggcggtttgtatcaagatcaccgcgctgatggcgaacgtggcgctgattgctccgctacttggtccgctggtgggcgcggcgtggatccatgtgctgccctgggaggggatgtttgttttgtttgccgcattggcagcgatctcctttttcggtctgcaacgagccatgcctgaaaccgccacgcgtataggcgagaaactgtcactgaaagaactcggtcgtgactataagctggtgctgaagaacggccgctttgtggcgggggcgctggcgctgggattcgttagtctgccgttgctggcgtggatcgcccagtcgccgattatcatcattaccggcgagcagttgagcagctatgaatatggcttgctgcaagtgcctattttcggggcgttaattgcgggtaacttgctgttagcgcgtctgacctcgcgccgcaccgtacgttcgctgattattatgggcggctggccgattatgattggtctattggtcgctgctgcggcaacggttatctcatcgcacgcgtatttatggatgactgccgggttaagtatttatgctttcggtattggtctggcgaatgcgggactggtgcgattaaccctgtttgccagcgatatgagtaaaggtacggtttctgccgcgatgggaatgctgcaaatgctgatctttaccgttggtattgaaatcagcaaacatgcctggctgaacgggggcaacggactgtttaatctcttcaaccttgtcaacggaattttgtggctgtcgctgatggttatctttttaaaagataaacagatgggaaattctcacgaagggtaaaaaaatgcctgactgctttgtgcgatcaggcattctcgaattaatggtgatggtcgtcaatctggtgttcgataaccatcccttcacctacgctggcaagatggcgaacataaggatgcgggcggtaagccggagctggcgcaggagccacatagacggtttgcggcacagtcgcgacgctgaccgcttgtggaacgctgactgaatcaggaaccacaaccactttgtatccactcggcacatcgacggtgacactttgcgccatcgccacaccagtaaagcccattaaaagcgcgcccaacagtagacaatttttcataatcatttcgcctgaaataatgcagcgggttaatttccgcgaattatgcagccttcattcaggcattgtgttgccgggcgtgctgccggttttattggtcaaatggcgcttcgtgtttaagaactttatcgatcacatccagtacgccttcacggttattggagcctgcgcggtattttgccgctgcgacgaccgcgctaccggcattttccattgcaaaactaaagcctgcctgacgcagcatctcaatatcgttaccgccatcgccaaagaccaccacttcgctgtcgtctattccccataatttctgcagttggcgaaggccattggctttatgtacgccggggataatcagatcgatgctgccgttgccggtgtggaccgacaccataatatcgccgatggcctcatgtaatgctttttgtacttgtggaatcagttcatcggaaagattcaggccaaacttaaagaagatatcctctaagttgtcaaagttatcgacgtattccagacggtgataatacatttccgccaccgttttcatggcatcgtcatattttttgagtgtataggcactattttttccgcaggcaataatttccacttccgggcgcgtcagcaaatgttccacgacagtagcaaacgcatccttcgatagctcgccattaaaaacatctttgccttcgctcactacccagccgccgttttcagccacaaaggcaatttcattagcaatttcagggaagaaagagatcaactgataatattgattcccgctggcgactacaaagcgaattccttgtgctttcatttgctgatactgagccataaaccgctcacggttataggttttttgatcgcttaagaaagtaccatccatgtctaccgcaattaatttaatgctcatcaactattctccatcgccgtctgcgttttggtatcgggtttggcgacggctttcgcgacaatagccgcgagaataaccagcgccagtacaaccagcattgcactacgtaatccataatgttcgccgagatagcccagcagcggcggcccgacgaggaaagccagataaccggtcgttgctaccacactgacgcgggttggtgcatcggggccggtatcgctggcggcagaaatggtcagcgggaagcccagcgaggcacccagtccccagagtacaacagacaccccagcgacccaggcgctatcgacaaaaataatcagcccaatacccaacgcccccattagtgcactggcccgaaccacggcaacgcgactgtaacggtcgatgaaccaaccgccggtgaagcgtccaacggtcatccccagggtaaaaccggcataaatcagcgagccggaagtagggctaaaaccgtgaccgtcaaccattaataagggtaaccagtcgttggcagaaccttcggcaaaggccatcgccagcaccacaacacctatcagcagcaactggatatcgcgataaaaaggtacgcctttttcgccatgctgggtgccatcggcagcatttttgcccgtaccgtcagggattgcctgaatggcgatataaataggtgcgatacctaccagcgccgccaataaaatgtgcaccgttgccggaacgccaaaggccgtcagtgccatcccgacacctgcgcctgccagcgtgcccaggctataaaaaccgtgcatcatcggcaaaaccgtcttattcatttctcgctcaacggcagcaccttcaacgtttatcgccacttccgcagaaccaaaacttgccccaaagacgccgagaccaacggcaaagagcaggggcgatgtcagccagagtgccagacttaatatcatcatcccgatcaatgcgcaggacatcgtgaccaggatgacattacgtgtcccaaagcgtttcactaaccacgccgagcagagaataccgctcatcgaaccgatcgacagaccaaagagaacaccgcccatttcagcgatcgagacagagagaatatcgcggatagcaggcgtacgggttgcccaggacgccattaacaggcctggcaaaaagaagaacataaacagcgcccaggttcggcgtttcaatgcattacgtgaagaatttacggtcatagatcacgtcaaaataagaagagggaagacaacattagcaaggttgtgtacatttgtacacaattgcagagagaggaaatgacatgcgtcgcgctaacgatccgcaacggcgagaaaaaattatccaggccacgctggaggcggtgaaactttacggaatacatgctgttacgcaccgcaaaattgctacccttgccggggtaccgttgggatcgatgacctactatttttcaggaattgatgagttgttactggaggcgttcagcagttttactgagatcatgtcccggcaatatcaggcattttttagcgatgttagtgatgctccgggcgcatgccaggctatcaccgatatgatctacagctcacaggttgcaacgccggataacatggagctgatgtaccagctctacgcgctggctagccgaaaaccgctattaaaaacggtaatgcaaaactggatgcagcgcagtcagcaaacgctcgaacaatggtttgaacccggaaccgcccgcgcgcttgatgcgtttattgaggggatgacgctgcattttgtcaccgaccgtaagccgctatcgcgcgaggagattttgaggatggttgagagggttgcagggtagtagataagttttagataacaaaaaacccatcaaccttgaaccgaaatggcggggttgatgggctccacaaaatggggacatcaaagaaaagcagtggcactaattaagactgatgccctgcggaaaagttctgcggttgtgcaaaaaaatttcattttcagggcaacttcagttttatcctaatcctggccataccatgacgatgattgtccctgccagcgtcagcaggacgttggcgattgcataggtgcccgcatagcccagcgccgggatgttactgcgagctgtatcactgatgatctccattgccggcgcgcaggtacgtgcgcccatcattgcgccgaacaacagcgcgcggttcattcgcaatacataagcaccgaacaagaaacagataaccacgggcaccagactgacaatcaatccggcaatcaacatctgaccgccaatcgcgcccaggccgttattaataccgctaccggcgctcagaccaacgcctgccataaacaccatcaagccgaactctttcaccatgcttaatgcaccctgcggaatgtaaccgaaggtcgggtggttagcacgcataaagcccagcataattccggcgaataacaacccggcagcgttccccatgccgaaactgaatgtgctgaactggaaggtgatcatcccgatcatcagcccaataacaaagaaggcgcagaatgccagcaggtcagtgacctggctgtgaatcgagataaagccgatgcgatcggcgatggtttttacgcggcgggcatcgccgctgacttgtaaaacgtcacctttgttaagcacgacgttgtcatctatcggcatctcaatctggctacgaatgacgcggttaaggaagcaaccgtgatcggtcaacttcagttgtgcgagacgtttacctacagcgttatggtttttaacgaccacttcttcagtgacgatacgcatgtcgagaaggtcacgatcgaaaacttctttaccgttacggaagctgggatcgagtcgggcatgggcgtcgggatagcctaccaacgctatttcatcgcccatttgtagcacggcatcaccgtctggatttgccagaatcccgttacgtcgaatacgttcaatgtagcagccggtttgtcgataaatacccagttcacgcagatttttgccgtcggtccaggccaccagttccgggccgacgcgataggcgcggatcaccggtaaataaaccttacggttggcatcagtgtccaggccacgttcgcgggcgatttgctgggcgctggtctgtaagtcctgatgctgcaatttcggcaagtaacgcgcaccaacaatcaaactcaccagaccgattaaataggttaaggcatacccgaggctcagattatccagtgccagtgagagctgcctgctttccatgccggaatgacgcagtgtatcgccagcaccgaccagaaccggtgtcgacgtcatagagcctgctaacataccggccgtcaggccaatatcccagccaaacagcttacctaaccctaaggcgatcaccagcgcactgccaaccatcaccagtgctaacattaggtaatttttcccatcgcgaaaaaaaatggaaaaaaagttcggtccggcttcgaccccgacgcagaaaataaacagcataaagccaagattaagcgcatcggtgttaatgctgaaatgttgttggcctaataacagcgatacgactaaaacgccaatggaattacccagttggatcgaaccaagtcgtaactttccgagacatagcccaagcgcgaggaccacaaataataacagaatgtaattcccatttaacaattcggcgacgtttatattcacggaggctaacttcttgtttactagtaagctgttgaaagaaatggtaatttacgataatgttttttaccagaattcagggcgcagattcattcagcgcacctaaacgatagtaaagtaacaatatattttactagtgtaatcacattaggtatcaacggctatatgaattgcgttggcctatattagcatggaatgcgaagcggctttatcttactgaacgccacactggcgaaaaatgtgttcgatagacgcagtgtcaggaggaacgagtgaaacataaacaacgttgggcgggggcaatctgctgttttgtcctcttcattgtggtgtgcctttttctggcgacgcacatgaaaggcgcttttcgggctgccgggcatcctgaaatcggcttgctatttttcattcttcctggagcagtcgccagcttcttttcacagcgtagagaagtcctgaaacctctgtttggcgcaatgctggcggcaccctgttcgatgctcattatgcggctgtttttttcaccgacgcgctcattctggcaagagctggcatggttactaagcgcggtgttctggtgtgcgctgggggcactgtgtttcttatttatcagtagtttgtttaaaccacagcacagaaaaaatcagtaaagccctcaacgcgagggcttgtcagacgatcaggcgtccagattttctttcacccatgcagcaaaatcggtatagccgccgatatgttgctgatcgacaaaaatctgcggcacggtttctacgggtttacctgccttttgttgtagatcttctttagtgatcccttccgcacgaatatctacatactgatactgaaaatcatcgcgttcattgctcaatttctcagccagatcttttgcacgcacacagtaagggcaacccgaacgaccaaaaataacggtttgcattatttctctcctcatagatttatgcctgtaatgatcacgctaaaatgtattcgctgaaagtaggtttaacctgttgcattaattgctaaaagctataactgttaaacacaatacagtgaaaagttttagactgaaggctcactttgcagagggaagcgtatgcgcgcgatcggtaaattgcctaaaggcgtgttgatactggaatttatcggaatgatgctactggcggtggcgctgctgtcggtaagcgactccctgtcgctgcctgagccattttctcggccagaagtgcagattctgatgatttttctcggtgttttgctcatgcttcccgctgcggtggtggttattcttcaggtggcaaaacgtcttgccccacagctgatgaaccgtccaccgcaatattcacgttcagaaagagaaaaagataatgacgccaaccattgaacttatttgtggccatcgctccattcgccatttcactgatgaacccatttccgaagcgcagcgtgaggcgattattaacagcgcccgtgcgacgtccagttccagttttttgcagtgcagtagcattattcgcattaccgacaaagcgttacgtgaagaactggtgacgctgaccggcgggcaaaaacacgtagcgcaagcggcggagttctgggtgttctgtgccgactttaaccgccatttacagatctgtccggatgctcagctcggcctggcggaacaactgttgctcggtgtcgttgatacggcaatgatggcgcagaatgcattaatcgcagcggaatcgctgggattgggcggggtatatatcggcggcctgcgcaataatattgaagcggtgacgaaactgcttaaattaccgcagcatgttctgccgctgtttgggctgtgccttggctggcctgcggataatccggatcttaagccgcgtttaccggcctccattttggtgcatgaaaacagctatcaaccgctggataaaggcgcactggcgcagtatgacgagcaactggcggaatattacctcacccgtggcagcaataatcgccgggatacctggagcgatcatatccgccgaacaatcattaaagaaagccgcccatttattctggattatttgcacaaacagggttgggcgacgcgctaaaaccgccacgtcgatgtatgatacgcgggcttttgaccaggtctgacagagaggtgcagggtgaaaattgccatattgtcccgggatggaacgctctattcgtgtaagcggctgcgtgaagccgctatacagcgcggtcacctggttgaaattcttgatccgctttcttgctacatgaacataaatcctgcggcgtcttctattcactacaaaggccgcaagttaccccattttgacgcagtgatcccgcgtattggcaccgccattaccttttatgggacggcggcactgcgccagttcgagatgctggggagctatccgctcaatgagtcggtcgccattgcccgggcgcgtgacaaattgcgttccatgcaactgctggcgcgtcagggcatcgacctgcctgtcacgggcattgcgcattcgccggatgataccagcgatttaatcgacatggtcggtggtgcgccgctggtggtcaagttggttgaaggcacgcagggaattggcgtcgtgctggcggagacgcgtcaggcggcggaaagcgtgattgacgctttccgcggtctgaacgcgcatattctggtgcaggaatatatcaaagaggcgcaagggtgcgatatccgctgtctggttgttggcgatgaagtggtcgctgcgattgaacggcgggcgaaagagggcgattttcgttccaatttgcatcgtggcggcgcggcaagcgtcgccagtatcacaccacaggagcgtgaaatcgcgataaaagccgcgcgaacgatggcgctggacgttgctggtgtggatattctgcgtgctaatcgcgggccgttggtgatggaggtgaatgcgtcgccggggctggaaggaatagaaaaaaccaccggtatcgacatcgcgggtaaaatgatccgctggatcgaacgccacgctacgacagaatattgcctgaaaacgggtggttagtcgcaatcacattactgatcatggttttgcctgcgctttttgcgtaagctgtgccggtctttttatcgaaagaggttgtacaaaattatgacatcgctggtcgttcctggtctggatacgctgcgtcaatggctcgatgacctggggatgagtttttttgaatgtgataactgtcaggctctgcatctgccccatatgcagaatttcgacggtgtctttgatgccaaaatcgatctgatcgataacacgatcctgttttctgccatggcggaagtccgaccttcagccgtattgccgctggcggcggatttatctgccatcaatgccagttcgctgaccgtgaaagcatttcttgatatgcaggatgataatctgccaaagctggtggtttgccagtctttatccgttatgcagggcgtaacctatgagcagtttgcatggttcgtgcgtcagagcgaagagcagatttcgatggtcattcttgaagctaatgcccatcaactgctgttaccgactgatgatgaagggcaaaacaacgttaccgaaaactatttcctccactgataactcctttcgagcacgcagtcgctggtgcagtggctgcgcgctgcaaaattatctgctgtttttaaccttttcttaaagattatttcacttctcttgtgtcgatttggctttatcacatagagcaaatatgcataaaaatttgttaaataccgttttttaatccgagctatagtctcaaaccctggctaaagttattcttgcgatgcttttatatagcgagcagtgctggccgggagaaagttctcttttcttacaccgcgccgataaaaaatatgcacgtttattgcatatctttcagtgtgacaacttttgttcgtttgttaacgaactttcagaaggaaagagatatgaccgccttaaataaaaaatggctatcgggtctggttgcgggtgctctgatggccgtctctgtcggcacgctcgcggctgaacaaaaaacactccacatttataactggtctgattatatcgccccggacacggtggccaattttgaaaaagaaaccggtattaaagtcgtctacgatgttttcgactctaacgaagtactggaaggcaaattaatggccgggagtaccggctttgatctggtggttccatctgccagctttctggagcgccagttgactgcgggagttttccagccgctggacaaaagcaaattgccggagtggaagaatctcgacccggaactgctgaagctggtcgccaaacacgatcccgacaataaatttgctatgccctatatgtgggcgacgaccgggattggctataacgttgataaagttaaagcggtgctgggcgaaaacgcgcccgtcgatagctgggacttgatcctcaaacctgaaaatctggaaaaactgaaaagctgcggtgtctctttcctggatgcgccagaagaagtttttgctaccgtgttgaattatctcggcaaagatcccaacagcactaaagcggatgattacaccggaccggcaacagatctgctgttaaagctgcgcccgaacattcgttatttccattcatctcaatacattaacgacctggcaaacggcgatatttgcgtcgctatcggctgggcaggtgatgtctggcaggcgtcaaaccgcgcgaaggaagcgaagaatggcgtgaatgtctcgttctcgattccaaaagaaggggcgatggcgttctttgatgtattcgccatgcctgcggatgccaaaaacaaagacgaagcctatcagttcctgaattacctgctgcgcccggatgtagtagcgcatatttccgaccatgtgttctatgccaacgccaataaagcagccacgccgctggtgagtgcggaagtccgtgagaacccaggtatttatccgcctgcggatgttcgtgcgaagctgttcactctgaaagtgcaggatccgaaaatcgaccgtgtgcgcacccgcgcgtggaccaaagtgaagagcggaaaataatccgcagtcgtagatgccggaggggcgcaccacacccgccggcaattcgcaccattatggtgcgcttgcacacattcaatgccggagagcagccgtgaatgacgctatccctcgcccgcaggcgaaaacccgtaaggcgctgacgccgctattagaaatccgcaacctgaccaaatcctacgatggtcaacatgcggtggatgatgtcagcctgaccatctacaaaggtgaaatcttcgcgctgctgggcgcatccggctgtggcaagtccacgctgctgcgtatgctggcaggtttcgaacaaccttctgccggacagataatgcttgatggcgtcgatttgtcacaggttccgccttacctgcgccccatcaatatgatgtttcagtcttacgcgctgtttccgcatatgaccgtggaacagaacatcgcttttggcctgaaacaggacaaactaccgaaagcggaaattgccagccgggtcaatgagatgctcggcctggtgcatatgcaggagttcgccaaacgcaaaccgcatcagctttccggtggtcagcgacaacgtgtggccctggcccgaagccttgcgaagcgcccgaaactattactgctcgatgagccgatgggcgcgctggataaaaagctgcgtgacaggatgcagcttgaagtggtggatattctggagcgcgtcggtgtgacttgtgtgatggtcacccacgatcaggaagaggcgatgaccatggcggggcgcatcgccattatgaatcgtgggaaatttgtccagattggcgaaccggaagagatctacgagcatccgactacccgctatagcgccgaatttattggctcggtaaacgtctttgaaggcgtactcaaagagcgtcaggaagatggcctggtgcttgattcgccggggctggtgcatccactgaaagtcgacgcggatgcctcggtggtcgataacgtgccggtacatgtggcgctgcgcccggaaaaaatcatgctttgcgaagagccgcccgccaatggttgtaacttcgcggtgggggaggtgatacacattgcctatctcggcgatctttcggtgtatcacgttcgtctgaaaagtgggcagatgattagcgcccagctacaaaacgcccatcgtcatcgtaaagggttaccgacctggggcgacgaagtgcgtttgtgctgggaagtggacagctgtgtggtgctgacggtttaaggagcaaagatgagtacacttgaacctgctgcccagtcgaaaccgccgggcggatttaagctgtggttgtcgcagctgcaaatgaagcatgggcgcaaactggtcattgcgttgccatatatctggttgatcttgctgtttctgctgccatttctgattgtctttaaaataagcctggcggagatggcgcgcgctattccaccttataccgaactgatggagtgggctgacgggcaactgtccatcactcttaatctcggtaattttctgcaactgaccgacgatccgctctatttcgatgcttatctccagtcgctacaggtggctgcgatttcgacattttgctgtttactgatcggctatccgctggcgtgggcggtggcgcacagtaagccttcgacccgtaatattttattactactggtgatcctgccgtcgtggacctcgtttctgatccgcgtttatgcctggatgggaatattaaaaaacaacggtgtgctgaataattttctgctgtggctgggggttatcgatcaaccgctgaccattctgcataccaatctggccgtttatatcggcattgtttacgcttacgtgccgtttatggtactgccgatttataccgcgttgattcgtattgattattcgctggtggaagcagcgctggatctcggtgcacgaccgctgaaaacgttctttactgtgatcgtgccgctgactaaaggtgggattattgccggatcgatgctggtgtttatcccggctgtgggcgagtttgtgatcccggaactgctcggtggcccggacagcatcatgatcgggcgcgtgctatggcaagagtttttcaataaccgcgactggccggtggcctcggcggtagcgatcatcatgttgctgctgctaattgtgccgataatgtggttccacaaacaccagcaaaaaagcgtgggagaacacggatgaataatttaccggtagttcgttcgccctggcggattgtgattttgctgctgggctttacctttctctacgcgccaatgctgatgctggttatctattcgtttaacagctcgaagctggtgacggtgtgggccggctggtcaacgcgctggtatggtgagttattgcgcgatgacgcgatgatgagtgcggttggtttaagtctgacaattgcggcctgtgcggcgacggcggcggcgatcctcggaactattgcggcggtggtgctggtgcgctttggcaggtttcgcggatcaaatggctttgcctttatgatcaccgcgccgctggtaatgccagatgtcatcacgggcttgtcgctgttgttattattcgtcgcgcttgctcatgccattggctggcctgcggaccgcggtatgctcaccatctggctggcgcatgtcactttttgtacggcttatgtggcggtcgttatttcttcaagattgcgggaactggatcgctcgatagaagaagcagcgatggatctcggtgcgacgccgctgaaagtgtttttcgtcattacgctaccgatgatcatgcccgcgatcatttctggctggttactggcttttactttgtcgcttgatgatctggtgatcgccagctttgtttccgggccgggagccaccacgttaccgatgctggtcttttccagcgtgcggatgggggtgaatccggaaatcaacgccctggcaacattgatcctcggcgcggtcggaattgtcggatttatcgcctggtatctgatggctcgcgcagaaaaacagcggatacgcgacatccagcgtgcaagacgtggctgaagacactaaaatttgccaacctggctacataatgccgcgcatgtcgcggcattgttttcatggaagacgaaacgttgggattttttaagaaaacatcttcatctcatgctcgcctgaatgtgcctgcgctggtgcaggtggcggcgctcgccattattatgatccgtggcctcgacgtgctgatgattttcaatacgctgggcgtgcgcggtattggcgagttcattcatcgcagcgtacaaacctggagtttaacgctggtctttttaagcagtctggtgctggttttcattgagatctggtgtgcgttttcactggtgaaagggcgtcgctgggcgcgctggctatatctgctgacacaaatcaccgccgcaagttacttgtgggcggcttcgctggggtacggttatccggagctgttcagcattcccggtgaatcaaaacgtgaaatcttccatagcctgatgctgcagaagctgccggatatgctcatcctgatgctgctgttcgttccctcgaccagtcggcggttcttccagttgcaataatgtgtataatcgtcgcccctgatgatgtgaaggtcaatgtatgcagtgcgcactttacgacgcgggtcgctgtcgttcctgtcagtggataatgcagccgattccagagcaactctccgctaaaaccgccgatcttaaaaatctgctcgccgactttccggttgaggaatggtgcgcgccggtgtcaggcccggaacaagggtttcgtaataaagccaaaatggtggtgagtggtagcgttgaaaaaccactgctcggtatgctgcatcgcgatggcacaccagaagacctttgtgactgcccgctttatcctgcctcatttgcgcccgtttttgcggcgctaaaaccgtttatcgcccgagcggggttaacgccctacaacgtggcgcgtaagcgtggcgaactgaaatacattctgctgactgaaagccagagtgatggaggcatgatgctgcgctttgtactgcgttctgataccaagctggcgcaactgcgtaaggcgctgccgtggttacacgaacaactaccgcagctgaaagttattaccgtcaatattcagccggtacatatggcgattatggaaggggagacggagatctacctgaccgaacaacaggcactggcggagcgttttaatgacgtaccgctgtggatccgtccgcaaagtttcttccagactaatccggcggtcgccagccagttgtacgccaccgcgcgcgactgggtacgacagctgccggttaaacatatgtgggatctgttctgcggtgtggggggctttggtttacactgcgcgacgcctgacatgcagttaaccgggatcgaaattgcatcagaggccattgcctgtgcaaagcagtcagccgctgaactgggcttaacgcgtttgcaatttcaggcgctggactccactcagtttgccaccgctcagggggatgtgccggagctggtgctggttaacccgccgcgccgcggcattggtaaaccgctgtgtgattatctctcaacgatggcaccgcgttttatcatctactccagctgtaacgcccaaactatggcgaaagatatccgcgaactgcctgggtttcgtattgaacgggtgcagcttttcgatatgttcccgcataccgcgcactatgaagtgctgacgctgctggtgaagcaataaaaaagccgcatgtgcggcttcagattgctgacaaagtgcgcgttgtttatgccggatgcggcgtaaacgccttatccggcctacaaaagcgtgcaaattcaatacattgcatgggccatgtaggcctgataagcgtagcgcatcaggcaattttacctttgtcatcagtctcaagccgcggttgcggctttctgaatcttactgtgggaaccactggtcactgattttttgataagtaccgtcagctttaattgctgccagcgcgttattcagtttttccagcagggctttgttatccggacgtacagcgatgcccaggccggtgccaaaatattgcggatcggtcactttctcagtagcaacaccaagttgtggattggttttcagccattcgtttaccaccgctgtgtcaccaaataccccatcaatacgaccatttttcagatcgataaaggcattctgataactgtcataagagacagttttcacttccgggtgctgatcctgaatatatttctggtgcgtagtaccgttttccatcccaatacgtttgcctttcagatcggcaaacgttttgtaggtatcttttttggcaatcacgacggctgagttttcatagtagggcgtggtaaacgatacctgtttgctacgctccggggtgatatccataccggagattacggcgtcatattttctgaatttcagggacgggatcaggctgtcgaacgcgtgattagtaaaagtacattctgcctgcatttgtttgcacaaggcttttgccagatcgatatcaaagccgacaatctcattattagcacctatagattcaaagggtggataggtggctgaaacgccaaaattgattttctctgcggcagaagcaccgaaagtaaaggaagcaagtaaagcggcaagaactaactttttcatgatggaactcccgtctgtcaatcttatgatttttggccgtgtctgcggcatgggataacaatgccatcaagtgaatttatatgcaataaacatgattaaataatttaaatgaaataaaaaagacggacaacttagtgggttgtccgtcttcattataagaatttatgcactatgtaggccggataaggcgtccccgccgcatccggcacaggcaccgtgctgatgtctgatgcgacgctggcgcgtcttatcagacctacaaaaccccccggcgaatgtacgcagccacattaatttcgccgttcgaatgccagcgctttgcgctcgatcagacgcatcatcagcgtcagcaggccgttaacgaccaggtaaataatccctgccgcaccgaacaccattacatcgtaggtgcgtccgtacaacaactggctgtatcccatcacttccatcagcgtaatggtgtatgccagagaggtacttttgaataccagcaccacttcgttggaataagaagagagcgagcgtttaaaggcatacggcagcaggatcgccagcgtatcttttttgctcattcccagggcgctacaggactgccactgaccttccgggatcgcacgaattgcaccgtaaaacagctgcgtggtatacgccgcactattcagcgacaacgcaatcagcgcacataaccacggttctgacaacaaatgccacagtgccggatactcctgcaaagtcggaaactggcccggcccgtaataaatcaggaagatctgcaccagcagcggcgtaccggtaaacagcgtgatataaccccgcaccagccacaccagcaccggcgttttcagcgtcaggatgatggtaaaaatcaatgccagaatcagtgccacaatcagcgaggcaacggttagcgtcaggctggtgtgtagccctttcatcagttcgggtaaatactcaaacattagctgggcctccgctcaaaacgtgtcgcgcgcaggtcaatgcgtttgagaatgtactgactgagcagggtgatcaccaggtaaatcgccgccgccacaatgtaccaggtaaatggttcctgggtacgagtagcgatgctttttgtttgcagcattaaatcattcacactaatcaaactgaccagcgcggtatctttcagcagcaccagccactggttaccgaggccaggcagcgcatgacgccacatctgcggcatcaccagacggaaaaagatagccgatttcgacagccccagcgcctgaccagactcccactgacccaccggcaccgctttcaacgcgccccgaagcgtttgcgaggcataggcggcatacagcagtgacagagcgatgacaccacaaaggaacgggctaacgtcgaagttctcaatgtccatctgcactgggatctgcacgaacccaagattgatagtgaagccatccgaaagcgtcagcagcagctgcgaggagccaaaatagataaacagcaccaccagaatttctggcaggccacgcagaatggttaccagcgctgaacctgcccacgcgacaggacgccattttgccgactcccataccgcaaagaacatcgccagcgccagcccgacaatcaatgcacaaacggcaaggccgacggtcatcccggcggcgcttgctaaaggaaaaaattcattcatcaggaattacttctggaaccatttgttgtagatggtttcgtaagtgccatctttcttcactttttccagcgcagtgttgagtttctgctgcagctcagtgttgccctgacgtaccgcgatgccgaggccagtgccgaagtaatctttatcggtcactttgtcgcccaccgccgccagtttcgggttatctttcagccactcagtgaccactgcggtgtcaccgaagacgccgtcgatacgcccgttttgcagatccagttttgcgttctggtagctgtcatacggaacggtagtgatttccgggtgcttatccataatgaatttctggtgtgtcgtcccgttctgtacgccgacttttttgcctttcagctgatcaacactggtgtatttgccttgctgacccacaaacagggcagagttgtcatagtacggggtggtaaacagcacctgcttttcacgctccggagtgatatccatgcccgccatcacggcttctacgcgacggaatttcaggcttgggatcaggctgtcaaacgcctggttagagaaagtgcaggttgcatcaatctctttacacagcgcttgtgccaggtcgacgtcaaaaccaacgatctggttgtttgcatcaatcgattcaaacggaggataggaggcttcggtagcaaaacgaatggtttcggcagctgtggcggaaagactaaaacctgcaattaacgcggcaatcagaacttttttcattgttgttatcccgaatcttagtgagagagatagtttttaaatgcttcggtttgcggctcggtaaagcagctcgcgtcgccttgttctacgatatgaccattttccatatacaccactcggctggcggttttacgcgccacttcaacttcgtgggtgacgatcacctgggtaatattcgtttctgccagctcacgaatgatgctgacgatttgtgccgtaatttccgggtccagtgcggcggtcggttcatcgaacagcagtacctgcggttccatcatcaacgcacgggcaatagcaacacgctgctgctgaccaccagaaagatgcagcgggtaacgatcgctataaggtttgagacgcagacgttccagcagtttttctgcacgggccagcgcctgatctttactcaaccccagtacacggcagggcgcttcaatcaggttttgctgcacggtcagatgcggccacaggttgtattgctgaaacaccatgccaacgttacgacgcaaatcgcgaatcgctttgtcagagggtgttttggtgaaatcgaaatggttgcctgcaatgttgagcgtaccggagcgcggcatctcaagcagattgagtacacgcagcagcgagcttttacccgcgccgctggggccaagtaacaccagcgtttcgccctgtgggcaatccagcgtgatatcgaacagcgcctgatgcgcgccgtagaagcaattaatgccgtttaattgaatactcattgacactcgtatactggcagtctgatagctattgaggtcgaagatagtacctttgacagaataattatgcaatatttctgctttaaaagttaaaagcaaagcgcattattcaataaacatagcacaaaataacgggggcggtggtcggcgagcataaatgtcggcattcctcacgaaatgccggacaatttacggggtttattggttgatcaaggcgttagcgattctcgatggactgacggagcgtacccgccgtggcatgaacgctaccgcctaagtaacgcacatcgtcgatgacccaacactggccttcctgaatcattaacacttcatcctgccaaccctggtcaccctgtttgagatccacgcgcaatggaatgttacgggcatcacgattagggatagtcgatgcactggcaacgtgggcgctatctggcaaggtggttcgactggagaatggatcgttggtcagtagttcccgatggttattatcccgggaggcatcgctaagcagtgtcgccagtttgtcgctcagataagggcgcaaggcggtgatgtcgttgctgcggtgcaaaatgcggtagtcataaaattgctgggccacgttatccgggcctccttcaacgcaaggaccactgcgtgtgccgttatctttataagctggagtgactgtggtgcaggcactgaggagcagtgcgcaggggataagcattgtcaatttgctgtagcgcataatgatttccttataagcgatcgctctgaaagcgttctacgataataatgatatcctttcaataatagcgtatcagtctgataatgcttttgagatcgaaggcttagcaaacaaggagatcgatcatgcaattttctacaaccccaactctggaaggccagaccatcgttgaatattgcggtgtggtgaccggcgaagcgattttaggtgccaatattttccgtgatttctttgccggtatccgcgatatcgttggcggacgttccggtgcgtatgaaaaagaactgcgtaaagcacgggagatcgcctttgaggaattaggctcccaggcgcgggcgctgggggccgatgccgtcgtcggtattgatatcgactacgaaacggtcgggcaaaacggcagtatgctgatggttagcgtcagcggtacggcggtgaaaacgcgtcgatgagaagattcttctggctggtcgctgccgctctgttattggcagggtgtgcaggcgaaaaaggcattgtcgagaaagagggatatcagcttgatacccgacgccaggcgcaggcggcgtatccgcgcattaaagtgctggtgatccactacaccgcagatgattttgatagctcgctggcgacactgaccgataagcaggtcagctcgcattatctggtccctgcggtaccaccgcgatacaacggtaaaccgcgcatctggcaactggtgccggaacaagaactggcctggcatgcggggattagcgcctggcgcggggcaacgcgccttaacgacacctctattggcattgagctggaaaaccgtggctggcaaaaatcggccggagtgaaatattttgccccgtttgaaccggcacagattcaggcgcttattccactggcgaaagatattattgcccgttatcacatcaagccggaaaacgtagtggcacatgcggatatcgcaccgcagcgcaaagacgatccggggccattatttccctggcagcaactggcgcagcaggggattggtgcctggccggatgcgcagcgggttaacttttaccttgccgggcgcgcgccgcacacaccggtagataccgcgtcattgctggagcttttggcgcgctacggttatgacgttaaacctgatatgacaccgcgcgagcagcggcgcgtgattatggcattccagatgcatttccgcccgacgttatataacggcgaagcggatgcagaaactcaggcgattgccgaagcattgctggagaaatacgggcaggattagcgcggcagttttccgtggtcgcgtagccaggcggcagttttctcgataccttcatccagggtgatgaccggctgataacctaactcttcctgcgcacgcgtaatatccagcgtaaagtcaaaattcaacttggagacgccgtagtgggtcagcggcggctcttttgctgacttgcggcctaaacgctccatgctgcgggcgatcatatccagcatcgggtaggggacggaacgaatacgacagtcaatattcaactcgtcgatcagcttctgcacgatgctgcgcagtgtgcgatgctcgccgttggtgatgttgtacacacgcccggaaggtagcttatcgcaggcttcctggcttgccagccacattgcgtgcacggcattttcatagtaggtcatatcgaccagcgcactgccgccatgcggtaacagaatactgccgtagtggtgcatcatatgcgccagacggggaataaagactttatcgtgcggtccgaacagactttgtgggcgcagaatagtaaagcgcgtttgtggattcgcctgcgaaagcatattgatcacttcttcgctggctgctttgctgcgggcaaactcgttggcgaagcggtgagggcgaaaatcttctttaatatcgcgatggtggtgataatcgaagtacagggagggggaagagatatgaataaagttacgcacaccccaggcgacagcccattcacccaggcggcgagtggcgcgaacgttagccagatcgaaagcctgttgtgtcccccagggtgaggtaaagctggagcagtgccacagcgtatcaatgcccgcgagcatcactttagcttgtgatgaaaccagctcggtcagatccgccggaacaaactctgcgcccattttttccagcaatttgcccattgcctcgttgcgaccggtcgctcgcacgctgatgcctttctggcataaaaactctaccgcgtttcgacctaagccgctggtggcgccggtaaccagtaccttcatatcaatccactgttgttgagaaaataacgtgcgcattcttccgtgatttcccccatgatgcaatgggaaacatgaaagaataacgcaggttttgtcgattaatctgtgctttgttctgccagtctggcgatttgttttgccattccgcgaaaaataaacagatgcgcggggatcatcaataaccagtaaaacagccccggcataccgtgcggatgccagaaagcgcggacatcgatagtacgatagtcgcctttatcttccaggctaaaacacagtcgtcccagccccggcgctttcatgccaaataacaacgtaagttgtttttccggttcaacgacaatcactttccagctatccaccgcatcgccagtctgtaaatattcgcgctccgggcggcctttcgccagcttatgaccgatcgcgcggtccatcaacgcccgtgtctgccacaaaatattgccaaagaaataacgctctttaccgccgatttggttcactacctgccataaagcagcaaggctggcggacgttttaacggtaaaccccgcctgtttggcaaaataaccgtactccggtcgccagcgggcaaaggcctgagcgtcgtagccccagtcgctggagttgaccagtttttcctcctctttcaacgtgctacgtaccgcgtcatcgaaagcgatcagccgttgtgggatgagtgcacgtagcgcggtatcatccgccagcagatcgtgtttcagcccctgaatcaacgccctggcggtggtgggcggtacggaagtaatcacattgagaaaccacaccgaaatccagcgggtggggagggggatggggatcaaccagcggcgcttaccgctcaccgccataaaatgttcaaactgttgctgataactgagcacctctggtccggcggcttcgaagatgcggtgttcgctggccggatgatctaacaacgcaaccagatagtgcagcaagttttccagcgcaatgggcgtggtgcgtgaacgaacccagcgcggaggcgttaagactggcaggttgtagaccatatcgcgcatgacttcgaacgccgcggaacctgcgccaacgataattccggcccgcagttcggtcacgggtacattcgcttcacgcagaatgtccgccgtagcctgacgagcacgcagatgatccgactgctcatgtggcggggcctgcaacgaactaagaaagattaattgcttaactggtacttcacgtagcgcatcgcggacgttgagagccacctggcgctcctgagcgataaaatcgccgccttcgcccatgctgtgcaccagaaaatagaccgtatcgatatcctgcaacagggccggtaggttatccggccagctgagatcgactttatggcaactgacgtttgccagttgcagctttgcaagcctgtcgacatgacgtgccgccgccaggatctgatgcccttgctggctgagtgtgcgcaccagatgctgaccaatgtagccactggcaccgagaactaaaatgcgttgcggcacgtctctctccttaacgcgccaggaatgcacgccagtgggcggcgacttccgccagttgttcgcgcgagacgtcaagatgcgtcaccaggcggacaatcggcgaggcgttaatcagcacgtttctcgctttcatgtattcgcctaacgcggcagcattttcttccccgacgcgaacaaacagcatattggtgtcctgacgcatcacatccgcgcctgcttcacgcagctgctccgccatccaggcagcgttgtcgtggtcttcctgcaagcgcgcaacgttatttttcagggcatatatcccggcggcagccagaatgccggactggcgcatcccgccacctgtcattttccgccagcgaatggcacgtttaatgtaatcacgattaccgacgagtaatgaaccgactggcgtcccaagacctttcgacaggcaaatggtgaacgaatcacaatattgcgtgatctctttcagttcgcagccgtaagccaccacggcattaaagatgcgcgcaccgtcaacatgcagcgccagattgcgctcgcgggtaaattcccatgcttctttcaggtattcccgcggcaacactttgccgttgtgggtgttttccagactgagtaatttggtgcgggcgaaatggatatcgtcgggtttgattttcatcgccactttatccagcggtagcgtgccgtcggcagccgcgtctatgggttgcggttgaatactgcccagcaccgccgcgccaccggcttcaaacagatagttatgcgcggcctgaccgacaatatactcttcgccgcgttcgcagtgactgagcagagcgaccaggttggcctgagtgccggtaggcagaaaaatggcggcttctttaccggaaagctctgctgcgtagtcctgcagagcattaacggtagggtcgtctccgtaaacgtcgtccccaaccggggcggccatcatcgcttcgagcatggcgcggcttggtcgggtaacggtatcactgcgtaaatcaatcatggcatgtccttattatgacgggaaatgccaccctttttaccttagccagtttgttttcgccagttcgatcacttcatcaccgcgtccgctgatgattgcgcgcagcatatacaggctgaaacctttggcctgttcgagtttgatctgcggtggaatggctaactcttctttggcgaccaccacatccaccaacaccggaccgtcgatggagaaggcgcgttgcagggcttcatcaacttcagacgctttttctacacggatacccgtaatgccgcacgcttcggcaatgcgggcaaagtttgtgtcgtgtagttcggtgccgtcagtcaaatagccaccagctttcatctccatcgccacaaagcccagcacgctgttgttaaagacgacaattttcactggcagtttcatctgcactactgagaggaaatcgcccatcaacatgctaaaaccgccatcgccgcacatggcgaccacctgacgttctggctctgtcgcctgcgcacccagcgcctgcggcatggcgttagccatcgaaccgtggttaaacgaacctaacaggcgacgcttgccgttcatttttagataacgtgccgcccacaccgttggcgtaccaacgtcacaggtgaaaatagcgtcatcggcggcaaaatgactaatttgctgcgccagatattgcgggtgaatggctttctcgctcggtttagctaaatcgtccagccctttgcgggcgtcgcggtaatcttccagcgctttatccagaaacttgcgatcggctttttcttccaccaatggaagcaatgcacgcagagtcgacttgatatcgccgaccagtgccatatccaccttgctgtgagcgccgatgctggctgggttgatatcaatctgaatgattttggcatcggtcgggtagaaggcgcggtagggaaattgcgtgccgagtagcactaacgtgtcggcgttcatcatggtatggaaacctgacgagaagccgattaacccggtcattccaacatcatacggattatcgtattcgacatgttctttaccgcgcagggcatgaacaataggcgctttaattttcccggcaaactcaactaactctttatgcgcccccgcgcagccgctgccacacatcagggcgatattgctggaataacgcagcagttgcgccagtttgcgtaactcttcttcttccggcgtcacgactggttgtggcgcatgataccagtgcatggttgccccttctggcgcaggttttaacgccacgtcgcctggtaacacgacaaccgaaacgccacggttaagcaccgctttgcgcatggcaatcgccagtacttgtgggatctgctccgggctggaaaccagctcgcaatagtgactacattcgcggaatagctcttgtgggtgggtttcctggaaatagccgctgccaatttcgctggagggaatatgagcggcaatcgccagtaccggaacgtgattgcggtggcaatcgaacaggccgttgattaagtgcaggttgccggggccgcacgatccggcgcagaccgccagttctccgctaagttgtgcttcagcgccagcggcaaaggccgccacttcttcgtggcgggtggacatccactcgatggtgcccatgcgattaagactgtcactaagaccgttcagagagtcgcctgtgactccccagatgcgtttcacccctgccgattcgagtgttttggcgatataagctgcaaccgtttgtttcatggttctccatctcctgaatgtgataacggtaacaagtttagttcatctgacggagggggaagggatgggagagaaaggaggcactaacggttaaatagcccgatgaaaggaatatcatcgggcataaggcgattatgcgagaaccaaatccccctgcggatggcaggagcaggccagtacgtaaccttcagcgatttcggcgtcggtcagcgtcattgtgctgctcaccgtatattcaccggaaaccacttttgtcttacagcagccgcaaacacccgcacggcaggcagcgacaaccggaacgttattgctttccagcgcctccagtagcgtggtgccaaccggggcgtaaaattctcgtgccggttgcagtttggtgaatttcagaccgctggtcgccgcttctgctactggggtgaagaatttctctttaaagaaacgcgtcacgccgagcgctttcacttcctgctctacccaatccatatacggagccgggccgcaggtcatcacggtacgtgaagctaagtcaggtacacctgccagcagttcgcgagtgagacgaccagcgataaagccttcggtaacgttattttctgccaccagcgttaccggatagttacgccactcatcggcgaaaataacatcctgcggcgtacgcacgttgtagatcacccgcacatcggcctgtggacggttcttcgcaagccagcgacgcatcgacataatcggcgtgacgccgcagcctgccgccagcaacaggaatttatcttctgctttatcgtcgcaggtaaattcccccatcgcgtccgaaagccagagataatcaccgcgttttacatcgcgcgtcagccactgggagccgacaccgtcatcaatccgccgcacggtcagggtgatatattcactcacgcctggcgtggaggaaatggtgtaagcacgcagcgtttccgctgagtttcgcacgctgaccagtgcatattgcccggcgcgatatgggtagtaatcgtggcaaatcagggaaatcgtccacacatccggcgtttcttgcgtaatgtgatgaacctgcatccgccacgggcattgattcgttggcatcgtcatcgacaaactccttacgcgctcaacagttgcttcatgtcttcttcaacagtggtgatagaacgcaggccgaatttctcgttcagcaccgccagcaggtctggtgtcaggaaaccaggtgcagtcgggccggtgacgatatttttcacgcccagagaaagcagcgtcagcagaatgacgatcgctttctgttcaaaccaggagagcaccagcgacagcggcagatcgttgacaccgcagcccagtttctctgccagagtgacagccagaataatcgctgagtaagcatcgttacattgacctgcatctaccagacgcggcagaccttcgatatcgccaaactcaagtttgttaaagcgatatttaccacaggcgagggtcaggatcaggcagtcatccggcacgctggtggcgaaatcggtgaagtagtggcgctcgccgcgtgcgccgtcacagccaccaagcaggaagatatgacgcagtttttcacggctcaccagatcaatcagcgtatcagcagcgccaagcagcgtctggcgaccaaaacccacggtgataaggtgcggaatttcgctgtacgggaagcctgccatctgttgcgcctgggtgataaccgcagagaaatcatcaccgtccagatgacgcacgccaggccagccaacaatgctgcgggtccagatacgatcgtcataagcgcctacggttgggtcgatgatgcagttcgaggtcatcacgatggggccagggaaacgagcgaactccacttgctgattctgccagccgctgccgtagttaccgaccagatgcttgaatttacgcagctccgggtagccatgcgcaggcagcatttcgccgtgggtgtagacattaacgcccgtgccttcggtctgttccagcaggttgtagagatctttgagatcgtgaccggaaatcagaatgcatttacccgccgtcgctttgacgttgacctgggttggcgtcgggtgaccgtatttaccggtttcgcctgcatccagaatgctcatcactttgaagttcatctggccgatttccattgaacactcaagaagcgcgttcatatcggcaggccaggtccccagccacgccatgattttatggtactgggcataaatatcgttgtcgtattgaccgagaacatgcgcgtgttccatataggccgccgcacctttcaggccatacaggcacagcagacgcaggccgagaatgttttcgccaatcgccgctttatctttgttaggggtaaattctgctgcctgacgttgcagctcgccgagatcgtcgctcaccagttgcaggtcagccatcgggttatcgacgcgcgcgttggcatctacagccaggcattgcgctttcagcgcctcgcgcagggcaatcgcttcacgagcgtagccgacaatacgcggagaatcgaagttaacgttggtcagggttgagaaaaaggcacgtggcgcgaagctgtcaacatcgtggttgatgatgccgtattcacgcgcttttaccgcccaggcagaaagcccttgcagcgccgcgatgagtaaatcctgaaggtcagaagtttccgccgttttaccacacatcccctgcgcgtatgagcagccgtttcctgccggagtacggatagtttgttcacattgcacacaaaacatgatcacaccttttaaagttatatttaatatacatgtttaaggttaagacgcttaacgcggggataaaagggatttttcatgcaactttaagggagattgatttagcgcaattttggcggcagggatctaccgccagagaggtattacgcagagaaaaaggcgatgaggatcggcactaacaggctaagaataaaaccgtgaacaattgccgccgggaccatatccagcccgccagtacgttgaagaacgggcagggtgaaatccattgatgtggcaccgcataagcccagtgcagtagagcggctgcggcgaatcagcccagggatcaacataatagcaatcagttcacgggccagatcattaaaaaacgccgcgctcccgattaccggaccaaaagattcggtcaataaaataccggaaagagaataccagccgaaaccggaggccattgccagcgcggtattgatggggagatcaagaataaaggcgttaattaaaccaccaattaatgaactgacaaccaccaccacggcgacaatcattccccggcgattaaggacaatctgctttaaggtcatgccattattgcgcaactgaataccaacgaggaaaagtagcaaaattaacgtgtattcactggcttcggtcgcgtgttgtaagaaagccagtccacttagaccaatggcaaaaccaatcactactacgccgcacagttttagcgactccagcgccatcgcaatacgcgacgggagtttttcttgctgatggtggttgcgccacggcaggcctcgctccagccacatcagggcggcaatattacacagtaaaataacggtaatactgacggcagaataatgcagaatcgccaacaggttactggcgaggttatcgagaaacgccagactgatacccataaaaaagagaataaggtaaaccatccagcttaatagctgattaataacttttaacgcagcttgttggcgaagcggaatgaggtaacccacaatcaggggaaccagaatgattaacagcccagaaaacatgaaaacccagtccttgcaaagatgaagtcgaaatgcgcgatgacacactactgaaagcggaaggacgagtaaagttgcaattaaaaggaaatgttatgcataaggagcagtagagtattcgttttcatttaaagatattcttgcgctttaattacaaactgcaccgatgttggtggcgtcaaaatcgccgaggcgttccctgaaggccggggcagcccacatggatgtgggctgagggcgcgttttacagggatgttacctcgcgcccgacccggtagccgtaagggataagtcgagggcaccgcgcagcggcgattttgttcgccagagcccgggggtgcagggggcggcggcgattggccgccccctgcgcgctccttgcgccagtggcaatatgttgcttagctcatgaaaggagcgcaacaagatgatgaatcaacatataacaacatcttaaaaaaaggcctgacattacgccaggccttctgcgttaattaatcacgcttttccagcagggtccggtaaatcagaccaccgataatgccgccgacaattggcaccacccagaagaaccacagttgttctaatgcccagccgccctggaagatagcaaccgcggtgctgcgcgccgggttaacagaagtgttagtcaccggaatactaattaagtgaatcagggttaaggccagaccaatagcgatcggcgcaaaacctgccggcgcgaatttgtcggttgcgccgtggatcaccaacaggaaacctgcactcaataccagttcaactaccagcgcggaaagcatggaataaccgcctggtgaatgctcgccataaccgttagaagcaaaaccgctggctgccgcgtcaaaacccgttttaccactggcaattaaatacagcagcgccgctgcaacaataccgccgacaacctgggcaattacgtagccaacgacttcttttgccggaaaacgtccgccagcccataaaccaatagtgaccgccgggttaaaatgaccaccagaaatatgaccaacagcaaaggccatcgtcagaacggtcagaccgaacgccaacgccacgccggcaaaaccaatgcctaattccgggaagcctgcggccagtacagcactaccacagccaccaaaaacaagccagaaagtaccaaaacattcagctgctaattttctgaacatatccaccacaattaaaaattgaccctgtgaaaaatatggtcgttttatagggtcgtcgtaaaaaagtgacgacggaaataatgcgcggctattttaaaaacgaaggcgagtcattcaccagataaataaatccagtaaatttgatttagggcaacagcgggttgccccatatagtcatttgtctgattgacagtgtagtgcacgcaaaagatttaatcctttaggcgtaataaaaaataatttatcatgctaattatttgattttgttgtttttgcagacttatcagcaagagggagtataacgcgattattcgctcatttttcagacatttgccatgcttaaatgtgatgtcatcacgtattagcaaggcctttcccgttatactgccagcgtaaaggataagtcacatatttctggaggggatatgattcttgagcgcgttgaaattgtgggttttcgcggtatcaaccgtttgtcgttgatgctggaacaaaacaacgtcctgattggggagaacgcgtggggtaaatccagcttgctggacgccttaactctgctgctatcgccagaatcagatctctaccattttgagcgcgacgatttctggttcccgccgggagatatcaacgggcgagaacatcatctgcatattattttgaccttccgcgaatcgctgccaggccgacatcgggttcgccgttatcggccgctggaagcgtgctggacgccatgcaccgatggctatcaccgtattttttatcgtctggaaggggagagtgcggaagacggcagcgtgatgacactgcgcagttttctcgataaagacggacatccgattgatgtcgaggatattaacgatcaggcacgccatctggtgcgtttaatgccggtgctgcgcttgcgtgatgcccgttttatgcgccgtattcgtaacggcacggtgccaaatgtccctaatgtggaagtcaccgcgcgccagctcgatttcctcgcccgtgagttatcctcacatccgcaaaatctctctgatgggcagattcgtcagggactttccgcaatggtacagctgcttgagcattatttctctgagcagggggccggacaggcgcgatatcgtttaatgcggcggcgagccagcaatgagcaacgaagctggcgctatctggatatcatcaaccggatgattgaccgacctggtgggcgctcgtatcgggttattttgctcggcctatttgctactttgttgcaggcaaaaggcacattgcgactggataaagacgcccgtccattgttgctgatcgaagatccagaaacccgtttacaccccattatgctttcagttgcctggcatctgttgaatcttctgccattgcagcgcattgccaccaccaactcgggtgagttgctttcgttaacgccggtagagcatgtttgccgactggtacgtgagtcctcgcgcgttgccgcctggcgtctggggccgagtggcttgagtaccgaagatagccgacgcatatcctttcacattcgttttaaccgtccgtcatcgctgtttgcacgctgctggttgctggtggaaggggaaacggaaacctgggttatcaatgaactggcgcgtcagtgcggacatcattttgatgccgaagggatcaaggtcattgagtttgcccagtccgggctaaagccactggttaaatttgcccgccgaatggggattgaatggcatgtactggtcgatggcgatgaagcagggaagaaatatgccgctacggtacgcagcctgttgaataacgatcgggaagccgaacgagaacatttaacggcgttaccggcgctggatatggaacattttatgtatcgccagggattttccgatgtgttccaccgcatggcgcaaatcccggaaaatgtaccgatgaatctacgcaaaattatctcgaaagcgatccatcgctcttccaaacccgatcttgccattgaagtggcaatggaggcaggacgtcgtggtgtggactccgtaccgacgctgctgaaaaaaatgttctcacgcgtgctgtggctggcgcgcggtcgcgcggattaaccgcgaaacatcgtggccatttgtggctgaatagcgtcgagcatctcatagcgccgacggtattcagcccgttttttactggcgatttcggcaatctcttttcgtgctatctgtgctggaaggcggtaatggcgttcagcatcacatacgccgccaaccgattcccagaaagcgttgtaatcagcgtggatcttgccttctttatcgcgataacgcaggctgcggtaaatatgcgtttcattgctgacggcaataatctgctctacctgcaaacgttgggcaaacagacaggccgcttccatcacgaggcgtttgggaaatagcccgtggcaggctttcgtcgcattctggatttcctgatgtggaatttcccattttgcgccttgcagtccgccaataaacatcgttcttttcccctgatattcacacagggtaaacgtgatctctgccagaggaataccttcgctgttgcggaacaggattgtgctgtcaccttctttatccattgagatcatcatggtcagctcaagcgtgaactgctcgccgtttttgccttccagcttcgccagttgcagcccgggggtattcaaatataagctgaattcttccgccgacatacattcgcggagtaacgcataatggtaacgtaacgcctccagcaattgcttacggctaagattcgccgcaaggtaagggcgatgcagacgcacaggcagtcgcggctggcgcgttaacaatacattgagattaggccagtgggaaagttcgttcatccactcaacgcttaaacgcggcataatcaacgagcgcagcaaaaatttctggcgaaaactacggcgatgccagaatttacccggccgacactgtccacgtgccagactaagaaaaagtgacaggctgctgagagattcagatggcgtaaaggtccgttcagttagctgcgacatattcatgaaatcaatggttatacatggcgtcgatttcaccattgcgtatcttaaccaaacatcaatagtgtgattactaacgtaaattttagggttttgttgatatttcgttgaagttaatgacccggattggcatatggagtattcagaaaatttatgaaaaagcggaaaaccgtgaagaagcgttacgttattgcgctggtgatagtcatcgccggactgattacgttatggagaattcttaacgcacccgtgccgacttatcagacgctgattgtgcgccccggtgatttacagcaaagcgtgctggcgaccggaaagctggacgcgctgcgtaaggttgatgtgggcgcgcaggtcagcggtcagttgaaaactctgtcggtggcgattggcgataaagtaaaaaaagaccagcttttaggggttattgatcctgaacaggctgaaaaccagattaaggaggtcgaagcaacgctgatggagctacgtgcgcagcggcagcaggcggaagcggagctgaaactggcgcgggtgacgtattcccgtcagcaacgtctggcacaaacgaaggctgtttcacagcaggatctcgacaccgccgcgacggagatggctgtgaaacaggcgcaaattggcaccattgacgcgcaaatcaagcgcaatcaggcttctctcgatacggctaaaaccaatctcgattacactcgcatcgttgccccgatggccggggaagtcacgcaaatcaccactctgcaaggccagacggtgattgccgcacaacaagcaccgaacattctgacgctggcagatatgagcgccatgctggtaaaagcgcaggtttctgaagcggatgtaatccacctgaagccggggcaaaaagcctggtttacggtgcttggcgatccactgacgcgctacgaggggcaaatcaaggatgtactaccgacgccggaaaaggttaacgacgctattttctattacgcccgttttgaagtccccaaccccaatggtttgctgcggctggatatgactgcgcaagtgcatattcagctcaccgatgtgaaaaatgtgctgacgatccctctgtcggcgttaggcgatccggttggcgataatcgttataaagtcaaattgttgcgtaatggtgaaacacgcgagcgtgaagtgacgattggcgcacgtaacgataccgatgttgagattgtcaaagggcttgaagcgggcgatgaagtggtgattggtgaggccaaaccaggagctgcacaatgacgcctttgctcgaattaaaggatattcgtcgcagctatcctgccggtgatgagcaggttgaggtgctgaagggcatcagcctcgatatttatgcgggtgagatggtcgcgattgttggcgcttcgggttccggtaaatcgaccctgatgaatattctcggctgtctggataaggccaccagcggcacctatcgcgtcgccggtcaggatgttgccacgctggacgccgatgcgctggcgcaactgcgccgcgagcatttcggctttattttccagcgttaccatttgctttcgcatttaaccgccgagcagaacgttgaagtacccgccgtctatgctggtcttgagcggaaacagcgactgcttcgtgcccaggagttgctgcaacggctggggctggaagaccgtacagagtattatccggcacagctttcgggtggtcagcaacagcgcgtcagcatcgcgcgggcattgatgaacggtggtcaggtaattcttgccgatgaaccaaccggcgcactggacagccattctggcgaagaggtgatggcgatcctgcatcagctgcgcgatcgtgggcatacggtgattatcgtcacccacgatccgcaggtcgctgctcaggccgagcgggtgatcgaaattcgcgacggcgaaattgtgcgcaatcctcccgccattgaaaaagtgaatgttactggcgggacggaacctgttgtcaacacggtgtctggctggcggcagtttgtcagcggttttaacgaggcgctgacgatggcatggcgggcgctggcagcgaataaaatgcgtactttactgaccatgctggggattattatcggtattgcgtcggtggtttccattgtcgtggtgggtgacgccgccaaacaaatggtgctggcggatattcgttctattggtacgaatactattgatgtctatcccgggaaagattttggcgatgacgatccgcaatatcagcaggcgctgaagtacgacgacttaatcgccatccaaaaacaaccgtgggtcgcctcagccacacctgccgtctcgcaaaacctgcgcctgcgttataacaatgttgatgttgctgccagtgccaatggcgtgagcggcgattattttaatgtctatggcatgaccttcagtgaaggaaacacctttaatcaggagcagctgaacggtcgtgcgcaggtcgtggttctcgacagtaatactcgccgccagcttttcccccataaagcagatgtggttggcgaggtgattctggtcggcaatatgcccgccagagtcattggtgtggcggaagaaaaacagtcgatgtttggtagcagtaaagtgctgcgtgtctggctaccttacagcacgatgtccgggcgagttatgggccagtcgtggcttaactccattactgtcagggtgaaagaaggatttgacagcgccgaggcggaacagcaactcacgcgtttactttcactgcgccacggaaagaaggatttctttacctggaacatggacggcgtcttgaaaactgttgaaaagaccacacgtactttacaactgtttctgacgctggtggcggtgatttcgctggtggtgggcggtattggtgtaatgaatattatgctggtgtcagtgaccgagcggacgcgggaaattggcattcgcatggctgtaggtgcgcgagcaagcgatgttttgcaacagttcctgatcgaagccgtactggtttgcctggtcggtggcgcgttgggaataacactgtcactgttaattgctttcaccttgcagcttttcttacccggctgggagattggtttttcaccgttggcgctgctgctggcgtttctctgctcgacggtcaccgggattttatttggctggttacccgcacgaaatgcggcacgactggatccagtagatgctctggcacgagagtaatttttgagataaaaatgccagccgatcgggctggcattttgcctttaggatgtacacaatgagacagaagagctatgcgactgccgcttctacttcgacgggcacaataacactggcgtgattgccttttggcccctggtggacatcaaactgaacggattgtccagcttttagcgttctgtaaccatccatctgaatggtggaataatgagcgaaaatatcttcgccgccgccttcagggcagatgaaaccaaaccctttggcattgttgaaccacttaacagtacccttttccatgcttcgacatccttcgcaaatcttatacaagtaagatggaataaaccggggtcagagagggggctgttcaaaacctcgccaactctagaaatacaatttagagaattagggcgagccgtcaagcatttgacaggggacaaggggcaggtatgaatcaaaaatttgaagcagttaacgctattgacaggaatgtgacagatgtcgctgatgccaacgatagatgatagttatctatcatgtggagtagattggtcaggcaaataagctcttgtcagcggcagggcgttctgccgataaccgtaaccgaagatgataactgacaatgggtaaaacgaacgactggctggactttgatcaactggcggaagaaaaagttcgcgacgcgctaaaaccgccatctatgtataaagtgatattagtcaatgatgattacactccgatggagtttgttattgacgtgttacaaaaattcttttcttatgatgtagaacgtgcaacgcaattgatgctcgctgttcactaccaggggaaggccatttgcggagtctttaccgccgaggttgcagaaaccaaagtggcgatggtgaacaagtacgcgagggagaatgagcatccattgctgtgtacgctagaaaaagcctgaatgcaggcataaaaattgggggaggtgcctatgctcaatcaagaactggaactcagtttaaatatggctttcgccagagcgcgcgagcaccgtcatgagtttatgaccgtcgagcacttgttactggcgctgctcagtaacccatctgcccgggaggcgctggaagcgtgttctgtggatttggttgcgctccgtcaggaactggaagcctttattgaacaaaccacacccgttctgcctgccagtgaagaggagcgcgacacacagccgacgctgagttttcagcgtgtactgcaacgtgcggtcttccatgtccagtcctccggtcgcaatgaggttaccggtgcaaacgttctggtcgctatctttagcgaacaggagtcgcaggcggcatatctgttgcgtaaacatgaagtcagccgtctcgatgtggtgaactttatctctcatggcacgcgtaaagacgagccgacacagtcttctgatcctggcagccagccaaacagcgaagaacaagctggtggggaggaacgtatggagaatttcacgacgaacctgaatcagcttgcgcgcgtgggcggaatcgacccactgattggtcgtgagaaggagctggagcgtgctattcaggttctctgccgtcgccgtaaaaacaacccgctgctggtgggggaatctggtgtcggtaaaaccgcgattgcggaaggtcttgcctggcgaattgttcagggcgatgtgccggaagtgatggctgactgtacgatttactctctcgatatcggttctctgttagcgggcacaaaatatcgcggcgactttgaaaaacgttttaaagcgttgctcaagcagctggagcaggacactaacagcatcctgtttattgatgagatccacaccattatcggtgcgggtgcagcgtctggtggtcaggtcgatgcggctaacctaatcaaaccgttgctctccagcggtaaaattcgtgtaattggttcgacaacctatcaggagttcagcaacattttcgagaaagaccgtgctctggcgcgtcgcttccagaaaattgatattactgaaccgtcgatcgaagaaactgttcaaatcatcaatggcctgaaaccgaagtatgaagcgcaccacgacgtgcgttataccgcaaaagcggtgcgtgcggcggtagagctggcggtgaaatacattaacgatcgtcatctgccggataaagccattgatgttatcgacgaagcgggcgctcgcgcacgcctgatgccggtaagcaaacgcaagaaaaccgttaatgtggcggatattgagtccgtggtggcccgtattgcacgcattccagagaagagtgtttctcagagtgatcgtgataccctgaaaaacctcggcgatcgcttgaaaatgctggtcttcggtcaggataaagccattgaggcgctgactgaagccattaagatggcgcgtgcaggtttaggtcacgaacataaaccggttggttcgttcctgtttgccggccctaccggggtcgggaaaacagaggtgacggtacagctttcgaaagctttgggcattgagcttctgcgctttgatatgtccgagtatatggaacgccataccgtcagccgtcttattggtgcgcctccgggatacgttggttttgatcagggcggtttgctgactgatgcggtcatcaagcatccacatgcggtgctgctgctggacgaaatcgagaaagcgcacccggacgtgttcaatattctgttgcaggtgatggataacggtacgctgaccgataacaacggacgcaaagcagacttccgtaacgtggtgctggtgatgaccaccaacgccggggtacgggaaactgagcgcaaatccattggtcttatccaccaggataacagcaccgatgcgatggaagagatcaagaagatctttacaccggaattccgtaaccgtctcgacaacattatctggtttgatcatctgtcaaccgacgtgatccatcaggtggtggataaattcatcgtcgagttgcaggttcagctggatcagaaaggtgtttctctggaagtgagccaggaagcgcgtaactggctggccgagaaaggttacgaccgggcaatgggcgctcgtccgatggcgcgtgtcatccaggacaacctgaaaaaaccgctcgccaacgaactgctgtttggttcgctggtggacggcggtcaggtcaccgtcgcgctggataaagagaaaaatgagctgacttacggattccagagtgcacaaaagcacaaggcggaagcagcgcattaatctgattgttaggtaggttggtcaagtccgtaatctcgaaagaggttacggactttttgtttatggggtggaggaggttcagaccctttttttaatgatgatggtaagttgttgataattagtgctgcgggaaggtaaggataaaaaagggtgctgcaggagaatgggatggttttgctttattaacaacgggctaaacgtgtagtatttgagttcactgccgtacaggcagcttagaaattcacaggtaacatactccacccgcccaccatgttcactgccgtacagacagataaaatgcgaaaaaaaagctcgcactttcgtacgagctcttctttaaatatggcggtgagggggggattcgaacccccgatacgttgccgtatacacactttccaggcgtgctccttcagccactcggacacctcaccaaattgttttgctaccaaacctcatgggtggcaacggggcgctactatagggagttggagtaaaacggtcaagaagaattttaatgataattattgtttgctcatactgtaaacaagttgtgcagtatatctacatcgagacaagttacggacttatacttccaaagtacttcatacatatcacaaaataaaaaggccggttaaaccgaccttttactcgttctttctcttcgcccatcaggcggtaaaacaatcagcgactacggaagacaatgcggcctttgctcaggtcgtacggggtcagttcaacagtcactttgtcgcccgtcaggatgcggatgtagtttttgcgcattttaccggagatgtgtgcagtaaccacgtgaccgttttctaactctacgcggaacatggtattaggcaacgtttcaagaacggtaccttgcatttcaatattgtcttctttggccatctaatcctctggggtatcactaccgtaatttgaaccggcaagataatgccgaagttctgtaaataagtaaagatttgcgcgctaaatcgcaacaaacaggttcggcacattactccgaaaacacacggctaagccgcaccaaaagcgcaacgtataagggagcggtgagataaacgatgggcgttacctgacgcgaaaaattccttatcggcagcggggtaatgagcgtaaccaactctgcgaccgcaattataacactctggggagaaatgtgccgaaaacattcattcttgtggtgaaaacaagcatcgtggtacccagaaattattcggcaatcgtccgaggcgcatttgattgagataattaaggtaatcccggcggggaatttcgcaggcaccaagcgatgctgtgtgatcgttaaggacctggcagtcgataagcttaccgccatgaccgataaattcctcacagaataccagaagcgccgttttagacgcattttccatccggctgaacatggactcgccacaaaatagcgttccctgggccacgccgtacataccgccgacaagctcatcttcacgccagacttcaatggagtgggcatggccgagttcgtgaaggcgatggtaggcttcgaccacgccacgcgtgatccaggttccttcttcgcgatcgctggcacagccttcaatgacctgaccaaaagcgtaattcatcgtgacacgatagggcgagcgtttatgaaatcgcttcatactacggctgatatgcagtgattctggccatagcaccgcgcggggatcgggcgaccaccagaggatggggtcgcctggagaaaaccacggaaaaataccacgctggtaagccattaacaggcgcgcagggctaagatcgcccccaagtgccagcaggccgttaggctcacgtaatgcgccttccggggaagggaaggctattgaatggcgagaaagctgaaccaggcgcatgaccgcaaaactccacgcaagtcggatcgttcaataatagcttacaaaccctgcttgaactggtaataacgcccctgtctggcaagcagttctgcgtgagtaccttgctcaataatttgcccgttgtccatcactattatttgttggaaacgagagagtccgcgaagtcgatgggtgaccattaacaccgttttctcacgcatcatttctgcaagcaattcaaggatctggctttcggttgtggcatctaagccttcggtaggttcatccagcaacaccagtggcgcatcatgtaacagcgcacgggcgatagccagacggcgcagttcaccaccggagagctggcgtccgccttcacctaaccaactgttgagacctgcatcctcgagcagcttttccaggccaacgcgacgcaagatctccgacagagcctcatcactactgccaggcgaggcgagtaaaagattatcacgcagcgtggcgctaaacagatgcactcgctgaggaacaacgctgatggtctgtcgtagagccgcttcattcaggctggctatggggctatcgttaagcaaaatctcgccctgttgcgggtcccatgcgcgggtcagctgttgtaacagtgttgatttgccgcatccggttcgcccgagaatcgctatatgttccccggcgtttacctgaagagaaatccctttaagtgcctgttgagattgctccggataagtgaactgaacatcccgtaacgtcagcgaaacgcgatcggcaacacgagtttgggtatcaggaaaggtgacctccggtttttgatccgttaagtcagagatacgtacggcagaggcaatgacttgccccagatgctgaaatgcacccgttactggtgccagtgcttcaaacgcggctaacgcgcagaagacaaacagggcaattaacgcgccgggttgagcattgccgccaacgccgccagacgccatccacagcatcaggatcaccgctaacgcgccaatgagcagcattatcgcttgcgacaatgcggtcagttcagattgacggcgttgcgcttccagccattgaatttctgtattctctagttgcgtgcgataacgatcgctggcaccaaaaatggtcagctcagcttgcccttgcagccaggccgtcagttgttggcgatactgtccgcgaagatgagtcagattttgcccggtgctttttcccgcacgataaaacagcggtggcatcaggaaaagcgtcagtaacataatgccgcccagcgtaaaggcgagggtgaaatcaaggaaacttaacccgattgtcaccaccataatcaccacaaaagcgcccaccagcggcgagataacgcgcaggtaaagatgatcgagcgtatcaacatccgccaccacgcgattgagcaattcgccctgacgatagcgcgccagtccggcaggggagaggggcagcaatttgctgaaggtgtaaatgcgcagatgctgcaacacgcggaaagtcgcgtcgtgacttaccagacgttcaaaatagcgcccggcagtacgggtgattgctgcgccacgcacgcccgcagcgggtagcatatagttgaagctgtacagtccggcaacccccgcaaccgctgaggccgagaggaaccagccggaaagtgtcaacagaccgatactggcgagcagcgtcacaattgccagcacaataccaagacttaacatccatttatgacgtttatacagtgccagatagggtagcaaagcgcgcatttaaatctcctcctgacgatgggccagtaatgtggcgaatgggccaccagccacacttaattccgcgtaacgtccttgctcaataatccggccatcctgcataacccaaatgacatcccagtcagcaagatcttctaactggtgggtgaccattaacgttgtctggcgcagagaggcggcattcagcgcctccattacgcgctgttcactgtgagcatcaaggctggcagcgggttcatccaacagtaatagcgaacagggatttagtaacgcacgggccaccgccacgcgctgcgcctgccccacggaaaggcgggcagcctggtcgccaacaggcgtatcaacgccttgtgggaggagcggtagaaactcgctgacccaggcgttatccagcgctgcttgtaattcttgttcgctggcatcaggtcgcgccagtagtacgttatcccgcaatgttgctgccggtaattgtgggttttgcccaacccaggagagatgtttacgccatgattctggtgataaatcgcgtaattctatcccgttgattcgtagcgatccctgatatgagagaaaaccagaaagcgcgttcagcagtgagcttttacctgaaccgctgcgaccaaccaacaccgcacgttggcctgctggcaaagtaaagttcagcggtccggccagcgttttaccttccggcgacgtgataaacagctcctcggcctcaatggtcaccggatcggtcgatgctaattccgcctcaccacgttgcggatgggcgagcggggtttccataaacgttttcagactgtcagctgcgccaacagcctgggctttagcatgataaaacgtaccgagatcgcgtaatggctggaaaaactctggcgcaaggatcagggccagaaaacccgcagccagcgtcacaccggtatcgtagtgaccaaaatccagctcgccgagataggaaaaaccaaagtagaccgccaccagagcaattgacagcgaggtaaaaaattcgagaatgccggaggataaaaacgccagccgtagcacttccattgtccgttggcggaaatcttccgaagcagaacgaatactttcaatttcagcttcaccacgaccaaaaatacgcaatgtttccatgccgcgcaggcgatcgaggaaatgcccacttaagcgagcaagagcgagaaagttacgtcggttagcatcggcagcccccattccaaccagcgccataaacaacggaattaacggtgcagtgcccagcagaatgagcgccgcagcccagttagaggggaagattgccaccacaatcagcaacggcaccgacactgccagcgccatttgcggcagatagcgtgcatagtaatcatgcatatcgtcaatttgctcgagtaccagcgtcgcccagctccccgcaggtttaccctgaatccacgctggccctgcttgttgcagacggtcgagaacctgacggcggatggcaaagcggatatgctgcccggcgtgataacccacccgttcgcgtaaccagaccacccatgcgcgcagtacaaaggtcagaaccagtaacgtaaagggaagcagcagggcttcacggggaatattctccataatcatatgttgcagaattcgcgccatgaaccaggcctgggcaatgatcaatatgccgctcacaaagcccagcagacgagaaatattcagccaacgttgggagatgacgctttgctgttttaaccagcgggttaactctttttgacgagatttattcattgcacgcttagcaggtgagttatcagaattatttgcagagcaatgttacaacggggaaaaaataaaggcgacccatagtcgcatggtgtcgccttctttacttttgttactgatttgtaaaattattttgcgtcagctaaaccatcgaggtagcgttccgcatcaagtgctgccatgcagcctgtaccggccgaagtaatggcctggcgataaatgtgatccatcacgtcgcctgcggcaaagacgccaggaatgctggtctgggtggcattaccatgaatacccgactgtactttgatgtagccgttttccagttccagctgcccttcgaaaatcgcagtattcgggctgtgaccgatagcaacaaacagaccggcaacgtcgagtgactcgatgttatcgctgttttgcgtatcgcgcagacgaacgccagtgacacccatttgatcgccggtcacttcttccagcgtacggttggtgtgcagaatgatgttgccgttctccactttatccatcaggcgcttaatgaggattttttccgcgcggaaaccgtcacggcggtgaatcagatgcacttccgaagcgatgttagacagatacagcgcctcttcaaccgcggtattgccgccgccgatgaccgcaactttctggttgcgatagaagaaaccgtcgcaggttgcacaagcagaaaccccacggcctttaaaggcttcttcagagggcaggccgagatagcgtgcagaagctccggtggcaataatcagcgcgtcgcaagtgtattcgccgttatcgccattcagacggaacggacggttttgcagatccaccttgttgatatgatcaaaaatgatctcagtttcaaacttggtggcatgttcgtgcatgcgctccattaataacggaccggtcagatcgtttggatcgccaggccagttttccacttccgtggtggtggtcagttggccgcctttttccatgccggtaatcagcacaggttgcaggttggcgcgcgccgcgtagacagcagcggtgtatcccgccgggcctgaacccaggataagcagtttactgtgtttggtcgtgcccatgagatccccatagttgttggcagacaatgggcaggattgtagggaatttacagacgtaaaaaaagagtatgacgattttgttaacaatttgtgcaatcggcagcatcgataagcaggtcaaattctcccgtcattatcacctctgctacttaaatttcccgctttataagccgattaaatgatgaataaacgcccctgttaatgaatatctggcatgttgtactaaaaatcgatgttttgctttgacaatcccctggtgttttgcgaaaacattcgaggaagaaaaaaaacagtattcttatatgcgcataaccatgcatgtaaataccatgtttaccgtgctagtgaaatctacgtatggcgtggacagacgccattcgtgatgtcgatagctgccacaaggcaacggtcttctcaccgtagacccaggcattgcgcgccgtgaatcttcatgatttcggtctatcgtgacgggtagcgactctgaacagtgatgtttcagggtcagacaggagtagggaaggaatacagagagacaataataatggtagatagcaagaagcgccctggcaaagatctcgaccgtatcgatcgtaacattcttaatgagttgcaaaaggatgggcgtatttctaacgtcgagctttctaaacgtgtgggactttccccaacgccgtgccttgagcgtgtgcgtcggctggaaagacaagggtttattcagggctatacggcgctgcttaacccccattatctggatgcatcacttctggtattcgttgagattactctgaatcgtggcgcaccggatgtgtttgaacaattcaataccgctgtacaaaaacttgaagaaattcaggagtgtcatttagtatccggtgatttcgactacctgttgaaaacacgcgtgccggatatgtcagcctaccgtaagttgctgggggaaaccctgctgcgtctgcctggcgtcaatgacacacggacatacgttgttatggaagaagtcaagcagagtaatcgtctggttattaagacgcgctaacacggaacaggtgcaaaatcggcgtattttgattacactcctgttaatccatacagcaacagtactggggtaacctggtactgttgtccgttttagcatcgggcaggaaaagcctgtaacctggagagcctttcttgagccaggaatacattgaagacaaagaagtcacattgacaaagttaagtagcggccgccgccttctggaggcgttgctgatccttattgtcctgtttgccgtctggttgatggctgccttactaagctttaacccttcggaccccagctggtcgcaaacggcctggcatgaacctatccataatttaggtgggatgcccggtgcgtggttggcagatacgctgttctttatttttggcgtgatggcttacaccattcccgtcattattgtcggcggttgttggtttgcctggcgtcatcagtccagcgacgaatacattgattattttgccgtttcgctacgcatcattggcgttttggcgctcatccttacctcctgtggtctggcggcaatcaacgctgacgatatctggtattttgcctccggtggcgtcattggcagcttactaagcactacgctacaaccactgctacacagtagcgggggaactattgcgctgctctgcgtttgggcagcgggcctgacgttgttcaccggttggtcatgggtgaccattgctgaaaaactcggcggctggattttaaacattctcaccttcgccagtaatcgtacccgtcgcgatgatacctgggtcgatgaagatgagtatgaagacgacgaagagtatgaagatgaaaatcacggcaaacagcatgaatcacgccgtgcccgtattcttcgcggcgcgctagcgcgtcgtaaacggttggcggaaaaattcattaatccgatggggcggcaaacagacgctgcgttgttctccggtaagcggatggatgatgacgaagagattacctacactgcacgcggtgtggctgccgacccggacgacgtcctattttcgggcaatcgtgcaacgcagccagaatatgacgaatacgatccattattaaacggtgcgccaattaccgaacctgtcgctgtagcagctgctgctaccacggcgacacaaagctgggctgcgccggttgaacctgtgactcagacgccgcctgttgcctctgttgatgttccacctgcgcaacctacagtagcctggcagcctgtaccgggtccacaaacgggagagccggttattgctcctgcaccggaaggttacccacagcagtcacaatatgcgcagcctgcagtgcaatataatgagccgctgcaacaaccagtacagccgcagcagccgtattatgcacctgcagctgaacaacctgcgcaacagccgtattatgcccctgcgccagaacaaccggtggcaggtaacgcctggcaagccgaagagcagcaatccacttttgctccacagtctacataccagactgagcaaacttatcagcagccagccgctcaggagccgttgtaccaacagccgcaacccgttgaacagcagcctgttgtggagcctgaacccgttgtagaagagacaaaacccgcgcgtccgccgctttactactttgaagaagttgaagagaagcgagcccgtgaacgtgaacaacttgcggcctggtatcaaccgattccagaaccggttaaagaaccagaaccgatcaaatcttcgctgaaagcaccttctgttgcagcagtacctccagtagaagccgctgccgctgtttccccgctggcatctggcgtgaaaaaagcgacactggcgacgggggctgccgcaaccgttgccgcgccagtcttcagtctggcaaatagcggtggaccgcgtcctcaggtcaaagaggggattggtccgcagttgccacgaccgaaacgtatccgcgtgccaactcgtcgtgaactggcgtcttacggtattaagctgccctcacagcgtgcggcggaagaaaaagcccgtgaagcccagcgcaatcagtacgattctggcgatcagtacaacgatgatgaaatcgatgcgatgcagcaggatgaactggcacgtcagttcgcccagacacagcagcaacgctatggcgaacagtatcaacatgatgtgcccgtaaacgcagaagatgcagatgctgcggcagaggctgaactggctcgtcagtttgcgcaaactcaacaacaacgttattccggcgaacaaccggctggggcgaatccgttctcgctggatgattttgaattttcgccaatgaaagcgttgctggatgatggtccacacgaaccgttgtttacgccaattgttgaacctgtacagcagccgcaacaaccggttgcaccgcagcagcaatatcagcagccgcaacaaccagttccgccgcagccgcagtatcagcagccacaacagccggttgcgccgcagccacaatatcagcagccgcaacaaccggttgcgccacagcagcaatatcagcagccgcaacaaccggttgcgccgcagcagcagtatcagcagccacaacagccagttgcgccacaaccgcaggataccctgcttcatccgctgttgatgcgtaatggcgacagccgtccgttgcataaaccgacgacgccgctgccttctctggatttgctgacaccgccgccgagcgaagtggagccggtagatacctttgcgcttgaacaaatggctcgcctggtggaagcgcgtctggctgatttccgtattaaagccgatgtcgtcaattactctccggggccggttatcactcgctttgaattgaacctggcaccgggcgtaaaagcggcgcgcatttctaacttgtcacgggaccttgcccgttcactttcgacggtggcggtgcgtgtcgttgaagttattcctggcaaaccctatgtaggtctggagttaccgaataaaaaacgacaaaccgtttatctgcgcgaagttttggataacgccaaattccgcgataatccgtcgccattaaccgtggtgctgggtaaagatatcgccggtgagccggtggttgccgatctggcgaaaatgccgcacttgttggttgcggggactaccggttccggtaaatctgtcggtgtgaacgcgatgatcctgagcatgctttataaagcacagccagaagatgtgcgtttcatcatgatcgacccgaaaatgctggagctttcggtttatgaaggcattccgcatctgttaacggaagtcgttactgatatgaaagatgccgccaacgcgctgcgctggtgtgttaacgagatggagcgtcggtataaactgatgtctgcgctgggtgtgcgtaatctggcgggttataacgaaaaaattgctgaagccgatcgcatgatgcgtccgattccagacccgtactggaagccgggtgacagtatggatgcccagcatccggtgctgaaaaaagaaccatacattgtggtgttggttgacgaatttgccgacctgatgatgacggtaggtaaaaaagtggaagagctgatagcacgtctggcgcaaaaagcccgtgccgcgggtatccacctcgtactggcaactcagcgtccatcggttgatgttattactggtctgattaaagcgaatattccgacccgtatcgcctttaccgtatccagtaagattgactcacgtaccattcttgatcaggctggcgcggaatcactgctgggtatgggggatatgctctactctgggccgaactccacgttgccggtacgtgtccatggtgcttttgttcgcgatcaggaagttcatgccgtggtgcaggactggaaagcgcgtggtcgcccacagtatgttgatggcatcacctccgacagcgaaagcgaaggtggtgcgggtggtttcgatggcgctgaagaactggatccgttgttcgatcaggcggtgcagtttgtcactgaaaaacgcaaagcgtcaatttctggcgtacagcgtcagttccgcattggttataaccgtgcagcgcgtattatcgaacagatggaagcgcaggggattgtcagcgaacaggggcacaacggtaatcgtgaagtgctggccccaccgccgtttgactaactaatgcatcgtatgccggataaggcgcggtagcgtcgcatccggcactctatcaactgaaaattcagtattttcttctttcctcaagctgattattagcctggaatagagagtagagggaactcccgatcgggagtgacgtaatttgaggaataatgatgaaaaaaattgccatcacctgtgcattactctcaagcttagtagcaagcagcgtttgggctgatgccgcaagcgatctgaaaagccgcctggataaagtcagcagcttccacgccagcttcacacaaaaagtgactgacggtagcggcgcggcggtgcaggaaggtcagggcgatctgtgggtgaaacgtccaaacttattcaactggcatatgacacaacctgatgaaagcattctggtttctgacggtaaaacactgtggttctataacccgttcgttgagcaagctacggcaacctggctgaaagatgccaccggtaatacgccgtttatgctgattgcccgcaaccagtccagcgactggcagcagtacaatatcaaacagaatggcgatgactttgtcctgacgccgaaagccagcaatggcaatctgaagcagttcaccattaacgtgggacgtgatggcacaatccatcagtttagcgcggtggagcaggacgatcagcgcagcagttatcaactgaaatcccagcaaaatggggctgtggatgcagcgaaatttaccttcaccccgccgcaaggcgtcacggtagatgatcaacgtaagtagaggcacctgagtgagcaatctgtcgctcgatttttcggataatacttttcaacctctggccgcgcgtatgcggccagaaaatttagcacagtatatcggccagcaacatttgctggctgcggggaagccgttgccgcgcgctatcgaagccgggcatttacattctatgatcctctgggggccgccgggtaccggcaaaacaactctcgctgaagtgattgcccgctatgcgaacgctgatgtggaacgtatttctgccgtcacctctggcgtgaaagagattcgcgaggcgatcgagcgcgcccggcaaaaccgcaatgcaggtcgccgcactattctttttgttgacgaagttcaccgtttcaacaaaagccagcaggatgcatttctgccacatattgaagacggcaccatcacttttattggcgcaaccactgaaaacccgtcgtttgagcttaattcggcactgctttcccgtgcccgtgtctatctgttgaaatccctgagtacagaggatattgagcaagtactaactcaggcgatggaagacaaaacccgtggctatggtggtcaggatattgttctgccagatgaaacacgacgcgccattgctgaactggtgaatggcgacgcgcgccgggcgttaaatacgctggaaatgatggcggatatggccgaagtcgatgatagcggtaagcgggtcctgaagcctgaattactgaccgaaatcgccggtgaacgtagcgcccgctttgataacaaaggcgatcgcttttacgatctgatttccgcactgcataagtcggtacgtggtagcgcacccgatgcggcgctgtactggtatgcgcgaattattaccgctggtggcgatccgttatatgtcgcgcgtcgctgtctggcgattgcgtctgaagacgtcggtaatgccgatccacgggcgatgcaggtggcaattgcggcctgggattgctttactcgcgttggcccggcggaaggtgaacgcgccattgctcaggcgattgtttacctggcctgcgcgccaaaaagcaacgctgtctacactgcgtttaaagccgcgctggccgatgctcgcgaacgcccggattatgacgtgccggttcatttgcgtaatgcgccgacgaaattaatgaaggaaatgggctacgggcaggaatatcgttacgctcatgatgaagcaaacgcttatgctgccggtgaggtttacttcccgccggaaatagcacaaacacgctattatttcccgacaaacaggggccttgaaggcaagattggcgaaaagctcgcctggctggctgaacaggatcaaaatagccccataaaacgctaccgttaatgttatcgttgcggtaatgttgttactgtatccctgtggtcgcaggctgtggccacatctcccatttaattcgataagcacaggataagcatgctcgatcccaatctgctgcgtaatgagccagacgcagtcgctgaaaaactggcacgccggggctttaagctggatgtagataagctgggcgctcttgaagagcgtcgtaaagtattgcaggtcaaaacggaaaacctgcaagcggagcgtaactcccgatcgaaatccattggccaggcgaaagcgcgcggggaagatatcgagcctttacgtctggaagtgaacaaactgggcgaagagctggatgcagcaaaagccgagctggatgctttacaggctgaaattcgcgatatcgcgctgaccatccctaacctgcctgcagatgaagtgccggtaggtaaagacgaaaatgacaacgttgaagtcagccgctggggtaccccgcgtgagtttgactttgaagttcgtgaccacgtgacgctgggtgaaatgcactctggcctcgactttgcagctgcagttaagctgactggttcccgctttgtggtaatgaaagggcagattgctcgcatgcaccgcgcactgtcgcagtttatgctggatctgcataccgaacagcatggctacagtgagaactatgttccgtacctggttaaccaggacacgctgtacggtacgggtcaactgccgaaatttgctggcgatctgttccatactcgtccgctggaagaagaagcagacaccagtaactatgcgctgatcccaacggcagaagttccgctgactaacctggtgcgcggtgaaatcatcgatgaagatgatctgccaattaagatgaccgcccacaccccatgcttccgttctgaagccggttcatatggtcgtgacacccgtggtctgatccgtatgcaccagttcgacaaagttgaaatggtgcagatcgtgcgcccagaagactcaatggcggcgctggaagagatgactggtcatgcagaaaaagtcctgcagttgctgggcctgccgtaccgtaaaatcatcctttgcactggcgacatgggctttggcgcttgcaaaacttacgacctggaagtatggatcccggcacagaacacctaccgtgagatctcttcctgctccaacgtttgggatttccaggcacgtcgtatgcaggcacgttgccgcagcaagtcggacaagaaaacccgtctggttcataccctgaacggttctggtctggctgttggtcgtacgctggttgcagtaatggaaaactatcagcaggctgatggtcgtattgaagtaccagaagttctgcgtccgtatatgaacggactggaatatattggctaatacccaatttttctgaatctaaaaagcgcctgcgggcgctttttttgtctccctttgataccgaacaataattactcctcacttacacgtaatactactttcgagtgaaaatctacctatctctttgattttcaaattattcgatgtatacaagcctatatagcgaactgctatagaaataattacacaatacggtttgttactggaatcaatcgtgagcaagcttgagtgagccattatgaaaacgaaaatccctgatgcggtattggctgctgaggtgagtcgccgtggtttggtaaaaacgacagcgatcggcggcctggcaatggccagcagcgcattaacattaccttttagtcggattgcgcacgctgtcgatagcgccattccaacaaaatcagacgaaaaggttatctggagcgcctgtacagttaactgtggtagtcgctgcccgctacgtatgcacgtcgtggacggtgaaatcaaatatgtcgaaacggacaataccggcgatgacaattacgacggcctgcaccaggttcgcgcctgcctgcgtgggcgttccatgcgtcgccgtgtctacaatccggaccgcctgaaatatccgatgaaacgagtcggggcgcgcggtgaaggcaaattcgagcgcattagctgggaagaagcctacgacatcatcgcgaccaatatgcagcgcctgatcaaagagtacggcaacgagtctatctatctgaactatggcaccggtacgctgggcggcaccatgacccgctcctggccgccgggaaataccctggtcgcgcggctgatgaactgctgcggcggctatctgaaccattacggcgactactcctccgcgcaaattgcggaaggtttgaactatacctacggcggctgggcagatggcaacagcccgtcggatatcgaaaacagtaagctggtagtgctgtttggtaataaccctggcgaaacgcgaatgagtggcggtggggtgacttactatcttgaacaggcacgccagaaatctaatgcccgcatgatcatcatcgatccgcgctataccgacaccggtgccgggcgcgaagatgagtggatccctattcgtccgggaacagatgccgcactggttaacggtctggcgtacgtcatgatcactgaaaacctggtggatcaggcattcctcgataaatattgcgttggctacgatgagaaaaccctgccagccagtgcgccgaaaaatggccactataaagcttatattctgggtgaagggccagatggcgtggctaaaacgccggaatgggcctcgcaaatcactggtgttccggcagacaaaatcatcaaattggctcgtgaaatcggtagtaccaaaccggcgtttatcagccagggatggggcccgcagcgtcacgctaacggtgaaatcgcaacccgtgctatctcgatgctggcgattctgaccggtaacgttggtattaacggaggcaacagcggcgcgcgtgaaggttcatacagcttaccgtttgtccgtatgccgaccttggaaaacccgatccagaccagcatttcgatgtttatgtggaccgatgccattgaacgtggcccggaaatgacggcgctgcgtgatggtgtacgcgggaaagataagctggatgtgccgatcaaaatgatctggaactatgccggtaactgcctgattaaccagcattctgaaatcaaccgtacccatgaaatccttcaggatgataagaagtgcgagctgattgtggttatcgactgccacatgacctcatcggcgaaatatgctgacatcctgctgcctgactgcaccgcttccgaacagatggactttgcgctggatgcatcctgcgggaatatgtcttacgtgattttcaacgatcaggtgattaaaccgcgctttgaatgtaagaccatctatgaaatgaccagcgaactggcaaaacgtcttggcgttgagcaacagtttactgaaggccgtacccaggaagagtggatgcggcatctgtatgcccagtcgcgggaagcgattcctgaactgccaacgtttgaagagttccgcaagcaggggatctttaaaaagcgcgacccacaagggcatcacgttgcttataaagccttccgtgaagatccgcaggcaaacccactgactacgccatcgggcaaaattgagatttattcgcaggcgctggctgacattgccgctacctgggaattgcctgaaggcgatgtgatcgatccactgccgatctacacgccgggctttgaaagttatcaggatccgctgaacaaacagtatccgctgcagcttacaggtttccactataaatctcgcgttcactcaacttacggcaacgttgatgtgctgaaagcggcttgccgtcaggaaatgtggatcaacccgcttgatgcccaaaaacgcggtatccacaacggcgataaagtcaggatctttaacgatcgtggtgaggttcatattgaggcgaaagtgacgccacgaatgatgccgggtgtggtcgcactgggtgaaggtgcctggtatgacccggatgcaaaacgtgtcgataagggtggttgtattaacgtactgaccactcaacgtccgtctcctctcgctaaggggaatccgtcacatacaaaccttgttcaggttgaaaaggtgtaaggagtaaccgatgacaacccagtatggattttttattgattccagccgttgcaccggttgcaaaacctgcgagctggcctgtaaagactacaaagatttgacgccagaagtcagcttccgccgcatttatgaatatgctggcggcgactggcaggaagataacggtgtctggcaccagaacgtgtttgcctactatctgtcgatttcatgtaaccactgcgaagatccggcttgtactaaagtctgcccgagcggtgcgatgcataaacgtgaagatggttttgttgtggtcgatgaagatgtgtgcattggctgccgctactgccatatggcttgcccgtatggcgcaccgcaatataacgaaacgaaaggccatatgaccaaatgcgatggttgttatgaccgtgttgcggagggtaaaaagccgatctgtgttgaatcttgtccgctgcgggcgctggatttcggccctatcgacgagctgcgtaaaaaacatggcgatctggcggccgttgcgccgttgccgcgagctcactttaccaaaccgaatattgtgatcaaacccaatgccaatagccgcccgaccggggataccactggctatctggcaaacccgaaggaggtgtgagatgggaagtggatggcatgaatggccgctgatgatcttcacggtcttcgggcaatgtgtagcaggtggttttatcgttctggctttggcgctgctcaaaggcgacctgcgagcagaagcccagcagcgtgttatcgcctgcatgtttggtttatgggtgctgatgggcattggctttatcgcctctatgctccatcttggttcaccaatgcgcgcttttaactcgctcaaccgggtaggggcttcagcactcagtaacgaaatcgccagcggttcgatcttttttgccgtaggcggcatcggctggttgctggcaatgctgaaaaagctgtcaccggcattgcgtacgctgtggctgatagtgacgatggttcttggcgtcatctttgtctggatgatggtgcgtgtgtataacagcattgataccgttccgacctggtacagcatctggacgccgatgggcttcttcctgacgatgtttatgggcggcccgttactgggttacctgttgttgagtctggctggcgtcgatggctgggcgatgcgtctgctgccagcaatttctgtactggcactggtagtgagtggcgtggtgtcagtgatgcagggcgcagagctggcgactattcatagttctgtgcagcaggccgcagcgctggtgccggactatggtgcgctgatgtcctggcggatcgtgcttttggccgttgccctgtgcttgtggattgcaccacagctaaaaggttatcagcctgcggttccgctactttctgtatcattcattctgcttctggcaggggaattaatcggtcgcggcgtattctatggtttgcatatgaccgtggggatggccgtcgcaagctaatcataacaaccggggtttcggccccggttctcttttatttctgcttcgttaacgtgtcataactggtcatcaaattacgataatcaggaatgtggttagagaacaacgtcgccagtccttcaatatcattacgccagtcgcgatgcagctcgcacgccacgccgaaccatgtcatcaattgcgcaccagcttgcgacaagcgatcccatgccgaatgccgggtaatttcattaaaggtccctgacgcgtcagtcacgacaaagacgtcaaacccttcttcaatggctgaaagcgccgggaatgccacgcaaacttcggttaccacaccggcaataattaactgttttttacctgtcgctttgacagcttttacaaaatcttcgttatcccaggcgttaatatttcccgggcgagcaatgtaaggtgtatcggggaattgtgctttcagttctggaactaatgggccgttaggaccggtttcaaaactggtggtaagaatagttggtaagttgaaatacttagccaggtcacccagcgccagcacgttatttttaaacttatcgggttcgatatcccgtacaagggaaagtaaaccagcctggtgatcaacaagcaaaacggcagcatcatttttatcaagacgaacatacggtttggtcatcctcttctcctttcgagagtcagtggtacgtctgaaatcgatcagacgcgatgcattgctctgaaagcatagacgggaaatatgagtttgctgtgaccatgaaatttttcgactgaacgaagcgtatgaaatttgtgttagttcaataaaaacaatcagatgagactaatcatctcttcagcattagcgttatgaatgagtaatataaatcgataataccgccgctgggatatcgcgtattttcacccattgacaatgtttttggcggtggcatgatgcgcatgaaatttgaacttcctcacggttttaattcatgtccacgtatacccagcctgtcatgcttttgctgtctggcctgcttttgttgactctggcgattgcggtgttaaatacactcgtgccgctttggctcgcccaggaacacatgtccacatggcaggtaggcgttgtcagctcatcctattttaccggcaaccttgtcggtacattgctgacagggtatgtcattaagcgcattggctttaaccgcagctattatctggcctccttcatttttgccgctggctgtgccggccttggcctgatgattggattctggagctggttggcttggcgttttgtcgcgggcgtcggctgtgccatgatttgggtggttgttgagagcgcgctgatgtgcagtgggacgtcacgtaaccgtgggcgtttgcttgctgcgtatatgatggtttattacgtgggaacgtttttaggccagttactggtcagcaaagtttcaaccgagctgatgtccgtattgccgtgggttacaggtttgacgttggcagggatcttaccgctgttgtttacgcgtgtgctgaatcagcaggctgaaaaccatgattcgacgtcaattacgtcaatgctaaaactccgtcaggcgcggcttggcgtgaatggctgcattatctcaggaatcgttctgggatctctatatggcctgatgccgctgtacctcaatcacaaaggggtgagcaatgccagcattggtttctggatggcggtactggtcagtgcgggtatccttggacaatggccgattggacgtctggcggataagtttggtcgactgctggtgttgcgtgttcaggtctttgtcgtcattctcggcagtatcgcgatgcttagccaggcggcgatggccccagcgttattcatcctcggtgccgctggctttacgctatatccggtggcgatggcatgggcttgcgagaaagttgaacatcatcaactggtggcgatgaaccaggccttactgttgagctatactgtgggaagtctgcttggcccgtcatttaccgctatgctaatgcagaatttctccgataatttattgtttatcatgatcgccagcgtatcgtttatctatttgctgatgctgctgcgcaacgccggtcatacgccgaaacccgttgctcacgtgtaaatgaattcaagcagagtgtgaacttactgtttcacactctgcttttttgtttcttctatctgacttgctttattccaaattttattcgtttaaaaataaaatgtgcagcaggttataattttgcatttcgctatttccgcacttcttatttgccgcgcataatccctcgttttaccgatgcccctttaattttggcgaaggatttgtctatggctgggaatgttcaggaaaaacagttgcgatggtacaacattgcgctgatgtcttttatcactgtctggggttttggcaacgttgttaataactatgccaaccaggggctggtggttgttttttcatgggtgtttatctttgcactctatttcacaccttatgcgctaattgttggtcagttaggctcgaccttcaaagatgggaagggcggggtcagtacctggattaaacacacgatgggacccggactggcttatctcgccgcgtggacctactgggtggtgcatattccctatctggcacaaaaaccccaggcaattctgattgcgctcggttgggcgatgaaaggcgacggttcgctaatcaaagaatattcagtcgtagcgttacaggggttaacgctggtgctgtttatcttctttatgtgggttgcttcacgcggtatgaaatcgctgaaaatcgtcggttctgtggcagggattgctatgtttgttatgtcactcctgtatgtggcgatggcggtaaccgcgcctgcaattactgaagtgcatattgcgaccacaaacattacctgggaaacgttcattcctcatatcgactttacctacattaccactatttcaatgctggttttcgcggttggcggagcagagaagatttctccttacgttaatcaaacgcgcaacccaggaaaagaatttccaaaagggatgttatgcctggcggtgatggttgcggtttgtgccattctgggctcgctggcgatggggatgatgtttgattcgcgtaatatcccggatgacttaatgaccaacggtcagtattacgcctttcagaagctgggcgagtattacaacatgggtaatactttaatggtgatttacgccattgcgaataccctgggacaagtagcggcgctggtattctcgattgatgccccgcttaaagtgctattaggtgatgctgacagcaaatatattccagccagtttatgtcgtaccaacgcttctggtacgcccgttaatggctattttctgaccctggtactggtggcgattctgattatgctgccgactctcggcattggtgatatgaacaatctctataaatggctgttgaaccttaattcggtagtgatgccgctgcgttatttatgggtatttgttgcatttattgcagtcgttcgcttggcgcagaaatataaaccagaatatgtctttattcgtaataagcctctggcaatgaccgtcgggatttggtgttttgcctttaccgcctttgcctgtttgacggggatcttcccgaaaatggaagccttcactgcagagtggaccttccagttggcgctgaatgttgcaacgccgtttgtgctggtaggattaggactgatattcccgctgctggcgcgtaaagcgaatagtaaataattattgtggtcggtgacgctgactctggcagatctgacccgtttttacataatcgagaaatgcgcgcaagccgcaggacatatactggcggtttggataatagatctggaagcctggacgctctgtgctccagtcttccagtacacattctaaacgaccagtatcaaggtactccttgatctgttcatagagcagatacccgataccagcacccatcaaaacggcctccagttcagcatcaacatcatccagaatgatatttcctgcgacagcaatttccagctcctttgcaaattgccagtggaaaggtttgccgctgggataacgaaaaacaacacattgatgattaagcagatcatgaggatggcggggtttgccatatcttgcaaagtactctggcgttgctgctacacataatttcactggcgggccgatcgccacgctgatcatatctttttcgacgatgcaactaagtcgaacgccagcgtcaaagccctgttggacgatatcgacaagagagtcgtcagttgtgagctcgactttaatatcaggatattcacgtgtgaaaccaaccagtaaagacattaaaaatatacgtgcagctacccgggcggcattgattttgagcgttcctgtcggtgtcagacgaaaatcattcatctcatctaacatgatctgaatttcgtcgaaagctgggcgcaatcgttcatagagattagaacccgcttccgttaacgatacgcttcgggttgtccgattgaataagcgaattttaagacgttgttccagtgttttaatactatggctaatggcggacgaggataagcctaactcatcgcccgctgcacgaaagctttgattacgggccacggcaaagaaagtggcaaagtcagacatattcatccgcattagtgaaaatccttcattaactcatcctgaatcatcacgtttacaggattatgccgcctgcgtaaagtgcgctccagaacttaacgtggaggtaaaattatgcagtctgaacgtatttatttggtatgggcccatcctcgtcatgattcattgaccgcacatattgctgatgcgatccatcagcgggcaatggagcggaaaatacaggtgacggaactcgatttatatcggcgtaatttcaacccagtgatgacgccggaagatgaaccagactggaagaatatggataaacgttattctccagaggttcatcagctttattcagagctgcttgaacatgacacgttagtggtggtttttcctctctggtggtacagcttcccggcaatgctaaaaggatatattgacagagtatggaataatgggctggcttatggagatgggcacaaattaccattcaataaagttcgttgggtggcgctggttggaggagacaaagaatcatttgtccagatgggctgggaaaaaaatataagcgattatttaaaaaatatgtgcagttatcttggtattgaagatgccgatgtcactttcttgtgtaatacagtggtattcgatggggaagaacttcacgcgagctattatcagtcgttattatctcaggtacgggatatggtagatgcactataagatgtgttaaaaacgctgtagcagaatgaagcgcggaataaaaaagcggcaactcaataaagttgccgctttacggggaaattagaacattaccttatgaccgtactgctcaagaatgcctttcacgcgttccatggtctctttcttcggtggtttaacaccgtcgagtttgtactcttcacccattgccacccatttgtgtttgcccagctcgtggtaggggagaagctcgattttctcaacgttgcccatatcacgggtaaattcaccgaggcgatgcgctgaatcgtcatcgtcagaccagcctgggacaacaacgtagcggatccacaccttcacatttttgttcgccagatatttagcgaactccagcgtgcggtggttggaaactccaaccagattttggtggatctcgtcgttcatctgtttgagatcgagcattaccaggtcggttacttccagcagttcatcaatcaccggatcgtaacgacgaacaaaaccgttggtgtccagacaggtatgaatgccttcttttttgcaggcgcggaaccagtcacgaacaaactcagcttgcaggattgcttcaccgccggatgcggtaacgccgccgccggaagcgttcataaagtggcgataggtcaccacttccttcatcaaatcttcaacggtaacttctttaccgccatgcgtgtcccaggtgtcgcggttatgacaatacaggcagcgcatcaggcagccctggaaaaaggtgataaagcgaatacctgggccgtctacggttccacaggattcaaaggagtgaatgcgaccaataactgacattgcggtgtttctccagatgtggcccatctgaggccgtgttggtgcgcagctcgaaggctacgtcgagtctgttttggcagtcaccttaaagtatagatagctgacaaaaaaggctctcgcgctaaaaaaggccccactttcgtggagcctttattgtacgctttttactgtacgatttcagtcaaatctaattacatagattgagtgaaggtacgagtaataacgtcctgctgctgttctttagtcagcgagttgaaacgtactgcgtagccagatacacggatggtcagctgcggatatttttccgggttttccatcgcgtcgagcagcatttcacggttcatcacgttaacgttcaggtgctgaccaccttcgatggatgcttcgtggtggaagtaaccatccatcagaccagccaggttggtcttacgaacttcgtcgtctttacccagtgcgttcggaacgatagagaaggtgtaggagataccatctttagcgtaagcaaacggcagtttagcaacggaagtcagagaggctactgcacctttctggtcacgaccgtgcatcgggttagcacccggtccgaacggcgcgccagcacgacgaccgtctggggtgttacccgttttcttaccatacacaacgttagaagtgatggtcagaacagactgagtcgggatagcgtcacggtaggtgtgcagtttctgaattttcttcatgaaacgttctaccaggtcaacagccaggtcatctacacgcggatcattgttaccaaactgcgggtattcgccttcgatttcgaagtcgatagccagaccgtcttcgtcacgaatcggtttaactttcgcatatttgattgcagacagggagtcagcagcaacggacagaccagcgataccacacgccatggtgcggataacgtcacggtcgtgcagcgccatcagagaggcttcgtagctgtacttgtcgtgcatgtagtggatgatgttcagtgcagtgatgtactgtttagccagccagtccatgaagtgatccatgcgctccatcacttcatcatagttcaggacatcgcctttgatcggttcagacttcggaccaacctgcattttcagtttttcgtcaacgccgccgttgattgcgtacagcatggttttcgccaggtttgcacgcgcaccgaagaactgcatttgtttaccaacgatcatcgggcttacgcagcaagcaatagcgtagtcatcgttgttgaagtccggacgcatcaggtcatcgttctcatactgcagagaagaggtgtcgatggacactttagcggcgaatttcttgaagttcagcggcagtttttcagaccacagaatggtcatgttcggttccggagacggacccatggtgtacagggtgttcaggaaacggaagctgtttttggtaaccagggtacgaccgtcgaggcccataccaccgatagattcggttgcccagatcgggtcgccagagaacagttcatcgtattccggagtacgcaggaagcgaaccatacgcagtttcatgaccaggtggtcaaccatttcctgcgcttcttgttcggtgatcttgccagctttcaggtcacgttcgatgtacacatccaggaaggtggaggtacgaccgaaggacattgcagcaccgttctgagacttaacagcagccaggtagccgaagtaagtccactggatagcttcctgagcgttggtagccggaccagagatgtcgtagccgtatttcgcagccatttctttcatctgacccagagcgcggtgctgttcagcgatttcttcgcgcagacggatagtctgttccaggtttacgccgttttccagatcagcctgcagagaagtgaactgtgccagtttgtctttcatcaggtagtcgataccgtacagcgcaacgcgacggtagtcaccgatgatacggccacggccatatgcatctggcagaccggtcagaacaccagatttacggcaacgcaggatgtccggagtgtaaacgtcgaacacgccctggttgtgagttttacggtattcagtgaagatttttttgatcatcggatccagttcgcggttgtacgctttgcaggaaccttcgatcattttgataccaccgaacgggataagagcacgtttcagcggagcttcagtctgcagaccaacgattttctcaagctgcttgttgatgtagccagcgtcgtgagaggtgatggtggaagcaacagcggtgtcaaagtcaactggcgcgtgagtgcggttttccagtttaacgccttccattactttgtcccacagggtggtggtcgcttcagtagcgccagccaggaaggactcgtcaccctcgtacggagtgtagtttttctgaatgaagtcacggacgtttacttcattctgccagtcacctttggtaaaaccttcccaggctgtggctaacttttcattaagctcggacatgtaacacctaccttcttaagtggattttttatttactgcgtacttcgacaaccattaatggtggtcgttttcacgcaggtaaatgacccagtatgtcaacccaaccaacaaaccaccaccgataatgttgccgatcgtaaccggaatcaggttatcagtgatgaaattcatcacggtcaggtgagaaaaattttccggtgcagaaccgactgcggtccaaaattccggggatgcgaagtcgcggattacaatacccatcgggatcataaacatgtttgcgatactgtgctcaaaaccgctggcaacaaacatcgcgaccggcagcaccataatgaacgctttgtccatcaggctgcggccagaataactcatccatactgccagacataccatcaggtttgccaggataccaagacagacggcctcaataaaagtatggtgcactttgtggtcggcggtttgtaggacgtttagtccccattgaccatttgcggtcatatactcgccggaaagccacattaaaagtacaaacagcagtgcgccgaccaggttgccaaaatagacatttagccagtttttcgccaactgaccccaggtgatgcgcccactcgccttagcaacaacaatcaacacggtggaagtaaagagatcggctccgcagacaacacaaagaatcagccccagagagaagcaaatgccgccaaccagttttgccatgccgaagggcattgtgcctgtgccagtggttgctgtgatatagaagacgaatgcgattgagatgaaaacaccggcggtaatcgccagatagaaagtcttaagcggatgtttcgttgctttatagacacccgcctcttcggccactttggccattgcagcaggaagtaaaagatcaaaagggttgtcagctttcacactaactctctctttattaagtcggcgacgagatactaacaaagcattatagatgagaaattgatatagatcatatctcgcctggcttataggcccgtaactcgcatggtttttatgcaaatacggagtaaatatttgattatccaaataaaaataaattttaaaaattaacaaatgagttgaattttttccgcatcctccgctaaaacagttaattaaaagggagcatcaggcgaataaagtaacaatatcgatcgtatttattaaatacaaattaccgatatttaaccttataattacaattattttattaatgcaaatatatgtaaagcggggcattaaaaaaacgccccgtaatataactcagactaatcattaagcctacattgcgtaggctatttgattttattttgcccagaatgctgctttggcgcgctgcagcttttcgtaggccttcaacaacgactgatgtgcagcaaacgcgtgcagatcgctatctaccggttgcaggccgtaaaacgccgcttcgccgctcattgccgcactggcggcttctacggcatctgcgccgtacatgcgaacaaacgcattcagatattgcagcggctggcgatcttcttcctgtgccagtaataacaacgtttgcaggcagcgataatagttggcgcgttccggactaaatactgatgagttaaactccatcgtccattcggtccagaccagagcctgttccagatcgccaccagccagcgccagcatggcttttaattcaccgatacgcagggtgtaccaaccgttatccgacccggtcgccagacccaacagctcacgcacgcgggtaaagtcatcaaaaccttcttcatccagttgctcgatgaggttcaggtaatcttctttttcccactcgctgcctggtagcgaaagaatcgtttcacgtaaatggctgcccatactgttattcgcgagccacagatcttcagccggataaatatcggacatgccaggcacgataatacggcaagcataaacgcccagatgctcgtaatcggcaatataaacttctttatcttctttgttgaagatagccatcagtgtggcgaactcttcttccgtggtgccggagaaattccagtccacaaacggataatcggcatcctgcttgaacaggtcccaggagattaaaccgctggaatcgataaagtgcgtttcgaggttggtatgttcagcgacttcttcatcatcgaaggttggcggagtaaacacatccaaatctttcaggccacgaccttgcagcagctcggtcacggtacgttccagtgctacgccaaaatcaggatgcgcaccgaaagaggcaaagcaggtaccgttagcaggattgaacagtaccacgcaaatcaccggatactggccgccaagcgaaccgtcataagcgaagattgggaaaccctccgcttccagcgtttcgatggcttcaactactgctgggtaacgcgccagcacgtctgccgggatctctggcaggctgatgctttcagcaataatgcggtttttcacgtagcgttcgaaaacttcagacaatccctgaacgcgtgcttcgttgcgggtattacctgcggacataccgttggagacgtacaggttaccaatgatattcatcggaatataaacggtctgattgtcggactgacgcgtaaacggcaggccgcaaataccacgatcttcgttaccggattgtaggtcaatcagcatgctgccggtcagttcattctccggatcataaaacgcgcgcagacggtcatcgagcagcccttctggcacatcgtcattttcggtcagtgggaaccatttttcgttgggataatgcacgaacggaccgttggcgatggtttcgcccagccagaagtccgcaaaaaagtagttggttgagagacgctcgaaatattcaccgagtgcagaagccagcgccgctttcttggttgcgcctttaccgttggtaaaacacagtgcgcactctttgtcgcgaatatgtacagaccagacgttaggcacgggattcagccaggaggcctcttcaatctgaaagccgaggtctgaaagtttttgctggaagcgagcgatggaatcttccagagcggcatctttgccggggataaatgtttgcgtcatgaaaatcactttagtcgtacggaaagcgcgcaataatacgggttttatctcaaaggcgctatcaccgccgccatgccgatgaactgttgactatgcttttagcggataaaccacgttaagagcataaaaatgaaggcgttcgatctccaccgtatggcatttgataaagtgccttttgatttccttggcgaagttgcactacgtagtctttatacctttgtactggtctttttgttcctcaaaatgaccggaagacgcggtgtgcggcagatgtcgctgtttgaagttttaatcattctgacgctgggatcagcggcgggagatgtggcgttttatgatgatgtgccgatggtcccggtacttatcgtctttattactctggcgttgttataccgcctggtaatgtggttgatggcgcacagtgaaaaactggaagatcttctggaaggcaagccagttgtcattattgaagatggcgagctggcctggtcgaaactcaataactccaacatgacggaatttgagttctttatggagctacgattgcgtggcgtggagcagctggggcaggtacgtctggcgattctcgaaaccaacgggcaaatcagtgtctatttctttgaagatgacaaggtgaaaccgggtttacttattttacccagtgattgtacgcagcgttacaaagtggtgccggagtcggcggactatgcctgtattcgttgtagtgaaatcattcatatgaaagcgggggaaaaacaattatgtccgcgctgtgcaaatccagaatggacgaaggcaagtcgggcaaaacgggtgacctgacagtaaaaacatcggctttttgctaataatccgagagattcttttgtgtgatgcaagccacatttttgccctcaacggttttactcattgcgatgtgtgtcactgaatgataaaaccgatagccacaggaataatgtattacctgtggtcgcaatcgattgaccgcgggttaatagcaacgcaacgtggtgaggggaaatggctcaaatcttcaattttagttctggtccggcaatgctaccggcagaggtgcttaaacaggctcaacaggaactgcgcgactggaacggtcttggtacgtcggtgatggaagtgagtcaccgtggcaaagagttcattcaggttgcagaggaagccgagaaggattttcgcgatcttcttaatgtcccctccaactacaaggtattattctgccatggcggtggtcgcggtcagtttgctgcggtaccgctgaatattctcggtgataaaaccaccgcagattatgttgatgccggttactgggcggcaagtgccattaaagaagcgaaaaaatactgcacgcctaatgtctttgacgccaaagtgactgttgatggtctgcgcgcggttaagccaatgcgtgaatggcaactctctgataatgctgcttatatgcattattgcccgaatgaaaccatcgatggtatcgccatcgacgaaacgccagacttcggcgcagatgtggtggtcgccgctgacttctcttcaaccattctttcccgtccgattgacgtcagccgttatggtgtaatttacgctggcgcgcagaaaaatatcggcccggctggcctgacaatcgtcatcgttcgtgaagatttgctgggcaaagcgaatatcgcgtgtccgtcgattctggattattccatcctcaacgataacggctccatgtttaacacgccgccgacatttgcctggtatctatctggtctggtctttaaatggctgaaagcgaacggcggtgtagctgaaatggataaaatcaatcagcaaaaagcagaactgctatatggggtgattgataacagcgatttctaccgcaatgacgtggcgaaagctaaccgttcgcggatgaacgtgccgttccagttggcggacagtgcgcttgacaaattgttccttgaagagtcttttgctgctggccttcatgcactgaaaggtcaccgtgtggtcggcggaatgcgcgcttctatttataacgccatgccgctggaaggcgttaaagcgctgacagacttcatggttgagttcgaacgccgtcacggttaatgccgaaattttgcttaatccccacagccagcctgtggggtttttatttctgttgtagagagttgagttcatggaatccctgacgttacaacccatcgctcgtgtcgatggcactattaatctgcccggttccaagagcgtttctaaccgcgctttattgctggcggcattagcacacggcaaaacagtattaaccaatctgctggatagcgatgacgtgcgccatatgctgaatgcattaacagcgttaggggtaagctatacgctttcagccgatcgtacgcgttgcgaaattatcggtaacggcggtccattacacgcagaaggtgccctggagttgttcctcggtaacgccggaacggcaatgcgtccgctggcggcagctctttgtctgggtagcaatgatattgtgctgaccggtgagccgcgtatgaaagaacgcccgattggtcatctggtggatgcgctgcgcctgggcggggcgaagatcacttacctggaacaagaaaattatccgccgttgcgtttacagggcggctttactggcggcaacgttgacgttgatggctccgtttccagccaattcctcaccgcactgttaatgactgcgcctcttgcgccggaagatacggtgattcgtattaaaggcgatctggtttctaaaccttatatcgacatcacactcaatctgatgaagacgtttggtgttgaaattgaaaatcagcactatcaacaatttgtcgtaaaaggcgggcagtcttatcagtctccgggtacttatttggtcgaaggcgatgcatcttcggcttcttactttctggcagcagcagcaatcaaaggcggcactgtaaaagtgaccggtattggacgtaacagtatgcagggtgatattcgctttgctgatgtgctggaaaaaatgggcgcgaccatttgctggggcgatgattatatttcctgcacgcgtggtgaactgaacgctattgatatggatatgaaccatattcctgatgcggcgatgaccattgccacggcggcgttatttgcaaaaggcaccaccacgctgcgcaatatctataactggcgtgttaaagagaccgatcgcctgtttgcgatggcaacagaactgcgtaaagtcggcgcggaagtggaagaggggcacgattacattcgtatcactcctccggaaaaactgaactttgccgagatcgcgacatacaatgatcaccggatggcgatgtgtttctcgctggtggcgttgtcagatacaccagtgacgattcttgatcccaaatgcacggccaaaacatttccggattatttcgagcagctggcgcggattagccaggcagcctgaatgaacaacgggcaataaatagccaaatctttctttatcaaaacgtcggcacattgtcggcgttttttttcggaccttgtgagtcattttgattaatggtagcgtcgcttgtcaatgtaagttgttgatacataatatttatatatgattaatcaacggatgattcacatgaagaatactaaattactgctggcgattgcgacctctgcagcattactgacagggtgtcaaaatacccacggtattgataccaatatggctatcagctccggtttaaatgcctataaagcagcaacattaagcgatgccgatgcaaaagcgattgccaatcagggctgtgccgaaatggacagcggcaatcaagtcgcaagtaaatccagcaagtacggtaaacgtctggcaaaaatcgccaaagcattgggtaacaatattaatggcacgccggtcaactataaggtttatatgaccagcgacgtcaacgcatgggcgatggcgaacggctgtgttcgtgtctacagtggcctgatggacatgatgaatgacaacgaaattgaaggcgttctgggccatgaactgggccacgtcgcgttgggtcactcgctggctgaaatgaaagcttcttatgcgatcgttgccgcacgcgatgccatttcagctaccagcggtgtggcttcccagctttcccgctcacaattaggtgatatcgcagaaggcgctatcaatgctaaatactcccgtgataaagagtccgaagcagatgatttctcctttgatctgttgaagaaacgtggcatcagcacccaggggctggttggcagctttgaaacactggctagcctggatggcggtcgcacccagtccatgtttgactctcacccaccatcaacagagcgtgcgcaacacatccgtgatcgtatcgcctctggtaagtaaatcattgtcatctttcgggctggtcttctgccagcccgctataattgcgcaataaatccccatctgaatacagacaaaactggtttttgcacacaacgttaacgatttgtggcgtcggcgcgtataatgcgcgcggttatgttaacggtacgcctgttttaaggagataaagatgacggcaattgccccggttattaccattgatggcccaagcggtgcagggaaaggcaccttgtgtaaggctatggcggaagcgttgcaatggcatctgctggactcgggtgcaatttatcgcgtactggcattggcggcattacatcaccatgttgatgttgcgtcggaagatgcgctggtaccgctggcatcccatctggatgtacgttttgtgtcgaccaatggcaatctggaagtgatcctcgaaggggaagatgtcagcggcgaaattcgtactcaggaagtggcgaatgcagcttcacaagtcgcggcattcccacgcgttcgtgaagcattattgcgtcgccaacgcgcgtttcgcgaattaccaggtctgattgccgatggccgcgacatgggaacggtggtattccctgatgcaccagtgaaaattttccttgacgcctcctcggaagaacgtgcgcatcgccgcatgctacagttgcaggagaagggctttagtgttaactttgagcgccttttggccgagatcaaagaacgcgacgaccgcgatcgtaaccgagcggtagcgccactggttccggcagccgatgctttagtgttggattccaccaccttaagcattgagcaagtgattgaaaaagcgctacaatacgcgcgccagaaattggctctcgcataagcgaccgaatttgcagtacccccgttgcaatggaatgacagcgggtatgttaaacaaccccatccggcatggagccaggtggacgttaaatataaacctgaagattaaacatgactgaatcttttgctcaactctttgaagagtccttaaaagaaatcgaaacccgcccgggttctatcgttcgtggcgttgttgttgctatcgacaaagacgtagtactggttgacgctggtctgaaatctgagtccgccatcccggctgagcagttcaaaaacgcccagggcgagctggaaatccaggtaggtgacgaagttgacgttgctctggacgcagtagaagacggcttcggtgaaactctgctgtcccgtgagaaagctaaacgtcacgaagcctggatcacgctggaaaaagcttacgaagatgctgaaactgttaccggtgttatcaacggcaaagttaagggcggcttcactgttgagctgaacggtattcgtgcgttcctgccaggttctctggtagacgttcgtccggtgcgtgacactctgcacctggaaggcaaagagcttgaatttaaagtaatcaagctggatcagaagcgcaacaacgttgttgtttctcgtcgtgccgttatcgaatccgaaaacagcgcagagcgcgatcagctgctggaaaacctgcaggaaggcatggaagttaaaggtatcgttaagaacctcactgactacggtgcattcgttgatctgggcggcgttgacggcctgctgcacatcactgacatggcctggaaacgcgttaagcatccgagcgaaatcgtcaacgtgggcgacgaaatcactgttaaagtgctgaagttcgaccgcgaacgtacccgtgtatccctgggcctgaaacagctgggcgaagatccgtgggtagctatcgctaaacgttatccggaaggtaccaaactgactggtcgcgtgaccaacctgaccgactacggctgcttcgttgaaatcgaagaaggcgttgaaggcctggtacacgtttccgaaatggactggaccaacaaaaacatccacccgtccaaagttgttaacgttggcgatgtagtggaagttatggttctggatatcgacgaagaacgtcgtcgtatctccctgggtctgaaacagtgcaaagctaacccgtggcagcagttcgcggaaacccacaacaagggcgaccgtgttgaaggtaaaatcaagtctatcactgacttcggtatcttcatcggcttggacggcggcatcgacggcctggttcacctgtctgacatctcctggaacgttgcaggcgaagaagcagttcgtgaatacaaaaaaggcgacgaaatcgctgcagttgttctgcaggttgacgcagaacgtgaacgtatctccctgggcgttaaacagctcgcagaagatccgttcaacaactgggttgctctgaacaagaaaggcgctatcgtaaccggtaaagtaactgcagttgacgctaaaggcgcaaccgtagaactggctgacggcgttgaaggttacctgcgtgcttctgaagcatcccgtgaccgcgttgaagacgctaccctggttctgagcgttggcgacgaagttgaagctaaattcaccggcgttgatcgtaaaaaccgcgcaatcagcctgtctgttcgtgcgaaagacgaagctgacgagaaagatgcaatcgcaactgttaacaaacaggaagatgcaaacttctccaacaacgcaatggctgaagctttcaaagcagctaaaggcgagtaattctctgactcttcgggatttttattccgaagtttgttgagtttacttgacagattgcaggtttcgtcctgtaatcaagcactaagggcggctacggccgcccttaatcaatgcagcaacagcagccgcttaatttgcctttaaggaaccggaggaatcatgaccaagtcagaattgatagaaagacttgccacccagcaatcgcacattcccgccaagacggttgaagatgcagtaaaagagatgctggagcatatggcctcgactcttgcgcagggcgagcgtattgaaatccgcggtttcggcagtttctctttgcactaccgcgcaccacgtaccggacgtaatccgaagactggcgataaagtagaactggaaggaaaatacgttcctcactttaaacctggtaaagaactgcgcgatcgcgccaatatttacggttaagttttttactcaaacttgaacgagagaaaagcacctgtcgggtgcttttttcatttctctaatctggaactggaagctgcctcgcagagttttgaacagttttcaccctttcgttaaattcttctgaatatgcctcggggaacgcaaaattcccaccagacaaccgctcaacaaagttgcacactttccataaacagggaggggtgcatgaaaataacgacagtcggtgtatgcataattagcggaatttttccgttgctgattttgccccaattgcctgggacattaacccttgcgtttctgactctcttcgcctgcgtactggcatttatccctgttaaaaccgtccgttatatcgcgctgacgttgctgtttttcgtttggggcatattatcagcaaagcaaattttgtgggcaggagaaaccttaactggcgcgacgcaggatgcaattgttgagatcactgcaactgacggcatgaccactcattacggtcaaattactcatctacaaggtcgacgtatattccctgcgtcaggtctcgtgatgtatggcgaatatcttccgcaagcggtttgtgctggacaacaatggtcaatgaaactcaaagttcgtgcagttcatggccaacttaatgatggcggctttgatagccagcgttatgccattgcccagcatcagccgctcaccggccgttttctgcaggcaagtgtcattgaaccgaattgtagcctgcgtgcacagtatctggcgtcactacaaacaacgctgcaaccctatccgtggaatgcggttattcttggtttaggtatgggggaacggttatccgtccccaaagaaatcaaaaatatcatgcgcgatactggaacggcgcatttaatggcgatatcgggattgcacatcgcttttgcggcgttgctggctgccggactcattcgcagtggacaaatttttctgcctgggcgctggatccactggcaaataccattaattggcggaatctgctgtgctgctttttatgcctggttgacgggaatgcaacctcctgcattgcgtaccatggtggcgcttgctacgtggggaatgcttaagttaagtgggcgacagtggagtggctgggatgtatggatatgttgtctggcggcaattttgctgatggatcctgttgccattctctcgcaaagtttatggctctctgccgctgcggtcgcggcattgatattttggtatcagtggtttccctgtcctgagtggcaactgccgccggtattgcgtgcagttgtttccctcatccatctgcaactgggaatcacacttctgcttatgcccgtgcaaatcgtcatatttcatggcattagtctgacctcgtttattgcaaatctattagcaattcccttggtgacatttatcacggttccgttgatcctcgccgcgatggttgtgcatttaagcgggccgttaatcctggagcaagggttatggtttcttgccgaccggtctttggctttacttttctgggggttaaagagtttgccggaagggtggatcaacattgctgaatgttggcaatggctatcattttccccatggttcttactggtggtatggcgattaaacgcctggcgaacgttgccagcaatgtgtgtggctggaggcttgctgatgtgctggccgctgtggcaaaaacctcgacctgacgagtggcagctgtacatgcttgatgtcgggcaagggctggcaatggtgatagccagaaacggcaaagcgattctctatgacacaggactggcctggcctgaaggggatagtgggcaacaactgattatcccctggctccactggcataatcttgaaccggaaggcgttattctgagccatgaacatctggatcaccggggagggctggattcaatattgcatatatggccgatgttatggatcagaagtccgttaaactgggaacatcatcagccctgtgtgcgtggcgaagcgtggcaatggcaaggattgcgtttcagcgcgcactggcctttacaaggtagcaacgataaaggaaataaccattcctgtgtggttaaggttgatgacgggacgaatagcattcttctaaccggtgatattgaagccccagctgaacaaaagatgctaagccgttactggcagcaagtgcaggcaacattgcttcaggtacctcaccatggcagtaatacctcatcatcgttgccattaattcagcgagtgaatggaaaagtggcactcgcatcggcatcgcgctataacgcatggcgactgccctctaacaaagttaagcatcgctatcaactgcaaggatatcaatggattgatactccacatcaaggtcaaacaacggtcaatttttcagcgcaaggctggcggattagcagcctcagggagcaaattttacctcgttggtatcatcagtggtttggcgtgccagtggataacgggtagaatatgcggctatttcaacaaatgctggttttttgaatgcataacgacaaagatctctctacgtggcagacattccgccgactgtggccaaccattgcgcctttcaaagcgggtctgatcgtggcgggcgtagcgttaatcctcaacgcagccagcgataccttcatgttatcgctccttaagccacttcttgatgatggctttggtaaaacagatcgctccgtgctggtgtggatgccgctggtggtgatcgggctgatgattttacgtggtatcaccagctatgtctccagctactgtatctcctgggtatcaggaaaggtggtaatgaccatgcgtcgccgcctgtttggtcacatgatgggaatgccagtttcattctttgacaaacagtcaacgggtacgctgttgtcacgtattacctacgattccgaacaggttgcttcttcttcttccggcgcactgattactgttgtgcgtgaaggtgcgtcgatcatcggcctgttcatcatgatgttctattacagttggcaactgtcgatcattttgattgtgctggcaccgattgtttcgattgcgattcgcgttgtatcgaagcgttttcgcaacatcagtaaaaacatgcagaacaccatggggcaggtgaccaccagcgcagaacaaatgctgaagggccacaaagaagtattgattttcggtggtcaggaagtggaaacgaaacgctttgataaagtcagcaaccgaatgcgtcttcaggggatgaaaatggtttcagcctcttccatctctgatccgatcattcagctgatcgcctctttggcgctggcgtttgttctgtatgcggcgagcttcccaagtgtcatggatagcctgactgccggtacgattaccgttgttttctcttcaatgattgcactgatgcgtccgctgaaatcgctgaccaacgttaacgcccagttccagcgcggtatggcggcttgtcagacgctgtttaccattctggacagtgagcaggagaaagatgaaggtaagcgcgtgatcgagcgtgcgactggcgacgtggaattccgcaatgtcacctttacttatccgggacgtgacgtacctgcattgcgtaacatcaacctgaaaattccggcagggaagacggttgctctggttggacgctctggttcgggtaaatcaaccatcgccagcctgatcacgcgtttttacgatattgatgaaggcgaaatcctgatggatggtcacgatctgcgcgagtataccctggcgtcgttacgtaaccaggttgctctggtgtcgcagaatgtccatctgtttaacgatacggttgctaacaacattgcttacgcacggactgaacagtacagccgtgagcaaattgaagaagcggcgcgtatggcctacgccatggacttcatcaataagatggataacggtctcgatacagtgattggtgaaaacggcgtgctgctctctggcggtcagcgtcagcgtattgctatcgctcgagccttgttgcgtgatagcccgattctgattctggacgaagctacctcggctctggataccgaatccgaacgtgcgattcaggcggcactggatgagttgcagaaaaaccgtacctctctggtgattgcccaccgcttgtctaccattgaaaaggcagacgaaatcgtggtcgtcgaggatggtgtcattgtggaacgcggtacgcataacgatttgcttgagcaccgcggcgtttacgcgcaacttcacaaaatgcagtttggccaatgatcgaaaaaatctggtctggtgaatcccctttgtggcggctattgctgccactctcctggttgtatggcctggtgagtggcgcgatccgtctttgctataaactaaaactgaagcgcgcctggcgtgcccccgtaccggttgtcgtggttggtaatctcaccgcaggcggcaacggaaaaaccccggtcgttgtctggctggtggaacagttgcaacagcgcggtattcgcgtgggggtcgtatcgcggggatatggtggtaaggctgaatcttatccgctgttattgtcggcagataccacaacagcacaggcgggtgatgaacctgtgttgatttatcaacgcactgatgcgcctgttgcggtttctcccgttcgttctgatgcggtaaaagccattctggcgcaacaccctgatgtgcagatcatcgtaaccgacgacggtttacagcattaccgtctggcgcgtgatgtggaaattgtcgttattgatggtgtgcgtcgctttggcaatggctggtggttgccggcggggccaatgcgtgagcgagcggggcgcttaaagtcggttgatgcggtaatcgtcaacggcggtgtccctcgcagcggtgaaatccccatgcatctgctgccgggtcaggcggtgaatttacgtaccggtacgcgttgtgacgttgctcagcttgaacatgtagtggcgatggcggggattgggcatccgccgcgcttttttgccacgctgaagatgtgtggcgtacaaccggaaaaatgtgtaccgctggccgatcatcagtctttgaaccatgcggatgtcagtgcgttggtaagcgccgggcaaacgctggtaatgactgaaaaagatgcggtgaaatgccgggcctttgcagaagaaaattggtggtatttgcctgtagacgcacagctttcaggtgatgaaccagcgaaactgcttacgcaactaaccttgctggcttctggcaactagttacgccgcggcagcgttcgattgatggagtcatgaatgtcgctgccgcacctctcccttgctgatgcgcgtaatcttcaccttgccgcacaaggcctgttaaacaaaccccgccgtcgagcgtcgttggaggatattccggcaacgatctcccgcatgtccttgctgcaaatcgataccatcaatattgttgcccgtagtccatatctggtgcttttcagtcgtctgggaaattatcctgcccagtggctggatgagtctctggcgcgtggcgaattaatggaatactgggcgcatgaagcctgctttatgccgcgtagcgactttcgtcttattcgccaccgcatgctggcacctgaaaaaatgggctggaaatacaaagacgcctggatgcaggaacatgaggcggaaattgcacagttaattcagcatattcatgataaggggccggtacgttcagccgattttgagcatcctcgtaaaggtgcaagcggctggtgggaatggaagccgcataaacggcatctggaaggtttatttactgccggaaaggtgatggtgattgaacggcgcaacttccagcgcgtttatgatttaacccaccgtgtcatgcctgactgggatgatgagcgcgatctcgtttcgcaaacagaagcagaaatcatcatgctggataacagtgcgcgtagcctgggaatattccgcgaacagtggctggcagattactatcggctgaaacgtccggcactggcggcgtggcgcgaagcgagggctgaacagcagcaaatcattgctgtgcatgttgaaaaattgggcaatctttggctgcatgatgatttgctgccgctactcgagcgagcgctggccggaaagctcactgcaacgcacagcgcggtactttcgccttttgatcctgttgtctgggatcgcaaacgcgcagagcagctttttgattttagctaccggctggagtgctataccccagcgccgaaacgccagtatggctattttgttctgccgttattacatcgtgggcaattagttgggcgaatggatgccaaaatgcatcgccagacaggcatccttgaagttatctctctgtggttacaggaaggtattaaaccaacgacaacgctgcaaaaagggctacgtcaggcgattactgatttcgctaactggcagcaggcaacgcgggtgacattaggatgctgcccgcaaggcctctttactgattgccgcaccggctgggaaatagaccccgtcgcataaatgattatgataagatttatgcattcataacccgatccatctggaggaactatggatcatcgtctgcttgaaatcattgcctgcccggtttgcaacggaaaactttggtataaccaggaaaaacaagagcttatttgcaaactggacaacctcgctttcccgctgcgtgatggcattccagtgttgctggaaacggaagcccgcgtgctgactgctgatgagagtaaatcatgagttttgtggtcattattcccgcgcgctacgcgtccacgcgtctgcccggtaaaccattggttgatattaacggcaaacccatgattgttcatgttcttgaacgcgcgcgtgaatcaggtgccgagcgcatcatcgtggcaaccgatcatgaggatgttgcccgcgccgttgaagccgctggcggtgaagtatgtatgacgcgcgccgatcatcagtcaggaacagaacgtctggcggaagttgtcgaaaaatgcgcattcagcgacgacacggtgatcgttaatgtgcagggtgatgaaccgatgatccctgcgacaatcattcgtcaggttgctgataacctcgctcagcgtcaggtgggtatggcgactctggcggtgccaatccacaatgcggaagaagcgtttaacccgaatgcggtgaaagtggttctcgacgctgaagggtatgcactgtacttctctcgcgccaccattccttgggatcgtgatcgttttgcagaaggccttgaaaccgttggcgataacttcctgcgtcatcttggtatttatggctaccgtgcaggctttatccgtcgttacgtcaactggcagccaagtccgttagaacacatcgaaatgttagagcagcttcgtgttctgtggtacggcgaaaaaatccatgttgctgttgctcaggaagttcctggcacaggtgtggatacccctgaagatcttgagcgcgttcgcgctgaaatgcgctaatttcacttcacgacacttcagccaattttgggaggagtgtcgtaccgttacgattttcctcaatttttcttttcaacaattgatctcattcaggtgacatcttttatattggcgctcattatgaaagcagtagcttttatgagggtaatctgaatggaacagctgcgtgccgaattaagccatttactgggcgaaaaactcagtcgtattgagtgcgtcaatgaaaaagcggatacggcgttgtgggctttgtatgacagccagggaaacccaatgccgttaatggcaagaagctttagtacgcccggaaaagcccgacaactggcatggaaaaccaccatgctggcaagaagtgggactgtccgtatgccgactatttatggtgtgatgacgcatgaagaacaccccggccccgatgtcctgctactggagcggatgcgtggtgtttcggtggaggcaccagcccgaacaccagaacgctgggaacaactcaaagaccaaatcgttgaagccttactggcctggcaccgtcaggacagtcgcggttgcgtcggcgcggtcgacaatactcaggaaaatttctggccctcatggtaccggcaacatgttgaagtgctatggaccacgctcaatcagttcaataacaccggtctgacgatgcaggataagcggatcctgtttcgcactcgcgaatgtctcccggcattatttgaaggctttaacgacaattgtgtgctgattcacggtaacttctgtttacgcagcatgttgaaagattcgcgcagcgatcagttactggcgatggtcgggccgggactaatgctttgggcaccgcgagaatacgaactgttccgactaatggataattctctggcggaagatttgctctggagttacctgcaacgcgcgccagtggcggagtcgttcatctggcggcgttggttgtatgtgttatgggatgaagttgcgcaactggttaataccggacgatttagtcggcgcaacttcgatctggcatcaaaatcactcttgccgtggctcgcctgacgaaccttttagccactgccagatacggccaagcgtttcatagccaacacgatcgctatgcatcaaccagaccggagaagggattgcccgttcccacgggttaagcggcgagtcgatggccaactgattcgccggggctggtagcggatttaacccttcctgctgaaaaaagatcatcgcccgcggcagatgtgatgcggaggtcaccagcaggaaaggggcgtcaccaatcgcctgtttcactgctgcagcttcttcttcggtatcttttggcaaatccagggtgataatttgctcgcgcggcacgcccagcgattgcgcaactctggcacctacttccgctgtactcaccgtattggtttttgctacgcctcccgtgaagatcagttttgatcccggattttcgcgccataagcgaataccttcattcaggcgtggcagactgttattgattaaattagagctcggtgcccactgcgggttccaggtataaccacctccgagcaccacgatatagtccactttttgcgaattattccatgtcggataggtgctttcgatgggacgcagcaggcggtcggctaccggttgcaaactcaataacaagagcgccagccacccaatgctaataaaaatcttcccggttttttgaaaacggctaaaccacagcagcgccaggccagcgccaataatcaacaacatcagcggaagtggcagcaacatattgccaatcacttttttcagtgtaaaaagcatcctttctggttccttttttaaccatatagcaagggatcgccagcgatattacaccagacgggttcattctcgccgtggctgtgacaaaatagcgtctttatcagaaaacgtcttagccaaccggtggagaaagcaatgcaggatcgcaattttgatgatattgcggaaaagttttcccgtaacatttacggcaccaccaaagggcagcttcgacaggctattctgtggcaggatctcgatcgcgtgctggcggaaatgggcccgcaaaaactgcgtgtgctggatgctggcggtggagaagggcagaccgcaatcaaaatggccgagcgtgggcatcaggtcattttatgcgatctttctgcgcagatgatcgaccgcgcaaaacaggcggcagaagcaaaaggtgtgagcgacaacatgcaatttatacattgcgccgctcaggatgttgcttcgcatttggaaacgcccgttgatctgatattgttccatgcggtgctcgagtgggtggctgatccccgcagcgtattgcagaccctctggtcagtgttgcgtccaggcggcgtgttgtcgttaatgttctacaatgcgcatggtttgttgatgcataacatggtcgccgggaattttgattacgtgcaggcgggaatgccgaaaaagaaaaaacggacgctttcgccagattatccacgcgacccggcgcaggtttatctgtggctggaagaagctggttggcaaattatgggtaagacaggcgttcgcgtgtttcatgattatctgcgcgagaaacaccagcagcgcgactgctatgaagcattacttgaattagaaacgcgttattgccgtcaggaaccgtatattaccctggggcgttatattcatgtcaccgcgcgcaaaccgcagagcaaggataaagtatgagtgaattttcccagacagtccccgaactggttgcctgggccagaaaaaatgacttctccatctcgctgccggtagaccgactctcttttctgctggcggttgccacgctgaacggcgagcgtctggatggtgagatgagtgaaggcgagctggtggatgcattccgccatgtgagtgatgcgtttgagcaaaccagcgaaaccatcggcgtgcgcgccaataacgcgatcaacgacatggtgcgtcaacgtctgctgaaccgctttaccagcgagcaggcggaagggaacgcaatttaccgtctgacgccgctcggcatcggcattactgactactacatccgtcagcgcgagttttctacgctgcgtctttctatgcagttgtcgattgtggcgggtgagctcaaacgcgcagcagatgccgccgaagagggcggtgatgaatttcactggcaccgtaatgtctatgcgccactgaaatattcggtagcagaaattttcgacagtatcgacctgacgcaacgtctgatggacgaacagcagcagcaggtgaaggacgatatcgcccagttgctgaacaaagactggcgggcggcgatttccagctgtgaattgttgctttcggaaacttccggaacgctgcgtgaattgcaggatacgctggaagcggcaggcgacaaattgcaggctaatctgttgcgcattcaggatgcgacgatgacccatgacgatctgcatttcgtcgatcgtctggtgttcgatctgcagagcaaactcgatcgtattatcagttggggccagcaatccatcgacttgtggattggctacgaccgccacgtacacaaatttattcgtaccgcgatcgatatggataaaaaccgcgtctttgctcagcggttacgtcagtcggtacaaacctattttgatgagccgtgggcgctaacttatgccaatgccgatcgtctgctggatatgcgtgacgaagagatggcactgcgcgatgaagaagtgactggggaacttcctgaggatctggaatacgaagagtttaacgagatccgcgaacagctggcggcgatcatcgaagaacaacttgccgtgtacaaaaccagacaagtgccgctggatcttggtctggtggtacgcgaatatctgtcacagtatccgcgtgcacgtcactttgacgttgcgcgtattgttattgatcaggcggtacgtcttggcgtagcgcaagcagatttcaccggactgccagcgaaatggcagccgattaatgattacggagccaaggtacaggcgcatgtcatcgacaaatattgaacaagtgatgccggttaagctggcgcaggcgctggcgaatccgttatttccggcgctggacagcgccttacgttcaggacgccatattggcctcgacgaactggataatcatgcattcctgatggattttcaggaatatctggaagagttttacgcgcgttataacgttgagcttattcgcgcaccagaagggttcttctatttacgcccacgttccaccacgctgatccctcgttccgtcttgtcggaactggatatgatggtcgggaaaatcctctgttatctctatctcagcccggaacggctggcgaatgaggggattttcacccagcaggaactgtacgacgaactgctcaccctggccgatgaagcaaaactgctgaaactggtgaacaaccgttcaaccggttcagacgttgaccgtcagaagttgcaggagaaagtacgttcttcgctcaaccgtctgcgtcgtttaggcatggtgtggtttatgggccacgacagcagcaagtttcgcattaccgaatcggtgttccgcttcggagccgatgtgcgtgctggcgacgatccccgtgaagcacagcgtcgcctgattcgtgatggcgaagcaatgccgattgaaaatcatctgcaactcaacgatgaaaccgaagagaatcagccagatagcggagaggaagaataatgattgaacgcggtaaatttcgctcactgacgctgattaactggaacggcttttttgcccgaacttttgaccttgacgagctggtcacgacgctttctggcggtaacggggcgggtaaatccaccaccatggcggcgttcgttacggcgctgatccccgacctgaccctgctgcatttccgtaacactacggaagccggggccaccagcggttcgcgcgataaaggtctgcacggtaagctgaaagcgggtgtctgttattcgatgctcgacaccattaactcgcgccaccagcgcgtggtggtcggtgtgcgtctgcaacaggttgccggacgcgatcgtaaagtggatatcaagccgtttgccattcagggactgccgatgtcggtgcagccgacacagctggtgaccgaaaccctgaacgaacgccaggcgcgcgtgctgccgcttaacgagctgaaagacaagctcgaggcgatggaaggcgtgcagtttaaacagttcaactccattactgattaccactcgctgatgttcgatctgggcatcatcgcgcgtcgtctgcgctccgcatctgaccgtagcaaattctatcgtctgatcgaagcttcgctgtatggcgggatctccagtgccattacccgttctctgcgcgactacctgttgccagaaaacagcggcgtgcgtaaagcgttccaggacatggaagcggcgctgcgtgaaaaccgtatgacgctggaagcgattcgtgtcacccagtcggaccgcgacctgtttaagcatctgatcagcgaagccaccaactacgtggcggcggactacatgcgtcacgccaacgagcgccgtgtccatctcgacaaagccctggagtttcgtcgcgagctacatacttcgcgtcagcaactggcggctgagcagtacaaacacgtcgatatggcgcgtgagctggcagagcacaacggtgccgaaggcgatctggaagcggattatcaggcggccagtgatcacctgaacctggtgcaaaccgcactgcgtcagcaggagaagatcgaacgctacgaagcggatctcgatgagctgcagatccgtctggaagagcaaaatgaagtggtggcagaagccatcgaacgccagcaagagaatgaggctcgtgcggaagctgccgaactggaagtggacgagctgaaaagccagcttgctgactaccagcaggcgctggacgtccagcaaacgcgcgcgatccagtataaccaggcgattgctgcgcttaatcgtgccaaagaactgtgccatctgccggacttaaccgccgactgcgccgccgaatggctggaaaccttccaggcgaaagagctggaagcgactgaaaaaatgctctctcttgagcagaaaatgagcatggcgcaaaccgcgcacagccagtttgagcaggcttatcagctggtggtggcaatcaacggcccactggcgcgtaacgaggcgtgggatgtcgctcgcgaactattgcgcgaaggggtcgatcagcgtcacctggcagagcaggttcagccgctgcggatgcgattaagcgaactggaacagcgtctacgcgagcagcaagaagctgagcgtctgctggcagatttctgcaaacgtcagggcaagaattttgatatcgacgaactggaagccctgcatcaggaactggaagcacgcattgcctctctttccgatagcgtgtctaacgcccgtgaagagcgcatggcactgcgccaggagcaggaacagctgcagtctcgcattcagagtttgatgcagcgtgcgccggtttggctggcagcgcaaaacagtctcaaccagttgagcgaacagtgcggcgaagagtttacctccagccaggacgtcaccgaatatctgcaacagttgctggagcgtgagcgagaggcgattgttgaacgcgatgaagtgggcgcgcgcaaaaacgccgtcgatgaagagatcgaacgtttaagccagcctggcggctctgaagatcagcgtctgaacgcgctggcggagcgttttggtggtgtgctgctgtcagaaatttatgacgacgttagcctggaagatgcgccgtacttctcagcgctgtatggcccgtcacgccacgccatcgtggtgccagatctgtcacaggtaactgaacacctggaaggcttgaccgattgcccggaagatctctatctgatcgaaggagatccgcagtcattcgatgacagcgtgttcagcgttgatgagctggaaaaagcggtagtggtgaaaatcgccgatcgtcagtggcgttattcacgtttcccggaagtgccgctgtttggtcgtgctgcgcgtgaaagccgtattgaaagcctccatgccgagcgtgaagtgctttccgaacgcttcgccacgctctcctttgatgtacagaaaactcagcgtctgcatcaggcgttcagccgctttatcggcagtcatctggcggttgcgtttgagtctgacccggaagcagaaatccgtcaactgaacagccgtcgcgtcgaactggagcgggcgttaagtaatcatgaaaatgataaccagcagcagcgtattcagtttgagcaggcgaaagagggcgttacggcgctgaaccgcattctgccgcgtctcaacctgttggctgatgacagcctggcggatcgcgtcgatgaaatccgcgaacgtctggatgaagcccaggaagccgcgcgttttgttcagcagtttggcaatcaactggcgaaactggaaccgattgtttcggtattgcagagcgacccggaacagttcgaacagttaaaagaagattacgcgtactctcagcagatgcagcgcgatgcccgtcagcaggcgtttgccctgacggaagtggtgcagcgtcgtgcgcactttagctattctgactcggcagaaatgcttagcggtaacagcgatctcaacgaaaaactgcgtgaacgtctggaacaggcggaagcggagcgtacccgcgctcgcgaagcgttgcgcggtcacgcagcgcagttgagtcagtacaaccaggtgctggcttcgctgaaaagttcttacgacaccaaaaaagagctactcaacgatctgcaacgtgaattgcaggatatcggcgtgcgtgctgatagcggggcagaagagcgggcgcgtattcgccgtgacgagctgcatgcgcaactgagcaataaccgttcacgccgcaatcaactggaaaaagcgcttaccttctgcgaagcggagatggacaacctgacccgcaaactgcgcaagctggagcgggattactttgagatgcgcgagcaggtagtgaccgccaaagcgggctggtgtgcggtgatgcgcatggtgaaagataacggcgttgagcgccgcttacaccgtcgtgagctggcttatctctccgctgatgatttgcgttccatgtcggataaggcgttaggtgcgctgcgtctggcggtggcggataacgaacatctgcgcgacgtgctgcgcatgtcggaagatccgaaacgtccggagcgtaaaattcagttcttcgtggcggtttatcagcatctgcgtgaacgtattcgtcaggatattattcgtaccgatgatccggtggaagctatcgaacagatggagattgaacttagccgtctgaccgaagaattaacctcccgtgaacagaaactggcgatcagttcccgcagcgtggcgaacatcattcgcaaaaccattcagcgcgagcagaaccgtatccgtatgctcaaccaggggttgcagaacgtatcgtttggtcaggtgaacagcgtgcgtctcaacgtgaacgtgcgtgaaacgcacgccatgctactggatgtgctctctgaacagcacgagcagcatcaggatctgtttaacagcaaccgtttgaccttctcggaagcgctggcgaaactgtatcaacgtcttaacccgcagattgatatggggcagcgcacgccgcagaccatcggtgaagaactgctggattaccgcaactatctggaaatggaagttgaggttaaccgtggttccgatggctggctgcgcgcagagtctggtgcattgtcgaccggtgaggcgattggtaccggtatgtcgattctggtgatggtggtacaaagctgggaagatgaatctcgccgcctgcgcggtaaagatatctctccttgccgcctgctgttcctcgatgaagcagcgcgactggatgctcgttctatcgccacgctgtttgaattgtgtgagcgtttgcaaatgcaactcatcatcgcagcgccggaaaatatcagcccggagaaaggcaccacctataaactggtgcgtaaagtcttccagaataccgaacacgttcatgtcgtcggcctgcgaggatttgcgccgcaactccctgaaacgcttccaggaactgacgaagcgccttctcaggcgagttaaaattaaggcggcagcaatgccgccttttctttttccgaaaactccgtttctgcactaaaaaagtggcacattacggcgcgcttttctttaaacttctttacattaggttatgtaaaaacgtatcggcgtttatatactgaagataagcctgatgagtaacaggcttgctcgtcatactttcgtgagtattggcgttgtacaggcaagtcgtaaaataacagcctggctattcagagtatgataaaaacagggggcaagggatgttgcttaatatgatgtgtggtcgtcagctgtcggcaatcagtttgtgcctggccgtaacattcgctccactgttcaatgcgcaggccgatgagcctgaagtaatccctggcgacagcccggtggctgtcagtgaacagggcgaggcactgccgcaggcgcaagccacggcaataatggcggggatccagccattgcctgaaggtgcggcagaaaaagcccgcacgcaaatcgaatctcaattacccgcaggttacaagccggtttatcttaaccagcttcaactgttgtatgccgcacgcgatatgcaacccatgtgggaaaaccgtgatgctgttaaagccttccagcaacagctggcagaggtggcgattgccggtttccagccgcagtttaataaatgggtagagttactgaccgatcctggtgttaacgggatggcacgcgacgtggtgctctctgatgcgatgatgggctatctccatttcattgcaaatattccggtcaaaggcactcgctggctatatagcagtaaaccttatgcacttgcaacgccgccgctctcggtgattaaccaatggcagctggcgctggataaaggtcaattgcctacgtttgttgcaggactggcaccgcagcatccgcaatatgcggcgatgcatgaatcgttactggccttactctgtgacaccaaaccgtggccccaactgaccggcaaagcaacgttgcgcccagggcagtggagtaacgacgtaccggcgttgcgcgaaatattgcaacgcacaggcatgttggacggggggccgaaaattactctacctggcgatgacacgccaactgacgcggtagtcagcccatccgctgttactgttgaaacagcagaaactaagccgatggataagcaaacgacgtctcgtagtaaacctgcgcctgccgttcgcgccgcctacgataatgaactggtggaagccgttaaacgttttcaggcatggcaaggattgggggcagatggtgctattggcccggcaacacgtgactggttaaacgtaacgcccgcccagcgtgctggtgtgttggctctcaacatccagcgattgcgcttgctgccaacagagctttctaccgggatcatggttaacattccggcctattcgctggtctactatcagaacggcaatcaggtgctggattcgcgagtcattgtcggtcgccccgatcgcaaaacgccgatgatgagcagtgcccttaacaacgtagtggtaaacccgccgtggaacgtacctccaactctggcacgcaaagatattctgccaaaagtgcgcaacgatccgggatatctcgaaagccatggctatacggtgatgcgcggctggaacagcagagaagcgattgacccatggcaggttgactggtctacaatcacggcctcgaatttaccgttccgcttccagcaggctccaggcccacggaactcgctggggcgctataaattcaatatgccgagttcagaggccatttatttgcatgacacgccgaaccacaatctgttcaagcgtgatacacgcgcattgagctcaggctgtgtacgagtgaataaagcttccgatctggcgaatatgctgttgcaggatgcaggctggaatgacaaacgtatttctgatgcgctgaagcagggtgatacacgttacgtcaatattcggcagtcgattccggtgaatctctactacctgacggcctttgttggtgcagatggtcgtacccagtatcgtacagatatttacaattatgatctgcctgcgcgatccagctcgcaaatcgtatcgaaagcggaacaattaatcaggtaaatgaagtagttcggggaaatcagttgtcgtaataattagcatgattgggggcgattctctgcagcccccgtcactgctggggttgagtcatcttgacgtctgctttacgggcggttaaggtgcctcttgtgcgccagaagtgcatataaacgataacattgacctgtagacttgattatcatggacaaattcgacgctaatcgccgcaaattgctggcgcttggtggcgttgcactcggtgccgccatcctgccgacccctgcgtttgcaacactctctaccccacgcccgcgcattttgacactcaataatcttcataccggagagtcaatcaaagcggagtttttcgatggcagaggctatattcaggaagaattggcaaaacttaaccattttttccgcgattaccgcgcgaacaaaataaagtccatcgacccaggattattcgaccagttgtatcgcctgcaagggttgttaggcacgcgcaaaccggtgcaactcatttccggttatcgttctattgataccaacaatgaactacgcgcccgcagccgtggagtagcgaagaaaagctatcacactaaaggccaggcgatggatttccatattgaaggtatcgcgttaagcaatattcgcaaagccgcgttatctatgcgcgcaggtggtgtaggatattatccacgtagtaactttgtgcatattgataccgggccagcacggcactggtagtaattgcttaacgaaacaggggcagtatgaactatcgtattattccggtcaccgcattctcccagaactgttcattaatctggtgtgaacaaacccgtctggccgcactggtcgatcctggcggcgatgcggaaaaaatcaaacaggaagttgatgacagcggcctgacactgatgcagatcctgctgacgcatggtcatctggaccacgttggcgcagcggcggaactggcgcaacattacggcgtgccggttttcggcccggaaaaagaagatgagttctggctgcaaggcttgcctgcgcaaagtcgtatgtttggtctggaagagtgccagccgctgacgccagatcgttggctgaacgaaggcgataccatcagcatagggaatgtgactttacaggtgttacattgccctgggcatacgccgggtcatgtcgtgttttttgatgatcgggcaaagctgctgatttctggcgatgttattttcaaaggcggagtagggcgcagtgacttcccgcgtggcgatcataatcaactgatttcttcaatcaaagataaattgctgccactgggggatgacgtgatatttattccgggtcacggaccattatccacacttggttatgaacgcctgcataatcccttcctgcaagacgaaatgcccgtctggtaaggcacataaaaaagcccgcttttaatgctggcctggatttctggcaaagtgcgctttgtttatgccggatgcggcacgagcgccttatccggcctacaaaatcgtgcaaattcaaaatattgcaggggacgcgtaggcctgataagcgtagcgcatcaggcaatgttgcgtttgtcatcagtctcagcccgcttttcagcgggcttcattgtttttaatgcttacagcactgccacaatcgcttcgcacagcggagccatgttatctggtgtcatcccggccacatttacgcgaccagaagcaaccgcatatacgccaaactcttcgcgcagacgcagcacttgttcttttgtcaggccactgaaggagaacatgccgttctgtttgatgataaagctgaagtcgcggtttgcgcctttttcctgcagcgtattgacgaacaactgacgcatacgctgaatacgctggcgcatatcagtcagctcttgttcccaaatcgcacgtaacgcatcgttgctcaggatggtggcaacaacagaagcgccgtgtgctggtgggttagagtagttagcgcgaatcgccgctttcatttggctgaatgcgcgatcaacggtttcactgtcggcagcaaccagagtacaagcgccaacacgctcgttgtacaggccaaagtttttagagtaggaactggcaacaatcagctctttatgcatagccgcgaaagcgcgcagtccttcagcatcttcttccagaccacgggcaaaaccctggtaagcgaagtcaaacagcggtaaccagcctttctcaacggagagttgtgccagtgtttgccattgttccagcgtagggtcgataccggttgggttatggcagcagccatggaacagcactacgtcgccagcctgagcttcattcaggctgttaatcagtgcatcgaagtcaagagtgtgattttccgcatcataataagcgtattcacgaacttccagacctgcagagttaaagacgctcttatggttcggccagcttgggttgctcacccacacacgcttaacgctggtattttttgccaggaaatcggcagccacgcgtagtgcgccagtgccccccggagtctgtgccgtgcgagcacgtttgtcattgatcagggcgctacctttaccaaacagcagttcctgagtgcagcgaccaaattcagggatgccgtcaatgccgaggtaatttttggtggtttcattttcgagcagatactgttcagcctttttcacgctggtcagtaccggggttttgcccgtctcatctttatagacaccaatcccgaggttaattttgccgggacgttcatcggcacgaaacagatcggccaggcccagaatcgggtcggcaggagcggcggtaatgttctcaaacatgacgaggttccattatggttacagaagggaagtccgctatcagggtaacgggagatttacaaaattccaactattactgatgaaaacgcaggctgtttttgcaagacgtgagattgctctggaaggtataaaaaaaacaggaccaaagtcctgttttttcggcatttaacaaagaggtgtgctattagaactggtaaacgatacccacagcaacggtgtcgtctgaacctacgcccagtttgttgtcagaatcgatctggttgatgatgtagtcaacataggtggacatgtttttgttgaagtagtaggttgcgcccacttcaaagtagttcaccagatcaacatcaccgataccttctacgtctttcgctttagatttggtgtaagcgatggacggacgcagaccgaaatcgaactggtattgcgcaactaacagaacgtcttgcgttttgttggcgaagccgctggtgtttgtaaatttattagtgatcggcgtagcgttacgggtttcaccgtagttcgctgccaggtagatgttgttcgcgtcgtacttcagaccagtagcccactgttcagcttttttaccgttgccaagaggttgagcttcttgcaggttggtacggtcagctgcaccataagcaccaacgataccaaagccttcgtattcgtagctgatagaaccgccaacaccgtcgccgttagaacggcgtgcagtgtcacgctcgtttttacccaggtactgaacagcgaagttcaggccatcaaccagaccaaagaagttggagttacgataggtagcaacgccgccaacacgaccaacgaagaagtcatcgctgtatgcagtatcaccaccaaattctggcagcatatcggtgtaacccagtgcatcataaaccacaccgtagttacggccgtaatcgaaagaaccaacgtcagcgtatttaagacccgcgaatgccagacgcgttttgttaccagtttgagcgtcagcgccttcagagttgttaccctggaagttatattcccactgaccataaccggtcagatcggaattgatttgagtttcccctttaaaaccaagacgggcataggtcatgtcgccattgccaccgtaactgttttcaccgttacccttggaaaaataatgcagaccaacagctttaccgtacagatctactttgttgccatctttgttatagatttctgcagcgtttgcagtacctgctactaacagagcagggacgatcactgccagaatattgcgcttcatcattatttattaccctcatggttttttttatgacacctgccactgccgtcaataagttctgtcaataaaaatttacggaactattgatgagagtttggtgtctttatgtgtctgcaggcatctttccattcaaactaacgtttcgctaccgtgaaagtgctacaaagataaagatttggtttcaaaaagaaaaaatatgtaaccaaaagtaaaatttaaggaactttgtgaacaccgtcatatttccatagagacgtgatgatatttacagcaattttaatctatttatatgatttccttatatttaaattaactaaacggaaattttgtttctgatggaaactttatcgacctggcacaaaatcttctttcagacatccagaatgccaaaaaatagtatgaaaattgtgctattagctaagaaaaaactaatccgcaataagaatgcggattagtttttgcgcgtaaatgttgcaatgtaatattccgtaacaggatgatcgttatggcggggttgcaaatagattgcttgacttaacaaacagataacttgacagaaaagataaaaaaagagccagcgggcgctggctcttgaagacgctaaattagaagctggcgttacgcggagtacgtgggaacggaatcacatcacgtacgttttgcacgccagttacgtaagcaatcagacgttcaaaaccaagaccgaaacctgaatgcggaacagtaccgtagcgacgcagatcgcgataccaccagtaatcttctttattcaggcccatttccagcatacgctcgtccagcacgtccagacgttcttcacgctgggagccaccaatgatctcaccgatgcccggagccagaacgtccatagccgcaacggttttaccgtcttcgttaaggcgcatatagaacgctttaatatctttcggatagtttttaaccactaccggtgctttaaagtgttcttccgccagataacgctcatgctcagaagagagatcgactccccagtaaaccgggttttcaaacttcctgccgcagttttcgagaatggtcactgcgtcggtataatccacctgcgcaaaatcggcttcaatgaagcgttccagacgtgaaacggcatctttatctacgcgttcagcgaagaatttcatgtcgtcagcgcgttcttcgagaaccgctttgaagacatatttcagcatggcttcagccagacccgcaatatcgttcaggttagcaaacgccacttccggctccagcatccagaattccgccaggtgacggctggtgttggagttttcagcacggaaagtcgggccgaaggtataaattttggacaatgcgcaagcgtaggtttcgccgttcaactggccagatacggtcaggaaagactctttaccaaagaagtctttgtcgaaatccactttgccctgatcgttacgcggcaggttttccagatccagcgtagaaacgcggaacatttcgcctgcaccttcggtatcagatgcggtaatcagtggcgttgaaacccagaagaatccctgctcgttaaagaagcgatgcagcgcctgcgccagcgtatggcgaacgcgcgcgacggcaccaatcaggtttgtgcgcggacgcaggtgagcgacttcacgcagatactcaatgctgtggcgttttgccgccatcgggtaagtgtctggatcttcaacccaaccagcaacttcaaccttgctggcctgaatttcaaattgttgcccctggcccggcgacgccacgactttacccgtcacaatgaccgagcagccggtggtcagacgcaggacgtcttcattgtaattgggcagagaattattgatgacagcctgtacaggatcaaagcaggaaccgtcataaacggcgaggaaggagatgccagcttttgaatctcggcgggtacgtacccatccgcgcacggtgacttcgctgtcaacggctacacggccctggagtacgtcggctacaggcacaacgctcataatattctctctgttaatagtcggaaaaaataaacacttgtccacccgtaaatggggggatacctatgttacctggcatctgcaatcagacaagcagaattcgcaaatgcagcgaaagatttcggaattaaaggtaaaaaaagggagccgattagctccctgatgatattaactggcttttttaatatgcggaaggtcgaacgctttgcgcagcgcccgaacaaacgctttatcatggcagatagttttgccagggctgtcagaaagtttcgccaccggtttaccgttacactctaccaacttaatgacaatattcaggggttttacctgggggatatcgcaggtcaggcgagtcccaataccaaaacttaattgcacgcgggaagagaagtggcggtatagctcaaccgctttgcgtaaatccagattgtcagagaaaaccagcgttttactctgtggatcaattcccagcttttcataatgtgcaatggctttttcaccccattcaaccgggtcgccagagtcatgacgcaggccctgataccgactagcgaactcgacaccgaaatcacgcaggaaagcatccatagtgatgcagtcggttaatgcaatgccaagttggtcgggatactcttccagccaggcagcaagtgcagctcgctggctgttggctagatccgggctgatttgctgatgtgcctggaaccattcgtgtgcctgtgttcccatcggcgtgagggaaagccgacgcgccagatcgtagttgctggtgcccacaaaccaggattcctgttgcagacgcttaacgatggtttcttgtacttcgcgagaaaaacggcgacgggtgccaaaatccatcagatggaagcgcgacatatcaagaccggcggttaacgccgagaagtcgactaatttgctttccagcgtgtcgagggcttgcgcaacgtcggcctgcggtgagcgatagcgatgtaccatttcactgataaccgccagcaaaggaacttcccagaggatgacttcacgccacgggccgcttaaacgaatatccagcttgccattatcgttggacacggtgacttgttccgggttaaagcggaactcgcgtaaccagttaagatagtcggccttaaagaaaggcagggcagaaagccactgatattcatcatcctgcaggcgcaggtgctgcatcgcctgaacctgttcacgaatagcatcggcataaatacccagcagatcgtcacctcggcaacgaaactccgccgcgacatgcacatcgtaatagtgatgaaacacggcttgctgcatatgcaacttataagcatctgtatccagcaacgagtgcagaacaggagaagcgaattgtgtcataggtgcgcagtagcgtcctcgtacaggagcgtttagtacaataaacatcttcaggaactgctggagtataccttgtttcgcaatttattgaaccccgatcacaccatatgccacctttctggtcgatggcattacgcggtgtatgttataaaaatgtagcaataaaggcgtttgtacctgaaaagatgaagattctgcatagcgcgatttacgcaacaggaatagactgaacaccagactctataaaagatgctaaaggttatttatgactcaacagccacaagccaaataccgtcacgattatcgtgcgccggattaccagattactgatattgacttgacctttgacctcgacgcgcaaaagacggtcgttaccgcggtcagccaggctgtccgtcatggtgcatcagatgctccccttcgtctcaacggcgaagacctcaaactggtttctgttcatattaatgatgagccgtggaccgcctggaaagaagaagagggcgcactggttatcagtaatttgccggagcgttttacgcttaagatcattaatgaaataagcccggcggcgaataccgcgctggaagggctttatcagtcaggcgatgcgctttgcacccagtgtgaagccgaaggtttccgccatattacgtattatctcgaccgcccggacgtgctggcgcgttttaccaccaaaattattgccgataaaatcaaatatcccttcctgctttccaatggtaaccgcgttgcgcaaggcgaactggaaaacggacgccattgggtacagtggcaggacccgttcccgaaaccgtgctacctgtttgcgctggtggcaggcgactttgatgtactgcgcgatacctttaccacgcgttctggtcgcgaagtagcactggagctgtacgtcgatcgcggcaaccttgatcgcgcgccgtgggcgatgacctcgctgaaaaactccatgaaatgggatgaagaacgctttggcctggagtatgacctcgacatctatatgatcgtcgcggtggatttcttcaatatgggcgcaatggagaataaggggctgaatatctttaactccaaatatgtgctggcccgcaccgacaccgccaccgacaaagattacctcgatattgaacgcgttatcggccatgaatatttccataactggaccggtaaccgagtgacctgtcgcgactggttccagctcagcctgaaagaaggtttaaccgtcttccgcgatcaggagttcagctctgaccttggttcccgcgcagttaaccgcatcaataatgtacgcaccatgcgcggattgcagtttgcagaagacgccagcccgatggcgcacccgatccgcccggatatggtcattgagatgaacaacttctacaccctgaccgtttacgagaagggcgcggaagtgattcgcatgatccacaccctgcttggcgaagaaaacttccagaaagggatgcagctttatttcgagcgtcatgatggtagtgcagcgacctgtgacgactttgtgcaggcgatggaagatgcgtcgaatgtcgatctctcccatttccgccgttggtacagccagtccggtacaccgattgtgaccgtcaaagacgactacaatccggaaaccgagcagtacaccctgaccatcagccagcgcacgccagccacgccggatcaggcagaaaaacagccgctgcatattccgtttgccatcgaactgtatgataacgaaggcaaagtgatcccgttgcagaaaggcggtcatccggtgaattccgtgctgaacgtcactcaggcggaacagacctttgtctttgataatgtctacttccagccggtgcctgcgctgctgtgcgaattctctgcgccagtgaaactggaatataagtggagcgatcagcaactgaccttcctgatgcgtcatgcgcgtaatgatttctcccgctgggatgcggcgcaaagtttgctggcaacctacatcaagctgaacgtcgcgcgtcatcagcaaggtcagccgctgtctctgccggtgcatgtggctgatgctttccgcgcggtactgcttgatgagaagattgatccagcgctggcggcagaaatcctgacgctgccttctgtcaatgaaatggctgaattgttcgatatcatcgacccgattgctattgccgaagtacgcgaagcactcactcgtactctggcgactgaactggcggatgagctactggctatttacaacgcgaattaccagagcgagtaccgtgttgagcatgaagatattgcaaaacgcactctgcgtaatgcctgcctgcgtttcctcgcttttggtgaaacgcatctggctgatgtgctggtgagcaagcagttccacgaagcaaacaatatgactgatgcgctggcggcgctttctgcggcggttgccgcacagctgccttgccgtgacgcgctgatgcaggagtacgacgacaagtggcatcagaacggtctggtgatggataaatggtttatcctgcaagccaccagcccggcggcgaatgtgctggagacggtgcgcggcctgttgcagcatcgctcatttaccatgagcaacccgaaccgtattcgttcgttgattggcgcgtttgcgggcagcaatccggcagcgttccatgccgaagatggcagcggttacctgttcctggtggaaatgcttaccgacctcaacagccgtaacccgcaggtggcttcacgtctgattgaaccgctgattcgcctgaaacgttacgatgccaaacgtcaggagaaaatgcgcgcggcgctggaacagttgaaagggctggaaaatctctctggcgatctgtacgagaagataactaaagcactggcttgataaataaccgaatggcggcaatagcgccgccattcggggaatttacccctgttttctcaggcgagtttcagattcaccacgttgcatcacccgttgcaacacctccgcttccagctccgctaatcgcaccgaccctaatcgacgcggacgggggatatccactgtcaaatccagaccaatttttccctcttcaattaacagcacccggtcagccatcgctaccgcttcgctcacatcatgcgtcaccaacagtacggtaaagccgtgctcctgccaaagtgacacaatcaaatcctgcatctcgagtcgcgttaaggcgtccagcgccccgagcggttcatcaagcaacaataatcccggtcgatgaatcaacgctcttgccagcgccactcgctgtttctgcccgccagaaagtgcggcaggccattcccctgcgcgattctccagtcctaccgcagccaacgctcgacgtgcggcatcgcgccactggcctttaaggcctaacccaacgttatcaatcaccgatttccacggtagcagacgcgcatcctgaaacatcattcgcgtgtcttcctgaatttcagccagcggtgtggtgcccgctaacacatcgcctgcggttggcgtttccagacctgccagcaggcgcagcagggtacttttgccaccaccgctgcggcccaccaccgccacaaactgacctgccggaatatgtaaatccagttggttcaggacgatattttccgcgtaatgtttgcttactgcattgagcaacaatggcgtgccctggttcagacgagcagtattcataccgtggcctccttcaaatgataagccgggttccagcgcaaccagaggcgctctaacagctgcgcgctgacgtcagccagtttgccgagcagggcgtaaagaataatagcgactaccaccacgtccgtttgcaaaaactcccgcgcattcatcgccagataaccaatgcctgaattggcagaaatggtttcggcaacaatcagcgtcagccacatcaggcccaacgcaaaacgcacgccgaccataattgagggcagggcaccaggcaggatcacatggataaacagcggtatgccggataatccatagctacgcgccatctccaccaacccgcgatcgatattacggatgccatgccaggtgttgatataaatggggaatagcgtaccgagcgccaccagaaagatttttgcggattcatcaatgccaaaccacaaaatcaccagcgggatcagcgccagatgcggcacgttgcgcaacatctgaattgaggtatccagcagccgttctccccagcgagatagcccgctaatcagtcccaaaatcaaccccagcgatccgccaattgaaaagccaatcagcgcccgccaggagctgatcgccagatgctgccacagttcgccgctggcggagagcgtccagaacgccgtcaccactccttccggtgaaggcaaaatacgcgtcgacagccagccaaccgaggaggccagttgccacaccgccacgatgcccaccggtaaaaaccagggggcaacgcgcaataaccacttcttcactggcgttgccattatttcttccttagctttgcgcgactttacgggggataaaatcattcgccaccgcttcgccttgcggattcagcggctgcggctggggaatttccgggatggcgacatccagaagcgggaacagcaactcgccaacccgatacgcttcttccagatgcggatagcccgaaagcacaaaactgtcgatgccaagcgcggcatattcgttgattcgcgcagcgaccgtaggaccatcgcccaccagcgccgtcccggcaccgccgcgcactaagccaacgcccgcccataaattggggctgatctccagattgtcgcgcttgccgttatgtaacgccgccattcgctgttgccctacggaatccgtccgggcgaatgcggcctgtgctttggcgatagtttcatcatcaagatgcgagattaaccgctcggcggcctgccacgcttcgtcgttagtttcacgaacaatcacatgcagacgaataccgaaacgaattttgcgtccatgcgcggcagctttcgcccgcacttgttcgattttctctttaaccagttccggcggttcgccccaggtgaggtagagatcaacctgttctgccgccagctcctgggcgacatctgacgatccgccaaagtaaagtggcggatacggctgttgaatcgccgggaagagcagttttgctccgcgcacatgaatatgtttaccgttgaaatcgacggtttctctctgcaataaacgccgccagacctgggtaaattccgccgaggcttcgtagcgctcgctatgatcaaggaacactccgtcgcctgccagctcttgtggatcgctgcctgtgaccaggttaaacaacgcacgtccatttgagagacggtcaagcgtggcggcctggcgggcggcaacggtaggtgaggttacgctgggacgcagggcgacaagaaacttcagccgctgcgtcaccgggatcatcgatgcggcaaccagccacgcatcttcgcaggagcgccccgttggaattagcacaccggtatagccaagacgatccgccgcttgcgcaatttgttgcagataaccgtgatcaaccgggcgtgaaccttcttccgttcccagataatgcccgtcaccgtgggtcggtaaaaaccagaacatattcagactcataattgttttccttccagttgagtgggctgccagatgcgctggcgaatatcgacttttttcggcaccagacgattttcataaaacagatctgccgtttgctgctgtaaggcggcaacctcggcgttaaccggtttgatggtggtaggagggcgatgatctaagtaagaggcaatcaccggtgccggtaagcccatcgtttttgccagtaaagcgatgctttgctcgcgctggctgcgggttaacgcatcggcctcactaaaggttgccagtacgccctgaataaaagcgccgtttttttctgcatagggacgagctgccagataaaacgatccagtttgattgagatcggtgccgtctttcagcacccgcacgccgccctgtaataatgcagcagagtagtagggatcccagatagcccaggcgtcaacgttaccttgctggaacgcggcgcgggcatcagcgggcgtcaggtaagtgggttggatatcggtaaacttaagtccggcctgacgcagtgcacgcagtaaaaggttgtgtgaactggaacctttctgaaaggcaactttgtgacctttaagatcggctacggttttgatcgggctgttttctgccaccagaatcacttcggctttgggcttcggtggctcgacgcccacgtacaccaaatcagccccggcagcctgggcaaagattggcggaatatccccggtactgccgagatcaatactgccaacgtttaacgcttccaacatttgcggacccgcggggaactccacccaggagatttttgattccggatagcgtttttccagtaactggtggctttttgccagcaccataccaatactgcctttctgatagcctatacgtaacgcttcaggcgaggattctgcagcaaccgcaaaagtagagacgctaagcaatcccgccagcgccagtttaatgatgttacgcatgggcattacctcgcagagacagaaggtcaggaacctgaacatcgcggcggtgcaatgcctgccagaaagtttctagcgcggtatcaagacgggtttgcagatttggcgtgaactggggtctgtgatggtaatcaattacttgtgagtcatcggcaaacacgccgtgcaggatctcctgagctttcagtgcgcttaaaactggtttaagggcataatcgaccgccagcagatgggccacggtaccgcccgtcgccagcggtagcaccactttgccttgcaaagcgcgttctggcagcaggtcgagcagggttttcaacgcaccggaataggcggctttatacacaggcgtggcgacaatcagcccatcggcctgttgcagctgttcggtgaaggtcttgagtgccggactatcgaaacgagcataaagtagatcttccggggcgaagttttgcagattccagtgataaacctctacatccaggccatttagtttttcccgcgcatattccagcaaggagctggagcgagaaggaaagcgaggactacccgccagggtgatgacacgcatactctctccttataaccaattgttctttttttgttaacattgataacaattcggtcagtctgtcggagagacaagaaaattccaaatataaattttgtgtatctttttctgaaaataaactaaagaaagggctttatatatcacgcatatttatttattggatagtcattagatgttgaatcaatgaattactcgttcagttaatatttaaatattcatgaaatctataaattaaagatttgtcacttattggatttagtatgcttgatttaaatggcggacaattattgttattattaagtctaatgtcatttaaaggcattatcatatttacgaagagatcaggatgataacgatgaaaaaaagtgtattgacggcgtttataactgtggtatgtgcaacgtccagcgttatggctgctgatgataatgctatcacggatggctcagtaacatttaatggtaaagttattgctccagcttgtaccctggtagctgcgacgaaagattccgtggtgactttgccagatgttagtgccacgaagttgcaaaccaatggtcaggtttctggcgtgcaaattgatgtgccaattgaattaaaagattgtgatactaccgtaacaaaaaatgcaacgttcacctttaatggcactgcggatactactcagattacagcgtttgctaaccaggcctcatctgatgctgctacaaacgtggccctgcaaatgtatatgaatgatggtacaacggccatcacgccagacacagaaaccgggaacattttgttgcaggatggagatcagacgttgacttttaaagttgattatatcgctacggggaaagcgacttcaggtaatgtgaatgcggtaacaaatttccatattaactattattaatagaactcattaattgttttattaattagtacccctccagtgttctggaggggatattcatattttttaagagtgactatttatgaaaacttgcataacaaagggaattgtgaccgtaagtttaacggcaatattactcagctgctcatccgcatgggcggcaggtaaaggcgggattggacttgcagcaacacgtcttgtttattcagaaggtgaagagcaaatttcactgggtgtacgtaacaccagtccggatgttccttatcttattcagtcatgggtgatgaccccagataataaaaaatcagcagactttattattacaccaccgctatttgtgctgaatccggcaaatgagaatctgttacgcattatgtacattggagcgccgttggcgaaagacagagaaacccttttcttcactagcgtacgggcagtcccttcaacaacgaagcggaaagagggaaataccctgaagattgccacacaaagcgtcatcaaacttttctggcgaccaaaaggtttagcgtatcccttaggcgaggctccggcgaaactgcgttgcacttcgtcagctgacatggttacggtcagtaacccaacaccttatttcattaccctgacagacctgaaaataggtggaaaagtagttaaaaatcaaatgatttccccctttgataaataccaattttctctgccaaagggggccaaaaatagcagcgtaacgtatcgaaccatcaatgactacggggcggaaacgccgcaactcaactgtaaatcgtaagccgtcttcagttaagagagcgagatgtatagaactcatcgacaacacagcctgttaagctctggtggagtgccatcgtttattggtgggctggtggtgtttgtgtcggcagcgttcaatgcacaagctgaaacctggttcgatcctgcttttttcaaagatgatccctcaatggtggccgatttgtctcgtttcgaaaaaggacaaaaaataacgccaggggtttatcgtgtcgatattgttctgaatcagacaattgtagatacgcgcaacgtcaattttgttgagataacgccagagaaggggattgccgcctgtttgacgactgaaagcctggatgcaatgggtgttaatactgatgcgtttccggcttttaaacaactggacaaacaagcgtgtgtgccattggcggagattattccggatgccagcgtaacgtttaatgtgaataaactccgtctggaaatttcagtaccgcaaatcgccatcaaaagtaatgcccgtggttatgtcccccctgaacgttgggatgaagggatcaacgcgctattactgggatattcgtttagcggggctaacagtattcatagcagcgcagacagtgattctggcgacagctattttctgaatttaaacagtggcgttaatttaggcccatggagattgcgcaacaattcaacatggagtcgtagtagtggccaaaccgcagaatggaagaatctcagcagctatttgcaacgggcggttattcctctgaaaggcgaactgaccgtaggtgatgattatactgcaggcgattttttcgatagtgtcagctttcgtggtgtgcagctggcgtcagatgacaacatgctgccagacagcctgaaagggtttgcgcctgtggtgcgtggtatcgccaaaagcaatgcccagataacgattaagcaaaatggttacaccatttaccaaacttatgtatcgcctggtgcttttgaaattagtgatctctattccacgtcgtcgagcggtgatttgttagttgaaatcaaagaagcggacggcagcgtcaatagctacagcgtaccgttctccagtgtgccattactccagcgtcaggggcgaatcaaatacgcggtgacactggcgaaatacagaaccaatagtaatgaacagcaggagagcaaatttgcccaggccacgttgcagtggggcggaccgtggggaacgacctggtatggtggtggacaatatgctgaatattaccgtgccgccatgtttggtctgggatttaacctcggcgatttcggagcaatttcgttcgatgcgacccaggcgaagagtacgctagcagatcaaagcgaacataaaggtcagtcatatcgttttctgtatgccaaaacgctcaaccacttgggcactaactttcaattgatgggctatcgctattcgacgtcgggtttctacaccctttccgacaccatgtataaacatatggatggctacgaatttaatgacggtgatgatgaagatacgccgatgtggtcgcgttattacaatttgttttacaccaaacgtggcaaactgcaggtcaatatctcccagcaattaggcgagtacggttcgttttatttaagtggtagccagcaaacttactggcatacggatcaacaggatcggctattacagtttggctacaacacgcaaattaaagatctttcgctggggatttcctggaactacagtaagtcccgtggtcaacctgatgctgatcaggtgtttgctctaaatttttccctgccgctcaatctgttgctccccagaagtaatgatagctataccaggaaaaaaaattacgcctggatgacctctaacaccagtatcgataacgaagggcacactacacaaaacctgggtttaacggagacattactcgatgacggtaacctgagctacagcgtgcaacagggatataacagcgaggggaaaacggctaatggtagcgccagcatggattacaaaggggcgtttgcggatgcccgagtgggctacaactacagcgataacggcagtcaacaacaactgaactacgctctttcaggcagtttagttgcccattcacagggcattaccctggggcaatcgctgggggaaactaacgttctgattgcagcaccaggcgcagagaatactcgtgtggcgaacagcaccgggctgaaaactgactggcgcggatataccgttgttccttatgccacttcttatcgggaaaatcgaatcgcacttgatgcggcgtcgttaaaacgtaacgtggatcttgaaaatgcagtagtcaacgtggttcccaccaaaggggcgttggttctggcggagttcaatgcccatgcgggtgcaagggtattaatgaaaacatcaaagcagggtataccgctgcgttttggcgcgatagcgacgctggacggcgtacaggctaatagcggcataattgatgatgatggctcgctctatatggcgggtttaccggcgaagggaacaataagcgtgcgctggggcgaagctcccgatcaaatttgtcatatcaattacgagcttaccgaacaacaaattaactctgcgattacgcgaatggatgccatatgcagataatctttggagaaaaatgcgtgtcattactacgactattttttgccgccgtcttaatgttatggtgcgctcaaaccgctgcttatagcgggcagtgtcatactactcaggggaatccgtatattggcgtcaattttggcgttaaaaccctggaggaagaagcaaatacggcaggggtagttaaagacaaattttatcagtggaacgaatcgaatgattattatgtttcctgtgattgcgataaagacaatgtcagaagtggccgatgggcattcgccgcggattcaccgttagtctatttaggcgacaactggtacaaaattaatgactatcttgccgccaaagttttattgcaggttaaaggcagttctcctactgcggttcctttcgaaaacgtgggcacagggggggatacccgatggcatatttgcgaccctggcggtcaacgtttaggtgggcagggggcaagcggtaatagcggtagcttttccctgaaaatattgcagccgttcgttggctcggtcgtcattcctcctatggcgctggcgcgattatatgaatgctacaacatacccgcaggtgattcctgcacgactacaggtacaccggttttagtgtattacctgtctggtacgatcaattcacttggctcatgttccgtcaatgccggagagacaattgaagttgatttaggtgatgtcttcgctgccaatttccgtgttgtagggcataaacctcttggggccagaacggcagaacttgcaattccagtcaggtgtaacacgggaaacgcgggattagttaatgtcaacctgagtctgacggcaaccacagaccccagctatccccaggcgattaagacgtcacgtcctggcgtgggcgtggtggtgaccgatagccagaacaacattatttcccctgctggtggaacattaccgctctctattcctgatgatgcagacagtatcgcgcgaatgaatgtctatccagtcagcacgacaggtgtaccaccagaaaccgggcgatttgaagccacggcaacggtgagaataaattttgattaacgcgtgaacgtatgaagaaaaaaacgatatttcagtgcgttatcttgttctttagcattcttaacatccatgtcgggatggctgggcctgaacaagttagtatgcatatttatgggaatgtggtcgatcagggctgtgatgtcgccaccaaaagtgcattacaaaatattcatattggtgattttaatatcagtgattttcaggccgcgaataccgtaagcactgctgctgatttgaatatcgatatcaccggttgtgccgctggtattactggcgcggacgtcctttttagcggcgaggctgacacccttgcgccgacactgctcaaactaactgacacaggcggaagcggtggtatggcaacggggattgccgtgcaaattcttgatgcgcaaagtcagcaagaaatcccgctcaatcaggtccagcctcttacgcccttaaaagccggggataacacactcaaatatcaacttcgttataagtccacaaaggcgggagcaacgggcggtaatgcgacggcggttctctattttgatctggtttaccagtgaaggagtgatgttgaaacggataatctggattctgttcttattgggattaacgtggggctgtgagctatttgcccatgatggcacggtcaacattagcggatcgtttcgccgtaatacatgcgtgctggcacaggatagcaagcaaatcaatgtgcagttaggcgatgtctcgctgacacgtttttctcatgggaattatggcccggagaaatctttcatcattaatttgcaggattgcggaacagatgtcagcacggttgacgtcaccttttcaggaacccccgacggagtgcagagcgaaatgttgtccattgaaagtggtacggatgcagccagcgggctggcaattgcgattctggatgatgcgaagatattgattccgcttaaccaggcgagtaaagactacagcctacatagcggtaaggtgccattaactttttatgcgcaattgcgacctgtcaatagcgatgtgcagtcgggtaaagtgaatgccagcgcgacatttgtacttcattatgactaatacgtggaacagattggcgctcttgattttcgccgttttatcgctgctggtggcgggtgaattgcaggcaggagtggtggtcggcggaacgcgatttatctttccggcagacagagaatcgatatctattttactgactaataccagtcaggaatcctggcttattaacagtaaaatcaaccgcccaacgcgttgggccgggggggaagcgtcgacagtgccagcaccattactggccgctccgccacttattctcctgaagcccggtacgacaggcacgttgcgcttgctgagaacggaaagcgacatcttgcctgtggatcgcgaaacgctatttgagttaagcattgccagcgtgccatccggcaaagttgaaaatcagagcgtaaaagtggcgatgcgctcggtatttaaactgttctggcgacccgaaggtttgccgggcgacccgctggaagcttatcaacaattacgctggacacggaattcgcagggtgtacaactcactaacccaacgccttattacattaacctgattcaggtgagtgtaaatggtaaagcgttaagtaatgtgggagttgtgccgcctaaaagccagcgtcagacaagctggtgtcaggcaatcgcaccgtgtcatgtcgcctggcgggcgataaatgattacggcgggttgagtgcaaagaaggagcaaaatctgccctgaaacaggttcggaaaacgtttgcgttttttttgccgcaggtcaattcccttttggtccgaactcgcacataatacgcccccggtttgcacaccgggaatccaggagagttcatgtactaccccttcgttcgtaaagcccttttccagctcgatccagagcgcgctcatgagtttacttttcagcaattacgccgtattacaggaacgccgtttgaagcactggtgcggcagaaagtgcctgcgaaacctgttaactgcatgggcctgacgtttaaaaatccgcttggtctggcagccggtcttgataaagacggggagtgcattgacgcgttaggcgcgatgggatttggatcgatcgagatcggtaccgtcacgccacgtccacagccaggtaatgacaagccgcgtctctttcgtctggtagatgccgaaggtttgatcaaccgtatgggctttaataatcttggcgttgataacctcgtagagaacgtaaaaaaggcccattatgacggcgtcctgggtattaacatcggcaaaaataaagatacgccagtggagcagggcaaagatgactatctgatttgtatggaaaaaatctatgcctatgcgggatatatcgccatcaatatttcatcgccgaataccccaggattacgcacgctgcaatatggtgaagcgctggatgatctcttaaccgcgattaaaaataagcaaaatgatttgcaagcgatgcaccataaatatgtgccgatcgcagtgaagatcgcgccggatctttctgaagaagaattgatccaggttgccgatagtttagttcgccataatattgatggcgttattgcaaccaataccacactcgatcgttctcttgttcagggaatgaaaaattgcgatcaaaccggtggcttaagtggtcgtccgcttcagttaaaaagcaccgaaattattcgccgcttgtcactggaattaaacggtcgcttaccgatcatcggtgttggcggcatcgactcggttatcgctgcgcgtgaaaagattgctgcgggtgcctcactggtgcaaatttattctggttttatttttaaaggtccgccgctgattaaagaaatcgttacccatatctaattatttcttcgaattcctctttataagataatcagggctttattttcagccctggttgttttatattcatcgctgttgcttatttagacattttgtacttttattgttgaggttattaagcgaagcgacaatggattgtgttgctgcggttttatagggtaggggagaggcagatgcgaattaaaccagacgataactggcgttggtattacgatgaagagcacgatcgaatgatgctcgatttagccaatggtatgctatttcgctcacgttttgcgcgcaagatgttgactccagatgccttttctcccgcaggcttttgcgttgacgacgccgcgctctatttctcttttgaagaaaagtgccgcgattttaatttatctaaagaacaaaaagccgaactggtgctgaatgcactggtagcaattcgctatctcaaaccgcaaatgccgaaaagctggcattttgtttcccatggtgaaatgtgggtgcccatgccgggcgatgcggcctgcgtttggttgagcgatactcacgagcaggtcaatttgctggtcgttgaatctggcgaaaatgccgcactatgcctgctggcacaaccctgcgttgttattgcgggtcgcgcgatgcagttgggcgacgccattaaaatcatgaacgacaggctgaaaccgcaggttaatgttgacagcttcagcctcgaacaggcagtctaacgcgccaacttaagtgcagtcttcggtacacagctacagcaaagaatggtgccatcatcgcccattgctgattttttcagcggcgtgacttcgccttctaaaagctgaacacggcaacttccacaaatgcccgcgcggcaagaataagggatacgaattccctgattttctaattgctccagcaacacctgttggttatttccacgaaatgcctgtccctgccagtcaatatctacatttgcgtccggttgttgcgtgatgttggcggtatcatcagcggcagctgcgccgtaaatttttgccggagccgttgccagaatttccacctcatcgccaacgcgaatcacgccgctattacgggcaattaaattctgaccaaaatcgacatcgccgttatcctgggcagtgcggaaagattgcaatgtttttaatggttcgcctgccggatgtttttgccctttttctgggctgacggtggtgaaaatacagcggctacaaggtttaaccacatcaaacaccacatcaccaatgcgaatcactttccagcgatcttcttcccaggctgacgcgccggaaaccaccagattggggcggaattgctccatttttacactggccggacaacgttgttggagatcacgtaacgaggcttcgttagcaagaaggtaaggatagccatcagcaaatgacagaggtacagtgttgtggcgtttcacgcgccgggtcatttgtggccccacccagcgtaattgcacttcgcgggagaaaaatccacttagccatttgttgatcgcgtctggcgcaattcgcgcggtaaaatgtgtgccccaaacttcggttggtgcgtcttgtgtggcgaaatcagcaaaacgaacatatgcgctactgccatctggtgcggtgagatgcaagccatcatgcacaggtgaaggagtaaaccgtaccatctggggaaactggcgagcggtaataaacgtaccgtcaggttccgtgatcataaagatgcgatcgaaggccagaccactgacatctgccagagcatgtgtaagaccaatgccgcgcatcgatttaacaggatgaataaaaagccggattaatgtcgccacggtgcggtcctcaaatgaaaataagccctcaactttatgacatgacgcgcttattagctataatgcgcaacaattttcttagcgcctgtcccattaggctattttatttgtcagtttggccctgggttatgctcgaaatcctcacgtacttgtgtacgctccggtttctccgcgctgtccatgtccagactgactgcaacaattacgcctactgcggtaggctcttagagtaaaagtgacgatatgaattctctgtttgccagtacggcccgtgggctggaagagctgttaaaaactgaactggaaaacctgggggccgttgaatgccaggtggttcagggtggggtccatttcaagggcgacacacggcttgtttaccagagcctgatgtggagccgcctggcctcgcgtattatgttgccgctgggcgagtgtaaggtttacagcgatttagacctctatctcggtgttcaggcgatcaactggacagagatgtttaatcctggcgcgaccttcgctgtccacttcagtggtttgaatgacaccatccgcaacagtcagtacggcgcgatgaaagtgaaagacgcgatcgtcgatgctttcacgcggaaaaatctgccgcgtccaaatgttgatcgcgatgcgccggatatccgcgttaacgtctggctgcataaagaaaccgccagtatcgctcttgatctgagtggtgatggtttacatctgcgtggctatcgcgatcgtgctggtattgcgccgatcaaagaaaccctggcagccgctattgtgatgcgatccggctggcagccaggaacaccgctgctcgatccgatgtgtggttccggtacgttgctgattgaagcagcgatgctggcgaccgatcgcgcaccaggcttgcaccgtgggcgttggggctttagcggctgggcgcagcatgatgaagctatctggcaggaagtgaaagcggaagcgcaaactcgcgcccgtaaaggcctggctgagtatagctctcatttttacggttcggacagcgacgcacgggtgattcaacgtgcacgcactaacgcccgtcttgcggggattggtgaactgatcacctttgaggtgaaagatgtcgcgcaactgaccaatccgctgccgaaagggccgtacggcacagtgttgagcaacccgccatacggggaacgtctggacagcgaaccggcgctgattgcgctgcatagcctgctgggtcggatcatgaaaaaccagtttggtggctggaatctctctttgtttagtgcctcgccggatctgctaagctgcttgcagctgcgtgcagacaaacagtacaaggcgaaaaacggcccgctggactgcgtacagaaaaattaccacgttgccgaaagcactccagacagcaaaccggcgatggtagcggaagactacaccaaccgcctgcgtaagaacctcaaaaaattcgagaagtgggctcgccaggaagggattgaatgttaccgcctgtatgacgccgatctgccagaatataacgttgccgttgaccgttatgccgactgggtggtggtgcaggagtatgcgccgccaaaaactattgatgctcacaaagcgcgtcagcgtctgttcgatattatcgctgcaaccatttcggtactggggattgcgccaaacaaactggtgctgaaaacccgtgaacgccagaagggcaaaaaccaataccagaaactgggcgagaagggcgagtttcttgaagttaccgaatataacgctcacttgtgggtgaacctgacggattatctcgatactggtctgttcctcgatcaccgcatcgcccgtcgtatgctcggtcagatgagcaaaggcaaagatttcctcaacctgttctcttataccggcagcgccaccgtgcatgcgggattaggcggtgcacgcagcaccaccaccgtggatatgtcgcgtacttatctggaatgggcagaacgcaacctgcgtctgaatggcctgaccgggcgtgcgcatcgcctgattcaggccgattgcctggcgtggctgcgtgaggcaaatgaacagttcgatctgatctttatcgatccgccaaccttctctaactcaaaacgaatggaagatgcgtttgatgttcagcgcgatcatctggcgctgatgaaagatttgaaacgtctgctgcgtgcaggtgggacgatcatgttctcgaacaacaaacgtggcttccgtatggatctcgacggcctggcaaaactgggactgaaagcacaagaaattacgcaaaaaacgctctcccaggatttcgcccgtaaccgccagatccacaactgctggctgattaccgcagcctgaaaggaatagtaatgtcattaatcagtatgcatggcgcatggctgtcgttcagcgacgcgccgcttctcgataacgcagaactgcatatcgaagataacgaacgtgtttgtctggtgggccgcaacggcgcaggcaaatcgacgttaatgaaaatcctcaaccgtgaacaagggctggatgacggtcgcattatttacgagcaagatttgattgtagcgcgtctgcaacaggatccgccgcgtaacgttgagggtagcgtttatgatttcgttgccgaaggcattgaagaacaagcggaatatctgaaacgctatcacgatatttcgcgcctggtgatgaacgacccgagcgagaaaaatctcaacgaactggcgaaggttcaggaacagctggatcaccacaacctgtggcagctggaaaaccgcatcaacgaagtgctggcgcaactggggttagatcctaacgttgcgctgtcgtcgctttccggcggctggttgcgtaaagcggcattaggacgcgcgctggtgagtaatccgcgcgtgctgttgcttgatgaaccgacaaaccacctggatattgaaaccatcgactggctggaagggtttttgaaaactttcaacgggacgattattttcatctcccacgaccgttcgtttatccgcaatatggcgacgcgcattgttgatctcgatcgcggcaagctggtgacctatccagggaattacgaccagtacctgctggaaaaagaagaagccctgcgcgtggaagaattacaaaatgccgagttcgatcgcaaactggcgcaggaagaggtgtggatccgccaggggatcaaagcacgccgtacccgtaatgaaggccgcgtacgcgccctgaaagcgatgcgtcgcgaacgtggtgaacgtcgcgaagtgatgggtaccgcaaagatgcaggtggaagaggccagccgctccggtaaaatcgttttcgaaatggaagacgtttgctaccaggttaacggtaagcaactggtgaaagatttttctgcccaggttctacgtggcgacaaaattgccctgattggtccgaatgggtgcggcaaaaccacgctgctaaaactgatgctcggtcagcttcaagcggacagcgggcgtattcacgttggcaccaaactggaagtggcttatttcgatcagcaccgcgcggaactggatcccgataaaacggtgatggataaccttgccgaaggtaagcaagaggtgatggttaacggcaagccacgccacgtattgggctatttgcaggactttctgttccatccgaaacgggcgatgacgccggtacgtgcgctttctggcggtgagcggaaccgcttgctgctggcgcgtttgttcctcaaaccaagcaacttattgattcttgacgaaccgaccaacgatcttgatgtcgaaacgctggaactgctggaagaactgatcgacagctatcagggcacggtattgctggttagccacgatcgtcagtttgtcgataacaccgttacagaatgttggatcttcgaaggcggcggtaaaattggtcgttatgtcggcggttatcatgatgcccgtggtcagcaagagcagtatgtggcgctcaaacagcctgcggtgaaaaaaaccgaagaagccgccgcggcaaaagcagaaactgtaaaacgcagcagtagcaaactaagctataaattgcagcgcgaactggagcagctaccgcaattgctcgaagatctggaggcgaagctggaagccctacagacgcaagtggcggatgcttccttcttcagtcagccgcatgagcagacgcaaaaagtgcttgctgatatggctgctgcagagcaggagctggagcaagcctttgaacgctgggagtatcttgaagcgttaaaaaatggtggctgatcgcaaaatagtcgatttaaacagagacagctgacaacggtaaaattgcctgatgaactgggtttatcaggcatgaaaaccaacactttgttagtcatctgtaaaatagcgcatcattaaggagtaccaatgtgcgaacatcatcatgccgcgaagcacatcctgtgctcgcagtgtgacatgctggtggcgttaccgcgccttgagcatggtcagaaagcggcatgtccccggtgtggcacaacgttaaccgtggcgtgggatgcccctcggcagcgtcccaccgcctatgcgttggctgcactgttcatgctgttgctgtccaacttgtttccttttgtgaatatgaacgttgcaggagttaccagtgaaattacattactggaaattcccggcgtgcttttttctgaggactacgccagcctcggcacctttttcctgttgtttgtgcaactggttcccgcgttttgtctgataaccattctgttactggtgaatcgcgcggaattaccggtccgtttaaaagagcaactggcacgggtgctttttcaactcaaaacctggggaatggcggagattttcctcgcgggtgtgctggtcagtttcgttaaactgatggcttacggcagcattggggtaggcagcagctttctcccctggtgtttattttgtgtcctgcaactgcgcgcttttcagtgcgttgatcgtcgctggttatgggacgacatcgccccgatgccagaactgcgccagccgctaaaaccaggcgtcacggggatacgtcaggggctgcgttcgtgctcctgttgtacggcaatccttcctgctgatgaacccgtgtgcccgcgttgtagtaccaaagggtacgttcggcgtagaaacagcctgcagtggacactcgcgctgcttgtaacgtccatcatgctgtatcttccggctaatattttgcccatcatggtgacggatttattaggctcgaagatgccgtcgacgattctcgctggggtcattctgttatggagcgaaggctcttatcccgtcgctgcggtgatctttctggccagtattatggtgccaacgttaaagatgatcgccatcgcgtggctgtgttgggatgccaaagggcatggcaagcgcgacagtgaaagaatgcatttgatttatgaagttgttgagtttgtaggccgctggtcgatgattgacgttttcgttatcgcggtgctctcggcgctggtgcgtatgggaggtttaatgagtatttatccggcaatgggtgcattaatgtttgctttagtcgtcataatgacaatgttttctgctatgacgtttgacccgcgtttgtcgtgggatcgtcaacctgaatcagagcatgaggagtcctgacagtatggaatctaataatggggaagccaaaatccagaaagtgaagaactggtctcccgtgtggatatttcctatcgtcacggcgctcattggggcctgggttcttttttatcattacagccatcagggaccggaagtgaccctgatcaccgcgaatgcggaaggaattgaaggtggcaaaaccaccattaaaagccgtagcgttgacgtcggcgtggttgaaagcgccacactggctgatgatttgacgcacgttgaaatcaaagcgcggctgaattccggtatggaaaaattgctgcataaagacaccgtcttttgggtggtgaaaccgcagattggtcgcgaagggattagcggcctgggaacgctgctgtctggagtttatatcgaactgcagccaggcgcgaaaggcagcaaaatggataaatacgatttgctggactcgccaccgttggccccgcctgatgcgaaaggtatccgtgtgattctcgatagcaaaaaagccgggcagctctcgccaggagatccggtgctgttccgtggctatcgggtaggttcggttgaaaccagcaccttcgatacacaaaaacgcaatatcagctatcaactgttcatcaatgcaccttatgaccgactggtgaccaacaatgttcgcttctggaaagatagtggcattgcggttgatctgacgtcagcagggatgcgtgtggagatgggctcattgacaacgctgctgagtggcggtgtcagctttgatgtgccggaaggtctggatttagggcagccagtggcaccgaaaacagctttcgttttgtatgatgatcagaagagcattcaggattcgttgtacaccgatcacattgattatctgatgttctttaaagattcggtacgcggtctgcaaccgggagctccggtagagttccggggtattcgcctgggtaccgtaagcaaagtgccattctttgcgccgaatatgcgtcagacatttaacgatgattaccgtattccggtactgattcgtatcgagccagagcggctgaaaatgcagcttggcgaaaatgcggatgttgttgagcaccttggcgaattgttgaaacgtggtttacgcggatcgctgaaaaccggaaacctggtcactggtgcactgtatgttgatctcgatttctatccaaatacgcctgcaataaccggtattcgtgaatttaatggttatcagattatcccgaccgttagcggcggcctggcgcaaatccagcaacgactgatggaagcgttggataagatcaacaaactgccattgaatccgatgattgaacaggcaaccagtacgctttctgaaagtcagcgcacaatgaaaaacctgcaaacgacgctggatagcatgaacaagatcctcgctagccagtcgatgcagcagttgccgacggatatgcagtcaacgttgcgtgaattgaatcgcagcatgcagggcttccagcctggctccgcagcctacaacaagatggtggcggatatgcagcgccttgatcaggtgttgcgagaactgcaaccggtgctgaaaacgctcaatgagaagagtaacgcgctggtatttgaagcgaaggacaaaaaagatccagagccgaagagggcgaaacaatgaaaaagtggctagtgacgattgcagcactgtggctggccggatgcagctccggcgaaattaataaaaactattaccagttacctgtggtgcagagcggtacacaaagtaccgccagccagggcaatcgtctgttatgggtagagcaggtcactgttcctgactatctggcggggaatggtgtggtttatcaaaccagtgatgtgaagtatgtgattgccaacaacaacttgtgggccagcccgttggatcaacagttgcgcaacaccctggttgccaacctgagtacgcaactgcccggctgggtggttgcctcccagcctctgggaagcgcccaggacacgctcaatgttaccgtaacggagtttaacggtcgctatgatggcaaggtcattgtcagtggtgagtggctgttgaaccaccagggacaactgatcaaacgtccgttccgtctggaaggagtgcaaactcaggatggttacgatgagatggttaaagtgctggccggtgtctggagtcaggaagccgcttctattgcacaagagataaagcgtctaccttaattataaagatttgtaaatataaccgtctccggtatgttgcctgaggcggtttttttgtctctaacgtgcggaaaaatttgttcctcttcacattttttgtacaaccgacatgcccgtgtagctcacaaatatgacagtggcgtgaattttgcgcattgacggcagttatgattcgcggtattgcttaactgtgattgcacatttagtaatcactgttttcttttccaccagaaaccagtatgagggaaacgaggcatgaagagacaaaaacgagatcgcctggaacgggcacatcaacgtggttatcaggccggcatcgccggacgctcaaaagaaatgtgtccctatcagacgctgaatcaaaggtcacaatggctgggaggctggcgagaagccatggcggacagggtagtaatggcctgattctgtctctttaaaaagaaacctccgcattgcggaggtttcgccttttgatactctgtctgattataatcagaaggcagacgtatcctggaacagaccgactttcaggtcgctggcggtatagatcagacgaccatcaaccagcacttcgccatccgccaggcccataatcagacgacggttaacaatgcgtttaaagtgaatacggtaggtcacttttttcgctgtcggcagtacctgaccagtgaatttcacttcgccaacgcccagcgcgcggcctttaccttcgccgcccagccagccgaggtagaaccctaccagctgccacattgcgtccaggcccaggcatcccggcataaccggatcgccaataaagtggcatccgaagaaccacagatccggattgatatccagttctgcttcaacataccctttgtcgaagttaccacccgtttcggtcattttgaccacacggtccatcatcagcatgttcggtgctggcaattgcgggcctttagcgccaaacagttcaccgcgaccagaggcaagaaggtcttcttttgtataggattcgcgtttatctaccatgttctctgtaagccttattttattgaagcacgcaggatagctaacacgtgtacgctgaacaagtccgatcagttcggaataaaccagttcagccaacgtaatggccatggaaaacggtgacgtccttcctgttgcgatgcttgcgcgatacgttcctggatggtttgcatcagcgtcgtttggccttcgccatcccacaccagatttaataataacggcagtgcgtcagtcacatcgtctactgcccagatggtgaatttgccttcttctaccgctttcaccagttcactgtgaagacttaaatggcgaacgttagctgtggggataatgacaccttgtttcccggttaactcacgttgctggcaaatagcaaagaagccttcgattttctcatttaaaccaccgaccggctgggcgcgaccgaactgatcgactgaacctgtgatagcgatactctgattcaccggcacatcggcgagggcgcttatcagggcgcagagttcagccatcgaggcactatctccatcaacttcactgtatgactgctcaaatgtcagcgatgctgagaaggggatctgttgctcaagctgtagttccgacatcaggaacgcttgcatgatcatcatccctttcgcatggatattgccgccaagctccgctttgcgttcgatgtcggtgaattcaccatcgccaatatgcacaacgcagctaatgcgagaaggttcgccaaaagcgcgtggatgacccggaaattcaatgaccgaaagggcgttaatttgcccgatgcgttcgccttcggtttcaatcaggatttgctcctgaaggatctcatcctgcatacgttcagcgaggaaaccttcgcgccattcacgctgctgcagcattaagtttagctgctcgccggagaaggtgtcgccatcacacagggaggcgacctctttacactggcggaggatccactgcgggctaagcggaagtgtttcttgttcaccggtgtagcgtgctgcttcgcggataagtatcggccaggcatccgctcccggtgcaggtaagtgattatgtctggcggtaaatgtcacccagcgacaccactgggttactgactccgcatcgacaatctgcagagtatcttcaaattcgctataaatagcctgctctgaaagctctggctccatctcctggaaatcagccaatgattcgcgttcgcctaccagaatgactttcagcttcaatggcatcgaaggcacagagacggggagagggcgcgactcatcaaacgcaacccagtcaaaacgctcgcggttaacgatatttttcagccgcatccacagcagaggttgcgccagcagtgtacgcaaagagataatgagaataccgccatttgcctgatgcaccagaccaggctgcagggtaatgtcgccattaaactggcgcaggcagccaaagagttgctccgcttctacccagtcggcagcgacaacttgcgttaaagtcgcaaaattatcatctgcactcactgcgtgacgtaagcggatggagtggccggaaacctcatagtgaccgcccaccagttggcctgcatcgctttgtagcgtacgcgcggcattggcaataagattcagatactcagactcttccggggccttcgccagcataaaagaggaggatgctcgcgtatgcagcaactgctccagcgcaaattgcagccgcggttgagtatcactgaataaaggatcgttttcgtcaatcaaatgtggctgagcaaatatttcctgatagctatcggtatcaggaaccaggtcacgccatgcaagtttcgtaatggtcaaagttgatgttttttagtctgttgtcaaagccgcgattataccgtaaccggcactacagcacacgtagaaagcaccgacaatactcctggcatgggcgttaaagctcacaggatggagattcttttcttcactggcctaaaaagctgatattctgtaaagagttacacggtaacattgagatcgctatgaaatatcaacaacttgaaaatcttgaaagcggttggaaatggaagtatctggttaagaagcatcgcgaaggggagttaatcacccgttacatagaagccagtgccgcccaggaagccgtcgatgtgttgctctcgctggaaaatgaacccgtgctggtaaatggctggattgacaagcatatgaatccggaactggtcaatcgcatgaagcaaaccattcgggcaagacgaaagcgccattttaatgcggaacaccagcatacgcgcaaaaaatcgatcgatctggaatttattgtctggcaacgtctggctggtcttgcgcagcgtcgcggtaaaacgctttctgaaacgattgttcagctgattgaagatgcggaaaacaaagagaaatacgcgaataaaatgtcttctctgaagcaggatctgcaggcattgctgggtaaggaataactgacgaaagtcagttcaatttactaaaggcaaaaaaaaccccgcagcagcggggtttttctaccagacgagaacttaagcctgcggctgagttacaacgtctttgatacctttaacttcgatctctacgcgacgatccggagccaggcagtcgatcagtgcagcacgctgtttcacgttgtcacaggtgttgccagtaaccgggttggattcgcccataccacgtgcggagatcttgtctgccgggatacctttggagatcaggtaatcaacaacagactgagcacggcgctcggacagaccctggttgtaagcgtcagaaccgatgcggtcggtgtaacccagaacaactacggaaccgtctttcggatccaggttgctcagctggctgtacagctgatccagagcagcctgaccttccggtttcagggttgctttgttgaagttgaacagaacgtcagacttcagagtgaagtgcttggtctgtacttccggtgccggagctggagccggagcaactactggagctgcttcgccctgaccgaaacggtaggaaacacccaggctcagcatgccgttgtccggacgagtgccgatggtgtgtgcgtcaccgatgttgttggtccactggtattccagacgggtagcgatttcaggagtgatcgcgtactcaacaccgccagcgaagaccggagaaacgccggtgtcgtggtttttaccataaacgttggatttagtgtctgcacgccataccatgccacccagacgagtgtagatgtccaggtcgtcagtgattgggtaacccagtttagcggtcagttgaacgccctgagctttgtatgcaccgttttcaacgctgcctttgtacggcatacgacctaaccagtcgtaacccatttcaaagccaacatacgggttaacctggtaaccaccaaaagcaccagcgcccagttggttttcatgggtcgggccattgttgttgatgaaaccagtgtcatggtactgggaccagcccagtttagcaccagtgtaccaggtgttatctttcggagcggcctgcgctacggtagcgaaaccagccagtgccactgcaatcgcgatagctgtctttttcattttttgcgcctcgttatcatccaaaatacgccatgaatatctccaacgagataacacggttaaatccttcaccgggggatctgctcaatattaactctaccgatatcttcggcttatgccgagcacccctggcgatgtaaagtctacaacgtagttgaaaacttacaagtgtgaactccgtcaggcatatgaaaaaaaagtcttgtataaggtatgtttaatcttttttgtcagcgacaatttacagaagagaatcgcggaaaccgcttcagacaagcctccgcaaggaaaattagtcacgactgaaagcattggctgggcgacaaaaaaagttccaggattaatcctaaatttacttaatgatacaaattagagtgaatttttagcccggaaagttgtctcgtggcgtgagaggatgcgcttaccggacgcataataaaccccatagcgttaccttcatttgccgcatcaacaagttcagcatgctcttcttcagtcaaatcatctgccaaccaaccgatcaccacactgtaattgcccgtgcgtaaagcgcgaaccattgactccacagtgtggcaaggggagagctggctaatctgcattactttcgttaagggtagcccagatgcctgaacccattcccgactcagtttttgttgcggtgttaaccagagttgccagcgcgattgctgaccgagttgctgtaacaatggcaacagtagaagttgcgtcatcatgggctgatcttcgcgatagacaacttcactgataagcccggctgtagtgttttccgtagagacacgcgcaattttacttgctgcggatgagaacgacgaagaacgatgtgcatagcctgaagtgtacataatcaatccagcccctgtgagttactgtatggatgtacagtacatccagtgacaacaaagatcaaccctattttcggaaagagcctcgcaaattttgtcgttggtgacgggaaaacataaattaatcttgccccttaagaataagttgcctattttcgtagttaacggatccgttaatgtgaatcattcttttatgttatgattttaaaaggaattttatgaaaagcctctcctataagcggatctataaatcacaagaatacctggcaacgttgggcacaattgaataccgatcattgtttggcagttacagcctgaccgttgacgacacggtgtttgcgatggtttctgatggtgagttgtatcttcgggcttgtgagcaaagtgcacagtactgtgtaaaacatccgcctgtctggctgacatataaaaagtgtggccgatccgttaccctcaattactatcgggttgatgaaagtctatggcgaaatcaactgaagctggtgcgtctgtcgaaatattctctcgatgcagcgctgaaagagaaaagcacgcgcaatacccgggaaagactgaaagatttgcccaatatgtcttttcatctggaagcgattctcggggaggtggggattaaggatgtacgggcgttacgtatacttggggcaaaaatgtgttggttgcgactgcggcagcaaaacagtctggtgacagaaaagattctgtttatgcttgaaggtgccattatcggcattcatgaagctgcgctcccggtggcacgccgccaggagcttgcagaatgggctgactctcttacgccgaaacaggagtttcctgcggaacttgagtaatctggcgttgcagacgaccaatctcaggcagtaatgcaatcaataatccaacttgttgtacgaccagaggttctttgctgtctgcccgtggttcaagttgctgcatccgctgtttcaggctagctaatgcctcattgacgcgttcttcatcagcaggttgatgatgtaacgcgtcatcaacatagcaaactgcgtcatcaagaaacgccagaatttcaggattagttaactgctcccggtgagcaccgagggctgagatatagctggtaaacgtatggttaaggcacagcaaccgaaacgcggcttcgcgaatttgcggggtaacgttcggctcgctggacatatttgataccaccgacgccagctcagcatcacggttgtgtgcatcgcggcgggcaatacgatacgccagacggttatcacgcccctgatggtattgctccagtatggcatcgagataccgacagttggcctctgtggcgcgttcgagcatgcgcggcagattgcgaaactgccagtcaggccagatgtagctcactgccgcccacgcaatggcacaaccaatcagcgtatcgattacgcgaggtaacgctacttcaaaaccttcacccagtaagttaaaacacagtagcaccaaaagtgtgatgaacatcgttgcatgagcgtattgcacgttacggaaggcaaaaaagagcacgccggtaataaccagcagcaccagctgcccttccagtgatggcacaaaccacagcacaggaatgccaatggcgatacctaccagcgtaccaataatccttaacttcaggcggtggcgcgtggcgttatagtttggctggcagacaaacaaacttgtcagcaagatccaatacccgtgatgcattccggttatctgaatgatggcgtagccgaagcacaacaccagcgacattcttaccgcatgacggaagagggcggattccggcgtgaagtgacggctaagacgcagccagatatcactcaacccgtgcgggctgtcatcagcgagctcattttcgtcattattatggggtagtgcctgggcctgttctgattcaattgttgccagttgggcatcaatggcgcgtaaattgttcagcaaaaatcccagtgttttgagtaaatcggcgggtgcgccgttatcgcgcatccgctccagcgcagcatcaatatgcgtaaaagcgcgctcaaaatgcggatcatgttgataaggctgacgcaacaaaatacagcgtgacagttgctggcacgcctggccctgcatcgacatcagccgctgaaaacggaacagcacgtcgctgtggcgaaaatgttcacgcaatgtttgatactgaatatgagaagagctggcacgctcgtgaatatcctgtgcgacaaagtaataatgcagcgtgcgacgcgttccccgttgaccacgatcgccacgtaagcgggtcagcagcgagagtttcgtctgattcaatgtcgccatcagcagaccgttggcgagagccaaatcgtacagcggtgcctggctttgatcttcaatatcaggatcaaacatgcgcgacttgagctcaagataacgcgccagttgttcatagcaacgcgccaggttgtcctgcagcgggcggaccgggaacagcagatgaccaataagtgtcaggacgttgtaccagacggcaccggccagcagatacatcggctgctgataccagtgctcatacagtgatgttcccaacatagtgtaaatggcgatcagcaatgcaccgaaggcaattgttgcatagcgttgacccagaccgccgagcaaaatgaagccgctggtagagagcgttaagccaatcgcaaatagccagggccagggaaacagcaattctactgaggccgaggcgataaaaaagcagaacagcgtaatgatgaggttacgcaaacgtcccgccagtcggtcatcgagatcggtcagcgccgctgccaccatccccagcgttagcggaatcgtcagttttacatcacccagccaccacggaaacgctgtggttccacaaagcgcaataaaaatacgcgcgtaatacagccaggcgctgttccaggtatagcgtttgagcaaaggacttagcataaaggccatattagtggattattcaaaacgacgacgtgcattggcttcacgcgcagcttgcgctgtttctaccgataccacgcgacgaccaaccggccatagtgcaatagcggcaattttaaagttcgcaatgccgacaggaatgccaatgattgaaatacattgtgcgatgcccgttgcaatgtgcatcaggcataaccaccagccaaagaaaatcagccagaaaatattcaataccgtaccgccagtattcagcagcacatttttgccagccgggttcagttcatcgacatgaatagcttcattgccataaggcaccagagacagtttagtgatctcccagcaggatcgtgtcagcggtaaggtaaaaatcagcacaatactgaccagagtcgccaacagccagcccagagtggtggcaaatccgccaagcacaaagttcagaatgttcaaaacggtacgcataaaacctcgctttactgtggttttcagtaatgggcggcaattgtaacgtttttttgggctggagcacgttttctctgacggttacactgataagaaataatttcgtgtggatctacagagtcatggaactgaaagcgacaacgcttggaaaacgtctggcacagcacccttacgatcgggcggtgatcctcaatgccgggattaaagtctccggcgatcgccacgaataccttattcctttcaatcaattactggcgattcactgtaagcgcggtctggtatggggcgagctggaatttgtactgccggacgaaaaagtggtgcgtctgcacggcaccgaatggggcgagacgcagcgtttttaccatcatcttgatgctcactggcggcggtggagtggcgagatgagcgaaattgcgtctggtgttttacgccagcaactggatttgattgccacgcgcactggggaaaataaatggctgacgcgtgagcaaacctctggcgtgcagcaacaaatccgccaggctttgtcggcgttgccgttgccggttaaccgactggaagaattcgataactgccgtgaggcgtggcgtaaatgtcaggcctggttgaaagatattgaaagcgctcggttgcagcataaccaggcgtataccgaagccatgcttaccgagtatgcggattttttccgccaggtcgagtcttcaccgctgaatccggcgcaggcccgggcagtcgttaatggcgagcattctctgttagtgctggcaggtgcaggaagcggaaaaacgtcggtgctggtggcccgtgcaggctggttgctggcgcgtggtgaagcgtcccctgagcaaattttattgctggcgtttggtcgcaaagccgctgaagagatggacgagcggattcgcgaacggctacataccgaagacattaccgcacgcacgtttcatgcgctggcgctgcatattattcagcagggcagcaaaaaagttccgatagtcagcaaactggaaaatgataccgctgcccgtcatgaactctttattgctgagtggcgcaagcaatgcagcgaaaagaaagcgcaggcgaagggctggcggcaatggctgacggaagaaatgcagtggtcagtgccagaaggtaacttctgggatgatgaaaaattacagcgtcgccttgcctctcgcctcgatcgctgggtaagtctgatgcggatgcacggtggtgcacaggcagaaatgattgccagtgcacccgaagagattcgcgatctgttcagtaaacgtatcaagttgatggccccgttattaaaagcctggaaaggtgcgctgaaggcagaaaacgctgtcgatttttcgggccttattcatcaggcgattgtgattctggagaaaggtcgctttatcagcccgtggaagcatattctggttgatgaatttcaggatatctcgccgcagcgggcagcgttgttagcggcattacgcaagcaaaacagtcagacgacgttgttcgctgttggtgatgactggcaggcgatttaccgattcagcggtgcgcaaatgtcgctcaccaccgctttccatgaaaactttggtgaaggcgaacgctgtgatttagacacgacttaccgttttaacagtcgtatcggtgaggtggcaaaccggtttattcagcagaacccaggccagctgaaaaagccgctaaacagcttaaccaatggagacaaaaaagccgtcacgttattggatgagagtcaacttgacgctttgctggataagctctctggttatgccaaaccggaagagcgcattctgatcctggcgcgttaccatcacatgaggcctgccagcctggaaaaagcggcaacacgctggccgaagttgcaaatcgactttatgaccattcatgccagcaaagggcaacaggcggattacgtcatcatcgttggcttgcaggagggaagtgatggttttccggctgcggcgcgggagtcgattatggaagaggcgctactgccaccggttgaggatttcccggacgctgaagaacggcggttaatgtacgtggcgctgacccgggcacgccatcgggtatgggcactgtttaacaaagagaatccctctccctttgtggaaatactgaaaaatctggatgtgccggtggcgagaaaaccgtaagaaacaggtggcgtttgccacctgtgcaatattacttcagacggtccgcgagataacgctgataatcggggatcagaatatcgaccgcgtcgttgaaatgcggcgactggattatgaagtctgccgttgccacgttggtggcgaccggaatgttccataccgtcgccagacgcagcaaggctttcacgtcaggatcgtgcggcacggcatttagtggatcccagaagaaaatcaatacatcaattttcccttctgagatcaatgcgccaacctgctggtcaccccccattgggccactcaacatcgcgttgacgttcatgccggtcgcgcgggaaattaagttaccggtagtgcctgttgcatacagtacgtgttgttccagtaacggttgatgccgttccacccagctcatcagcatttgtttgcagtgatcgtgtgccaccagcgcaatatgtttccgcgcaggtaaagtgcgagtcgtcagttccataatgtacatccgtagttaactttcctacagattactgtaagcacttatcgctgcaagataaagaccgaaaaagcctgcgcacaggcacaaaaatctcaggaagatggttgtttttccgcccactgcaggaaagtatttcgcgtttgtgggtcagccagtttaaaccaatacttcagccgttgttctgtgagcacctgagactgcggtggaatagcatccagctcggaaacacccgaaagcagcgtactgtcatctgccatcatcgtggcaaattgcggtagtgaagcgcgtttcgcggatttgttatagcgttcaacctcgacctcataatcaatcgtttttgccgttgaggtaatggcgagaatatccagctttaccggaatcggcgtcgcatcgccatccaacaattcaaggcgcggcgcggcatcaaaatggttagcttcccgctcattctccaggcgaggcaggcgaaaattgacctggttgatgagctgggtattaaaactgaccaccagcggtggggagatatacagccgttcttcactattggaaagatgaatcgtcttctcaacgcgaaacactaactgatgcggtccattatccagttcaatgctgtccgcaccgcgcagcagagagctggaaaccttcttgccgtcgagtaccagaagatcgacatcggttgaaagccgcagcgtggtggcaaaaacggataccggcaaacataatgcaatcaaggtggtcacgatgccggttttcataggtagctcctgtcaaaagaccgcccgaataataatgtgtcaaaatttttctttaatcatacttactaacatatagacatatttcccgcttttgctctcattcattcgtattagctgcatggttggcatgtcggctttgtcgtacactttgttaaacagtctggaggaaataatgaaagaaaccgatattgcaggcattttaacgtccactcacaccattgcgctggtgggggcaagcgacaaacccgatcgtcccagctatcgcgtgatgaaatatctactcgaccaggggtatcacgtcattccggtttcgccaaaagttgccggcaaaacgctgctgggccagaaggggtatggcacgctggcagacgttccggaaaaagtcgatatggtcgatgttttccgtaattcagaagcggcgtggggcgtggcacaggaagctattgccattggcgcgaaaactctctggatgcaactgggggtgattaatgagcaagcggcagtactggcacgggatgccgggttaaatgtggtgatggatcgctgcccggctattgagatccctcgcctgggcctggccaaataaaaaatccccggaaggcaaaaaccttccggggatttgttcagggattagttacgcagacgcggggcctggagttgtttgcggatggtctgcgccagctcatccatggatggctgttcaggatgttcatcctgcaattcgctacttagctgggcttcagccaggtaggtatgaaccggtaggccgttatcgtcctccatcactacgtgataccacggagcggcgcgaagctcgtcattcaccgccagctcatcaggcgacggttcagagagcgaataaaccgggtcgatatccacgaccactccgagataacctaacagggaatggcggacctgctggccgataccgaatttgctggcaatcatagtcacctcccgggaaatctttacctttgatataagggtaaaattccacatttcaagttacatgacgcgacaggcaaaccctttcagatatagcccttccggataggtagcgatcaccggatgatcggctgcctgacggaactgctctataaattgtacatcacgaccggcatcaattgcggcatccgcgatgattttctgaaataaatcgctggtcatcagaccggaacaggagaaagtcaggagaataccgccttcattcagcagctgaatcgccagcatgttgatgtctttataaccacgacacgcgcccatcaactggcttttattctcaacaaacttcggcgggtccatcacgataacgtcaaatttttcaccgcgatcgcgataagtacgcagcaatttaaagacatcatcacggacaaactcagccttgctcagatccagtttgttcagctcaacgttctgccgtgcaatatccagcgcttcctgggaggtatcaacgctgacaacctggctgcaaccgcccatcagtgccgatacggcgaaaccaccggtataggagaaacagttcagcacacgtttattttcaacgtagcggcgggtagccaggcggctatcacgctggtccaggtagtagcccgttttgtgtccgtgctgaatatccaccagcagtttcattccgtgttcttcaatcggcagcagggcaggtggcaactcgccggtgacggggccctgggtcagctccattccttcttttttacgtaccgcgacgtcgctgcgatcgtaaatcgaacattccgggtacagcgtttgcagggcactaattaatgccgcgcgctgatattctgccccagcactcagcagttgcagcaccagaaaattaccgaaacgatcgatagtaatacccggcaggccatcagattctccggcgattaaacgatagctgtcgaggccatctttttgcgccagccagtcacgccatttttgtgcttgttgcaaacggcgggaaaaaaaagcaatgtcgatagactcagacgggtcaaacgtccagacgcgcgcccggatttgcgaagctggcgaataagcgccgcgtgctaaccattttccctgatgatcaacaatatcgatggtttcaccgaggctggctttaccttccatgcgggcaacggccccggaaaagacccacggatggcgacgaagtaatgatttttcgcgccctttggctaacactaaacgtacactcataatttacttttctgtcgatgcaaagaaatgggcgtcattgtccggagttttccatggatttgcaacgcgtccattaaggataaggagagcagcaatgtcgaaagtctgcataattgcctgggtttacgggcgagttcagggcgtaggatttcgctacaccacacagtacgaagcgaaaagactgggtttaaccgggtacgccaaaaatcttgacgatggcagcgtggaagtggttgcttgcggtgaagaagggcaggtggaaaaattaatgcagtggttaaagagtggcggcccgcgttctgcgcgtgtagaacgggtgctcagcgagccgcatcatccctcgggggaattaaccgattttcgtatccgttaaatacattttaccggttttggcaggccagcaattttggtggcttgcttagccggacctttcggaaacagtcggtataaatagcggctgttacctttttcttcgccaaatttattcgccatcgcttttaccagcatacgaatcgccggagaagtattgaattccagatagaaatcacgcacaaaacgcaccacttcccagtgttccggtgacagcgaaatcccttcgttctctgcaatcaccacagccagcggctcactccactggctgctttctttgagatagccttcggtatccgtttctatctctttaccttcgaagatcagcataattattactaccttaatcagactggcggcagtgtaacaaaaaacaaagccccgcataaagcgaggctatgaaagtgttagcgggtgagattaatcgcggctagcgaagcccagaatgctcagcaggctgacgaagatgttgtacagcgaaacatacaggctaaccgtggcacgaatatagttcgtctcaccgccatgaatgatgttgctggtttcaaacaagatagcgccagaggagatcagaatgaagaccgcgctgatcgccagatgcagagcaggcagctgcaggaagatattcgcaaccataccaatcagcaccaccacaatacccgccatcagcataccgccgaggaacgacatatctttgcgggtggtcagcacatatgcagagcagcagaagaacactaacgccgttccgcccagtgccatagcgattacgtcacccattccggcagacagataggtgttcagaataggtccgaggatataacccagaaaaccggtaaaggcgaatgcggagataatcccggtcggcttattcgccgttttataggtcaggaacatcaaaccatacatacccaccagcgtcagaatcagacccggagatggcagcatcagcaccgtactggcagttgcggtaatcgccgaaaaggccagcgtcaggctcagcagaaaataggtattacgcagcaccttatgggtgctaagcagtgatgtacggtcatgtgaagaactaacaatacgatccattgagtcactctctatgacagatgtaattaattaagcagcataatgataatgcgtaagggcacccagaagttttacccatctttacgcatttgatctggaacaggtttaacagcggattatcaggtcattaagcaaatataacgccctgagaatttcgacaggcaaaagaaaaaggggttagcatttagctaaccccttatcttatttggcggaagcgcagagattcgaactctggaaccctttcgggtcgccggttttcaagaccggtgccttcaaccgctcggccacacttccggaatgacgcgcactataaacatcccgatgcggcgtgtaaacccctaatttgtttgtttgcctgaaaaacagccaaaagtgcattgatagcgtgaaataacagcagattgatcatttcatcaccatgaattccttctcttttactcgtttagcaaccggctaaacatccccaccgcccggccaaaagaaaaataggtccatttttatcgctaaaagataaatccacacagtttgtattgttttgtgcaaaagtttcactacgctttattaacaatactttctggcgacgtgcgccagtgcagaaggatgagctttcgttttcagcatctcacgtgaagcgatggtttgccttgctacagggacgtcgcttgccgaccataagcgcccggtgtcctgccggtgtcgcaaggaggagagacgtgcgatatgaataacgaggaaacattttaccaggccatgcggcgtcagggcgttacccggcgcagctttctcaaatattgtagtctggctgccacgtcgctgggattaggcgcgggaatggcaccaaagattgcctgggcgctggagaacaaaccgcgcattccggtggtatggatccacggtctggaatgcacctgctgtaccgaatcttttatccgctccgctcacccactggcgaaggacgtcatcctttccctgatttccctcgattacgacgatactttgatggctgccgccggaacccaggcggaagaagtctttgaagacatcatcacgcaatacaatggcaaatatatcctcgcagtagaaggtaatccgccgctgggcgagcaggggatgttctgtatcagcagcggtcgaccgtttattgagaaactcaaacgtgccgctgccggagccagcgcgattatcgcctggggaacctgcgcgtcctggggctgcgtgcaggccgcgcgacccaatccgacgcaggcaacgcctatcgacaaagtcatcaccgacaaacccattatcaaagtacctggctgcccgccgatcccggatgtgatgagcgccatcattacttacatggtgacctttgatcgcttgccagatgtcgacagaatgggccgtccgctgatgttctatggtcagcgaatccacgataaatgctatcgccgcgcccacttcgacgccggagagttcgtccagagttgggatgatgacgctgcccgcaaaggttactgcctgtacaaaatgggctgcaaagggcctaccacctataacgcctgttcctccacacgctggaatgatggcgtttctttcccaatccagtctggtcacggctgcctgggctgtgcggaaaatggtttctgggatcgcggttcgttctacagccgcgtggtcgatattccgcaaatgggtactcattccaccgccgataccgtcggtttaaccgcgcttggcgtggtggcagcggctgttggtgtgcacgcagtcgccagcgccgttgaccagcgcagacgtcataaccagcaacctacagaaaccgaacatcagccaggcaatgaggataaacaggcatgagcactcagtacgaaactcagggatacaccatcaataatgccggacgccgcctggtggtcgacccgattacgcgcatcgaaggccacatgcgctgcgaagtgaatattaacgatcagaatgtgatcaccaatgccgtctcctgcggcaccatgtttcgcgggctggagatcatcctacaagggcgcgacccgcgcgatgcgtgggcgttcgttgaacgtatctgcggcgtctgtactggcgtacacgccctggcttcggtttacgccatcgaagatgctatcggtattaaagtgccggacaacgccaatatcatccgcaacattatgctggcaacgctctggtgccacgatcatctggtgcacttctatcagcttgccgggatggactggatcgatgtgttagatgcgctgaaagccgacccgcggaaaacctccgaactggcgcaaagtctctcctcttggccgaaatcatcccctggctatttcttcgacgtacaaaaccgcctgaaaaaatttgttgaaggcgggcagttggggatcttccgcaatggctactgggggcacccgcagtacaaactgccgccagaagctaacctgatgggctttgcccactatctcgaagctctcgatttccagcgtgaaattgtcaaaatccacgcggtctttggcggtaaaaacccgcatccaaactggattgtcggcgggatgccttgcgccatcaacattgacgaaagcggcgcggtcggggcagtcaatatggaacgcctgaacctggtgcagtcaattatcacccgcacggcggacttcattaacaacgtgatgatccccgacgccttagccatcggtcagttcaacaaaccgtggagcgaaatcggcactggtctttctgataaatgcgttctcagctacggcgcattcccggatattgccaacgactttggcgagaaaagtctgctgatgcctggcggcgcggtgattaacggcgacttcaacaatgtgctgccagtggatttggttgatccgcagcaggtgcaggagtttgtcgaccacgcctggtatcgatatcccaacgatcaggtcgggcgtcatccgttcgatggcatcaccgacccgtggtacaaccccggcgatgtcaaaggcagcgataccaacattcagcagctgaatgaacaggaacgctactcgtggatcaaagcgccacgctggcgcggtaacgcgatggaagtggggccgctggcgcgcacgttaatcgcttatcacaaaggcgatgctgcgaccgttgagtcggtcgatcgcatgatgtcggcgttgaacctgccgctttccggtatccagtcaacgttaggccgcattttgtgccgcgcgcacgaagcgcagtgggccgcaggtaagttgcagtatttcttcgacaagctgatgaccaacctgaaaaacggcaatctcgccactgcttccacggaaaaatgggaacctgcaacctggccgacagagtgccgtggtgtcggttttaccgaagcgccgcgcggggcgttaggccactgggccgccattcgcgatggcaagattgatctctaccagtgcgtggtgccgaccacctggaacgccagcccgcgcgatcccaaagggcagattggcgcttatgaagcggcgctgatgaacaccaaaatggcgatccccgagcaaccgctggagatcctgcgtactctgcacagctttgacccgtgcctcgcctgttcaacacacgtgctgggcgacgacggtagcgagctgatctccgtgcaggtgcgttaacagcgaaggagaatcatcatgcaacagaaaagcgacaacgttgtcagccactatgtctttgaagcgccagtgcgcatctggcactggttgacggtgttatgcatggcggtgttgatggtcaccggatactttatcggcaagccgctaccttccgtcagcggcgaggcgacgtatctgttctatatgggctacatcaggttaattcacttcagcgccgggatggtttttaccgtggttttgctgatgcggatctactgggcttttgttggcaatcgatactcccgcgagctgtttatcgtgccggtatggcgtaaaagctggtggcagggcgtgtggtatgaaatccgctggtatctgtttctggcaaaacgtccgagtgccgatataggccataatcccatcgcccaggcggcgatgttcggctatttcctgatgtcggtctttatgatcatcactggttttgcgctgtacagcgaacacagccagtacgctatttttgcgccgttccgttatgtggtggaatttttctactggacgggtggcaactcaatggacattcacagctggcatcggctggggatgtggctgattggcgcgtttgtgatcggtcatgtctacatggcgctgcgtgaagacatcatgtccgacgacacggtgatctccaccatggtcaacggctaccgtagccacaaatttggcaaaataagtaacaaggagcgttcatgagcgagcaacgcgtggtggtcatggggctgggcaacctgctgtgggccgatgaaggcttcggcgtgcgggtggcggaacggctgtatgcccattaccactggcccgagtatgtggagattgtcgatggcggtactcagggactgaacttgctggggtatgtcgaaagcgccagccatctgttgattctcgatgccattgactacgggctggaacctggaacgctgcgaacctatgccggagaacgcattccggcttatctcagcgcgaagaaaatgagcctgcatcagaacagtttctccgaagtgttggcgctggcggatatccgcggacatctgccagcacatattgccctcgtcggtctgcaacccgcaatgctcgacgactacggcggtagcctgagcgaactggcacgggagcaactgcccgctgcggaacaggcggcgctggcgcagcttgctgcgtggggaattgtgccgcaaccggctaatgaatcgcgctgtctcaattatgactgtctgtcgatggaaaattacgaaggcgttcgcttgcgccagtaccggatgacacaggaggagcagggatgagcaacgacacgccatttgatgcgttgtggcaacgaatgctggcgcgcggctggacgccagtcagtgaatcccgtcttgacgactggcttacgcaagcgccagacggcgtggtgttattaagcagtgacccgaaacgcacgccagaggtcagcgataatccggtaatgattggcgaattactgcgcgagtttcccgactatacatggcaggtggcgattgctgaccttgagcagagcgaagccatcggcgatcgctttggcgtctttcgctttcctgccactttagtgtttaccggcggaaactatcgcggcgtgctgaatggtattcacccgtgggcggaactgataaacctgatgcgcgggcttgtcgaaccgcagcaggagcgtgcctcatgagcgaaacttttttccatctgctggggccaggaacgcaaccgaacgatgacagtttcagcatgaatccactgccgatcacctgtcaggtgaatgatgaaccgagtatggcggccctggagcaatgtgctcacagcccgcaggtgattgcgctgttaaacgagttacaacatcaactaagcgaacgccaaccgccgttgggcgaggtgctggcagtcgatctgttaaatctcaacgccgacgatcgtcactttatcaatacgcttctcggggaaggggaagtgtcagtgcgcattcagcaggctgacgacagtgaaagtgaaatacaggaggcgatcttctgcggattatggcgggtgcgcagacgtcgcggcgaaaagttgctggaggacaaactggaggctggctgcgcgccgctggcgttgtggcaggcggcaacgcaaaatctcttgccgacagattcgctgttaccgccgcccattgatggcctgatgaatggcctaccgttggcgcatgagttactggcacatgtacgtaaccccgacgcgcagccgcacagcattaatctgacgcaattacccatcagcgaggctgatcggctttttctctcacgtctctgtgggccgggaaatattcagattcgtaccattggctatggcgagagctatatcaacgccacggggttacgccatgtctggcatttacgctgtacggacaccttaaaaggcccgttactggaaagttatgaaatctgcccaataccggaagtggtgctggcagcgccagaagatttggtcgactctgcgcagcggcttagcgaggtatgtcagtggctggcggaagctgcaccgacgtaaaaagacggtaagtatcgctttcagtcttatgaatatcgcaatcggcgaatacctctggtcgtagagtttcaggataaagagggagatctaccattatcgggttatttttctctcttcgcctacaggagtgcgcatgtgggatgtcattgatttatcgcgctggcagtttgctctgaccgcgctgtatcactttttatttgtaccccttaccctggggctgatttttttgctggctattatggaaaccatttacgtggtcaccggcaaaacaatctaccgcgatatgacgcgcttctggggtaagctcttcggtatcaattttgctcttggcgtggctaccggcctgaccatggagtttcagtttggtactaactggtcattctattccaactatgtgggcgatatttttggcgcaccgctggcgatggaagcattaatggccttcttcctcgaatccacctttgtcgggctgttcttcttcggctggcaacggctgaataaataccagcacctgctggtgacgtggctggtggcgttcggttcaaatctctctgcgttgtggatattgaatgccaacggttggatgcaatacccgaccggtgcgcattttgatatcgacaccctgcgtatggagatgaccagcttcagcgagctggtctttaatccggtcagccaggtgaaatttgtgcacaccgtaatggcgggctacgtgaccggggccatgtttattatggcgatcagcgcctggtatttactgcgcggacgggagcgcaatgtcgcattacgctcgtttgccatcggttccgtcttcggtactctggcgattatcggtaccctgcaactcggagacagttctgcgtatgaagtcgcgcaagtacaaccggtaaaactggcggcgatggaaggggagtggcaaacggaacctgcacctgcaccgttccatgtggttgcctggccggaacaggatcaagagcgtaacgcctttgccctcaaaattcccgcgctgctagggatcctcgccactcactcattagataaacccgtgccgggtctgaagaatttgatggctgaaacctacccacgcttgcaacgcggacgtatggcctggctgttaatgcaggaaatatcgcaaggcaatcgtgagccgcatgtgttgcaggcattccggggactggaaggtgacctgggctacggcatgttgctctcccgctatgcgccggatatgaatcatgtcacagccgcacagtaccaggcggcgatgcgtggcgcgatacctcaggttgcgccggtattctggagtttccgcatcatggtgggctgtggttccctgctgctactggtgatgctgattgcgcttgtccagacgctgcgtggcaaaatcgaccagcatcgctgggtgctgaaaatggcgctctggagtttgccgttgccgtggattgcgattgaagccgggtggtttatgaccgagtttggtcgtcagccgtgggcgatacaggacatcttaccgacatactccgcgcactccgctttaaccacaggacaactggctttctcactgatcatgatcgtagggctttacaccctgttcttaatcgccgaagtctacctgatgcagaaatatgcccgtctggggccgagcgcgatgcagagtgaacaaccgacgcagcaacaggggtaaaggagaaaatcatgtttgattatgaaacattgcgcttcatctggtggctgctgattggcgtgatcctggtggtctttatgatctccgacggatttgacatggggatcggctgtctgctgccgctggtggcgcgtaatgatgatgaacgccggatagtgataaacagcgttggtgcacactgggaaggcaaccaggtctggttgatcctcgctggtggggcattatttgccgcctggcccagagtgtatgcagcggcgttttccggcttttatgtggcgatgatcctggtgctgtgctcactgttcttccgcccgctggcctttgattatcgcggaaaaatcgccgatgcacgctggcgtaaaatgtgggacgccggtctggtcatcggcagtctggtgccgccggtagtcttcggtatcgccttcggcaacttgttgctcggcgtgccgtttgccttcacaccgcaattacgcgtggagtatctcggcagcttctggcaactgctgacgccattccctttattgtgcggattgctcagccttgggatggtgattttgcaaggtggcgtctggttacaactgaaaactgttggtgtgattcatctgcgttcacagctggcgaccaaacgcgctgcactgttggtgatgctgtgctttttgctggcgggttactggctgtgggtcggtattgatggctttgtactgctcgcccaggatgctaacggtccttccaatccgttaatgaaactggtggcagtgctacctggtgcctggatgaataattttgtcgagtcgcccgttttgtggatcttcccgctgctgggattcttctgcccattgctgacggtgatggcgatttatcgtggtcgcccgggttggggatttttgatggcatcattgatgcaatttggcgtgattttcacggcaggcatcacgctgttcccctttgtcatgccgtcaagcgtgagtccgatctccagcctgacgttgtgggacagtacttccagtcagctgacgctgagcattatgttggtaatcgtgctgatatttttgcccattgtgttgctctacactctctggagctactacaaaatgtgggggcgcatgacaacagaaactctccgccgtaacgaaaacgagttgtactaaggagcagaaacaatgtggtatttactttggttcgtcggcattttgttgatgtgttcgctctccacccttgtgttggtatggctggacccgcgtctgaaaagttaacgaacgtaggcctgatgcggcgcattagcatcgcatcaggcaatcaataatgtcagatatgaaaagcggaaacatatcgatgaaagcgatcttaatcccatttttatctcttctgattccgttaaccccgcaatctgcattcgctcagagtgagccggagctgaagctggaaagtgtggtgattgtcagtcgtcatggtgtgcgtgctccaaccaaggccacgcaactgatgcaggatgtcaccccagacgcatggccaacctggccggtaaaactgggttggctgacaccgcgcggtggtgagctaatcgcctatctcggacattaccaacgccagcgtctggtagccgacggattgctggcgaaaaagggctgcccgcagtctggtcaggtcgcgattattgctgatgtcgacgagcgtacccgtaaaacaggcgaagccttcgccgccgggctggcacctgactgtgcaataaccgtacatacccaggcagatacgtccagtcccgatccgttatttaatcctctaaaaactggcgtttgccaactggataacgcgaacgtgactgacgcgatcctcagcagggcaggagggtcaattgctgactttaccgggcatcggcaaacggcgtttcgcgaactggaacgggtgcttaattttccgcaatcaaacttgtgccttaaacgtgagaaacaggacgaaagctgttcattaacgcaggcattaccatcggaactcaaggtgagcgccgacaatgtctcattaaccggtgcggtaagcctcgcatcaatgctgacggagatatttctcctgcaacaagcacagggaatgccggagccggggtggggaaggatcaccgattcacaccagtggaacaccttgctaagtttgcataacgcgcaattttatttgctacaacgcacgccagaggttgcccgcagccgcgccaccccgttattagatttgatcaagacagcgttgacgccccatccaccgcaaaaacaggcgtatggtgtgacattacccacttcagtgctgtttatcgccggacacgatactaatctggcaaatctcggcggcgcactggagctcaactggacgcttcccggtcagccggataacacgccgccaggtggtgaactggtgtttgaacgctggcgtcggctaagcgataacagccagtggattcaggtttcgctggtcttccagactttacagcagatgcgtgataaaacgccgctgtcattaaatacgccgcccggagaggtgaaactgaccctggcaggatgtgaagagcgaaatgcgcagggcatgtgttcgttggcaggttttacgcaaatcgtgaatgaagcacgcataccggcgtgcagtttgtaatgcataaaaaagagcattcagttacctgaatgctctgaggctgatgacaaacgaagaactgtctaatgcgtagaccggaaaaggcgttcacgccgcatccggccactttcagttttactctttctcggagtaactataaccgtaatagttatagccgtaactgtaagcggtgctggcgcgtttaatcacaccattgaggatagcgcctttaatattgacgcctgcctgttccagacgctgcattgacaaactcacctctttggcggtgttcaagccaaaacgcgcaaccagcaggctggtgccaacagaacgccccacgaccgcggcatcactcaccgccagcatcggcggcgtatcgacaatcaccagatcgtaatggtcgttcgcccattccagtaattgacgcatccgatcgcgcatcagcagttcagacgggttaggtggcacctgaccgcgagtaatcacatcaaagcctcctttgccaaaatgctggatcactttgttgagctcatctttacctgccagatattccgacaagccatgttcattactcacggtaaacaggttatgcgaataaccacggcgtaagtcggcatcaataaataacactttttgatcggactgggcgatcaccgctgccagagttgaactgacaaacgttttaccactgtctggcgtcgcaccggtgatcattagaatgttattctccgtctccatcatagcgaaatgcagactggttcgtagcgcacgtacggcttccacagcagaatccgccgggttatccaccgccaggaaggggatatttttagtacgatggcgctgctgattagaaaataaatttttcttacgcagacgggtgcgtttatccagccactcggacattgggatagtggcataaacgctgatgccgtgctcttccagttgttccggggcttctacaccacgacgcaacatcgcacgcgccagcacggcacccacagaaataaacaggccaagaataaaaccaagcaccacgttcaacgcttttttcggtttcactggctgcggctgagtgactgccgggtcgataatccgcacgttaccaatggcactggatttcgaaatactcaactcctgctggcggttaagtaattgcagatataccgcacggcccgcttctacgtcacgacttaaacgcaacacttcctgttgggtggaaggcattgccgatacccgcttattcaggcgtttgcgttcttgctccagcgtctggcgtttttccagcagcgcacgataagttgggtgatctttcttatacagctgggagatctctgcctcgcggaaggtcagctcattgagttgattatcaacgttcacaatctgctcaagaacggctttggcttccaggttaaggtcaaccgaatcgcgctgctggcgataaacgttgagtttttcttccgcttggtccagctcgctgcgcacttcaggtaactggcgctgtaagaattcaaggctttgtgaatcctgcgccgcctggcgagcgatattctgttgcaaatagttgttagcgatgctgttcagaatacgagtaatcaactggggatcatcaccagtcatggtaagttccagcatcccgctttctttactgcgttcgctaacggtaaaggtttcctgcaatgcgttaatcgcttccagttcggtacgctggctcaggacaaactgtgttcctggtttggccttaatgtccgcgatagtcagcgcaacgccatctttttccagacgctggccgaccataccattgacggtgaactcttcaccttccagtgtatagtggccgttttccccaaccgtgagtgtcagttgctgatcctgaccattcagttgtggaatatgcatccagctgatcgccagctcacctggtttttctttggttaatctcgcccagccgcgacccacaatcggaaaatacttctgctcaactatgtcgcgcagattcagttcagcaatggttttaccgagaatcatgcgcgattgcagcagttggatctccggtgcagactcgggcgatgagttagggatcatatcgctcaggccgctgagaatggcgttgccctgtttttgctcaacctggaccagagtatctgcctgataaattggtgtgcttaacagcgagtaagcgacagcgatcagcgtgaataacgcggtcacgctgataataaacttacggtgatcccataactcgccgaccagacgaagcagatcgatctcattttcctgagtgctgcctggtggcgtattcatatttttagttgtcatcgtattttataaactcaaattaccggctgaggcgcttcgcccattcctgactggcgcgctccaacataccgtagacatgttcaaatgcgtcctgacttttacgatagggatccgggatctctttctgttccagccattgcccaaacagcattgtcttcccgcggacctcgggagcaattgcggtaacctgagcaatatgttccgactccattgccagaatcagatcgtaatttcgtgccatctcagcagtgagcttacgtccggcatgtccttcaagagatacgccatgattagcggcaacatctgccgctgtcgcatctgcagggtgttttaccagaccatgaacacctgccgatttgacttttacgcccggcagacgtttacgcagcaagcgctcgccaatgggcgaacggcaaatgttgccggtacaaaccaccaggattgagttaaattttagttgggccatgtttgaatccaccgtgaagtctctgtcaggtcatgcaccccggaaatcgtcggtaccagcagagaaatcacacggttccaacgagccagcggcgcggtagtgacataaacaatgtcgtaaggttcaagctggaattccgttccgagtatcattgccgatgcgtccttcgcattcagctgataaatattggcgattttgccattctgcttgttttgcgttgcacgaataacaaaaatccccgtcgcatcagcgacatcctgattcataccctcagcgttacccagcgcttccgccagggtcataccgctgcggtccattttcagcgtgctctgtttacccacttcacccatcacgaagactttcagatcatcgttgcgcggaataaataaaatatcgcccgggtgcagcagtttgttctggcgcaagtcgccacgctgcatcagcgcatagaggttcactttggtctttacgccattctgggtgagcaccacgttgcgccagtctgcatctgcggtcagaccgcccgcggcgttaatcgcatccatgatggtcagaggaatattggtaatcggctgctgacccgatttgctgacttcgccggtgacgtacgctttttgcgatcggaacgccgcgacgctgacatcgacttgcgggctttcaatgactgaatcgagacgcgctgtaatctcgttgcgtacctgggtaagtgttttcccggccactttcaggcgaccaatataggggtagaaaatcgcaccatcggcgttaacccagttgccggtatcactggcgctacggtattgccctgcgggggtggttagttccgggtgatcccagaccgtaaccatcaacacatcaccaatcccgatacgatattcatagtttgcgatttgctgctccagctccgggttagcctgcgacataatcggtttggcgcgcaactgatcaatcaatcctggcgtgacgggatagatattgaccattttgtccaggtcatactgattgtcaggtagttcaatgacatccttgttactggtcgataaattctgaccaggaacaagggtacatgctgtcaaagacagaacagccaatgtcagtaccgaaaacttaaaaatgttctttttcattggtttatatttatcagtcaatgtaatgttatgaattacgtcaggttattgtccaaccggtacttctcgctctgccgtcattggatagagctggtatttgcgtgacagcatttgtccaccatcacgcgtcaatggtgtccacgaaaccaccgcgcggttgcggttaggtccaatggtcatcaagtcgaatggaatcgagatataaaaacctttactaaagccgccttcgccgtagtcatctttagatacgttactgattgccgcccatacccctaccgccacgccgctgtcaaagcgtttggcgacgtcgatcgttgcgcctttatcttttgccagatattgcccaacgctaagtttcatcagtacgccattgagcgtcggcgggttccagtaagccgtcacgaaacctgttggcgtggaataatcggtgaaacgcatcatgttgtcccagtcacgttgcttcacgtagttaacgtccacacccagcgcccagcaggcatctagcgggcgataaagcagctcggaaccgacaccggcgtacatcgtttccagataaccgccatacacctggccatagaaaccattgcctaagtcagcaaaatagttcgcctgcaagttgttgagataaacgtcattgcgaacgtagtcacggatatgcgtgcgcacgcggggcagggtagagtccgcgggcaacagcgaagacttaaacttgtcgtagttgttgtaaatattggtgaaaataccgccatcaagcagcaggtggtcggtaaaccagtagcgggcactggacatcagccccagctggaacatatagaaatcttccgggccgcccagcgactgtgaaagtgttgggttgaaagagtagctaaagcgatcttcacgaatacggtagccccgaccaaaggcagaaagatcttcagcttcaacacgttgttgttgcagtggctctgattgaccaggcgctgtacctgccagctgtttgcgcaggctggctacgtcggtttcggtagtcaccatcgccatatgctcgcgcttttgcgtcacgctaatcttctcaacgccttgcggcaggttattcaccagaatccggttggcacgatcgaccgcttcacgagagtcacggtatttgtattgctgaccagacatatacagtgtcttatcgcgtagctgaatttctggcgcgtcaaagcccgcgttatacttcagggcggtaagttggtttgctaccgtggtgtactgcaatccttcagattcaggcgcaggttgatatgccggttttggcgtatcgcgcagggcagggcgcagatcgttgaaattggtccgtaacgtgaagccaaacatcaacgtgttaccgcgttcataactcaggttgagatctgcccagctggcagcgcgataaactgcgccgacgttgaaatggcttgcctgaggcagtttgccagcgaaatcattctggtaattgtttccatcgtattcgagtttcagacgcaggggattccacggcgtttgatactcaatgccgccaaagatggaagccgggccacgaaagatatcgctaaagctgatatcgcccgcatcgtgagactctgcgcgatgacaatatttatcgctcacccggcaaaacgggttggtaatattgcccgcattaccggcgtagccccatgccatcccgagggtgaaatcaaatggccccgcttgcttgctggccaccagatactcaccgtcaaacagacccgtaccagcaatatcacgtttaccaaacgccacttgcggtagccagtaaccttcttcccacaggcgaagtttaaaatcgaatgatttgtctttgtatgactgatcgccgctgaaatcttcccactggctatatttgcgtgtgcgcacatccgtataacgaatggtgccttccagccatgggaacagcgccacggaggtggagtagaaccggtattgatcgttatcccggtagttgacgctgaattcaccttccggtgcgatgcgcgcatttggcatctgcaacaatcctgtgccgccaaagtctgattgcgacgaacccagcggatccgggtaggttaatacttcagcatgacaggcactggagacggcaatggccaggcagcttaaaagataagaattcttcttcatcagtcaggaacacgttgcgttaaaacagacacaatctggtcatttaaatcagcatatttttcgggcagtacatgcgcagaaaagcccaaccaaagctggctgccaggcggtggttccacatgtcttttattccacagggcaacaggggcgacgacagtctcaccctcaggcgtaatcaccataacgttattcttgtccgcgcctgcaaggcgggggtgatcttgcagataatcggtaacgctacggcctgcctgccagggcaattgcccggccccagaaaccgcacccagcagagtaatagtcaccggacgctgtacggtatagagcgtatagtccccgaccaacgggggattgctgttctcatccactcgtacaaaatcagggtccagtttgaccggtaagcgaccagtgatattgagattgagtaactgctggcgcacggatttaatcgttgccgccacatcgtcgtcagcttctgcttcccaggaagcaagctgtgccatgacatgttggtagtctttaagcgctttagctttcgccgcagagtcggtcagcaaggcaccaggccaccagaggcgatcgcgcagttgcggttgtgtcaccaactggacaacattttccacggggccaacggaaagtgtctgttgttcgccaggcagataaatagtcaccgttccttgcgcaaaggcatggggtgtcattacgtaaagtacgctggcaatgaaatacgactgtaatttattcatggtgcgggtttaagaaacgtcatttctacgggaataacccctgcgcctaacatttgccgactttgacgaacctggccagtagccgaatcgacccagaatgtgttttgccactgtttttctggccgcgtggaagtcacctcttcctgccagacattacacagcacattgcgacccgcaatattcagcgtctctaatccagcaaaggaaaaagtagaactcagggtcgcagagcgaaaatggttgtcttcactccagagaatatcgcgcgtccagcggctgccatcttttattgccagcgcgttacgcagagggtcctgcccggaatttgtcacttccagcagattattattaagtttgacggtttttaaaagacgtccattgtgggtaaccagcatggcgttatcctgggataaccatttgctttgttcttgttctatatatcccagtaccacaaagattcgttgcccttcattaaggcgtaaatacatagtggaataaggcaacgcctggatctgctgatccgctacggtgatatcctgattatcgaaaaggctggcgcgaaatgtatcgaccatactttgctggctgtgcgtacatcccgcaagaaatagtgcgaaaatcgataaaataagagggcgcacctttaatccttgaaaggttaattaaaaaaatgcaaatctctaaagcccggtacgaatatcgcaaccgggtatcatttaactttaatttcgacgcgttaaagcagtattagcgtgtagtggacgtggtggttgaggtgttatgagaaccgccatcgccactgtcatttgctgcaacaactgccaacgtcgccacaccaacagccgttgccacaccgacaactgtcgccgtgccgacagcgccagcagccacgccaccagtggtagtagcagtcgtggttgcgccggtagtggtcgttgtggtgccagtagtacccgtcgttgcctcggtcccgtttgttgcttcaggggcagcaaacgcagctggcgtcgtcaacatgaaggccataaggattgcagaaagcttgtgtttcataacttttcctttattcatcgcatggacaatacgggtgatgctgccaacttactgatttagtgtatgatggtgtttttgaggttctccagtggcttctgtttctatcagctgtccctcctgttcagctactgacggggtggtgcgtaacggcaaaagcactgccggacatcagcgctatctctgctctcactgccgtaaaacatggcaactgcagttcacttacaccgcttctcaacccggtacgcaccagaaaatcattgatatggccatgaatggcgttggatgccgggcaacagcccgcattatgggcgttggcctcaacacgattttccgccatttaaaaaactcaggccgcagtcggtaacctcgcgcatacagccgggcagtgacgtcatcgtctgcgcggaaatggacgaacagtggggatacgtcggggctaaatcgcgccagcgctggctgttttacgcgtatgacaggctccggaagacggttgttgcgcacgtattcggtgaacgcactatggcgacgctggggcgtcttatgagcctgctgtcaccctttgacgtggtgatatggatgacggatggctggccgctgtatgaatcccgcctgaagggaaagctgcacgtaatcagcaagcgatatacgcagcgaattgagcggtataacctgaatctgaggcagcacctggcacggctgggacggaagtcgctgtcgttctcaaaatcggtggagctgcatgacaaagtcatcgggcattatctgaacataaaacactatcaataagttggagtcattaccgacaatacgtacgcttgagatcaggattgtctactttgagtataacatccttgtgaaatctccctttcctcataccgcttgcactatatactgcgggtaggaaaggcgcgcagagggaaatataagattgttaactatccccctctggaaatacgacttgtgagcataagataaatcttagcaaaatacaaattaaagataaggaaattgttacgaaagctattaattattgttggtaatatagtttcaagtggtactataactggctgttaaatggcatttataactattaggtgcagagatattcgcttaaatggattagtttctttgtggaaaagtaactgatgttataatgtatgatgttgactatttcactattccaataaaaccagtcagctttaaacaagcagcgtcatattaagagagataaacatttgccgctgttggtcctcgcaggccatttacgcggcaaaattccacacgtaatcctggtataagcacttctgcgtcgcggggagtgaatgcggaaatatggacctgaacttctttacgaccgtcggaggggataatgaatcctttgccgcttttgcgatcaaaggttttgacaattcctgtcattttacgggacaaacaaattccttactgaaaatactgcgctgcactatacggggttaataaaataaagccagcgatatttaagaccgccggacggctaaaataaaatttgcttaatctcaattatcatgcgttaatagctgcgtcggtttgaaagacagacagcatacaaagtagtttactaaagcagttctcattatcaggcattatccccttcttttgagtctctctcctgaacactaagtagtttctgtattaaagccctgtttgccgaaaggcccaaaatgaaggaagtaaaatatgtctaataaaatgactggtttagtaaaatggtttaacgcagataaaggttttggctttatcactcctgatgatggcagcaaagacgttttcgtccatttcaccgccatccagagcaatgaattccgcacgctgaacgaaaatcagaaagttgaattttctattgagcaggggcaacgtggccccgcggcagcgaacgttgttacgctctaaggttgccattattactcaacatctccatttccgctgtccatgttgtcatggttcacagtaccgcacatcggcattcgatgtgacggagcgaaaccctttgggcgctaagtgtattttttgtaaatcgacgatgatcacctttgataacgtcgcgctgcaaatacgcactgaccatgcgccgctggatttcacaaaataatatcaggctccctcgtggagccttttttatatctgccttatttttcttcaacgctgtatgtatagtaagcgataacctgttgattattgaatctttcggggagatggcttataacatttcttacctgaccagggtaccgggaaccaacaccttactggcgtgttgctgtcttttaagaccagaagaggttaacagtgaatattgaagagttaaaaaaacaagccgaaacggaaatcgccgactttatcgcgcaaaaaatcgccgagctgaacaagaatacagggaaagaagtctctgaaattcgcttcaccgcacgagaaaaaatgaccgggcttgaaagttatgatgtcaaaatcaaaataatgtgattttgtgaacatcaccccgtgcgaggtgatgttccgcttgttgctaatttagtgaccaatcattggcgcttgtggaattaagcgtcggtacaattcctccggcaccgggctttgccatactcccgcatacattgcgtaaccaatcaccgcaaacataatccccagaaccagtagcgtcattaaccagccagacaacgcaaaggcttttttatttgccgcaggtttttgcagtgaaaaggtcaatgttgaggctaccggacatgactctacgcaagtcatacagccggtacattccactgttcgtacctgaattaatttatcgaccgggatccgtgatgggcaattttttgcgcatttgccacagtcgatacaactttcggcattgcgacgaatcttaaacggcgacaatagcgaaaccacgcccatcagcgcgccatatgggcaaagataacgacaccaggcatggcgaataaacaggctggcaatcagcaaaacggtcacgctgattaatgtcgcggtccccatatgacgaaagaaatcgagcattttaacgtccatcaccacgctgtagggcgacaacataaaatagtgaatcgcctgagcgggcatcaataacgcgatatagataaaaaaactcaacagcaaatacttcacgccgcgcagaggaatatccagccagcggggaaggacacattgccgaccaaacagtttgttaccgagatcgccgattaattcagaaagcgtaccaaccgggcataaccatgagcaaaaggcctttttgagtaatagactgatgacgataaaagcgaccaataacagcatcgcggcggcgtggacggacggtaactgacctgttacaaggctatatttcagattcatcagcccggcaatcggtagccagccttcgatacctcccggtctggcgacaaatgtcgtgctacttgccgtttcgtaatagcgcacccaataccagaacgtgatggcaatataaatattcattgccaacagtaataattgcgtcgctttacgccaggtcgtggcattacgccagtcattccacggtaatttgccgcccgtcgtgcctggccgccgctgccagcgggttcttttattctctgccatgattttgccagtccgttaagttgtataccaaatgccactattctagttgttcttaactggctgatattgattcaaatcgcgttcaggtctttcttatgcaaccatgcttccagagcggcaacactgcgtgtaatttcttcgtgtggaaggggggcagataatggctgctgctccagttgtgcgcatagctggctggcgatatgcattcccagactcgagcaactgctttttagctgatgcgcggcacgctttattttctcgctatcctgactggcgcgggcaatgtcgatttcatcgagaagcggcagggcatgttgtgtaaataataccagccattcgtggatcttctccgtccccattaactgagcatcttcattgagttgcgatacatccagcgattgatcattattgacttgcagttggagatagtgcgccagtaactgaccgagcacttcacgcggcaccggtttagggataatcccgcggaataatgaactggtacgctggcgcagcgtttcgtcaatgacatgggcgctaaagccaatcaaaaccagcgacggatattgctgtgccagttgtcgggcaagcgtaatgccgtcgatatccggcagatcaaaatccaccagtgcggcagcaaacggttcgctattttgcagtgtctctaaagcctgcgcggcattgccaacagcaacaatctgcgcaccactggttttcagcatctcaatggtaattcgctgggttagcgggttatcttcaattaacagcaaacgtaaaccgtcaagacgcaccgcctgattgactgtttttggcacgggtgccgtggcaacacgtaacggcaagcgtaaacaaaaacagcttccaacctccggcgtgctggtggcgctcagttcgccgcccatcgcctgggccagacggctactgatagtcagtcccagcccggtgccgccgcgtttgccgcttacctgcacaaatggctggaagatttctgccagtttcgcgggatcaataccgcagccgctgtcttccacttcgaccagccattgctcgccatcagtgcgactacgcaggataatgtacccttcgtcagtaaaacgcagggcgttgctcaacaggttggttataacctgacgaatacgtcgtggatcgcccattaacgcgcacggcatatcatcggcaattgccgttgccaggcgaatcgggcgacctttcacccgtccgctcattaattgcagggtactttccagcagcgggcgcggttcaaagggctcatcgctgaccgaaacattcttgccacctgcttcgatagcggaataatcgagaatatcgttgaggatggtcagcaacgattcaccagagtcagtaattgcccgcaaatcatcacgctgggcgttaagtgcggggttatctgccagcagttgagcagtgccgagaataccgtacagcggtgtgcggatctcatggctcatcgccgccagaaacgccgattttgcctggctggctttttctgcttccgcccgtgcctgtcggtgttctatcaccagttcctgcaattcagctgtacgcgctttgacctgcgccgccagctgttcgcggtggcgattcagtgcatgaacattgctgcgaaacgcatccatcagccgcccgatggtatccagctcccgtacgccagcggtttccgggaaaggggagtcaatatcaccgtccagcagccgttgcagcgcctgcgtttgttcggcaagtggacgcgtgactgagcgataaaccacgcgccagaggatcagaatcagtgcgcaaagtgaaaccatccccagcaataacaggctgtattgcccgcgtgcactcgctttttccagatgcgccagtccgtgctgattacgcagctcaatggtgtcgaccagctgactgacttcgctactaaactgcgcgaactgggcgatgttattttgtgcgagagtttgtaggtgattgctgatttcactgtcctgctgatacagcgccagcaaatcgctatattggctaacggtagttaacgttgttgcgacctgcgcacgaacacccggatcttcaatgcgtatttgccgacgttgcagaattttcaccgcattattgagctgcttttccagcgttggtgcatttttctggatctgctccagccccagattcatcaccatttgctgcacccgcagagcgctaaggcgcagttcattcatctggttaacatactcaagatcgatatcaatcagccgatcgagtgcactttcagcagcctgacgctgatcttgttcgatcaaatcgtaaatcccggcctgggtcgctccagcggaagttgtcgcattattcgcctgaccttgcgccaggcgtgcgatctcatcggcggcagcgactatctgctgactgagttgctgttgttgctggcgcagttgcaaacgctgccccaccagttccccttgctgacgtaacgaacgggagatctcctgctcctgttgttcaatagcggtggtatcaaaaccttgttcccgtaacgcttgcagcaacgcattaatcttcaggctttgtgcggtgagcattcgcccctgcgcctgccacatcttttcgttatcggcactggtcaggttctgcgcggcgaaaagttcccaggcgctggcttcgctcaactggcgcgccatattcatggtaggaatcaatgcctgagtgttgtctttttccacctggctgataaagcgcaggttgtaccatcccaccagggtactggtcagggttaacagcgccatcagggcaaagcccatccagagtcttcgggtcagggttaaattcacggtcggtgcactttaggtgaaaaaggttgagtcgcaaagcggaatgcatctagcataaagccttattattgatgaggctatcatgcgcgtactgctatttttacttctttcccttttcatgttgccggcattttcggctgataacctgttgcgctggcatgatgcgcagcatttcacggtgcaagcctctacgccgcttaaagccaaacgcgcatggaaactgtgcgcgctttatcccagcctgaaagattcatattggttatcgttgaactatggtatgcaggaggctgctcgccgctacggtgtggatttaaaagtgctggaggcaggcggctacagccagttggctacccagcaagcacaaatcgaccagtgtaaacagtggggcgcagaggccattttgctcggtagtagcacgacctcatttcccgacctgcaaaagcaggtagcaagtctgccggtgatcgaactggtaaatgctattgatgctccccaggtgaaaagccgcgttggtgtgccctggtttcagatgggctatcaaccggggcgatatctggtgcaatgggcgcacggtaaaccactgaatgtgctgttgatgcccggacccgataacgccgggggcagtaaggagatggtcgagggttttcgcgcagccattgccggaagcccggtgcgtattgttgatattgcgcttggtgataacgatattgaaatccagcgtaacctgttgcaggagatgctggaacgccatccagaaatcgacgtcgttgccggaacggccattgcggcagaggcggcaatgggggaagggcgtaacctgaaaacgccgcttaccgtggtgtcgttttatctttcacatcaggtgtatcgcgggctgaagcggggaagagtgattatggctgccagcgatcaaatggtctggcagggggaactggcggttgagcaggccatcaggcaattacaggggcaatcggtttctgataatgtcagcccaccgattttagttctgacgccgaaaaatgccgaccgtgaacatattcgccgctcgctgtcaccagggggatttcgtccggtctatttttatcagcacacatcagcggctaagaaataaccttcaccatgttgcgtcaccagtaaatccgcgctgagtttatgacgtaaacgacgaattaacacatcgacggtgcgcaggtcagggttttccacccgacgcgcagaaagcatacgtagcagacgttcacggctgagaatttcgcccggattcgtcacaaatgccaccaacatttcatactctgcgcgggtcagtttaatcggctcgccatcccgctccagcgtatggcgcgacacattcaggcaataaccggcaaagcgatagcagttgtcctgagtgtgcggttgagcttgtcgcgcgaggtcgattcgccagagcagatttttcacccgtactaccagttcgcgcagttccagcggtttggtgacgtaatcgtctgcgcccatttccagcccaacaatacggtcaatccgatcgctgcgtccggtaaccagaataatccccaccgttgagcgttctcgcagggcgcgggttaacatcaggccattttcatcgggtaagttgatatccagcagaattaaatctaccgactgattctgcataatttcccgtagcccagcaccgctcgccgtaacggaaacggtatacccctcctgagtgaagtaggattgtaatcgcgcctgggtaaccggctcatcttcaacaataacaatgtgatgtggcatcagagggttttactcattctgttcatatctgttcatattctgccgtaagccgttcatcctgaccagtgccgctgttcatatttgctcattaagatcgcttcactaaaccataattctacaggggttattatgcggaaactctggaacgcgctacgccgacccagtgctcgttggtcggtactggcgctggtcgcaattgggattgtgattggcattgcgctgattgtattgccacacgttgggatcaaagtcaccagcacaaccgaattttgtgtcagttgccacagtatgcaaccggtgtatgaagaatataaacagtcggtgcatttccagaacgcctccggcgtgcgagctgaatgccatgactgtcatatcccgccggatattccaggcatggtgaagcgcaaactggaagcgagcaatgatatctaccagacctttattgctcactccattgatacacctgaaaaattcgaagccaaacgcgcggaacttgccgagcgtgaatgggcgcgaatgaaagaaaacaactcggcaacctgccgctcctgccataactacgatgcgatggatcatgcgaagcagcatcctgaagcagcacgtcagatgaaggtggcagcgaaagataatcaatcctgcatcgactgtcataaaggtattgcccaccagttaccggatatgagtagcggcttccgtaagcagttcgatgagctgcgcgccagtgctaatgacagtggtgacacgctgtactctattgatattaagccaatttatgcggcgaaaggcgataaagaagcctctggttctctgctgcctgcttcggaagtgaaagtccttaaacgtgacggcgactggctgcaaattgaaattaccggctggacggaaagcgccggacgtcagcgtgtactcacccaattcccaggtaaacgcatctttgttgcctcgattcgtggtgatgtgcagcagcaggtaaaaacgctggagaaaaccaccgttgccgacaccaataccgagtggagcaagttgcaggccactgcgtggatgaagaaaggcgacatggtgaacgatatcaaaccgatctgggcttatgcggattcgttgtacaacggcacctgtaaccagtgccacggcgcaccggaaatcgcccactttgacgctaacggttggatcggcacgctcaacggcatgattggctttaccagtctcgataaacgtgaagaacgcaccttgttgaaatatctgcaaatgaatgcgtctgacaccgcaggtaaggctcacggcgataagaaggaagaaaaataatgaacaataacgatctctttcaggcatcacgtcggcgttttctggcacaactcggcggcttaaccgtcgccgggatgctggggccgtcattgttaacgccgcgacgtgcgactgcggcgcaagcggcgactgacgctgtcatctcgaaagagggcattcttaccgggtcgcactggggggctatccgcgcgacggtgaaggatggtcgctttgtggcggcaaaaccgttcgaactggataaatatccgtcgaaaatgattgccggattgccggatcacgtacacaacgcggcgcgtattcgttatccgatggtacgcgtggactggctgcgtaagcgccatctcagcgatacctcccagcgcggtgataaccgttttgtgcgcgtgagctgggatgaagccctcgacatgttctatgaagaactggaacgcgtgcagaaaactcacgggccgagtgccttgctgaccgccagtggttggcaatcgacggggatgttccataacgcttcggggatgctggcgaaagctattgccttgcatggtaatagcgttggtacgggcggagattactctaccggtgctgcgcaggtgatcctgccgcgcgtagtcggttcgatggaagtgtatgaacagcaaacctcctggccgctggtattgcagaacagcaaaaccattgtgctgtggggctccgatttgctgaaaaaccagcaagcgaactggtggtgcccggatcacgatgtttatgaatattacgcgcagctaaaagcgaaagtcgccgccggtgaaattgaggtcatcagcatcgatccggttgtcacatccacccatgagtatctggggcgcgagcatgtgaagcacattgcggttaacccgcaaactgacgtgccgctgcaactggcgctggcacatacgctgtacagtgaaaacctgtacgacaaaaacttccttgctaactactgtgtgggttttgagcagttcctgccgtatctgctgggtgagaaagacggtcagccgaaagatgccgcatgggctgaaaaactgaccggcattgatgccgaaaccattcgtgggctggcgcggcagatggcggcgaacagaacgcaaattattgctggctggtgcgtgcagcgtatgcagcacggtgaacagtgggcgtggatgattgtggttctggcggcgatgctggggcaaattggcctgccaggtggtggttttggttttggctggcactacaacggcgcaggcacgccggggcgtaaaggcgttattctgagtggtttctccggctctacgtcgattccgcctgttcacgacaacagtgactacaaaggctacagcagcactattccgattgcccgttttatcgatgcgatcctcgaaccggggaaagtgatcaactggaacggtaaatcggtaaaactgccgccgctgaaaatgtgtatttttgccggaactaacccattccatcgccatcagcagatcaaccgcattattgaaggcttgcgcaagctggaaacggttatcgccatagataaccagtggacctcaacctgccgctttgccgatatcgtactgcctgcgaccacgcagtttgagcgtaacgatctcgaccagtacggcaatcactccaaccgtggcattatcgccatgaaacaggtggtgccgccgcagttcgaggcgcgcaacgacttcgatattttccgcgagctgtgccgtcgctttaatcgcgaagaagcctttaccgaagggctggacgaaatgggctggctgaaacgcatctggcaggaaggtgtacagcaaggcaaaggacgcggcgttcatctgccagcgtttgatgacttctggaataacaaagagtacgtcgagtttgaccatccgcagatgtttgttcgccaccaggcattccgcgaagatccggatctcgaaccgctgggcacgccgagtggcctgattgagatctactcgaaaactatcgccgatatgaactacgacgattgtcaggggcatccgatgtggtttgagaaaatcgaacgctcccacggtgggcctggctcgcaaaagtatccgttgcatctgcaatctgtgcatccggatttccgacttcactcgcagttatgtgagtcggaaacgctgcgtcagcaatatacggtagcgggtaaagagccagtattcattaacccgcaggatgccagcgcgcgcggtattcgtaacggtgatgtggtacgcgtctttaacgctcgcggtcaggtgttggcaggggcagtggtttctgaccgctatgcacccggcgtggcacgaattcacgaaggggcatggtacgatccagataaaggcggcgagcctggtgcgctgtgcaaatacggtaaccccaacgtgttgaccatcgacatcggtacatcgcagctggcgcaggcgaccagtgcgcacactacgctggtggaaattgagaagtacaacggaacagtggagcaggtgacggcgtttaacggccccgtggagatggtggcgcagtgcgaatatgttcccgcgtcgcaggtgaaatcatgaccacgctgacagcacaacagattgcctgtgtttacgcctggctagcgcagttgttctcccgtgagctggacgatgaacaactgacgcaaatcgccagtgcgcagatggctgaatggttttcgttgctgaaaagcgaaccgccgctcactgcggcggtgaacgagctggaaaaccgtattgccacgctgacagtacgtgacgatgcccgtctggaactggccgcggacttttgcggcctgtttctgatgaccgacaaacaagcggcgctgccgtatgcatcggcctacaaacaggacgagcaagagattaaacgcttgttagttgaggcagggatggaaaccagcggcaatttcaacgaaccggcagatcatctggcgatctatctcgaattgctcagccatctgcatttttcgctgggagaggggaccgttcctgcgcgaagaatcgacagtttgcggcaaaaaacactgacggcgctgtggcaatggttaccagagtttgttgcgcgttgtcgtcagtatgacagctttggtttttacgcggcactaagccagttattgctggtgttagtggagtgcgaccaccaaaacagataacgtcgtttgtgcgcctgaaaagacgcgtttagcgtcgcatcaggcattatggcgcagttgccggatgcggcgtgaacgtcttatccggcccacaggaactgtaatctttgtagaccggttaagatgcgtcatcgcatccggcaaacacacatcacggatgagctacaaaccgggaaagccgctggcgcagcaggcggttttcctgcttcaggtgcgcaatatcatccattaacgtcagcgccaccgcgatccccggccagtccagagccagttcatgacgcaggcgtaccgcgcgttgcaccacaatggcggcatggtcgtcaaatacccaggttgtttcctggatctcacgcggttcaaccacccccaaaccgacaatttcattcaactcctcttcagagatgccggtatgcaggcaaaattcggtaatagtaaaagtcaccgtaacattagccattatgctttcccccaatctttacgtggatcaaaagacgactgggcgtctgccagttgctgccacagcgcggcagtgttttcatccggtttcggcggcatcacgattttcagtaccgcatacagatcgccggtctgttttttgctcaccagacctttgcctttaacgcgcaatcgttgcccggcctggctgcctggcgggatagtcagcaaaatgctttctttcagtgttggaacggtgactttagcacccagcgccgcttcccacgggctaaccggcaccacaatttccagatcctggccgacaatatcaaacagcggatgtggcgcaatatgaatcaccagccacaaatcgccatttggaccgccgttttcgcccggcgtcccctggcctttcagacggatgcgttgaccattgccgacgcccgccgggatcttcacattcagcgttttcggaatttcctgttcgatcatgccaaaggcgttataaaccggcaggttatagctgatggtacgcttatgctcagtaagcgtttcttcgaggaataccgccacttcgatttcaatatcgtggccgcgtgtggcggggcgttgacggctctggcgggcatgctgaccgaaaattgacgagaagatatcgtcaaaatcttcggcgttaaaactctgaccgtcgccatggtggaactgacggttaaattgcggatcgttgcgatgttgccacatctgatcatactcagcgcgacgttgttcatcacttaacacttcccaggcttcagcgacctctttgaagcgggcttcggcatccggttctttgctgacatcaggatggtatttgcgggcaagtcgacgataggcggtcttgattgtcttgagatcgtccgtcggtttcacgcccatgatggcgtaataatcctttaattccatagcgttatctcgcgtaaatcaacacaaattgaaggaacccctgtaaggtaactcctataagtgtagggtaatcctcaaaatttcatatgccaacacagaatatgttattgaaatcatcgcggagaggaggtcgccatcaagatgggttgctgaacatattttaaacaggtgaaaaagggtgagcgatttttgatagttgaaccaggcactttaagtttaactagggcgtcattatttattaaattttatagacgctatatatgggtagtaatatacatggaattagttgcactgcaaataattatttgaaacaggcctggaacgatataaaaaatgagtacgaaaaaaatcaaacatattcaatcacgctttttgaaaacacactggtgtgttttatgcggttatacaatgaactcagacgtaaagtaaatgaagaggatactccatgtctggaatgtgaatcactagaaaaagaatttgaggaaatgcagaatgataatgatctatcattatttatgagaatattgcgtactaatgatacacaaatttattcaggggtttcaggaggtattacatatactatacaatatgttcgagatattgatattgttagagtgtccttgccgggcagagcttcagagtctatcacagattttaaaggttattattggtataactttatggagtatattgaaaacattaatgcgtgtgatgatgttttttctgagtattgttttgatgatgaaaatataagtgtccagccagagcggataaatacgccgggaatatctgatttggattctgacattgatttgtctggtatatcttttattcagcgtgaaactaaccaggcattaggattaaaatatgctcctgtagatggcgatggatattgtctgttaagagctatactggttttaaaacaacatgattattcatgggcgctggtcagttataagatgcaaaaggaagtttacaacgaattcattaaaatggttgataaaaaaacgatcgaggctcttgttgatacggcattctataatctcagggaagatgtaaagacgttatttggcgttgatctacaatctgacaaccaaattcaggggcagagtagtcttatgtcatggagctttctgttttttaaaaaacaattcattgatagttgcttgaataacgaaaaatgtatcctgcatttacccgagtttatatttaatgataacaagaacttgcttgctttagataccgacacgtcggataggattaaagcggtgaagaattttcttgttgttctttcagatagcatttgctcattatttattgttaatagtaatgtggcatcaatctccttggggaatgaatccttttcaacagatgaagatcttgagtatggttatttaatgaacactggcaatcattatgacgtttacctccctcctgaactttttgctcaggcttacaagttaaacaataaggaaatgaatgcgcaactcgactatttaaatcgttatgcaatttaatggcaaaggcatatgctaaaaaccattgttattagtctcacacttttttattggtaaatattgtctctgtattggtaacgccgcagatattctgtttagccacaggtgcaattatcagcggcgtacgcgaggcaggggctaatcaggcatagtttgcgtcaaaccttgcctgtttttgaagatgtatatagaaaaacaggcgttcaacaagccattttgcgaacctgttcccggaaaaaagtcatatttctgtcacactctttagtgattgataacaaaagaggtgccaggaatgaacaaaacgctaatcgccgcagctgtggcagggatagttttactcgcttcaaacgctcaggcacaaaccgtaccggaaggctatcagctacagcaagtgctcatgatgagccgccataacttacgtgcgccgctggcgaacaatggcagtgtgctggagcagtcgacgccgaataaatggccagaatgggacgtccccggtgggcaactcaccaccaaaggtggcgtgctcgaagtgtatatgggccattacatgcgtgaatggctggcagagcaggggatggtgaaatcgggggaatgcccgccgccgtacaccgtttatgcctatgccaatagtctgcaacgtaccgttgcgaccgcacagttctttattaccggcgcattcccggggtgtgatattcctgtgcatcaccaggaaaaaatgggcactatggacccaacctttaacccggtgatcaccgatgattccgccgcattcagtgaacaggcggtggcggcaatggagaaagagctcagcaaactccagcttaccgacagctaccagctactggaaaaaatcgttaactataaagattcccctgcctgtaaagagaaacaacagtgttcgctggtggatggcaaaaatacctttagcgccaagtatcaacaagaaccaggtgtttccgggccgctgaaagtcggcaactcgctggtagatgcgtttactttgcaatattacgaaggttttccgatggatcaggtggcctggggagaaatcaaatctgaccagcagtggaaggtgttgtcgaagcttaaaaacggctaccaggacagcctgtttacctcaccggaagtggcgcgcaatgttgcgaaaccgctggtcagttatatcgacaaagctctggtcaccgatcgcaccagcgcaccgaaaattacagtgttggttgggcacgactccaacattgcctctctgttaacggcgctggatttcaaaccgtatcagttgcatgaccagaacgaacgcacgccgattggcggcaaaatcgttttccagcgttggcatgacagcaaagccaatcgcgatttgatgaaaattgaatatgtgtatcagagtgcggaacagttacgtaatgccgatgcgttaaccctgcaggcacctgcgcagcgtgtgacgctggaattaagcggttgcccgatagacgctgatggtttctgcccgatggataagtttgatagcgtgttgaatgaagcggtgaaataacagaaaactcccccgcgagaagcgggggagtcgctggttaaacgtttttacgttcgatggtctgttcgccccaaaaaagcgaatctttatcggtcttagcaaaggctttgactaacacttcatcactaccttcttcccaaatcttttccgccattttttcgtcgtacccggcgacttcgaaaatggcctcggctatttccggcgacgtattgcgcagagatgcccattcaccgacgtgatgagctttcgcttcttgagttggcatgcgtatcctcctgttgaagattagccgttaagtttaactgccagacctgcgacatattccccttgataacgagcaatagacagttcttcctggctgggctggcgtgaaccgtcaccgcctgcgatggtggttgcgccgtacggcgtaccgccgcgaacctgtgaaacgtcaaataattcctgcgctgcgtagccaatagggacaattaccatgccgtgatgcgcaagggtcgtccaggtggatgtgatggtttgttcctgaccgccgccagtaccggtggaactaaagacgctcgccagttttccgtatagtgcgccggaagcccacaggccgcccgtctggtcgaggaaggtacgcatttgaccggacatgttgccaaagcgggtaggtgtaccaaaaataatggcgtcgtaatcggccagttcttgcggggttgcaaccggtgcagtttgcgttttaccgcctgctttttcaaataattgcggcggcatggtttccggtacacgcttaacgacaacttcagcgccatccactttgcttgcaccctcagcgactgcgcgtgccatcgtttcaatatgtccgtacatggaataataaagcaccagaactttagccatttctaaccactcctcgtgttatctctattccgtagcgattcgctaccacttatttaaagataagacgtccttttcagagtgcaaatttcacaaccacttatttgatttataacaactttcacaagcacgtaattttgtcgcaaaatgacacatttttatctcatcgcgtttttttaatcataagagcggcttatggataattattggagatgatatctattctcgctaagaagctgttgcaggatattaccaaacgcgggtctgcccgcgtcagttcactaagcttagtcccacgtagcgaaaatatggcagccgccatacgccgcgttaattctatgcaatatgatgtctatacccagacggaggtcagtaatggcaaaccatcgaggcggttccggcaattttgcagaagaccgcgaaagagcatcagaagcaggtaaaaaaggtggacagcacagcgggggtaatttcaagaatgacccgcagcgcgcatctgaagcaggtaaaaaaggtggtaagagcagtcacggcaaaagcgacaactagccgggctaatcaatgacgaatgcatttttgtctgtagctcgtcaaaaagccatcaccgccggttacccggtggttgatactgatgacaaatgtaagcttgcctgatgcgcgatgcttatcaggcctaccagaagattgcaatatattgaatttgcactgttttgtaggccggataaggcgtttacgccgcatccggcatgaacaatgcgtacgttgtcaacaatctgcaccgccggtaaccccggcggttttctgtttatggctcctgatgaacaacttctggcggtggaacgtcaaccaactttctgcttaacaacgcattgagtaaaatcgcgccaaaggttgctgtaccaatccctcccaacgtaaaaccgcccagcgtgagagcaaaatcacccgcgcccagcactaaggttactgcgaccataatcaaattaccgttctggcttaaatcgacacggttttgtacccatatccttgcgcctgcgacggcaatcagcccgaacacaacaattgatgcaccaccaataaccgcggccggaatggtatgaatcagcgcaccaaatttcggtgaaaagcccaacagcatggcgatgacggcagcagcaacaaacaccagcgtcgagtagactttggtcacggccatcacaccgatattttcagcataggtggtcacgccgctaccgccgacagagccggaaagcatcgttgccagaccatcgcctacgaatgcccgccccatatacgggtccatattgcgtccggtcatcccggcgactgccttgagatgacctaagttttccgccaccagaatcaccgccacgggcgcaatcagcatcattgcctgaccattaaaagcaggagtggaaaaatgtggcagaccgaaccaggcagcatggctgacgagagtaaaatcgacggcttttcccagccctaaaacgttggtcatcacgccatacagcagacaggcgacaattaatcctacgagaatcaataaccgctggatcatgccacgggtaaacaccgccaccagcccaatacacagcaccgtcattaccgccatccagctatcaaaggccgaagccgatacacttttcactgcgataggcgctaagttcaggccaatcgccatcaccaccgcacccgtcaccaccggcggcatcagtcgttcaatccagcgcgtaccgattttcatcaccaccaggccaatgacggtataaaccagcccacaggcgataatcccgcccagcgcaatgctgatattcgggttaatgccctgaccgttaaagcccgtcgcggcgatcaccacgccgacaaaagccgcgctggagccgagataactggggacgcgcccgccggtaataaagaaaaacagtaacgtgccgatccccgacattaaaatggaaagattgggatccagccccatcagaatcggcattaacaccgtcgcgccaaacatcgccaccgcgtgttgaacgcccattactgccgtctgagcaaacggcaatcgttcatccggcgcgaccacgccgctctctgtagaggtcgattttaactgccagtgaggaaaaccgaacattgccatcagctgtctccttaaggaggttaacaagcagggcgcatcagcgcgtgataactgcgatcgaaccacaccagcccgtagggtgtggtgtgacgatgaatcgcttcgatggcgcaaaacagaatgtcgtgggtgccgacgctcaccacctggctgatacggcagtcaaacgaaaccagagcctcttccagttgcgggcatccggtcacccccgtctgccagcgggcggcggcaaagcggtgttccatgggcgttttgccgccaaaaaggtttgaaagcggctcctgcccggcgctaagtgtatttacacacagcgttcgattttcattgaatgccggccagacggacgccccacgattcaggcacaccagtaatgtgggcggcgtatcggtcacactgcagacggcgctggcggtgaacccggcgcgcccggctggaccgtccgtggtgataatattgaccgccgcgcccatgcaggacatcgcatcgcgaaaagtttgttgatcgacaatgttcatagtttgctccttacaacagcccgcaggcttcttcaaaggacagacgtggcaggcgcgcataaagcttgctgctatcgccatagccgatattaatcagcagattgctcttcagcgtgctgcccgtaaaaaaggcgtcgtccacgtgttgacggtcaaagcccgacatcgggccggtatccagtcccagcgcccggcaggcgacgatcagataggccgcctgcatggaactgttgcgaaacgctgtttcttcggcaagttgtgggctggaggtaaaccaactgcgggcatcaccgtggggaaacagtagtggtaaccgttcataaaattcactgtcccaggcgacgatagcggtgacgggcgcggtcagggttttttgcagattgccgctggaaagtgccgggcgcagacgttcttttccttctgccgtgcgggtaaacacgatccgtgccggagaacagttagctgatgtcggcccccatttcatcagggcataaatctcccgtaacgtctcatcgctgacgggtgtctcccgccagccgttgtgagtgcgggcatcggtgaacagggtgctaagcgcacctgggctaacggcttcgttcatagcaattccttacagggcggcttcacggtgatgtaacaggctggcaagcccgttgagtaacagagcattaaacgtttcgggatcggtcacgttgcaggcgtgtccgccatagggcatcaccattttctggctatcgggcagggcggcatgaagttcactggaacatgctgttggcaccagcagatcatcactggcgcagatgatttgcaccgggcagcggatgcgatccgcatggtgactaaagtcagcgcgtttgagggcgttaagtcgacgcagtaaattatttttgccctgaaaatgcgccagtgccagcgcgtcttctgcctccaggcgaggtgcgcgggccgccatccagtcggcgggatagaggaacaacggctgcgcttccacccatgcctgcgcgccgccgctatacagtaatcgttcgcgaacctgaaaacagcggcgcgtatgggcgtttattcgtagccagccgttaacgctgatcagcacagttaccgacgcgggataatccagcgccagctgcattcccaccagcgcaccgagcgcatggccgaccactgcgtaatgctcaatccctgcggctaccagcgcctgatgcagttccgctgccatctgggcgatactgtaatcttctgccagcgtgtcgggattattgccggtgccgcgctggtcgtaacagactacctgatactcctgctccagcaccgccagttgcggtaaccagtaactgccgctacccccaagacccgaaatcaacaccactacgggcgcatcagcataagggggaggtgagagtgaaagtttcatcgcggcctcacttggcgatatgcgcaattgtggcgatttccaccagcgcgtcaggttttaccagtccgcactgaatgcagaatcgcgccggtttatcacccggaaaaaactcggcgtagatttcgttaatcgcggcgtaatttttccagtcggtaataaagatgctgttgaaggtcacatccgccatcgtgccacccgccgtctcgatcaccttgcggatagtttccagaacgtggcgggtttgcgcctttgggtcatcggcaaacagcacgttattatgttgatcaaaagccagcgtaccggagacatacaccacgccatcagccagcgtgccgggaacgaagggggccagcggtgcgctgctgccagcgggaataattacggattttggcatcgttaaactccttaagcgatatgagcaaaggacgtgggagaaagcgcgtcgcagaatgtttcgacgtcgctgacccagccaaaaaaggtttcgatattgaacaacgcggctttctgcgcaaatttcggccccgcctggtgagttgcgtcttcaagcaccacgccgaaatactccagaaaaaagccgtcgcgtagcgtcgattcgacgcagacgttggtagcgatgccggtgaaaaccagatggcgtattccgcggctgcgcaaaatgctgtccagcggcgtattgaagaaaccgctgtagcgcggcttcggcagcacaatatcgccaggctgcggcaccagttcatccaccagttgataatcccaggagcctttcgccagcaatttcccctgcagctgcggctgcttacgcatggttttcagggcgttcgatttatgaaaattcggtgagccgggtccgccagcctcgacatactgttcatcccagccattttgaaaccagatgatcagcatccctgccgctcgcgctgcggtcacggcggtttgaatgttggcaatgaccgggcgagtggttgagacatcaaacccggcgagatctaagtagccgcctggcgtggcataagcgttttgcatatccaccacgatcagcgcactttgctgcggatcgaaggtaatggcttccggtcgagcggttaaggtcgtcatcatgccacctcctgagtcagcgcaggtagatgggcgcggcattgcatcagtggttgaatgcgctcgccgaaggtttcgattcccgacagaaaatcgtcgaaggttaacagcacgccttcggcaccaggcacgcttgcgacttcatctaacatgcgcgcgacactggcgtaagaaccgactaacgtccccatattgatgtttaccgccgaagtgggatcggccatctgacgaacgttggtgtcagtaccggagcgggtatctttctgactttgttcggttagccagcttaacgcctcttcatccgcgcccgctttgtagtgttcccatttggcgcgagcggcatcgtcggtttcatcggcaatcaccataaacaacacataagagccaacgtcgcgtccggtttgctctgcggcctgtttcatccgcgcagcggtcggggcgaaagccgtgggtgtatttacgcctttgccgaaacagaagttgaaatcggcataccgggcggagaacgccatgccagcgtcgctttgcccggcgcagatcactttcatggggacactcggttgcggactcacgcgacaatcattcatggtgaaaaaatcgcctttaaaatcgcttttccccgtgccccacaggtcgcgcagcacctgaacatattcggtgagatagtcgtaacgacgggagaaatagtcatcgccaggccagatacccatctgctcatactcgggcttttgccagccagtcacgaggttgacgccaaaacgcccgccagagatggagtcgatggttgcggccatacgggcgacgattgccggaggtaacgttaaggtggcagcagtggcgtaaatctgaatgcgcgaggtcacggccgccagccccgccatcaaggtgaacgactcaaggttgtgatcccagaactcagttttgccgccaaagccacgcagtttgatcatcgacagggcgaaatcgaaatggtagtgctccgctttttgcacaatggctttattcagttcaaaggtcggcatgtactgcggcgcgtgggtcgaaatgagccagccgttgttgccaataggtacgaatacgccaattttcatcatcaacctctcttcgtctcgtaaagtgaaagtcagacggggcgctgcatcctgcatatccttttcagccgcgtattggcttgtttgcaaagcggatgccagtttttaaaaagttaatgttattaatctgttaacattacgttatctaaaatatctggtaaaaagtggactaaacggtcaaaacagttgcacataaaacatgcatctgtgcgcgatgagagtgcagaaggtcgaggccgggcgggggttttgctatcctgttgccaatctacaagaggggagagcgcatgacgcaaggcgcagtgaaaacaacgggtaaacgttcgcgcgcagtaagcgcgaagaaaaaagcgattcttagcgcagcactggacactttttcacaattcggttttcacggcacaaggctggagcagatcgcagagttggcgggtgtttcaaaaaccaatctgctgtattactttccgtcaaaagaggcgctgtatattgccgtgctgcggcagattctcgatatctggctggcaccgttaaaagcgtttcgtgaagatttcgccccgctggcggcgatcaaagagtacatccgtctgaagctggaagtctcacgcgattatccgcaggcttcgcgcctgttctgtatggagatgctggcaggcgcgccgctgttaatggatgaactgacgggcgatttgaaggcattaattgatgagaaatcggcgctgattgccggttgggtcaaaagcggcaaactcgcgccgattgatccgcagcatttgatttttatgatttgggcttccactcaacattacgccgatttcgcccctcaggtggaggcggtgacaggcgcgacgttgcgcgatgaggtatttttcaatcaaacggttgaaaacgtgcagcggattattattgaggggattcgaccacgttaaagatgccggaggaggttgtaacatcctccggctacctgtttaacctatagtcattaagctggcgttaccgccagcggcagcggtattcacactcagcgaacgctcgatatacagccgttccagaaggatattgctttcgccacgggcaaaaccctgcaccgaaacaattgtgccatcccgcgcggcaactgcttcacacaatgcgcgaagctgatccgaatcaccgtggaagatcaccgcatcaaacggttgagcggttatattttccgctttcgccagttgaatacgttcgctgactgccgatggcaatgccttcactaactgacgatgcagcgcgtcatccggccacagtacctggctgcccaccgccagcacggcggcgagctgagtcagcgcatcctgctcatcatcggcaatacacaacacgcgctcacgcggcagcagcgtccaggtgttgcgttcacccgtcggccccggcagcaatcgttgtgttcctgcctgcgccagctcgccatattgcgtacataacgcctgcaattctggacgatttgctgcccattcccgcagtgcatttagcggctgagtcaatgcggctttcaactgcgcatcgaccggatactttgcatcctgacgcgcgagcgtcactgccagcgcactttccgggcgattcgccagcagacggtagagatagagcggaccgcctgctttcggcccggtaccggacaacccttcgccgccgaacggctgcacaccaaccactgcgcccaccatattacggttaacatacaggttaccaacatgggccgagccagtgacctgggcgatggtttcatcaatgcgcgtatggacgccaagcgtcagaccataaccggaagcgttaatctgctcgatcagctctggtagctggttacggttgtaacgcaccacatgcagcaccggaccaaagacctctttttgcaattcggcaaagtcatccagttcgatcagcgtcggggcgacaaaggtgccgctttgccattcacgggcatcttcgctgttttcccgcaccgcctggaacaccggacggcctttgctacgcatggtctgaatatggcgctcaatattggctttcgcttcgctatcaatcactggaccgatatcggtggtcaggcgacccggattacccatccggcattcggccattgcgccgcgcagcattttcaacgtgtggtcggcaatctcatcttgcaggcacagcacgcgcagcgccgaacaacgctgacccgcactgtcgaacgccgaggccagtacatccacgacgacctgttcggtcagtgctgaagaatcgacaatcatcgcgttcatgccgccggtttcagcgatgagcggaatagggcgaccctgagcgtccaggcggctggcgatattgcgctgcagtaacgtagcgacttcggttgaaccggtaaacatcaccccgcgcacgcgatcatcacccgtcagttgcgcgcccacggtttcaccccgacctggcagcaattgcaccacgcctggcggtacacccgcttccagcaaaatggcgatcccttgcgcggcaatcagcggcgtttgttctgccggttttgccagcacgctgttacctgccgccagtgcggcggcgatctgcccggtgaaaatagccagcgggaagttccacggactgatacacaccacaggccctaatggacggtgggtttcgttagcgaaatcatcccgcacctgtccggcgtagtagtggagaaaatcgaccgcttcgcgcacttcggcaatggcgttactgaaggtttttccggcctcacgcaccagaataccaatcagttgctgcatctggctttccatcagcacggcagcgcggtgcaaaatcgctgcgcgttcagccggaggcgtggcaaaccagattggcgcgttattaaccgcactttccagcgcctgttctacttcacgcggcgtggcttcacgcacatagcccacaatatctttcggttccgcagggttaataacgggcgacatctcacctgccgctaccggttgttccagcattggcaaggcctgccatttttgcagtgcactattgagcagggcagaggagagcgaggccaggcggtgttcgttagcgagatccagccctgccgagttgtcgcgcccgtgaccgtaaagatcgcgcggcaggggaattttcggatgcggtaatccagtttgcccttcctgttgcgccagtttttctacagcagtgaccggatcggcgaccagttcatccagtggcaaagaggtgtcggcaatacggttaacaaacgaggtgttagcaccgttttccagcaggcgacgcaccagatacgccaacagcgtttcatgtgtgccaaccggagcataaatacgacacggacggttaagtttgccgtcggcaactttcccggtgacctgctcatacagtggctcgcccataccatgcaggcactggaactcgtactgacccgggtagtagttctgccccgccagttgataaatcgccgccagcgtatgggcgttgtgcgtcgcgaactgcgggtagattagattcggcaccgccagcagctttttcgcacaggcgagataagaaacgtcggtatacaccttgcgggtataaaccggataaccttcaaggccgtccatctgcgcacgcttaatttcactatcccagtacgcgcctttcaccaggcgaatcatcagacggcgacggctgcgggtggcgagatcaatcaggtaatcgatcaccaacgggcagcgtttttgataagcctgaataacaaaaccgatgccgttccagcctgccagttccggctcgaaacagagtttttccagcagatcgagggagatctccaggcgatcggactcttcggcgtcaatgttgataccaatatcgtactgacgcgccagcagggtgagtgatttcagacgcgggtaaagctcttccattacccggtcatactgggcgcggctataacgcggatgcagcgccgacagtttgattgaaatgcccggcccttcatagatgccacgaccgttagacgctttaccgatggcgtgaatcgcctgctgataggaaaccatatacgcctgtgcatctgcggcggtcagcgcggcttcgcccagcatatcgtaagagtaacggaaacctttctcttccagcttgcgggcattggctaacgcttccgcgatggtttcgccagtgacgaactgctcacccatcaggcgcatcgccatatccacacctttgcggatcagcggttcaccgcttttaccgataatgcggttcagcgagcgggagaggctggcttcgttatgggtggaaaccagtttgccagtaaacagcagcccccaggtggcggcattaacaaacagtgacgggctacgaccaatgtgtgactgccagttaccgttgctgattttgtcgcgaattaacgcgtcgcgggtggctttgtcgggaatacgcaacaacgcttccgccagacacatcagcgccacgccttcctgcgatgacagcgaaaactcctgcaataacccctggaccatacctgcgcgaccactggcatttttttgattacgcagtttatcggccagctgatacgccagtttgtgcgcctgttcagcaactggctgcggcaggcgggcttgttccagcagcatagaaaccgcttcggtttccgggcggcgataggccgcggtgatcgcggcgcgggaaaccgactggggcaatatttgctcggcaaagtcgaggaatggctggtgtggttcctctgccggagtcggtgcttcatcgctctcattggccgcgccagaaagcagcgcaggtagctccggcagagtatcgctgttttccagttgttcgagataagaaaaaatcgcctgcttaattaaccagtgtggtgtgcgatcgatacgtgtcgcggcagacttaatacgctcacgcgtcgcgtcgtccagcttaacccccatggtggtggttcccatgccattactcctgttgttcagaaaggtgcaacttaacgttatcgtgaaatatccatgatgttgcaactttgtgcaaccatgttaaatgtgacatgcgtagcaagcttaaaaatgaatgaaatgttaataaaagaaatcgatatgacagggattaaaaaaataactcagactttttctctgcggcagttaacatttttgaaaggtgcaaccgcaaaaaatgtgagagagtgcaacctgatgaaaaatagtgtcgctgagcactaaaatttaatgtaaatggtgtgttaaatcgattgtgaataaccagcgcttccggcaggatacggtcgccctggtaaaacataaactctgttaccccgttccggtggcagatataacggcaagtttcgacattgccgataataattttttggagactttagatggctattagcacaccgatgttggtgacattttgtgtctatatctttggcatgatattgattgggtttatcgcctggcgatcaacgaaaaactttgacgactatattctgggcggtcgtagtcttgggccattcgtgacggcattatcggcgggtgcgtcggatatgagcggctggctgttaatggggttgccgggcgctgtttttctttccgggatttccgaaagctggatcgccattggcctgacattaggcgcgtggattaactggaagctggtggccgggcggttgcgtgtgcataccgaatacaacaataacgccttaacactgccggattatttcaccgggcgctttgaagataaaagccgcattttgcgcattatctctgcgctggttattttgctgttcttcaccatttattgcgcttcgggcattgtggcaggcgcgcgtctgtttgaaagtacctttggcatgagctacgaaacggctctgtgggcgggcgctgcggcgacgatcctttacacctttattggcggtttcctcgcggtgagctggactgacactgtacaggccagcctgatgatttttgccctgatcctgacgccggttatcgtcattatcagtgtcggtggctttggtgactcgctggaagtgatcaaacaaaagagcatcgaaaacgttgatatgctcaaaggtctgaactttgttgccattatctcactgatgggttgggggctgggttacttcgggcagccgcacattctggcgcgttttatggcggcggattctcaccacagcattgtccatgcgcgtcgtattagtatgacctggatgatcctctgcctggcaggggcggtggctgtcggcttctttgggattgcttactttaacgatcatccggcgttggctggtgcggtaaatcagaacgccgagcgtgtgtttatcgaactggcgcaaattctgtttaacccgtggattgccgggattctgctgtcggcaattctggcggcggtaatgtcaaccttaagttgccagctgctggtgtgctccagtgcgattaccgaagatttgtacaaagcgtttctgcgtaaacatgccagccagaaagagctggtgtgggtagggcgtgtgatggtgctggtggtggcgctggtggcgattgcgctggcggcaaacccggaaaaccgcgtgctgggcttagtgagctacgcgtgggcaggctttggcgcggcgtttggtccagtggtgctgttctcggtgatgtggtcacgcatgacgcgtaacggtgcgctggcggggatgatcatcggtgcgctgacggttatcgtctggaaacagttcggctggctgggactgtacgaaattattccgggctttatcttcggcagtattgggattgtagtgtttagtttgctgggtaaagcgccgtcagcggcgatgcaaaaacgctttgccgaggccgatgcgcactatcattcggctccgccgtcacggttgcaggaaagctaagggacttagcctgcggcggttttgtttggcttcagcagcgggttgcgctcccttaatgtgcctcgccatataaattgaatggtgcagggagcgcgcagggggcggccaatcgccgccgccccctgctgtcccggccttcggggaacgcttcagcgattttgacgccaccaacacccgagctgttattatgttccgggcaaaaagttagatttgataatcgcggatggacgaaattgcttgatacacccgcttatcagttttacatggaagctctgatgcattgagtctggacagttttgtcggctggatacggcgtttacgcggcatccggcaagaacacatggttctttgcaaacaatcccatctttctaccctggaataatcgtttatatcccttggcattacctctctttgtttacattccaacatcattttataaacattccgcttgtgtttttctttgccgtaatgataatcgctatcactgcgatttacttttctttgcatagattgactcagaaaaacgtttaagggtgggtggcatgtttgttccgtttctcattatgttgcgcgaaggacttgaagccgcgctgattgtcagtttgattgccagctatcttaagcgtacccagcgaggccgatggattgtgtgatgtggattggcgtgttgcttgccgctgcgttgtgcctgggcttgggtatcttcattaacgaaaccaccggcgaatttccgcaaaaagaacaggaactgtttgaaggtatcgtggcggtgatcgccgtggtgatccttacctggatggttttctggatgcgcaaagtgtcgcgcaacgtcaaagtgcaactggaacaggcagtcgatagcgcattgcagcgtggaaatcatcatggctgggcgctggtgatgatggtcttttttgccgttgcaagggaagggctggagtcggtctttttcctgctggcggcatttcaacaagatgtcgggatctggccgccgctgggtgcaatgctcggtcttgctactgccgtggtgctaggcttcctgctctactggggcggtattcgcctcaatcttggtgcattttttaaatggaccagcctgtttattctcttcgtcgccgcagggctggcagctggtgccattcgcgcatttcatgaagccggattgtggaaccactttcaggaaatcgccttcgatatgagtgcggtgctctcaactcactcgctgtttggcacgctgatggaagggatttttggctatcaggaagcgccgagcgtcagcgaagtcgccgtctggtttatttatctcatcccggcgctggtggcatttgctctgccaccacgcgcaggggcgacagcgtctcgctccgcgtaacaaatacgacgcaaactcttgcttagttacaacatactttaaagggatagtctcgtcatgaccattaacttccgccgtaacgcattgcagttgagcgtggctgcgctgttttcttctgcttttatggctaacgccgctgatgtgccgcaggtcaaagtgaccgtgacggataagcagtgcgaaccgatgaccattacggttaacgccgggaaaacacagttcattattcagaaccacagccagaaggcgctggagtgggagatcctcaaaggcgtgatggtggtggaagagcgggaaaatatcgcccctggctttagccagaaaatgacggcgaatttacagcctggcgaatacgatatgacctgcggtctgctgactaacccgaaagggaagttgatcgtcaaaggtgaggcaacggcggatgcggcgcaaagtgatgcgctgttaagtcttggtggtgcaattactgcatataaagcgtatgtcatggcggaaaccacgcagctggtgaccgacaccaaagcctttaccgacgcgattaaagcaggcgatatcgaaaaagcgaaagcactgtatgcaccgacgcgccagcactatgagcgtattgaaccgattgctgaactgttctccgatctggatggcagcattgacgcccgtgaagatgattacgagcaaaaagccgccgacccaaaattcactggtttccaccgtctggaaaaagcattgtttggcgacaacaccaccaaagggatggatcagtacgctgagcagctttataccgatgtggtcgatttgcaaaaacgcatcagtgaactggctttcccaccttcaaaagtggtcggcggcgcagccggactgattgaggaagtggcagccagcaaaattagcggtgaagaagatcgctacagccacaccgatctgtgggatttccaggctaacgttgaaggctcgcagaaaattgtcgatttgctgcgtccacaactgcaaaaagccaacccggaactgctggcaaaagtcgatgccaactttaaaaaggtcgataccattctggcgaaataccgtactaaagacggttttgaaacctacgacaaattgaccgatgccgaccggaatgcactgaaaggaccgattactgcgctggcggaagatctggcgcaacttcgcggtgtgctgggactggattaagcgttatgcagtataaagatgaaaacggcgtgaatgaaccgtcacgccgacgtttactgaaagtgataggtgcactggcgctggcgggaagttgtccggtcgctcatgcacaaaaaacgcaaagtgcgccgggtacgctttcaccggatgctcgcaatgagaaacagccgttttatggtgagcatcaggcagggatcctgacgccacaacaggccgcaatgatgctggtggcgtttgatgtgcttgccagcgataaagccgatcttgagcggttgtttcgcttgttgactcagcgttttgcttttctgactcagggcggagcagcaccagaaacgccaaatccgcgcctgccaccactcgattccggcattcttggcggctacattgcgcccgataatctcaccatcacgttatcggtgggtcactcattgtttgatgagcgctttggccttgcgccacagatgccaaaaaagctgcagaagatgacgcgtttccccaacgactcgctggatgcggcgttatgtcatggtgatgtgttgctacagatttgcgccaacacccaggacacggttatccatgcgctgcgcgatatcatcaaacacacgccggatttgctcagtgtgcgctggaagcgggaagggtttatttccgatcacgcggcgcgtagtaaaggcaaagagacgccgattaatttgctgggtttcaaagacggcactgccaatcccgatagccagaatgataagttgatgcaaaaagtggtgtgggtaacggcagatcagcaggagcctgcgtggacaatcggtggcagctatcaggcagtacgcttgattcagtttcgagtggaattttgggacagaacgccgctgaaagaacagcagacgatttttggccgtgataagcaaaccggtgcgccgctgggaatgcagcatgagcatgatgtgcctgattacgccagcgacccggaagggaaggtgatcgcgctggacagccatatccggctggcgaatccccgcacggcggagagtgagtccagcctgatgctgcgtcgtggctacagttattcactgggcgtcaccaactccgggcaactggatatggggttgctgtttgtctgctaccaacacgatctggaaaaaggcttcctgacagtacaaaaaaggctcaatggcgaagcgctggaggaatacgttaaacctatcggcggcggttatttttttgcgctgccgggggtgaaggacgcgaacgattatttcggaagcgcgttattgcgggtttaatgtttttaggcggataaggcatttgtgcgcagatgcctgatgcgacgcttgcgcgtcttatcatgcctacaatcagtgcgggtttggtaggctggataaggcgttcacgccgcatccggcgatcgtgcactgatgcctgatgcaaatcctgctgaaagcacacagcttttttcatcactgtcatcactctgtcatctttccagtagaaactaatgtcactgaaatggtgttttatagttaaatataagtaaatatattgttgcaataaatgcgagatctgttgtacttattaagtagcagcggaagttcccggcagtgatagtcagtcactatggagatcgcggatggtaacgtcctgtactggacatgttttagataatcaacgcgccaccactcgcggagttttctcctccggtagtcatctcgtcactttgcattttcaacctcatcctttcttttcatgtgttaccgacgccgtaaacggtgcgcgtagccgtttttcggcattttatccaaaagcaaactatggcttacaaggaagccaaccctctgatgttcgtgcgcataatcgcgctgccaacggcgcgtgtgatgaatacaaacaactcaaggtgctctccatgggaagacaaaaagcagtgatcaaagctcgtcgcgaggcaaaacgtgtgctgagacgggattcgcgcagccataagcagcgtgaagaagaatcggtcacctcgcttgtgcagatgggcggcgtagaagccattggtatggcccgcgacagtcgcgatacttcgcccatcctcgcgcgaaatgaagcgcaattgcactatctgaaggctattgagagtaagcagctgatattcgccacgggcgaagccgggtgcggaaaaacctggatcagcgcagcaaaagcggcagaggccctgatacataaggatgtcgacaggattatcgtcacccgtccagttctgcaagccgatgaagatcttggcttcttacctggagatatcgcagaaaagtttgctccctattttcgcccggtctacgacgtgctggtccggcgcttaggggcttcctttatgcagtactgcctgcgaccggaaatagggaaggtggaaattgcgccgttcgcctatatgcgtggacgtacctttgaaaatgcagtcgtcattcttgacgaggcgcagaatgtgactgccgcgcaaatgaaaatgtttttaacccgcctcggggagaacgtgacggttatcgtcaacggtgatatcacgcaatgcgatttgcctcgcggcgtgtgctccggattaagtgacgcgctggaacgtttcgaagaagatgaaatggttgggatcgtccggttcggtaaagaggactgcgtacgttcggcactttgccaacgtacgctgcatgcctacagttaagtgtgttatcggtgcagagcccgggcgaaccgggctttgttttgggtgtttatgcccggactagcgctttttctgaaacaaccatttttatttgcccctggctggtgaagtgtacgctcatcctgtggcttttttgtagttgctgatagagctcatcaggtattgctaagctctctgcatattcttgcggcgtatattggtaggctgcatgatgctgctgtttttgaaaacgcagcttattgtacagcgcccagacaattaacacgacggcattcgccactgccagcaaaaaatagaactgaagtcggcttctggcctcgctttgccagtaataacccgtcagcagatccatggcgaataagaatatgaacaacgcaaataatgtccacaagatggttgtggcaacataatcaaccagtaaacgtactggtgattgtcgggtcgtaataattaaattgttcatattaacctctcagaatcccgcgatcgggacttacccaacgggcgcgttgctttttaggcatcaacatgactcgtgtaaatgataccaatgtcgttgccaggctcagcatccagaaaataaccgggaaccaaataatccagaaaagcgatgaagtcagattatgctcatagcgattctcgatcatcaggctgacaataaattgcagtaaacataacgtacacaataatattccggcagtatgtgtcgcagcgatatgtgtcaattcaatatttaacggtacaccggcaagttggactgcgtaaataatgaaaccgaccaggcaggtgaaggcccatattgtcgtcaggcagtattcaaaaaacagcggccacattcgaaagttttctttgcgccacaaccttgtcatatttttgaggaatacttctgcaccgccctgagcccagcgcaggcgctgtttccacagcccttttaacgtttcaggcattaatatccagcacagtgcccgtggctcgtaaaaaatcgtccactgattcaactgcagcttccagctaatatcaatatcttcggtgatcatatcgtcactccagtaacccacttctgccagggcgctgcgacgaaatgcggcaataacaccggaaacggtaaatacgtttccatagatacgctgggttcgcttgatcaaaccaataattgaggaatactcgccaacctgaattttacccaccagggtagaacgtgttcgaatacgaggattaccggttacggcacccacacgcgggttgtacaacatcggttccacaatatatgccgccgcatcgcggtctaataacgcatcgccatcaatgcacaccagatattcacttttcgccgcggcagctccggttttaagcgcaatggctttcccctggttttgcgccagatgaatgacccgcaaatggggaatttgtgcagccatgcgatccaggatggcacgggttttatctgttgaaccgtcatttacggcaataacttcaatgttctcataacgctgtgctaaagcggcgtgtatggtttcctcaacgtttttctcctcattaaaacagggaatgataatggagatagacggattatctttcaactggggagctggtgcgttttctccccacggccagtggcgttcacgatagacccagaaatagacgccgccaacaatccacataatggacataaaaaacggccagaagaaaacgaacctcatcatcagttcaccagagtgaaagtacgctacgcataggggtatgcataacaccagacataatataaaaaacgatacgatgcgattaatcatttttcggataccaggctgttgaaaactcaggacgaataaggtctatttcaggttggttatgcagaaaattgtcgggataataaccatagtttttcactccattcagttgtaataggctcatccagtgagcgagttgttgcgaagaaatagcctgatgctgaccatttttctgccagttttgtgcctgtaattctaaaatagatttgtctttagcctgagggatgtttttaatttgattggtcaattgtattaaccattggtcagccgatttttctgcgacaccttccagataaggcatagccataatagcggtccagtcatagctttttaggaaatcagcataattctgtgcaaaccaggcttcactttcaggttgtattaccggaagtgcaaaaatatttcgtgcagttttaatatgtggaccgcgaatggcttttacgcgcgcactaagttctaaagtgaagtcagttaacgcacgacttttaaagcgggcccactgtttaaattgctccgggttttgtcgaatttcgctcagactcccgctaaagcctgcttgctgataagccgtgatagccggtgcactggcatcttcataatctgaaagcaaagcatcatcgtggaacaatatgccatcaaaagcagcatgtccggcaagatcttcatataacatgccaacttgtgctctgactctgtcatcgaaaggagagagacggtgatattgttcaggatgaatttgtgcttttttctcccctgttggtaagtattttactcgcgttaatgtgggatctaaatcccagcttaataccggcatccacgcatagatgtttacacctgagcgggtacgtaattgccaggcaacccgactaaaaatatctgctttcattggtagcaaacgatttggaaaccagacctctttgaccagcccatcaccatcgggatcagcaaatgcctgcaaatacacggttgatatttgcatatctttcacccgctgaattagcacatcaatattgcgatccatttgctggaggttttcgtcataaacgtaatcaagatcgatatgcattatccgttgtggtgatttttcctgtacggtaataatttgctgggcaaactcttttaatgagggattattggcgattaatacccgcggaatggaatccaattgcgacgcatttgccaaacctgattcaagggtgaagaacatgtcataaccgagtttttttaattcctctatcgctatgccattcgcttcgccataaggccaaacaaaaacgtgtggatttacctcaacctttgtacgcaggtattccgtcatttttacagcatccagacgaattctttcccggtattctgctgcggtttcataccgtgcgtggtcagtaaaatatgcacgatttacatatacaggcaataagctgccggtggcattagcctgaataccgtagtgagaattccatgtatgagaagcgagctcaacgagccgggaacgcgcaacttctcgcacttgttgccacgtggcaaaatattctcgatcgaccaactcatcgccaaattttacttgtttatccgctggcgtatcgacccaactgccgacgggggcccatacagcaggccactggaaggcctgaagaattgggaagacgcgggtataaaaactctggtagccgtcatcaaaagtcagcactacagctttttccggtagcggttttcctcctcgatgtgcttcacgaatttgagcaatactgaccggttgataaccgttctcgcgcagccaggcaaattgttcacgcagtgctgatgtccgcactgacataaaacgctggtcggcagcttcgtcttcaacgttatgccatgaaatcgctacaaaaccattatgcggccacggttgctcggcgagtaaagattcgcgatcctgtggcggtataaatgatgttcttgactggctaatgcacgcggtgagcataattatactcaccagcatcaggagatatttatttccattacgtaacatatttatccttaaaatctgaatgtcatatcgaattcaacgtataagttgtgttctctgtcaccgtcataaggtcgtttttcccagcgtagcgttgcgccagcatcaatcacgtcattccaactaatgcgttgcccgtagccgagttgggtgacgacatccgtgccataatgtttttgccaggaggcaccaacacctgcgctgaatatttgctcccagctattttcatagcttcgccataacaaatggcttgcctcaaatgccggaacaatatcgaacgtttttatagggttgtagtatggggtatcgtgttctgtattttgttcgtaatacagactgggtaggaaatcgacaatcaaatatggtgaagaccagatgcgttcctgaccctcaagtgagacttcatgacgctggttactgtcggaaaaatcagtgaaagcccaggagacaccgtacttacgccgctcattttgataccagcgaacataagcctgagcactgttgcctgtaacaccatttttcattgcccgtaatggaacgcggtgagagaggcgttccagttgcgaaccaatacgccagttatcattaaaatcataccagccagacaggcgcgcgccgggtttatgctcatgattgaaaacgcgttcagcgtactctgcctcgagccagatattacgtgaccgccactcaacacccgcaagccagtcgcgaacaatcccttttccttcgctaaattgtccatcggcataaccgaatccagcaaaaccgcgccagttatccttcagcggtggtgaataaacgatggtggttaagtcgacatcatgtttaccactatccgggccttcggcatcaattcctgttgagccagcgatacgaagctctgcaagattatgtacatcaaccgcacgttttaatcgtacaacgccgggatcttgcggttcacgttcgacaacatcgtgcgttaagacagctgcctgctgccattcttgtaacgttaatgctgtccaggcttgttcaacctccagattaatattacgtggctcgatcacttctgctttttttaattcattttctgctgcacgaggccaaccgcgggcttgtaacacactcgcgtaatcaatgcgcagtccctgatttcctggtgcgttataagcaagctctctggctgtcatttcagcctgaggaagatcattactatattttgctacggttgagagaaacgaatgcccctgtaaccaggtatcattcgggatgctcgtaggcgtgcccattaaccgaaggaaaggcggcgaagtattaatggtatgttgggtgacagttagcgcgcccggataattttcactctccaggtggctgtaaaagagatccgcaagttcttcatcggataaatccggggcaatggtctccttgtgataaaagagctcggtcattattgactgtgcttttttcggctgatgatctttgagataagccgatgcaacccaatattgcccccagggcggaataatttgccccgtcttttttaatcgctgatagtgagaaataacgtctttataacgatcgcgagttaataacgcgccaagatgatcaacctgaatacgctggtactgggcagtgcggtctgggttatcgtgccacagaatttctaatgcagcgtattgggcgagggcgcgatcggcaatggcataacgttcactttcactgcgcgtaggcataaacgacagtctgaccagttcggcatgaatatcagcgcgaatatctggcgttaaattggcatcgtcaatcgcggcagcaagttgattattacgtaatgcctgcacgtattctgtgggatattgttgcgtagatgcattttcaggtaatgactctgtcatcgcccgtaattcatcctgatgacgccccgccagtttatagatataggcttctgcgagtaaattggctttgtccggtgctccagagttaagctgcttaagtttaaccagcgcagtatcatagtgaccagcatctgccagggttaaaatttgtccccgttgataatccttattttgcggctccagagagagcgccttttgccacagtgtaagcgagttttgccattgttgcaggttacgataagcgacggcgacagctgcataaccacgcgctggtaattgctgatgacggtagcggttgtaaacggtaataacctgtttatcttgcccggcccataaggcaatctgtaaccagtcagcaatttggttattgctgagtgctgattttagtgcaaaccatgacaaagctggctgagtattacccttgcgagcttcaataatcaatgcatcataggcgttattaacagcactcttcgccgcgggactcgctgctaaaaatgcggcagtaagaagtttcaaagcccatttggttttcgggcacctttttctgctacttgaatacatcctgtattactccatgtattgccaaaatctctctctgtatctaattacaggtaactgaaaagaaagatatttttgcacctcataatccgttattaaacgcggaagagagacgtgaattgttgatgatgagaagaagaaatgatgagcagagtgtccatataaaatccttttctcgcccgaaaatccattccaatgatgaggatcttcaggaatacggcataaatcccaatgcctttttcaaaataaattaggattaaaataattaaatcagtaaattccgatgcatgatttcggatttttcgaaagtcctgatgaaaggctgcgctacggcactcacggatttaattgttattcctaatgtatctatgaattaatgttttataaggattttctataaccatttataagtattttcaagcctggcttgttgcaaacaatgtataaagcacttaggcaataataattacattcagcaactatcatcatcggtattgtttgtgggcggaatttcatattgacaacagtacagttcttatatctattaataatagaaagggatctacaacctacagattggtgtagctttatggaaaaagactatttgagaattagtagtactgtattagtgagcttattgtttgggcttgctttggttttggtgaatagttggtttaatcagccaggcgttgaggaagttgttccacgatcaacctatctgatggtaatgattgctttattttttatcgatactgttgcatttatttttatgcagttgtatttcatttatgaccgtaggcaattttcaaactgtgtacttagtttggcttttctgagttgtttgatttactttgttataaccgtcattatcattcagcaaattattgaggagcgtttgacaagcagtgttgtccaaaatgacattgcaatctattatttgtttcgtcagatgagtttgtgcatattaatatttctggcattggtgaataaagttagtgaaaacacaaaacagcgcaatttattttccaaaaaaatgactttgtgcataagtttgttttttgtttttggggggccgatagttgctcacatactttctagtcattatgagagctacaatttacacattgccgagttaaccaatgaaaatggtcaggtggtttggaaagcctcatatgttaccataatgattttcatgtggttaaccttgctttcggttaatctatactttaatggtttacgctatgatatctggaatggagtgacggtgattgctttttgtgccgtactgtacaatatctctctgttatttatgagcaggtatagcgtgtccacttggtatattagtcgcactattgaagtagtcagtaagttaaccgttatggtaatatttatgtgccatatattcagtgcgctacgagtaacaaagaacattgcacatcgcgatcccttaaccaatatatttaacagaaattatttttttaatgaactgacagttcaatcagcatcagcccaaaaaacgccttattgcgtcatgattatggatatcgaccacttcaaaaaagtcaacgacacctgggggcatccggttggcgatcaggtgataaaaacagtggtgaatatcattgggaaaagcatacgaccagatgaccttttagcgcgcgtcggcggcgaagagtttggcgtcttgctgacggacatcgatactgaacgtgcgaaagctttagcggaaaggattcgggaaaatgttgagcgtttaactggcgataatcctgaatacgctataccacaaaaagtgacgattagtattggcgctgttgtgactcaggaaaatgcgttaaacccaaatgagatctatcgactggctgataacgcactttacgaggcgaaagagaccgggcgtaataaggtggttgtgagggatgtggtgaatttttgtgagtcaccataaagcggcattttgatcctacccacgtaatatggacacaggcctaagcgaggttcttgttttcaaattgttccggactgaggccgccacaccaactgtgccgccgccaccgattgtaatcacattcgatataattaaacaccgttgcccgcattatttcccggctgataaagtgttctccatggatacattccactttcagcgaatgaaagaagctttccacgcaggcattatcgtagcagcaaccttttgcgctcatacttccacgcagattatgccgcttcagttgcgcctgataatctgctgaacagtactggcctccacggtccgtgtgaacgataacgttccggggcctcttacgccgccacagcgccatctgcagggcatcgcaggccagttgcgccgtcatgcgtggcgacattgaccagccaataacggcacgtgaccacaggtcaatgaccactgccagatacagccagccttcatctgtacgtaagtacgtgatgtctcctgcccacttctggttcgggccactggcgtaaaaatcctgctccaacagattttctgacacaggcaggccgtgtgcgcggtagctgaccgggctgaacttccgggaggcctttgccctcagtccctgacggcgcaggcttgccgccacggtttttacgttaaaggggtaaccctgagcacgcagttcatccgtcaggcgtggggcaccgtaacgctgttttgaccgggtaaaagccgcgaggacaacgctgtcgcagtgttggcggaactgctgacgcgtgcttatccttgtccgccgctgacaccacgtataccagccgctgcgggccacccggagcacgcggcacattgctttgatgctgaactcagcctgatgtttttcaataaagacatacttcatttcaggcgcttcgcgaagtatgtcgcggccttttggaggatagccagctcttcatcccgttctgccagctggcgtttgagacgtgcaatctcggtagacatctccagttcacgttcagaagacgtctgctgattttgctgtttactgcgccagttgtagagttgtgattcatacaggctgagttcacgggctgcggcagtaacaccgatgcgttcagcaagcttcagggcttcactgcgaaattcaggcgaatgctgtttacggggttttttactggttgatactgtttttgtcatgtgagtcacctctgactgagagtttactcacttagccgcgtgtccactattgctgggtaagatcagtgcctggcacacgcgtttgatggaagacggcgttcaggcaatgcgcgattatcttgccggactggatatcgcttcgccagagcatcaggttctgatgaacgtaacagcaaaaagcgaggtcgctccgtcaattatcaaagaaaatctctcattacacttaactcatacggtgaaatggactgaatctctcgatacatttctgaatatgccaaccccggtagctttccttgaaataagtaataagccctatttggggaatatgttaaatgattttgctggcgtggatcagcaacgagttatgcattgtcgtaaagcatttagtgatgcaaaggtattcaaatgattcctgattatttaacttttattcgctttcaggataaacgaaatctgatatacatttatgctattggacttattctgataggcttttattggaagaatgcagggtttacttttccatcagaggatattggtgtagttagtgggattctggctctggtgctgtataattttatttttgatctcaaggcgtactgggcttataaatgcgtcacgaagaatatcgatttttcgtggtttaagaaaaagcagaaccacaaaatagaattatttcttacacaacctctggtggcaggatttctgtcgttaatcatgttgagtgcaatgagttgggggctataccagcttctaccctcgttatatgcgctgttcctgatttcgttacttgggccgttggtcatctttctgctgtttcggatgatccgcaccagttatgtcaagcaggtcgctatttcagtagcgaaaaaagtaaaatataaaagtctgactcgctatgtgctgctttcggtgtgcatctcaacggttgttaacctgcttactatcagcccgttgcgtaacagtgattcttttgtgacagaggggcagtggttaacgtttaaatcgataattgcattgctcattctttgtggcgtagtgttggcgattaatctgttttttctgcgcttctccaagcggtacgcttttctgggcaggctttttttgcaggaaatcgatctgtttttctccagtgaaaatgcgttgtcgaccttttttgccaagccgctttggcttcggttattcatattgctggttattgaagtgatgtggattacgctggtgtcggtattggcaacgcttgtagaatggcggatttggtttgaagcctattttttactctgctatgtaccgtgcttaatttactattttttctattgtcgattcctctggcataacgattttatgatggcatgtgacatgtatttccgttgggggcattttaataagtgaggaagtgataggaagtgaccagataatacatatatgttctgtactctcttgcgcattttgattgttgactgagtaaccagacagttgatgtgcacgatttcccctcgccctaacagacgtgggcgggggcacccggtgtgtgcaatatacgaaaaaaaagcccgtactttcgtacgagctcttctttaaatatggcggtgagggggggattgactcgcttcgctcgccctgcgggcagcccgctcactgcgttcacggtctgtccaactggctgtcgccagttgtcgacccccggtcggggcttctcatccccccggtgtgtgcaatacacgaaaaaaaagcccgtactttcgtacgagctcttctttaaatatggcggtgagggggggattgactcgcttcgctcgccctgcgggcagcccgctcactgcgttcacggtctgtccaactggctgtcgccagttgtcgaaccccggtcggggcttctcatccccccggtgtgtgcaatatacgaaaaaaaagcccgtactttcgtacgagctcttctttaaatatggcggtgagggggggattgactcgcttcgctcgccctgcgggcagcccgctcactgcgttcacggtctgtccaactggctgtcgccagttgtcgaaccccggtcggggcttctcatccccccggtgtgtgcaatatacgaaaaaaaagcccgtactttcgtacgagctcttctttaaatatggcggtgagggggggattcgaacccccgatacgttgccgtatacacactttccaggcgtgctccttcagccactcggacacctcaccaaattgtcgttcctgtcttgctggaacgggcgctaatttagggaaatcatgacctgaggtcaacaaactttttgaaaaaatcgcgcgtttattcaaacttcaatcaatgtgtggttttaataagcgaaatctgctttttttgccaccgaccacggatttgttatgctggtggcctttgtagatcataacgataagtgcgaataaatttcgcacaacgcttttcgggagtcagtatggatatcatcttttatcacccaacgttcgatacccaatggtggattgaggcactgcgcaaagctattcctcaggcaagagtcagagcatggaaaagcggagataatgactctgctgattatgctttagtctggcatcctcctgttgaaatgctggcagggcgcgatcttaaagcggtgttcgcactcggggccggtgttgattctattttgagcaagctacaggcacaccctgaaatgctgaacccttctgttccactttttcgcctggaagataccggtatgggcgagcaaatgcaggaatatgctgtcagtcaggtgctgcattggtttcgacgttttgacgattatcgcatccagcaaaatagttcgcattggcaaccgctgcctgaatatcatcgggaagattttaccatcggcattttgggcgcaggcgtactgggcagtaaagttgctcagagtctgcaaacctggcgctttccgctgcgttgctggagtcgaacccgtaaatcgtggcctggcgtgcaaagctttgccggacgggaagaactgtctgcatttctgagccaatgtcgggtattgattaatttgttaccgaatacccctgaaaccgtcggcattattaatcaacaattactcgaaaaattaccggatggcgcgtatctcctcaacctggcgcgtggtgttcatgttgtggaagatgacctgctcgcggcgctggatagcggcaaagttaaaggcgcaatgttggatgtttttaatcgtgaacccttaccgcctgaaagtccgctctggcaacatccacgcgtgacgataacaccacatgtcgccgcgattacccgtcccgctgaagctgtggagtacatttctcgcaccattgcccagctcgaaaaaggggagagggtctgcgggcaagtcgaccgcgcacgcggctactaataaagcatcaggattcctgctatccttggcgggaattgaatacaggagagagttatgtatcccgtcgaccttcatatgcataccgttgccagcacacatgcatatagcacattaagtgattacattgcccaggccaaacaaaagggcattaaactttttgcgatcaccgatcatggcccggatatggaagatgcgccgcatcactggcacttcattaacatgcgtatctggccgcgagtggttgatggggtagggatcctgcgcggcatcgaagctaacattaaaaatgttgatggtgaaattgactgcagcggtaaaatgtttgactcgctggatctaattattgccggttttcatgagccggtttttgcgccacatgacaaagcgaccaatacacaagcgatgatcgccactatcgccagcggcaatgtgcatataataagccatcccggaaatcccaaatatgaaatagatgtgaaagccgttgctgaagcagccgcgaaacatcaggtggcgctggaaatcaataattcctcatttttacactcacgtaagggcagtgaagacaactgtcgtgaggtagccgcagcggtacgtgatgctggaggttgggtggcattaggctcggattctcacaccgcgtttaccatgggggaatttgaagagtgtcttaaaatcctcgacgcggtagattttccgccagagcgcattttgaatgtttctccgcgccgcttactgaacttccttgaatctcgcggtatggcaccgattgcggaatttgcagacctttaattactagtaatggaaatatattaatgaacgagttttctatcctctgtcgtgtgctgggttcgctctattaccgccaaccacaagatcctttactggtgccgctgtttaccctgattcgtgaggggaaactggctgcgaactggccactggagcaggatgagttgctgacacgtttgcagaaaagctgtgatatgacgcaagtctctgccgattacaatgcgttgtttatcggcgatgaatgtgctgtgccgccatatcgtagcgcatgggttgagggcgcgacggaagcggaagtgcgcgcttttctttctgagcgagggatgccattagcggatacgccagccgatcacatcggcacattgctgctcgcagcttcctggctggaagatcagtcaacggaagatgagagcgaagcactggaaacactgttcagtgagtatctgttaccctggtgtggtgcgttccttggcaaagtggaggcccatgcaaccacgcctttctggcgcaccatggcaccgctaacccgcgatgccattagtgcaatgtgggacgagctggaagaagattctgaagaataagtgtgatctacgtcactcataactgcaacggataatttgttgttgcataaaatgtgtgctcgatctcattcatggccgcgttttctgctatcatgcgcggcatgaacatacttctctctattgcaatcacaacaggcattctctccggtatctggggatgggtggctgtttccctgggcttactaagctgggcgggcttcctgggctgtacggcctactttgcctgcccgcaaggtgggctgaaagggctggcgatctccgctgcaaccctgcttagtggcgtggtgtgggcgatggtcattatttacggtagtgcactggcaccacatctggaaattctcggttatgtcataaccggtattgtcgcgtttctgatgtgtattcaggccaaacagctgctgctttcatttgttccggggacgtttataggcgcatgcgcgacgtttgccgggcagggtgactggaaactggtgttaccttcgctggcgcttgggctgatatttggttacgcaatgaaaaacagtggcctgtggctggcggcgcgtagtgcaaagacggcgcaccgtgagcaggaaatcaaaaataaagcgtgaggggcactcacgctttcgcttaaacagtaaaatgccggatgataattccggcttttttatctgtcaggattccggtggaaccgacatatggcggtatttcaccagaatgtcattctgccgttctgctttattttgcaaatcccacagaccacggtcgataccatcattaatcaggaaaatgacccctgtttcgatagccgacatcaggcacagcataacaggttcgttcgaggtgtaacccacttccccttcaagcaagcgctggtagtcaataaagcggaaaaccccggcctgaacttcataggaaagtatcgtcttactggtgttcaccgaagaaaggatctcgccggtactcacattgacgacgcgcaggttcacggcaatctgatcgagctggtattgcgtgtcggcaccgatgccaaaatatcttgccccaaccccgccagatttgacgttgctttcataaccgataatcgaaccttcaaccatgatatttgccgccgttaaagattgcagcgggattcggttattaatggcaaccgtgccgttttcttgtgccgcacgaataatcttgcgctcgttaagcaggttttgtaagccctggcgctccagcggtataaaccagcgagaatctttcagtgccgtgaccagcattgccgtggcgctttgcggaacagcagtggagaagttacttgccgggtagggtttaaattgcccggtttcgtcctgaatgttgtataccgaaacaaagattttacccgtcggcgctggcagatgggtcaaatctttgtagctctgagcacgaggcattaatgtcggtctggcggcttctttaggcggggcggttaagcatccgctcagtaacatgacggcaaccaaaagaaataagcgctgcatgattattttccttatgaagctggggcttaaaaatcggttgagttattttgtaaacccgaaacctggatggtcgaggtttgtccggttttacgatctgtcacgttcaactgcaattgaccatcgcggttggcaatatcgacaatataatcgttggtcaccatgcggcccggtttaccggtattaatattcgacagtagcccacctaaaatttgtgactggatggcctgagtaaagttatctaacgctgagggtgtttcaataccaaagtcatcgttatagctcggatctttataagagttttgggcctgagcgctatttaataaaaaagcgccattatttgggttaccaccaaagtttggattacggaactggaaagtcatggttccagcccaacttaatggcgaaataagcatgagtagaactactgcatgtttgacacgcattgcagcctccgaacaattttttatttagaattcatcatgcgccaaatcgcccgtacttaataacgcctgatttatctggcgacgatttagtgcttcttcagtttgaatcagtgcaaagacgacagttttctcgaagtctcttttcaacggaaataaaaaagtctggaaaataacgtcctgattgaccgttatagtgatccagcttccccatcgtgcactgggcctttcattaatcgttaagttacccgtatagtcactttcccatttatcactaaaggctcggtaaaaatcatggccaatagatgaaacagtatggtcagttagcaatcccgggacttctacctcaacggcgtgaagattccctgcggcgaacagaaattctgccgccacaatccagcgtaaataacgtttcatggctttatcgcctgaggttatcgtttgcccaggaaaccgcttgtgtccggttttttacggctatcttcttgaaaagattataaagatgcgttttaaccgtattttcgctgatgaacaacgaacgagcgatctcgttattagacgcgccgatacgcagcttattcaggatctctttttcccgatgagtaaggagggctgattccgtgctgttataacgatagttacctgaatgcgtaatcaggtagctggcaagcttttgcgtaaagtagcattcgccgcgcaggacgccttgcaacccattgacaacacgttcttgatcctccatggaataaaaaacgccgttgatatgaggccagttttcaatgtcgcggtacgggtaatcttcaggcgtatttagcaacaatattttgatattgttgtttttcctgctcaaagtatcctgccaataatggataagctttttatccgcttccatcatatccagaagaataatagagcctgaagagatatcgtccagagaacgttgaatattatgtaattttcctgtaattgccagcgattgtttaaggtgctgcaagagagctgtcgcctgcaaagaagatttagtgatcaacaataatgtatgaccatgaatactatggacttcattaaacatgatgaaaccccgctttttttattgatcgcacacctgacagctgcctctaaaatagaagcaccagaagtactgacagatgttgcactgctgtgtgtagtaataaatcagccctaaatgggtaaaatataaaactaatggattacatctgatttcaatctagccattacaaatcttaaatcaagtgttaaacatgtaactaaatgtaactcgttatattaaaatgttaaccttaaggttttattaagtttagaaatgatagaaaagttgtacatttggtttttattgcacaattttaaaaaatcatacaaatggtgataacttactaataatgcatataaaaaatatttcggtgtagtcctttcgtcatgtaaaacgttcttgttttttctccacacctccgtggacaattttttactgcaaaaagacgaggtttgtcacggcttgtgcgcaagacatatcgcagcaatcagcgacgggcaagaagaatgactgtctggtgctttttgatagcggaaaacggagatttaaaagaaaacaaaatatttttttgcgtagataacagcgtatttacgtgggttttaatactttggtatgaactaaaaaagaaaaatacaacgcgcgggtgagttattaaaaatatttccgcagacatactttccatcgtaacgcagcgttaacaaaatacaggttgcgttaacaaccaagttgaaatgatttaatttcttaaatgtacgaccaggtccagggtgacaacatgaaaaacaaattgttatttatgatgttaacaatactgggtgcgcctgggattgcagccgcagcaggttatgatttagctaattcagaatataacttcgcggtaaatgaattgagtaagtcttcatttaatcaggcagccataattggtcaagctgggactaataatagtgctcagttacggcagggaggctcaaaacttttggcggttgttgcgcaagaaggtagtagcaaccgggcaaagattgaccagacaggagattataaccttgcatatattgatcaggcgggcagtgccaacgatgccagtatttcgcaaggtgcttatggtaatactgcgatgattatccagaaaggttctggtaataaagcaaatattacacagtatggtactcaaaaaacggcaattgtagtgcagagacagtcgcaaatggctattcgcgtgacacaacgttaatttccattcgacttttaaatcaatccgatgggggttttacatgaaacttttaaaagtagcagcaattgcagcaatcgtattctccggtagcgctctggcaggtgttgttcctcagtacggcggcggcggtaaccacggtggtggcggtaataatagcggcccaaattctgagctgaacatttaccagtacggtggcggtaactctgcacttgctctgcaaactgatgcccgtaactctgacttgactattacccagcatggcggcggtaatggtgcagatgttggtcagggctcagatgacagctcaatcgatctgacccaacgtggcttcggtaacagcgctactcttgatcagtggaacggcaaaaattctgaaatgacggttaaacagttcggtggtggcaacggtgctgcagttgaccagactgcatctaactcctccgtcaacgtgactcaggttggctttggtaacaacgcgaccgctcatcagtactaatacatcatttgtattacagaaacagggcgcaagccctgttttttttcgggagaagaatatgaatacgttattactccttgcggcactttccagtcagataacctttaatacgacccagcaaggggatgtgtataccattattcctgaagtcactcttactcaatcttgtctgtgcagagtacaaatattgtccctgcgcgaaggcagttcagggcaaagtcagacgaagcaagaaaagaccctttcattgcctgctaatcaacccattgctttgacgaagttgagtttaaatatttccccggacgatcgggtgaaaatagttgttactgtttctgatggacagtcacttcatttatcacaacaatggccgccctcttcagaaaagtcttaatttgttgaaatatcgagcataagatgaatctggagagaatggtctgctgcgaatcagccaacctgaaagtatggataacacaaccctcaaggatgactaatcattgaggaaatagaataaatgttcagaccttttttaaactctcttatgctcggcagtttgttttttccttttattgccattgctggaagcaccgtgcaagggggcgtgatccatttttatggccaaattgtggaaccggcatgtgacgtcagcacccagtcatcacccgtagaaatgaactgcccacagaatggttctattccgggcaaaacctactccagcaaagcgttaatgagcggcaatgtcaaaaacgcgcaaatagcctcagtaaaagtgcagtatcttgataaacagaaaaagctggctgtaatgaacatcgaatataactaagtttctgaacaactcacgttgctgagcagaaaaatgcgatttaaccaaaaagcctgctgtacacttaagaaacaagaaggtgtaaggaggcgttatgaaaacgcgtattcatgttgtgcagggtgatattaccaaactggccgttgatgtgattgtgaatgcggctaatccgtcattaatgggaggcggcggcgtcgatggggccattcatcgcgcagcgggtccggccctgctggatgcttgtttaaaagtcaggcaacagcagggcgattgccctacggggcatgccgttattacgcttgcaggcgatcttcccgctaaagccgtagtgcacaccgtcgggccagtctggcgtggtggtgaacaaaacgaagaccagcttttgcaggatgcctatctcaatagcctacgactggtggcggcaaacagctatacgtcagtggcttttcctgcaatcagtactggggtttatggttaccctcgtgcggcagcggctgaaatcgcagtaaaaaccgtttcagaatttattacccgtcacgctttacccgaacaggtatactttgtctgttatgatgaagaaaacgcccacctctacgaaagactccttacccaacaaggagatgaatgatttgccccggctggcgagcgcggtgctgccactgtgttcgcaacatcccggtcagtgtggcctttttcctctggagaaaagtctggatgcgtttgccgcccggtatcgtctggccgaaatggcagagcatacgctcgatgttcagtattacatctggcaggacgatatgtcgggtcggttactgttttccgccctgttagccgcagcaaagcgtggcgttcgcgtccgtttgttgctggacgacaacaatacgcccggacttgacgacattttacgcttgcttgacagtcatccacgcattgaagtccggctttttaatcctttctcgtttcgcttgctgcgtccgcttggttatatcaccgacttttcccgtcttaatcgccgtatgcacaataaaagtttcactgtcgatggcgtggtgaccctggtgggaggacgaaatattggtgatgcctattttggagcaggggaggagccacttttttcggatttagatgtcatggcaataggacccgtggtagaggacgttgccgatgatttcgcccgctactggtattgcaaatcggtttcacccttacagcaggtgctggatgtcccggagggtgaaatggcggatcgcatcgagttacccgcctcctggcataacgatgccatgacgcatcgttatttacgcaaaatggaatccagtccatttataaatcatctggttgatggaacattgccgcttatctgggcgaagacacgtttattaagtgatgatccggcgaaaggggagggcaaggcaaaacggcattcactgttaccgcagcgcctgttcgatatcatgggctcacccagtgaacgcatcgatattatctcttcctattttgtaccgacacgcgcaggtgtggcgcaactcttacggatggtgagaaaaggggtaaagattgcgatcctaaccaattctcttgccgctaacgatgttgctgtcgtccatgccggatacgcgcgctggcgcaaaaaattgctccgctatggcgtggaattatatgaactcaagccgacgcgtgaacaaagtagtacgttacacgatcgcggcataaccggtaattccggagccagcctgcatgctaaaacctttagcatcgatggtaaaacggtgtttatcggctctttcaatttcgatccgcgttcaacattgctcaatactgaaatgggcttcgtgatagagagcgaaacgctggcacagttaattgataaacgctttattcagagccagtatgatgcggcctggcagctccgtctggacaggtggggacggatcaactgggttgatcgtcatgcaaagaaagagattattctcaaaaaagaacccgccaccagtttctggaagcgggttatggtcagactggcgtcgatattgcccgtggaatggttattgtaaatgtggcttaacgggctggtgctttatcgttctcacgcttaacaaccggtttaccagagaacaaaaacttcagtaacgggatgcgcaaatgaatttcatacagaattatcgcaatccctactacaaatatcaggccacagagaaaaccaagccagttggaggtgatgtgcggtgtaatgtatgcgccgaaaaacagcgttaacgggtggtgaaccagatagataaacagcgatgcgttaacaaaataagtcacccgcgctgactggaagttaagcaaacggtggccaaaggagaagaccacattcaccatccacagaccgaggaccatggtgatcaccgactcggtttcgtacatccaggcatcgccactgccatagcgctggttgagtaaataagcgacaaacgccaatgctgctgcaagggtacagccacgagacggcgtggtaaacaaggctttaagatgagggaaaatgaaagccagtgcgccgaggataaagaacggcaaataaaacagcgtttgcatgacaataaaattgaacatgccattactcagaatgggcggatacacaataaaaatcgttcttcttattaccgcataaccgatgccgaggcataaaaaaatcaccgatagttttaccatcgagaattttttattcgttttatcagaattttctaaattatttctgatgcgcttaaatatccatacgcacagcgtcgtcatgaccactaacaccagtaaaaaccacaggtgtgatattaattcccaggccaacgtattatatttgtcatacaatgacagcccaggccaactttccgcttttcctttgacatattgcagcataataaattgcggtaatgtcagtagggggatggctgttaacatcgggatacctacacgttcgacacgtactttccaccattttttcaagggatagcgtaaaaaaagcatgtaggaaaagtagccggatataacgaaaaatacctgcatgcggaacgagtggatgaagtcattaaaaagggtcagccacaatgatgattcggcgctattcacatgccatgtatggctcgaatagattaaagaaatatgaaaaggtatccctaacaacatcagccaggcgcggatggagtcgaggaaatattcacgttgcgcgggtactgggttcatatatggttaactaatctcggatttttcgtcttatccctgtcgggttatgcctttaggcttgttgccatagtgacaccgacctgaccgcgccaggcgcaggcttcaaggtttttatgcatagcatcatcgctaccactaaccagaatggaagcgtctgtaagacggttgataaataaatttgctggcaaaccctacacgaagtcgatgcttctgtctttaggagaagcacggaaagtgaaaacggttgcaatcaggtgcttaatccatgagccagcgtgctgaacgataccgggattctgttgtcggaatggctggttatccattaaaatagatcggatcgatataagcacacaaagggggaagtgcttactaattatgaaacataaactacaaatgatgaaaatgcgttggttgagtgctgcagtaatgttaaccctgtatacatcttcaagctgggctttcagtattgatgatgtcgcaaagcaagctcaatctttagccgggaaaggctacgagacgcccaaaagcaacttgccctccgttttccgcgatatgaaatacgcggactatcagcagatccagtttaatcatgacaaagcgtactggaacaatctgaagaccccattcaaactcgagttctaccatcagggtatgtacttcgataccccggtcaaaataaatgaagtgactgccaccgcagtcaaacgaatcaaatacagcccggattatttcactttcggcgatgttcagcatgacaaagatacggtaaaagaccttggctttgccggttttaaagtgctttacccgatcaacagcaaagataaaaacgatgaaatcgtcagcatgctcggggccagctatttccgcgtgattggtgcaggtcaggtttatggcctttctgcccgcggcctggcaattgataccgccttgccatcgggtgaagaatttccgcgcttcaaagagttctggatcgagcgtccaaaaccgactgataaacgtttaaccatctatgcattgcttgactcgccgcgtgcgacaggtgcttacaaattcgtggttatgccagggcgtgacacggttgtggatgtgcagtcgaaaatctatctgcgcgataaagtcggcaaactgggggttgcaccgttaaccagtatgttcctgtttgggccgaaccaaccgtcgcctgcaaataactatcgtccggagttgcacgactctaacggtctctctatccatgccggtaatggcgaatggatctggcgtccgttgaataacccgaaacatttagcggtcagcagcttctccatggaaaacccgcaaggctttggtctgttgcagcgcggtcgtgatttctcccgctttgaagatctcgatgatcgttacgatctccgtccaagcgcatgggtgactccgaaaggggagtggggtaaaggcagcgttgagctggtggaaattccaaccaacgatgaaaccaacgataacatcgtcgcttactggacgccggatcagctgccggagccgggtaaagagatgaactttaaatacaccatcaccttcagccgtgatgaagacaaactgcatgcgccagataacgcatgggtgcaacaaacgcgtcgttcaacgggggatgtgaagcagtcgaacctgattcgccagcctgacggtactatcgcctttgtggtcgattttaccggcgcagagatgaaaaaactgccagaggataccccggtcacagcgcaaaccagcattggtgataatggtgagatagttgaaagcacggtgcgctataacccggttaccaaaggctggcgtctggtgatgcgtgtgaaagtgaaagatgccaagaaaaccactgaaatgcgtgctgcgctggtgaatgccgatcagacgttgagtgaaacctggagctaccagttacctgccaatgaataagacaactgagtacattgacgcaatgcccatcgccgcaagcgagaaagcggcattgccgaagactgatatccgcgccgttcatcaggcgctggatgccgaacaccgcacctgggcgcgggaggatgattccccgcaaggctcggtaaaggcgcgtctggaacaagcctggccagattcacttgctgatggacagttaattaaagacgacgaagggcgcgatcagctgaaggcgatgccagaagcaaaacgctcctcgatgtttcccgacccgtggcgtaccaacccggtaggccgtttctgggatcgcctgcgtggacgcgatgtcacgccgcgctatctggctcgtttgaccaaagaagagcaggagagcgagcaaaagtggcgtaccgtcggtaccatccgccgttacattctgttgatcctgacgctcgcgcaaactgtcgtcgcgacctggtatatgaagaccattcttccttatcagggttgggcgctgattaatcctatggatatggttggtcaggatttgtgggtttcctttatgcagcttctgccttatatgctgcaaaccggtatcctgatcctctttgcggtactgttctgttgggtgtccgccggattctggacggcgttaatgggcttcctgcaactgcttattggtcgcgataaatacagtatatctgcgtcaacagttggcgatgaaccattaaacccggagcatcgcacggcgttgatcatgcctatctgtaacgaagacgtgaaccgtgtttttgctggcctgcgtgcaacgtgggaatcagtaaaagccaccgggaatgccaaacactttgatgtctacattcttagtgacagttataacccggatatctgcgtcgcagagcaaaaagcctggatggagcttatcgctgaagtcggtggcgaaggtcagattttctatcgccgccgccgtcgccgcgtgaagcgtaaaagcggtaatatcgatgacttctgccgtcgctggggcagccagtacagctacatggtggtgctggatgctgactcggtaatgaccggtgattgtttgtgcgggctggtgcgcctgatggaagccaacccgaacgccgggatcattcagtcgtcgccgaaagcgtccggtatggatacgctgtatgcgcgctgtcagcagttcgcgacccgcgtgtatgggccactgtttacagccggtttgcacttctggcaacttggcgagtcgcactactggggacataacgcgattatccgcgtgaaaccgtttatcgagcactgcgcactggctccgctgccgggcgaaggttcctttgccggttcaatcctgtcacatgacttcgtggaagcggcgttgatgcgccgtgcaggttggggggtctggattgcttacgatctcccgggttcttatgaagaattgccgcctaacttgcttgatgagctaaaacgtgaccgccgatggtgccacggtaacctgatgaacttccgtctgttcctggtgaagggtatgcacccggttcaccgtgcggtgttcctgacgggcgtgatgtcttatctctccgctccgctgtggtttatgttcctcgcgctctctactgcattgcaggtagtgcatgcgttgaccgaaccgcaatacttcctgcaaccacggcagttgttcccagtgtggccgcagtggcgtcctgagctggcgattgcactttttgcttcgaccatggtgctgttgttcctgccgaagttattgagcattttgcttatctggtgcaaaggaacgaaagaatacggcggcttctggcgcgttacattatcgttgctgctggaagtgcttttttccgtgctgctggctccggtacgcatgctgttccatacggtcttcgttgtcagcgcgttccttggctgggaagtggtgtggaattcaccgcagcgtgatgatgactccacttcctggggtgaagcgttcaaacgccacggctcacagctgctgttagggttagtgtgggctgttgggatggcgtggctggatctgcgtttcctgttctggctggcaccgattgtcttctcgttgatcctgtcaccgtttgtttcggtgatttccagccgtgccaccgttggtctgcgcaccaaacgctggaaactgttcctgatcccggaagagtattcgccgccgcaggtgctggttgataccgatcggttccttgagatgaatcgtcaacgctcccttgatgatggctttatgcacgcagtgtttaacccgtcatttaacgctctggcaaccgcaatggcgaccgcgcgtcaccgcgccagtaaggtgctggaaatcgcccgtgaccgccacgttgaacaggcgctgaacgagacgccagagaagctgaatcgcgatcgtcgcctggtgctgctaagcgatccggtgacgatggcccgtctgcatttccgtgtctggaattccccggagagatattcttcatgggtgagttattacgaagggataaagctcaatccactggcattgcgtaaaccggatgcggcttcgcaataaaaacgtagttgcctgatgcgctacgcttatcaggcctacatcgttcctgcaatttattgattttgcaagactttgtgggtcggataaggcgttcacgccgcatccggcaaaaacaacgagccaataaaaataccggcgttatgccggtatttttttacgaaagaggtatcaaatgcgtttaattgtggtgagcatcatggtgaccttgctgagtggctgtggcagcattattagtcgcactataccggggcaggggcatggcaaccaatattatcccggtgtgcaatgggatgtgcgtgactccgcctggcgttatgtcacgatccttgatctgccattctctctggtttttgatactttactgctgccgatcgacattcatcatggcccgtatgagtgattaacgttcatcccactcatcagctgctgcgcgtccttcctcggtatccagcggtggctcaagctgaaattccccctcgtcccattcatgtaatgtattctcttcctgccactcctggcgtatctctatctcatcatagtcgccatcaaaaacactttgcgcggcttcaccgctaagcataggtaaacattcaccttcttccccttcgtcggcaaaaaactcaacttgccacatgatgtcgccgtcctgcaaaacgtatttttgggcattgaactgttgcacattcgcatcttcggcgtcgatgccggggttgtctgcaagaaattcttcgcgtgcagcgtcaatggcttcttcaagcgttgcgtacatggtcatcacgattctccctttgagttgatgaggtttcagggaaaaggatagctgattctccgcttttgcaagtatgaaaggcgaaaaatcagttcgatacctggggtattcgacgacgacgtagactgttccatgaatagactgcgttgaataacactacgccagcggtgacgagaaataccgctctgaaaccgtagttcgctgaaatcgctgctcccatcaatggtccggtaacgttgccaatatcacgaaacgattggttatagctgaagatacgcccggcgatctggttgctcgagttgtaaaccaacagtgtctgtacggcggggagtagtgcaccatcggcggcaccgagcaaaaaacgtaaaatcccaagttgcaatggcgtctgaacgtaagacattgggatcaacagcagtacagaaaagatcagcgctgtaatcaggatcttttcgggtccgattcgatcgccaagtttgccgagtcgtggtgcacttagcagagccgccacgcctggcaccgaggcgatcatgccactgataaaggcgacgttactgacgttacccgccagttcgcggacatacagcgtcagaatgggggcaattgagcccgtcgccacctggatgattaacgtagtgacaaacaggctgagtaccagtttcgggtttttaagtgatgtcaccacttcccgcatgtgcagcatctcttttttgctgaccggctggaatttttctctgatgcaaaacagggtgacgaaaaagcagagtatgagcacactggcggtaataaagaataccggacgtaagccgtagctatcggcgagcaggccgccagccattgggccgagcaacgcaccactaacgccgcctgtggagagcgtacccagcgcccagccgcttttattacgcggtacttgtgtggcgataagagcattagcgttggggacaaatccgccaagtaacccaagaagcgcccgcaggatcaaaaactgccagatattttgtgccagccccatcaacaccatcacgatgcccatgccgagggcagagcgtaatagcatgagttttcggcctttacggtcggcgagtccaccccaaaacggtgaggcgatggccgaaaataaaaatgtaatgctgaagacaataccggaccacatattcagggcggagtgaccggtaacgccaagctgctcaacgtagaggggtaagaagggcattaccagactgaaggcggcaccggtaagaaaacagcctagccaggcgacgatcaggtttcgtttccagtttataggggtgtcattttcacagggtgacatagcaatccgctgttggtgcgccaggcgcggtgaacataagaagaaaagataagcacactaattatgcgcccgacttccagggggcgcaatccagagagcttttatcgctaaatcagggggatttgctgtggtaatgccggatgccattctgaagcatccggcatgggagatttaatagcgtgaaggaacgccttccgggcgtgttttaaagcgacggtgtaaccacatatactgctctggtgccatcatgatgcatttttcgaccactttgttcatccacgcggcggtagtttcggcatcatccagtggcggagaacactctggcggcagcataatcaattgataccctttgccatctggcttacggcgtggaacgaagggcaccagacatgcgccggacatccgtgccagcatccaggttccggtcgtggtcgcagcctgctcaacggcaaacaacgggacgaaaacgcttgagcgcgggccgtaatcatgatccggtgcgtaccagaccacttcgccttttttcagggctttaatcatgccttttaaatctttgcggtcgagcatcgatttatttgagcgcaaacggccccaggtttgtagccagtcaatcagtggattatcgttcgggcgataaacgccaatacccggttcctgcataccaaactgccgcgcacccagctccagtgtcagaaaatggatgccaactaacaggatgccgcgtttttgcgcctgcacgtcacgaatgtgttccatgccgatcacttccgtccagcgggcgattcggcggtccggccagaaccacgccatgccggtttccatcaggcccatgccaacggattcgaaattcttcaccaccattttacggcgttcttgttcgctcatttccgggaagcacagttccaggttgcgatgcacaatttttgcgcgtcgtttcataaaacgtaacgccagttttcctaatccacaaccgaggcggtagataaccgggtagggcaattgcacgactaaccaaagtacgccaatacccaaccaggttaaccaataacgcggatgaagcagtgcggtggagaacttgggtagattcgtcatatcaatcctgtttttcaacctattcgggcaattgtatgtattgtcgcattttttcgcccgcaaccaaaatttgtggctgaagactgggcgaaattgccgcgcttgtaaataacaaataatttttaatgcgcaaatgtagcgtaaaatgtgtggatgttaattatcgataattgctatatcatgccgcggatttttactttcccatctcgcaggaaccgtacaccatgccagtgttacacaaccgcatttccaacgacgcgctaaaagccaaaatgttggctgagagcgaaccgcgaaccaccatttcgttttacaagtatttccacatcgccgatcctaaggcgacccgtgacgctttatatcagctgtttaccgcgctgaatgtttttgggcgagtgtatctggcgcatgagggcattaacgcgcaaatcagcgtacctgcgagcaatgttgaaacatttcgcgcgcagctctatgccttcgacccggctttagagggtttacgcctgaatatcgcgttggatgatgacgggaaatccttctgggtactgcgcatgaaggtacgcgatcgcattgttgccgacggtattgacgatcctcactttgatgccagcaatgttggtgagtatctgcaagcggcggaagtgaacgccatgcttgacgatcccgatgcactatttatcgacatgcgtaaccactatgagtatgaagtggggcactttgaaaacgcgctcgaaattccggcagataccttccgtgagcagctgccaaaagcagtcgagatgatgcaggcacataaagataaaaaaatcgtcatgtactgcaccggcggcattcgttgtgaaaaggccagtgcctggatgaaacataacggattcaacaaagtctggcatatcgagggcggaattattgaatacgcccgtaaggcgcgcgagcagggcttgccggtgcgttttattggcaaaaattttgtttttgacgagcggatgggcgaacgtatatcggatgagattatcgcgcattgccaccagtgcggcgcgccgtgcgacagccataccaactgtaaaaatgatggctgccacctgctgtttattcagtgtccagtatgcgcggaaaaatacaaaggttgttgtagtgagatttgctgcgaagaaagcgcgttaccgccagaagaacagcgacgccgtcgggcaggacgtgaaaatggcaataagatctttaataagtctcgtggacgtctgaatacaacactgtgcattcctgatccaacagaataaatatcattgccggatgcgtgccatccggcaacatttcacgcttacttctgctgtacgccttccactgaaataatcagatccacttcctgagaagctggacctaaatctgtcttgatattgaagtccttgagcttaattttgccttcggcctcgaagcctgcacgtttaccaccccatgggtcgtcgccctgaccaattaatttcgcttccagcgtgacgggtttggttacgccattcagcgtcagatcgccggtaatatccagttcgtcaccgtctttcttcacgctggtggaggtgaatgttgcctgtggatattttgcggtattgaggaaatctgcactgcgaagatgtttatcgcgttcggcgtgattagtatcgacgctggtggtgttaattgtcacattcactttatcggcagccggatttttttcgtcaaaggtaaaagtaccgtcgaaatctttaaaggtgccgtataaccagctatagccaaggtgctggatgcggaaattaacaaaggcgtgctgaccttctttgtcaattttgtaatcggcggcaaccgctgaaccggcagagaacatcagggacgcgaaggttaaaccaagcaggctttttttcattttttatactccatagtcagatgacgactttcccagcatgcgcttcagagtgtcgtctttatcgatgaaatgatgcttcagggccataaatccgtgcataacggacagtactacgacgctccacgcgagccaaaaatgcagggcaccggcaaagtctgcctgtgcgccagcgtcggcaagggtcgcggggacgtcaaaccagccaaaaacgctgatcggtttaccatcggcagttgagatcagatagccgctgatgccgatggcgaaaagcaataggtacaatgcgagatgtccagctcttgcggcaagacgagtcatgggcgaataactcggcagcggacccggcggtggagatatgacacgccacagaacgcgaataaccagccccatcattaacaaaataccgatgcttttatgcagttcgggtgctttgtgataccagccatcgtaataactgagcgtgaccatccacagacctaaagcaaacatgccgtagacaataattgcgcttagccaatggaaggccgcagatataacaccatagcgttcaggggtatttgtgaatgacataagtgcatccaaaacgaatttgcgagagaaagaaaatggcgtgtcggagaatgaattgcaacacaaaaataacaaattgaatgatatttatttttatttcaataattttgaattaataatgaaagaatcttcataagtttagtgggttcagcatcagagatgtctggtgagtgctgtagaagcaggaataatctcattcaatttttcacgctaaatgaaagggagattaaatatttgtcagtttatgtcagtgcggaaaactaaaaataaaacacatagatcagatccataattgccaacaatccccagagaaaaagataaagcatcagatgctcgcgaatattattgatgagatagtgcaacagccgacgcattaaatactcctgtaaaaacggcctcattctggaggccgtaatgatgattattggaagcgggaaagcctgaatggcgtcaaatcaaaatcgctttttttgtcttgcgcaaaatcggcagctatttcccctaaaactgacgcaaatttaaaaccgtgcccactcaggccggtaatgagcagtgtattatcgtggccgggtagggtatcgataataaaatcttcgtcaggcgaattatcataggtgcaggcagcgccgtacaggcagcaaccgatacccggcaatacattgcgcaagaacgggaaggcttctgacccatcactggccacttccgcaaacggaacacgttcatccgctgaatggataacctggcctccgttatgtttgccaatcttcaacgcgtcgttttctgccggaaaaccataatattgatcgccattgggcagttcaccggtaaacgccgggaatttattcttcacgctatagcggccatcggcctgataccaggcaaatactttgcgtacgggctggacaggcagctccgggagcaggtcttttacccatgttcccgcgcagacaatcgcttttttcgcctgatactcaccgtcagccgtttcaatagttacgccatcatcgtcatgacgaattgcggtgaccgggcagttgaacagttgcgcacagcccgcttccttcgccagttggatccaggttttaatcgccagttcgctgcgcaaaaaaccggaatcagtttcaaataagccgatgtagttgtccgggacgcgtatttccggccagcgggccataatcccttgcgcatcgagcttttcaacgttgagttgccattgttcggcgctgtgggcgacgttggcgagaaatgtggaatcagccgggccaaggttaatgacgccagagcgtacaaaaatgggatcttcttcgttgtggcgggagagttcatcccacagcgtttgcgcgcggaggaccagcgggacatacttttcgccttcaccataagcatggcgaattaatcgcgtatcgccgtggtggctgccgtgttgatgcggtggcatatgggcgtcggtcattagcacgtttaaaccggcgcgggttgcataatacccggcggcagcgcctacggaaccgctgccaataatgatgagatcgtatttcatttttttctctctgctctcatggtttaagcagagtaattaactgaatgcagatatacaacccagaaatggtaaaggcaccggtgaggtgccttttgggtggatggtcatgtcatgttaatgacgccgatactcgtttacctggaaatcaccggattcaattttggcgattcctgcttctaatatcgaaataaattgtctggcaacatcagtggttaaccagagcgtctgaccaacttcagtcccttcctgctcggacttatttggggtctggtagtgcaaacgcaacatcagcgcatcatagctatcaacggtgctgatgtcccaccctacgagcggatgagtctgaatgacttcattatttttttccatcatggccccctaattcgtgttactagacaacgttattcgaggttcaatgcgtttttatctgaagcaacttcagtataccaataagtaagggtattcaccgaatttttaaagggggaaacagataaatttctgcttttaagatttatatgaacaataaaacagcatgtcattcatatttttttagcatattgtgcaattattttgaggaagtgtagaaattttgtactcaaaattcgtaagtaaaataaaaaagccggggcgacccggcaaaaaaaatcactgcatattattcgctgacaaaccagtcatcggcgctttcccacgtttcctggagaatttcactaatgcgctgtttatcttcttttgtcgcgccaataaccgataaattattcgctgcggcataacgtaccgatacgtggccttcattatcaggaaacgcatactgaatacggcgggaaagttcgccagccagggcgtcaatagccccagctggcaatggagaagttttcgctatggtgacttcaattcgcataatagccccctgttgaatatactggttatttatacaggtaaaataacctaatgacaacaggaagctacgatttttattgtttaacggaccagcgtaccgtttccccggcgaggaatggcaccagcgtgtcatcagtcagtgcgatgctttcagcaacctgttgctcttcacgtaccagttcgatgaatgtgtcgttgaccggcaacccatagaactgcgggccgtttacagaacagaatgcttcaaagtgctgcaaagcattcatttcttcaaagacggtagcgtaactgcccagcgcggttggggcgttgaagcagcccgcgcagccgcaactgctctctttgcgatgacgtgcatgtggcgcagaatccgtaccgaggaatactcgattaaaaccgctggcgaccagttcacgcaatgcctgttggtgaatattacgtttgaggatgggtagacaatacaggtgcggacgcacgcctccaaccagcatatggttgcggttaaacatcagatgctgcggagtgatggtggcagccagccgttcatttccgtcacggacatagtcggcagcatctttggtggtgatgtgctcaaaaacgactttcagcgcagtcaggcgctggcgcagaggttccatcacgctttctataaagcgcgcttcacgatcaaaaatgtcgatatctgcatgtgtcacttcaccatgcaccagtagcggcataccgattttttccatgcgctcaagtaccggcatgattgcgtcaattgacgtcacgccgtggctggagttagtggttgcgtttgccgggtaaagttttgcagcggtgaacacgccttcgttaaatccgcgctccagctcattaggatccagcgaatctgttaaataacaggtcatcaatggggtgaaatcgtgcccggcaggtacggcgtcaagaatacgctggcgatacgccacggcagcctcaacggtggtcacgggcggagccagattgggcattacgatagcccgtccataaatttcgctggtatatggcacgacagtttttaacatgtcgccatcgcggaggtgaaggtgccagtcgtctgggcggcggatctttaatacctgggatggtgcagtcattaatctctatgctccggctgaagggatgtttttgccggacacaaaggataagcggaaacgttttcctttgcacgaaaaataaagggcgcgaatgcgccctcgtgattaatcagtaaatggaatgacaatttcgcctggcttcacttcaatgcctttcgccagttttttcgccattgcttcgccctggctgccatcttcgcgcaggacgtaagcaggttgctggttaaagtaattgcgtaatgcctggttcaaatagggaagcaacgtttgcatcaccgtttgcattttttccggttgtaccgtcgcatcgaccacttccatctctttcaggaagatcgcacctttttctttatcaaacacgggcagcgctttcagcttcagtttcatggtcgctttctgactaccgaacagggagttcatgtccagattggcgtctccggttagggtaaccttattcggctcttcgcgaccaatttggctggtcaggtttgtcagaacaatatgggcgtcagccacgccgggtaaaccgatatcttttgagaaattattatgtttcgcaagcgactggttaatttcttgttcggtgatggtgtattgggtgagttgattacagccaacgagcaggccactgacgatcaatgcagcggcaaataaaaacttgttcatggtagtcctcgacatgaaatctgcgtcaatatcctgacacaacgcagcatgtgtcaccagcgataaactcgccagcagaaaaaactgaaaacggcggcaacccgcgaatacaggctgccgcggcgggtcaggattaaatcgccattgatgataacaaattgatttgtgtctgtttcgccatattatcgcggtaatcagcaacgcggcttggccagttaattccggctaccagcgtcagattacgcagtagcgggaatagctgaatatcatcttccgaaagttcgccattcacggcgttcggtttgacgatcagtttgtccagcgcacgtaaatcatcgctgatattcttaatcagaccgtcagagtgggccagcaggtcggcaaaattacccgcgctggcctctttcttgtcgacgaaatatttgcgcgcggcgggagtagaaaactcatcaaatgccgatttggcaaaacgcggcaacagcagtttgttggcgtagccattgaccttgcgcagccactcttcaatggcaggggaacgtttgccggtcagtaacggtttgccgtcgagtttatcgacatagtgaacgatgtccatgctttctggcatatagcggctgtcatctttttgcagaatgggaacctgtttttgaccgaccatccgggtgggtgtttctgcgtcgtcgttgagcagaacatgtaattcgacggggatatttttcaggccgaaaatcatgcgggctttgaggcagtaagggcagtgatcgtaaatgtatagcttcacgtgactcctccatttggctgtcagttcactttcagtatgaaggagtcaggggggagtatcaaatcaggcgtcgcgttcaagcaaacgacgcgcggcgcgtttctggctaaactgccaacccagcgcaaggaaagtgaagatgccaataatgcccagcatcatccacggaagctctggctggtgcgccgatttgcccaggtcaaacagccagccgccaccgatataaccaatagcgccgccaatcgccagacccagacggctaaaccccatatagctgccgcgagctcttgcgtccgccagcgaagcacttaaggtttcacgcgcaggctcggcaatgatcgacccgatataaaacagacaaatcagggtgaaaagttgttgcaggccgctgaccatgcccaccggcatcatgcttaatgacattatcaacagcccagccatcaaccggtgttccagacgaaaatgcttttcactccagcgggcgatagggtagagcaacgttaacgacagacacgcttcaatggcatacatccatttaacggcagagggcgcgccagccacgtcgttgaccataattggcagcatcagcatcacttgtacagccagcatgtagtaacccgccagcgtcagaacataggtgacaaaacgcttgtcacgcatcacgcgggtcatgccttcgcgaacgggcgtgcgtacggtggagagtttccatgctggtaacaaccacgcattgaacgccgcacatagcacaaatagaactgcccctgtggcgcagaccaggcgaaagtcgtattgcaacagccagctccccaacaatgcgccaatgaccgcaccggcactgtcctgcatcatcaacagcgagaaaaaacgaccacgctgctgtggacggattaatttcaccaccagcgccgaacgcggcggatcaaacaacgtgccaccgagtcccgagagcaggcatgaaaaccacaatagccacggttcgtgggcgatacccattgtggcgaatccggcggcgcgcatcagcataccggtaacaatcatcggtttggcaccaaagcggtcggcaattgcaccgccgaaaatacccagaccttgctgaataaattggcgtagaccgagagcaataccgaccatgacggcggcccagcccatttgatcaacgaagcggatagagatcagcgggaagacaacaaagaaccccagcacgaccagcatattatcgatgagcaggaaatatttacccaggttcctcgcctgcgacacgcgggacatttcccctcccgggaaataaaagatgagcactttctattctgcattgccgctaagacttttcccatcacttcggggacaatatttttttatcaaaacgtcgctttgatagagagtttttatcaaatatgtgaataatgcagaaaatggcattttggacttttcacagggtctggttgcgcaggtatagtaatacttacagcgtattaaagacgttacgggaaggagtaggtatagaatgtttggctatcgcagtaacgtgccaaaagtgcgcttaaccacagaccgactggtcgtgcgtctggtgcatgatcgtgatgcctggcgtcttgcggattattacgcagagaatcgccatttcctcaagccctgggagccagtgcgcgacgaaagccactgttatccatcaggctggcaggccaggctggggatgattaacgaatttcataaacaaggttcagctttctactttggcttattcgacccggacgaaaaagagattattggcgttgccaatttttccaatgttgttcgtggctcttttcatgcctgctatctcggttattcgattgggcaaaaatggcagggcaaaggactcatgtttgaagccctgaccgcagccattcgttatatgcagcgcacccaacatattcatcgcattatggctaattatatgccgcacaataaacgcagcggtgatttactggcgcgactgggttttgaaaaagaaggctatgcgaaagactatctgttgattgatggacaatggcgcgatcacgtactgacggcattaactaccccagactggacgcccggccgctaaggagaatctcatgaaatatcaacttactgcccttgaagctcgcgtgattggttgcttgctggaaaagcaggtgaccacgccggagcaatacccgctctcagtcaatggtgtagtcacggcctgtaatcagaaaacgaaccgtgaaccggtcatgaatctgagtgaatccgaagtgcaggaacagctggataatctggtcaaacgtcattatctacgcacagtgagcggttttggtaatcgggtcaccaaatatgagcaacgtttttgtaattcagaatttggcgatctgaaactgagcgcagcggaagtggcgttaatcaccacgttgttattgcgtggtgcccagacgccaggtgaactgcgcagccgcgccgcgcgaatgtatgaattcagcgatatggcggaagtggagtcgacgctggaacaactggcaaatcgcgaagatggtccttttgtggtgcgtctggcccgcgaaccgggtaaacgcgaaaaccgctacatgcatcttttcagtggtgaggttgaagatcagccggcggtgacggatatgtcgaacgcggttgacggtgatttacaggcccgcgtcgaagccctggaaatcgaagtggcagaactgaaacagcgtcttgattcgttgctggcccatctgggagattaaagtgaaaaaattacgtatcggcgtagtgggattaggtggcattgcgcaaaaagcgtggttaccggtgctggcggcagcgtctgactggacgttacaaggagcctggtcgcctacgcgcgcgaaagccctgccaatttgtgaaagctggcgcattccttatgccgattcgttatccagccttgccgccagttgcgatgcggtttttgtgcattccagcaccgccagccactttgacgtggtcagtacgttactcaatgcgggggtacatgtctgtgtcgataaaccgctggcagaaaatctgcgcgatgctgaacggctggtggaactggcggcgcggaaaaaactgacgttgatggtcggttttaaccgtcgtttcgcaccactctacggtgagttaaaaacgcaactcgccaccgcagcctcgctaagaatggataaacatcgtagcaatagcgtcgggccacacgatctttatttcacgttgctggatgattatctgcatgtggtggataccgcgctgtggttgtcgggcggcaaagcctctctggatggcggtacgctactgactaacgacgctggcgaaatgctgtttgccgagcaccatttttcggctggtcctttgcagatcaccacctgtatgcatcgccgtgccggaagtcagcgtgaaaccgtgcaggccgtgactgacggtgcgctcatcgacattacggatatgcgcgaatggcgtgaggagcgcgggcagggcgtagtgcataaaccgattcctggttggcagagtacgcttgagcaacgtgggtttgtcggctgtgcgcggcacttcattgaatgtgtgcaaaaccagacagttccgcaaaccgccggcgaacaggccgtgctggcgcaacgtatcgttgacaagatctggcgcgatgcgatgagtgaataaaccctgtaacatctggcggtagcaattcaccataatccaggtagactattcgcctctttcagcgcctgccttgcaggcgttttgcccgtgggtctggattagaacaccgatgaatttattaaaatcgctggccgccgtcagctcgatgaccatgttttcgcgtgtgcttggcttcgcacgagacgcaattgtcgccagaatctttggcgcagggatggcaaccgacgcctttttcgtcgcttttaaacttcctaacttgttacgccgtatctttgccgaaggggcattttcccaggcatttgtaccgattctggcggaatataaaagtaagcagggtgaagacgccacgcgggtctttgtctcttatgtttctggcctgctgacacttgcgctggcggttgtgacggtcgctggcatgctcgccgcaccgtgggtgatcatggtgaccgcgccaggcttcgctgacacagctgacaaatttgccctgaccagccagctactaaagattacctttccctatatcttgctgatctccctggcgtcgctggtgggagcgattctgaatacgtggaaccgcttctcgattccggcgtttgctccaacactgcttaacatcagcatgattggtttcgcgctgtttgccgcaccgtactttaacccaccggtgctggcgctggcgtgggctgttacggtcggcggcgtcctgcagctggtgtatcagctaccgcacctgaagaagatcggcatgctggtcctgccgcgcattaacttccacgatgccggagcaatgcgcgtggtgaaacagatgggaccggcgatccttggcgtctctgtgagccagatctccttaatcatcaacaccatttttgcctcgtttcttgcttccggttcggtgtcttggatgtattacgccgaccgcttaatggagtttccgtccggtgtgctgggcgtggcgcttggcaccattttgctgccgtcgctgtcgaaaagttttgccagtggcaatcatgatgaatacaaccgtttgatggactgggggttgcgtctttgtttcctgttggcgctgccgagtgcggttgcgttgggcattctttccggtccgttgaccgtttcgctgttccagtacggtaaatttaccgcgtttgatgcgctgatgacccagcgggcgttaattgcctactcggtgggtttgattggcctgattgtagtgaaagtgttggctcctggcttttattcccgccaggacattaaaacgccagtgaaaattgccatcgttacgctgattttaacgcaattgatgaacctggcgtttattggtccgttgaaacatgccgggctgtcactttctattggtctggcggcgtgtctgaatgcttcgctgctttactggcagttgcgtaagcagaaaatctttaccccgcaacccggctggatggcgtttctgttgcgtctggtggtggcggtactggtgatgtctggcgtgcttttaggtatgttacatatcatgccggagtggtcattgggtaccatgccctggcgtttactgcgtttaatggcggtcgtgctggcggggattgccgcgtacttcgctgcactggcggtactgggcttcaaagttaaagaatttgcccgccggacggtgtaacaatgcattccggcctgcagtgcaggccggagataatcttcagatcgaaatctttttaccgccgcgatgggttgttgaggtctgaccgttcgccccatatagcgtcggttcctgatgcggtttcaacatttccagcgcctgttgattgcgctcaatctgtccttccagtaaccagccgttatgttgattcatttggcgtagttgctgcgttttcacagtaatttcctgccagcgttgactaatatcaacgctatttgctgtattgggttctttcctgcgtaactgttcgaggtaatccagcgtcgccagcagtgagcttttttgttctgtaatccattgcaactggctgccgttgatctgccccatagagagatgttgctgctcttgatccattaccgttttgagatcgttaagcacagcggacatctggtcgaggatctctgcaagacgtgtcatacgatcagttactctgcaagtcttgctgcgcttcgttgatcagcgcatcggcaattttgccggtgtccatttttagttcaccgttacgaatcgccagttttaacgcttcgacacgttcaagattgatatcactgctgccgggttgcatcagttttgcttgcgcgtcgcttaacgtcacactggtgctggtggaggcggttgtttttgccgcccggctgttcgttaccggcgcgtcagtggtttcgcgcggttgaacggtgcttacaggcttcagaggcgaagtgcgatcaatactcatggtttattcctcattgagggcgcttttatcatgtgttgcttatttatcggcaagggacgggtaatctttaacagcttacaggtttataagaatattcccatctgcatcaacaacgccgctgactacctgtcccgataccatgcgcacccgcgcattctgtgcgacggctgcattgttcagcgcctgaccttctgcgttggcgctaaacccatcaccgctggcgatcacattgacgcgttgtcccgcttttacccgccatgcctggcgaaactgggttaactggataggttgatcgggtgatagatcgcgcaggctaatggcatcaacaagttgattgatatccagcaccgtacgcggtggcagggtatccagccgtccgcgtttcagtttgacattgccagcttccagctttcctccccgcgcaatgggcatcgcggcaaccacataatttcctgtggcctgtacattaacctgtaaatatcgtttgtcgttaccgcagcgtgccaacacattcacattgccccacaggcgggaattattgctcatcgaaagcaatggctgctcgcatggcggtagtagattgggcgctgtacgaatagaaacacgaacctcatcacttacccccgcgagttgggcgctaaaaaagttgtgcaattgcgatgtgagattgctcgccgtacttaacggactgaacagtatcgcgatgatcgccacgctacgttttattatcagcattttcgcccccagccatttctacaacgtgaattgtacctgtccgcaatgaccatcaacggcataaatagcgacccattttgcgtttattccgccgataacgcgcgcgtaaaggcatttaagctgatggcagaattttgatacctgcggaggagatatgctcgataagctcgacgccgccttacgttttcaacaagaggcgctcaatctgcgcgcccagcgtcaggaagtgctggcagcaaacatcgccaatgccgatacccctggttatcaggcgcgcgatatcgattttgccagtgaacttaaaaaagtcatgcaacgtggacgggatgcaaccagtgtggttgcactgacgatgacctcaacgcaacacattccggcgcaggcgctgacgcctcctaccgcagaactgcaataccgtattccggaccagccttcgcttgacggtaataccgtcgatatggatcgcgaacgcacccagtttgccgataacagcctgcaataccagatgagccttagcgcgttgagcgggcaaatcaaaggcatgatgaacgttttacagagcggaaattaacggatggcactgctgaatatttttgatatcgccgggtcggcgttaactgcccagtcccagcgcctgaacgtggcggccagtaatctggcgaatgctgatagcgtgaccggtcccgatggacagccatatcgggcaaaacaggtggtattccaggttaacgctgcaccaggtgctgcgacaggcggcgtaaaggttgccgatgttatagaaagtcaggccccggacaaactggtttatgaaccgggtaatccgctggcagatgcaaagggctacgtaaaaatgccgaacgttgatgttgtcggagagatggttaacaccatgtcggcgtcacgcagctatcaggccaatgttgaagtgctcaacacggtgaaaagcatgatgctgaaaacccttacgctcggtcaataaaggagaaagctatgtccattgcggtaaccaccaccgatccgacaaataccggcgtcagtaccaccagcagtagttcgctcacgggcagcaacgccgcagatttacaaagcagttttctgactttgctggtggcgcagctgaaaaaccaggacccgaccaatccaatggaaaacaacgagctgacgtcgcaattggcacaaatcagcacggtcagcgggattgaaaaactcaataccacgctcggatctatttccggacagattgataacagccagtcgttacaggccagtaacctgatcggtcacggcgtgatgatccccggcaccactgttcttgcgggaaccggcagtgaagaaggggctgtgaccacgaccacgccgtttggtgttgagctgcaacaggcggcagacaaagttacggccaccatcaccgataaaaatggcgcggttgtgcgcaccattgatattggtgaactgaccgccggagttcacagtttcacctgggacggtacgttgactgatggcagcactgcgccgaacggttcttacaatgtagcgattagcgccagtaacggtggtacacaactggttgcccagccgctgcagtttgctctggtgcagggtgtgatccgcggcaacagcggtaatacgctggatctcggcacttacggcaccaccaccctcgacgaagtacggcagataatttaagccttcacatttcaggagtcagtcatggccttttctcaagcggttagcggattaaacgctgccgccaccaacctcgatgttattggcaacaatatcgccaactccgccacctacggctttaaatcaggcacggcctcttttgccgatatgtttgccggttcgaaagtgggactgggggtaaaagttgccggtatcactcaggactttaccgatggcacgaccaccaacaccgggcgaggtctggacgttgctatcagccagaacggttttttccgtctggtagacagcaacggttcggtgttctacagccgtaacggacaatttaagctggatgaaaaccgtaacctggtgaatatgcaaggtttacagctgacgggttacccggcaaccggtacgccgccgactattcagcaaggggcgaatccgaccaatatttcgatcccgaataccctgatggcagcgaaaactaccaccacggcatcgatgcagatcaacctgaattccagtgatccgcttcctactgttacgccattcagcgccagcaatgcggatagctataacaaaaaaggttcggtgactgttttcgacagtcagggtaatgctcatgacatgagcgtctactttgtgaagaccggggataataactggcaggtctacacccaggatagcagtgatccaaacagcattgcgaagacagcgacaacactggaatttaatgctaatggcacattagtggatggtgcgatggcgaataatatcgcaaccggcgcaattaacggtgcagaacccgccacgtttagtctgagcttcctcaactccatgcagcaaaataccggcgctaacaatattgtggcaaccacccagaacggctacaaaccgggcgatctggtgagttatcaaatcaatgatgacggtacggttgtcggcaactattccaacgaacaaacccaactgctggggcagattgtactggcgaactttgccaacaacgaaggtctggcatccgaaggcgacaacgtctggtctgcgacgcaatcttctggcgtggcgctgttggggacagccgggacgggaaactttggcaccctgaccaacggtgcgctggaagcgtccaacgtcgatctcagtaaagaactggtcaatatgatcgttgcccagcgtaactatcagtctaacgcccagaccatcaaaacccaggaccagatcctcaacacgctggttaacttacgctaatcgctgacgggatagctcaatggatcacgcaatttataccgcgatgggagcagccagccagacactgaatcaacaggcggtaaccgccagtaatctggccaatgcctcaacgcccggttttcgcgcgcagttgaatgctttacgcgcggtgccagtggaagggctttctctgcccacgcgcacgttggtcacggcgtcaacgccgggcgcagatatgacgcccggcaaaatggattacacctcgcgcccgctggacgtcgcgttgcagcaggatggctggctggccgtgcagaccgctgacggcagcgaagggtatacgcgtaatggcagcattcaggttgatcccaccgggcaactgacaattcaggggcatccggtgataggcgaggctgggccaattgctgtgccggaaggggcggaaatcactattgctgccgatggcacaatctcggcgctcaatccgggcgatccggcaaatacggttgcgccagtagggcgtcttaaactggtgaaagccacgggcagcgaagtgcagcgcggtgacgacggcatttttcgtttaagcgcagaaacccaggccacgcgtgggccggtactgcaggcagatccaaccttgcgtgtgatgtcgggggttctggaaggcagtaacgtcaatgccgttgcggcaatgagcgacatgattgccagcgcgcggcgttttgaaatgcagatgaaggtgatcagcagcgtcgatgataacgcaggccgtgccaaccaactgctgtcgatgagttaattgaaaggatacatgacaagtataagttgcccgatgcgcaagtttatcgggtctatgggggcaatcgcaatttatcgattttgcgagcacttgtaggccggataaggcgtttacgccgcatccggcaagaagacatatgcactttgtcactaatccactacaggacattttatgatcagttcattatggatcgccaaaacgggccttgacgcccagcaaaccaatatggacgtcattgccaacaacctggcaaacgtcagtactaacggttttaagcgtcagcgcgcggtgtttgaagatctgctttatcaaaccattcgccagccgggggcacagtcttccgaacaaaccaccttaccctccggattacaaatcggcacgggggtacgcccggtcgccactgaacgcttacacagccagggaaacctgtcgcagaccaacaacagcaaagatgtcgcgattaaagggcagggctttttccaggtgatgttgccagatggttcatcagcctatacccgtgacggctctttccaggtggatcagaacgggcagctggtgacggctggtggttttcaggtgcagccagcgatcaccattccggcgaatgcgttaagtatcaccatcggtcgtgatggcgtggtcagcgtaacccaacaaggccaggcagctccggttcaggttgggcagctcaatctcaccacctttatgaatgacaccgggctggagagcattggcgaaaacctctacaccgaaacgcaatcctctggtgcaccgaacgaaagcacgccgggcctgaacggcgcgggactgctgtatcaagggtatgttgaaacgtctaacgtcaacgtggcggaagaactggtcaatatgattcaggtgcaacgcgcttacgaaatcaacagtaaagcggtgtccaccaccgatcagatgctgcaaaaactgacgcaactctaaggcttaaccggtggcaggttcaccggtttactgatttttgaagatgatagccatgcaaaaaaacgctgcgcatacttatgccatttccagcttgttggtgctttcactaaccggctgcgcctggataccctccacgccgctggtgcagggggcgaccagtgcacaaccggttcccggtccgacgcccgtcgccaacggttctattttccagtctgctcagccgattaactatggctatcaaccgctgtttgaagatcgtcgaccacgcaatattggcgatacgctgaccatcgtgttgcaggagaacgtcagcgccagcaaaagctcctctgcgaatgccagccgtgacggtaaaactaattttggctttgatactgtgccgcgctatttgcaggggctgtttggtaacgctcgtgccgatgtcgaagcctccggtggtaacacgttcaacggaaagggcggggccaatgccagcaatacctttagcggcacgttgacggtgacggttgaccaggtactggtcaacggcaacctgcatgtggtgggtgaaaaacagattgccattaatcagggtaccgaatttattcgcttctctggcgtggttaatccacgcactatcagcggcagcaataccgtaccgtctactcaggtggcggatgcgcgcattgaatacgtaggcaatggctacattaacgaagcgcaaaatatgggctggttgcagcgtttcttccttaacctgtcgccaatgtaagtgaggctgtggtgattaaatttctctctgcattaattcttctactggtcacgacggcggctcaggctgagcgtattcgcgatctcaccagtgttcagggggtaaggcaaaactcactgattggctatggtctggtggtggggctggatggcaccggtgaccagacaacccagacgccgtttaccacacaaacgcttaataacatgctctcacagctgggaattaccgttccgacgggcaccaatatgcagctaaaaaacgtcgctgcggtaatggtgacagcgtcacttcctccgtttggacgtcaggggcaaaccatcgatgtggtggtttcttccatgggaaatgccaaaagcttgcgtggaggtacgttgttgatgacaccgcttaagggcgttgacagtcaggtgtatgcgctggcgcagggcaatattctggttggcggcgcaggagcctccgctggcggtagcagtgttcaggttaaccaactgaacggtggacggatcaccaatggtgcggttattgaacgtgaattgcccagccagtttggcgtcgggaatacccttaatttgcaacttaacgacgaagatttcagcatggcgcagcaaatcgctgacaccatcaaccgcgtgcgtggatatggcagcgccaccgcgttagatgcgcggactattcaggtgcgcgtaccgagtggcaacagttcccaggtccgcttccttgccgatattcagaatatgcaggttaatgtcaccccgcaggacgctaaagtagtgattaactcgcgcaccggttcggtggtgatgaatcgcgaagtgaccctcgacagctgcgcggtagcgcaggggaatctctcagtaacagttaatcgtcaggccaatgtcagccagccagatacaccgtttggtggtggacagactgtggttactccacaaacgcagatcgatttacgccagagcggcggttcgctgcaaagcgtacgttccagcgccagcctcaataacgtggtgcgcgcgctcaatgcgctgggcgctacgccgatggatctgatgtccatactgcaatcaatgcaaagtgcgggatgtctgcgggcaaaactggaaatcatctgatgatcagcgacagcaaactactggcaagtgcggcctgggatgcgcaatcactcaacgaactaaaggcgaaagcgggcgaagatccggcggcaaatatccgtccggtggcccgtcaggtggaagggatgttcgtgcagatgatgttgaaaagcatgcgcgacgctttaccaaaagatggcctgttcagcagcgagcacactcgcctgtataccagtatgtatgaccagcagattgcccaacagatgacggcgggcaaaggtctggggcttgcagagatgatggttaaacagatgacgccagaacaaccattgccagaggagtccacgccagcagcaccgatgaaattcccgctcgaaactgtggtgcgttatcaaaatcaggcgctttcgcagctggtgcaaaaggccgtgccacgtaactacgatgattcgctgccgggtgacagtaaagcattcctcgcgcaactctcgctgcccgcccaactggcaagccagcaaagcggtgtgccacatcatttgatcctcgctcaggcggcactggaatctggttgggggcaacggcaaatccgccgcgaaaacggcgagccgagctataacctgtttggtgtcaaagcctctggcaactggaaagggccagttactgaaatcaccacgactgaatatgaaaacggcgaagcgaagaaagtaaaagcgaagtttcgcgtctacagctcgtatctggaagccttgtcggattacgttgggctgttaacgcgtaacccgcgctacgccgccgtgacgaccgccgcgagtgcggaacagggggcgcaggccctacaggacgcgggctatgccaccgatcctcactatgcccgcaaactcaccaacatgattcagcagatgaaatcgataagcgacaaggtgagcaaaacctacagtatgaacattgataatctgttctgaataactcaagtccggcgggtcgctgccgataatactctgtaattgaaggcttataaggaacctccatgtccagcttgattaataacgccatgagcggactgaacgcggcccaggcggcgttaaatacggcaagtaataatatctccagctataacgttgccggatatacccgccaaaccactattatggcgcaggccaatagcacgttgggcgctggcggctgggttggcaatggtgtctacgtttctggtgtgcagcgtgagtatgatgcgtttattaccaaccagttacgtgcggcgcagacgcaaagtagcggtctgactgcccgctatgagcagatgtcgaaaatcgacaatatgctctccaccagtacctcttcgctggcaacacagatgcaggatttcttcaccagcctgcaaacgctggtgagtaacgcggaagacccggcagcgcgccaggcgctgattgggaaatcagaaggattggtgaatcagtttaaaaccaccgatcaatatctgcgcgaccaggacaaacaggtcaatatcgcgataggtgccagcgttgatcagatcaacaactacgctaaacaaattgccagcctgaacgatcaaatctcgcgcctgacaggcgtgggggcaggggcgtcacctaacaatctgctggatcaacgcgatcaactggtgagcgaattaaaccagattgttggtgtagaagtcagcgttcaggatggcggcacttataacatcacgatggccaatggttactcactggttcagggaagtacggcgcggcaactggcggcagttccttccagcgctgacccttctcgtacgactgtcgcttatgttgatgggacggcaggcaatattgagatcccggagaaattactgaataccgggtcgctgggcggcattctgacattccgttctcaggatctggaccagacgcgtaatacgcttggacaactggcgctggcatttgccgaggctttcaacacccaacacaaagccggatttgatgctaacggcgatgccggtgaagatttctttgctatcggtaagcccgcggttctgcaaaacacgaaaaacaaaggtgacgttgcgatcggtgccacggtaactgatgcctccgcggtactggcgacagattacaaaatctcgttcgataataatcagtggcaggtcacccgccttgccagcaataccacttttacggtgacgccggatgccaacggtaaagtggcatttgatggtctggagttgacgtttacaggaacgcctgccgttaacgacagcttcacgctgaaaccagtaagtgacgccatcgtcaacatggatgtattaatcaccgacgaagcgaaaatagcgatggcgagcgaagaagatgcgggtgatagcgataaccgcaacggtcaggccctgctggatctgcaaagcaacagtaaaacggtgggcggtgcgaaatcctttaacgacgcttatgcctcgttagtgagtgatatcggtaataaaaccgcgacgttgaaaaccagtagcgccacgcaaggtaatgtggtgacgcagctttccaatcagcagcagtcgatttccggtgtcaatctcgatgaggagtacggaaatctgcaacgttttcagcagtattacctggcgaatgcgcaggttctgcagacggcaaacgcgatttttgatgcgctgattaacattcgctaaggggagataagatgcgtttcagtacacagatgatgtaccagcaaaacatgcgtggtatcaccaattctcaggcagaatggatgaagtacggcgaacagatgtcgacgggtaagcgagtcgttaacccttctgacgatcccattgctgcatcacaagccgtagttctctcccaggcacaggcgcaaaacagccagtacacgctggcgcgtactttcgccactcaaaaagtgtcactggaagagagtgtacttagccaggtcaccactgctatccagaatgctcaggaaaaaattgtctacgccagcaatggcaccttgagtgacgatgaccgggcctcgctggctacggatattcaggggcttcgtgaccagttgctgaatctggcaaacaccactgacggtaacgggcgctacatttttgccggttataaaacagagactgcgccgtttagcgaagagaaagggaaatacgtcggtggagcagaaagtattaaacaacaggtcgatgcttcgcgttcgatggtgatagggcacacgggtgacaaaattttcgacagtattaccagcaacgcggtagcggaaccagacggtagcgcttctgaaaccaatctttttgccatgctggatagtgccatcgcagccctgaaaacgccggtcgcggatagcgaagcggataaagaaaccgccgctgcggcgttagataaaaccaaccgcggactgaaaaactcgctgaacaatgtgctgactgttcgcgcggaattaggcacgcagctgaacgaactggagtcgctggattcattaggtagcgatcgcgctttagggcaaacgcagcagatgagcgatctggttgatgtggactggaatgcaactatttcatcttacatcatgcagcaaacggcattgcaggcatcgtataaagcatttaccgatatgcagggattgtcgctcttccagctcagcaaataatttcgctttaaaacatatcatgaaactgggtatgttttgtctgcctgctctgggatcgctggggcgggcatttttttgcctattttgcattgttggttagcaaggatgccattcgatgaattttaatatgttgattcaaagatgaaataaaaaagccctggcagttaccagggcttgattactttgagctaattattactcaacaggttgcggacgcgcaggagcggcagaggcatgatgtgttgccgtatgaccacctgcggcacctttaccttcgaaggcaaaagtagggcgctgccagtcactgtgacgcggtgcctccggaacatattccggtgctggagcgcgcgtcattggcgcggtagcgtggttatgctcaacggtgacctcaggttcgaccgcagctaccgtttcaacttctgctgcgacttcagcgactactggcgcggcaggttgagcaacaacttcaggttcagcaactacaacctcagcagtttcgacaacttcttcaatatctgccgtctcttcctgcggttcaaccaccggttctgcttgttctgcaacttcctgggctacggcaacatcagactcggtaatcacctgcggctgttcagttaccgcggcagcgatcacttcaggatgcgtcgtttcaaccacttccggttgcggttcggcaacctgaacgggggcttctacgacaccggccacttcttcaacaactggcgcgctaacaaccggttcgatagcggcggcgacagggacctcagtcaccatcggctgcacatgtacttcttcctgttcgcgctgctcttcaacctgtacatcttgcggacgtacaattggatagcggatccagactttgccagaggccagttccggagacgcgcacgctacggtcaacggcattggcgactgggttggataacgctcgtcacgatagcgacgacgacgctgaccacttacgcgcaggtgacgaggcgagcggcgagaacgacgcggcatgccaccgttgtcacggttatcagcattgttctcttcttgctgttctggtgcagtttgcgctacgactggcagcgggactttcaccagttctgtgcgtggagctggcgcttcctgaacaattggttcggcagcgacagtttcttcaaccaccggtgcgactaccgcttcttcggctacgctttgctcgtaacgcactttctgattgagctgacgctgtttacgacgcggctgaaccggacgtacacgttcttcctgttcggtttcctgaacagattgctcttcaacattcagcgccttcgcttcttgttgcgcctgacgtttatcatcattacggcggcggctacgttcacgacgcggcgcttgctgctcgtcggcggtacgcgctttttccgttacctcagcctgctgacggctctcacgcgtctcggcagtctgctgctgtgcctggcgacgattacgacggttttcttcgcgattatcgctgccttcagtacgttcactacgggtgtcgcggcgctcattacggtcacggcggttgttctgacgaggcttgcgacgatcctgttgacgttccggtttcgcttctgctttcggtgctggttgctcggtcggtttggtttcttcaccaccgctgaacagcgctttcagtgcgccgaagaagcggctcaacagcccaggttgtgcaggagctgctggtgttgccggtgcagctttcggtgctggagctacaacaggcgcggcaggttcagctggcgttggcgcaggcggcacatccggcatggcaaaggttgccagcgcaggttgttccggacgcttacgttcagcgaactcttcttcagacggcagcgccatcgcttcttcatgcagcttcggcagcatgtagcttaaggttggggtttcttcccctttacgcacgcgcagcacgtggtagtgcggggtttccatctgatcgtttggcacaattacacagcgcacaccgtcctgacgagtttcaatggcatttaccgcagaacgtttttcattcagcaggtaagaagcgattggcacaggaacaatggcgtgaacttcctgggtgttctctttcagcgcttcttcttcgatcagacgcagaatagagagcgacagcgattcgttgtcacgcacggtgccagtaccagaacaacgcggacaaacgtgatgactggattcacccagtgatgggctcaggcgctgacgggacatttccagcaggccaaagcgagaaatatggctgatttgaatacgcgcacggtcctgacgcaccgcttcacgcagacggttttctaccgcacgctggtggcgtactggcgtcatgtcgatgaagtcgataacaatcaggccgccgaggtcacgcaggcgcagctgacgagcaatctcatcggcagcttcgaggttagtgttaaacgcggtttcttcgatatcgccgccgcgggtcgcgcgtgcggagttgatgtcgatggccgttaacgcttcggtgctgtcgataacaatggaaccaccagacggcagacgaacttcacgctggaaggcggactcgatctgtgactcgatctggtagtggctgaacagcgggatctcgccggtgtacagtttgattttgctgctgaaatccgggcgacctaatgcagcgatatgctgacgtgccagttcgagcactttcgggttatcgataaggatttcgccgatgtcctgacgtaagtaatcgcggaatgcgcgaacgattacgttgctctcctgatgaatcaggaacggggccgggcggctttcagcggcttttttgatggcttcccagtgtttcagacggaagcttaaatcccattgcagcgcctcagcagatttgccgacgccagcggtgcgcacgataagccccatgccttccggcagttcaaggcttgccagtgcttcttttaattcggtacggtcgtcgccttcgatacggcgagaaatgccacccgcgcgcgggttgttcggcatcagaaccagatagctacccgccagactgataaaggtggttaatgccgcgcctttgttgccgcgctcttctttatcgatctgaacaatgacttcctgaccttcacgcaacacatctttaatgttgggacgaccatgagcactgtagttagcagggaaatattcgcgggcaatttcttttagtgggaggaaaccgtgacgttcagcgccgtaatcaacaaaagcagcttccagactcggttcaatgcgggtgattttacctttgtagatgtttgcctttttctgctcgtgccctggactttcgatatccaggtcatacagacgctgcccatctacaagggcaacgcgcaactcttcctgctgagttgcgttgattaacattcttttcatcgtaacttactcattattcttacattgacgactaagctgcgggcaaagtaacgcctttccgggtgtgaaccgatggcctcgtgtctagtcgcgtcgccaacctcacggttatcgtcagctcaaagaggcgcagagtgtcggttgcccgtttttcatgcggaaaaacagcgcaattatcaaagaaacagactgggtattactctccagaaatatttccatctaccggtaaggactgcaacccgcagcccgctaactgcctgaaagatcaatacgtcttacgccattgctgcgtggatgatcggtcgggcaaaatgggttattccgtaaaatttcttgttttaacaaggatggacacggaaacggcctcattattccactgcaagccttgttatagcaagatgacttttaccatttatcacccgcttactcacagttttttcacttcttgctggtgattggtttaataaccatcaataaagtgatcacgcagtgaagtaataaggtgcaaaagtaaatataagcatagaaaaatgagtggcgcgaatcctgttggctaattagaatcgccaaccatgaaaacagagactccatccgtaaaaattgttgctatcaccgctgacgaagcggggcaacgtatcgataactttttgcgtacccaattgaaaggcgtaccaaaaagtatgatttaccgtattttgcgtaaaggcgaagtgcgggtgaacaaaaaacgtattaagcctgaatataaactcgaagcgggtgatgaggtgcgtattccaccggttcgcgttgctgagcgggaagaagaggcggtttcgccacatctgcaaaaggtggcggcgctggcggacgtcatcttatatgaagatgatcacatcctggtgctgaataaaccttccggtacggcggtacatggcggcagtggtttaagcttcggcgttattgaaggtttgcgggcgttgcgcccggaagcgcggttccttgaactggttcatcgtcttgaccgggacacctcaggtgttttgctggtagcgaaaaaacgctcggcgttgcgttctctgcatgagcaattacgtgaaaaagggatgcaaaaagattacctggcgctggtgcgcggtcagtggcagtcgcatgtgaagagcgttcaagcaccgttactgaaaaatattctgcaaagcggcgaacgtatcgtgcgtgtgagtcaggaaggcaaaccgtcggaaacacgctttaaagtggaagaacgctatgcatttgccaccctggtgcgttgtagcccggtaacagggcgtactcaccagatccgtgtgcatacacaatatgcgggtcatccgattgcctttgacgatcgctacggtgaccgtgaatttgacaggcagctcactgaagcaggcacgggattaaatcgcctgttcctgcacgctgcagcgttgaagtttactcatccggggaccggtgaggtgatgcgtatcgaagctccgatggatgaaggtttgaagcgttgtttgcaaaagctgcgtaacgcgcgctaatacaagcatataaacctgataatgggcggttggcctgataaggcgtttacgccgcatcaggccgccagcaccgattgccggatgcgacgtaaccacatccggcgcaaaaaactatcccatcagcgggtttttcccttcccgacgtaacatctgacacagcgcgattagcggtaaaccaaccagcgtgttaggatcacgcccctctaaacgctcaaacagcgtaatgccaaatccttcactcttaaagctacccgcgcagtgcaggggatgctctttacgcacgtaattatcaatctccgcctcgctcaggtgacggaaatggacgtcaaaaggctccacttctgtttgcagatgcccattcgccgaattaaacaacgccagtccagtatagaaggtgacgatattgccgctggctttgcgtaattgcagacgggcattttcttccgttaacggtttaccggtgatttcgccatcaagaacacatacctggtctgaaccaataattaaatgatccggataacgtgacgccagagattgcgctttttcttgtgccagtcgaagcaccaactgtcgcggtgattcgtcgctgcgtggggtttcgtcgacctctggtgctgcacattcaaaagagatttgcagtttttccagaagagcgcgacgccatggcgaggtggaggctaaaataagtttaggcatatttttttccatcagatatagcgtattgatgatagccattttaaactatgcgcttcgttttgcaggttgatgtttgttatcagcactgaacgaaaataaagcagtaacccgcaatgtgtgcgaattattggcaaaaggcaaccacaggctgcctttttctttgactctatgacgttacaaagttaatatgcgcgccctatgcaaaaggtaaaattacccctgactctcgatccggttcgtacggctcaaaaacgccttgattaccagggtatctatacccctgatcaggttgagcgcgtcgccgaatccgtagtcagtgtggacagtgatgtggaatgctccatgtcgttcgctatcgataaccaacgtctcgcagtgttaaacggcgatgcgaaggtgacggtaacgctcgagtgtcagcgttgcgggaagccgtttactcatcaggtctacacaacgtattgttttagtcctgtgcgttcagacgaacaggctgaagcactgccggaagcgtatgaaccgattgaggttaacgaattcggtgaaatcgatctgcttgcaatggttgaagatgaaatcatcctcgccttgccggtagttccggtgcatgattctgaacactgtgaagtgtccgaagcggacatggtctttggtgaactgcctgaagaagcgcaaaagccaaacccatttgccgtattagccagcttaaagcgtaagtaattggtgctccccgttggatcggggataaaccgtaattgaggagtaaggtccatggccgtacaacagaataaaccaacccgttccaaacgtggcatgcgtcgttcccatgacgcgctgaccgcagtcaccagcctgtctgtagacaaaacttctggtgaaaaacacctgcgtcaccacatcactgccgacggttactaccgcggccgcaaggtcatcgctaagtaatcacgcatctgcgtgatgaagcttagtgaggattttccccaggcaactggggaaagaccaaaccgggcggcgacgataccttgacacgtctaaccctggcgttagatgtcatgggaggggattttggcccttccgtgacagtgcctgcagcattgcaggcactgaattctaattcgcaactcactcttcttttagtcggcaattccgacgccatcacgccattacttgctaaagctgactttgaacaacgttcgcgtctgcagattattcctgcgcagtcagttatcgccagtgatgcccggccttcgcaagctatccgcgccagtcgtgggagttcaatgcgcgtggccctggagctggtgaaagaaggtcgagcgcaagcctgtgtcagtgccggtaataccggggcgctgatggggctggcaaaattattactcaagcccctggaggggattgagcgtccggcgctggtgacggtattaccacatcagcaaaagggcaaaacggtggtccttgacttaggggccaacgtcgattgtgacagcacaatgctggtgcaatttgccattatgggctcagttctggctgaagaggtggtggaaattcccaatcctcgcgtggcgttgctcaatattggtgaagaagaagtaaagggtctcgacagtattcgggatgcctcagcggtgcttaaaacaatcccttctatcaattatatcggctatcttgaagccaatgagttgttaactggcaagacagatgtgctggtttgtgacggctttacaggaaatgtcacattaaagacgatggaaggtgttgtcaggatgttcctttctctgctgaaatctcagggtgaagggaaaaaacggtcgtggtggctactgttattaaagcgttggctacaaaagagcctgacgaggcgattcagtcacctcaaccccgaccagtataacggcgcctgtctgttaggattgcgcggcacggtgataaaaagtcatggtgcagccaatcagcgagcttttgcggtcgcgattgaacaggcagtgcaggcggtgcagcgacaagttcctcagcgaattgccgctcgcctggaatctgtatacccagctggttttgagctgctggacggtggcaaaagcggaactctgcggtagcaggacgctgccagcgaactcgcagtttgcaagtgacggtatataaccgaaaagtgactgagcgtacatgtatacgaagattattggtactggcagctatctgcccgaacaagtgcggacaaacgccgatttggaaaaaatggtggacacctctgacgagtggattgtcactcgtaccggtatccgcgaacgccacattgccgcgccaaacgaaaccgtttcaaccatgggctttgaagcggcgacacgcgcaattgagatggcgggcattgagaaagaccagattggcctgatcgttgtggcaacgacttctgctacgcacgctttcccgagcgcagcttgtcagattcaaagcatgttgggcattaaaggttgcccggcatttgacgttgcagcagcctgcgcaggtttcacctatgcattaagcgtagccgatcaatacgtgaaatctggggcggtgaagtatgctctggtcgtcggttccgatgtactggcgcgcacctgcgatccaaccgatcgtgggactattattatttttggcgatggcgcgggcgctgcggtgctggctgcctctgaagagccgggaatcatttccacccatctgcatgccgacggtagttatggtgaattgctgacgctgccaaacgccgaccgcgtgaatccagagaattcaattcatctgacgatggcgggcaacgaagtcttcaaggttgcggtaacggaactggcgcacatcgttgatgagacgctggcggcgaataatcttgaccgttctcaactggactggctggttccgcatcaggctaacctgcgtattatcagtgcaacggcgaaaaaactcggtatgtctatggataatgtcgtggtgacgctggatcgccacggtaatacctctgcggcctctgtcccgtgcgcgctggatgaagctgtacgcgacgggcgcattaagccggggcagttggttctgcttgaagcctttggcggtggattcacctggggctccgcgctggttcgtttctaggataaggattaaaacatgacgcaatttgcatttgtgttccctggacagggttctcaaaccgttggaatgctggctgatatggcggcgagctatccaattgtcgaagaaacgtttgctgaagcttctgcggcgctgggctacgacctgtgggcgctgacccagcaggggccagctgaagaactgaataaaacctggcaaactcagcctgcgctgttgactgcatctgttgcgctgtatcgcgtatggcagcagcagggcggtaaagcaccggcaatgatggccggtcacagcctgggggaatactccgcgctggtttgcgctggtgtgattgatttcgctgatgcggtgcgtctggttgagatgcgcggcaagttcatgcaagaagccgtaccggaaggcacgggcgctatggcggcaatcatcggtctggatgatgcgtctattgcgaaagcgtgtgaagaagctgcagaaggtcaggtcgtttctccggtaaactttaactctccgggacaggtggttattgccggtcataaagaagcggttgagcgtgctggcgctgcctgtaaagcggcgggcgcaaaacgcgcgctgccgttaccagtgagcgtaccgtctcactgtgcgctgatgaaaccagcagccgacaaactggcagtagaattagcgaaaatcacctttaacgcaccaacagttcctgttgtgaataacgttgatgtgaaatgcgaaaccaatggtgatgccatccgtgacgcactggtacgtcagttgtataacccggttcagtggacgaagtctgttgagtacatggcagcgcaaggcgtagaacatctctatgaagtcggcccgggcaaagtgcttactggcctgacgaaacgcattgtcgacaccctgaccgcctcggcgctgaacgaaccttcagcgatggcagcggcgctcgagctttaaaagaggaaaatcatgaattttgaaggaaaaatcgcactggtaaccggtgcaagccgcggaattggccgcgcaattgctgaaacgctcgcagcccgtggcgcgaaagttattggcactgcgaccagtgaaaatggcgctcaggcgatcagtgattatttaggtgccaacggcaaaggtctgatgttgaatgtgaccgacccggcatctatcgaatctgttctggaaaaaattcgcgcagaatttggtgaagtggatatcctggtcaataatgccggtatcactcgtgataacctgttaatgcgaatgaaagatgaagagtggaacgatattatcgaaaccaacctttcatctgttttccgtctgtcaaaagcggtaatgcgcgctatgatgaaaaagcgtcatggtcgtattatcactatcggttctgtggttggtaccatgggaaatggcggtcaggccaactacgctgcggcgaaagcgggcttgatcggcttcagtaaatcactggcgcgcgaagttgcgtcacgcggtattactgtaaacgttgttgctccgggctttattgaaacggacatgacacgtgcgctgagcgatgaccagcgtgcgggtatcctggcgcaggttcctgcgggtcgcctcggcggcgcacaggaaatcgccaacgcggttgcattcctggcatccgacgaagcagcttacatcacgggtgaaactttgcatgtgaacggcgggatgtacatggtctgaccgcgatttgcacaaaatgctcatgttgcgcgcagtctgcgtggttatgagtaataattagtgcaaaatgatttgcgttattggggggtaaggcctcaaaataacgtaaaatcgtggtaagacctgccgggatttagttgcaaatttttcaacattttatacactacgaaaaccatcgcgaaagcgagttttgataggaaatttaagagtatgagcactatcgaagaacgcgttaagaaaattatcggcgaacagctgggcgttaagcaggaagaagttaccaacaatgcttctttcgttgaagacctgggcgcggattctcttgacaccgttgagctggtaatggctctggaagaagagtttgatactgagattccggacgaagaagctgagaaaatcaccaccgttcaggctgccattgattacatcaacggccaccaggcgtaagtgaacatctccaggcggtcgttcgaccgcctgagttttatctttttgtcccactagaatcattttttccctccctggaggacaaacgtgtctaagcgtcgtgtagttgtgaccggactgggcatgttgtctcctgtcggcaataccgtagagtctacctggaaagctctgcttgccggtcagagtggcatcagcctaatcgaccatttcgatactagcgcctatgcaacgaaatttgctggcttagtaaaggattttaactgtgaggacattatctcgcgcaaagaacagcgcaagatggatgccttcattcaatatggaattgtcgctggcgttcaggccatgcaggattctggccttgaaataacggaagagaacgcaacccgcattggtgccgcaattggctccgggattggcggcctcggactgatcgaagaaaaccacacatctctgatgaacggtggtccacgtaagatcagcccattcttcgttccgtcaacgattgtgaacatggtggcaggtcatctgactatcatgtatggcctgcgtggcccgagcatctctatcgcgactgcctgtacttccggcgtgcacaacattggccatgctgcgcgtattatcgcgtatggcgatgctgacgtgatggttgcaggtggcgcagagaaagccagtacgccgctgggcgttggtggttttggcgcggcacgtgcattatctacccgcaatgataacccgcaagcggcgagccgcccgtgggataaagagcgtgatggtttcgtactgggcgatggtgccggtatgctggtacttgaagagtacgaacacgcgaaaaaacgcggtgcgaaaatttacgctgaactcgtcggctttggtatgagcagcgatgcttatcatatgacgtcaccgccagaaaatggcgcaggcgcagctctggcgatggcaaatgctctgcgtgatgcaggcattgaagcgagtcagattggctacgttaacgcgcacggtacttctacgccggctggcgataaagctgaagcgcaggcggtgaaaaccatcttcggtgaagctgcaagccgtgtgttggtaagctccacgaaatctatgaccggtcacctgttaggtgcggcgggtgcagtagaatctatctactccatcctggcgctgcgcgatcaggctgttccgccaaccatcaacctggataacccggatgaaggttgcgatctggatttcgtaccgcacgaagcgcgtcaggttagcggaatggaatacactctgtgtaactccttcggcttcggtggcactaatggttctttgatctttaaaaagatctaagttgtcattttccacccttataaaaggtccgcttgcgggccttttttcttagcttttattccgacttgttccgtagtgaacatgctgccacactaacaattctctgataaggagccggtatgttcttaattaacggtcataagcaggaatcgctggcagtaagcgatcgggcaacgcagtttggtgatggttgttttaccaccgccagagttatcgacggtaaagtcagtttgttatcggcgcatatccagcgactacaggatgcttgtcagcggttgatgatttcctgtgacttctggcctcagcttgaacaagagatgaaaacgctggcagcagaacagcaaaatggtgtgctgaaagtcgtgatcagtcgcggtagtggcgggcgagggtacagcacattgaacagcggaccggcaacgcggattctctccgttacggcttatcctgcacattacgaccgtttgcgtaacgaggggattacgttggcgctaagcccggtgcggctggggcgcaatcctcatcttgcaggtattaaacatctcaatcgtcttgagcaagtattgattcgctctcatcttgagcagacaaacgctgatgaggcgctggtccttgacagcgaagggtgggttacggaatgctgtgcggctaatttgttctggcggaagggcaacgtagtttatacgccgcgactggatcaggcaggtgttaacggcattatgcgacaattctgtatccgtttgctggcacaatcctcttatcagcttgtcgaagtgcaagcctctctggaagagtcgttgcaggcagatgagatggttatttgtaatgcgttaatgccagtgatgcccgtatgtgcctgtggcgatgtctccttttcgtcagcaacgttatatgaatatttagccccactttgtgagcgcccgaattagtcatgaaaaaagtgttattgataatcttgttattgctggtggtactgggtatcgccgctggtgtgggcgtctggaaggttcgccatcttgccgacagcaaattgcttatcaaagaagagacgatatttaccctgaagccagggaccggacgtctggcgctcggtgaacagctttatgccgataagatcatcaatcgtccacgggtttttcaatggctgctgcgtatcgaaccggatctttctcactttaaagccgggacttaccgctttacaccgcagatgaccgtgcgcgagatgctgaaattgctggaaagcggtaaagaagcacagttccctctgcgactggtagaagggatgcgtctgagcgattacctcaagcaattgcgtgaggccccgtatatcaagcatacgctgagcgatgataagtacgccaccgtagcgcaggcacttgaactggaaaacccggagtggattgaaggttggttctggccagacacctggatgtataccgccaataccaccgatgtcgcgttactcaagcgagcgcacaagaaaatggtgaaagcggtcgatagcgcctgggaagggcgtgcggacggtctgccttataaagataaaaaccagttggtgacgatggcatcaattatcgaaaaagaaaccgccgttgccagtgaacgcgataaggttgcctcagtatttatcaaccgtttacgcattggtatgcgcctgcagaccgacccgaccgtgatttacgggatgggagagcgttataatggcaaactttctcgtgcagacctggaaacgccgacagcgtataacacctataccattaccggtctgccgccaggtgcgatagcgacgccgggggcggattcgctgaaggctgctgcgcatccggcaaaaacgccgtatctctattttgtggccgatggtaaaggtggtcacacgtttaataccaatcttgccagtcataacaagtctgtgcaggattatctgaaagtgcttaaggaaaaaaatgcgcagtaagtatatcgtcattgaggggctggaaggcgcaggcaaaactaccgcgcgtaatgtggtggttgagacgctcgagcaactgggtatccgcgacatggttttcactcgggaacctggcggtacgcaacttgccgaaaagttaagaagcctggtgctggatatcaaatcggtaggcgatgaagtcattaccgataaagccgaagttctgatgttttatgccgcgcgcgttcaactggtagaaacggtcatcaaaccagctctggctaacggcacctgggtgattggcgatcgccacgatctctccactcaggcgtatcagggcggcggacgtggtattgaccaacatatgctggcaacactgcgtgatgctgttctcggggattttcgccccgacttaacgctctatctcgatgttaccccggaagttggcttaaaacgcgcgcgtgcgcgcggcgagctggatcgtattgagcaagaatctttcgatttctttaatcgcacccgcgcccgctatctggaactggcagcacaagataaaagcattcataccattgatgccacccagccgctggaggccgtgatggatgcaatccgcactaccgtgacccactgggtgaaggagttggacgcatgagatggtatccatggttacgacctgatttcgaaaaactggtagccagctatcaggccggaagaggtcaccatgcgctactcattcaggcgttaccgggcatgggcgatgatgctttaatctacgccctgagccgttatttactctgccaacaaccgcagggccacaaaagttgcggtcactgtcgtggatgtcagttgatgcaggctggcacgcatcccgattactacaccctggctcccgaaaaaggaaaaaatacgctgggcgttgatgcggtacgtgaggtcaccgaaaagctgaatgagcacgcacgcttaggtggtgcgaaagtcgtttgggtaaccgatgctgccttactaaccgacgccgcggctaacgcattgctgaaaacgcttgaagagccaccagcagaaacttggtttttcctggctacccgcgagcctgaacgtttactggcaacattacgtagtcgttgtcggttacattaccttgcgccgccgccggaacagtacgccgtgacctggctttcacgcgaagtgacaatgtcacaggatgcattacttgccgcattgcgcttaagcgccggttcgcctggcgcggcactggcgttgtttcagggagataactggcaggctcgtgaaacattgtgtcaggcgttggcatatagcgtgccatcgggcgactggtattcgctgctagcggcccttaatcatgaacaagctccggcgcgtttacactggctggcaacgttgctgatggatgcgctaaaacgccatcatggtgctgcgcaggtgaccaatgttgatgtgccgggcctggtcgccgaactggcaaaccatctttctccctcgcgcctgcaggctatactgggggatgtttgccacattcgtgaacagttaatgtctgttacaggcatcaaccgcgagcttctcatcaccgatcttttactgcgtattgagcattacctgcaaccgggcgttgtgctaccggttcctcatctttaagagagacatcatgtttttagtcgactcacactgccatctcgatggtctggattatgaatctttgcataaggacgtggatgacgttctggcgaaagccgccgcacgcgatgtgaaattttgtctggcagtcgccacaacattaccgggttatttacatatgcgggatctggtaggcgaacgtgacaacgtcgtattttcttgtggcgtgcatccactcaaccagaatgatccctacgatgtagaagatttacgccgtctggcggcagaagagggtgttgtagcgctgggtgaaaccgggctggattattattacacgccggaaactaaagtacgtcagcaagagtccttcatccatcatatccagattggtcgtgaactgaacaagccggttatcgtccatacccgtgacgcccgtgccgatacgctggcaattctgcgcgaagaaaaagtgacggattgcggtggcgtactacactgttttacagaggacagagaaacggcgggtaaattactggatctcggattttacatctccttttccggcattgtgaccttccgtaatgcggagcaactgcgcgatgctgcgcgttatgtccccctggatcggttactggtggaaactgactcaccttaccttgcgccggtaccgcatcgaggaaaagagaatcaacctgcgatggttcgtgacgttgcagaatacatggctgtgttgaaaggtgttgccgttgaagaactggcgcaggtaaccaccgataacttcgcccgtctgtttcacatcgacgcttcccgccttcaatccatccgttgaatgagtttttttaaagctcgtaattaatggctaaaacgagtaaagttcaccgccgaaaattgggcggtgaataaccacgtttgaaatattgtgacatatgttttgtcaaaatgtgcaacttctccaatgatctgaagttgaaacgtgatagccgtcaaacaaattggcactgaattattttactctgtgtaataaataaagggcgcttagatgccctgtacacggcgaggctctccccccttgccacgcgtgagaacgtaaaaaaagcacccatactcaggagcactctcaattatgtttaagaatgcatttgctaacctgcaaaaggtcggtaaatcgctgatgctgccggtatccgtactgcctatcgcaggtattctgctgggcgtcggttccgcgaatttcagctggctgcccgccgttgtatcgcatgttatggcagaagcaggcggttccgtctttgcaaacatgccactgatttttgcgatcggtgtcgccctcggctttaccaataacgatggcgtatccgcgctggccgcagttgttgcctatggcatcatggttaaaaccatggccgtggttgcgccactggtactgcatttacctgctgaagaaatcgcctctaaacacctggcggatactggcgtactcggagggattatctccggtgcgatcgcagcgtacatgtttaaccgtttctaccgtattaagctgcctgagtatcttggcttctttgccggtaaacgctttgtgccgatcatttctggcctggctgccatctttactggcgttgtgctgtccttcatttggccgccgattggttctgcaatccagaccttctctcagtgggctgcttaccagaacccggtagttgcgtttggcatttacggtttcatcgaacgttgcctggtaccgtttggtctgcaccacatctggaacgtacctttccagatgcagattggtgaatacaccaacgcagcaggtcaggttttccacggcgacattccgcgttatatggcgggtgacccgactgcgggtaaactgtctggtggcttcctgttcaaaatgtacggtctgccagctgccgcaattgctatctggcactctgctaaaccagaaaaccgcgcgaaagtgggcggtattatgatctccgcggcgctgacctcgttcctgaccggtatcaccgagccgatcgagttctccttcatgttcgttgcgccgatcctgtacatcatccacgcgattctggcaggcctggcattcccaatctgtattcttctggggatgcgtgacggtacgtcgttctcgcacggtctgatcgacttcatcgttctgtctggtaacagcagcaaactgtggctgttcccgatcgtcggtatcggttatgcgattgtttactacaccatcttccgcgtgctgattaaagcactggatctgaaaacgccgggtcgtgaagacgcgactgaagatgcaaaagcgacaggtaccagcgaaatggcaccggctctggttgctgcatttggtggtaaagaaaacattactaacctcgacgcatgtattacccgtctgcgcgtcagcgttgctgatgtgtctaaagtggatcaggccggcctgaagaaactgggcgcagcgggcgtagtggttgctggttctggtgttcaggcgattttcggtactaaatccgataacctgaaaaccgagatggatgagtacatccgtaaccactaatccgtaagacgttggggagactaaggcagccagatggctgccttttttacaggtgttattcagaattgatacgtgccggtaatgctgaaattacgcggtgtgccgtagacgatagaaccttccacgttggtatcgtaggttttgtcgaacaggttattgacgttcccctgtaacgagaagtttttcgtcacctggtagcgggtgaagagatccaccagcgcgtagctaccttgctcggcgcggaaggtgccatacggcgtcacggtgtcggtatacacgcgattttgccagttaacaccaccgccgaccgtcaactctggcatgacaggcaaccgatagctggtgaacattttaaccgtggtgcgtggcagattaggattaacggcgtttccttcgttatcctctgcaatatagcgcgttgcgccaaatgtcagctgccagttgtcggtaattgcgccgttgagttcaaattccacccctttactgactgtcccatccaccgctttataggcggtttcgccgttgctgccggggataggtgtaccggtggactgagcgacattatcctgctcaatacggaagatggctaacgtggtggtcagacggctattcatccagtccgatttcagacccagctcgtagttgttaccggtgattggagccagatatttgcctgaactgtcacgatcattttgcggctggaaaatagaggtatagctggcgtaggtcgaccagttgtcattgatgtcaaacaccagaccagcgtaaggcgtggtgtggtttttctccatgctgtaagtcagcgtatcaacccgccagttggtataacgtgcgccgaggatcagatgcagcggatcggcaagggtgacacgagtggcagcatataacgatttcatatgtgtggtatcgtcctgcgccaggctctgtggtgaccagtcggtttgtgggaaattgccattaaagttgtagaaactgccaatttcatccgggaagatgttggcccatgaactgaagtaacgattgttttgtttgctgtaactgccaccaaacattagattgtgctgacgaccaaacaattcataactaccgtcagcgaacaaatccagcgcatcaactttacgtttgccactgttccaaccggtgccgccgacataatcaaagccaggtccataattactgtatggcccaaccagcataccatccgctttgtttacataggcatcgacatacatcattttgctgtcaaattcgacttcagagtgggtggcattcagtgtcgcttgccaggtatcagcaaactgctgcttcagggtcataaagaccttgttgatctctttatcgttgtacgcccagtcaggtgcggtactgcgtgcgcgatcgtaactgttgctgctgccatcagtattccagcgcggtaaaccgccccaggtagggctattaacatcaatgcgctgatattcgtaaccggctgaaagcgtcgtaagatcgcctaaatcagcatcgacaatgcccgagaagaaggtcttttcactgttgtagcggtccagccatgagtcgttattctggtagccgccgacaattcgcgcgcggattttaccgtcttcggtgagtgggctttgtaaatccgccacataccgttctttgttccagctaccgtattccgccgagacatcgcctttaaattcacgactggtcgcgtgttttcgaaccatattaattgccgcagatggattacccgtcccggtcatgagtcctgtcgcgccacgcactacttctacgcgttcaaagagtgccatatcagaaagtgcgtcgcccagattccagcgcgattcaaaataggtggggataccatcaaccatatagttatcgatctggaatccgcgggaataataaagagcacgatcggaatccgcctgacttttgctgatccccagcgtgttttccatcacttcgcccagcgtttgtaactgctgatcttccatccgctgctggctaacaatagtgaccgactgaggaatatcacgttgagtcatctgcattttggtacccgcagaggtagacgttacgctgtaatcattttcgccatcatctggagctgtggctgaaccctcaacaatcaccgtttcttcagtggctggtgcagcaaaagcggcagaaggtaatagtgccagtgctatgcaaccggcaagtagtgacggtttggtgatggcttgatattgattatccctgttaaattgtgttgaaagcatttgaaatctcttggtttatgttgtcgtcaggctcatgccggaggagggtgatgagcgattatatttagtgtgcgaataattttgtttgtaaatgcaaatgagaaatatacgcattcatatttgtcatgtaaaccaaacagagaatgtcttttcagcgcattcgcaggcagaaatgggaataatggcgatatatacggcagcaaaacgattttttgcttaagaaatcgtgagttaaggttgaaagagcaggtttaactcgaccatactctatactcgcagtgtggcgcggcgtagcatggcgcaacgcatggctatttgaaaaaggaaaatgtcgtggcagaagaaactatattcagcaaaattattcgtcgtgagatcccctccgatatcgtctaccaggatgatctggtaacggcgtttcgcgatatttcgccgcaagcgccaacgcatattctgatcattccgaatatcctcattccgactgtgaacgacgtctcagctgagcatgagcaggcgctgggacgcatgatcaccgtagcggcaaaaattgctgagcaagaaggtattgccgaagatggctatcgtctgatcatgaataccaaccgccatggcggacaagaggtttaccacatccatatgcacttgttgggtggccgtccgctgggaccaatgctggcgcataaaggtctgtaacgatgagaaaaggatgctttgggctggtgtctctggtgttgttactgctggtgggctgtcgttcacatccggaaattccggtgaatgatgagcaatcgctggtgatggagtcatctttattggctgcgggcatcagtgcagaaaagcccttcctttcgacgtctgatattcaaccttcagcatcctcaacgctttataacgaaaggcaagaacccgttaccgttcattatcgtttttactggtatgacgccagagggctggagatgcatcctctggaaaggccacgcagcgttaccattcccgcacattcggcggtaacgctgtacggcagcgccaattttctgggggcgcacaaagtcagactttatctatatttgtaaggggtgaatcttgatgacaaaaatgagtcgctacgccttgattaccgcgctggcgatgtttctcgccgggtgtgtggggcaacgtgaacctgcaccggtagaagaagtgaaaccagcgccggaacaaccagccgagccacaacagcctgtccccacagtgccctcggtgccgacgatcccgcagcagccaggcccaattgagcacgaagatcaaactgcaccgcctgcgccgcatattcgccattatgactggaatggcgcaatgcagccgatggtcagtaagatgcttggggctgacggggtgactgcgggtagcgtcctgctggttgatagcgttaacaaccgtactaacggttcgctgaatgccgcagaagcgaccgaaacgctgcgaaatgcgctggctaataacgggaaatttaccctggtttccgcccagcaactgtcgatggcgaagcaacagttaggtttgtcgccgcaggacagtttaggcacccgtagtaaagccataggcattgcccgcaatgtcggcgctcattacgtgctgtactccagcgcctctggcaacgttaacgctccgaccctacaaatgcagctgatgctggtgcagacgggcgaaattatctggtcaggtaaaggtgccgtttcgcagcaataatcccatcacgcgcgacgaattgctgtcgcgctttttcccgcagtatcatcccgtcacgacgtttaatagtgggcttagtggcgggagttttctcattgaacatcagggccagcgttttgttgtgcgtcagccgcacgatcctgatgcgccgcagtccgcgttcttgcgccagtatcgggctttatcacaactacccgcatgcattgcaccgaagccgcatttatatctccgtgactggatggtagtcgactatctgcccggcgcggtaaaaacgtatttgccggataccaacgaactggcaggcttgctgtattatctacatcaacaaccacgttttggctggcgaataacgctgttgccgttactggaactgtactggcagcaaagcgatccggcgcggcggacagtgggttggctgcgaatgttaaaacgtctgcgcaaagcgcgggaaccacggcctttacgcttaagtccattgcatatggatgtccacgccggaaatttagtgcatagcgcgtcagggttaaaactcatcgactgggagtatgccggagatggtgatatcgcgctggaactggcggcggtgtgggtggaaaatactgaacagcaccggcaattggtcaatgactatgccactcgcgcgaagatttatccggcgcaattatggcgtcaggtcaggcgatggtttccctggctgctgatgctcaaagcagggtggtttgagtaccgctggcgacaaaccggcgatcaacaatttatcaggctggccgatgacacctggcggcagctattaataaaacaataaggagagcagtgtgggtccagtaatgttggatgtcgaaggttacgaactggacgcggaagagcgtgaaatactggcgcatccgctggtgggagggctgattctctttacgcgtaactatcatgatcctgcccagttacgtgaactggtgcgccagatccgcgcagcttcgcgcaatcgtctggtggtggcggttgatcaggaaggtggacgcgtgcagcgttttcgtgaaggttttacccgcttgccagcggcgcaatcattcgctgcgctgtcaggaatggaagagggtggcaaactggcgcaggaggcaggttggttgatggccagcgaaatgatcgctatggatattgatatcagctttgcgcctgtgctggatgtcgggcatatcagcgcggcgattggcgagcgttcttatcatgccgatccacaaaaagccctggcaattgccagccggtttattgatggtatgcatgaagccggaatgaaaacgaccgggaaacacttcccaggacacggtgcagtaacggcagactcacacaaagaaacaccgtgcgatccacgtccacaagcggagattcgcgctaaagatatgtcggtcttcagttccttaatccgcgaaaataaactcgacgccattatgcctgcgcatgtgatctacagtgatgttgatccgcgtccggcgagcggttctccctactggctgaaaaccgttttgcgtcaggaactgggttttgacggcgtgattttctctgacgatttatcgatggaaggtgccgcgattatgggcagttatgccgaacgcgggcaggcttcactggatgcgggttgcgatatgatcctggtctgcaataatcgtaaaggggccgtcagcgtgttagataatctgtcaccgatcaaggcagaacgtgttacacgtttgtatcataaaggttcattttcgcgacaggaactgatggactcggctcgctggaaagcgatcagcacccgtctgaatcagttacatgaacgctggcaggaagagaaagcaggtcactaaccctggcttatgtgaggaagcgatgattatctatttacacggttttgactctaacagtccgggtaaccacgagaaagtcttacaattgcagtttattgacccggatgtacgcttgataagctacagtacgcggcatccgaaacatgatatgcagcatctgcttaaagaagtggacaaaatgttgcaactgaacgttgacgagcgtccgctaatttgcggcgttggcttgggcggatactgggcggaacggattggttttctttgcgacatccgccaggtgatcttcaaccctaatttgttcccttatgagaacatggaaggcaagattgatcgcccggaagagtatgccgatattgccactaagtgtgtgaccaacttccgtgagaagaatcgcgatcgttgcctggtgattttgtcgcgtaatgatgaagcgcttaacagccagcggacatctgaagagttgcatcattattacgagattgtctgggacgaagagcagacgcacaaattcaagaatatctccccgcatttacagcgcattaaagcgttcaaaaccctcgggtaaatgccctcgtcgcatcaggtaaccttgccggtacctgatgcgctccgaattctgtgggtcggataaggcgtccacgccgcatccgacagtcgagcatcaatgcctgatgcgcttcttatcaggcctaccgaacgccctgcatacacccctcactctatatcactctcacaaattcgctcaaataataaacaataaactctgttttttgatctcacccggtaaagtcgcctatcttttcagcaacaaaacttgattaacatcaattttggtatgaccaatgcaccattcatgttattctcaatagcgaagaacattttcattgctgtaacctgttgttaattaagagctatgttaataaccattaattaacaattggttaataaatttaagggggtcacgttgactacgccattgaaaaagattgtgattgtcggcggcggtgctggtgggctggaaatggcaacacagctggggcataagctgggacgcaagaaaaaagccaaaattacgctggtcgatcgtaaccacagccacctgtggaaaccgctgctgcacgaagtggcgactggctcgcttgatgaaggcgtcgatgcgttgagctatctggcccatgcgcgcaatcatggtttccagttccagctgggttccgtcattgatattgatcgtgaagcgaaaacaatcactattgcagaactgcgcgacgagaaaggtgaactgctggttccggaacgtaaaatcgcctatgacaccctggtaatggcgctgggtagcacctctaacgatttcaatacgccaggtgtcaaagagaactgcattttcctcgataacccgcaccaggcgcgtcgcttccaccaggagatgctgaatttgttcctgaaatactccgccaacctgggcgcgaatggcaaagtgaacattgcgattgtcggcggcggcgcgacgggtgtagaactctccgctgaattgcacaacgcggtcaagcaactgcacagctacggttacaaaggcctgaccaacgaagccctgaacgtaacgctggtagaagcgggagaacgtattttgcctgcgttaccgccacgtatctctgctgcggcccacaacgagctaacgaaacttggcgttcgcgtgctgacgcaaaccatggtcaccagtgctgatgaaggcggcctgcacactaaagatggcgaatatattgaggctgatctgatggtatgggcagccgggatcaaagcgccagacttcctgaaagatatcggtggtcttgaaactaaccgtatcaaccagctggtggtggaaccgacgctgcaaaccacccgcgatccagacatttacgctattggcgactgcgcgtcatgcccgcgtccggaagggggctttgttccgccgcgtgctcaggctgcacaccagatggcgacttgcgcaatgaacaacattctggcgcagatgaacggtaagccgctgaaaaattatcagtataaagatcatggttcgctggtatcgctgtcgaacttctccaccgtcggtagcctgatgggtaacctgacgcgcggctcaatgatgattgaaggacgaattgcgcgctttgtatatatctcgctataccgaatgcatcagattgcgctgcatggttactttaaaaccggattaatgatgctggtggggagtattaaccgcgttatccgtccgcgtttgaagttgcattaatcgacgtacactggcggatgtggcataaacgcctcatccgcccttgaggaacagcgcgatcggcagccgcgttgtatcaggcatcctttcagactcctccgaatccttaagtatttccagccattcccgcgcttttcatcttctgtctgatagctgcttttctccttcgcttgcatgattggcataactgcaaagaaggaggtgttcccgtgaataaatcaatgttggcgggtatcgggattggtgtcgcagctgcgctgggcgtagcggcagtggccagtctgaacgtgtttgaacggggcccgcaatacgctcaggttgtttctgcaaccccaatcaaggaaacggttaaaacaccgcgtcaggagtgtcgcaacgtcacagtgacccatcgtcgaccggtgcaggatgaaaatcgcattaccgggtcggtgctcggcgctgttgctggcggcgtgatagggcatcagtttggtggtggtcgcggtaaagatgtcgccactgttgtgggggcgctgggtggtggatatgccggtaaccagatccagggctctctccaggaaagcgatacttacacgactacgcaacagcgttgtaaaacggtgtatgacaagtcagaaaaaatgctcggttatgatgtgacctataagattggcgatcagcagggcaaaatccgcatggaccgcgatccgggtacgcagatcccgctagatagcaacgggcaactgattttgaataacaaagtataacaaggctgtactctgcaatttggcccctcattcgctcaggctgaggggctttttttgcgacttatttcaccagttcgggccataaacgcaaagtcgttccggcaatctgcatcagtttttccagcgatgcaccttcgcgtgcgctgatcgacatcccctgaataatacaattaaggaattctgccagatgtgtcacgtcacagtggggcgggatttccccgcgcgcttgtcgttgacataaaaactgctgcaaagtgcgctcttgcatcgcatggcgtgatttcaacgtattggcgatatctcctgaatctggggagagggtggtgcagttgttgatcatgaagcagcctgccggggtgtctttgctggtaaagcagttggcgatggcagcaaaatagtcagccagcgcagactccacgcttttctcttcacaaaacagctgtgcttcatgcttagcggcaaaacgatcgatatagcggtcgagaacggcacgaaataacccctctttgttggtaaattccgcgtatagcgtgggcgctttggctccggtcgcttcgacgaggtccgcaagagaagtcgcttcataaccgtgttgccagaacaatttcatggccttatcaagcgcggcatccctgtcgaacacttttgggcggccacggcttttttttacacattgtgttgagtcagttgccatgatgccgttgtacctggtgactgtgaatgaaaggttattataaaaataatcacctccgttcaccagtccagatcccataaaaataattgctttctatttaactgaaatttaaagatttttaaattaattaatgattgttataaaaaatatcttgtatgtgatccagatcacatctatcatttagttatcgatcgttaagtaattgcttgcgacgtcattcatctgcataaggccactattatgaaaaacgtaaaaaccctcatcgctgcggcgattttaagctccatgtcatttgccagctttgcggctgtcgaagttcagtcaacgccagaaggccaacaaaaagtcggtacaatcagtgctaacgcggggacaaatctgggatcgctggaagagcagctggcgcaaaaagcggatgagatgggcgcaaaatctttccgtattacttctgtaaccggtccgaataccctccatggaacagcagtaatttataaataagcattaaccctcattaatgcctgctactgctgattttttccccgcgacatgccgtgtcgcggggatttttttatccgggctttacagcgtttgtgggctcacttgatgacggcggacatccaccggcatcccggaacggacatccatcacatgttgcatcacttcagcgtcagtttgtgctgcatctttaaatgattgcattgcgctattcagcgtaattggcagcagctgcggatcgtcatcaatcttctctgacagcggctgatgtacttcaaccagacgcgcaccgtttggttcggcagagacttttatcggagtgttgatgatattcactttggtgcctggggtgacctggctaaagagtgttttgatatcgtcatcccgcagacgaatacagccagaacttacccgcatgccaatgccgaaatcggcgttcgtaccatgaagcaaataaacgccgccataggccgccagacgaatcgcatgatggcccattgggttatccagtccagccggcactaccgcaggcaactcaattccctgtgctttataacgggcgcggatgtttgccgttggcgtccaggttgggtttgcacgtttgtctgaaacggtggtcaccattgtcggtgtcagcgtgtcaccacctaactgaccaatacctattggatacacggttaccgaatttttacccggcgggtagtaatagagacgcagctccgcaatgttgatcacaatgccttcgcgcggcgcatctggaagtagggtttgcaacgggatcgttaacacgctgcccgcgcgcggtacgtaaggatcaacgccggggttagcctgtaacagagcgagaaagccgacgttgtattttttggcgatggcttccagagaaccaccgtcattttccaccacatgaaatttgttttcgccaaccagacgactgcccgctggcggcagcggccaggtgttggcttttgccggtagcgccagcgccacggcagcggcgaacgtaaaaaacgttagccagcgagaaaaacgcgttttgatcatcaccaaaaatccataataaatataaggttattgtaataaacagataagcctgaattatggatggtgacagtgtcggatagtgcagggaagtgcaaagaatttgtaaatgttgcagatgggggcgcagaaacgcccccgatttaccattaagcgatcgcgttctcttccagttcacgcataaactggcgtacccattcgatacgcgttttccgctcactcaaatcctgaataaatttcaggcgcgtcggaccatcaaggcggtaatgctgcggctgtttttgcagcaaaccaatcaaccaggccggattaacgtgattcttctcggcaaattcgatcaccccgcctttctcattaccttccagcttcctgatccccagtttctgcgcttgctggcgcagacgggcaatatccagcagggtacgcgccggatctggcagcaggccgaagcgatcgataagctcgactttgatctcttccagttcgttttccgttttggcgctggcaatacgtttgtagaacgacagacgcgtgttcacgtcagggatgaaatcatctggcaatagcgacggcatccgcagctcgacttctgtttgctggctggtgagatcttccagcgacggctcgcgtccggctttcagtgcatcgacggcgttttccagcaactccatatacagcgagaaaccgatggtttccattgagccgctttgttcttcgccaagcagttcacccgcgccgcgaatctccagatcgtgcgttgccagcgcaaaacctgccccgagatcttccagcgaggcaattgcttcaagacgtttttgtgcatcggtagtcatcgcttttggatgcggtgtcagcaaccatgcatatgcctgatgatgcgaacgtccgacgcgaccgcgtaactggtgcagctgcgccagaccgaagtgatccgcgcgttcaatgataatagtgttggctgtcgggatgtcgatcccggtttcgataatggttgtacaaaccagcacgttgaaacgttgatgatggaaatcattcatcacccgttccagttcgcgctcgcgcatctgcccgtgaccgatggcgatccgcgcttctggcaccagttctgccagccgttcggcggctttctgaatgttttccacatcattgtagagataataaacctgtcctccgcgcaaaatttcacgcaggatcgcctcccggaccaccatgctgtcatactcacggacaaaggttttaactgccagacgacgggcgggcggcgtggcgataatcgacaggtcacgcattccgctcattgccatattcagcgtacgtgggatcggcgttgcagtaagcgtcagaatatccacgttcgcgcgcatcgctttaatgcgctctttatgacgcaccccgaagcggtgttcttcatcgacaatcagcaggcctaaatctttaaacttgacgtcactttgcagcagtttgtgcgtaccgatcagaatatcgattttcccttccgccacttccgcaaggatttgcgtctgctctttggcgctgcggaaacgggagatcatttcgatacgtaccggccagttggcgaaacggtcgcggaagttgtcgtaatgctgctgcgcgagaagggtggtaggcaccagcaccgccacctgcttgtggttatctactgccaggaaagctgcgcgcatcgccacttctgttttaccaaagccaacatcgccgcacaccagacgatccattgccagcggctgacacatgtcgctaagtaccgcattaatggcctgcgcctgatccggcgtggtttcaaacgggaagctgtcgcagaacaactgatactgctcacgatcgtgtttaaacgcgaagccctctttggcggcgcgttgcgcgtagatatccagcaattccgccgccacatcacgcactttttccgccgctttctgccgcgcgcgtgaccacgcatcgccgccaagtttatgcagcggggcgttttcttccgcgccacctgcgtaacggctaatcagatgcagtgacgacaccggaacatacagtttggcgtcgttggcataggtgagcatcagatactcgccagtaatgccacccgcttccagcgtggtcattccggcataacgaccgacgccgtgctccagatggaccaccggctgaccaatatgcagttccgcaaggttacggatcagtgtatcggggttgatggtgcggcgagaatcctgacgacgacgggcaacgcgttcaccgagcagatcgctttcgcaaatcagcgccagattacgcaccgtatcgacaaaaccatgttcggcagcgccaatcatcagataacgcccacggtcgctggcttcatcaagacgcataatgcgttgcggagcaattttaattcgtgcgagcagttcacccagcgcttcacggcgaccttcactttctaccgagaacaccaccggaccgtcgaaagtctcgaggaacttacgcagcgcatccagcggcgctttttgttgtgcctgaacggccaggtctggcagtttctggaaacctaaattggcattcgcggcttttgtcggtaaatgttcagtttttagctgcacccggggccagtttttcagctctgagaagagctcgtccacccgcagccagagcgattgtggtggcaacagcgggcgcatcggatcgacgccgcgattctcaaaacgcgccagcgtgtcagcctggaaacgttcggcactggtttccagatcgccagtattcacgagcaaggtattggcagggaaataactgaacagcggcggcagtggttcgctgaagaacaatggctgccagtactcgatcccggcaggtaatgtgcctttactcacttgctggtaaatatgttctggatcgcgcttcacttcgaaggtatcgcgccactggctgcggaacagttcaattgccgctttatcggtcggaaattcgtgcgcgggcagcagattgatcgcttctacttcctccagcgtgcgctggctgtcgacgtcaaacacccgcaggctgtcgatttcatcatcaaagaaatcaagacgataaggcagctcactccccatcgggaagagatccagcaacgcgccgcgcgtggcgtattcgccgtgctccatcacctggtcaacatggcgataaccggcgctgtccagttgggttcgtaatgcatctcgtgacaggcgctgaccttttttcatcaccagcgcatgaccgtggagaaaactgtgtgggcaaacgcgctgcataagcgtattcaccggaacaatcagtacgccacgctgcatcgtcggtagctggtaaagggtggaaaggcgcgaggagataatgtcctgatgaggcgaaaaactgtcgtagggaagagtttcccagtccgccagattcatcaccatttgatcggtaaactggctgatttcatcatgcaaacgcagagcattttgcatatctggtgcaatgagtaccaccggaccggcgtgacgttcggcaatttccgctaccagcgttgcacaggctgcgccggttaactcgcccagcagacgctgctcacccgctttgacgggcagcgtataacgatattgttcaggcataacggttgtcagattctcgttaggatatgcctcaacatatgggggcatatctctgataagcaatgctgttcattatccgtaatcgacatggtttagcaaattgaatcgccccggctggggcgatggcttagcgggagtaactgacggcagcgggcagtgaaggcggggagaacaacagatcgctgaatgcacgctgtgaaagttttcttaccagcaagcccgcaacagtacagatgaacaaactgacaaagggataaaccagcaggagtgtcagttcgacttgcggcgaccagcgtgctgcgttcatttgcgcaagcagagttaagctgaatatttcaaccagaatgcgatgggtggtgtagatagcaatggtgttggagccaatcacattcagcaggctggtggagcgcataccgaatcgttgctcgtattgataaaacagcttcatgatcaccacaatcgataccagcgacaacagcagcgagatagtaaacaaccaggcaccgaccgccagaacggtaagcaaagaagccatcagcagatggcggcgcaacggcacctctttaacacaggtcattattgttgcgccaaaccatgcgccaaggctgtaataaggcaaattgcggatcacactgttcattccccaccacggcgtgggaacgaaattaaccgccacactcagcagtacaaacaaggcgaatagtggcagcgccagacggctaaaaattttacataccacgaaatagacaattaacgcatacagataccacaagctggtgctggcggtgatcatcccgtgcaggaactcaccggtggaatcggcataagcggcattggaggcattgcttaaatcgcgctcaggtgccagccactggttcagcgcacttaacgccagccactgcaccacgccccaaagcgccagcacccagaagatgttccagatccgtttatcgagacaatttccccacggtacgctgtcgatatagcggcgaatcaaatagccggatataaagaaaaaaaccggcatacgaaagggggcaaggtaaagattgaaatagatccagcatttgctcaggacttccgataacggatgctgaaaagtggtcagatgcggataaaaggtaatgaccgagtgataaatcaccaccagacaaatacataaccctttgatctggttaatccatagctctttttgtttcatcaggacaacacgctcttttttaatttacatgcggttgatcctgcgggttatgacccgaggtgtaatgggtatctgtctgtattggatgatttttcagattaagatcaggcggcaagattgatgataaaacatggcaatttagccgattgatttacgggggcttttcagattagccctgacgatcacttacagttcagacgtttacccatcttgctttcgcttatatactcgtgtctttgctacagcaaccagacggatttcatgtaccaacctgtcgctctatttattggcctgcgttacatgcgtgggcgtgcagcggatcgcttcggtcgtttcgtctcctggctttctaccatcggcattaccctcggggtgatggcgctggtcacagtattgtcagtgatgaacggctttgagcgcgagctgcaaaacaacatccttggcctgatgccacaggcaattctctcttctgagcatggctctcttaacccgcagcaactcccagaaacggcagtcaaactggacggcgttaatcgcgtcgcacctattactaccggtgatgtggtactgcaaagcgcgcgcagcgtggcggtcggggtgatgctcggtatcgacccggcgcaaaaagatccacttacaccgtatctggtcaatgtgaaacaaactgacctcgagccggggaaatataatgtcatcctcggcgaacaacttgcctcacagctaggcgttaatcgcggtgatcaaatccgcgtgatggtaccatctgccagccagttcacgccgatggggcgtattccaagccagcgcctgttcaatgtgattggcactttcgccgccaacagtgaagtcgatggctatgaaatgctggtgaatattgaggatgcctcgcgtctgatgcgttatccggcaggcaatattaccggctggcgtttgtggctggatgagccgctgaaagtcgactcattaagtcagcaaaaactgcctgaaggcagcaaatggcaggactggcgtgatcgtaaaggcgagttgttccaggccgtacgcatggaaaaaaatatgatgggtttactgctgagcctgattgtcgccgttgcggcgtttaacattattacctcactagggctgatggtaatggagaagcagggcgaagtagcgatcctgcaaacgcaaggcttaactccgcgacaaatcatgatggtctttatggtgcaaggggccagcgccgggattatcggtgcgatcctcggagcggcgcttggcgccctgcttgccagccagttaaataatctgatgccgataatcggcgtcctgcttgatggcgcggcgctgccggtggctatcgaacctttacaggtcattgttattgcgctggtggcgatggctatcgcgctgctgtctacgctttacccttcatggcgcgctgccgccactcaacccgctgaggctttacgttatgaataagatcctgttgcaatgcgacaacctgtgcaaacgctatcaggaaggcagtgtgcaaaccgatgtgctgcacaatgtcagtttcagcgtcggcgaaggtgaaatgatggcgatcgtcggtagctctggttccggtaaaagtaccttgctgcacctgctgggcgggctggatacgccaacctccggcgatgtgatttttaatggtcagccaatgagcaaactgtcgtcggcagcgaaagctgaactgcgcaaccagaagctgggctttatttatcagtttcaccacctgctgccggattttaccgccctggaaaacgtggctatgccgctgctgattggcaagaaaaagcccgctgaaatcaacagccgtgcacttgagatgttaaaagcggtggggctggatcatcgtgcgaatcaccgcccatctgaactttctggcggcgaacgccagcgtgtggcgattgcccgtgcgctggtgaataacccgcgcctggtactggcggatgaacctaccggtaacctcgatgcgcgtaacgccgacagcatcttccagttgcttggggaattgaatcgcttgcagggcaccgccttcctggtggttactcacgacctgcaactggcgaaacgtatgagccgccagttagaaatgcgtgatggtcgtctgacggcggaactgagcctgatgggggcggagtaatggcgatgcctttatcgttattaattggcctgcgttttagtcgcggacggcggcgcggcggcatggtgtcgctgatctccgttatttctaccattggcattgccctcggcgtggcggtattgatcgtcggcttaagcgcgatgaacggctttgaacgcgaactgaacaaccgtattctggcggtggtgccgcatggtgaaatcgaggcggtggatcagccgtggactaactggcaggaagcactggatcacgtgcaaaaagtgccgggtattgccgctgccgcgccgtatatcaatttcaccgggctggtggaaagtggcgcgaatcttcgcgcaatccaggtgaagggcgttaacccgcaacaggaacagcgtctgagcgcattaccctcgtttgtccagggcgatgcgtggcgcaattttaaagcgggcgaacagcaaattatcatcggcaaaggcgtggcggatgcgctgaaagtgaagcagggggattgggtgtcgattatgatccccaactcgaatcccgagcataaactgatgcagccaaaacgtgtgcgtttgcacgttgccggtattttgcagttgagtggtcaactcgatcacagttttgccatgatcccgctggcggatgcccaacaatatcttgatatgggttccagcgtgtcaggtattgcccttaaaatgacggatgttttcaacgccaataagctggtacgcgatgcgggtgaagtgaccaacagctatgtttatattaaaagctggattggtacttacggctatatgtatcgcgatatccaaatgatccgcgccattatgtatctggcgatggtactggtgattggcgtggcctgtttcaacatcgtctccaccttagtgatggcggtgaaagacaagagtggcgatatcgcagtattaagaacgctgggggcgaaagatggtttaattcgcgccatctttgtctggtatggattgctggcagggctgttcggcagcctgtgtggtgtgattatcggcgtagtggtttcactgcaacttaccccgattattgagtggattgaaaagttgatcggtcatcagttcctctccagcgatatctattttattgatttcctgccatcggaattgcactggctggacgtcttctacgtactggtcacagcattgttgctgagtcttttggcaagttggtatccggcgcggcgcgccagtaatattgaccctgcgcgagtccttagcggccagtaaaggcagtacattaaaacaaggagcggcaatgtattacgggtttgatattggtggaacaaaaattgcgcttggcgtgtttgatagcggtcggcagttgcagtgggaaaagcgggtgccgacaccgcgtgacagctatgacgcatttttagatgcagtgtgtgagctggtagctgaagctgaccaacgttttggctgtaaaggttctgtcggcatcggtattccgggaatgccggaaacagaagatggtacgctgtatgccgccaatgtccccgctgccagcggtaaaccgctgcgtgccgacctgagcgcacgtcttgatcgcgatgtacgccttgataacgatgccaactgttttgccctttcagaagcctgggatgatgaatttactcaatatccactggtgatggggttgattctcggcaccggtgttggcggcgggctgattttcaacggcaaaccgattaccggtaaaagctacattaccggcgagtttggccatatgcgtctgccggttgatgcgttaaccatgatggggttggatttcccgttacgccgctgcggctgtggtcagcatggctgcattgaaaattatctgtctggtcgcggttttgcgtggctgtatcaacactattatcatcaaccgttgcaggctcccgaaattattgcgctttatgatcaaggcgatgagcaggcaagggcgcacgttgagcgttatctggatttattagcggtttgtctgggaaatatcctgaccatcgttgaccctgacctggtcgtcattggtggtggcttatcgaatttcccggcaatcacaacgcaactggcggacaggctgcctcgtcatctcttacctgtagctcgtgttccgcgcattgaacgcgcgcgccacggtgatgcgggaggaatgcgtggtgcggccttcctacatctaaccgattaaacaacagaggttgctatgctgtcgcgtcggggtcatcggttaagtcgttttcgtaaaaataaacgccgcctgcgcgagcgtttgcgtcagcgtatttttttcagagataaagtggtgccggaagcaatggaaaaaccaagagtactcgtactgacaggggcaggaatttctgcggaatcaggtattcgtacctttcgcgccgcagatggcctgtgggaagaacatcgggttgaagatgtggcaacgccggaaggtttcgatcgcgatcctgaactggtgcaagcgttttataacgcccgtcgtcgacagctgcagcagccagaaattcagcctaacgccgcgcatcttgcgctggctaaactgcaagacgccctcggcgatcgctttttgctggtgacgcagaatatcgacaacctgcatgaacgcgcaggtaataccaatgtgattcatatgcatggggaactgctgaaagtgcgttgttcacaaagtggtcaggttctcgactggacaggagacgttaccccagaagataaatgccattgttgccagtttccggcacccttgcgcccgcacgtagtgtggtttggcgaaatgccactcggcatggatgaaatttatatggcgttgtcgatggccgatattttcattgccattggcacatccgggcatgtttatccggcggctgggtttgttcacgaagcgaaactgcatggcgcgcacaccgtggaactgaatcttgaaccgagtcaggttggtaatgaatttgccgagaaatattacggcccggcaagccaggtggtgcctgagtttgttgaaaagttgctgaagggattaaaagcgggaagcattgcctgatgcactacgcttatcaggcctgcaaggggacgcaattaattgaatttgcgggttttgtgggccggataaggcgttcgcgccccatccggaataatacacgcgcacttttccggcctcttttatcgtttactcgtcaataacaatgcggcaataaacgtacagacaccaattagccctgcccagagtggcgatattctggtaatcgcaaagctattatcgatatacaaacataaagcctgataacccatattggcaatagtcatcgccactgcaaattttaacgcataaataaaacgagtcgtgtagtaaaagatcctggaaaataagataaacgtcgcagcccaggcgataaaacctaatgtgttggtgctgccggggggagcattttcatgctgttgtcctggatgcggataatacgttagtggcggcgtcgattgttttaatatctgtgcttgtagaacagccaatgcattattgattccctgataccagagatctgcatttaaataagccagcgtgtgattttctatcagaaggccgagatgtttatcgtccagaccactttcaacctggccgttggtgatcataattaaccgtggttcgcgggtagtaaatagtaacagaacacttccttttacatcactcaatgaagatgacgcatgcgccagcatcgctttaccattttgtctgagactggcttcattattaatgtcgggtaaaaccacaataaacggtgcaattcccgtttgttggcgaaaaagctcggctttatgcgcgatctcttcagcatctggtacagtaccggtaacgtccgtaaaaagtgtcttcattattggaattaatggcttgctggctgctgtcagaggcaggagtatcagtaaactgagcagtataatgaattttttcatgggcgggacttccgtttcctgcgtgattttttagaggagggcatacttattaataaaccgacggcgataaaaataacgcccataatgccgataaacccccatttaaaaaaattaacccacgggttatttatctcagccttttcaggatgcccgggagaataataaacattaactttatcgccttcgctgtcttcataaaaatcgctgccgatactcgaattgaaaattagcgtgtaatctggcgtcggtcgaaaggcaacgacgggataccacgaaccatctttacccgtgcgatgagaatgactggagtgccagacggtatcaacaatgacgccttcggtatgaatcgcgtctttgctataggtgaactggttataaaagacaacaacagaaatgaggatcagtaccagaccgataccgaggaatatacgaaagaaaactttactgtcctgactcattagccacatccttgctaactaaaaaacgggcggtaataccaccgcccgcttgctgaattaacgtcctgctttcagcttctgataatactcttcataaatgctgctggctgcgccaacgtcattctgccattcgccatttttaatggtttcagcatccgggtagagtgttttatcgttcgccacttctggacttaacagcttacgcgccgcaaggtttggcgttggataaccgatagtttcagcaacctgttttgccacatccgggcgcagcaggaagttgatcaatttcagcgcgccttctttgtttttggcatttgccgggatcgccaggctgtccatccagaaaatgccgccttctttcggccacaccacgtcaattggcgtacccgcctggcgtgcaacgaaagcagaaccgttccagatcatgccgaggttaacttcgccttccatgtacgggttcgccgggttatcggagttaaaggctgccacgtttggcatcagttttttcagctcgttatatgcagcttcaatctctttcggatcggtggtgttaccggagtagcccagcttacgcagcgccatctggaacacttcacgggcatcgtcggtcaacagcaggctgcctttgtactctggcttccacagatcggcccagctggtgacagatttcggatccaccgcatcaccgttaacaccaatcgccgtcgcaccccagatatacggaatggagtagtcgttattcgggtcaaaaggcttgttgagcatgtctggatcgagattgctgaagtttgttaacttcgacttgtcgatcttctggatcatcccttctttacgcattttatcaacgtaataggttgaaggaaccaccagatcataggcaccgtctttgtatgttttcagcttggcgtacatggtttcgttcgactcgtaagtcgaatagataaccttaataccggtttctttggtgaactgttcaagcagtcctggcggcacgtactcggtccagttgtagaaatacagcgtgttgttgtcatcggcgtgagcggcgctcatgcccagtgccagagcacccgccgcgagcaggtggcgtgaccattttttcatttaacgtcccctgtgttacctttcgttttatcacgagcaataagctggctggcaataaccatcaccagcgacagcaccagtaatatggttgccagcgcgttaacttccggcgatacgccgactttgaccatcgaataaatttttaacggcagaatttcataacttggtccggtgacgaacgaagaaactaccacatcgtccatcgacagggtaaagcttaacacccagcccgccgccaccgctggcattgccagtggcagaatgatttttcgcagaatggtaaattcgctggcaccgagatctttcgccgcttccagcattcgcacgtcaaaacctttcaggcgcgaatacaccgtcaccaccacaaatggcaggcagaaggtgatatgcgagaacagcagcgaccagaagccaagctgaatacccagcagcataaacagcaccagcagcgaaatcgccatcacgatatctggtgacatcatcaccacaaacagcattccgctaacgaacggcttaccacgaaagcgataacggtacagcgcaactgccgtcagtgaaccgataagcgtagcaaacgtcgccgaaaacaccgccattgttagtgaatgctgcgctgcctgtaacaggctgtcgttgttcatcagcaggctataccatttggtggtaaagccctgccagttgatgccaaagcgcgagctgttaaaggagttcacaatcaaaataatgattgggatatacaggtacgcgtagatagcggtcataaaaccgccgcgaagcagtcgaccgatcattcgagttccaccttcttattcagcaaacgagaagcgcgccagtaaaccagcaacatcaggcccattacgatagtcagcgtaatgctggtagctgcaccaaacggccagtcacgaatattaaggaactggaccttgatgacgttaccgatcagcaggtttttcgcaccgcccatcaggtcggatacatagaacaggcccatcgctggcagcatcaccagcagacatccggcaataattcccggcatcgtcagtggaataatgatacggataaaagtctgtaacttgctggcaccgagatcgcgcgccgcctcaagcaacggcttatccagtttttcgatactggagtacagcggcatcaccataaacggcagcagaatgtaaaccagaccgataatcaccgcactgggcgtgaacatgatacggattggtgtgtcgataacgcccagccagagcaaaaactcgttgagatagcctttggtgctgaggaaaattttcagcccgtagatacgaattaatgagttggtccagaacggaacaatcagcagaaacagcagcagcggacgcaccttgtgtggcaacttcgccagaaaccaggcaaacgggtagcccagcaccaggcaggcgagggtggcgatcagcgccatattcagcgagtgcaatagcacttcaaaatagagcggatcgagcagacgcgtgtagttatccagcgtaaagaccattttgacaaaactggcgtcgtcgcgggtcaaaaagctggtgccaatgatcatcaggttgggcagaaagacaaacaacacaagccaaccgacaatagtgacaatcactacattctggaacttacttgtgttcttcatcagccagtacgacctcccagctttctacccaattaatggccattttttggtcgagagagtggtcaaagtcaggatcgtcttcattgaagaattcgctgaccatcaccatcttgccattttccagttcaacaaccgactccagcgtcatgcctttgtagttacgctcgcgaacgtaaccaatcagcccttcagcgtggttgtcgtcgttaatctcttcaacacgtaagtcttccgggcgcagcagaacatgcagtttttgccccggttcaacggcgaagttaacgtagatattacattcgcggccttcaacgttggcgcgtacgcgctgctcgtctagacgttcgatgacagtggcgttaaacatattgatttcgccaatgaagccggcaacaaacaggtttttcggctcttcgtagatttcacgcggcgtgccgtcttgctcaatgcgaccatcgcgcatcaccacaatcctgtctgacatggtgagtgcttcttcctggtcgtgagtcacaaagacgaatgtaatgccaagcttacgctgtaacgctttcagctcgttctgcatttgcttacgcagtttgtaatccagcgctgagagcgactcatccagcaacaacagacgaggcttgttaaccaccgcgcgagcaatggcgacgcgttgctgttgaccaccagagagctgatgcggtttgcgttgagcgaaggtttccaactgcaccatccgcagggcttccatcacgcggggcgtaatttcagcagcgggggttttttgcatgcgcaacccaaaggccacattttcgaacacggtcatgtgggggaaaagtgcgtagctttggaaaacagtgttcacatagcggttttccgccggaacgtgggtgatgtcctcgttatccagcatgatgcgtccggaatcaacagtttccagacctgcaatcaggcgaagaacggttgttttaccgcagccagaagggccaagcagcgtgaggaactcgccattgttgatagtcagatccagctggggaatgacctctttaccatcaaagcatttgcgaattcccgccaattgcaccagcggtgaaagcgaactcggttgtttattcaattttttactctgtcccatgtaaacgcaacggatggcttaccgatgcggggtttgtggttaaccaccttggtgactcttaatgagggcggtaattctacggcaaaccgcttgaatcgccaatctttgttgtgaattactggcttagctttatattcattaaggtaatgctgataaatattcccgcttgcaggggtaaaagtgacctgacgcaatatttgtcttttcttgcttcttaataatgttgtcacaaaaagtgagggtgactacatggataaactacttgagcgatttttgaactacgtgtctctggatacccaatcaaaagcaggggtgagacaggttcccagcacggaaggccaatggaagttattgcatctgctgaaagagcagctcgaagagatggggcttatcaatgtgaccttaagtgagaagggcactttgatggcgacgttaccggctaacgtccctggcgatatcccggcgattggctttatttctcatgtggatacctcaccggattgcagcggcaaaaatgtgaatccgcaaattgttgaaaactatcgcggtggcgatattgcgctgggtatcggcgatgaagttttatcaccggttatgttcccggtgctgcatcagctactgggtcagacgctgattaccaccgatggtaaaaccttgttaggtgccgatgacaaagcaggtattgcagaaatcatgaccgcgctggcggtattgcaacagaaaaaaattccgcatggtgatattcgcgtcgcctttaccccggatgaagaagtgggcaaaggggcgaaacattttgatgttgacgccttcgatgcccgctgggcttacactgttgatggtggtggcgtaggcgaactggagtttgaaaacttcaacgccgcgtcggtcaatatcaaaattgtcggtaacaatgttcatccgggcacggcgaaaggagtgatggtaaatgcgctgtcgctggcggcacgtattcatgcggaagttccggcggatgaaagcccggaaatgacagaaggctatgaaggtttctatcatctggcgagcatgaaaggcaccgttgaacgggccgatatgcactacatcatccgtgatttcgaccgtaaacagtttgaagcgcgtaaacgtaaaatgatggagatcgccaaaaaagtgggcaaagggttacatcctgattgctacattgaactggtgattgaagacagttactacaatatgcgcgagaaagtggttgagcatccgcatattctcgatatcgcccagcaggcgatgcgcgattgcgatattgaaccggaactgaaaccgatccgcggtggtaccgacggcgcgcagttgtcgtttatgggattaccgtgcccgaacctgttcactggcggttacaactatcatggtaagcatgagtttgtgactctggaaggtatggaaaaagcggtgcaggtgatcgtccgtattgccgagttaacggcgcaacggaagtaagcgaaaagggatgcggcatgtgatgccgcatccggcttaaatccaaacttacccttcgaagaaccaatacccgctattgaccagcgccgcgagcatcgcgaggaatgacggatcttccagcgcatcgccaaaattctccgcagtcagcgcaatgttgctggcgagtgcatccagtgccggacggtgcggggaatcgatcttctcaccattggcatacacgtcgtcgccaatgcgcaatacgcgcagaccacccaggcgcaccagcacttcaccttgtttcagcgcatcgtagatttcatccggctgataaggcggctctggcggcgcgatatccagttcatgacgtgactgggatataaactcgccaaaccattgcttaaagtgttccggctggttgatcaattcgagcatcatctcacgcagtttatccatctcttgcggcagaacatccgcaggatgagcgcgaggtggaacatccggatcgctgtagtagttgccgcccagttcacgttgcagcacataatcggcaaatccactaatcagttcccgcgtatttggcgcgcgaaagcccacggaatagttcatcgcattttccagcgcgtagccttcatgcgggaatcctggcggaatataaagaatatcaccaggctccagctcttcatcgatgatggcttcgaacggatcgacctgtaacagatccggatgtgggcagtgctgtttcatttgcagcttttcgcccactcgccagcgacgacgtccggtaccctgaatgataaacacgtcgtactgatcgagatgcgggccgacgccgccgccgggtacagaaaaagaaatcatcagatcatcaatacgccagtccggtagttcacggaacggtcgcatcagcgcggcggtcggctcatgccagtggttcactgcctgtaccagtaatgaccagttggtttcaccgagatgatcgtagctttcgaacgggccgtggctgacctgccatttgccatcctggtgactgaccagtcgactgtcaacttcgctttccatcgccagacccgccaactcgtctggagagatcgggtcaataaaattattaaagccgcgttttaacaccaccgggcgtttctgccagtgacgttcaagaaaatcgggccagttaagagtgagttggtattccatgttaagcatccacaggctggtatctgcaaccgattataacggatgcttaacgtaatgcgtgaagtatgggcatatttattcatctttcggcgcagaatgctggcgaccaaaaatcacctccatccgcgcaccgcccagcatgctctctccggcgacgattttaccctcatattgctcggtgatttcgcgggctaccgccagccctacaccttgcccagggcgtaaagtatcaacccgttgaccacggtcgaaaatgacctctcgcttgcttaatggaataccggggccatcatcctcgaccacaatatagagatgctcgtcggtttgccttgcagaaatttcgacaaactcgaggcaatatttacaggcattatccagcacgttgcccatcacctcgacaaaatcgttctgctcaccgacaaagctgatctctggcgaaatatcgagagagatattgacccctttgcgttgatacactttgttcagcgctgaggtgagattgtccagcagtggggcgaccggatgcagctcgcggctgagcaatgtcccgccgcgcatactggcacgatgcaggtagtagccaatttgctgtgaaatgcggctgatttgctccagcattaccggctcagcatcactgacgctcatcttttcactacgcagagaacgcagcgtactttgcagcaccgccagtggcgttttcagactatgggtcaggtcggtgagcgtcgtacggtatttgtcgtaacgttcgcgttcactttttaacaatcggttcaggtttcgtaccagactggtcagttctcgcgttgtggctggattgagcaattcgcggttatgttcttccagttcgcggacttcttttgccagggcttcgatggggcgtaaactccaccaggcggcgacccacagcagcgggatcactaacagcagattggctgagagcacatagataaaccagctccagaccatataggaactttttagctccaccggaatggtatccaccaccacaatggttaattttggcatccgcgatgttgccgggtagacgtttactgccaccgagtgggtcatctccgcgtcgtcatcatcttcccgcacttcctgcaactgttgctgtatcgaatgatctccactcagcaagaggctggtatcgttaacatccgcttcaatttcatgaaaaccattcgatttcagccagtcaggctggatcatcttcatcagccagggcacgtcacgttgcgcccataaaagctgcccgttctcatcataaattagcgtcatggtggggctttgcttgtcgatattttcgggtaactcgacatgcaacttattgttttcccacttcgcaagggtatagaacagattgctctcgccacgtaacagccgaaacgtagttttatcgaaactgacgctataaccgatcagcgcgaccattccgtaggcaagcgaaagcaccagtactaccgctgccgttgccaacagaaaacgtacccgcagcgagagcgggaaaaaaagacgcagtaattttttcatcagcgcaattcgaacagatagccctggccgcgaacggtggtaatcacttcttggggatattgtgcctgaatttttttgcgcagacgtcccatcagtacatcaatggtatggctttcccgcagctccgcatccggatagagttggagcattaacgaatctttgctgaccactttgccattattgcgtatcaacgtttccataatagtgtattcgaacgcggtcagtttgatcacttcgtcattaatagataattcacggcgagagagatcaacctgaaacggggggagcgaaatgacctgtgaagccagaccgctattacgccgcattaatgcctgcattcgcgccatcacctcttcaatatgaaacggtttagtcacataatcatcagcaccggcacttaatacttcgactttgtcctgccagctttcacgggcggttaataccagaatcggcagtgaaacatcgttgctacgccagcggcgaatcagtgacagaccgtcctcgtctggcaatccgagatcgacaatcgcaatatccggtatatgttcattgagataataatcggcttctttggcatcttctgcgtcatcgacctgatgaccagcatcctgaatctgaactttaaggtggtgacgtaacaacgcattgtcttcaacaaccagtacgcgcatttttatttctccctgtcttaattattaaaatagtgtaacgcgattatgtggttatgggggtaaacattaaataaaccagcggggaggggaggtaaagtgaaaaaataaaaagcggataatcttaataagcaggccggacagcatcgccatccggcactgatacgaggtttatttcagctcatcaaccatcgtgatagctcgaccaatatagttagccggcgtcatcgctttcaggcgggctttctcttcttctggcaacgccagaccatcgataaactgcttcatgccttcggcgtcaacgcgcttaccgcgagtcagctctttcagcttctcgtacggtttttcgatgccatagcgacgcataactgtctggattggttcagccagcacttcccagttgtgatccagttcatccagcagatggtcacggttcacttccagtttgctcacgcctttcagggtggattgatatgcaatcaaggcataaccgatacccacgccgaggttacgcagcacggtagagtcggtcaggtcacgctgccagcgggaaaccggcagtttgcttgccagatgctgcaataccgcgttggaaaggcccagattcccttcggagttttcgaagtcgatcgggttaactttatgcggcatggtggaagaaccaatctcaccagcaatggttttctgtttgaagtggttaagggcgatataaccccagacgtcacggtcaaagtcgatcagaatagtgttgaagcgcgcaacgcaatcaaacagttcggcaatgtagtcgtgcggttcgatctgggtggtgtacgggttccactgaatacccagcgaggtgacgaactcttcgctgaactgatgccagtcaacttccgggtaagcggcgatgtgggcgttatagttaccgaccgcgccgttgattttgccgaggatctccacctggttaagctggcggtactggcgctccatacggtaggcgacgtttgccatctctttaccgatggttgacggcgtggctggctgaccgtgggtacgagacagcagcgggatatcgcgatactgaacggcgagatctttaatgccatcaatcagttgacgccagtatggcaggatcacttcatcacgcgcggttttcagcattaatgcgtgggagaggttattgatatcttccgaagtacaggcaaagtggatgaattcagaaaccgcgtgcagttccgggatctccgccactttttctttcaggaaatactcaaccgctttaacgtcgtggttagtggtacgctcgatagttttgatgcgcgccgcatcttcttcgctgaaactggcgacgattgcatcaaggtaaccgattgcgtcggcagcaaaagcaggaacttccttgatcgctgcgtgcgcggccagtttttgcagccaacgtacttcaacttgtacacggaatttcagcaaaccatattcgctgaaaatcccgcgcagcgcgctgactttatcgccgtagcgtccatcgacaggggaaacggcggtcagtgaggataattccatagatcacaactccggggttaaatgagcaagaatttgttttgcctgagtggtcaggcgattacgagaaaacatcagttgcagacgtccgccgccgacctggtgccagagcacggcggcgcgaatgcctgccagcagggttgcgcgaactttcgcctgcacttgtgggctttgcagtacagcaggggaaccggtgacctgaatgcgcgggccaagcgggctaatcacatcaacatagatagcagccatcgcgctcatcagcgtttcggactgtaaatcgaagtgttcgagctggcgttgcaggccgttgatccggttgcccagagtgtcgagcgcgcctttcgctgaggagagtttgcgctcaagcaccatcaagctgagtgtgtagcgggttaattcggcgtttaagccctggcgactgctggcattgagcacgccgagcagggtttccagcccgacgcgcaggttggcttcgctaccgccaaaaaccgccagcgtcgagctggggttcatatcaataatactgttgagtgagacgtgtagcgcatcggcatcacaatgcccctggtgagcgagttgttgcaccaggcgtgccgactgacaaataccggccagggcgagggtgatgtcatagtaattctttgccacgttcactgcttccttgttttaagtaaagataataatcagaccggcagcggcagacgctgctcaataataccgccaccgaggcacacttcaccgttatagaagacggcagactggcccggcgtcacggcggcaaccggttcatcgaaaatcacttcaatgcgatcatcgtccagcgccttgacggtgcaagggatatcggtctggcgatagcgggtttttaccgtgcaacgcatagtgccggtgaatggttcgcgatcgacccagtgcaactgctgggcaatcaacccgacagacatcagccgcgggtgttcatggccctgagcgacaaccagaatgttgttttcgacgtctttgtccaccacataccacggttcttcggtaccttctttggtgccaccgatacccagacctttacgctgaccgagagtgtgatacatcagcccctggtgctcaccaatttcatcgccatcgacggtaatgattttgcccggttgcgccgggagataacggcccaggaactcgcggaatttacgttcgccaatgaagcaaatgccggtagagtcttttttcttcgcggtgaccagaccaagatcttcagcaatcttacgcacctgcggtttttccagttcgccgaccgggaacaggctttgcgcaatctgctcatggctgagcgtataaaggaagtagctctggtctttattgctgtccagaccacgcagcaggcggctcttgccatcgacatcggcccgacgtacgtaatgaccggtagcgatataatcggcacctaaatcttcggcggcaaattcgaggaaggctttaaatttgatctctttgttgcacagaatatccggattcggcgtgcgaccggctttatattcggcaaggaacagttcgaagacgttgtcccagtactcggcagcaaagttaacggtgtgcagttcaatgccgagcttgtcgcagacagcctgggcatcagccagatccgctgccgctgtgcaatattcctcaccgtcgtcttcttcccagttcttcataaacaggccttcgacctgatatccctgttgttgcaacagccaggcagaaacggaggaatcgacaccgccggacatgccgacgattactttttttgcggtttcagacattggatcactcacgacattgaacttcaaggcggcgtattctatcacgcagccttttagatgacaccctttgtaaaaggccagttaaaatcgccaatcatctccagcggataacgttgcccgctttgataacaacgaatactttccgccaccagcggcgaacgaagatttgacgcctgtaaaatttcttcggcgctgacccaacggcagcagtcgatatcgctgtcatgaggctgggtcgggcatatttgctcaagctcaatggcaaagaggaaacgcaaaaacggcgttttatctggcgcaatccactgatgcatacgaataaagtgttgcggctgcgcgctgatgccggtttcttcccacagttcacgggcggcggcttccactaaggtttcatcggcttccagatgcccggcaggttggttccataacgctttaccattaatcgtctcttcaacgactaaaaatttgccttctgcgtgcaccacgcaagcaacggtaacgtgcggtttaaacattttgcatccttaatctgtcacttctcgccattcaccattggcaagattatccaaagagtaatcacccatcgcatagcgaatcagtcgcagcgtggggaagccaacatgggcggtcatgcggcgcacctggcgattacgtccttcatataaggtgatcttcagccagctggtgggaatacttttgcgttcacgaattggtggattccgcggccataaccacgcgggttcgtcaaccagctccgcgccggcgggcagggtagggccatcatttaaggttacgccattgcgcaaggcttcaagtgcgtcttgtgtgggaataccttccacctgcacataatagatttttccggtgcgtttacccggctgggttaaacgcgcctgcaacgcgccgttattggtcagcaccagcaacccttcgctatcgcggtcaaggcgacctgctgcataaacaccctgaaccgggatgaattcttttaatgttttgcgtccggcttcatcggtgaactgcggaagaacatcgtagggtttattgaacaggatcacacgcgtgggctggttttcaggtttacgcctggtagaacgttgcgagctgaatcgcttaacctggtgatttctaaaagaagttttttgcatggtattttcagagattatgaattgccgcattatagcctaataacgcgcatctttcatgacggcaaacaatagggtagtattgacaagccaattacaaatcattaacaaaaaattgctctaaagcatccgtatcgcaggacgcaaacgcatatgcaacgtggtggcagacgagcaaaccagtagcgctcgaaggagaggtgaatggaaagtaaagtagttgttccggcacaaggcaagaagatcaccctgcaaaacggcaaactcaacgttcctgaaaatccgattatcccttacattgaaggtgatggaatcggtgtagatgtaaccccagccatgctgaaagtggtcgacgctgcagtcgagaaagcctataaaggcgagcgtaaaatctcctggatggaaatttacaccggtgaaaaatccacacaggtttatggtcaggacgtctggctgcctgctgaaactcttgatctgattcgtgaatatcgcgttgccattaaaggtccgctgaccactccggttggtggcggtattcgctctctgaacgttgccctgcgccaggaactggatctctacatctgcctgcgtccggtacgttactatcagggcactccaagcccggttaaacaccctgaactgaccgatatggttatcttccgtgaaaactcggaagacatttatgcgggtatcgaatggaaagcagactctgccgacgccgagaaagtgattaaattcctgcgtgaagagatgggggtgaagaaaattcgcttcccggaacattgtggtatcggtattaagccgtgttcggaagaaggcaccaaacgtctggttcgtgcagcgatcgaatacgcaattgctaacgatcgtgactctgtgactctggtgcacaaaggcaacatcatgaagttcaccgaaggagcgtttaaagactggggctaccagctggcgcgtgaagagtttggcggtgaactgatcgacggtggcccgtggctgaaagttaaaaacccgaacactggcaaagagatcgtcattaaagacgtgattgctgatgcattcctgcaacagatcctgctgcgtccggctgaatatgatgttatcgcctgtatgaacctgaacggtgactacatttctgacgccctggcagcgcaggttggcggtatcggtatcgcccctggtgcaaacatcggtgacgaatgcgccctgtttgaagccacccacggtactgcgccgaaatatgccggtcaggacaaagtaaatcctggctctattattctctccgctgagatgatgctgcgccacatgggttggaccgaagcggctgacttaattgttaaaggtatggaaggcgcaatcaacgcgaaaaccgtaacctatgacttcgagcgtctgatggatggcgctaaactgctgaaatgttcagagtttggtgacgcgatcatcgaaaacatgtaatgccgtagtttgttaaatttattaacgggagcgtaacgctcccgttgttttttgttaggctgctaacggttatcaaaattttatcaaaaaaagttatcaaaacccctcggtagttttggggtaggctggccggtcaggtggtagttctactactagtctcccacatagatattccttagctttttattattgctggcggacgctcgttaatatttaaggtcttcattgattaagacatccccaaagttagttatgtattcactgttattaggacaattatgaattaccactccttacacccgctcaaatattgttaaattgccggttttgtatcaactactcacccgggactcgccaggggacagccaacaggcattgggtgcaatcaccttagcgttcaggtacatgcggaatgtaaaaaaggccgcgagcgcggccccttcacatacatctttagtactgagactgtttaacctagggaattattatcgtattatattgcattacaactcccaacagtgacatatgaacttcctgctttactccacgactttaatatttcaaggccatgtgaagaacatatttcttgcactgcgagttcatcgagtaatccatagtaagaaacactttttgaatttttgtaaatgtatccgtaaagatgttttcttcctgtttcgtattttttgaagtatgagcttttatattgatttacaataagagtctcacctcctgattttagtaatctcttgatgctaagaactattttgtcgattgtatcccgacaaggaacggcagagagaacattagagcaaaggatgaaatcgtaacccccaattattttgtcgacatcctcgaaagcaactgtatttgcatttttataatatcgtgggacatagtcaataattttagttttaattcctctaataatttgctctctttcaagttgccttttcgagtctagaaaagtaacttcatcaaatttactgattaattcatcagaatatctaagttttccgcagccaaaatcaagggcgtggccatttttctcaatgcttctaatatactcgcaaagatatctagagggcatcgtatgaggttttgctgcattctctgagcgaatattaactccgtgcatattatagttcaaagcaagtaccattcaattaatgttatttttagtgaaaaattcttttattttatcgtccgggatttttccgacttgactttcagttctgggcttaactgtcaaagcaaagataataccactcactgagaatgataaaattacaaaaaagaataaagacagcaaagaaccttcaacatgaaaaatatccatttgtttgcaaaaaaagattattaggaaggaaattaatgcaattatcgaaaattcaaaaaatatccaaaaatagtatactttattccagaagagttcaatataatgtttgtcttcaatttttcttacttcagggtaatatagattgctcattacattgtgagcttcatctttatttaattttctgttgactccagctctccgtgataacggttttataattagatgcttatcccaaagatatcgcacccgaagtagtttggctgcattgttatgtaggtctaacgcaccgctaattaaatatgcaaaaatcgcaaaagcacaaggtaatataccaaaagatagtgcccaattaataaagctctcatgatctttaataggtgggacatacttggttggtaatgttattaaagggatgtattcgtaaataactagaagtatgcaatatattagcgtatttaagaaagttgctttatgaagtttaggcaacatttcattataatttttggggggttcgaacatattattcacctgagtcacgctttaggatagtgtaatggtaatatttaattaagtgtcattatatacttttcagtaggttagttacaattttttgtatctgttcaggctgacctagcttcgctgacagacaatattgtgatcagtagcacgtatcgaggaggagtagcgctacaaatttgacgctgggtgagaatctgaaattgatagaaatgaaataatgaaataatgaaatgatgaaatgatgaaatgatgaaatgatgaaatgatgaaatgatgacagagtgtccagtgggcacggatggtgtcttacgacatgcttaccttaatcgttcccagtgtgcctatagcagatattctaaacatgtcgataattcattacgcatatagtatcgaacatagaaaaaactgaagattcatcttattttgtatatactacctagcccaacaatgtagaggttaacgaaaaatgcgctcaccaatttgtcatcttttctcagcaattaattcatcaccatttaagattgcaccagagaaggagcaagatcttaaaacgatagttgacgacaaaaaaattataatttcagttgtgagtgaacctggttttaatatccgagtcaggaagaatgagagtaataattcacatgaaatagttctaacagtagcttcacttgaatatatttgggcattttccaatttcttttgggtttttacgcaagagtactccaaatctcagaaaaataatgatgagcactttgatttaacaggaaaaaataggcttaaaaagtctgatgaacttcttaaatgggcaaggaaaaacttgcaaacaacaggttgcgaatcatggcctaaaaaatgtcccaagccagaagcatatttacaaggaagcgaagactcacaagttgctagcgagatatttctttgtgctattgcttggattcttcatcatgaaataagtcatgttgttttacagcatccattggtcactacagcattctccactcaagaggagcgtgaagcagattcacatgctacaaaatggatattaggcaacctgtatgaatccgctcctgaattaaagaaacgtgcacttggcattgctacggcagtgctttgtatacaaagcttagaagttgaaaattacttctgtttacaaaatacacacccagctgcatatgagcgtatatattcgaatatttcatgctaccctgtcggaaatgaagagttgattgaagctctatgtacagtgatgcttcaatatcttttccatggcaaaaatatcaatgtgaatctagatggggagtccttttcatcgattttaggtgatcttctctgtgatatttcacgtcttaccagtaactgatatggctgtccgccgctcgcttaaagtggactttttagtttttatcatgtgcggtgagaaattcaatgtggcgttgagatgcttaaaggttcacaacgctactttgctccatcctttacctcgatcatcatgataacgatcggtttgttgttgtgttttatgaccaagtagtttttgtgtgtctaacccctgttctttatacagacgttcagataaagacctttgctcatggaatgtcgcaggtgaaccctctccccagtcaattcttgctaaatctctcgctttactaaaattcatcgtcaatgtattggctttaacctgcgctccgcgctctgcttgtgaagttgaacgaaaaaaatgcactaagtatgcactgactgcatagtcacggcagcgggctactacatcgcgtaaactccagttaatcgcattgaggcgaagagaaagaggaattgcgattttgctcccggtcttttcctgaatgacatgaagatgatcatcccaaatatcgctaaatttcatacgcgaaatatcacctaaccgctgaccagtaaccagcgctaacagcatggcatttcccatgtaacgatgagtagcgtctgcgatatcgaagatttttttccattcttcaaggctcagccgttgtcgggtaatttttcttcttggttgtttagtggctaatgctgggttatagccaggaggtacttctccgtagtgctgcgcctctttgaaaacatcaatcaggacggagcgaactacttgtgccattcttggccgcccagcggcgatatactcatcaagcaattgtgctatatctctgacatcaacggctgagatcaacttcattcctgctcgttctctgagcaaggatactggtttagctttttgtttataggtgttgagtcttatatcaccacttttaagcctgtcatcctggatcgcttgatagcgatctaaccaggttgacgttgtgatagcctttcctttgctggttgcgatcctgtcactgatagccagaatctgccgggttctttgttcagccaggcgagtgttggcctcagtggcaatagcgatagcttcagcttcgtttgttcccaaagcatggaattttcctgtcactggatgcttataccgccaatagactttatttaccttcctactataaagcggatataagttagggactgaaacattattcttacgcggtctggctgccattactcaaaatccgttgcaaaagtaatgagtcatttttcttgattacaggtgttaccaactccccaactaactcggcgtcctcacgcactcgccataaccggccttgtttcatggccggtggacaaaataaattctgcttagcataacgacgcaatgtggacacacttggaggattacttctgtatttttcagcagcccattcttcaagagttaacatttgaagcatatgcgatcaccttattactacactaactgcttagtctcagcatatcgaccctgcacggtcggttagtttctccacaaaacagagaagagcacctgtggccacagctatcaggatgggtcgggttattaacccgtcatccggggatactcttctctgttttgtaaaaagggcggtaccagaaaggactaaggaaaaaactggtaccgccaagactacacacagcataaagttgtggtgtcgggtgcccccggtgcctggcgaaggttgcacaccaggcgggtgggtatccacagaaggtcgattgtcagcctcaaccttaacccgcgtgcgctgagccgcattcaccacaacgctaaggattctctctggttgaaaatacttagctgttatgtgcctgtcttttcaccacttcaggctcggtggtatgctggagttctcacacagccagcaagcaaggaaacttaatgaaccagttttatgttcacgttcgtctatttgaagacacagccgaacagaccaaaaaatttgaagaattaatgcttaactttctgtaccagaaaacagttaaagagtctgacgatagctgctgcagactgattccagagggatatatcctcaaaagtacaatgaactgccaacaaatccttgatcaaacattttcaattgctaacagtgccggtgttgacgcaaatatatttgtctgtaaatttgaacaaagcgcatgcttacttccgtctgcttccttagttggtaacgatttcgttcattacgatcttacgcctaagcccatcaagctcgattcttaaagccttaaccattgtgtcgtgataaacacggctcaccttctctccattgcatggcagaggggtgagtgtgttagccatgaaattcatgaactcggttcgaccaggggcttgcgccccgcaagtctttaatgcctgttttgctaacaaaatgcgggcctcagtgcctgcatttggctctatctgctgcaaacgtttagcgtcttccagcaacaatgcgatcacatgcttcaaattctgctcattcatctattctctccactgaaatcatccgctaacgaatcatcccggtcttcgtacgtaccgggcgggctacttcgtgggcgtcctgcctgtttgttgtttctcttgggtacattatgtatctcaaaggtacattgtcaagtataaaaaaacctgccgaagcaggttcataaacattgattaggctttgattttgtatcttcttggttttcctgagaaaatcacagtaccaattatagagcaattaccgttgatcttaatgtaaggctcaggccagtttgggtttaacgctttgagataacgctgtgtcccatcttctatcaaccttttgaaggtggtttcacctgtatcgtgcatcaatgcaataacgtcgtcaccgtggcaggcaggtacttcaggatcgacaaaaatcatgtctcccgggcggtactcatcaatcattgaatcacctattacccgcaagatataagtcatttccccacagggtacagggcagggatacgtttctgctgtgctcaaatcaacctcagaatatccaacttctttccatgctccggcctgtacccatgatatgacagggactaatgtgatttgtttattagtgattgaaacatcaggtttttttgtgatgttcgttgtctggtgttcttgatcgagccatcctacaggcaggtcgaaacatttttcgatgtgtcgtgccatgctgtcaccgatatttttagtagcaccatctcccataaacctgctggtctgggttggctcgcgatcaatcatagtggcaaaggaagaattcccgccaacaccatctctcagttttctggcgttagaccgccggatgtcatggattgttttcataacgaaattaaaacccttgtaccgttaaggtacaagtatcttgaaggttcatttcaatcatgtaatatgtacaccggaggtacatattgtatgaaagcgtattgggactctttaaccaaagaacagcagggcgagttggccggaaaagttggctcaacacctggctacttacggctggttttcaatggctataaaaaagccagttttgtgctggctaaaaaacttgagcaatacacatcaggtgcaattacgaaatctgacttaagaccggatatctatccgaaagattagcagaacactttcaatttttaaccacagaacgatgaggctaatcgtgggtaagcatcactggaaaatagaaaaacagcctgagtggtacgtgaaagctgtcagaaaaactatcgcggcgttgccgagtggttacgctgaagcggctgactggctcgatgtaacagaaaacgctttattcaaccgccttcgtgcagatggcgatcagattttcccgctgggatgggcaatggttttacagcgtgctggtggcactcacttcattgctgatgctgtggcgcagtctgcaaatggcgtctttgtgtctcttcctgacgtcgaggatgtggacaacgccgatattaaccagcgtctgctggaagtcattgaacagatcggcagttattcaaaacagattcgttcagcaatcgaagacggtgtagtggaaccgcatgagaagacagcaattaacgacgagctgtatctctcaatttcgaagctgcaggagcatgcagcacttgtctacaaaattttttgcatttcagaaagtaatgacgcccgcgagtgtgcagctccgggcgtcgtggcgtcgattgcttctggttgtggagaaactaacgcatgaacagtttaacaacacactaccgtcgctcgcaactgattgcgcttcctgtaccgggtggaaaagcgaaggtggaatattgctatgcagtgaatgtaccaggtgacagggaaattgtaacccacagctttgcagagtgggctgtgggtgatttcaaccggcagaaggagacagtcctttgcgacaagttaaccgctggttcaaagatcactacggagtgcccgtcagagtcattcgttgggagccggaaacacaacgggttatctacctccgcgaaggttatgagcatgaatgcttcagcccgctcgaacagtttcgtcgtaaattcagggaaatagaggtcggtcatgagcactaaattaaccggctatgtatgggatggttgcgctgcatcaggcatgaagttatccagcgtggcaattatggcccgcctggctgatttcagtaatgacgaaggtgtgtgctggccatcaattgaaaccattgcccgtcagattggcgcggggatgagtaccgtcagaacggctatcgcacggctggaagcagaaggctggttaacgcgtaaggcgcgtcgccagggtgatggttcatcaccccactgtgccgtggtggatgaatatcacgagcacgccacagatgcgctttacaccacgatgcttaccgggatgggggcgcgacgccagccactgatgtgggccattaccaccgccgggtacaacattgaggggccgtgctacgacaaacggcgggaagtcatcgagatgctcaacggctcggtgccaaacgatgaactgttcgggatcatctataccgttgatgaaggtgacgactggaccgacccgcaggtgctggaaaaagccaatccaaatattggcgtgtcggtttatcgcgaatttttgttaagtcagcagcagcgtgcgaaaaataacgcccgtctggcaaacgtctttaaaacaaaacacctcaatatctgggcgtcggcgcgttcggcgtatttcaacctggtgagctggcagagctgcgaggataaatcactgacccttgagcagttcgaggggcagccgtgcattctggcctttgacctggcgcgtaagctggatatgaacagcatggcgcgactttatacccgcgagattgacggtaaaacgcattactacagtgtggccccgcgtttctgggtaccgtatgacacggtgtacagcgtcgagaaaaatgaagatcgccggacagccgaacgctttcagaaatgggtggaaatgggcgttctgaccgttaccgatggtgcggaggtggattatcgctacatcctcgaagaggccaaagcggcgaacaaaatcagcccggtcagtgagtcacccatcgaccccttcggggcgaccgggctgtcacatgaccttgctgatgaagacctgaaccccgtcaccatcattcagaactacaccaacatgtccgatccgatgaaagagctggaagcggcgattgaatcggggcgctttcatcatgacggcaatcccatcatgacctggtgtatcggcaacgtggtcggcaaaaccattccgggtaacgatgatgtggtgaagcccgtcaaggagcaggcggaaaacaaaatcgatggtgcagttgcgctgattatggcggttggcagagccatgctgtacgagaaagaagacacgctgtctgatcacattgagtcctacgggatccgctcgctttaactgaggtaattatgatcatgctgattctcgcgcctctggtgggcgtgctgggtgcgcttttgctggcgtatggtgcctggctgatttatcccccggcgggttttgttgttgccggggcgctgtgcctgttctggtcgtggctggtggcgcgatatctcgaccgtacacagtcgtctgtcggcggaggtaaatagtgttcttttcgggattatttcaacgaaaaagtgacgcaccggtgaccacgccagcagagctggcggatgccatcgggctgtcgtatgacacctataccggaaagcagatcagcagtcagcgggctatgcgactgacggcggttttttcctgcgtcagagtgctggcagagtcggtcgggatgttgccctgcaatctgtatcacctgaacggcagcctgaagcagagagccaccggcgaacgtctgcataaactgatctccacgcatcccaatggctatatgacgccgcaggagttctgggagctggtggtcacctgtctgtgcctgaggggaaacttttacgcctacaaagtgaaagcatttggcgaagtggctgaactgctgcccgtcgatcccggctgtgtggtatatgcgctgggaaggtgtcagcgatggcctgaaggtgaccgccgggagtgttattcagcgcgatgacctggtgcagtacacgacaactgacgatgcaaccagctccggtggtgtcctgcgcgtgccgatcgcctgctcaagtgcaggtgcggtcggtaacgctgacgacggtacggcattaatcctggtcacgccggtgaatggtctgccgtcttccggtgtggctgacaccctgacaggcggatttgatactgaagagctggaaacgtggcgcgcccgcgtcattgagcggtattactggacgccgcagggcggggctgacggggactatgtcgtctgggctaaagaagtgcccggcattacccgcgcatggacataccgtcacttgatgggaacgggaactgtcggtgtgatgattgccagcagtgacctgattaatcccattccggaagaatcaacggaaacggcggcaagacaacatatcgggccactggccccggtggcaggctctgatttgtatgtgttcaggccggtggcacatacggtggattttcatatccgcgtgacgccggacacaccagaaatacgggctgccattaccgcggagttgcgttcgttcctgctgcgtgatggttatccgcagggagaactcaaggtatcgcgtatcagtgaggcgatttccggtgcgaacggggaatacagccatcagttgcttgcaccggtggacaatatctccattgcgaaaaacgaactggcggtactggggacgatttcatggacgtgacaaacgatgattacatccgcctgttatcggcactgttgccgcccggtccggtgtggtcagccagcgatccggcgattgccggtgcggcaccgtcattaacccgtgttcatcagcgtgcggatgccctgatgcgggagctggatccgcgcaccaccactgaactgataaaccgctgggagcgtctgtgcggtctgccggatgaatgtattccggcgggaacgcagacccttcgccagcgtcagcaacggctggatgcgaaggttaacctggcgggcggcatcaacgaggatttttatcttgcacagcttgctgccctgggcagaccagatgccaccatcacgcgatacgacaaaagcactttcacctgctcatcggcctgtactgacgcggtgaatgcgccggaatggcggtattactggcaggtcaacatgccagccaccaccaactccacctggatgacatgtggcgatccctgtgattccgcactgcgtatctggggtgacaccgttgtcgagtgtgtgcttaacaaactctgcccgtcgcatacctacgtaatttttaaatatccggagtaatccatgcatcgtatagacacgaaaaccgcgcagaaggataagttcggcgcgggtaagaacggttttacccgtggtaacccccagaccggcacgcctgccaccgatctggatgatgactactttgacatgttgcaggaggaactttgcagcgtggtggaggcatccggtgccagcctggagaaggggcggcacgaccagttacttaccgcacttcgcgcgctgctgttaagccgcaagaatccgtttggcgatatcaaatcggatggcactgtgcaaacggctctcgaaaaccttggtttgggagaaggagcaaaactcaatgcagcaacggctacattaggacgcaccggtttcatagctataccggttatgattggtggtattgagcaatcagtaatcattcagtgggggtggaatgccgcaaaagcatctgcctctgggggggatggaaatacagttgtattcccggttgcgtttaataatgcctgtgttgccgttgttgcaaattatgacaatgtcagcgcacctatcaatgcagtggcaacggggggatatacaaccacttcgtttttattacggtgcgcagctcaaacgggtagttattactataactggattgctattgggtattaagatgaaaatatactgttgcttaaataccgttggtttttttatggatggctgtggcgtcattccgccagattctaaagaaataacggcagaacactggcagtcattattaaaatctcaagctgaaggaggcgtgatcgatttttctgtttttcctccttctattaaagaggttatccgtactcatgatgatgaagtcgcagatgcgaactttcaaaagcagatgcttatctctgatgcaactgattttatcaatagcagacagtggcagggtaaggctgcattgggaagacttaaagaagatgagctgaaacaatataatttgtggctggattatctggaagcactggaactggttgatacatccagtgcgccagatattgaatggcctacgcctccggcagttcaggccagatgacatccggcgcggtgctggtatctgttgccgtcaccgcgtcaatgtaatccagcacagcgttaagtctggttgtttctgcctgcgtcagtttacgtccggcctgcaatttcagttgaatcagactaatggaagccattgcagcatcaatcagtgactggcgctgtgcttctgccgcgtctactgcggcgctatgctgtgcttcagtatcggtcacccatttctcaccatcccatttatcgtatggagataaaggggcgatagtggttgtattttcagggtaatcacccggagctttgatttcttttgattctccagttttggtgctatagaccgtttcaccgcgatggtctggcacatattcccatgagttaaaatctgcagaacggcagattgcataaccagccttatgtgtaccaggggcatctaaacaggaacatgccggaatgccgacaccaacggcaagatattcatttgaagtggaaatatattcccgtgtttcaccatcgtagttataaacggtaacatcccctgcctttgttgcaataaggtcactatttaatattgctttatgcatcaggctgccctcacgatatagttaaatgcaatattacgcggacgcgtttctgaggctgcggcacctaaaccatccactgattgtttatatgttttaaaggttccataatccggggctggtaatccggcatcgtttgtgtttcctcttttgataatgtcagtgccactatttacccatatttcatcaaaatagaaattaatcgttgcatcagtcacaatcgtggatcttgacggtaatccatgagcatgatcctccgttgcatacccctgaatacttaaaatagagcgacctgtatcaatcccccgcccgtcatcccagccacgaataaactcaccacgtaaatcaggcaatttatttgtcggataagcctttgccagttccgggtattcttcagcagaaaaagcggcaccattgcatttcagccagcctgttggcggagtggctgaaggccacggaaccgggacaccaacaggtaatgcagagccttctcccaaaccaacgtttatgaaaatgaagaaataacaagcaaatggcatcattcctgcttttaccagggggatttaacatgcttattggctatgtacgcgtatcaacaaatgaccagaacacagatctacaacgtaatgcgctgaactgtgcaggatgcgagctgatttttgaagacaagataagcggcacaaagtccgaaaggccgggactgaaaaaactgctcaggacattatcggcaggtgacactctggttgtctggaagctggatcggctggggcgtagtatgcggcatcttgtcgtgctggtggaggagttgcgcgaacgaggcatcaactttcgtagtctgacggattcaattgataccagcacaccaatgggacgctttttctttcatgtgatgggtgccctggctgaaatggagcgtgaactgattgttgaacgaacaaaagctggactggaaactgctcgtgcacagggacgaattggtggacgtcgtcccaaacttacaccagaacaatgggcacaagctggacgattaattgcagcaggaactcctcgccagaaggtggcgattatctatgatgttggtgtgtcaactttgtataagaggtttcctgcaggggataaataaagttaaagacactttgtgtacaaaagaaagtaaaacaacagcaacttgttgcaattttatcaataaaagtagtattgtcgtgaaaaattgattaaagattaatattatgcatgtttttgataataatggaattgaactgaaagctgagtgttcgataggtgaagaggatggtgtttatggtctaatccttgagtcgtgggggccgggtgacagaaacaaagattacaatatcgctcttgattatatcattgaacggttggttgattctggtgtatcccaagtcgtagtatatctggcgtcatcatcagtcagaaaacatatgcattctttggatgaaagaaaaatccatcctggtgaatattttactttgattggtaatagcccccgcgatatacgcttgaagatgtgtggttatcaggcttattttagtcgtacggggagaaaggaaattccttccggcaatagaacgaaacgaatattgataaatgttccaggtatttatagtgacagtttttgggcgtctataatacgtggagaactatcagagctttcacagcctacagatgatgaatcgcttctgaatatgagggttagtaaattaattaagaaaacgttgagtcaacccgagggctccaggaaaccagttgaggtagaaagactacaaaaagtttatgtccgagacccgatggtaaaagcttggattttacagcaaagtaaaggtatatgtgaaaactgtggtaaaaatgctccgttttatttaaatgatggaaacccatatttggaagtacatcatgtaattcccctgtcttcaggtggtgctgatacaacagataactgtgttgccctttgtccgaattgccatagagaattgcactatagtaaaaatgcaaaagaactaatcgagatgctttacgttaatataaaccgattacagaaataaaattatttattaaagtcacatttaagacgtaataccctacagggtaaaaattttctctgatcttaacttctgcaaatgttaactgctatttttatgctaaaaatggttatcaaaactcaaaaacacatgtttataatcaatgagttatagaaatgctaagggctaatgagttatatgcaaattagtaaaattatgttgctatgtcagatagttacgatttagtcatctaactaatgctgcgccatatgggttggactgaagcggctgacctgattgttaaaggtatggaaggcgcaatcaatgccaagaccgtaacttatgacttcgaacgtctgatggaaggcgctaagctgctgaaatgttcagagtttggtgaagcgatcatcgaaaacatgtaatctctccatgtgttaaatattgaaacgggcgtataacacgcccgttgttttatttatgtggatattattaatagcatatcgagcatatttatatgaagcccattacttgagcccatatgggcatatttttataatgcaactattatgtaaacatttatttgttattttgctttctcctggaggacactcttgactgcttttgagtaaactccataaatccttgttgaatggtgcgatgtgataaatagtaataggatattctttatccttaaggataataccagacttaaccggtgtaaatatactgccaggagggagaaatatagtagattgataccagatgatcattttcatattaccccatatggctgaaaaagatataccacatgtaggttgaattaccgtgtcaattactatccacttcatttgttatgtcttatcccacggtatttaatatggttcattaggatgtttatttcttgattttgcatatgagtatattacccccccctcaaaaaaataaattaattaaaatgatggcttatataaaataaaatttaaagcaaggaatctcaatggatgttaaacaaaatgagattttgtgaaagcaataaattattgacttcgttttagatttgtttagctataatgttatacattcaaatgactgaacatcctgtaattaaaacatagcctttatgctactttgtgccaatttgctaaacattatggttgcctttttatataacgataataatgaatataagcatgacatgagaataaggtttcaatttttgagttatataggaatgatttaacctgttcctggctaaaatacatataaccggatgatgactaaaccaaaatacatgtgcgttaagtattgaaacggacgtgtggcacggccgttgtttttataaatatgttaaccgttataaaataacgtatcaaaagtcaagtgatcacatttcaaatatcaagttgatagtattagtctggtgattatttatgggtgacaataaaaagacagtattaatcatccatagagatagtctctgcacttttatttccattatgctaatgccttactgaattatgaagcatttcttaagtatccaactttagctagattaatggtttattattttctacatcttcaatatataaaagcgtattatcaatggcgtagtaactgcgtttgttatgattaacatcagtaacccaccggaaaacgcccgcgcctgccagtgttgaacagtattcccgaaatgtagattttccgcaaatatgaagcaatgcggcctcttttattttagcagggttcttggtcgtactaacttttaacaggttcctggttcctcttaataacaaaaccgtatcatcgtgagtaataattctgatgttatccgtagccagataataaatgtaatgtgcaatacggtgatgttttaattctgaataaaaccaggagaagttttgctcttttctcacttgctcaaacatcttttgaaaaacaacgacctgatccatcaggataataacctcttgttagttgtgagactgcgtagtgtgcacgatcggttttaccacttcaatctggtctgtcctttggctgtgatatgtacagagtgtgatagagggaatatctgaattctcccggtgagcattttgcaacggaccagctccggtacaaacgctgttgtgggttcagattataacattctgtctaaggggcgggataaaggtgaaattagggggcatgaaagatgactttataaccttgctcaccccagtgttgtaaaagttcgttttgccttctcgttggtgccatgcctgtccagacaatcaatgtttgcgtcgggaacagttccgggcgcggcgattcaatgggatcagcaagaacagaaatgtgccatcctgacaatgataaacgccatgcttccagccacaatcgtgctctctcttcaacattccacgccatcagaatggcttctttaccgggcttacggcgcatttcgaaaagcgaggttgctgcgtattcaattaatgcgccgtcaaacatactgctcataatgcgggaggtgttgtgatcaagcacgagacgctggcgaacaggaaggtaaacatgattaatcaattgatctactgggtactctcgacccagtgaaataattctcgcgcgtagtttggcaggattagccatgcgaagaattgacatcatctcttcttgcaggcggctccagtcatcttccgtatcctggctggtggtttccagtaatgctttaactttgcctacagggacgccattacttatccaacgcttgatctcttcgatgcgttgtatgtcttcttcatcaaagagtcggtgtccgccttcactgcgctgtggttttaacaaaccgtagcggcgttgccaggcccggagagtgacaggattaatcccgcaacgttcagcaacatcaccaatgctgtaataagccacaattcctccttgcggtcacaaatctccgtcgcctgtacacgacccaataatactttgtacaatatacgctaaaattgtacaaagtataaataagatttcagctaaattggatgaaacattatttttaatgtggattaaatttaaacgtaacgtattcattttcacgatgatttactgaaatcatgtgaaagaatgtgctgaaaattattttttctctggccacgctatggaagggataccattcaatttagctttagcaaacagatctccctgaaacatctcaattcctgcggattcaagccacatccactcttctggtgttgccacgcccatagcactgacttgaatttcaagtgatgtacagcattttatgatcgcctgaataattgcctgccgtggcccacttttatgaacattggtaatcaattcctgactgattttaattctgtcaggctggaagcgtgacaggagtaacaaaccagcaaaacctgcgccaaaatgatcaattgctacactgataccagcagcctttagcgatttaatcgcttcggcaaactcatcaaaccgagatatgacttcactttcagtaaattcaacgatgatttgttcaggcaccagagcattggcctttatttcattaagtaaaaaagagactgcgtcaggttcgttaaccagggtcataggtaatagattgattgaaatcattttatcaccgagctcaagtgcgtgtgccatcgtgaatgcaagcgccttacttttgagatccgctgtgtagatttccccgtctttacgctgcccaaccgctatggctgatgggctatcttcatttttttgcacaatggcttcaaaagcgattatccgccgcgataagggatcgacaataggatgaaaggcaaagtggtcgtttatagttggtgaaagggcacaggaatcaagttctttatcagatccgtcagcgataaaaagccaggagtcttcggcagggatctcgaaataggttgattgttcggttgcaaggacaaaagtacgaaaaaattgtagcgctctgtcatcataagttagctgaaattttgatgtgcctttgtcgaatacggcctgtaaaacgtcatctcgctcgtgcaggcgcaaatcaaataattccattcccgctttgccaaaacggcgagcaggcgcgtaatcgcacagcagctcaacaatattatagtgccgtggatcctggcatatagcccgatatatcattttaacctgttcttccggaccttccagaagctggaaaaaatgagaaccattaaacagtaagatccctgttacgtcagactgcatgttcctgcgatttgctatcgaaaccatttcttcgatttttttgacaggttcgtcgtcacgtatatggctacgataaataagggtggtaagcattaacaatccagggtaatgggtgaggcgagagtaagacggtaacagacatatcttcttgtgtctttcttttaataccaaaacataaccgtttctttacattgataaaaaatggaaaaagttgaacactagttggcgaaaaatcttgtatagattgtcagttaaatgatgcaatatgttttatcataacacattgttttatatgcattagcactaattgcaaaaaattaatttatcattctgtacacatatttcgtacaagtttgctattgttacttcacttaacattgattaacatttttaacagaggcgtagcatgcatcaaaattcagtgactttagattctgcgggagcaatcactcgttactttgcaaaagctaacttgcatactcagcaggaaactctcggggaaattgtgactgagattttgaaagatggacgtaatctgagtcgaaagtcgctttgtgccaaacttctttgccgactggaacacgcgactggggaagaggaacagaaacattataatgcactaattgggttgctttttgaataatgcaacagcctgattatttaacaggttagctatgaagtcgttatgaagacatctgataatgaacgtataaaatatgaaattactggccaggcggtgctccagatactgcgcatgaagataaatttttcattgcagactcttattaagcaattactcgtaatgaaatcggctgaggaagatgctttccgacgcgatttaattgacagcataattcgtgattttagcaatagtgattcaggagggccaaaccgaagaacagcgacagctgacaataaaagtatgttcaatggtaagaaaataaacagaatacattaaaatttcataagtaagatgagaggttaccatgcttgaagatactacaattcataatgcaataactgataaagcgttagcaagttactttcgcagttcgggtaatttgttagaagaagaatcagcagtgttagggcaggctgtcaccaatttaatgctttcaggcgataatgttaataataaaaatattatcttaagtctgatacactccttggaaacaacaagtgatattctcaaagctgatgtgattagaaaaacactggaaatcgtgttgcgatacacagctgatgatatgtaacttctaattattaagtataagtttatagaaaactcattcatcttatttttgtctgtcgctttagactatacacagcataattttattgggttaatatttctacgaggctgacatgaataattcaatcccagagagatttatttttcaatgtgctttgtttaaaaatctcgagagggaggtgttcatgacgcatgggtatgttgatagtcatattattgatcaggctttacgcttgcgtttaaaagatgaaaccagtgtgattctttctgatctctatctgcaaatattgcagtacattgaaatgcataagactacactaacggatatcattattaatgacagggaatccgtgctctcttagaacttgagtaaggttttagaataaacatcagctgtatcaccatgctgatgcaaagtgagcatttcaggcgttatgctttcttattatgtccgcaatatcaggtgtcaagaatggagagttctcgctctccattcttgacgcctgatatcccgcctaacttattttgtactgcctacattatgctcaataattaatgggttagatcaagatggagaaaattttatcttcggcgtggatatttcttatgctctctaccatgctctctgtagatgccagcgcgagcgaatgaatggcattttcatgtattaaaccctttggccgggacaagcaaatgcgcaatacactcatacccatcctcgttgcgatatgcttgtttattaccggtgtcgctattttgaacatccagctctggtattccgcaaaagcagagtacctggcgggagcgagatatgccgccaacaatatcaatcatatacttgaagaagcgtcacaagcgactcaaacagcggttaacattgccgggaaggaatgcaacctcgaggagcaatatcagcttggcactgaagcagctctgaaacctcacctgcgcacaatcatcattctcaaacagggaatagtctggtgtacatccctgcctgggaatcgggtcctgttgtctcgtattcctgttttcccggacagtaatttactgttggctccagcaatcgacaccgttaatagattacctatcctgctctatcagaaccaatttgcagatacgcgcattttggttacgataagcgatcagcatattcgtggggcacttaatgtacccttgaaaggggtaaggtatgtattacgcgtggcggatgacattattggaccaacgggtgatgtgatgacgcttaatggacattatccctataccgagaaggttcactccacaaaatatcatttcactattatctttaacccgccgccactctttagcttctacagacttatcgataaaggctttgggattttaatatttattctgttaatcgcctgcgccgctgccttcctgcttgatagatatttcaataaaagcgcaacgcctgaagagatcctgcgacgggcaataaataatggggagatcgtccctttttaccaacctgtggtaaatggtcgggaagggacattgcggggagttgaggtgttagcccgctggaaacaacctcacggtggatatatatcacccgcggcatttattccacttgctgaaaaatccggattaatcgttccgcttacgcaaagcctgatgaatcaggttgccagacagatgaacgctatcgcgagtaaattgccggaaggttttcatattggaattaattttagcgcttcgcatattatttcgccgacgtttgtcgacgagtgtttaaatttccgtgacagttttacccgccgcgatttaaaccttgttctggaagtcaccgagcgtgagccattgaatgttgatgaaagtctggttcagcggttgaacatactgcatgaaaatggttttgtcatcgcactggatgatttcggtactggctactcagggctttcttatcttcatgacctgcatattgattatatcaaaattgatcacagtttcgttggccgcgtaaacgcagacccagaatcaacccgaattctggattgtgtattggatctggcgcgtaaactttcgatcagtatcgtcgctgaaggtgtcgaaacgaaagaacaacttgactatctgaaccaaaattatatcacatttcagcagggttattatttctataaacctgttacatacatcgacctggtcaaaattatcctttctaaaccgaaggtgaaggttgtggttgagtgaaaattgatcagtaaggccatagtgcggtgtaattatagacagctaattagctcgttgcctcttgttactattgttcattattttgtttgctataattgtttgaaagttttgacaggattgccattagtagcatgaacaatagtaataatctggattatttcactctctatatcatattttccattgcatttatgctgatcaccctcctggtcatccttattgcaaaacccagtaccgggctgggagaagtgcttgtgacgataaatttgcttaatgcccttgtttggctggcgatcaatctggttaatcgattaagagaaagactcgtcaaccacagggatcagcaataatctttcagtttctcactgtcagtatgcggctgaatgggttgctggcagtgaacgcctggatcattgaaggaaaggcattattgcgcaaatagttgtcaaccctggtgttatcacggttgtttttatatatcaccgaaataatcctcatcgcaactattaacaattttgatgtcgaagagttatttgttaaacaaaatcgtcacctcaaagtgatcaatgtcatgaaaataaggtgaaaaatgataatgccgacttatttatcatttatatattgtcgctgtttatctatttaaattttttgtgcttttgtttttgtctttaccctccgttttggtaatctgagctcataggttatttgaccaggaatgtttgttaatccaatgaatggatggttaatctatgaaactgaaaaaactccccgggtttagtttgggacttattgctctggcggtgggtaatgcatatgcaacacaattgttggatgattatagtataatttcctatatgactgatgaagaatcgccgattgaaatcaaagataataatccgataagtaatggagagtatctaaccactgaagacgaaagccatgctgtgaaagtggatgacggtgtaactggatatataaataatgccagtgtgatgactagtggtgatggatcttatggtatttctgttgatagtcaaaacaaagtattatatataagcgatagcgatattaagacctctggaagcgtatctgacaaagaaaatggagggataacagccagcgcagtagtcagtgaatttggtggcaccatctttatgaatggtgataattcagtcgagtcgggtggggcatattcagcgggacttttaagccaggttaatgattctgaaaagatggtaaataacacccgtcttgaaaccacagataaaacgaacattgttacctctggggaaaatgcagtaggtgttcttgcatgttcaagtcctggagagtctcgaacatgtgtcgatgctgtagatgatgaagttagtgattctaacagttacgaagttattagccgtgctgatttaaaaatgaatggtggttccataacaactaatggcattaatagctatggtgcttatgctaatgggaaaaaagcatatattaatttagattatgtggcacttgaaactgtggctgatggaagttatgcagttgctattcgacaaggtaacattgatataaaaaatagttctattacaacaacaggcactaaagcccccattgcaaaaatatacaatggtggagagttatttttttccaatgtcaccgcggtatcaaaacaagataaaggaatatcaattgatgcatcaaatatcgattctcaagccaaaatagcactattaagtgttgaactttcaagtgctttggatagtattgatgttaacaaaactacaacggatgtaagtatccttaatcgaagtattatcacacctggtaataatgttctggttaataatactggaggtgacttaaacataatttcgtccgactctattctaaatggagcgactaaactcgtcagcggcacaaccacgctgaagctttcagaaaatacaatctggaatatgaaagatgactccgttgttacccatctgactaattcagacagtattatcaatctttcgtatgatgatggtcaaacatttacccaaggaaaaacattaaccgtaaaaggtaattatgtcggtaataatggtcagcttaatatccgcaccgtattaggtgatgataaatcggctacggacagacttattgttgagggtaatacttcgggttcaactaccgtctatgtgaaaaatgctggaggaagcggcgcggccacgctaaacgggatcgaactcataactgtgaatggcgatgaatctccagcagatgccttcagataaggtgatgcaaggattgcagctggagctttcgaatatcaactaaaacaacaaggcaaaaactggtatttgacaagttatcagtcagtgaatgaggaggataacagctcagagggaaattcagaatcaacagaaacgcctacccccgtcctgcgccccgaagctggaagttacgtcgctaacctggcagctgctaacactctttttgttatgcgtctgaacgaccgtgcgggtgaaacgcgctacatcgatcctgtaactgaacaggagcgttcaagccgactttggctacgtcaaattggcgggcataatgcctggcgtgacagcaacggacagttgagaacgacctcgcatcgctacgtctcgcagttagggggcgatctgttaaccggtggttttaccgatagtgacagttggcgtttgggagtgatggctggttatgcccgcgactacaacttaactcattccagcgtgtcggattatcgttcgaaagggagtgtcagaggctatagcgcagggctgtatgccacctggtttgccgatgacatcagtaaaaaaggcgcatacattgactcctgggcgcaatatagctggtttaaaaactcggtgaaaggggatgaattagcctatgaatcctatagcgcgaaaggtgcaaccgtctcgctggaagcgggttacggttttgccctgaataaatcctttggtctggaagcggcgaaatatacgtggatcttccagccacaggcacaggctatctggatgggcgtcgatcataatgcgcacacggaagccaatggctcacgtattgagaatgacgcaaataacaacatccagacccgactcggcttccgcacctttattcgtactcaggagaaaaacagcggtccgcacggtgacgactttgaaccttttgttgaaatgaactggatccataacagtaaagattttgctgtctcaatgaacggtgtgaaagtcgaacaagatggggcgagtaatttgggggaaattaaacttggcgtaaatggcaacctgaatccagcggccagcgtctggggaatgtgggcgtgcagctgggtgataatggctacaatgacaccgcagtgatggtgggcctgaaatataagttctgatcccgccgttagctaaaaaaccgcgtcgtattcatcgacgcggtacatatgaaatattattttttgccgatagcacgcatggtgtcatcaattgccgtgatcaacagcatttgcgggtctttagcgcaaacctgattcagtttttctaccactttggcgctcagttccggagattgctcaatttttaaatcacggctggcaacgctggcattacccattaccgcaacaatttctgcaacctgtgcgctgtcagtttttgccatttcgttggcttctgcgcaagtaatataggtttctgacggcaaaccgtttttaatattgtagtcctgcgcccaggtcattggtgcgaaaacaaacaggcccgccagtaaagcaaattttttcatcatcattccttatttcattttacccagaattgcaccacccgtaccgccaatcacggcacctttaatcgccccttcgaggccattgccggtcagaacgccagtgacagcaccaacggcggcacccacttttgcacctttacgcgcatttttaccgtcgcggcctttttctgttactgcaccaacaccagcgccaacagctgcacctttcagtacgccattaacaccattgccagtaagtaaaccaacgcctgcgcctagcaatgcacctttcgtggtgcggttcatatccgccatcgctggcgtggagcagaacaatgctgagataagcccgaaggcaagtatttttttcttcaacttagatgtccggtattaagtaagttgcacacacaataatttcgtcttcaattaagatctgcttaactaaagaacgctcgctattattcagataattcaaaatgagcgtggctgtgatgataggaattatgttttttacgtgaatgagaataatcttaaatgaggaataactcattgattgacaatatttttattcaagaagtgtcattgactgttaacgcaatgttgtaaaggtaagataatctgatttatcaatattattgtgtgatttttatgtgagcagaagatattcatcagcaacgattacattagtcattttattttgccgacggcctcattgtcgaaagataagcgtacgacagtattatcagaaaagagtgattttttatccaactacacttcagcgcactgcgtgtaaaaaatgcctctttcttatgcgggatatcatcatttcatcatgatgtctttggtgagcggtgaacacaatacacctgcgctgtctcttcaggatgaatcccctggtctggtgcctgcgggctgatgttgcagcagagcttaggtcacttagacgctactatcatttatccaatggcatggaatcgaaatcagtcgatacccgcagtatatatcgtgaactgggtgcaacgctgagttacaacatgcgcctggggaacggtatggaaatgaaccctggctgaaggcggctgtgcgcaaagaatttgtcgatgataaccgggtgaaggtgaataatgacggtaatttcgtcaatgatttgtcgggcagacgtggaatataccaggcagctattaaagcctcattcagcagtacgtttagcggacatctcggggtggggtatagccatggtgccggtgtggaatccccgtggaacgcggtggctggtgtgaactggtcgttctgaccatcaacgattaaactgcgcttcggcgcagttttcgtttacaggatgttgaaagggaaaattctggggcaaaaaaagcccgccagttacggcgggaaacctcatcctatgggagaacaatgaataatgaaattgcggggttatcatctcccagtatatccatactaacaataaggttatttactcaaccaggcataaacattttgttttgtgcgtgggaacagccttaaggtgtaaagggggaggtggaaatagcaatgaggagtatcagcaagaatactcgccgctttaccacaacgtggatgagagggatgaaaaactcaaggcagagataactctgccttgaagataaatgcgcttttacagcgggcttatttcagctcttctgcttccggtaaggtcacgttcagctcaagaatagaaatatcgccatctttttgctcaagctgtacggttaccatctcaggatcaatttgtacgtatttacaaatgacctcaagaatatctttacgcaactgcggcagataatgcggttctgcatcgctgcgacggcgttcagcaacaataatctgcagccgttcttttgcaatgttggctgtgtttttcttccgcgagagaaagaaatcgagtaatgccataacttatcctccgaacaagcgtttgaggaagcctttcttctcttcttcaatgaagcggaaaggacgttcttctcccaacagacgttctacggtatctgcgtaggctttacccgcatcggcgttaatgtcgagaatgaccggttcaccctggttagaggcgcgcaatactgattgatcctctgggatcacgccgacgagtttgatgcgcaggatctccagcacatcttccatgctcagcatgtcacctctgcttacgcggcctgggttatagcgcgttaacagcaggtgctctttaataggctcttcgccattttctgcgcggcgtgatttcgacgccagaatgcctaaaatacggtcagagtcgcgtactgaggagacttccgggttggtggtaataatggcttcgtctgcaaaatagagtgccattaacgcaccggtttcaatccctgccggggagtcacaaacgataaattcaaaatccatcgctttcagatcatcaagaactttggcgaccccttcacgggtgagggcatctttatcgcgtgtttgcgatgccggcagaatatagagattttcagtacgcttatctttaattaacgcctgatttagcgttgcatcgccctgaatgacgttgacgaaatcgtaaacgacccggcgttcacaacccataatcaggtcgagattacgcaggccgatatcaaaatctatcacgacagttttctttcccttctgggccaaaccagtggcgatggccgcgctggaggttgtcttaccaacaccccctttgcccgaagtaacaacaataatgcgtgccatagaaattccttgttaaaaagggatcaatttaacggttgaacggtcaaagcgttttcgactaactgcagtcgcgccgctttgccataaaattctgctgggatttgatcactcagccagtattcacctgcgatggacaccagttccgccatcaggttcgtacaaaatatttgcgtttcccggtcaccacttgcccctgccagcgcacgaccgcgcatcatgccatagacatgaatgttcccatcggcaatcaattcggccccagcgctaacgtggcttgtaacaatcagatcacattgtggagcataaatacgctgaccggaacgcaccggggtatctattaaacgcgtttttgtgaccggcgttgtattttgcgctggagcctgcggtgtgggagctggacgtggcgctttttcctttccttccgtcaggataggcagccccatcttttcaatttcggctttaagttgcgcatctttgcagccacttacgccaataacccgcaaaccggttgccgaaaccgccttatgcatcgctgaccagtttaccgggtcttccagtgcactgacgttgagtacaacgggggcatgttttaaaaatgcgggggcctgagcgattttgtcttccagcgcctgatggataaccttaggttctgcctcatgcagatgaaccacagataaagtgaagctactgcctttaagctcgattggcgtgtttgacatcctggccttactcaattagctattaatcatcgccagcgcgcgatgatgttccgaagactataaggcatgttatagtctggattatattgaggcaagtcaccctcccatttattcagagtaaaagtctattctgtgataaatggcgctgattcatagcttaaaaaatacccttgtcaatcaacccattgccgtcgtacttttgattgttcttatttacgcttcctttttccgcaccctaatcgtgacagcatctccagacctgtttaaatatccagtattgaggcaagtgtattttttcaccacgccaggctttcttaactttccattttttgcggcatcattaaagaacagatacccgttatcttaatatccgccacagaattgctctatcatagaaaccgcagaagacgtctgatacttctgtcaggtcatcgtaactcgtccaggtcagcggttttgattacggattgatgatgaaatgagcataagtgttgtacggttggattatcaggatgtgctatgaatatgatgcgtattttttatatcggattgtcaggtgtggggatgatgttctcatcaatggcgtctggaaatgacgctggcggacttcaatctccggcgtgcggcgttgtttgcgacccgtatatttgtgtgaactcagatggcatttccccagagttaacaaggaaatatctcggcgaaaaagccgctgaaaacttacaatcattacaaggctacgatcccagcgaatttacattcgctaacggtgtattttgcgatgttaaagaaaaattatgtcgtgatgatcgttattttggtgtggatggtaagcggagtggaaaaatcaatcaaaccaccacaaagatgttatttatgtgtcgtgagtgatgtcttgtttacattatgttctattcgtcattaacctcttgagcgacagagaggagtggggcattaacgtttatgacggggagagtccccgtcggttgacatttacttaatttgaatatcgacgttatattttttagttttgtttttacgggcgtcgtttcgggtttgcaacactcgcagctcatatttgccagaagcagggagtgagtattgtccgtgactatcgagttctggggaatatctggataaatcaactgaatcatcgattcctggcccgaagaggtaagtatcagcgccttcattagagatactcacatgcactttctgaccttttttggcatagaaggtatatgtatcgtaatcgtatccctttatttcgccggagtactgagcgctgctatggccttttctgaactcaacattgacattcttacccgcagcaaagctcgtggaggttagcagtgcaagcagcaatacagccttcctgatgctcttgattttcattggtagtctcctgttcagaatgagtacgatgaactgttataatataacaatccctaacgggagaattccagtggctttcctgcgttcggtaaaatcacgttgcggcatttttgccggggggattacttataaagggggcatggactcaacaaaccgtagaaatctacagctggctggcttgtggcgcgggtttcattgatgttagcttatgccaaaacctggcatcttaaagagtaaaagtatgttttgtgtgatttatcgaagcagcaagcgtgaccagacctatttatatgtcgaaaaaaaagacgatttttcgcgtgttcctgaggaactgatgaaaggttttggtcagcctcagttagcgatgattctgccgctggatgggcggaagaaactggtcaatgccgatattgaaaaggttaaacaggcattaaccgagcaaggttactatttgcagttaccgccaccacccgaagatttgctgaagcaacatctttccgtcatggggcagaaaacagacgacactaacaaataaccgatatccggcggtggcattatctttgtcggcgcgggttttcatatccacgataaggtgaggggaacgttatgtatcaacatcacaactggcaaggtgcgctgctggattatccggtgagtaaagtagtctgtgttggcagtaactatgccaaacatattaaagagatgggcagcgcagtgcccgaagagccagtgctgtttattaaaccagaaacggcactgtgcgatctgcggcagccattggcgatcccatccgatttcggttcagttcatcatgaagtcgaactggcggtgttgattggcgcgacactgcgtcaggctacggaagagcatgtccgcaaagccattgccggttatggcgtggcgctcgatctgacattgcgtgatgttcagggaaaaatgaagaaagccgggcagccgtgggaaaaggctaaagcgtttgataactcttgtccgctttccgggtttattcccgcggcggaatttaccggcgacccgcaaaatacaacgctgagcctgagcgtaaacggcgaacaacgccagcaaggtacgactgcggacatgatccataaaatcgttccgctgatcgcttatatgagcaagttttttaccctcaaggccggtgacgttgtgttgacaggcacgcctgatggcgtcggcccgttgcaaagcggtgatgagctgacagtcactttcgatgggcattctttgacaactcgcgttttgtaatactttttgccgcctgaaagcggcggcaaaacttgcatcgctgtgccagactggttataaggtgcgttttaacgtaatggcggaacacctgatgagcgatgtacctttctggcaaagtaaaaccctggacgaaatgagcgatgcggaatgggagtcgttgtgtgatggttgcggtcagtgttgcctgcataaactgatggatgaagacaccgacgaaatctacttcactaacgtcgcctgtcgccagctcaatattaaaacctgtcaatgtcggaactacgaacgtcgtttcgagtttgaacccgactgcattaaattaacccgtgaaaatctgccaacattcgaatggctgccaatgacctgcgcttatcgtttgctggcggaaggtaaagatttacctgcgtggcatccgctacttactggttcgaaagcggcaatgcatggtgaacgtatctctgtgcgtcatatcgcagtgaaagaatcagaagtgattgactggcaggatcatatcttaaataaacctgactgggcgcagtgataaatttaatagatgctgatgggggctttcttaatatacgtctggatgctcgccatttcgtagccctgtttttgaaagcgctctgtcataatgagagttacccgataccttattatcaacaggtaactctcaatctttaaaaaacgtctgtgtttttaaatgtgataaaccttataccttgagtacatggagagaataatcgcttatcagacttcaggtacctcaaagagtgtctttttaccgtgtcttttctgatactcattacaggtgttaatcatttttttggccgcttcttttagcaaagaaagcattaaatcatcataatcaacgtagaatctggttgtttcagtttccgtttttatctcaccgatggcggctatttcggtggttaatttcaatttggcggcatcgatatctttattcgcttgtttaaccgtgttagacagggtggtaaagaaattctgcacagattttaacttgttcttcaattctggaatcagttttccttcaactacgcccgcagcaatagaataggaaatgattaatccaaatggaccggcgacgacaccggctgcggcaccggcatatgcttccttcctgattttatctacctgtgactggaaatagctgcttttttctgaaaaatcattggttaactggctatctaacgccagcagtttcccggaagcgttgttgaaactttgtgagcttaccagcagggatttttgcgcttcattcagcttcgtgatgccgtcatccagtaccttaatgagaatgtctttctgggcggatgctttcttctcattgtactcatcaaatagcaaaatatacgctgcgagcaattgcgtcgcaacaccacaccattcatacactgtttgggttgcttcaaaatacttatcctggctatccataagtaaggttttaatatcgccgactaaaacggaggctgcctgtgaatactcctgtttaaagcgacttaactcttttatggtttcatcaaaggtctgccaggggatgacctgatcgagatatttattataaagatctaatgctccatctgcggtttcgattgcgtttttaactacttctaccgttttatctgcaacgatttcagtcataatcattcgcctctttaaatatataaattgtaatgaaactcctgttttacaactattaataaattttacttcatctaattcatagttagccgggcgggatgcgtcaatgtctttatttctattaatatgataaatatcaaacaatgtttaatgtcattatggcgaatgcttctattctattttttagccgggtgatatttttcatttctgctggatgagcgtcgtcgccagaaggccacgtgagcacaagataagagaacgaaaaatcagcagcctatgcagcgacaaatattgatagcctgaatcagtattgatctgctggcaagaacagactactgtatataaaaacagtataacttcaggcagattattatgttgtttatcaagcctgcggatctccgcgaaattgtgacttttccgctatttagcgatcttgttcagtgtggctttccttcaccggcagcagattacgttgaacagcgcatcgatctgaatcaactgttgatccagcatcccagcgcgacttacttcgtcaaagcaagtggtgattctatgattgatggtggaattagtgacggtgatttactgattgtcgatagcgctattaccgccagccatggtgatattgtcatcgctgctgttgacggcgagtttacggtgaaaaaattgcaactacgcccgacggtacagcttattcccatgaacagcgcgtactcgcccattaccatcagtagtgaagatacgctggatgtctttggtgtggtgatccacgtcgttaaggcgatgcgctgatgtttgccctctgtgatgtaaacgcgttttatgccagctgtgagacggtgtttcgccctgatttatggggtaaaccggtggttgtgctatcgaataatgacggttgcgttatcgcccgaaacgctgaggcaaaggcgcttggcgttaaaatgggcgatccctggttcaaacaaaaagatctgtttcgtcgctgtggcgtggtttgctttagcagcaattatgagctttacgcagacatgagcaatcgggtgatgtcgacgctggaagagctatcgccccgcgtcgagatttacagtattgatgaggcattctgcgatctgacaggtgtgcgtaattgtcgcgatctgactgattttggcagagaaattcgcgcaacggtgctacaacgtacccatcttactgttggtgtggggatcgcccagaccaaaacgctggctaagcttgccaatcatgcggcaaaaaaatggcagcggcagacgggtggggtggtggatttatcaaatctggaacgccagcgtaaattaatgtctgctctccccgtggatgacgtctgggggattggacggcggatcagcaaaaaactggacgcgatggggatcaaaaccgttctcgatttggcggatacagatatccggtttatccgtaaacattttaatgtcgtgctcgaaagaacggtgcgtgaactgcgcggcgaaccctgtttgcaactggaagagtttgcaccgacgaagcaggaaattatctgttcccgctcgtttggtgaacgcatcacggattatccgtcgatgcggcaggccatttgtagttacgctgcccgggcggcggaaaaacttcgcagcgagcatcaatattgtcggtttatctccacgtttattaagacgtcaccatttgcgctcaatgaaccttattacggcaatagcgcgtcggtaaaactgctgacgcccactcaggacagcagggatatcattaacgctgctacgcgatctctggatgccatctggcaagcgggccatcgttaccaaaaagcgggcgtgatgctgggggatttcttcagtcagggagtcgcgcagctcaatttattcgatgacaacgcaccgcgccccgggagtgagcaattgatgacggtaatggatacactgaatgctaaagagggcagaggaacactctattttgccgggcaggggatccagcaacaatggcagatgaagcgagccatgctttcaccacgttatacaacgcgaagttctgatttactgagggtcaaataaatatagcggcaggaaaaaagcgctcccgcaggagcgccgaatggattagcgaccgaacagatcacgttttttcgctttaaacggctgggaaatcaccaccagcactgcgacaatcaggtaagcgataaaaataccgagcagccactgcggcatttccagacctaaaaaatcccactgacgctcggcgcaatcgccagaggcgacaaacacttgcggcacccacttatccagcggcagccattccgggaaacgaaccataaaatcacaggtggcaaacggcgaaggatagagctgaagcatggtgtgctcgtaagttaactgcacaccgcggaacgcactatacaaccagataaccatcgctacataacgcagcggagttttcggggcgatcgcgccaatcagcgcagcacccagaacgccgaataacgcgcagcgttcataaatacagagcacgcaaggtttcagtaacatcacatgctggaaccacagcgccgtcagttccagtgccagagcagtaaacgccatcaacagccacgcgccccggccttgtgaacattggttcaaaaatcgcaacataatcatttccctgcaatatgcatagagtgcgcagtttaaaccaattcattcgctgcgccaccaggaggcagcaaaaataggacgcaattggacaattatcgggcgaaaaggcaaaccgggcatttatatgcccggtaagttgttatcaaagcgttgctatccagcccatttgcataaaccattcggttacaggggcaagcgtaaactcgacgcagagcaagccgacgagtgtcaggacgagggtgtaaggcagggccatccacaccatgcggccataagagaggcgaatcaatggcgcgagtgcagaggtcagcaggaacaggaacgcagcctgaccgttcggcgtagcgacggagggcagattggtaccggtattaatggcgaccgccagcagctcgtattgcttcaacgtgatagcgccactttccattgccgctttcgcttcgttgatataaatcgtccccacgaagacgttatccgaaatggatgacagcagaccgttgaaaatatagaacagcgacagctgagcatgttccgatgcctgcaacacaaactgaataattggcgaaaacagttgttggtcgataatcaccgcgactaccgagaaaaacaccgtcaacagtgcggtgaatggcagagattcggtgaaggctttaccgatagcatgctcatcggtgacaccggtcaatgatgttgccagaataatgactgacaaaccaatcaagccaacttccgccagatgcaacgccagcgcagtcaccagccagacgccaataatcgcctggacaatcagacggattttatcctgacgggtacgctggtggcggctttgatcgtcaaactgttgcaacacttcgcggactttctccggcagcgtttcaccgtagccaaaccaacgcagcttctctaccagcaggcaggttaacaggccacaaatcagaaccggaacggtcaccggcgacatgcgcaggaagaaatcgccaaaatgccagccagccgctttagcgatgatcaggttctgtggttcgcccaccatggtcattacgccgcctaatgcggtgccgacaccggcatgcatcatcaggctacgcagaaagccacggaactgttccagaaccactttgtaatgcttgtcgatatgactatcgtcttgcaggtcggtgtcttcggtacgggaagaggctacgcggtgataaataccataaaaaccgactgcaacgctgatcaccaccgccacgacggttaaggcatcgaggaacgcggagaggaacgcagccgccacgcaaaaagagagcgacagcagcattttggagcgaatgcttaacagcaaacgggtaaatatgaacagcaacagctgtttcataaaatagatacccgccaccataaacatcagtaacagcaagacttcaagatttgccgccacctcttcacggacgtgttccgcgctggtcatgccgatgaataccgcttcgatagccaacagaccaccggggagcagcgggtagcatttcagggccatcgccagagtgaaaataaattccgctaccagcaaccagcccgcgacgaaagggctgatgaggaaaattaacgggtttacgattaagaaaatgatgagggcgagtttgtaccagtcgggggactggcccaaaaaattgcgccatagcgcgcggccccaggagatctccatgatggtttcccttaccttacaaataatcaatgatgtttttatgtttaaacgcaaagcttaacggtcaggcaggagtgaggcaagtcttgatagtcaaggggaaagagatgcggaaaatgaagccttgatccctttttcttctttttgtctgctatcagcgtagttagccctctggtatgatgagtccaactttgttttgctgtgttatggaaatctcactatggtcattaaggcgcaaagcccggcgggtttcgcggaagagtacattattgaaagtatctggaataaccgcttccctcccgggactattttgcccgcagaacgtgaactttcagaattaattggcgtaacgcgtactacgttacgtgaagtgttacagcgtctggcacgagatggctggttgaccattcaacatggcaagccgacgaaggtgaataatttctgggaaacttccggtttaaatatccttgaaacactggcgcgactggatcacgaaagtgtgccgcagcttattgataatttgctgtcggtgcgtaccaatatttccactatttttattcgcaccgcgtttcgtcagcatcccgataaagcgcaggaagtgctggctaccgctaatgaagtggccgatcacgccgatgcctttgccgagctggattacaacatattccgcggcctggcgtttgcttccggcaacccgatttacggtctgattcttaacgggatgaaagggctgtatacgcgtattggtcgtcactatttcgccaatccggaagcgcgcagtctggcgctgggcttctaccacaaactgtcggcgttgtgcagtgaaggcgcgcacgatcaggtgtacgaaacagtgcgtcgctatgggcatgagagtggcgagatttggcaccggatgcagaaaaatctgccgggtgatttagccattcaggggcgataatcccttccgtttaaagagcaaacccctcaaacgaggggttttttgttgtttttacagatttcccattcttggcgggcaacgttccagcaactcgatgctgccgtcttcgttttgctgttcgagcatcacatcaaatccccacaggcgatgcacatgcttcaggacttctttgcgcccccgatccagcggtgcgcgattatgtggaatataacgcagcgtcagcgaacggtcgccgcgcaaatccacgttccagatctgaatattcggctccagattacttaagttatattgcgacgataaccggttacggatctcccgataaccttcttcattatgaatagcggaaatctccagataattatgccgatcgtcatccagcacggtgaagaagcggaaatcacgcatcactttcggtgacaggaactggctgataaaactctcatctttgaaatcacgcatcgcgaaatgcagcgtttccagccagtcggaaccggcgatatccgggaaccagtatttgtcttcttccgttggcgactgacaaatccgtttaatatcctggaacatggcgaacccgagggcatacgggttgatgccgctgtaccacgggctgttataggggggctggaagaccacattggtgtggctgtgcaaaaactccagcataaaacgttccgttactttcccttcatcatacagatggttaaggatggtgtagtgccagaaggtcgcccagccttcgttcatcacctgagtctgtttttgcggataaaaatactggctcaccttacgcacaatacgcaggatttcacgctgccatgattccagcagtggcgcatttttctccataaaatagagcaggttttcttgtggttcggacggatagcggcgcgcttcagcaaccgttttctcttcctcgcgcttcggcagggtacgccagagcatattgacctgactttgcagatactcttcgcgacttttctgccgggctttctcttcttgcagcgagattttttgcgggcgtttgtaccggtccacgccgtagttcatcagcgcgtggcacgagtccagaagccgttctacttcatcaacgccataacgctcttcgcactcggtaatatatttacgggcaaaaatcagataatcgacaatcgaactggcgtcggtccagctacggaataagtaattgtttttgaagaaagagttatgcccatagcaggcatgagccatcaccagcgcttgcatggtaatggtgttctcttccatcaggtaagcgatacacgggttagagttaatgacgatttcataggccagtccttgctgaccgtgcttatacagccgttcagtctcgataaactttttaccgaatgaccagtgcggatagttaattggcatgccgacgctggagtaggcatccatcatctgttctgaggttatcacttcaatctggtgcgggtaggtatccagccggtagagtttcgccacccggtctatctctgccagataaacatccagcaggtcgaacgtccagtcgggtccatcgctcaaacgtgtggtgtccttattcatagaatcgatcgtcgccatacgcgcacctcattgttgtcggcgctctctgtgtggagcacctcatttcaagcatagaacacctgttaaaaaccgcgtcgccggagaatttttttctttgcgatttcttattatcagagtgccactaatccgcttctgaacggaattttatgctggataaaaagggcgttcagcaggagatactaaagacgccatattgccgcagagtcagggagatgtgagccagctcaccataaaaaagccgcatgttgaataatattttcaactgagttatcaagatgtgattagattattattcttttactgtatctaccgttatcggagtggctatgcgagttgtcatactgggaagtggtgtggtaggcgttgccagcgcctggtacttaaatcaggcaggacatgaggtcaccgtcattgatcgggagccgggggccgccctggaaaccagtgccgcgaatgccgggcaaatctcccccggatatgctgcaccgtgggcggcaccaggtgtgcctttaaaagcgattaaatggatgttccagcgccatgcgccgctggcggttcgtctcgacggtacgcagttccagttgaaatggatgtggcaaatgttacgtaactgcgacaccagccactacatggaaaacaaagggcggatggtgcgtctggcggaatacagccgtgattgcctgaaagcattgcgcgccgaaaccaatattcagtatgaagggcgtcagggtgggacgctgcaactgttccgtaccgaacaacagtatgaaaatgcgacccgcgatatcgccgtgctggaagatgccggcgtaccgtatcagctgctggaatccagccgcctggcggaagtggagcccgcgctggcagaagtggcgcacaaactgacgggcggcctgcagttacccaatgatgaaaccggagactgtcagctatttacccagaatctggcgcggatggcggagcaggcgggggttaaattccgctttaatacgcccgttgaccaactgctttgcgacggcgagcaaatctacggcgtgaagtgtggcgatgaagtgattaaggccgatgcgtatgtgatggcgtttggttcttactcgacggcgatgctcaaaggcattgttgatattccggtgtatccgctgaaaggctactcgctgaccattccaattgcgcaggaagatggtgcgccggtatccaccattcttgatgaaacctacaaaatcgccattacccgtttcgataaccgcattcgtgttggcggaatggcggagattgttggttttaataccgagctgttgcaaccgcgtcgtgaaacgctggagatggtggttcgcgatctctatccacgcggcggtcatgtcgagcaggcgactttctggactggtctgcgcccgatgacgccagacggcacgccggttgtcgggcgtacacgctttaaaaatctgtggctgaataccggtcacggcacgctcggctggacgatggcttgcggttccggtcagttgttaagcgatctgctctctggtcgcacgccagcgatcccatatgaggatctaagcgtagcgcgctacagccgtggatttacgccatcacgtccgggccatttacatggcgcacacagctaaggaaacgagatgacccgtccgatacaggccagcctcgatctgcaggcattaaaacagaatctgtccattgtccgccaggccgcgacgcacgcgcgcgtctggtcggtggtaaaagcgaacgcttacgggcatggtattgagcgtatctggagcgcgatcggggccaccgatggctttgcattgcttaacctggaagaggcaataacgttacgtgagcgcggctggaaaggaccgatcctgatgctggaaggatttttccatgctcaggatctggagatttatgaccagcaccgcctgaccacctgcgtacacagcaactggcagctcaaagcactgcaaaatgcgcggctaaaagcaccgttggatatttatcttaaagtgaacagtgggatgaatcggttgggcttccagcccgatcgcgtgcttaccgtctggcagcagttgcgggcaatggcgaatgttggcgaaatgaccctgatgtcgcattttgccgaagcggaacatcctgatggaatttccggcgcgatggcgcgtattgagcaggcggcggaggggctggagtgtcggcgttcgttgtccaattcggcggcgactctgtggcacccggaagcgcattttgactgggttcggcctggcattattttgtatggcgcttcgccgtccggtcagtggcgtgatatcgccaataccggattacgtccggtgatgacgctaagcagtgagattattggtgtccagacgctaaaagcgggcgagcgtgtgggctacggcggtcgctatactgcgcgcgatgaacagcgaatcggcattgtcgccgcagggtacgccgacggttatccgcgccacgcgcctaccggtacccctgttttagtggacggcgtgcgcaccatgacggtggggaccgtctcgatggatatgctagcggtcgatttaacgccttgcccgcaggcgggtattggtacgccggttgagctgtggggcaaggagatcaaaattgatgatgtcgccgccgctgccggaacggtgggctatgagttgatgtgcgcgctggcgctacgcgtcccggttgtgacggtgtaacttgttgtaagccggatcggaggcaacgtcttctgggtgcaaaaaaatcatccatccggctggtcagcaactgtagttgttaatgtgacagagccattgcccatgatagtgtccattaaaaggatggacactatttccccggaacctgaactcaccgcacaggcgttctacataaaacgcttacgcttcattgttgactcgaactcgacttcagataaatcacgctttacccttgatggagcctgtacatagatttgtgtaattgcctgattttgatatgttcaattcaacatcaaatgaaggttaaattatggacgacaaacaattgcaggctcaggctgcgttcagcaaagcatcgcaaccggcgatagatgcttcattaaatttaagattcagcttcctcttcagccacccgtacgccaatcttcaacacttcattatcttctttctcggccaccgtccagatcatcccggcaaactctacctggtcaccgacaaccggtgccgcgcctaacaactgctggacaatttcacccagcgtttgctgcttatcacgatattctcgcccgtcttccaggccatatatcagcgcaacatcagcatatttggcgctggcttcgagaatgaagtcaccaaagaagcgttgatccagcgcgaccggcggcgactggctgaacagtttaccgagcgccggaagatcgcgttcccgaccaattacacacaacacatcgccttcgcgcagtcgggtgctgccggtaggatgaagcaactggttatcacgaaacagtgccgcaatacgcgtctcttttggcatatgcaaatcgcgcagtgccgcgcccacgcaccatttatcggcactcaattgataaacaaactgctcccacggattttccggatgaatatccaggccaacgcgtgacaccggacgtcccactggcggaaccaccactttggcttttttagccgcccacgagagtgatgttccctgcaagagcagtgaaaccagaaccacaaagaaggcgacattaaagaacagacgtgcattctccagccccgccatcatcgggaacacggccaggatgattggcaccgcgccgcgtaatcctacccagctgataaacacgcgctcacgcagattgaaaccgcggaaggggagcaatccagcaaataccgaaaggggacgggcgaagaatatcatccatgcggacaaaatgagcgccggaatggcaataggcagcagatcgcttgggttaaccaacagccccagcaccaggaacatggcgatttgcgccagccaggcgaggccgtcgaaattttgcaggatgccgtagcggttgcgaatagggcgattacccagcagaaaaccgcacagatacaccgccagaataccgctaccttccagcgcagtagttaatgagaaaatcagaataccgccacttaatgccagcaatggatataatccggcgggcagggcgatgcggttgatcatttgcagtagtaaataaccgccgccaagacctattacaatgcccagaccaaattgttgcagaatatcgacaatgaacatccagctaatattgctctcatgatgctggatcatcgcaattagggtaatcgtcagaaagaccgccattggatcattactgccggattcaatttccagcgtcgagccaacacgttcgttaagccccttaccacccagcagagaaaagaccgctgcagcatcggtagagccgacgatagcgccgattaataagccttcaatcaaatcaagattaaacagccacgccgccatcatgccggttaaaccagaggtgataagcacgcccagcgtcgccagcgacagtgccggtcctaacgccacacgaaaggaactggcctgagtgcgcatcccgccgtcgagcaaaataatcgccagtgccaggttacttaccatgtaggcgaaggggtaattatcaaacgggataccgccgacgccatcgactcctgccagcatgccgatcgccagaaaaataaccagaataggaatgccaagacgggaagaaaatgaactaagtaatatactgctggtgacaaggatggatcctaagatgaaaaggctaattattgttgtggcatccaacggtcggttactcctgattacgctgtctcttatataaaccctaccatattagcggcagagacagcgttttacttagccctgaagcgtgatttttttacattttaagaacaggatgaccgctaatcgtcaactgagtgccttcccgggtgttattcagaatggcatgtgcgcccaacggcagcgtaaccgtgcgttgttcatgaccaaaatcgaggccggtaatgagtggaatcgacaggcgggaacgcaaaaacgcgtacactgactccaggttgtaacctgcgtcataatcattgggcgtgctgccgctaaagctaccgagaataatcgccttctgacgtggcaaaattcccgcatgatagagctgcaacagcatacgttcgacccggaaagggtgctcgttaatatcttccagcaccagaataccgttctcaatttttggcatccacggtgtaccgatcagtgaaatcagcatcgcaagattgcctccccacaacgtgccttcggcccgacatgtcgggccttccccttgccattcaatggtgaaggtttcattgcgtaacgccagccagaaatggtgctcggtaaaggcgttcagttcatccgcgccaaagtttgctaccagcatggggccgctaaaggtgatgacattgccatgcgccagaagaccgcactgaatggcggtaaaatcgctatgtccgcaaatgagcaacgggtcatgttgttggcgagccaccagtgcctgccagtcaatatctgccagtaaacgactggcaccgtaaccgccgcgtacagccagcacgatggtgttgggggtagtcagtctggcaagggaattgagatcttccagacgctctgtttccgtacccgcaaaacgctcacaacgacgggcaataacctcgacgttattgacttgatgccccgcgtcggtaaggcgctggataccacgcagcgcggcgtgctgtttaatgcagtaacccgatggggcaattaagtgaaacagagacatggcaattccttgctgacaacagaaacgaaatgtatatcatgccgcttaggtgtgccgttgtcacctcaacggcgattccaggctataaggatagaagaagtgaaattgagatggtttgcctttttgattgtgttattagcgggttgttcatcaaagcatgactatacgaacccgccgtggaacgcgaaagttccggtgcaacgtgcgatgcagtggatgccaataagccagaaagccggtgcagcctggggcgtcgatccacaattgatcacggcgattatcgctatcgaatcgggtggtaatccgaacgcggtgagtaaatcgaatgccattggtttgatgcagttaaaagcttcaacctccggacgtgatgtttatcgccgtatgggctggagtggtgagccgacgaccagcgagctgaaaaatccagagcgtaatatttcaatgggggcggcttacctgaatattctggaaaccggcccgctggcaggcattgaagatccgaaggtactgcaatatgcgctggtggtgtcatacgctaacggggcaggtgcgctgctacggactttctcgtcagatcggaaaaaggcgatcagcaaaatcaacgatttggatgctgacgagttcctcgaacacgtagcgcgaaatcaccctgcgccgcaggctccgcgctatatctacaaacttgagcaggcactggacgcgatgtaaatcagtcgcgcactttgtccgctttttcccgggcttctcgctcgagagagaaaataatccgctgtaattgccgctccaccgtcgggctgacgttaagaaaacggaagctcagacggggagtggtgatggtttcattcttgccatcaatcactttgcgctcgctgatggagattaactgggcgtcaaagtgaaaaacaccccattgccccatgttgacttcaatctgagcgaagcgcatgccttcttgtaattcggcaggctttgctgtttccagtaatgcgcccatgccgcctaacgacaaatcatacaggcggaaacgtaacgtactgttatccgccagtttggtctggcaaaaataaggcggatggagtggggcggagatgcggaaatatcggcgtcgttgtacaaaccataaggtgggaggcggtacggtaataaatgccggaagctgcaagtattcactctgctgtagttgttcaacagtaaactcgactttcgcaccctgagtttcggcggtaatggtaatgtgctgtgcctttagcacggcgatgttgtcttcggcttgactgccgaaatccagcaccagtttatccggggttattgccagtaatttgctgatcagctgcccgccattccaactgagacgcaaaggaattgcggctttgtgcaaatcgcgtaacacgcccaggacggctaacggattttgtttcaggaactgctcatggtaatgactcacgcggaaaaactcctgactgacaaactgtctttggtttatcggtcacagttaacaaaacttaatacaaatgcgtgaatattttttacatgttgttcttaaatcagccgacatacgcccagcatcgatcccgcccttgcctatacttagagcgttgatgtaagcatttcttgcgtccgattcatcgaaacgagggcctgaacatgggaattattgcctggattatttttgacctgatagccggcattatcgccaagctaatcatgccggggcgtgatggtggtggatttttcctgacctgtattctcgggatagtcggtgcggtggtcggcggctggctggcgaccatgtttggcattggcggctccatcagtggttttaatctgcacagcttcctggtggcggtggtgggagctattctcgttctgggcatattccgcctcctgcgaagagaataagattttcataaggcggatagcgatacagatgccgctatccgctttcacatcagaacgtatactcgacacctgctttacgggtgaaaaaaatcaatatagcacttcgatatccgataaagtcggttcccggtaacaacaacagaatccttttttaattattgtttcgttgtttttggtgtgattcagaaaataaatattttagacagtagccagtcaggcgttaaaaatggggcggatagtgaggcggttttggctgcgcttattgaacatttagaattgatcaatccttctggcagattaagccaaaatacccgttcggcaatgcttcagttacgcgaagaggaatggtctgaattctttttttggttgctaaattctctggagtgtctggattatgtgattattaatttaactccagaaagcaaaaaaacgttgatgagtgaacaccgtaacaatattcaggtagcaattgatgctttatatagccaacgtcggcgtaaatcgccgggtgatgaaagtgaaacacttacccgtagaaatgacgctatcttcggcaaccacgtatggcaaacatttgcgcaatacttcccgccaggacttgaaaaaccgtctgtgtagaaaaaaccatagctatggtgttatctgccgacaacgccatccggagaagccgaatgacgttgtcggagtaagcgctggttaaggtgtgggttgtgcctctttggttgagggttgcgtcgttgctgacttaacggtcggacgcgtcgccggaacattgtcacacggttgctctttcgggcagatcaaatccagcattttcagcgtcacgccattggtccagccaaagccatcctgtaatggatattcgccaccgccgccccccgttccggtggtgctgacatcatatttttccaccagctttttctcccggtcataggtgtgctgaacattggtcaggaagtgccagctaatgtccatcgccacctctttttgcccgtagttttgtaatccttctgtcgcgacccactgtaacggtgcccagccatttggcgcatcccattgttgcccacttttcaccgacgtggtgttcaggccgccgggttgcagcagatgtgttttcgtcgccgtcgccattttgttggcgcgatctttcgctgccgcattgacgtacagcgggaacagggcggccgcggttaactgattgcgcactttatgacttttcaggtcgtaatcggcataccagccttgttgatcgttccacaggtatttttcgatccctttttgacgggcatttgccagcgtttcgtactggtttgccatcgcgttatctccggcagctttgctggcgcgggcgaggattttttccattttaaacatcaggctgttcagatcgaccggtacgatgctggtggtgcgtaaggtatttaactgctgcgggttgtccatccagcgcgagctgaaatcccagccagacgcagcggcagagcgcaggtcgcggtaaatttcagtggcaggtcgattcggattgcttttggcggtggcaatatcttccacccatgactctggtcgtggcgtatcgcgatcgtcccagtagcggttgagaagggtaccatcctgaagtttgacaacgcgtttttcctgttgtccggcttgcaggttttcaacaccgtccatccagtaagcatattctttttgcatttgcggcaggtattgcttcaacgcggcatcgccttcatgctgcgccagtaactctaccatcagggcaaagaagggcggttgcgagcggcttaaatagtaactgcggttgccgttgggaatatgaccgtaagtgtctatttcatgagcaaaattggccaccatatccgcgactttatcccagtgaccgctttcggcaagtcctaacatggtgaagtaactgtcccagtaatatacctcgcgaaagcgtccgcccggcacgacataaggttccggcagcggtaacagagaatcccatttttcggtgttttcggtagaacgcgttaataccggccaaagtccgtcaatatgttcgcgcagtgactgcccctctggcggaacatatttctcgccttctttcggcagggtgaaattgacgttaacgaaatggcgcagatcaaatccgctctggttttgctgcatccgataatcagcaaggatcatcagcggatcgctgttcggcacggcatcggcaaaggttttttggtccggaaaaagtttggcgttttgcacatcattaaacagcggccctaataaaatatcaggcggctgtggtgttaccggtgtttcttctgcctgcaccgatagcgcagcgaaacacaaaaagatacaggctggaattaacgccattttttgcgggcgagaaggtgcgggggatttcatcaatcattctcctttggcgaaaccgaataaaacggtattcaagtatcagaaaaccttagttcaggatcgcactagctgcatgatcgaaatctcattctgcgaactgtcaggcattttagaaaagggaattaaagggataaataacggcgaaatagagtgatcaaataacgtctgtttattagccagccagcggcgttgggttcgtgattagcgaagaaaaatcatcataaattggtgaaaaatataacaggtagttaaaaaccattagtgctgagtaaattgccggatgacatcagaacgatgccatccgaacagtggcttaaccctgacggttgaaacgttgcgttttaacgtccagcgttagcgtttcttctggttgtatcgcatacagtttctcaccctgctggcaaatccagccaatccccagttcacgggcgattagggcgctgtgggataccggacttccggcgctaaggcagataccttttacaaccgccggatccagttgcagtactgtggaaggataaatgttctccgccagtagaatagttggcgagttaaactgcgggagttcttctttcgtttgggtcaggtggaccagggtgcgatgcagaagatcgtccacatcaatatagcgagcttgtagatattcatcatccagttgctggtattgctggctaagttctttaagaacttgctgccaggcatattctgccgtgcaatgttcatgctgaaggagttcgcttgccgccgccagcagttccggatcatctaacagtgtatggtgaccagaaaagattgcggcaatatcgtcaagcccgctggcttctgctttcgctgttaacgtcatcagatctaataacgtgaagtcaatagcctggcgtaatcgatcttgttcttcttccacggtcagggttgattttgcctgtaccgtacataaaactggttgataataaaaggctttacccgaaacaggcggaacgggacgcagagtaggtggagcgacttcctccgtttcaccaaagttatcttcagccagctgacggaaagcgatcagtgcctcttcagcttctggccctttcgcaatcaggcgcagcgtatcgttatagcgaacttgtagtaacgcaatctggttaatactctctggtgtgacgcatttgccgtttttttccagcaacatatcggcattaaatgtcgataaggtataaaccagccgggaggccggacgtacatgcaggccgttacggttttttatgaccaccgccagagaacgggcttcttcatcgtacgcaggacatgtgtcagagatttcagtgtcggaggacggtaaacccagttgttcacgtttggcttccagcgcatgcatggcgtcaaagataactttgtcgatatccgcccccgaggccgcgctgaccgttgctgccagtgtaccttcgaccaacggcgcagcacacaaacgtacttttgcggcgatctcgggagccagcaattccagcgcagtttcagcactcaataatgcgctacccatatccatcatgaccagcacatggtcggcatcagcaacagattcgatggcctccatcactttgacggcatcggtaccaatgggattttgtggatcgtcaattcccgcggcaatggcgattttacaactatcactcattaacatctgacgggctaattcaccgacaccttctcccagtcggctgctatgtgaaactatgaccaggtttaccatcaccaattccttactcttttgcggctaacgccaacatttgcatcataaacatcaccgaggtcgcgccgggatcctggtgaccaatactgcgttcaccgagataactggcgcggcctttgcgggcttgcatcgtaatcgtactttgtgcagcggattcggcgatgctactggcagcttcgagcgccaccggaacagagagattttgctcgctggactgacgtaacgattccaccaccggcacccacacatcacacatggttttatcgccaggttcggctttcccgcgactgattacgccgtccgcgccatcgcggaacatctgataaagctcttccagtgtcaggctttgccgtgcctgggtcgcctgtgcggcgcggataaagaaggtaccgaacagcggaccactggcaccaccgacgctggaaagcagcgtcataccggtattcttgagaatgaaaccgatatctttatctgcgatagcagggagtttttccaccactttgctaaagcctcggttcatatttagcccgtggtcagcatcgccaatttcgcgatccagtccggtaagatactcgctctcggtgctgaaaatatcgccacaacgagtgagccagttaacaatttgagttctgctcagtgacattgctttctccttatttaccccagttaagggccggggtgtggaccggggcgtcccagagtgccagcgtttcgtcatcaactttcagtaaggtgattgagaaaccggtcatatccagtgaggtgcagtacgcgccaattaaattacgttcgatagtcaatcccgcttgctggcaacgtgtggtcaggcggttatagacgccgtacagctcagaaagcggagttgcgccaagattgttaaccagcgcaatcacccgatcgccagactggagcggttgtttggtttgttgttcttcctgccaactgccttgttgataatcccagaaacgcaaagtgcgatggtatgagccatttaccagcagggtgtcgaacatttcatcgacggtttgatcaagggaagagaaggggcggcggtcaatacccggctcaccatgaatgccgacgccaaactccatctcattatccgccagggtaaaagaaggtttgcccgcggcaggaacggtacaggcaccgagagcgatacctattgagtggccttgattattcagcttacgccccagttccgcacaggcgtccagtgagtcgccacgctccgccgctgcgcctacgagtttttcaattaatacggtgttggcaacgccgcgtcgcccggcagtataaagactgtcttttaccgcaacgtcgtcatcaatgaccacagtggtcacttttacgccgctatcgtgcagtaactcggtcgctgtttcaaagttaagaatatcgccggtgtaatttttgataatcaacagtacaccttcgccgccatcaacttgcatggcgcattcaaagattttatcgggcgtcggtgaggtgaaaatttcgcccggacaggcccccgaaagcatcccctgaccgatataaccacagtgcatcggctcgtgtccgctgccgccacccgacagcagggcgacttttcctgcaacaggggcatcagctcgggtgacatacaccggatcctgatgcagtgtcagcgatggatgcgctttcgccagtcctgccagttgttcgtccagtacgtcttgcacatcattgatcaattttttcattattttgctccagcaattacggtagggcatggatgatgttcaacgacacggcgaccactgactgccgatgaatccattgtgcatcaggcaagggaaaagaaaattagcccaaattatgtttcatagtgaaacatatgctttaatgaatgttccatattgaaacttttacgtgtattaatacttaaaattgcgagccggaacaccttttgtcataagggatgcgggatatgagtggcgcttttaacaacgatggtcggggcatatctcccttaattgcaacctcctgggagcgatgcaataagctgatgaaacgggagacatggaacgtaccacatcaggcccagggcgtgacatttgcttctatttatcggcgtaagaaagcgatgctgacgctcgggcaggctgcgctggaagatgcctgggaatatatggcaccgcgagagtgtgcgctgtttatcctcgatgaaaccgcctgcattctcagccgtaatggcgatccgcaaaccttgcagcagctaagtgcactgggattcaatgacggcacgtattgcgccgagggaattattggtacttgtgcgctatcgttagcggctatctctggtcaggccgtgaaaacgatggccgatcaacatttcaaacaggtactctggaactgggccttttgtgcaacgccgttgtttgacagcaagggccgattgacgggaacaatagcgctggcgtgtccggttgagcaaactaccgcagctgatttgccgttgacgttggcaatcgcccgcgaggtcggaaatttactgctgacggacagtttgctcgctgaaactaaccgtcatttaaatcaacttaatgccctgttagaaagtatggatgatggcgtgattagctgggacgagcagggtaatttgcaatttattaatgcccaggcggcgcgggtcttgcgccttgacgcgacggcaagtcagggacgggcaatcactgaactcttaacgttacccgccgtattgcaacaagcaataaaacaggcacatccgctcaaacacgtagaagcaacctttgaaagccagcaccagtttattgatgcggtgataacccttaaaccgataatagaaacgcagggaaccagctttattttgttgctccatcctgtggaacagatgcggcagttgatgaccagtcaattaggaaaagtcagccataccttcgctcatatgccacaggacgatccgcaaacccgccgcttgattcattttggtcgccaggcggcgcgcagtagctttcctgtcctgctttgtggagaagagggcgtgggcaaggcactgctaagtcaggcaattcataatgaaagcgagcgtgctgcaggtccttatatcgccgtcaattgtgagttatatggtgatgctgcgctggcggaagaatttattggtggcgatcgcacggacaatgaaaatggccgtctgagtcggctggaactggcacacggcggcacgctgtttcttgaaaagattgaatatctggcggtggagttacagtctgctttgcttcaggttatcaagcagggggttatcacgcgactggatgcgcggcgtttaataccaattgatgtcaaagtgattgcaacaacgaccgcggacctcgcaatgctggtggaacaaaatcgttttagtcgccagctgtattacgcgctgcatgcatttgaaattaccatcccgcctctgcgtatgcggcgtggcagcattccggcgctggtgaataacaaattacgcagtcttgaaaaacgcttctctacgcggctgaaaattgatgacgatgccctcgctcgcctggtttcttgtgcatggccaggcaacgattttgaactttacagcgtcatcgagaatcttgctctgagtagtgataacgggcgcattcgcgtcagtgatttgccggaacatctgtttaccgagcaggcgacagatgatgtcagcgccacccgcctttccaccagtctgtcatttgcggaagttgaaaaagaggcaattattaacgcagcccaggtcacaggcggtcgcattcaggaaatgtcggctttacttgggatcggccgcactacgctgtggcggaaaatgaagcaacatggcattgatgcagggcagtttaagcgccgggtatgaaagacagaaacgatttctgatacatcagagtgatctgtatttcattccggcgcacgctaacaattttcagcatcgtttaagggcttgtctatcccgcacttaaaagctgaagcgatatcctccgttgacttgcttctgatcaaagaggttaccctgcgtgtaatccgcttcgagatagaatgtgtgctgtttgttatactgtgcactgactcccacgccgttattccagccattacctttgaaactgtacttctcccgggagttgttcaacagatattcggtatcccctgaaaactcgcggatagcgccagtcttcacatagacattcagctggctgttgcctgcggtgatgtcataccccagtatcatgctggcacgccccagcagcgattcgtagtgattcagatgtatattgaggccattactcgccttcatagtcatctcattctggtggctgtatgtaagctgggtttgcggctctatatagaacccataaccagtaggggacaggttgaacctctgcccggcttccagggagatgctcattccattcgcagtgccgttggcgttaacgccgttgttctgactgtccagtacgtggaaactatttttctggcgcgatgcttttataacgagatcgctgtaaaaaccgttttgtgccatgtaactggcgtacattcccatgtagtctgaacgtgcggtaccgtcgcctccgctatagtccggcgatgcatgtgttgagccaatatacagaccgacatacaacggcattacatcagagagacgtttatccccaccaaactggataccgctgtaacccatgtcaaagccgctcagtttgccactggcaaaggagtccaggcttcccccataactgcgcaaccagatattaccgtctttactctgatttcgcaggtcacccatccgttgcatcagcgtacggttttcaacatagttcaataagtaaccgacattgagataattgccgccagcatctgcggtcgtggtgggtttaggcgtgggagcgggttcaggcgtaggatcggggttgactatgggaggctgagcgggagctggtgtgggttcaggattaggagtcggttccggaactgtcccggaagcgtaaagctcccagttagtgccatttttacgcacatcgtacagatatccccccaactcaacctgagaagacgcgctgaacgaggccgcgccgtcagtggtttttaccactgtcagaacttcatttcccgttgtggcctcgctgccctggttgcggatagccaatacgtgattaccagcactactcccgctgatattcaataaatcccctttattattaacgccattaccctcgccaacaacatcagcacgcataataaaggtactgttaccgctcaggttctctacgtttaatgtggcaaatgtgccggcagttgacccgtggctggcaaaatcgacagttgaatggctcagcgccagcgtgtcgagattagaattacttgttacgttccagacgctgttattcattgcaacgtccagttttccgccattgacattatcgctgagggaggaacctgtccaaaccgacccagggtgcatatccagattgattagcccacctttggaaagaacgctaccgttgataagcatacgacccgaggcgttgatgcggctggcggcataaccatcgtcatgttgcgttgcgatggccatctggtcgggtgtactcatatcaatgaccagatcgctcgtgaggtcgatctggctgttggtcatggcataaattcccctggctcctgccgcgccggtgatagccaaactgtctccggttattctaccgccgctgagagcccacaaacccagcgccagactgccattacgatcaactgtaatatcggtattttgcatgttgacaacagccgttgccgtctgggccgaggcaccataagaaccgccggaaaagatgctgtttcgttgcgctgccgtgccagtaaaattgattatcgcgtctgaaccactggtgacgaggccaccgccctgcgcggaagaaatatggctatctgcaccgatagtggttgtaccaccacgaacttcgacgccattggccgcggctccagttacatcaacagtgagtgcattcgcgctaacctggccaaagctccagaggccgtgagcattatcgccattggttttaatggtactgtttgttccgagatcgacaacagagtttttctgtacgtttatccccatggcgctgtagccctgaacatcgattgtcaggtctgtagccgtaaaacgcgcagcaccattggcgttattgccgttgagaccaccgatataaacacctgtacttccatcggtcgtgattttacttccgcttccaagatcgacactggtgccatagtcattgatggttaggcctataccgttcgagttttcaatggtgaattgagtggctgttagtgttgagctatgcccaataatgatgccgtcatcgttactcttaatggtgctgcctgtgcctaagtcagcatgggtatagtcaccaattaagttaatgccgatggcagaggtttgaccaacaacatctactgtgagtcggttagctgtcagggagctgtttttgccctgaataatgattccttttgcatatccagaggcgtcgttgacattgacggtgacatcattacccaggttgatattgccaggcgtgtttcctgctggggtcattacaccatagaggtttcctgatggatcggcggtatctcctgtaattctgtcaccatcattaatagtaatattggtgccatattgacttcctgtatcagcagctatcagcaggggggaaaagataattgcattcaaaccaatagcgccaaattttatcagttgaattgagggcgaacggatttttaattcagcgagacgatctgctttggtattcccattgtgttgtttgatgcccataccactcctatatagtacccagactatgggtctatggattttgtcattttgtttaaatcaatgaataatatcctcttatcatcatgatatttgtatggtgcaatcatgatgagcttctcagagaataattctctattaccgggcaaaatcaggaacacaggaattaatatatatttaacatcccccttacaaaggtgagtttatatcgagttattccctaagttgtcgttacttattccaattcgttactataaatatggcaaaaatattacaacaaacagcggttaaaaaatttggtgaagattttttgtaataatcctaattagttatgggaatttcgcttgatgtatctgcataacaaaaacaatatgcgccatttttgcattactaataagaaaaagcaaaaaacatcgatattcatttttggtcaatgggttttctggcctatcgttgttattgtgctactggttatcattttcatcttgccagcatattggagcgtgatcaattttgatcagctgtgaagggggctgatgtgtagtgatacaaaaacttacgttatatcactgctaatgagatatccggcatctgaacacttatgtctttaattattctcgtggttcactataggcaataagcacaaaagtgtaggatgttacaagaatgattaggactcggtgaaatgaaaaatccacgcaattgcgtggattttatatacttttgcgctcttcatgagatttagcgaaacctcatgagacaataaattaattagacgttgaaaaggaagttcatcacatcgccatctttcacgatgtaatctttaccttctgcacgcattttgcctgcttctttcgcgccttgttcacctttgtaagtgatgaaatcttcaaacgagatggtttgtgcacggataaagcctttttcaaaatcagtatggattttgcccgctgcctgcggcgcggttgctccaaccggaatggtccatgcacgcacttctttcaccccagcggtgaagtaagtttgcaggttcagcagtttataaccggcacggatcacacggttcaggcccggctcttccagcccaagctcctgcataaactcgtcacgttcttcgtcgtccagttcggcaatgtctgcttcaacagcagcacaaaccggaaccacaacagaaccttctttcgccgcgatttcacgcacctggtcaagatatgggttgttttcaaaaccgtcttcgttgacgttggcgatgtacattgttggtttcagcgtcaggaagctcaggtaacgaatagccgctttctcttcagcgcttaaatccagcgcgcgcagcatacctgcattttccaactggggcaggcatttttccaggaccgccagctcagctttcgcgtctttatcgccacctttggctttcttctgtacgcgatgaatcgcacgttcgcaggtgtcgaggtctgccagcgccagttcggtgttgataacttcaatatcgtcagccgggttaactttgccggaaacgtgaatgatgttgtcattttcaaagcagcgaacaacgtgaccgatcgcttcggtttcacggatgttggtcaggaactggttacccagaccttcgcctttcgatgcgccttttaccagaccggcgatatcgacaaattccatggtcgtgggaagcgtacgctgcggttttacgatttcagccagttgatccaggcgaggatcaggcattggtacgacgcctgtgttcggctcaatggtgcagaatggaaagttggccgcttcaataccggctttggtcagcgcgttgaacagggtagatttcccgacgttgggcaaaccgacgataccgcatttgaatcccatgatttaaatcaccttaatatcttaataatcaacctgttattgctaacagattgcagaaatggaaataactttgcctattatacacggcactcggcaaaaatgccgcagacaacgacttattgcgctttaaaggcgtgcaatcggttcgttgctttggtcaagccatctgtaaaccacatttcagtacaacgcgccgcttcgtcaatggcttcatcaattaacttctgttcactaacaggcggtttgcctaacacaaaaccgacaactttatttttatcgcccggatgaccgattccgatgcgtaaacggtgaaagttagggttattacccaatttactgatgatgtctttcagtccattgtgaccaccatggccaccgcccaatttaaatttggcgacgccaggaggcagatccagttcgtcgtgggccaccagaatttcgtccggattaatgcggaaaaaactggccatcgccgcaacggctttgccgctgagattcataaatgtagtcgggactaacaggcggacatcttcgcctccaagagtgactcgcgaagtataaccaaagaatttagcctcttcgcgcagcggagcgcgcaaacgctctgccagtaagtcaacgaaccaggcaccagcattatgtcgcgttgcggcgtattcagcaccggggttcgccaggccgacaatcaatttaatcgtcacgtttttttgtcctgagtgtgtacataactggcgcgtagtttactggttgcggccccgcttgacaaaaaactgcgtatcaaatgcagataacgtaataattgcctgagtggactattagaaagtcaaggtgttcaggcgtttatttgtaaagttttgttgaaataagggttgtaattgtgatcacgcccgcacataacccactgggtgttgtctatactttacacataaggaagaggggtattccctgttacaacccagaaagttccggaggtgacatatgaaacgcaaaaacgcttcgttactcggtaacgtgctcatggggttgggtctggtggtaatggtggtcggcgtggggtattcaatcctcaaccagttaccacagtttaatatgccccagtatttcgcacatggtgcagtgctaagtattttcgtcggtgccattctctggctggcgggtgcccgtgttggcgggcatgaacaggtgtgcgaccgttactggtgggttcgccactatgacaaacgttgccgccgtagcgataatcgccgtcatagctaacaaataatgcagtttgctgaccagtcagtttgcgctgactggtcaatctcgtacttataaatccgccatcgccgcgcgacgattcgggaagaacgccaggcgtcccgggatcggttgaatgccagcgcgagccatagtgcgcagtggctggaattccacgttgcacacgcgcagttcacatccctcgggcagacgcttcacaaaacgctggaacgcatcaagaccaccagcatcaagtaccggaacggcatcccacttcagaatcacaatccgtttgccttcaagacgtgactccaggtccgtgaataagccttcagcagcagcaaaaaacagcgggccaataacgcgcagaaccaggacatcgtctggaacatctacgactaccggtgccaggcgagtcatacgtgcgatacgacgcataaacagcagcgatgccagcacgatccccacgctgatggcaataaccatatcaaacaacacggtcagcgacatgcacagcagcatgacgatgatgtcatctttcggcgcatgacgcagcaagtcgaccactttgtgcgcttcactcatgttccacgccaccatcaacagcagggctgccatggcggaaagcggcagccaggagagcagcggtgccagtaccagcagggcaagaataaccagaatagagtggatcaccgccgagataggggacgttgccccggcacggacgttagcggcagaacgcgcgatggcagctgtagcggtaataccaccaaagaacggagcgataatattccccagtccctgtccaaccagttcgctgttcgccttgtgtttcgtcccggtcataccatccagcaccacggcgcagagcagagattcgattgcgccgagcattgccattgagaatgccgcaggcagcagtgtgcgaatagaatcccaggttagcgtgaattctgaattaggcagatcccacggcagcaccagttgcggcagcagttgcggaataccgttaccctgagaaccatcggccaggacgtagtggaattgcgaaccgatggtagcaacatgtccgccgagcaggttaacaatccccatcaccgcgcaaccagccagcaaggccggaaggtgaccgggtaaacgaatgcccagacgcggccaaaaaacaagaatacctagcgtcacaatgccaatggcagcatcacccacattaatggtcggcagcgccataaataatgcgccgactttttgtagataatgttccgggacatgggccatttgcagaccgagaaaatctttaatctgcatggtaccgatggtgatcccgatacccgaggtgaaacctaaggtgacggaaaccggaatatactcaatcaggcgaccaaagcgtgccagacccatcagaatcaaaaagatccccgacagcaaggtcgcaaccagcagtcctgccagtccaaactgttgcgacacgggatagagaattaccacaaatgccgcagtcggaccggaaacgctaaagcgtgacccacccgtcagagcaatgacaatccccgcaacagctgcggtatataaaccgtactggggtgccacaccactaccaatagccaacgccatcgccagcgggatagcaataatcccgacggttatcccggcaatcaggtcacgggtaaaccgtgcggcagtatatttttctttccagcaagcgtcgatcagagcgcggaaaggcatcacatgtgaggaaaatattttgttcacaataatgtttcatccgtgagcgcatcatctgtcaactaaatggcaggtgaaggaggcataggtcatacaaatggatattacagacaaaaaaacccgccgcagcgggtctttgagccgggttcgattagtgttcgaacatggcagagatcgattcttcgttgctgatacgacgaatcgcttcggccagcatacctgacagggtcagagtacgcacgttcggcagtgatttgatttcatcgctcagcggaatggtatcgcagacaacgacttcatcaattacagagttacgcaggttgttcgccgcgttgccagagaagatcgggtgagtcgcgtacgcaaatacacgtttagcaccacgttctttcagagcttcagcagctttacacagcgtaccgccagtgtcgatcatatcatcgaccagtacgcagtcacgacctgcaacgtcaccgatgatatgcatcacctgtgaaacgttcgcacgcggacgacgtttgtcgatgattgccatatcggtatcgttcagcagcttagcgatagcgcgggcacgcacaacgccgccgatgtccggagaaaccacaattgggttatccagattcagctgcagcatgtcttccagcaggatcgggctaccaaatacgttatcaaccggaacgtcgaagaaaccctgaatctgttcagcgtgcagatccactgtcagcacacggtcaacaccgacgctggagaggaagtctgcaaccactttcgcagtgattggtacacgagcggaacggacgcgacggtcctggcgcgcatagccaaagtaggggataacagcggtgatacgacctgcggaagcacgacgcagggcatcaaccataacgactaattccatcaggttgtcgttagtaggggcacaagtggactggatgatgaaaatatcaccaccgcgtacattttcattaatttgtacgctgacttcgccatcgctaaagcgacctacagcggcgtcgccgagtgaagtgtacaggcggttggcaatacgttgtgctagttccggggtggcgttaccagcaaaaagcttcatatcaggcacgagaagaacctcaggcatgcgtccattggtggaaagaatctgccgaaaactgtgcgggccaggcatgatcctttccaggcggtgtattaaagagcgcgatgcaacgtctggaacaaggtgacgttgtcaccgaaactcagcttgcccggcttaaagcatggctctgtgcaatggggaaagattagcgcctttcgccacaaagccattgagccattccggggcttgctctagcacctggcgggcttcagactctgtatcaaattcagcaaagacacaggcccctgtcccagtcaggcgcgacggggcgtattctaacagccaggaaagcaccgcatcaacctcgcgaaaacgttttcttgcgataacctcgcaatcattgctgaattcacattttagcaacgtttctattgacctttttggcgtattgcgcgggagttcaggatctttaaaaatcaccggagtcggaatacttacaccagggtgcgccaccagataccacttctctggcggatccaccggcgttagtatttcaccaacgccttcggcaaacgcggcatgcccccgaacaaagacaggaacatctgcgcccagcgtcagccccatttccgccagctcatccatgcttagcccgcattgccagagatgatttaatgccaccaggaccgtcgcggcattggatgaaccaccgccgagaccgccgcccatcggcaaacgcttgtcaatgctgatattcgcaccgcttcccgtcggaagacgcccgctgtctgccgcagttttcatcaacaatcgcgctgcgcgaacgatcaggttatcttcatgttccacgccttcaacgggcgttaacagacgaatatccccatcgtcacgaagctcaatgctgatggtgtcgccgtaatcaagaaactgaaacagcgtttgcagcgtgtggtaaccatccgcacgctgaccggtaatgtataaaaacagattaagttttgccggagagggccactgtgtccgcattatttcactatccagttatccatttttaacttgatgcgttgaccaccgtcggtgagttccatattggctggcatcgcaggttgcgttttggtgtcataaccaccataaacaaccttccagtttttgccattctggctgtaggtaatttcgctcaggcggtactggtcgtccagtttgtagtcggttgcatcacccggtaaacctaaaatccactggcgcaagctgttgagcggaattggcattccggtcaatttgccaatcatctcttcggcgtcatcggcggtataacgctgacctttattgtcgactaactgcacgttacccggttgagcattcagctccagttccgtgctgcccaatgggttagtgagcagcagacggtagcgatcctggccggtttgctgccagaaaaagcgggcgtacactttttgttggtcagaaatataagcgaacgcgccgcgagtctgatactgattaagattgcgcacgtcttgctgatgctgacgccattgtggcgaatccgggcttttgccaggacctttgggcgtggtaacggaacaggcagtgagcacaagagcagccagcggtagcaggcggataagacgaaaatcgggcaggggcatagtgatgacaagtccttgagatacgttgcagttataacccttaatgctagcgttaccgtccgctatcgtctatgttcaagttgtcttaattgccagaatctaacggctttcggcaattactccaaaagggggcgctctcttttattgatcttacgcatcctgtatgatgcaagcagactaaccctatcaacgttggtattatttcccgcagacatgacccttttagcactcggtatcaaccataaaacggcacctgtatcgctgcgagaacgtgtatcgttttcgccggataagctcgatcaggcgcttgacagcctgcttgcgcagccgatggtgcagggcggcgtggtgctgtcgacgtgcaaccgcacggaactttatcttagcgttgaagagcaggacaacctgcaagaggcgttaatccgctggctttgcgattatcacaatcttaatgaagaagatctgcgtaaaagcctctactggcatcaggataacgacgcggttagccatttaatgcgtgttgccagcggcctggattcactggttctgggggagccgcagatcctcggtcaggttaaaaaagcgtttgccgattcgcaaaaaggtcatatgaaggccagcgaactggaacgcatgttccagaaatctttctctgtcgcgaaacgcgttcgcactgaaacagatatcggtgccagcgctgtgtctgtcgcttttgcggcttgtacgctggcgcggcagatctttgaatcgctctctacggtcacagtgttgctggtaggcgcgggcgaaactatcgagctggtggcgcgtcatctgcgcgaacacaaagtacagaagatgattatcgccaaccgcactcgcgaacgtgcccaaattctggcagatgaagtcggcgcggaagtgattgccctgagtgatatcgacgaacgtctgcgcgaagccgatatcatcatcagttccaccgccagcccgttaccgattatcgggaaaggcatggtggagcgcgcattaaaaagccgtcgcaaccaaccaatgctgttggtggatattgccgttccgcgcgatgttgagccggaagttggcaaactggcgaatgcttatctttatagcgttgatgatctgcaaagcatcatttcgcacaacctggcgcagcgtaaagccgcagcggttgaggcggaaactattgtcgctcaggaaaccagcgaatttatggcgtggctgcgagcacaaagcgccagcgaaaccattcgcgagtatcgcagccaggcagagcaagttcgcgatgagttaaccgccaaagcgttagcggcccttgagcagggcggcgacgcgcaagccattatgcaggatctggcatggaaactgactaaccgcttgatccatgcgccaacgaaatcacttcaacaggccgcccgtgacggggataacgaacgcctgaatattctgcgcgacagcctcgggctggagtagcagtacatcattttctttttttacagggtgcatttacgcctatgaagccttctatcgttgccaaactggaagccctgcatgaacgccatgaagaagttcaggcgttgctgggtgacgcgcaaactatcgccgaccaggaacgttttcgcgcattatcacgcgaatatgcgcagttaagtgatgtttcgcgctgttttaccgactggcaacaggttcaggaagatatcgaaaccgcacagatgatgctcgatgatcctgaaatgcgtgagatggcgcaggatgaactgcgcgaagctaaagaaaaaagcgagcaactggaacagcaattacaggttctgttactgccaaaagatcctgatgacgaacgtaacgccttcctcgaagtccgagccggaaccggcggcgacgaagcggcgctgttcgcgggcgatctgttccgtatgtacagccgttatgccgaagcccgccgctggcgggtagaaatcatgagcgccagcgagggtgaacatggtggttataaagagatcatcgccaaaattagcggtgatggtgtgtatggtcgtctgaaatttgaatccggcggtcatcgcgtgcaacgtgttcctgctacggaatcgcagggtcgtattcatacttctgcttgtaccgttgcggtaatgccagaactgcctgacgcagaactgccggacatcaacccagcagatttacgcattgatactttccgctcgtcaggggcgggtggtcagcacgttaacaccaccgattcggcaattcgtattactcacttgccgaccgggattgttgttgaatgtcaggacgaacgttcacaacataaaaacaaagctaaagcactttctgttctcggtgctcgcatccacgctgctgaaatggcaaaacgccaacaggccgaagcgtctacccgtcgtaacctgctggggagtggcgatcgcagcgaccgtaaccgtacttacaacttcccgcaggggcgcgttaccgatcaccgcatcaacctgacgctctaccgcctggatgaagtgatggaaggtaagctggatatgctgattgaaccgattatccaggaacatcaggccgaccaactggcggcgttgtccgagcaggaataatggaatatcaacactggttacgtgaagcaataagccaacttcaggcgagcgaaagcccgcggcgtgatgctgaaatcctgctggagcatgttaccggcagagggcgtacttttattctcgcctttggtgaaacgcagctgactgacgaacaatgtcagcaacttgatgcgctactgacacgtcgtcgcgatggtgaacccattgctcatttaaccggggtgcgagaattctggtcgttgccgttatttgtttcgccagcgaccttaattccgcgcccggatacggagtgtctggtggagcaggcactggcgcggttgcctgaacaaccttgccgtattctcgatctcgggacgggtaccggggcgattgcgcttgcgctggctagcgagcgcccggactgcgaaattatcgctgtagatcgtatgcctgatgctgtctccctggcacaacgtaatgcccagcatctggcgatcaaaaatatccacattctgcaaagcgactggtttagcgcgctagccgggcagcagtttgcgatgattgtcagcaatccgccgtatattgacgagcaggaccctcatcttcaacaaggcgatgtccgctttgagccgctcactgcgctggttgcggcagacagtggaatggcagacatcgtgcatatcatcgaacagtcgcgtaacgcgctggtatccggcggctttctgcttctggaacatggctggcagcagggcgaagcggtgcgacaagcatttatcctcgcggggtatcatgacgtcgaaacctgccgtgactatggtgataacgagcgcgtaacgctcggccgctattatcaatgacaagtttttctacactgcttagtgttcatcttattagtatcgcgctttctgttgggctattaaccttacgtttctggctacgttatcagaagcatccacaggcatttgctcgctggacgcgcattgtgccgccggttgtcgatacgctgttactgttaagcggcattgcgttgatggctaaagcgcacatcctgccattttccgggcaggcacagtggctgactgaaaagctgtttggagttatcatttatatcgttttgggttttattgcactcgattatcgtcgtatgcacagtcagcaggcgcgcattattgccttcccgctggcgttggtggtgctgtacatcatcattaaactcgccaccacaaaagtaccgttactggggtaagtcatgagatcgttagctgatttcgaatttaataaagcgccattgtgcgaaggcatgatcctggcttgcgaagcaatccgccgcgattttccctcgcaagatgtttacgacgaactggagcgtctcgttagtctggcgaaggaagaaatcagccagcttctgcctttagaagagcagttggaaaaactgatcgcgctgttttacggcgactggggatttaaagcctcacgcggtgtttatcgtctttccgatgcattatggctggaccaggtgttaaagaatcgacagggcagtgcggtatcattaggtgcggttttattatgggtcgcgaatcgtctcgatttgccgctgctgccggtgattttccctacgcagctgatattgcgcattgaatgtccggatggcgaaatttggctgattaatccttttaacggtgaatcgttaagcgaacatatgctggacgtatggttaaagggaaatatcagcccgtcggcggaactgttttatgaagaccttgatgaagctgataacattgaggtaatccgcaaattgctggatacactcaaagcctcgttgatggaagaaaatcagatggagctggcgttacgcaccagcgaagctttattacaattcaaccctgaagatccctatgaaattcgcgatcgcgggttgatttatgcgcaactggattgcgaacacgttgcgttgaacgatttaagttatttcgttgaacagtgtccggaagacccgatcagcgaaatgatccgtgcgcaaataaataacatcgcgcataaacatattgtgctgcattaattaatcgacattttactcaagattaaggcgatcctatgaaacaaaaagtggttagcattggcgacatcaacgtagcaaatgacctgccgttcgtactgtttggcggtatgaacgtgttggaatctcgcgatctggcgatgcgcatttgcgagcactacgtaactgtgacccagaaactgggtatcccttacgtgttcaaagcctcttttgacaaagccaaccgctcctccatccactcttatcgtggaccgggcctggaagaagggatgaaaatcttccaggagttgaagcagacttttggcgtgaaaattatcaccgacgttcacgaaccaagtcaggcacagcccgttgctgatgtcgtggatgtgattcagttgccggcgtttcttgctcgccagactgacctggttgaagccatggcgaaaaccggtgcggtaattaacgtcaagaaaccacagtttgtcagcccgggacagatgggtaatatcgttgataaattcaaagaaggcggcaacgaaaaagtgattctttgcgatcgcggtgctaacttcggctatgacaacctggttgtcgatatgctgggcttcagcattatgaagaaagtgtctggtaactcgccggtgattttcgacgtgacccacgcactgcaatgccgcgatccgtttggcgcagcttccggtggtcgtcgtgctcaggtggctgagctggcacgagccggtatggcggtaggtctggcggggctgtttattgaagcgcatccggatccggaacatgcgaaatgtgatggtccatccgcgctgccgctggctaaactggaaccgttcctcaagcagatgaaagcgattgatgatctggtgaaaggtttcgaagaactggataccagcaagtaatcttttttgcttgaaaaataaagtattagcgttctgcgttaagacttttttcatgggtgccggatacaaaaaaggccgcaggctgttacccctgcggccggtttcgggcgcatattgccatcacggcagcctgacgcccgttttcaccttacttccggttacgccaccagctgacaatcgctgcggtaataattcccgccaggatcggtgctgccaggtcgtgccagaaaatcatggcaaactgcgcgagcgtcatatagccgccttgttgtaatgacaacattttgcggctattcttgaattgttctggttcaagattagcccccgttctgttgtcaggttgtacctctcaacgtgcgggggttttctctttccagcaaccaatgccaccagggataaagcccccgcaacattgcgcctcaccggataacgccggcttggtgtggatactacgactcaattcatcttcacttcatccctgaaatgtttgcaatgaagagtgcattccggtttttcaacagctgttacagtcatttcatgagtgctctggatgaggcttccagctcgggttgccaatatttacttgtggaagtgataaagacaaaaatggccgcaggctgttacccctgcggccggtttcgggcgcatattgccatcacggcagcctgacgcccgttttcaccttacttccggttacgccaccagccgacaatcgctgcggtaataattcccgccaggatcggtgccgccaggtcgtgccagaaagtcatggcaaactgcgcgagcgtcatatagccgccttgttgtaatgacaacattttgcggctattcttgaagtgtctggtttcaagattagcccccgttctgttgtcaggttttacctctcaacgtgcgggggttttctctttccagcaaccaatgccaccagggataaagcccccgcaacattgcgcctcaccggataattccggcttggtgtggatactacgtctcaattcatcttcacttcatccctgaaatgtttgcaataaagagtacattccggcttttcaacagctgttgcagtcgtttcatgagtgctctggatgatgcttccagctcgggttgccaatatttacttgtggaagagataaagacaaaaatggccgcaggctgttacccctgcggccggtttcgggcgcatattgccatcacggcagcctgacgcccgttttcaccttacttccggttacgccaccagctgacaatcgctgcggtaataattcccgccaggatcggtgctgccaggtcgtgccagaaaatcatggcaaactgcgcgagcgtcatatagccgccttgttgtaatgacaacattttgcggctattcttgaagtgtctggtttcaagattagcccccgttttgttgtcaggttttacctctcaacgtgcgggggttttctctttccagcaaccaatgccaccagggataaagccccgcaacattgcgcctcaccggataacgccggcttggtgtggatactacgtcgcaattcatcttcacttcatccctgaaatgtttgcaatgaagagtacattccggcttttcaacagctgttgcagtggtttcgtgcagggtgtggtacaggctcgcaattctgattaacgacctgtccaggtagtatgaagaaatacaataagcaggaatttatattatctcccccgattaccgtcatcggaggagatataactgtcaggcaaatatcgtcatcaaataggcggcaaacagtgccagatgcgctgcgccattgagcacgttagtacgtccggtggagaaggagatatggcacagcactaaagaggccaccatcaccaccatttctggcgcaccaagtgcaaactgcaattcgttacccgtcataaaggcaattagcgtgacgacaggtacggtaagcgaaatggttgctaacactgaaccaaagaacagattcatcgcgcgctgaacctggttgttcaacactgcttttaatgcacctaaaccttccggcgacagaatcaacagtgccaccaggaagccagtaaaggcgacaggggcattcatgctgtcgagcaatgtctccagcgagctggcgttcattttggtcaccgcaataacggcaatcagatggataatcaaccagatagcatgccacaggctgctatgggcagacggtttaccgtgatgcgggtcgtcatcatcactgtcatcttcgtgctcgtagacaaacaaactttgatgcgttttggtctggatcagcaaaaatacgccatacattgccgcagaaattaatgctaccagtaacgcctgaccggttgaaaaattcgccgcaggcagagccattggaaataccagtacgattatcgccagggggaacagcgcaattaaatactgcttgataccaaacagattcatatattgggtggcaaacttacgaccgcccaacaataatgaaaagccaaccagcccaccggtaacaatcataatgattgaatagagcgtatcacgcattagcgttggcgcggcgtcgccggttgccattaaagctgaaatcaaactgacttcaagaataaccactgaaaggctaagaataagcgaaccgtaaggttctcccaggcgatgggctaatacgtccgcatgacggacaacactaaaggcgctacttaaaataccaataagcgcaagaagattgatggcaatgaccactggtagtgtctggctgcttccccacaggaacagcactaccagcgccagaaccgggaaaataagcgaagtctccttgtggcgggtttttaccgcctcttgagcatttgacattatggttatccctttgcagatgaatttatcgaaaatgtaaaaaataggtaggaaaaataacagaaagtgtctggatatcggtaacattttacgaatttttaccccgctgtcgattttttactcattggggcataaaaataagtattacgtttagacaatgtttgttttagcgtctcttaagaagagtctgacctgaaaattcttatgttttggcaagagtagatattgttgaccacacttaatgttcaactttgtaaaaggagtcaacgatgccgtataaaacgaaaagcgatctgccggaaagcgtaaagcacgttctaccgtctcatgcccaggatatctataaagaagcgttcaacagcgcatgggatcaatataaagataaagaagatcggcgtgatgacgccagtcgcgaagaaaccgcgcataaagtggcctgggctgctgtgaagcatgaatatgccaaaggggatgatgataaatggcataaaaaatcgtaaaaccggtcgcttagttaaagctattcgtgcggtgttgccttgcaagtggtccgtggattgcatattgtcccgttagtggtttcaaaatgagcagtaaaaatgtccggaagacaccaaaaagttgtcgcagggaagtatgcagtggcggaagtgtaaggtgataacgcgtgatttcttgatgaatgccgattgtaaaacggcatttggtgccattgaagaatcactcttatggtcagcagaacaacgggcggcttcgctggcggcgacgctggcttgtcgacctgatgagggaccggtgtggatcttcggctatggatcgttgatgtggaatccggcactggagtttaccgaatcgtgcaccggtacactggttggatggcatcgcgcattttgcctgcgcctgaccgccgggcgcgggactgcgcaccagccgggacggatgcttgcactgaaagagggcggacgcaccacaggcgtcgcctatcgactgccagaagagacgctggagcaggaactaaccctgttgtggaagcgagagatgattaccggctgttatctgccaacctggtgtcagcttgatcttgatgatggacgcacagtaaacgccattgtgtttattatggacccgcgacatccagaatatgaatctgatactcgcgctcaggtcatcgcgccgttgattgcggcggcgagcggtccgctgggaaccaacgcacaatacctgttttcactggaacaggagcttatcaaactgggaatgcaggacgatgggctgaatgatttgctggtatcggtaaaaaaactgctggcggagaattttccggatggtgtgttacgtccgggattcgcctgagtaaacttcccgcatagtggggcgtcagacgccccctcaaacattaaaatgtgagcactttatcggctgacagcgtccattgcgccagttccacaagagtaccgatttccaccccatcaatcagaggaagtgtactaatcccgcgcccgtcggtacaggttttgcacaatttcaccggtacattctgagcggtaaggatctccagcatttgctgaatgttgtagccttcccctggtttttgcccgcgcaacccggctgtgaccgcatcagacatgaggaacagacgcagatccagattgctctcctgctctcgtaacgcaatggccagccgcaagctgttaaacaaggattcgctcccgtaaggtgcgccattggcaacgatcacgattttttgcattatttactcctgtattcagggaattagacactcatcttctatcttactgcttctgcagcgtctgaccaatcggtcacatttttaaggattttcctgaaagcgcgagaaaatacgacaaaagttgccagtaatcgttattctttaaggctatggtttttcattattaccggaagttaccgacgttttgagccgtttcgttcctcgcattatcccgttttatttactcttgcttgtagcaggcggtacagctaacgcacaatctaccttcgagcaaaaagcggcaaatccctttgataataacaatgatggtctgccggatttaggcatggctcccgaaaatcatgatggggaaaaacactttgctgaaattgtgaaagatttcggcgaaaccagtatgaatgataacgggctggatactggcgagcaggcaaaagctttcgcattgggaaaagtccgcgacgcgcttagtcaacaggttaatcagcacgtagagtcctggctatcaccgtggggaaatgccagtgttgacgtcaaagtggataacgaaggacatttcaccggcagtcgtggaagctggtttgtgccgttacaagataatgatcgttatctcacctggagccagcttggtcttactcagcaggataatgggttggtgagcaatgtgggcgttgggcaacgctgggcgcgcggcaactggctggtgggttataacactttttatgacaacttgctggacgaaaatcttcagcgagcgggctttggtgccgaagcgtggggcgaatatttgcgattatcggcaaacttttatcagccgtttgctgcatggcatgaacagacagccacgcaggaacaacggatggcgcgcgggtacgacctgacagctcggatgcgcatgccgttctatcaacacctcaataccagtgtcagcctagaacagtattttggtgatcgtgttgatttgtttaactctggtacgggttatcacaatcccgtcgcgttgagtctgggattaaattacacccctgtgccattagtcactgtgacggcccagcataaacagggtgaaagtggcgaaaatcaaaataacctcgggctgaatcttaattaccgctttggtgtaccgctcaaaaaacaactttctgcgggcgaggttgccgaaagtcagtcgttacgtggtagtcgctatgacaatccgcagcgaaataatctaccgactcttgagtaccgacagcgaaaaacgttaacggtgtttctggcgacaccgccgtgggatctaaaacctggcgaaacagtgccgctgaaattacaaatccgcagtcgttacggtattcggcaactgatttggcagggcgatacgcagatattaagtttgacgccgggcgcacaagccaacagcgcggagggctggacgctgatcatgcctgactggcagaacggggaaggggcaagcaatcactggcgattgtctgtggtggtggaagataaccaggggcagcgtgtctcctccaatgagatcacgctaacgcttgtcgaaccgttcgatgcattgtcaaacgacgaactgcgctgggaaccgtaatcagaaaatgcgctcctgatgcacccataccgctgcttccacgcgagacttgagcttcattttcttcagcatgtgcttgacgtgcacttttactgtgctttcggtgatatccaggcggcgggcaatcatcttgttcggcaaaccctgggcaatcagcttgagaatatcgcgctcgcgtggggttaactggttaacatcgcgctcagtagtggcacggttagcgcgcaagctggcggccagaacaggcgttaatgcttcgcttaataccatttcgccagcagctgcctgatgcaatgctttcagcagatcttccggttccatatcttttaacagatagccatccgcgccgcgtttcagtgcggtgaccacatcttcttcatggttagagacgctgaataccacaatgcgccctgagagggacttttcgcgcagtttatccagcgtttccagaccgttcatgccgggcatattgagatctaacaggatcagatcgggatcaagagactccgccagttcaataccctgttcgccattactcgcttcgccaaccacggtgatatctggtgccatactgataagctgttttacgccagttcgcagcatcgggtgatcgtcaatcagcaggatagtagccggttcctgattactcatgggtatctccttggacgtctgtgaaagttttttcgggaataaaggtgaccaccacttcggtgccacctgattcacgacggcggacgcggcaatcgcctcgtaaactttgcgcacgatcgcgcattattatcatgccgtagtgattgctgcggatggcattttcaggcacgccgcagccgttatcctggacggtcagtttgacctgattatcgttttgcgccaccgtcaccacgacttcactcgcttgcgaatgtttgagggcgttacttaatgcctcacgggcaatttgcaacaagtggattgcctgatgcgaaggcaccaggcgaggcggcaattgataatccagcttcaccgggaagccaaatttggcgctgtactcttcgcaactcgcctccagcgccggacgtaatccaggctcggtgagctgcaagcggaatgtggtgagcaattcacgcaactgcgcccaggatgcattcagttcgttacggatctgacttaacagttcgcggctgctttctggcagcgcatcgccctgcatctgtaaacaactcacctgcatcttcatgcaagagagagattgggcaatagaatcatgcagttcgcgcgcaatggtggcacgctcttccatcacgatcaactgttgctgacgttcctgatggcgatccagcgccagcgtggcggtgagttgttcaaccagggtatccaccagttgttgttgatcatggctaagatgacgcccctgcggcagggtcgccagcaaaataccgtactgcgtatgagagtcagccagccgccacttcagggtcgtgccgcgatcaccaacgggtaatacgccgcgcgggcagagctggcagcctttatcatcacaagtcatatctggctggcaggtaaactcctgatgattctcttcatcatcagtgtcatacacccgcaattcgatatcacgtagcagggttaaattctgtaagccgttgagtacaggtgacaggcgttcacacagcggggcgcgggaatgcaaacggcggttagcctgccataaaaaagagaggatctgatttttatgctccagcccggcggttttctcctgaacccgctgctcaagtacggcataactttcggccagttctgcagacatattgttcaacgcagttccaagcatcgccatttcgttgcgcccgctgatgtttgcgcgttgggtaaaatcgcgatgactgacggcactcgccattgccagcagttgccgccacggttgtagcagtcgcgcccgcaaccagataatagtgaacaccagtaaaagtgccataaataccgccattacccgatggaccagtaccactgtctcgatgcgcatttccgtggtgcggtcaaaaccagataccagttgatcaagcccggcaacaaactggctgacatccgctgacaccgtttctcggttttgtgcacgcatcagcgcagggatcagttcattacgccagtaatcttgtaaaccctgtaattgcgccagttgtccgtctcgttctgctgctcgagtcaactcggcgctaaatgccgtttgttccatctctttaattaagggcttgtctttctcgcttaatggcactgccgccaacagacggtaactttgcatgcgcagcgatcccgctttgttgatcgcatgggcgctgccctgaacgccttgcaccagccagccagaaaccgccatccctgccagtccaatagcagtagaaagcaacacaataagcgcaacctgattaaccagggtgagcggagagagacaacgtttaagcatgtaaacctcttccttcaggctttaaatgagcaataaccttaatgaatgtgacgatacattctggaatggcagtattctcggctattggctgaagtatacccatacccggaaagagttactccttatttgccgtgtggttagtcgctttacatcggtaagggtagggattttacagcaccgtgaaaaatctcataatttttatgaagtcactgtactcactatgggtaatgataaatatcaatgatagataaagttatcttatcgtttgatttacatcaaattgcctttagctacagacactaaggtggcagacatcgaaacgagtatcagaggtgtctatgagtcactcatccgcccccgaaagggctactggagctgtcattacagattggcgaccggaagatcctgcgttctggcaacaacgcggtcaacgtattgccagccgcaacctgtggatttccgttccctgtctgctgctggcgttttgcgtatggatgttgttcagcgctgttgcggtgaacctaccgaaagtcggctttaattttacgaccgatcagctatttatgttgactgcgctgccttcggtttctggcgcgttattacgtgttccatactcctttatggttcctatcttcggtggtcgtcgctggacggcgttcagcaccggtattctgattattccttgcgtctggctgggttttgccgtgcaggatacctccacgccttatagcgtcttcatcatcatctctctgctatgcggctttgctggcgcgaacttcgcatccagtatggcaaacatcagcttcttctttccgaaacagaagcagggtggcgcgctgggtctgaatggtggtctgggaaacatgggcgtcagcgtcatgcagttggttgctccgctggtggtatcactgtcgattttcgcagtatttggtagccagggcgtcaaacagccggatgggactgagctgtatctggcgaatgcgtcctggatatgggtgccgttccttgccatcttcaccattgcggcgtggtttggcatgaacgatcttgctacctcgaaagcctccatcaaggagcagttgccggtactcaaacggggtcatctgtggattatgagcctgctgtatctggcaaccttcggctccttcatcggcttctccgcgggctttgcaatgctgtcaaaaacgcagttcccggatgttcagattctgcaatacgctttcttcgggccgtttattggtgcgctggcgcgttctgcaggtggtgcattatctgaccgtctgggcggaactcgtgtcacgctggtgaactttattctgatggcgattttcagcggcctgctgttcctgaccttaccgactgacgggcagggcggaagcttcatggcgttcttcgcggtcttcctggcgctgttcctgacagctgggctgggtagtggttccactttccagatgatttcagtgatcttccgtaaactgacaatggatcgcgtgaaagcagaagggggttctgacgaacgtgcgatgcgtgaagcggcaaccgacacggcggcggcgctgggtttcatctctgcgattggcgcgattggtggcttctttatcccgaaagcgtttggtagctcgctggcattaacgggttcgccagtcggcgcaatgaaggtatttttgattttctatatcgcctgcgtagtgattacctgggcggtatatggtcggcattctaaaaaataaaccgttactcgtcatacttcgggttacatgtgctgcggctgcgttcattcaccccagtcacttactttagtaagctcctgggattcattcacttgccgccttcctgtaaaccgaattatatagagtaaaatatttgattatcctttgcgcggcatgatgtcgcgctttttttatgcgtcatttagttacaacatactaatgttatatggtttatttcgccggatttcattaagagccattaatatgttacccatggggaatactccttaatacccatctgcataaaaatcttaatagtttaaataactacaggtataaaacgtcttaatttacagtctgttatgtggtggctgttaattatcctaaaggggtatcttaggaatttactttatttttcatccccatcactcttgatcgttatcaattcccacgctgtttcagagcgttaccttgcccttaaacattagcaatgtcgatttatcagagggccgacaggctcccacaggagaaaaccgatgagtaaattcctggaccggtttcgctacttcaaacagaagggtgaaacctttgccgatgggcatggccagcttctcaataccaaccgtgactgggaggatggatatcgccagcgttggcagcatgacaaaatcgtccgctctacccacggggtaaactgcaccggctcctgcagctggaaaatctacgtcaaaaacggtctggtcacctgggaaacccagcagactgactatccgcgtacccgtccggatctgccaaaccatgaacctcgcggctgcccgcgcggtgccagctactcctggtatctttacagtgccaaccgcctgaaatacccgatgatgcgcaaacgcctgatgaaaatgtggcgtgaagcgaaggcgctgcatagcgatccggttgaggcatgggcttctatcattgaagacgccgataaagcgaaaagctttaagcaggcgcgtggacgcggtggatttgttcgttcttcctggcaggaggtgaacgaactgatcgccgcatctaacgtttacaccatcaaaaactacggcccggaccgtgttgctggtttctcgccaattccggcaatgtcgatggtttcttacgcatcgggtgcacgctatctctcgctgattggcggtacttgcttaagcttctacgactggtactgcgacttgcctcctgcgtctccgcaaacctggggcgagcaaactgacgtaccggaatctgctgactggtacaactccagctacatcatcgcctgggggtcaaacgtgccgcagacgcgtaccccggatgctcacttctttactgaagtgcgttacaaagggaccaaaactgttgccgtcacaccagactacgctgaaatcgccaaactgtgcgatctgtggctggcaccgaaacagggcaccgatgcggcaatggcgctggcgatgggccacgtaatgctgcgtgaattccacctcgacaacccaagccagtatttcaccgactatgtgcgtcgctacaccgacatgccgatgctggtgatgctggaagaacgcgacggttactacgctgcaggtcgtatgctgcgcgctgctgatctggttgatgcgctgggccaggaaaacaatccggaatggaaaactgtcgcctttaataccaatggcgaaatggttgcgccgaacggttctattggcttccgctggggcgagaagggcaaatggaatcttgagcagcgcgacggcaaaactggcgaagaaaccgagctgcaactgagcctgctgggtagccaggatgagatcgctgaggtaggcttcccgtactttggtggcgacggcacggaacacttcaacaaagtggaactggaaaacgtgctgctgcacaaactgccggtgaaacgcctgcaactggctgatggcagcaccgccctggtgaccaccgtttatgatctgacgctggcaaactacggtctggaacgtggcctgaacgacgttaactgtgcaaccagctatgacgatgtgaaagcttataccccggcctgggccgagcagattaccggcgtttctcgcagccagattattcgcatcgcccgtgaatttgccgataacgctgataaaacgcacggtcgttcgatgattatcgtcggtgcggggctgaaccactggtatcacctcgatatgaactatcgtggtctgatcaacatgctgattttctgcggctgtgtcggtcagagcgggggcggctgggcgcactatgtaggtcaggaaaaactgcgtccgcaaaccggctggcagccgctggcgtttgcccttgactggcagcgtccggcgcgtcacatgaacagcacttcttatttctataaccactccagccagtggcgttatgaaaccgtcacggcggaagagttgctgtcaccgatggcggacaaatcccgctataccggacacttgatcgactttaacgtccgtgcggaacgcatgggctggctgccgtctgcaccgcagttaggcactaacccgctgactatcgctggcgaagcggaaaaagccgggatgaatccggtggactatacggtgaaatccctgaaagagggttccatccgttttgcggcagaacaaccagaaaacggtaaaaaccacccgcgcaacctgttcatctggcgttctaacctgctcggttcttccggtaaaggtcatgagtttatgctcaagtacctgctggggacggagcacggtatccagggtaaagatctggggcaacagggcggcgtgaagccggaagaagtggactggcaggacaatggtctggaaggcaagctggatctggtggttacgctggacttccgtctgtcgagcacctgtctctattccgacatcattttgccgacggcgacctggtacgaaaaagacgacatgaatacttcggatatgcatccgtttattcacccgctgtctgcggcggtcgatccggcctgggaagcgaaaagcgactgggaaatctacaaagccatcgcgaagaaattctccgaagtgtgcgtcggccatctgggtaaagaaaccgacatcgtcacgctgcctatccagcatgactctgccgctgaactggcgcagccgctggatgtgaaagactggaaaaaaggcgagtgcgacctgatcccaggtaaaaccgcgccacacattatggtcgtagagcgcgattatccggcgacttacgaacgctttacctctatcggcccgctgatggagaaaatcggtaatggcggtaaagggattgcctggaacacccagagcgagatggatctgctgcgtaagctcaactacaccaaagcggaaggtccggcgaaaggccagccgatgctgaacaccgcaattgatgcggcagagatgatcctgacactggcaccggaaaccaacggtcaggtagccgtgaaagcctgggctgccctgagcgaatttaccggtcgtgaccatacgcatctggcgctgaataaagaagacgagaagatccgcttccgcgatattcaggcacagccgcgcaaaattatctccagcccgacctggtctggtctggaagatgaacacgtttcttacaacgccggttacaccaacgttcacgagctgatcccatggcgtacgctctctggtcgtcagcaactgtatcaggatcaccagtggatgcgtgatttcggtgaaagcctgctggtttatcgtccgccgatcgacacccgttcggtgaaagaagtgataggccagaaatccaacggcaaccaggaaaaagcgctcaacttcctgacgccgcaccagaagtggggtatccactccacctacagcgacaacctgctgatgctgactttaggtcgcggtggtccggtggtctggttgagtgaagccgatgccaaagatctgggtatcgccgataacgactggattgaagtcttcaacagcaacggtgctctgactgcccgtgcggttgtcagccagcgtgttccggcagggatgaccatgatgtaccacgcgcaggaacgtatcgttaacctgcctggttcggaaattacccaacagcgtggtggtatccataactcggtcacccgtatcacgccgaaaccgacgcatatgatcggcggctatgcccatctggcatacggctttaactactatggcaccgtaggttctaaccgcgatgagtttgttgtagtgcgtaagatgaagaacattgactggttagatggcgaaggcaatgaccaggtacaggagagcgtaaaatgaaaattcgttcacaagtcggcatggtgctgaatctcgataagtgcatcggctgccacacctgttcagttacctgtaaaaacgtctggaccagccgtgaaggcgtggaatatgcgtggttcaacaacgtggaaaccaagccgggccagggcttcccgactgactgggaaaaccaggaaaaatacaaaggcggctggatccgtaaaatcaacggcaaactgcagccgcgcatgggtaaccgtgccatgctgctgggtaaaatcttcgctaacccgcatctgccggggatcgacgattattacgagccgttcgattttgactatcagaacctgcataccgcgccggaaggcagcaaatcgcagccgattgcccgtccgcgttcgctgattaccggggaacggatggcgaaaatcgaaaaagggccgaactgggaagatgacctgggcggtgagtttgacaaactggcgaaagacaagaacttcgacaacatccagaaggcgatgtatagccagttcgaaaacaccttcatgatgtatttgccgcgcctgtgcgaacactgcctgaacccggcatgtgtggcgacctgcccgagcggtgcgatttacaagcgtgaagaagatggcatcgtcctgatcgaccaggataaatgccgtggctggcgtatgtgcatcactggatgcccgtacaaaaaaatctacttcaactggaagagcggtaagtctgagaagtgcatcttctgctatccgcgtattgaagcgggtcagccgaccgtgtgctcagaaacctgtgtcggtcgtatccgttatcttggcgtgctgttgtacgatgccgacgctattgaacgtgcagccagcaccgagaacgagaaagatctttaccagcgtcagctggacgtgttcctcgatccgaacgatccgaaagtcatcgagcaggcgattaaagacggtattccgctgagcgttattgaagccgcacagcagtcgccggtttataaaatggcaatggaatggaaactggcgctgccgctgcatccggaatatcgcacactgccgatggtctggtacgtgccgcctctgtctccgattcagtctgcagcagacgcgggtgagctgggtagcaacggcattctgccagacgtcgaaagcctgcgtattccggtacagtatctggcgaatctgctgaccgccggtgataccaaaccggtactgcgcgcactgaaacgtatgctggcgatgcgtcattacaaacgtgctgaaaccgttgacggtaaagttgatacccgtgcgctggaagaggtcggtctgaccgaagcccaggcacaggagatgtaccgttatctggcgattgctaactacgaagatcgctttgtggtgccgagtagtcatcgtgaactggcacgggaagccttcccggagaaaaatggctgcggctttacctttggtgatggctgccacggttcagataccaaattcaatctgttcaacagccgtcgtatcgatgccatcgatgtgaccagcaaaacggagccgcatccatgatcgaactcgtgattgtatcgcgtctccttgaatatccggatgctgccttatggcagcatcaacaagagatgtttgaggcgattgccgcgtcgaaaaatctgccaaaagaggatgcccatgcgctgggcattttcctgcgcgatttaacgacgatggatccgctcgatgcccaggcgcagtacagcgaactgttcgaccgtggccgcgccacgtcactgttgctgtttgaacatgtgcacggcgaatcccgcgaccgcggccaggcgatggtggacctgctggcgcagtacgagcagcacggcttgcagttaaacagccgcgaattgccggaccatctgccgctgtatctggagtacctggcgcagctgccgcaaagcgaagccgtggaaggtttgaaagatatcgcgccgattctggcattgctgagcgcgcgtctgcaacagcgtgaaagccgttatgccgtgctgtttgatctgctgctgaaactggcgaataccgctatcgacagcgacaaagtggcggaaaaaattgccgacgaagcgcgcgatgatacgccgcaggcgctggatgctgtctgggaagaagagcaggttaaattctttgctgacaaaggctgcggtgattcagcaatcactgcgcatcagcgtcgctttgccggtgccgtcgcgccgcaatatctgaatatcaccaccggaggacagcactaatgcaattcctgaatatgttcttctttgatatctacccgtacatagccggggcggtcttcctgattggtagctggctgcgttatgactacgggcagtacacctggcgcgcggcgtccagccagatgctggatcgcaaagggatgaacctggcgtcgaacctgttccatatcgggattctggggatttttgtcggtcacttcttcggtatgctgacgccgcactggatgtatgaagcctggctgccgattgaagtgaaacagaaaatggcaatgtttgctggtggtgccagcggcgtgctgtgtctgattggcggcgtgctgttgctgaaacgtcgtctgttcagcccacgcgtgcgtgcaaccactaccggagcggatatcctgatcctgtcgctgctcgttatccagtgcgcgctgggcctgttgaccattccgttctccgctcagcatatggacggtagcgagatgatgaaactggttggctgggcgcagtcggtggtgaccttccacggtggcgcttctcaacacctcgatggtgtggcgtttatcttccgtctgcacctggtgctggggatgacgttattcctgctgttcccgttctcgcgtctgatacacatctggagcgtaccggtggagtatctgacacgtaagtaccagctggtgcgcgctcgtcactaagcgaattttagttcacatagaccctgcttcggcggggtttttttatgggcacggtgcggggtgagttgtcggatgcgcttcgcttatccgacctacaggggaggatattgtaggcccggtaaacgtggtgccatcgggcaaaattagctcggagtaacaggttttgattatttaaggaagcgatggtggtgggggaaggattactcagcgctgcgcgcttcgcccttcgggtcgttgcctgcggcaacgctctctcgctggcgctcaagtcgaaccttggtcgaagcttctcatccttccccgcttgggcagaatatttgattgcggattcgtttgagaattccggggcttttgaaagtgatggtggtgggggaaggattactcagcgctgcgcgcttcgcccttcgggtcgttgcctgcggcaacgctctctcgctgacgctcgagccgaaccttagtcgaagcttctcatccttccccgcatgggcagaatatttgattgcggattcgcttgagagttcagggacttttgaaagtgatggtggtgggggaaggattactcagcgctgcgcgcttcgcccttcgggtcgttgcctgcggcaacgctctctcgctggcgctcgagtcgaaccttggtcgaagcttctcatccttccccgcatgggcagaatatttaattgcggattcgttgggaagttcagggacttttgaaagtgatggtggtgggggaaggattcgaaccttcgaagtcgatgacggcagatttacagtctgctccctttggccgctcgggaaccccaccaggggtaattcaaattttgaggtaatgcttgagatggtggtgggggaaggattattcgtcgcttcgctcctcacccttcgggccgttgcctgtggcaacgttctctcgctttcgctcgaatcgaaccttagtcgaaggttctcacccttccccgatgagtgcaaactttcacaatctcaccgaagttaccacatcgctgtggtgaattatggtggtgggggaaggattcgaaccttcgaagtcgatgacggcagatttacagtctgctccctttggccgctcgggaaccccaccacggggtaatgctttttactggcctgctcccttatcgggaagcggggcgcatcatatcaaatgacgcgccgctgtaaagtgttacgttgagaaaaatgaactggttgcgtaattttcatccgtaacggattaaaggtaaccagttatttttgctggcgattaaagaataatcgttcgattaccgtaaacaaagacgcgctgtgccagtactttgtatagtgcacgacttaagacgtttttctcgacgtcacgacctgcgcgcatcatatcttcagctgtgtaggtatgatcgacatgaataacgtcctgcatgatgattgggccttcgtccagattgtcattcacatagtgagcggttgcgccaataatcttcacaccacgttcataggcctggtgataaggacgtgcgccaataaacgctggcaggaatgaatggtgaatattgatgatcttattcgggaagcgtgccacaaattccggcgttaatacccgcatatacttcgccagcaccacgtagtcaggttgataagcatcaatggcatccgccatcttttgatcgtgctcgttgcgggttaacccttcatggcttaccagctcaaacggaatatcaaaacgctcaaccagagaacgtaaagtatcgtggttaccaataactgccgcgatttcgacatccaggccgccgtaattggctttcatcaacaaatcgccaaggcaatgcgcttctttagtgaccagaatcactatccggcgacgaccggcaggattcagctcacgcacggagccttctggcaatgcgctatcgagatccgccagcagggtggaatcattaaaaatcccttccagttccgtgcgcataaaaaagcgcccggtacggtgatcaacaaattcattgttctgtacgatatttaactcgtgcttgtagcaaatattggtaatacgtgcgatcagacctttttggtccggacaaatagtacgcagaactttacgttggagtgaatgcattgctggaaaaaccttgttgagagtgtttgctaaaccgtaccgtcaaccattattggccgcagcactttttaaattttttacctgaaccacaagggcagggatcgttgcgaccaaactgcggacgtgtaccgtcaatatagtaccattgaccgttttctttcaaaaatcgcgaacgttcaattattgcacctgttttaccaccttcggtaaatcgagcaacaaaactgacaaatccgatattgtcggcgtcctgccaacaatgttcaaatacggtcaatcccaaccattcagtatgcgcaaatccggccatcaattcggcacgtaacgccgctgctccacaagagggatgccaggtctttattaaataatctgcgtcttgcatcacaaaagcgcagtaacgcgaacgcatgagatgttctggatcaggtgcaaccttttcaccagacacataagggtggcaacataggctatactcgacagcactaccacagggacaaagctgagacacaaataatctccctggaaacaataacggcgtattaaccgcctgagtagcactatgttaaccgagcagtagcgatgtggctacgattgcattccaggggaatcttgcgggaataatgagaaagataaaaatagggctggcgctgggatctggcgcggcgagaggttggtcgcatattggcgttattaatgcgctaaaaaaagtgggtattgaaattgatatcgttgcaggatgttcaattggttcgctggtgggcgctgcctatgcatgcgatcgattatctgcgctggaagattgggtgacctctttcagttattgggatgttttacgcctgatggatctctcctggcagcgcggtgggttactgcgcggcgagcgtgtcttcaatcaataccgcgaaataatgccggaaacagagatcgaaaattgttcccgtcgctttgcggctgttgccaccaatttaagtacgggacgtgaattatggtttactgaaggcgatctccatcttgctattcgcgcatcatgcagtattccaggactcatggcacctgttgcacataacggctactggctggttgatggagcagtcgttaacccaattcctatttccctcacgcgtgcattgggggctgatattgtgatagcggttgacctgcagcacgatgctcatttgatgcaacaagatttgctctcctttaatgtcagtgaagaaaatagcgagaatggtgattctctgccgtggcatgcgcgtctgaaagaaaggttaggcagcataacgacacgtcgggcggtgacagcgccaacggcaacagagattatgaccacttctatccaggtgctggagaaccgccttaaaaggaaccgcatggcaggtgatccgcccgatattctgattcaacctgtttgcccgcaaatatctacgcttgatttccatcgcgcgcacgctgccattgcggccggacagctggcagtggaaaggaaaatggacgaacttttgccgttggtacgcaccaacatttgaccagaatttttatctacacttaagttaattctgacaggcgcaggtggcaatagcatgccactattgagtaaagccagtcaggggagagaacatgacgcagccattggtcggaaaacagattctcattgttgaagatgagcaggtatttcgctcgcttctggattcatggttttcctcattgggagcgacaacggtactggcggctgatggggtggatgcccttgagttgctgggaggtttcactccagacctgatgatatgtgatatcgcgatgccacgaatgaacgggcttaaactgctggagcatatacgtaacagaggcgaccagaccccagttctggtgatatctgccactgaaaatatggcagatattgccaaagcgttacgtctgggcgttgaagatgttttgctgaaaccagttaaagatctgaatcgcttgcgcgagatggtttttgcctgtctctatcccagcatgtttaattcgcgcgttgaggaagaggaaaggctttttcgcgactgggatgcaatggttgataaccctgccgcagcggcgaaattattacaggaactacaaccgccggttcagcaggtgatttcccattgccgggttaattatcgtcaattggttgccgcggacaaacccggcctggtgcttgatattgccgcactttcggaaaacgatctggcattttattgccttgatgtcacccgagctggacataatggcgtacttgctgccttgttattacgcgcattgtttaacggattattacaggaacagcttgcacaccaaaatcaacggttgccagagttgggcgcgttattgaagcaggtaaaccatttacttcgtcaggccaatctgccggggcagtttccgctattagttggctattatcatcgcgaactgaaaaatctcattctggtttctgcgggtctgaatgcgacgttaaataccggcgaacaccaggtgcaaatcagtaatggtgttccgttaggcactttaggtaacgcttatttgaatcaattgagccagcgatgcgatgcctggcaatgccaaatatggggaaccggtggtcgactgcgcttgatgttgtctgcagaatgagcaaacgataacgcgggctaaatttgcattacctgctaatgtcggctggtggtactatcgtcgccattcgtataagtaattgtcttaattatgctaactcgcctccttttcagaacttagccccttcggggtgctgatatactgggatgcgatacagaaatatgaacacgttcaaaacacgaacagtccaggagaatttaaatggctgccattaatacgaaagtcaaaaaagccgttatccccgttgcgggattaggaaccaggatgttgccggcgacgaaagccatcccgaaagagatgctgccacttgtcgataagccattaattcaatacgtcgtgaatgaatgtattgcggctggcattactgaaattgtgctggttacacactcatctaaaaactctattgaaaaccactttgataccagttttgaactggaagcaatgctggaaaaacgtgtaaaacgtcaactgcttgatgaagtgcagtctatttgtccaccgcacgtgactattatgcaagttcgtcagggtctggcgaaaggcctgggacacgcggtattgtgtgctcacccggtagtgggtgatgaaccggtagctgttattttgcctgatgttattctggatgaatatgaatccgatttgtcacaggataacctggcagagatgatccgccgctttgatgaaacgggtcatagccagatcatggttgaaccggttgctgatgtgaccgcatatggcgttgtggattgcaaaggcgttgaattagcgccgggtgaaagcgtaccgatggttggtgtggtagaaaaaccgaaagcggatgttgcgccgtctaatctcgctattgtgggtcgttacgtacttagcgcggatatttggccgttgctggcaaaaacccctccgggagctggtgatgaaattcagctcaccgacgcaattgatatgctgatcgaaaaagaaacggtggaagcctatcatatgaaagggaagagccatgactgcggtaataaattaggttacatgcaggccttcgttgaatacggtattcgtcataacacccttggcacggaatttaaagcctggcttgaagaagagatgggcattaagaagtaacatccgtatcggtgttatccacgaaacggcgttgagcaatcgacgccgtttttttatagcttattcttattaaattgtcttaaaccggacaataaaaaatcccgccgctggcgggattttaagcaagtgcaatctacaaaagattattgcttgatcaggaaatcgtcgagggatttaccttgctcatccattgcttttttgattacagctggagtacggccttggccagtccaggttttagtttcgccgttttcgtcaacgtagctatattttgccggacgctgagcacgtttagctttggtgccagatttaacggcagcaaggctattcagcagttcgttcgggtcaataccgtcagcgatcagcatttcgcgatattgctgcagtttacgagtgcgctcttcaacttcagcagcagccgcgctttcttcttcgcgacgttcgttaacaacaacttctaatttttccagcatttcttccagcgtttcaagtgtacattctcttgcctgcgcacgaagagtacggatgttgttcagaattttaagtgcttcgctcattgtagtaatctcaaacttatattggggtggtttgttgaggtaataatagagccttaaattcagttgtgcaatagccaggaatgtaaggaattcaaaattgttctttattttgtgccgccaataaatatcttttcataaaattagccagaaaagacgcggcatatagccctatttacaccgatgatttcgcagcacgtgaggttaaaacttcctgattcatgtcacattttatggggagattatcgtaggctgacgacctttcagtcttctgtattagttgtgtttacgagaattccctattaagcgaatgatgaaaagtagaacagtcgcaataagagcatggacttagtattgcactatctcctggaggtcaacagagggctattacttgcgcaacaggttaaagattgtgaatagttaccagcagtcatttacccgcttataacaagcgaggcagttgtaatgatagctcagaaggattatgcaaggcttcgtaagggagaacgcatatacccacttctgtgcatactgttgagctgaaaaactgacgaattatgataaactccagccaactttatttcatatcattgagggcctgtggctgatggcacagctatatttctactattccgcaatgaatgcgggtaagtctacagcattgttgcaatcttcatacaattaccaggaacgcggcatgcgcactgtcgtatatacggcagaaattgatgatcgctttggtgccgggaaagtcagttcgcgtataggtttgtcatcgcctgcaaaattatttaaccaaaattcatcattatttgatgagattcgtgcggaacatgaacagcaggcaattcattgcgtactggttgatgaatgccagtttttaaccagacaacaagtatatgaattatcggaggttgtcgatcaactcgatatacccgtactttgttatggtttacgtaccgattttcgaggtgaattatttattggcagccaatacttactggcatggtccgacaaactggttgaattaaaaaccatctgtttttgtggccgtaaagcaagcatggtgctgcgtcttgatcaagcaggcagaccttataacgaaggtgagcaggtggtaattggtggtaatgaacgatacgtttctgtatgccgtaaacactataaagaggcgttacaagtcgactcattaacggctattcaggaaaggcatcgccacgattaataagaatttctttactgacagggtgagcagggcacttttatcctgtcagttcgttttacgcacttcttccgggctatatacccttctcggcagttttttaacgccgctatacgcctcacagggctcttaagcaccgacgttgacttgtgacctgtaaagtacaatatccctgtgtttaggcgttatacatcgtcgcaaatatgatgaaggctaatgctgtcggtttatggaaaagttgctttgggtaaacaaaaaatacggccccagaagggcaatgccgttcacttaagaggagcggcactatgtttcacaggataacgggtttttgatatcttaaccgacctcggccttgatggtcgggggcgttttgttatgaacaccacttccagagcaccccgaagatgctccagtcgtttcgggatggtccctggtgacgccgtgtttcccagctctatcatttctgatgcgatattcttccacgcaggcagtagccagtggcggttacaacccttctggttcagcgtcagcagcaggtcttcgctgtaaaaaagtttatcaaacaacgtaatagagttatccgggatggtggcgagcatggagtgggccagcacagtttcgctctgccggtaaggtgcggtcacggcattcagcagaatgtgacttcccaggttcattaaggccaccagacgcataaccgggtaggcgttctgccgcttagtggatgtgttggcagacccataatattcacgcagctcgggtttatcaggtgtcctgaactgtgcgccatcaatggcaaaaagttgcaggccgtgccagtcatccttcaggtaacgttccgcgcccctgtctgtgcggtctggcggaagagccattccactggggcggcccccacgcgctgacgcgcctgggtgacagcgctgcgggccagcaggttcatccccgcttcgccatccgcgctcaggttcagacggcgaacaacatcggtaattggctcattgcaccaccatccagataaccatgtcccccggtaaacgacggcggcgaacggtcgcatgagcagaaagcgtcaggcagtgttgtatccactcggtgggaaggtgttctgcaaatagttgtgcagagggcggaggcataagcggatggtcactgaaatcgagcagatcattgagaagtggcataagaaaacggctccctgttgtggaagccgttatagtgcctcagtttaaggatcggtcaactaatccttaactgatcggcattgcccagaaggggccgtttatgttgccagacagcgctactgattaagcggattttttcgcttttttctcagctttagccggagcagcttctttcttcgctgcagtttcaccttctacataatcacgaccgtagtaggtatccagcagaatctgtttcagctcggagatcagcgggtaacgcgggttagcgccggtgcactggtcatcgaatgcatcttcagacagtttatccacgttcgccaggaagtctgcttcctgaacgccagcttcacggatagatttcggaatacccagttcagctttcagcgtttccagccatgccagcagtttctcgatcttagcagcagtacggtcgcccggtgcgctcagacccaagtggtcggcaatttcagcataacgacggcgagcctgcggacggtcatactggctgaatgcagtctgcttggtcgggttgtcgttcgcattgtagcgaataacgttacaaatcagcagggcgtttgccagaccgtgcggaatatggaactgggaacccagtttgtgcgccattgagtgacatacacccaggaaggcgttcgcaaacgcgatacccgcgatagtcgctgcactgtgaacacgttcacgcgctaccggatttttagacccttcgtggtaggacgctggcagatattctttcagcagtttcagtgcctgcagagcctgaccatcagagaactcagatgccagtacagaaacataagcttccatggcgtgagttactgcgtccagaccaccgaaagcacacagggacttcggcatgtccataaccaggttggcgtcgacaatcgccatatccggagtcagcgcatagtctgccagcggatatttctgaccagtagcgtcgtcagttacaaccgcaaacggagtgacttcagaacctgtaccagaagtggtggtgacagcgatcattttcgctttcacgcccattttcgggaacttgtagatacgtttacggatatccataaagcgcagcgccagctcttcgaagtgagtttccggatgttcgtacataacccacatgatcttcgcggcgtccatcggggaaccaccacccagcgcgataatcacgtctggtttgaaggagtttgccagttctgcacctttacgaacgatgctcagggtcgggtccgcttctacttcgaagaagacttcagtttcaacgcctgctgctttcagtacggaagtgatctgatcagcataaccattgttgaacaggaagcggtcagtcacgatgagcgcacgtttgtggccatcagtaatcacttcatccagcgcgattggcagggagccacggcggaagtagatagatttcggaagtttgtgccacaacatgttttcagctcgcttagcaacggttttcttgttgatcaggtgtttcggaccaacgttttcagagatggagttaccaccccaagaaccacaacccagagtcagggaaggtgcgagtttgaagttatacaggtcaccgataccaccctgagacgctggggtgttaatcaggatacgcgccgttttcattttctgaccgaagtaagaaacgcgagccggttggttatcctggtcagtgtacaggcaagaggtatgaccgataccgcccatagcaaccagtttctctgctttttctaccgcgtcttcgaaatctttagcgcggtacattgccagagtcggggacagtttttcatgtgcgaacggttcgctttcatcaacaacggtcacttcaccgatcagaatcttggtgttttctggtacagagaagcctgccagttcagcaattttataggctggctgaccaacgatagccgcgttcagcgcaccgtttttcaggataacatcctgaacagctttcagctctttaccctgcaacagatagccgccgtgggttgcaaaacgttcacgtacagcgtcataaacagagtcaacaacaacaacagactgttcagaagcacagattacgccgttgtcgaaggttttggacatcagtacagatgcaactgcacgtttgatatcagcagtttcatcgataacaactggagtgttgcccgcgcctacaccgatagctggtttaccggagctgtatgcggctttaaccatgcccggaccaccagtcgcgaggatcaggttgatgtctgggtggtgcatcagtgcgttagacagttcaacagaaggttgatcgatccagccgatcagatctttcggagcaccggcagcgatagcagcctgcagaacgatatcagccgctttgttggtggcatcttttgcacgcgggtgcggggagaagataatggcgttacgggtcttcagactgatcagcgatttgaagatagcagttgaagtcgggttagtggtcggaacgataccgcaaataataccgattggttcagcgatagtgatggtaccaaaagtgtcgtcttcagacagaacaccacaggttttttcatctttataggcgttgtagatatattcagaagcaaagtggtttttgatcactttatcttcgacgatacccatgccggattcggcaacggccattttcgcgagtgggattcgagcatctgcagcagccagagcggcggcgcggaagattttgtctacttgctcttgagtgaaactggcatattcacgctgggctttttttacacgctctacgagtgcgttaagttcagcgacattagtaacagccataatgctctcctgataatgttaaacttttttagtaaatcatctgctcgaatacgagagtatagtcagtgcggtgatgatttgcttaacctatgaaaatcaaaagcttactcgcgctcacactcactgtgatttactaaaagagtttaaacattagagttattatctctaatgcgtcacttccaggtggcgtaagcaagattactcacttctgggtactgattacgtgatccaaatcaaatttttgcaaagctgacacctttcagcatcgcttttcgccattatagctaacagttaataaattgtagtatgatttggtggctacattagcatgttttgcacaactagataacaataacgaatgatagcaattttaagtagttaggaggtgaaaaatgctgtcaaaaggcgtattgtcagcgcgtcttttcaaccttatttatggctaacattatccggcttttgcttcggagctaaccgtgattcagaccttttttgattttcccgtttacttcaaatttttcatcgggttatttgcgctggtcaacccggtagggattattcccgtctttatcagcatgaccagttatcagacagcggcagcgcgaaacaaaactaaccttacagccaacctgtctgtggccattatcttgtggatctcgctttttctcggcgacacgattctacaactttttggtatatcaattgattcgttccgtatcgccgggggtatcctggtggtgacaatagcgatgtcgatgatcagcggcaagcttggcgaggataaacagaacaagcaagaaaaatcagaaaccgcggtacgtgaaagcattggtgtggtgccactggcgttgccgttgatggcggggccaggggcgatcagttctaccatcgtctggggtacgcgttatcacagcattagctatctgtttggtttctttgtggctattgcattgttcgctttatgttgttggggattgttccgcatggcaccgtggctggtacgggttttacgccagaccggcatcaacgtgattacgcgtattatggggctattgctgatggcattggggattgaatttatcgttactggtattaaggggattttccccggcctgcttaattaattcctttcaaatgaaacggagctgccatgctccgtttacttcgtcattatttttactttgttcccgcgcagttatcaaaagcaaaaggaataggtaaaaatattcttctcaaattacagttagttataaggatttccttaactgcttctcctcaccatcatgttattttcgccacatcataatcctgggcttgctgaagaataattgaaatgatattattaattccactgcctttggtagaggaaagtgctaaggaaggtgcgaacaagtccctgatatgagatcatgtttgtcatctggagccatagaacagggttcatcatgagtcatcaacttaccttcgccgacagtgaattcagcagtaagcgccgtcagaccagaaaagagattttcttgtcccgcatggagcagattctgccatggcaaaacatggtggaagtcatcgagccgttttaccccaaggctggtaatggccggcgaccttatccgctggaaaccatgctacgcattcactgcatgcagcattggtacaacctgagcgatggcgcgatggaagatgctctgtacgaaatcgcctccatgcgtctgtttgcccggttatccctggatagcgccttgccggaccgcaccaccatcatgaatttccgccacctgctggagcagcatcaactggcccgccaattgttcaagaccatcaatcgctggctggccgaagcaggcgtcatgatgactcaaggcaccttggtcgatgccaccatcattgaggcacccagctcgaccaagaacaaagagcagcaacgcgatccggagatgcatcagaccaagaaaggcaatcagtggcactttggcatgaaggcccacattggtgtcgatgccaagagtggcctgacccacagcctggtcaccaccgcggccaacgagcatgacctcaatcagctgggtaatctgctgcatggagaggagcaatttgtctcagccgatgccggctaccaaggggcgccacagcgcgaggagctggccgaggtggatgtggactggctgatcgccgagcgccccggcaaggtaagaaccttgaaacagcatccacgcaagaacaaaacggccatcaacatcgaatacatgaaagccagcatccgggccagggtggagcacccatttcgcatcatcaagcgacagttcggcttcgtgaaagccagatacaaggggttgctgaaaaacgataaccaactggcgatgttattcacgctggccaacctgtttcgggcggaccaaatgatacgtcagtgggagagatctcactaaaaactggggataacgccttaaatggcgaagaaacggtctaaataggctgattcaaggcatttacgggagaaaaaatcggctcaaacatgaagaaatgaaatgactgagtcagccgagaagaatttccccgcttattcgcaccttccctaaataataatcaattgttaaattattgtgcatttcactactggaactgtaatcagaaaagatagacatgcttagccaatctctatttgattgaattgaaagatgtttgttaaggcatggatgcaagctatagattctgatacggtcaataaaagagaattgcttaacaattttgcaaaatgtattggcgagtaagaaccgcatttggtactttccgggcaaccgccagacgattctttattggtaatgagaataattaacaattaaagagcgtcgcgaaagaataatgtgtctcgacaggggagacacagtacgaatcgacataaggtgatcgtctgaatcaccagaataaataaagtcggtgatagtaatacgtaacgataaagtaacctgacagcagaaagtctccgagcctgtgcagggtcccaatccgggattacacatgctggttaataccagtaattataatgagggagtccaaaaaacaatgaccaacatcaccaagagaagtttagtagcagctggcgttctggctgcgctaatggcagggaatgtcgcgctggcagctgatgtacccgcaggcgtcacactggcggaaaaacaaacactggtacgtaacaatggttcagaagttcagtcattagatccgcacaaaattgaaggtgttccggagtctaatatcagccgagacctgtttgaaggcttactggtcagcgatcttgacggtcatccagcacctggcgtcgctgaatcctgggataataaagacgcgaaagtctggaccttccatttgcgtaaagatgcgaaatggtctgatggcacgccagtcacagcacaagactttgtgtatagctggcaacgttctgttgatccgaacactgcttctccgtatgccagttatctgcaatatgggcatatcgccggtattgatgaaattcttgaagggaaaaaaccgattaccgatctcggcgtgaaagctattgatgatcacacattagaagtcaccttaagtgaacccgttccgtacttctataaattacttgttcacccatcaacttcaccggtgccaaaagccgctatcgagaaattcggcgaaaaatggacccagcctggtaatatcgtcaccaacggtgcctataccttaaaagattgggtcgtaaacgaacgaatcgttcttgaacgcagcccgacctactggaacaacgcgaaaaccgttattaaccaggtaacctatttgcctattgcttctgaagttaccgatgtcaaccgctaccgtagtggtgaaatcgacatgacgaataacagcatgccgatcgaattgttccagaagctgaaaaaagagatcccggacgaagttcacgttgatccatacctgtgcacttactattacgaaattaacaaccagaaaccgccattcaacgatgtgcgtgtgcgtaccgcactgaaactaggtatggaccgcgatatcattgttaataaagtgaaagcgcagggcaacatgcccgcctatggttacactccaccgtatactgatggcgcaaaattgactcagccagaatggtttggctggagccaggaaaaacgtaacgaagaagcgaaaaaactgctggctgaagcgggttataccgcagacaaaccgttgaccatcaacctgttgtataacacctccgatctgcataaaaagctggcgattgctgcctcttcattgtggaagaaaaacattggtgtaaacgtcaaactggttaaccaggagtggaaaacgttcctcgacacccgtcaccagggtacttttgatgtggcccgtgcaggctggtgtgctgactacaacgaaccaacttccttcctgaacaccatgctttcgaacagctcgatgaataccgcgcattataagagcccggcctttgacagcattatggcggaaacgctgaaagtgactgacgaggcgcagcgcacagctctgtacactaaagcagaacaacagctggataaggattcggccattgttcctgtttattactacgtgaatgcgcgtctggtgaaaccgtgggttggtggctataccggcaaagatccgctggataatacctatacccggaatatgtacattgtgaagcactaatggcaatacgtggggcaggagtgtcctgctccacggtgtctgatttttatcgcattacagaaggcacaggccagaaggtagggcaatgttaaaatttattctacgtcgctgtctggaagcgattccgacgctatttattcttattactatttcgttctttatgatgcgcctcgcgccgggaagcccttttaccggcgaacgtactttaccgccagaagtgatggccaatatcgaagcgaaatatcatcttaatgatccgatcatgacacagtatttcagctacctgaaacaactggcgcacggtgatttcggtccatcgtttaaatataaagattattcggtcaatgacttggttgcatccagttttcccgtttctgccaaactgggagccgcagcatttttccttgcggtaatactgggtgttagtgctggcgttattgccgcattaaaacaaaacaccaaatgggactataccgtgatggggctggcaatgaccggggttgttatccccagttttgtggttgcaccattattagtcatgatatttgcgatcattttgcattggctgccgggcggtggctggaatggtggggcgcttaaattcatgatattgccgatggtggcgttgtcactcgcttatatcgccagtattgcgcgtattacccgtggctctatgattgaagtattacactccaattttattcgtactgcccgggcgaaagggttacctatgcggcggatcattttacgtcacgcattaaaacctgctctgttacccgtgctctcttatatgggccccgcatttgtcggcattattaccggttctatggttatcgaaaccatttatggtttgccggggattggacaactgttcgttaatggcgcattgaaccgtgactattccttagtgttaagcctgaccatcctggttggtgctttaaccattttgtttaatgccattgtcgatgtgctatatgcggttatcgacccgaaaatccgttactgatactggagctcgcgatgatgttaagtaagaaaaacagcgagacgctggaaaatttcagtgaaaagctggaggtcgaagggcgcagcttgtggcaggacgcacgtcgacgttttatgcataaccgtgcggcggttgccagtctgatagtgctggtgctgatcgcgttatttgtaatcctggcaccgatgctttcccagtttgcctatgacgatactgactgggcgatgatgtccagcgccccggatatggagtccggtcactactttggtactgactcatccggtcgcgacctgcttgtgcgcgttgcgattggcgggcgtatctcactcatggtcggtgttgctgcggcactggtggctgtggtcgtcgggacactttatggttcgctttccggttatctgggcggtaaagtggattcggtaatgatgcgtctgctggaaatcctcaactccttcccattcatgttcttcgtcattttgctggtgacctttttcggtcaaaacatcctgctgattttcgtggcgataggcatggtttcctggctggatatggctcgtattgtgcgtgggcaaaccctgagtctgaagcgcaaagagtttattgaggcggcacaagttggcggtgtatcgacatcgggcattgttattcgccacattgtgccgaatgtactcggtgtggtggtggtctacgcatcacttctggtgcccagcatgatcctctttgaatctttccttagcttcctggggttgggtacgcaagagccgttaagcagctggggtgcattgctgagtgatggcgcgaactcgatggaagtctctccatggttattgttgttcccagcgggattcctcgtggtgacgctgttttgtttcaactttatcggcgatggcttgcgtgatgccctcgacccgaaagatcgttaaggagtgcagccatgagcgtaattgaaactgcaactgtgccgctcgcacaacaacaggctgacgcactgctgaacgtgaaagatttgcgtgtcacctttagtaccccggacggcgacgtcacggcggtcaatgatttgaatttttccctacgtgccggagaaacgctgggtattgtaggtgagtctggttcgggtaaatcgcaaactgcatttgcgttgatgggcctgttggctgccaacggacgtattggcggatcggcaaccttcaatgggcgtgaaatcctcaatttgccagagcatgaactcaataaactgcgcgctgaacaaatctcaatgatttttcaggacccaatgacttcgttgaatccctatatgcgcgtcggtgagcagttgatggaagtgctgatgctgcataagaacatgagcaaagctgaggcgtttgaagagtcggtgcggatgctcgatgcggtaaaaatgccggaagcgcgtaaacgcatgaaaatgtacccgcacgaattttctggcggcatgcgtcagcgagtcatgattgcgatggccttgttatgtcgacctaagctgctgattgcggatgaaccaacaactgcgctggacgtcaccgtacaggcgcagatcatgacgctattaaatgaactgaagcgggaatttaataccgccatcattatgatcacccacgatcttgtcgtggtggcggggatctgcgacaaagtgctggtaatgtacgccgggcgcacgatggaatatggcaacgcgcgcgatgtcttttatcaacccgttcatccttattctatcggtttgctcaacgcggtgccgcgtctcgatgcggaaggtgaaacaatgttgaccatcccgggtaatccgccaaacctgctgcgattaccgaaaggttgcccgttccagccacgttgtccgcatgcgatggaaatttgtagtagcgcaccgccgctggaagagtttacgcctggccgtctgcgtgcttgctttaaaccggtggaggaactgttatgaatgctgtaactgaaggaagaaaagtcctccttgaaatcgccgatcttaaagtgcactttgaaatcaaagatggcaaacagtggttctggcaaccgccgaaaacgctcaaagccgtcgatggtgtcactcttcgcctgtatgaaggggaaacattaggtgtggtaggggaatcgggatgcggtaagtccacctttgctcgcgccatcatcggtttggtcaaggcgaccgacggtcatgttgcctggttaggtaaagagttgctgggcatgaaacccgatgaatggcgtgccgttcgcagtgatattcagatgattttccaggatccgttggcatcgctaaacccgcgtatgaccatcggcgagatcatcgctgaaccactgcgtacttatcatccgaaaatgtcacgccaggaagttcgcgagcgcgtgaaggcgatgatgctgaaagtcgggttattgcctaacctgattaaccgctatccgcatgagttctctggtgggcagtgccagcgtatcgggattgcgcgtgctcttattcttgaaccgaagctgattatctgtgatgagccggtgtcggcgctggacgtgtcaattcaggcacaggtggtcaacctgctccagcaattgcaacgtgagatgggattgtcattaatttttatcgctcatgacctggccgtggtaaaacacatttccgatcgtgtgttggtgatgtatctcggccatgcggtagaactggggacctatgatgaggtctaccacaatccactacatccttacaccagggcattgatgtcggcagtccccatacctgatccggatctggagaagaacaaaaccatccagttactggaaggggaattaccgtcgccgatcaacccgccttccggttgtgttttccgtacccgttgcccgattgccggtccagagtgcgccaaaacacgtcctgttctggaggggagtttcagacactccgtttcttgcctgaaagtcgatccgctttaaaaacaataagggctgacagttgtcagccctttttcacgctaaaagcgattatttattcccgccagatgatatggcaaagtttgtgatctttttcgcggcataacagaatgcgggcaaaaacatcgttgatttcaccatcttcactgtccgccagaccaatcaccacttcggcaaaaaagtccgggttcaaatcgaaatcaacatgttcctgccagtcttccgccggatcgaataactccgcgccgccgcgctcttcaaactgaagattgaacagcagaacatcagctggatcgagattgtcggcagccagttcgagaaaaatatcgtaggcctgttcaagcgtttcatcttcagtcaggcgattgtttagatccatatccatagttactacctgtttaacctctgttggcgacgttttacagcaacggactgaagaagtaaaacagtcgctcggcgacacgttgccataatggacgttttagccataaacgggcatcgagcagacgtgaacgcgaaatataatcgtcctgaacggcggcgaggtcagcaccaaaacctttatcgtcgattgccagggtaatctcgaaatttagccacagactacgcatatcaaggttaactgtgccaaccagacttagttcgccatcgaccagcacgctcttggtatgcagtaacccgccttcaaactgataaattttaaccccagcagccagcagttccgtaaagaatgcgcgactggcccagccgaccagcatcgagtcattttttcgcggaaggataatactgacatccaccccgcgctgcgccgccgtgcaaatcgcatgaagtaaatcatcgcttggcacaaagtagggcgtggtcatgatcaaatattcacgcgccgaataagccgcagtcaataatgcctggtgaatgagatcttccggaaagccggggccagaagcaattgtgtgaatggtgtgaccgctggcctgttcaaacggcataatattgacatctggtggtggcggcagaatacgttttccggtttcaatctcccagtcgcaggaataaataatccccatcgcggtggcgatagggccttccatacgcgccatcagatcaatccattgccctacgcccgcatcttgtttgaagtagcgaggatcgaccatattcatgctgccggtgtacgcgatgtaattatcgatcatgatcatcttgcgatgttggcgcaggtccatacggcgtaaaaacacacgcatcagattgacctttaaggcttcgaccacttcaataccggcattacgcattagctcgggccacgggctgcggaaaaaagccacactcccggcggagtcgagcatcaatcggcaatgaatgccgcgtcgcgcagccgccattaatgattcagccacctggtccgccatgccgccgggctgccagatataaaacaccatctcaatattatggcgcgcgagctggatgtcgcggattaacgcctgcatcacatcatctgactcggtcatcagttgtagctgattccctttgaccccagcgatcccctgacgacgctcgcaaagcttgaataatggcgcagcgacactgctattttcttcggcgaagatatgcttacaggctttaaggtcgttaagccattttgcggtggaaggccacatcgctctggcgcgctcagcgcggcgtttgcctaaatggagctcgccaacggcaagataggcaataattccgactaacggcagaatgtaaataatcaacagccaggccatcgcggagggaactgcgcgtcgtttcattagaatgcgtaaagttacgcctgcaatgagcaaccagtatcccagaatggccaaccaactcaccaacgtataaacggttgtcatagattagaaatccttttgaaagcgcattgttatgagtttacgcatatggattcatctggcaaataaaaacgcgggaaaagcactggtcagcgtcgggggtgggggtataatgaccattctgttattgcatagagtagttaacatgaagcggagtagaacggaagtggggcgctggcgcatgcagcgtcaggctagccgacgtaaatcgcgttggcttgaggggcaatcgcgccgaaatatgcgtatccacagcatcaggaagtgcattctaaacaaacagcgtaactcgttattgtttgcgatctacaatatctaaatgtactgggcaccattgcggtgcccaataagtttactcttccgtctttaaactctatttttgcgccgattctttactgtcagctttcgtttctagttcatcgttatcgctgaaaataccatgacctgagttcaacaacattgaaacgagcatatcattattaatctcttcaccatttaaaactcgcgccagaatttcgctgccaaacagttgcggtgagagaatgatatccggatgtaccatcttaatcttattcaggtttttgctatcactgacggcgagaactgttttgacatcactgctcatatcttttgccgagagtacaacaaacgcgttatctgcatcgttatcactcagcgccagaatggcccggcaacgatcgattcccgctttctttaatacagaactgtcattactgtcaccggggataacatcagcattatcgcctaagcgttgctcaagttgcttgatatcatcttcaggcaagttgctgataaccgttacgttttgtccgcgttgattcagttgcaggatcgtattgatggcgagaatcgaatgtccgcaaacaataaaatgatctttacgatgcattgtatgattgtttccttttacaagtttgttgaatcccccgcggataagcggaccaaaaattgaggtcatagatgtggcaaaaacggtaatgccggaaataatgaccgaaatagtgaacaatcgtgctgattcagaaacagggacaatatcgccatagccgacggttgacatggtttctatcgaaaaatagaacgcggtcatcaaactttctattcgcggattaaaaccttcgcttaaataaagcgcaccgtaggttgagtaaaacagtaatgtcgtgaaactaataaatgcaaaaattgtcccggctgcggcgctactgtgggagaagtctttgcgcagtatcagcaaaaacaccagcgtaaaaatgcaaaatccaatactaaatttcagccagggataaaaatgcagggtgtaaattagcgctatcaacaacaaaatgatactgattgcccatgcgagctttgcccggaacagtaagccaatggagttcaggacaagaaagacgccgagcataaagagtggggcgtttgccagcaaggagagatccaactctgaaaatgctttgatatggaaaatatcaagcaaattgaccgacataccatagattgttttaaaaataagcaatccatttaaaaagacggccagcgcgagaatgtcgtgccgaagggtcacccataaatttgttgctgtttgtttgaatgtagcccagtgactcactgatacctctgtaaccacaattttgtttaattatcttagcgtgcacattttctgaacatacatgcagcgcgtgaatgtgttaaacaatagtagatgactttatccgcagtaatcaaaggatttgagcgagcaactgtacctcaggaaaggtcatttttcctgaatatgctcacatcatataaagaaatacagataaagttattatctgcttgtggtggtgaatgcactgaccggctataaggaaaggccaaacaagaacacggttgcaaaaaccgtgcccttaaatattgaatctctattcagaacactttcttaaatggtttcactgaaacgtgttcatagactcctgccgctacgtacgggtcagcatcggcccaggcctgagctgcttccagcgattcaaattcagcaataacggttgagccagtaaatcccgcagcccctggatcgttactgtctaccgctggcattggaccagctgtcaacaaacgaccttcatcatgcagtaactgtaaacgtgctaaatgtgccggacgaacggaaaggcgtttttcgaggctatcagctttgtcttgagcgtaaataacatacaacacgggcacaactccttgttcgggaaagttgtaaagtacgttatttgaaagggcgaagatctgcaacggaaagatgatgtctttgttaaggccatgcataaagtaagggtaattacgccaaaaatgacattttcactgatcctgatcgtcttgccttattgaatatgattgctatttgcatttaaaatcgagacctggtttttctactgaaatgattatgacttcaatgacccttgatttacctcgccgcttcccctggccgacgttactttcggtctgcattcatggtgctgttgtggcgggtctgctctatacctcggtacatcaggttattgaactacctgcgcctgcgcagccgatttctgtcacgatggttacgcctgctgatctcgaaccgccacaagccgttcagccgccaccggagccggtggtagagccagaaccggaacctgagccgatccccgaaccgccaaaagaagcaccggtggtcattgaaaagccgaagccgaaacctaagccaaaaccgaagccggtgaaaaaggtacaggagcagccaaaacgcgatgtcaaacccgtagagtcgcgtccggcatcaccgtttgaaaatacggcaccggcacgcctgacatcaagtacagcaacggctgcaaccagcaagccggttaccagtgtggcttcaggaccacgcgcattaagccgtaatcagccgcagtatccggcacgagcacaggcattgcgcattgaagggcaggttaaagttaaatttgacgttacgccggatggtcgcgtggataacgtacaaatcctctcagccaagcctgcgaacatgtttgagcgtgaggtgaaaaatgcgatgcgcagatggcgttatgagccgggtaagccaggcagtgggattgtggtgaatatcctgtttaaaattaacggcaccaccgaaattcagtaagcagaaagtcaaaagcctccgaccggaggcttttgactattactcaacaggtaaggcgcgaggttttccttcaggatcaaccgcgacatacttaaataatgcttctgtcgctttatagcgttgcccaattggttcagacgctacttttttcacccacacttcaatattaatgctgaccgatgtcgtccctttctggacacagcgtgcatagcagcacaccacatcgccgaccgcaaccggccgtaagaaagtcattccttcaacccgcacagtcactacgcgaccgtgggcaatttcttttgccagaatagcgccgccaatatccatttgtgacattaaccaaccaccaaagatgtcaccattggcattggtatcggcgggcatggctaaagtacgtaaaacaagatcgccctgagggacgttatgtgttgtagacatggtaaaaccgacttaaaaggaaaatcacaggcgcgatgctactatgattttcctgaggagaacagaggagatacagcgccagccccgaaggactggcagtctggttaggatttatcttcctgcggcatgtggcggtagatatagataccgcttaacaatgtgaagattaaggtaagggcggtcaggccaaagactttaaagttgacccaaatattttgcggcagccagaatgcgatgtagatgtttgccagaccgcaaaggataaagaaaacagcccaggccagattcagcttcgaccataccggttgcggcagcgtgagttctttacccagcatccgctgaattagcggctttttcatcacccattggctgactaacagggctcccgcaaatagagcataaatgacagtaaccttccatttaataaactcatcattgtggaagaacagcgtcaagccaccgaagacgaccaccagaacaaaagtgatcagggccatcttctcaaccttacgaaagcgaacccagctatagataagcacaatcgccgtggcgacgatcagcgccgcagtagccgcatagatgtcataaatcttgtaaaacgcgaaaaagacaaccagcggtaaaaaatcaagaaactgcttcattttacgattccgtaatcaaatgcttaaggttattggcgaatcaacatatacaggcggaacagatagatgagcaatatggctgaaatcaggttgctcaaggtgttcgccagtacggcaccaatttccggggttaatgcggcaaaagaagaggcaaaaagcagcaacagtgtttttgccagcaaccagctcagtactgcgggtgccaccagacgcatattcgcccaagtcagccgcatactgctacgcatcgaggcaaaaacgcccattttgtcctgtaccaacatcaccggtgccagggccagtaaaatggccatgataattcccggaacgaccaccagcatgatgccaatctgtactaaaagggtagtcagaaaaatcagaataaataactttggcaatatcggcgcactggcaccaatagctcgcagcgcactgactctctgacccgcagacaccagctggataattaatattacgcctccggcgagaatggcgttaccgattaatcctgaaaaagtggacgccgctgaagcctgcagcaaaatttgttgctgttccggtgacatattctgaaccaggtcgaacaacccactactgccgctaacgggcacgccgtcattgagctgcgcaagctgtgcatcactgggtgagaaaacatgccctaacaccactgtgataaacgcacatagcaacgataccaacagaatggtcataaattgattacggaagaaatttccggtgtcacggtatacggactgcgccgtgatagacatgcactctccttgagttttatgcaggtgttaattagcgggcaattgtaccctggttaagcctcgggtggcagcatcaggtcttgtatggaaaagcatatctttgtaaagcggaggtaattgctggccttcaggcatgggcaaatcgcggcaagtggcgaccgagttaatatttgcgtagcgaaaatatttaaaaattgatttaaatcacattaaccaggattctcaatgcaacttctaaattaatccagatcaataaagggtgaattatcatatgtaatgtgatctatgtaggatcatttgttactccaatgtaggtatattcgtcacgtttttataaccataacgacggagcggatatgaaaaagttaacagtggcggctttggcagtaacaactcttctctctggcagtgcctttgcgcatgaagcaggcgaattttttatgcgtgcaggttctgcaaccgtacgtccaacagaaggtgctggtggtacgttaggaagtctgggtggattcagcgtgaccaataacacgcaactgggccttacgtttacttatatggcgaccgacaacattggtgtggaattactggcagcgacgccgttccgccataaaatcggcacccgggcgaccggcgatattgcaaccgttcatcatctgccaccaacactgatggcgcagtggtattttggtgatgccagcagcaaattccgtccttacgttggggcaggtattaactacaccaccttctttgataatggatttaacgatcatggcaaagaggcagggctttccgatctcagtctgaaagattcctggggagctgccgggcaggtgggggttgattatctgattaaccgtgactggttggttaacatgtcagtgtggtacatggatatcgataccaccgccaattataagctgggcggtgcacagcaacacgatagcgtacgcctcgatccgtgggtgtttatgttctcagcaggatatcgtttttaattccgcacaaaaacgaccccgtaatatacggggtcaataaggacatggtataaagggtattatttcttcgcttctacgccatcagtttcagagcgaattaaaaatttctcagttgtttgcggaatattctgaatcagccagtcggccatttgcttttcctcatttaaaatcgcttcgatggttggaattgaagctgtatcaccggcattttttgctgctgctaatagtgaggtgtaacaggcgatttcaaattgctcgaagacatatccgctaatagagcctttgactatttcatcagaagggaatataccaccgattgactgcccaagcgcagccattttactcatggaatctttaatgactgaacgtgaaatgtcattacgatcaagaatagtttccagttgaacaatctggtttttggtttcactaagatgttgttcaatacgagcgcgtagttcaggataattatctatacggctggccatggattcaagcatagattcggcttgcttttccattgcgtgggcgtcacgtaaccagtcatgataatgttcaatacgattcatgaaaatgtcctctttataaaatgactaaaagttaaaattcatatttcaggctttattttcggctttcttatttacgttattaatggccagatcagtcagtttgatgtcggtggccttttcttcttccagggtttctttcagaagcttcgctgctttacggtaacctaattgttcagccagcgtcgctaatgtcccgtaactggcaatctcataatgctcgactttctgtgctgcggcaatcagtgcggcatcacgcacttcgtttttctcggtactttcgatgacctcattagcttcttcaataagaccttccattgccacacatttcatgcgcttaattttcaggttcgattcggactccacaacttgatcaatacgttcaatctgtccatgagtttcctcgaggtgcgcatgaaaagcctgacttaatttttcatttgatgttgctcttgcgagttttgccagtgcccgggttaattgtttttctgcgctgtaggtatctgaaagcaggtgaataaatacatcttcaatggtcttcatattcatatttttctccagtgaaatcactgcgagccatacggcccgcagatgcaattatctttatcagctgatattaataattaacggtgaatcaggatttgcctgatttattaccaccgctttgttgaccgccttttttacccgcttcagatgcgcgttgcggatcatttttaaaattaccgccgctatgctgaccgcctttacggcctgcgtcggatgccttctcacggtcttcggcgaaatttcctgaaccaccacgatgttcggccatgttatttctcccgttgcgttgcattgtttcattaatatgagtgttgtgtgtcgacactcattaaaattagtcgctaatgagaattagtcaaattaagcgcaacgagaagatagagggaaaatatattttgaggaacattctggatatattaacaattacctgaggaataagtgacttagagaaaattattgattttactggtgttatgttgcgggattaatttgtttgattatattactgttgggcggaaaaatgacgtaagttgacgttcgaccggggtaagcgaaacggtaaaaagataaatattaaatgaatttaggatttttccggcttcattaaagaaagttaaaatgccgccagcggaactggcggctgtgggattaactgcgcgtcgccgctttcatcggttgtacaaaaactttcagtgccgccagcattttctctggctcattaatatgttgctcgatgattttaacaatggccgaaccagaaatcgcgcccgcagctcctgcatcaatcgctgcttttacctgatccggggcggaaataccaaatccctgcaatggaggtgcagcgttgtactctttcagcttcgcaaccagatgattgaggggtaacgcggcgcggttttctgcgccggtcacgcctgctcgtgacagcaaataggtgtaaccacgaccgtaagaggctatctggcgcagcaggtcgtcatcggcatttggcgggcagatgaagataggtgcgacattatgacgcaacgcggcctggcggaagggcgcggactcttcaactggcacatcggcaaccagcaccgaatcgacgccgactttttcgcactgggcataaaactcatcaatgcctttgttaaacaccagattggcatacatcaacaggccaatgggaatggtcgggtgtttctggcgaatcagtgccagcatttcaaaacattgtgccggagtcacacctgccgcaaaggcgcgcagagtggcgttttgaatcgtcgggccatccgccagtgggtcggagaaggggatacctaactccagcgcgtcagcaccggcttcaattagcgtatcgataattttcaatgactgctcaatgcccggatcaccgagcgtgacgaaaggaacgaatgcgccttctttgcgctccttcaactgggcaaacagagattcgtagcgttccatcagatttcccctcgtgctttcaaaatatcgtgaacggtgaagatgtctttatcgccgcgaccggaaaggttaaccaccagtagctgctctttatccgggttttcgcgcatcattttcaacgcatgggccagggcgtgggaggattccagcgccgggatgatcccttcgtgcaggcacagcgttttgaaggcttcaagggcttcatcatcggtaatagacacgtaatcagcgcgtccagtgctgttaagatacgcgtgttgtgggccgacagacgggaaatccagtccggcggagatggagtaagattcttcaatctgcccgtcttcggtttgcatcatcggcgctttcataccgaaatagatacccacgcgaccatgttttagcggtgcgccgtgctcgccagtttcgataccgtgaccacctggctccacaccaatcaggccgacgttggtttcattgatgaaatcagcaaacatgccgatggcattcgaaccgccgccaacacaggcgataacggcatccggcaggcgaccttctctttccagaatctgcgctttggtttcttcgccaatcatccgctgaaactcacgcacaatggtcggataaggatgcgggccagctgcggtgcccagcatatagtgcgcggtttcgtaactaccggaccagtcgcgcagcgcctcgttacaggcatctttcagcgtcgcggaaccgctatgcaccgggatcacttccgcacccattaagcgcatacgaaaaacgttaggcgactggcgttcaacgtctttggcacccatataaatacggcatttcaggccgagcagggcgctggcaagggccgacgccacgccatgctgaccggcaccggtttcggcgatgatttcggttttacccatccgcttcgccagcaacgcctgccccagcacctggttagttttatgcgcgccgccgtgcagcaaatcttcacgcttgagatacagcgtggtgttcgtcccggctgtaatgttctggcatttggtcagcgcggttggacgcccggcatagtttttcagcaggtcgttgaactgagcctgaaattcaggatctttttgcgcactgacaaaagcttcttccagctggcgcagagcaggcatcaggatttgtggcacgtacatgccgccaaactcaccaaaataggggttaagtaatgttgtcattgttcctttccttaatatgcgcgcagcgtctggaaaaccgaggccaaaagacgtgcgtctttgatgcccggttgcgactctacagcagaattaaaatcaagtccggcgcagccggtttgtgccgcttccacgcagttatctgcgcctaagccccccgccagcagaacgttgccaagcgattgaccatttaatagtgaccagtcaaaacgttgcccgcttccaccctggccgttgtctaaaacatatttatcaacgtgctgaaactcgcgggcgggcagggtttcaccgacgcttaatgctttccagatggcaacatgtgctggcagagcttcacgcagcgtatcgatatacagctgttcttcattaccatgcagttgcactgccgccagcgataacaccttagctttgtccaccacatcggcaatatcgtgattgcggaacacgccaacatactgcaacggtgccgcagccatcacttcctgcgcctgttcaacgttgacgcaacgcggtgatgtcgcaacaaaaatcaacccaccgtaaatcgcgcccgcgtcataagctgctttagcatcttgcccacgcgtcaggccacatactttattctcacccagcaacacccggcgcacggcggcgtgcaaatcgtcatgggccatcaacgccgaaccaatcagaaaaccgttagcgaagtggcttaactcgcgcacctgagcgtaagtattgatgccggattcgctgattaccgtcacgttgtgccccagtttcggcgcaagctcgcgggtacggttgagatcaatcgacaaatcacgcagatcgcggttgttgatgccaacgacctttgctcccaatgcaatggcgcgctcctgttcctcttcattactgacttcggtcagcacccccatctccagactgtgagcgacggcggcaagctggcgatattggtcgtcatccagtactgaaagcattaataagcaggcatcggcctggtaatagcgcgccagatagatctggtaagggtcgataatgaagtctttacataaaatcggctgcggggcgatttggctgacgatggggaggaaattaaagctcccctgaaaatatttctcatcagtcagcaccgaaattgccgaagcgtaatgtttataaatggcggcaatgcgtgctggatcgaaatcatcacggatcacgccttttgacggcgacgctttcttgcactccagaataaacgccgtgcgcgcaccctgtagcgcatcataaaaatgtcgcgtgctcggctgaacctcattctgaaaactggccagcggttgctgctgtttgcgggcttctacccaaatcgccttgtctgcgacgattttcgctaaaacggtttgcatcatttaccctcgtgccgccagtgcggtgactctgtcgtaagcggaaccactgcgcagtacctcaagaacggtttgcgcattggcttgcagatcttcatggccatgcaggcgcattaacatggcgacgttcgcagcgacggctgcttcatgggcggcgtcgcctttaccttgtaacaaacgtgttaaaatgtcacggttttcttccggtgttccgcctgccagttgctcctggtggtagggtgtcaggccaaagtcttctgcggtgagctgatagcttttaatttcgccgtcatgcagttcggcaacgattgtcggcgcgtgtaatgaaacttcatccatcccgccgctgtgcaccaccgccgcgcgttgataccccagcacgcgcaaggtttcggcaatcggcagcaccagttccggactataaacaccaattaacgccagcggcggatgcgccgggttaatcaatggccccagcacattgaacagggtgcgggttttcagttgctggcgaaccggcatcgcgtggcggaatccggtgtgatacttcggcgcaaagaggaaacatacacctaactcatccagcgcctggcgcgatttatcggcgttcatatcaagattaataccgaacgccgccagcagatcggacgaaccagatttactggagacgctacggttgccgtgtttcgccactttcagcccacaggccgcggcgacaaacgcactggcggtagaaatattgatactgttgctgccgtcaccgccagtaccgacgatatcagcaaacagataatccgggcgcgggaacggcgctgcgttttccagtagcgcggttgctgccccggcgatctcgttcgggtgctcaccgcgaattttcatgctcaccagcgccgccgccagttgttccggcttcagctcgccacgcaccaccgctgaaaacagctggtggctttcttgttggctaagcgtctgcgcctgatacagtttttccagaatcggttgcagcgtgttggctggctctagtttctgctgcgcccaggccagcgtttgttccagcaggcgagcgccctgggtggtgagaatggattccggatggaactggaatccacaaacgcgatccgcatcgtgacgtactgccatcaccatgccattaaaatgggcgttgatggttaaaccggccggaatgttactgccaaccagcgagtgataacgcgccaccggcagcgggtttgttaatccggcaaacatcgcctgaccgtcatgttcaatgctggaggctttaccgtggagaatttcgcccgcctgaccgacatagcccccgtaagcttcgacaatcgcctgatgtccgaggcaaatgccaataatgggcagcttgccacgcaagcgggtgaggagttccggcatacaaccggcttcgctcggcacaccggggccaggagaaagcatcagcaccggattgctcatggtcgccaggcgttcaattaaggtttgcgccggaatatggttgcggtaaatcaccacgttatgcccattgctgcgcaactgatctgccaggttgtacgtaaaagagtcgatattatcgagcagcagaatgtcagccatcagaaagtctcctgtgcatgatgcgcggtggcaatagcgcgcagtacagcgcgggctttgttacgggtttcgtcggcttccgactgcggaacagaatcaaggactacaccagcacccgcttgcacggtggcgataccgttttccaccagcgccgagcggatcacaatgcaggtgtcgagatcgccatgcgcggtgaaataacctaccgcgccgccgtagctgccgcggcgacgaccttccgcctcggcaattaactgcatagcgcgtactttcggcgcaccgcttaacgtccccatattcatacaggcgcgataagcgtgcagggcgtcaagatcgtgacgcagttcgccgactacgcgagagacgaggtgcatcacataggaataacggtcaactttggtgagatcggcgacgtagcggctgccgggggtgcaaatgcgtgccagatcattacgggcgagatcaaccagcatcagatgttcagacagctctttatgatcggtacgcatttccagttcaatacggctgtcgagatctctgtccagtgaaccatcggcgcgacgaccgcgtgggcgtgttccggcaatcgggtagatctcaatctggcggctggtggcatcatacttgagcgagctttccggcgacgcgccaaatagggtgaaatcattatcctgcataaaaaacatgtacgggctgggattactctttttcagcacgtaataggccgccagcggtgacgggcagggcagagagaaacggcgagatggcaccacctggaaaatttctccagcgcgaatcgctttttgcaacaaacgcactacgccaccgaactcttcatcgctctgattacattcacaacgcatatgcggcacggaaaccactggcagcggcggcgcggcttcggtcagttgctgacgtagttcgttcaggcgagcagtgagacgttgtttttcttcttcattcggagcaaacaggctggcctgaatacgggtgctttttttctgatggtcaatcaccatcagcgtttcagcgagataaaaacagaaatcagggcagttattttccgctgacagttgcggtaaatcttcaaatcccgccacaaggtcataagagaacaggccgccgaagaacatggcttctcgttcttccttcggtacattcaacagattctgcaataaacggaaagcgtcaaaaaccgaaagggagcataagcgggcgtcttcatccagcagtggactgacaggggggaagcgcagcacacggcagtttggtgattgttcactttccacacccgcaggcagggcgttatccagtagtgccaggagggcttcgccgttgccggaaagtgcctggattgtgacagtgtcacctaaagctgtaatgcgcagcgcactgtctaccagcagcaggctttttaaatcatctttgctgtcgatatctgcggattccagcagcagcgttgccggacgatccccacacaactggtgaaaaagcgcggtgggattgtcgcgataagcgccttcgcaggttagcagttcgagagtcggtttttgtgtttgcattgttattctctaattttgttcaaaaaaaagcccgctcattaggcgggctgggtatctgattgctttacgcatggtgaatacactgcccgtttcaggaagtgcgccaccaacctttcagtacgaaaattgctttcattgtcgataccctttttacgtgaacttgcgtactagttaactagttcgatgattaattgtcaacagctcatttcagaatatttgccagaaccgttatgatgtcggcgcaaaaaacattatccagaacgggagtgcgccttgagcgacacgaattatgcagtgatttacgacctgcacagccataccacagcttccgatggctgcctgacgccagaagcattggtgcaccgtgcagtcgagatgcgcgtcggcaccctggcgatcaccgaccatgacaccacagctgcaatcgcgccagcaagagaggaaatttcacgttcgggactggcgttgaatcttattcccggcgtggaaatttccacggtctgggaaaatcatgaaattcatattgtcgggctgaatattgatattactcatccgctaatgtgtgagttcctcgcgcagcagacagaacggcgcaatcagcgggcgcagctgattgccgaaagacttgaaaaagcgcaaatacctggggcgctggaaggcgcacaacgactggcgcagggcggcgcagtgacgcgcggtcattttgcgcgtttccttgttgagtgcggcaaagccagttcaatggcggatgtctttaaaaagtatctggcgcgcgggaaaaccggatacgttccgccacagtggtgtacaatagaacaagctattgatgtcattcatcattctggcggtaaggcggtgctagctcatcctgggcggtacaatcttagtgctaaatggctgaaaagattggttgcgcattttgccgaacaccacggtgacgcgatggaagtcgcgcagtgccagcaatcgcccaatgaacgtacccagctggcggcccttgcgcgtcagcatcatttatgggcatcacaaggatctgattttcatcagccatgcccgtggatcgaactgggtcgtaaactctggctgcccgcaggcgttgaaggcgtctggcagctatgggaacagccgcagaacaccacagagagggaattatgagccagtttttttatattcatcctgataacccacagcaacgtctgatcaaccaggcggtggagatcgtgcgtaaaggcggggtgattgtttatccaactgattccggctatgcgctcggctgtaaaattgaagataaaaacgcgatggagcgtatttgtcgtattcgccagctgccggacggtcacaactttaccctgatgtgtcgcgatctttctgaactctcgacctattcatttgttgataacgttgcgtttcgtttaatgaaaaacaacacgccgggcaactataccttcatcctgaaggggacgaaggaagtgccacgccgtctgttgcaggaaaaacgcaaaaccatcggtatgcgtgtgccttctaaccctatcgctcaggcgttacttgaagcattgggcgaaccgatgctttccacttcgctaatgctgccaggcagcgaatttaccgaatcggacccggaagaaattaaagatcgtctggaaaaacaggtagatttgattattcacggcggctatctcgggcagaaaccgacaacggttattgatcttaccgatgatacgccggtcgtggtgcgtgaaggcgtaggtgatgtgaagcctttcttataacaaattgcgttccacggatggaagactatggcagggaagtttcgctgcattttgctgttgatagcagggctgtttgtatcatctctaagttatgcagaaaacacggagatcccttcttatgaagaagggatctcgctctttgatgttgaagccactctgcaaccagatggggtgctcgacatcaaagaaaatattcattttcaggcgcgaaatcagcagattaagcacggcttttatcgtgatttaccacgactatggatgcagcctgatggggacgctgcactgctgaactatcatattgttggcgtcacccgtgatggtattcctgaaccctggcatcttgactggcatatcgggttaatgagtattgtcgtgggcgataaacaacgtttcttgcctcaaggcgactatcattatcaaattcattatcaggttaaaaatgctttcctgcgtgagggggattctgatctgctaatctggaacgtgaccggtaaccactggccgtttgaaatttataagacccgtttttctctccagttctctaatattgcgggtaatccatttagcgaaatcgatctttttaccggagaagagggcgacacatatcgtaatggccgcatccttgaggacggaagaattgaatcccgcgatccgttttatcgtgaagatttcacggtcctctaccgctggcctcacgctttacttagcaatgcctcggctccgcaaacgacgaatattttcagccatcttcttttaccctccacgtcatcgttgttaatttggtttccgtgtctgttcctggtttgtggatggttatatctctggaagcgcaggccgcaatttacgccggtagatgtgattgaaaccgatgtcattccgccagattacacgcccggcatgttacgtctcgatgcgaagctagtttacgacgataaaggtttttgtgccgatatcgtaaatctgattgtgaaaggaaaaattcatctggaagatcagtctgacaagaaccagcaaatcctgattcgtgttaatgaaggcgcgaccagaaataatgcggtattactgcccgcagagcagttattactggaagcgttatttcgtaaaggcgataaggtcgttcttacggggagacgcaacagagtcttacgcagggcatttttacggatgcagaaattttatctgccgcgtaaaaagtcttcgttttaccggtctgatacttttttgcaatggggtggactggcaatattggcggtcattctttacggtaacttgagtcctgtaggctgggcaggaatgagtctggtgggcgatatgtttattatgatctgctggattattccttttttattttgttcccttgagcttttgtttgcccgcgatgatgacaagccttgcgttaatcgtgtaatcatcactttgtttttaccactgatttgttcaggcgtggccttctattctctctacatcaatgtcggagatgtattcttttactggtatatgccagcgggttattttaccgctgtttgcctgaccggttatctcactggcatggggtatatttttctgccaaagtttacccaaactggacagcaacgttatgcccacggtgaagctatcgttaactatcttgcgcgtaaagaggcagcaacacacagtggacgtcggcggaaaggggaaacacggaaactggattacgcgttgctaggttgggctatatcggcaaatttggggagggaatgggcgttacgcattgccccttcgctttcttcggcgattcgcgctccagagattgcccgtaacggcgttttattctcattacagacgcacctaagttgcggggccaataccagtttgttggggcgaagttattccggtggtggtgctggcggcggcgcgggtggcggaggcggtggtggctggtaattaagctgatgttaatcgaaacaagctttaaccataaagatagtgtagtatgttgcgcctcaaagccaggccgataaacgtcgagtcgtttacttaaggcctgaagagttcaaacagactttactatcagtgagtcagatgtaagttctgactcactgttgcacaaaagcatatcagacgcctgggaaggcgacaccaaaaggaagctctatgagcgaaaagctacagaaagtgctggcgcgtgccggccacggttctcgccgtgaaatcgaatctattattgaagccggtcgtgtgagtgttgatggcaaaattgctaaactcggcgatcgtgttgaagttacccctggattgaaaatccgtatcgatggtcacctgatttcggtacgtgagtccgctgaacaaatttgtcgcgttctggcctattacaaaccggaaggtgagttgtgtacccgtaacgatccggaaggacgtccaacggtgtttgaccgtctgccaaaactgcgtggcgcacgctggattgccgtgggtcgcttggacgttaatacctgtggtctgctgctgttcaccaccgatggtgaactggcaaaccgtttaatgcacccaagccgtgaagttgaacgtgaatatgccgtgcgtgtatttggtcaggttgacgacgcgaaactgcgtgatttgagtcgtggcgtgcagttggaagatggtccggcagcttttaaaaccatcaagttcagcggcggcgaagggatcaaccagtggtacaacgtgactctgaccgaaggccgtaaccgtgaagttcgtcgtctgtgggaagcggttggtgtgcaggtgagccgcctgatccgtgttcgttacggtgatatcccactgccaaaaggtctgccacgcggtggctggacggagctggacctcgcccagactaactatctgcgcgaactggtggagctaccgccagaaaccagctctaaagtcgctgtagaaaaagaccgtcgtcgcatgaaggcgaatcagattcgtcgtgcggtgaaacgtcacagtcaggtgagcggcggtcgtcgttctggcggacgtaataataacggttaatcaaagtatgccggacgtcatatccggcatttttacagattaataatcgatccctatctgcgcttttacaccggcatcaaacgcatgtttgacggggcgtaattcacttaccgtatctgccagttcaagaatatcccgatgacaaccacgacccgtgataatcaccgtctgttgatgtggacgttcatttaacgcctgcaccacttcttccagtggcaaatagtcatacgccaccatatacgtcagttcatcaagcaaaaccatatccagtgaggaatcagcaagcatccgctttgcatgttgccagacttcgcggcaggcggcggtatcagactcgcggttttgtgtatcccaggtaaagcccgttgccatcacctgaaactcaacgccatgtggctccagcagattgcgttcgccattaggccaggtgcctttaataaactgcacgacgcctactttttttccgtgaccaactgcgcgtgttgccgtaccaaatgccgcggtggttttgccttttccattgccggtaaagacgatgataataccgcgttcatcctgggcctgggccacacgagcatctactttttctttcactcgctgctgacgctgttggtagcgttcatcactcattgggaaattcctggtttacggcccggttgggcgtcaaaggtcatgccggttttacggcggctgtcatcgcccatcagccagaggtagagcggcatgatatcagcgggtgttttaagtttctgtggatcttcggtcgggaaggcgctggcacgcattgcggtgcgcgtaccgcctgggttaatgcagttgacacgcaggcgctgctgatattcatcggccagtacctgcatcatcccttcggtggcaaatttcgacgctgcatatgcaccccagttggctcgtccctgacgtccaacgcttgatgaagtaaagaccagtgaaccggcgtccgatttgagtaataaaggaagcagtgcctgggtgagcataaaggtggcattaacgttgacctgcatgacgtcctgccagacctgcggattttgttcgctcattgggcaaacatcgccgagcaatccggcattatgcaaaacaccatccagacgcggataattaacggcaatgcgctgtgccagttgttggcaattttcggacgtgcaggtcagcaaatcgagaataaaccactgtggctgacgcccagtttcttcgtttatgtggctggctacctgacgtaatttttcttcattacggcccaacagaatcactgtcgcaccatagcgtgcatacgtcatcgcggcttcacgaccaataccatcgctggctcccgtcaccaggataatgcgatcattgagtaaatcttgttttggctggtaatgcatggctactcctcaacgacgttgtctgtcgcgctgccagtgtactttatgactttggggctttatgcctgaaacagaagggcatttcaatcagcctggggcgataacaccgcaaaatggatactttgtcatactttcgctgcaataacatctctgcgagacggcttaacatgcctgttgtaaactgtgagccaaagcgttgtttaaccaaggtggggactcgtggaattgttgtctgaatatggtttgtttttggcgaaaatcgttaccgttgtgctagcgattgcggcgattgccgccattattgtcaatgttgctcaacgtaataaacgccagcgtggcgagttacgggtcaacaatctcagcgaacagtataaggagatgaaagaagaactggccgcggcgctgatggactcacatcagcaaaaacagtggcacaaagcgcagaagaaaaagcataagcaagaagcgaaagcagcaaaagcgaaagccaaactgggcgaggtggcaactgacagtaaaccccgcgtctgggtgctggattttaaaggcagcatggacgcccatgaagtgaactcgctacgtgaagagataacggctgtactcgcagcattcaaaccgcaggatcaggttgtgctccgtctggaaagccctggtggcatggtgcatggttacgggctggcggcttcgcaactgcagcgtctgcgcgataaaaacattcctttaactgttacggtagacaaagtcgctgccagcggcggttacatgatggcctgtgtggcggacaaaattgtttccgcaccgtttgctattgtgggttccattggcgtggtggcgcaaatgcccaactttaaccgcttcctgaaaagcaaagatattgatatcgaactgcacactgccgggcagtataagcgcacgctgacgttgctgggtgaaaataccgaagaagggcgggagaaattccgcgaagagttgaacgaaacgcatcagttgtttaaagattttgtgaagcgtatgcgtccttctctggatattgaacaggtggcaacgggtgaacactggtacggacaacaggcggtagagaaaggcctggttgatgaaatcaacaccagtgatgaagttattcttagcctgatggaaggccgtgaagtggtcaatgtacgctatatgcagcgtaaacgactcattgaccgattcaccggcagcgcggcagagagcgccgatcgattgttgctacgctggtggcagcggggtcaaaagccattgatgtaaaagacaaacgcgaggctaagacctcgcgttttgctttaatcaaccagatgatatttttctgaaagcacatgggccaggtgtttgaacatattaaacaccgcggtgcttttggctgttggcaatccttgttcatctaaaaagtagtcgccggtaaataccagcacgccattacgctgcgtgacgccggtggcttcaatccctgcgagcgtatcctcatgctcacgaatgattttgttggcctctttcaacagcgtttcgcggtcgatgggttgtgtctctttgttcattatttactccttaaacaaggacattagtctacgccaggcatggcttgcagacaaatataccacgctggtggcaagagcgccttactggcaactttggattttgcatgctaataaagttgcgtatcggattttatcaggtacagtgtgacgctttcgtcaatctggcaatagatttgcttgacattcgaccaaaattccgtcgtgctatagcgcctgtaggccaagacctgttaactcagtcacctgaattttcgtgaacagagtcacgacaaggggttgatatccgcagagagcgagtccatatcggtaactcgttgccagtggaaggtttatcaacgtgcgacgcattcctggaagaatcaaattaggtaaggtgaatatgggtaaagctcttgtcatcgttgagtccccggcaaaagccaaaacgatcaacaagtatctgggtagtgactacgtggtgaaatccagcgtcggtcacatccgcgatttgccgaccagtggctcagctgccaaaaagagtgccgactctacctccaccaagacggctaaaaagcctaaaaaggatgaacgtggcgctctcgtcaaccgtatgggggttgacccgtggcacaattgggaggcgcactatgaagtgttgcctggtaaagagaaggtcgtctctgaactgaaacaactggctgaaaaagccgaccacatctatctcgcaaccgaccttgaccgcgaaggggaagccattgcatggcacctgcgggaagtgattgggggtgatgatgcgcgctatagccgagtggtgtttaacgaaattactaaaaacgcgatccgccaggcatttaacaaaccgggtgagctgaatattgatcgtgttaatgcccagcaggcgcgtcgctttatggaccgcgtggtggggtatatggtttcgccgctgctatggaaaaagatcgctcgtggcctgtctgccggtcgtgtgcagtcggtggcggttcgcctggtggtcgagcgtgagcgtgaaattaaagcgttcgtgccggaagagttctgggaagtcgatgccagcacgaccacgccatctggtgaagcgttggcgttacaggtgactcatcagaacgacaaaccgttccgtccggtcaacaaagaacaaactcaggctgcggtaagtctgctggaaaaagcgcgctacagcgtgctggaacgtgaagacaaaccgacaaccagtaaacctggcgctccttttattacctctacgctgcaacaagctgccagcacccgtcttggatttggcgtgaaaaaaaccatgatgatggcgcagcgtttgtatgaagcaggctatatcacttacatgcgtaccgactccactaacctgagtcaggacgcggtaaatatggttcgcggttatatcagcgataattttggtaagaaatatctgccggaaagtccgaatcagtacgccagcaaagaaaactcacaggaagcgcacgaagcgattcgtccttctgacgtcaatgtgatggcggaatcgctgaaggatatggaagcagatgcgcagaaactgtaccagttaatctggcgtcagttcgttgcctgccagatgaccccagcgaaatatgactccacgacgctgaccgttggtgcgggcgatttccgcctgaaagcacgcggtcgtattttgcgttttgatggctggacaaaagtgatgcctgcgttgcgtaaaggcgatgaagatcgcatcttaccagcagttaataaaggcgatgctctgacgctcgttgaacttacaccagcccagcactttaccaagccgccagcccgtttcagtgaagcatcgctggttaaagagctggaaaaacgcggtatcggtcgtccgtctacctatgcgtcgatcatttcgaccattcaggatcgtggctacgtgcgagtagaaaatcgtcgtttctatgcggaaaaaatgggcgaaatcgtcaccgatcgccttgaagaaaatttccgcgagttaatgaactacgactttaccgcgcagatggaaaacagcctcgaccaggtggcaaatcacgaagcagagtggaaagctgtactggatcacttcttctcggatttcacccagcagttagataaagctgaaaaagatccggaagagggtggtatgcgcccgaaccagatggttctgaccagcattgactgcccgacttgtggtcgcaaaatggggattcgcacagcgagcaccggggtattccttggctgttctggctatgcgctgccgccgaaagagcgttgcaaaaccaccattaacctggtgccggaaaacgaagtgctgaacgtgctggaaggcgaagatgctgaaaccaacgcgctgcgcgcaaaacgtcgttgcccgaaatgcggcacggcgatggacagctatctcatcgatccgaaacgtaagttgcatgtctgtggtaataacccaacctgcgacggttacgagatcgaagagggcgaattccgcattaaaggttatgacggcccgatcgttgagtgtgaaaaatgtggctctgaaatgcacctgaaaatggggcgtttcggtaaatacatggcctgcaccaacgaagagtgtaaaaacacacgtaagattttacgtaacggcgaagtggcaccaccgaaagaagatccggtgccattacctgagctgccgtgcgaaaaatcagatgcttatttcgtgctgcgtgacggtgctgccggtgtgttcctggctgccaacactttcccgaaatcgcgtgaaacgcgtgcgccactggtggaagagctttatcgcttccgcgaccgtctgccggaaaaactgcgttatctggccgatgcgccacagcaggatccggaaggtaataagaccatggttcgctttagccgtaaaaccaaacagcaatatgtctcttcggaaaaagacggaaaggcgactggctggtcagcattttatgttgatggcaaatgggttgaaggaaaaaaataacctttaattctgtcaggtttttataaacaaagggtcgcgaaagcggcccttttttattgcatattattttttcttcacacctatacactaaggctataaatgatatagtggttatagttagcaccttttttattattaaatcgtattagtcacccgccaggtgtgacgaaaaaacgatgttctgatggcgtctaagtggatggtttaacatgaaattacaacaacttcgctatattgttgaggtggtcaatcataacctgaatgtctcatcaacagcggaaggactttacacatcacaacccgggatcagtaaacaagtcagaatgctggaagacgagctaggcattcaaattttttcccgaagcggcaagcacctgacgcaggtaacgccagcagggcaagaaataattcgtatcgctcgcgaagtcctgtcgaaagtcgatgccataaaatcggttgccggagagcacacctggccggataaaggttcactgtatatcgccaccacgcatacccaggcacgctacgcattaccaaacgtcatcaaaggctttattgagcgttatcctcgcgtttctttgcatatgcaccagggctcgccgacacaaattgctgatgccgtctctaaaggcaatgctgatttcgctatcgccacagaagcgctgcatctgtatgaagatttagtgatgttaccgtgctaccactggaatcgggctattgtagtcactccggatcacccgctggcaggcaaaaaagccattaccattgaagaactggcgcaatatccgttggtgacatataccttcggctttaccggacgttcagaactggatactgcctttaatcgcgcagggttaacgccgcgtatcgttttcacggcaacggatgctgacgtcattaaaacttacgtccggttagggctgggggtaggggtcattgccagcatggcggtggatccggtcgccgatcccgaccttgtgcgtgttgatgctcacgatatcttcagccacagtacaaccaaaattggttttcgccgtagtactttcttgcgcagttatatgtatgatttcattcagcgttttgcaccgcatttaacgcgtgatgtcgttgatgcggctgtcgcattgcgctctaatgaagaaattgaggtcatgtttaaagatataaaactgccggaaaaataatttcttgcgttattttcggcaccttttatgtagcgaaggtgccggaatatattctcttttgttacttatttctataccgtgcacaatatttttatccctcatatttatagggtaaattacctgtaaagtagtgtctaattacccgcctcgcaaactccagttttcaaatatctatttcaggtcaaaagattgaattattcactggagacgattcgtaaattcgctggatttttgactaaagtttctttaggatttgtctcatcgtatgattaattacaccaatcgttcaacgtcttgctgataagtgatggcgattatatgaggttagcaatgccttctggaaatcaggaaccccgccgcgatcctgaattaaaacgtaaagcctggctggcggtttttcttggttctgcacttttctgggtggttgtcgcactgctgatttggaaagtgtggggataactatggtcggtcaggagcaactggagtcgtcaccattatgccagcatagtgacaatgaaacagaaacgaaacgggaatgttccgtcgttattccagacgactggcaactaacatcgcagcagcaagcctttatagaactgtttgctgaagatgatcagccgaaacaataattatcatcattcttattacccatttttaatgaattaaagggcttttaatacaccgcagcaataacagcttgagttatctcaacacaaaataataaccgttaagggtgtagcctatgatcaacacaaatatgaaatattggtcctggatgggcgcgttttctctgtcgatgctcttctgggccgaactcctctggatcattactcactgatccttgaccccgctgcggcggggttgtcatttgctttgccacaaggtttctcctcttttatcaatttgggttgttatcaaatcgttacgcgatgtttgtgttatctttaatattcaccctgaagagaatcagggcttcgcaaccctgtcattaaggaggagctatgtcgtcaaccctacgagaagccagtaaggacacgttgcaggccaaagataaaacttaccactactacagcctgccgcttgctgctaaatcactgggcgatatcacccgtctacccaagtcactcaaagttttgctcgaaaacctgctgcgctggcaggatggtaactcggttaccgaagaggatatccacgcgctggcaggatggctgaaaaatgcccatgctgaccgtgaaattgcctaccgcccggcaagggtgctgatgcaggactttaccggcgtacctgccgttgttgatctggcggcaatgcgcgaagcggttaaacgcctcggcggcgatactgcaaaggttaacccgctctcaccggtcgacctggtcattgaccactcggtgaccgtcgatcgttttggtgatgatgaggcatttgaagaaaacgtacgcctggaaatggagcgcaaccacgaacgttatgtgttcctgaaatggggaaagcaagcgttcagtcggtttagcgtcgtgccgccaggcacaggcatttgccatcaggttaacctcgaatatctcggcaaagcagtgtggagtgaattgcaggacggtgaatggattgcttatccggatacactcgttggtactgactcgcacaccaccatgatcaacggccttggcgtgctggggtggggcgttggtgggatcgaagcagaagccgcaatgttaggccagccggtttccatgcttatcccggatgtagtgggcttcaaacttaccggaaaattacgtgaaggtattaccgccacagacctggttctcactgttacccaaatgctgcgcaaacatggcgtggtggggaaattcgtcgaattttatggtgatggtctggattcactaccgttggcggatcgcgccaccattgccaatatgtcgccagaatatggtgccacctgtggcttcttcccaatcgatgctgtaaccctcgattacatgcgtttaagcgggcgcagcgaagatcaggtcgagttggtcgaaaaatatgccaaagcgcagggcatgtggcgtaacccgggcgatgaaccaatttttaccagtacgttagaactggatatgaatgacgttgaagcgagcctggcagggcctaaacgcccacaggatcgcgttgcactgcccgatgtaccaaaagcatttgccgccagtaacgaactggaagtgaatgccacgcataaagatcgccagccggtcgattatgttatgaacggacatcagtatcagttacctgatggcgctgtggtcattgctgcgataacctcgtgcaccaacacctctaacccaagtgtgctgatggccgcaggcttgctggcgaaaaaagccgtaactctgggcctcaagcggcaaccatgggtcaaagcgtcgctggcaccgggttcgaaagtcgtttctgattatctggcaaaagcgaaactgacaccgtatctcgacgaactggggtttaaccttgtgggatacggttgtaccacctgtattggtaactctgggccgctgcccgatcctatcgaaacggcaatcaaaaaaagcgatttaaccgtcggtgcggtgctgtccggcaaccgtaactttgaaggccgtatccatccgctggttaaaactaactggctggcctcgccgccgctggtggttgcctatgcgctggcgggaaatatgaatatcaacctggcttctgagcctatcggccatgatcgcaaaggcgatccggtttatctgaaagatatctggccatcggcacaagaaattgcccgtgcggtagaacaagtctccacagaaatgttccgcaaagagtacgcagaagtttttgaaggcacagcagagtggaagggaattaacgtcacacgatccgatacctacggttggcaggaggactcaacctatattcgcttatcgcctttctttgatgaaatgcaggcaacaccagcaccagtggaagatattcacggtgcgcggatcctcgcaatgctgggggattcagtcaccactgaccatatctctccggcgggcagtattaagcccgacagcccagcgggtcgatatctacaaggtcggggtgttgagcgaaaagactttaactcctacggttcgcggcgtggtaaccatgaagtgatgatgcgcggcaccttcgccaatattcgcatccgtaatgaaatggtgcctggcgttgaaggggggatgacgcggcatttacctgacagcgacgtagtctctatttatgatgctgcgatgcgctataagcaggagcaaacgccgctggcggtgattgccgggaaagagtatggatcaggctccagtcgtgactgggcggcaaaaggtccgcgtctgcttggtattcgtgtggtgattgccgaatcgtttgaacgaattcaccgttcgaatttaattggcatgggcatcctgccgctggaatttccgcaaggcgtaacgcgtaaaacgttagggctaaccggggaagagaagattgatattggcgatctgcaaaacctacaacccggcgcgacggttccggtgacgcttacgcgcgcggatggtagccaggaagtcgtaccctgccgttgtcgtatcgacaccgcgacggagttgacctactaccagaacgacggcattttgcattatgtcattcgtaatatgttgaagtaacaactatttgcttgccggttattttgcttccggcaagcaaatgaattacacaatgcaagagggttatttgttcagcaaatggcccattttctcggctttggtatcgagataatgttcgttattggggttacgacctacaatcaatggtacgcgttcaacaatattaatccctgcttcggtcagaatttcgacttttttcgggttattggttaacaagcggacttcattgacgccaaggagtttgaacatatcagcgcaaagagtgaagtcgcgctcatcagcggcgaagcctaactggtggttagcctctacggtatcgtaaccttgatcctgcagtgcgtaagcgcggattttattcagcagaccaatgttacgaccttcctgacggtgatacagcaaaataccacggccttcctcggcaatttgcgtcaatgccgcttcgagctggaagccacaatcgcagcgcaagctgaacagggcgtcaccggtcagacattcggaatggacgcgcgcaagtaccggggtatgcccggaaatatcgccatagactagcgcgacatgatcgtgtccggttgccagttcttcaaatcccaccatcaggaaatcgccccatggggttggcagtttggcttctgccacacgtttaagctgcatgaaattctccagataatgctggttctgtattggcttattttgccataacgagaaggggttcacctaatcacgacgcgtcgatcgttcacggaatggcacaaatctgtcaatttttcctggaactggcgttttcagttatgattgtgggacttatcaaaaaggagaggccatgcgttcgattgccagacgtaccgcagtgggagctgcactattgcttgtcatgccagtagccgtatggatttctggctggcgttggcaacctggagaacaaagttggctactaaaagcggctttttgggttactgaaactgtcacccagccctggggcgtcattacacatttgattttattcggctggtttctctggtgtctgcgttttcgcattaaggctgcctttgtattatttgccattctggcggccgcaatccttgtgggacaaggcgttaaatcctggatcaaagacaaagtccaggaaccacgaccttttgttatctggctggaaaaaacacatcatattccggttgatgagttctacactttaaagcgagcagaacgcggaaatctagtgaaagaacagttggctgaagagaaaaatatcccacaatatttgcgttcacactggcagaaagagacggggtttgcctttccttccggtcacacgatgtttgctgccagttgggcactgctggccgttggtttgctgtggccgcgtcggcgaacgttaaccattgctatcttgctggtctgggcaacgggagtcatgggaagccgcctgctgctcgggatgcattggccacgcgatctggtagtagctacgttgatttcgtgggcgctggtggcggtggcaacgtggcttgcgcaacgaatttgtgggccattaacaccacctgcggaagaaaatcgcgaaatagcgcaacgagaacaagaaagttaacgctggttgattttccgaatttagcccttaaatcatcaacaatgcgtgtggatgccatttcgcagacggcgcgaaaatggtactttaaagggctattgcggtaagttgaccataatttattcgctctaaccacataacgggaagtaatgtgaaatatttactcattttcttactggtgttagcgatcttcgtgatttcggtcacgttgggtgcgcagaacgatcaacaggtgacgtttaattatctgttagcgcaaggggagtaccgtatttccacattgctggcggtattgtttgctgcggggtttgctatcggttggttgatttgtggcctgttctggctgcgagttcgtgtttccctggcgcgcgctgaacgtaaaataaagcgactggaaaaccagctttcacccgcgactgacgtggctgtagtgccgcactcgtcagcggcgaaggaataactttctatgctggagttgttgtttctgcttttgcctgtagccgctgcctatggctggtatatgggccgcagaagtgcgcaacaaaacaagcaagatgaagccaaccgcttgtcgcgtgattacgtagcgggggttaacttcctgcttagtaatcaacaggataaagcggtagacctgtttctcgatatgcttaaagaggatacaggcaccgttgaagcccaccttacgctcggaaacctgttccgttcgcgtggcgaagttgatcgcgctattcgcatccatcagaccctaatggaaagcgcctcgctgacctatgaacagcgtctgttggcgattcaacaactggggcgtgattacatggccgccgggttatatgaccgcgcggaagacatgttcaatcagctgaccgatgaaactgacttccgcattggcgcgctgcaacagttgctacaaatctaccaggctaccagtgagtggcagaaagcaattgatgttgccgaacgcctggtgaagctgggtaaagataaacagcgcgtcgaaattgcccatttctactgtgagttagccctgcagcatatggccagcgacgatctcgatcgtgccatgaccttgctaaaaaaaggggcggcggcagataaaaacagcgcccgcgtatccataatgatgggacgcgtgtttatggcgaaaggagaatacgccaaagccgtcgaaagtctgcaacgcgtgatatcccaggacagagaactggtcagcgaaacgctggaaatgttgcaaacctgctatcagcagttgggtaaaactgccgaatgggcagaattcctgcagcgtgcggtggaagagaacaccggtgccgatgctgaattgatgcttgctgatatcatcgaagcgcgcgacggtagtgaggccgcacaggtctatattacgcgccagcttcagcgtcatccgaccatgcgtgtgttccataagttaatggattaccacttaaatgaagcggaagaagggcgtgccaaagagagcctgatggtgctgcgtgacatggttggcgagaaggtacgtagtaagcctcgttatcgttgccagaaatgtggttttaccgcatacaccctctactggcattgtccgtcttgtcgggcctggtcaaccattaaaccgattcgcggtcttgatggcctgtaatttttaaaaaaaatccgactttagttacaacatactaattattaatgttccattgtgctccggcaacgacggcgcagaaaaagcctgccaggggagaaatcgcaactgttaattttttatttccacgggtagaatgctcgccgtttacctgtttcgcgccacttccggtgcccatcatcaagaaggtctggtcatgacgttaactgcttcatcttcttcccgcgctgttacgaattctcctgtggttgttgcccttgattatcataatcgtgatgacgcgctggcctttgtcgacaagatcgacccacgcgattgtcgtctgaaggtcggcaaagagatgtttacattgtttgggccacagtttgtgcgcgaacttcaacagcgtggttttgatatctttcttgacctgaaattccacgatatccccaacactgcagcgcacgctgtcgctgctgcagctgacttaggcgtgtggatggtgaatgttcatgcctctggtggggcgcgtatgatgaccgcagcgcgtgaggcactggttccgtttggcaaagatgcaccgcttttgattgctgtgacagtgttgaccagcatggaagccagcgacctggtcgatcttggcatgacactgtcacctgcagattatgcagaacgtctggcggcactgacgcaaaaatgtggccttgatggtgtggtgtgttctgctcaggaagctgtgcgctttaaacaggtattcggtcaggagttcaaactggttacgccgggcattcgtccgcaggggagtgaagctggtgaccagcgccgcattatgacgccagaacaggcgttgtcggctggtgttgattatatggtgattggtcgcccggtaacgcaatcggtagatccagcgcagacgctgaaagcgatcaacgcctctttacagcggagtgcatgatgagtgattccaacagccgtctggtctactcaacggaaaccggacgtattgatgagcccaaagcggcccctgtacgccctaaaggcgacggtgtggtgcgtattcagcgtcagaccagtggacgtaaaggtaagggcgtttgcctgattaccggtgtcgatctcgatgatgccgaactgacaaaacttgcagcggaactgaagaaaaaatgcggctgcggcggagcagttaaagatggagttattgaaatccagggcgataagcgtgatttattaaaatcactacttgaagcgaaagggatgaaggtaaaactcgcaggcggttaacataaaaagccacggatatatccgtggctttcgaatattttactgtgcgtattattcagttatttcgtactgaacagaatcaagcgtattataattgcgagtcgataatcgacatttatttacgattatttaccgacctggtgaccaataacacctccgacagctgcaccacctaatgtacccaacgtactgccatcggtcagtactgcaccgcctaatgcccctgcacccgcgccgattgcggtgttgcggtcccgtttagaccagttagaacaggcactcagagacattgccaaagtaattgccagaacagccgcggtcatttttttgctcgttacaaacataatactctctcctgaatttatgattcacggaagtaagctctctataactataatagctaagaataagtctggtgaaattattccgtgaaatctgctcgcgcgcagggttatatcacgcaggtgataatgacttcctgttatatcgctgataataattttatatcttgagagtgttaataacaggtaaatagtcttaattatcaaccaggaatcatcttagagcggatgatttgccaaactgcaaatcatccgtagagaagggaaatggttaaatgtcaacgacgtgaatggtgagtttactgtgctcaagatgcatcagatcgctggcgcgtattttcgaatcggtaatcacgcgattgaatcgctcaacgggaccgatggagtatgaatgtacagcaccaaatttcgagctgtcagtcaggactatcgcttcgcactctttttccagcacggcattgaccacatcggtacgcatcatatcgcgaccggtaaatccagtttcaggttgccagccatcaataccaataaatgctttgctgaaatgcacctgttggatgcactggcgtgtcaaagggccaaccatactttcgctttttttctgatacacgccaccgagcaaaataacttcacaaggcgcgtctttcagcaaatgcgcgatgtagctgctgaccgtgatgatagtgacatttttcttctgctcgcccagagtccgggcgagtagggcattgctgctgccattttcgataaagatggtttcgcccggttgaaccagcgacgcggcaaactcggcgagttcacgcttcagcgtatagttgctcatcatacgggtttcgacgtcatcactatcaagcgaaacagcaaagccatgtgcacggcggaggtaactcagtttttcgagtgtgttgagatcctggcgaatggtaacttcagaaactccagtggcttttgccagatcggttacgctaacctgaccctggtcaatgaccatctgtagaatagtttgttgtcgggaattcatcgctgtaattcttataacgttataatacttaataaaaaaatactgacgcgccgggcatcctcaaataggaaaacctgaaggcacgattgttaaatctcccacggtgccttcgggatgtctggcgtagattcagcaacctggcgcaagagttctgctttaagtatctcgagattatggatcgcagagtggtaatcgcctgccacaaggatatctaacacaatatcaatacgttcggcaacgcgctgggcatcaaattcagacatcaaggacatccttatagcaaaagggggaaaatgaataatgcaaaaattgccgctaaaagagaagtgtttaacagcaacggctaattatcatccaggaatacgatatataatgacgggatatagcgctaagtatatatattcatctacttatgcgcgcttcagatagcgtttataccagcgttcgaaggcgacggcgggcatcggtttggcaaacaaaaatccttgccgctcattgatcccgttcttggttaaaaaagcatcttcctttgcactctctacaccttcggcgatcacctgaagattcaatgcctgggccacagcgacgatcgcccggaccagtgactgcgagacaggttgtttgtgaatatctcgaacaaaaacctggtcaagtttgatggcatcgatcggaaagcgcgccagttgcgaaagtgaagagtagccggtaccaaaatcatccagatgcacttgcgcacctagttggctaaattgttgaataacagacagtgccagttcatcattctcaatcagacaactctctgtcagttcaacatctatagggcagtattcaaaattgagttcctggagaacctgtttcagggcggtgaaaatggtttgatcggcgagctgacgtgcagaaatatttaccgccactcgcaggtttatgcctttatcccgccactttgccacctggcgtacgacatcgagaatcacccaacggcctaaaggcacaattagccctgactcttcggcgtaggaaatgaagtccaacggtggaatcaacccacgttcaggtgactgccaacgtactagtgcttccagactgcgcacttcgccacgccaggtgattttcggttgatagtgaataaccaactgatcgttttccagtgctttacgcaagttggtatccagccagagatattcaaatacccgttgattcatttctggggtaaaaacgcaaaattgtcctcgtccgccttccttcgctgtgtacattgctgtgtcggcgtgacgaataatagccgtgctgtctgaaccatgttcgggagagagtgcaatacctactgaacagctggtataaacttcaattaaaccaatgcgaaaggggagccgtaagcgggtcaaaattcgtgatgccattgcttccagcgcgctttgtgaggtgttggatgccagtaccagaaactcatccccacctggacgcgccaacacctggtcatgttcgagacagcttaaaatagccaatgacacgtcgcgtaataactggtcaccaaacaaatgcccataggcgtcgttgacctttttgaaattatccaaatcaagatacacaaccccaactttattgttatctgcatgattaatagcgtgatcgattaaatcctgcattgcgttacgattcggcagtccggtgatactgtcggtatttgccagaatacgcagtcgctcctgagcgcggcgctcttcggtaatgtcggtgccggaacagattaaaaaaatctcgtttttgccactgccgctgtggacaaatttattgcgaaacagaaacagccgctggcctttacatgttggtatccacagttcgacttcatatgcattgccgcttcgaaaaaatacacggttattgcgcctggatgccgcagcttcacgacggctcataaacagtttaaacacgctttgcccaatgacgtcgtgttctttcaaccctgtgtaatcttcacataaccgattgaagcgttggatattcccccggctgtcgagaatcactattgcggaatgtgcttcagaaactacctgctcagcaaaggaaagcccgtgtgataaatcacgagcaaccgccggtgtgtcatgccatgcagacgcgttgccagcccattcccgtttattgatttttcgtcctaccagatgcacagaaagatcgctttcatcgacggtcagactcatcatcaggctggaggtgatgaccgtcatttccctgatgcgagcagcctgttcggcagataactgcaatgtacgatcaggttctgtggtttcggtggtagaaaagcgcaaaacatcgctgctttccgtcaaccgccagtatggattgtgcgatccgagaaagttgtacaacgttgtggactccctaacggttttcatgatgcatatcctccggttaacagcggagtccgcggttaaataaaaggaacaacatgacttacatgaaattaacggcggctaaacgcattgttttttttatatatttatttgtaatccagttttggaaaaacgccagttttcaaacgaaagtcagttaaaaaatctgcctggatataacgaaggtagagcggggaaataaacggcccatccatgaggaatgggccgtgaaaggagattacgcgaccgggcgcgcaataatgctgcgggtttccatgcggacttcggcaatagtgacgtcaataacgtcagtcactttgtaaaccgtttcacctttaatttgtacagtgccgttttcctggctgcaaaccagttcatcgcgcacagcgtgtaagaaaggtgccggaataaaggcgatagcgccgttatcaaccaaacgaacacgcatgccgccacggctgatatcgacaatttccgctgcgaaacgggtgtcggtcccggctttgtctttcaggaagcgtgcgtataaccagtcaccaacatcacgttctgccatccggttgagacggcgacgctcggccatttggacagtgatttcatcctgtgggcgcgtcgcagtttcgcctttgataaccgctttcagcagacggtggttgatcatgtcgccatatttacggatcggcgaagtccaggtggcgtatgcttccagaccgaggccaaagtgaggaccgggttcagtgctaatttcagcaaatgactggaagcgacgaatgcggctgtcgaggaaaccagttggttgcgcgtccagttcacgacgcagtttgcagaaaccgtccagcgtgagcacttcttcggcatcgacatgcagaccgtgcgttttcagcaacgctgccagcgcgtcggcattcgccggatcaaagcccatatgcacgttatagatgccaaaaccgagcttatcgcgcagtacgcgggccgcacaaatgttagcggcaatcatcgcttcttcgacgatacggttggcaatgcgacgaggctcggcgacgatatccagcacttcacctttttcaccgagaataaagcggtaatccgggcgatctttaaacaccagtgcgtggttatgacgccactcgccgcggcgttggcaaatttgcgctagcaaacggacttgttcggcaattgcttcactttcaggctgccagtcaccggtattttccagccagtcagaaacctggtcatacaccagctttgctttggattcgatggtggcggcaaagaattcgatattatcttcaatggtgccatcagcggagagcgtcatgcggcatgccagtaccgggcggacttcattggcgcgcagtgagcagagatcgtcagaaagctcgcgaggcagcatagggatgttgaagccaggcagatagttggtgaatgcgcgaattttcgcggctttgtccagcttgctgccttcagcaatccacgcggttggatcggcaatcgccacaatcagctgaagtttgtcatccggcaacgccttagcgaaaagggcgtcatccatatcttctgtgctggcactgtcgatggtgacaaaatccagcgcggtcagatcttcacgaaccagaccttcatcgagcatttcggtagcgacgccgtctggtgcttctttttccagattatggcgtgcaagggtaacccaccacggtacaaagtgatcgtcaccaaaagtgatgtattgtgtcagttctgcatagaaagaacgatcgcctttcagcggatgacggcgcatttcggcaaccgcccagtcgccttctttaaactcgtggttcaggccacgggctgcgcggcaaggaatggcgtcttttaagagtggatgatcaggaacgatggccagacggtcatttttgccctgaaccttacccacgaaacgagtcaggaacggttcaaccagttcttctggctctgcggattcacgttctttttcactgtggatcaccgcgataattcggtcgccatgcatgacttttttcatctgcggcggcggaatgaaataacttttttgcgcgtcgacttccaggaagccaaagcctttttctgtggcttttaccaccccttcagcgcgtggcgtctgggaatgcagttgctgtttaagctgcgctagcagcgggttgtcctgaaacataattgtctattttggtggccattagagcggctgacagttttacgcgaatctgtctgacgcggcaaggttaatatgtctcacccaacgcgatttttaagcgatttatccagccacacagcccgctccataccagcagattaataatctgcgttgatgatttttcgtgttcgagtaaagggctgaactgggcggcgctaaagcgatcgggtgctcgggtcagccattgtatcgcctgaacggtagcgcgctcaacagaatgacggtcagcccattggttaatttcattttcgcccttgcgcataagggtgctgatttttttatattcatttgatgaatccatacaggtggcaaaacaagcaggactgccatttatacgcgcgcataacaacgccgcaagctgattatccggctgtgtattgccccgtgtgctgtttaacaacttttcgagaagggaaagtgaaatagggtggagagagagtatttcggccagttggcaaagttctgcagttgaactttttgtgtgctcttcaggtagtttttccacctcatagctgcttcgccagcgtaatgattcatcagcaaacagtgacgcgtcggcgtagttttgtatctccagcccgggtaaccagcgtaccggatgcccgagataagcctgaaatgtcgcaattgtccgcgcctgaaagccaataaaaccaatgatttggctaatgatcacacagtcccaggcagtaagaccgacgtcattcagatgctggcgcgatcggttgtcgataatagaaggcgagctagccagttggcgggcatattgcgtgatttgtgccaaccgatgattactttccctggtggaatcaggcccggggagcggcgtaagtcgcgccgaatagtagttacataaccgctggacgccgcaaacctgagcaaccgtcagggccgtcgacaagcgttcataagcggtgaaggtctgtgaacgggtcacggtaagctggtcagggaacaaatccactgcaagaacacgcgcagggtccagccatgaaaggaagggggccagcgtttctttttcaaggatcacgtcgagtagaaagggatcgctgacctttgcggcttccgggaccagaggcagaacgtcatactccgtagtactggattgcgtttcatgataccagtggcttttgccggtgatgtggcgttgttccatgggcgctccttggtcgtaaaggaaatcgttatcctgacgcaaggcgggaaggggagaaagacggatcggcgataacaaatatcagaaaggtataacagagataacgggcggcagaacgccgcccatctttaccaacagaacgattatttcagttcgagttcgttcattgcagcaatgctgaaaccgccgtcaacgtggaccacttcaccggagataccggcagagagatcggagcacaggaatgccgcagagttacccacatcttcaatagtaacggtacggcgaatcggggtaacggcttcgcaatgagccagcattttgcggaagtctttgataccggaggccgccagagtacggatcggaccagcagagatggcgttaacacgcacaccttccggacccatcgcgttcgccatatagcgcacgttcgcttccagagacgcttttgccagacccataacgttgtagttcgggatagcgcgctcagcgccaaggtaggaaagggtcagcagggcagaacccggattcagcatggagcggcaagcttttgccattgcaacgaagctgtaggagctgatgtcgtgggcaattttgaagccttcacgggtaacggcgttaacatagtcaccatccagctgatcgccaggtgcaaaaccaatagagtgtacgaaaccgtcaaatttcggccaaactttccccagttcagcgaacatggtgtcgatgctggcatcttctgcaacatcgcactgcagaacgatgtcagaacccaattgagcggcaaattcttctacgcggcctttcagtttgtcgttctggtaggtgaatgccagttcagctccttcgcggtgcatcgcctgagcgataccgtaggcgatggatagtttgctggcaacaccggttaccagaatgcgcttaccggaaagaaaacccatagctttaatccttattgttgatgcttgttgtgcctgaaaatcaggcgattcgtcgttttagtaaacagtacgaacagataaacggttattataatcaacctggctgtgagtagctatagttgccaggtccgaccggagcaggctgcggcagggggggcgcttttcccctcaccctaaccctctccccagaggggcgaggggaccgtattgtgcaaatattgttaccccagcaacaaacaggctcatacagcccctaaccctttcatggcgatggctgggacggttcagaccttgccgaatattctccagcaccgtctccatgttttcaccacaacagctattcggctcggtctgccccctcgctctttcagggagagggtgaccggcggttcagttcctgcagaatattctccagcaccgtctcctcattacaatcaatctcgttattccagaaacgcagcacggtccagccctgcgactcaagccagctagtgcgcctggaatcataggcaactgctaaatcatgctgcccaccatccagctcaacgactacacgcgccgagcagcaagcaaaatcgagaatgtagctccccactggatgttgacggcgaaatttgaaatcactaaaacgtcggctgcgaagatatcgccagagctttcgttcctgcaaagtgagattgcgtcttaaatcacgcgcatttgatttaattttatctatcacctcattctgacaagatttaatcttttgtcagaatgaggtgaataatctggaaggaggattcagaaaattagcgatctttacgccacgcatccgccgtcaatgcctcgccaaaatgaccggcaatcagccgtttggtgagttcatgcagcggcgatgccagcacatccgcggtgctgcctcgctcgacaacctcgccctgatgcatcaccagcacctggtcgctaatgtgcttcatcattccgatatgctgggtaacataaatatacgaaatgccctgtttttcctgtaattccagcatcagattaatcaactgcgaacgcatcgacatatccagtgaagcgagggcttcatcggcaataatgacttttgggcgcaatatcagcgcgcgcgccagacccagacgctgtttttgtccgggtgccaacatatgcggatagtaactgacgtgatccggtagcagcccaaccatacgcatcgtttcaataatctgtttgcgacgctgttccggttccaggtcggtgttcaggcgcagtggaaaatccagaatttgcgagatacgttgacggggattcaacgaggtcgaaggatcctgaaaaatcatgcgaatacgctgactgcggaaggaataatcgccaaaatgcagtggatgatcgtcaatcaataactcgccgctggtaggctctatcattcccgccagcatttttgccagcgtggatttacccgaaccattctcgccaataatcgccagtgtctggccttcacgtagcgtaaagctcaagggttttaccgcttctacggtctgacgacgaaaccagccggtccggtagcggaacgttttacttaaattacgcacttcaagcagcgtttcgatcatctcactctttctccatgttcagcgggaaatgacaggcatagagatgatttttcgcccccgtcaaacgtggcgtcacaatgcattctcgttgtgcatacgggcaacgtggccccagacgacaaccaatcggtaactgttccagcagtgggatagcgccgggcagcgtattgaggcgacttttatgcggcatcgcgctgccgaagtctggtatcgcgcggatcagcgcctgggtataaggatgatgtggcatcgtcaccaactccttactcggcgcggtttccactgtttgaccgcagtaaagcacgttaattttatccgcccattggctaagcatttgtaagtcatggctgataagcaaaatagtggtattgctgttttggttgagacgcgtcagcaggcgaaagatttgcgcctgggttgttggctccattgagttggtcggttcgtcagcaatcagcagacgcggttgattcgccagtgcaatggctatcatcactttctgacattcaccttcggtcaactcatagggaaaactgcgcatcgcatctttgtgatctttaatccccacgcggtgcagcagttcaatggcacggcgtttgcgccagccaaaacgctgccaccaacggcctttataggtccaggctgggatgttttgcatcaactggcggcccacacgttctgaagggtcaagacacgactgcggttcctggaaaatcatcgacacgttatggccaaccagtttgcgccgttcgcgtgcggagagacgcagcaaatcgatatcatcaaaacgcatacggtcagcagtaacacgccagttatctttattcaccccacaaatcgctttcgcaatcaaactcttgccggaaccggattcaccaacaagaccgcggatttcaccttcggttaaggtcatacttacccggtcgacggctttaacccactcatcaccggttttaaattcaatggtcaggttacgaatatcgagtaatggcattattccacccccgcaataatcgcacgacgaacgccatcgccaaggaggttaaccaacaacacgctaatcataattgccgcacctggcagcatgacagtccacggggcgacataaatcagttccagcgcatcaccgagcatcgctccccattcaggcgaggggagttgtgcgccgagatcgagaaagcccagcgcggcgatatcgagaattgccatcgacagtgcgcgggtgatctcggtgaccagcccggcggtgatgtttggcatcacagcaaaccagagaatattcagcgttgatgcgccatccagacgggcggcgataacgtactctttttccagttcgtcatgcaccatgctgtaaatcgaacgtaccatacgcggcagcaatgccagccagacagcaaacatagcgtgggacaaactcggtccggcaaacgctacaacgataattgccaacagcagcgaagggatcgccagtaaggtatccagaatatggttaagcaccgctgagcggaggccgtgtgtcgccccggcgaaggtgcccagtaccaggccacagatcgtcgcggcaagcgtcaccacaaatgcgccacccacggttggcgcagctccgctcagtaaacggcttaaaacatcgcgtccgaggtcgtcagtccccaggaagaaagaaacttcgccatagcgcgaccatgacggcggcaataattgataaccgagaaattgctggtcgatgccgtaaggcgcaaaccagccgccaaaaatacacagtacagccagccccgcgcagccgtacaggccgaccatcgcagaggcgtcactataaaatttgcgccaggcggtacgcagcgtgcccggcgggcgcttttcgctgtatacgctatcgtaaggcataccattccttatgtttcagagggttagccatggcacccaaaatatcagaaatcacgttaacaataatgaccagtgagccacacaccatcactccggcggaaatggctgcgtaatcctgctggcggatggcgttaattaaccagcgccctaaacccggccagctaaaaaccatttcggtgatcatcgccagcgtcagcatggtggaaaactgtaagcccaggcgaggaataaccggcggtaacgcgttatgcagaacgtggcgacgcaaaatagtaaagcgcgacaaaccgcgggtcgccgccgcttttacatagttctggtcatacacttcgatagtgctgatacgcatcaggcggatcacttcagttgttggcgcaaccgacagggtgatcacgggcaatatcatatggcggattgcgctcatgatcatttcatcccgccatggtgagtccgaaagccaggcatcaatcaacgcaaaaccggtaatcggtttcacttcgtagagcagatcgaaacgccctgaaacgggcaaccaacctagcgtgagtgaacaaaacagcgtcaacagaagcgccagccagaacaccgggattgaaaagcccagtaaggcgatggcgttgatcaagttatcctgccacttatggcgcgtaatcccggcaatcatccccacggggatgccaacaatcagcgcaaaaccgaaggcgaggatgcacagttccatcgtcgccgggaagacctcttttaactgttcggcaatcggttgaccgttaatgctggaaacaccaaaatcccagtggatcaggccgttaaaccagaacacccaggcattccacagtgacgcgccttgtaacggcgcatgaggggtgaaatagctcaagctgaagccaacgaaggtcagcaggaacaaggtgacaatcaataacaaaatgcggcgtaaggtgaagataatcatggttttttcacctcatcctgtttctcgcgatacaccccagcaaaggaggcgttaccaaacgggctaagtaccagacctttgatatcgtaccgataggcctgcaaacgcaatgacgacgccagcggcaaaatgggcaattcctgcgccagaatactctgcgcttcgtcataggcttcaatacgcgccgccagctgctgcgaagagagcgccttacgcaatacgctgtcgaatttcggatcgcaccagtgggcgaggttggtctgcgaatgaattgccgcgcagctcagtaacggacggaagaaactgtccgggtcgttactgtccgtcgcccaaccggataacgtcagatcatggctcatatccatcaaccgcgcctcctgaaagcgaccttctaccggcacaatcaccacttttacgccaacctgcgccatatccgcctgaatcagttcggcagttttcagtggactggggttccacgcctgcgaacgtgtgggcacccacagtttcagcgttaaattttccagccccaacgacttcaactgttcgcgcgatttcgccggattgtattcagtaattttagcctcgttgtcataggcccacgaggcgcgcggtaaaatagaggccgccgtttcagccgtaccataatagatggattgcatcaggcgctggttattaatcgccagtgccagcgcatggcggacagcgggattatttagcggcggtttggcggtgttaaatgccagataggcgacgttcatcccaggacgcagcgttaaacgcaagcgcgggtcgtcacgcaaaatggatagctggctggcagcaggccaggccagaacgtcgcattccccggtcaggagtttcgacagacgtccggtgccgccggagcctaaatccaccactacctgcggcattaacggtttaccgcgccagaagtcatcatgacgttgtaggcgaataaattgcccggcgcggtattccgacaactgatacggaccggtgccgaccggttgacggtcgagttgctcctggcgatcttctttctctaacttccgggcatattctgccgacatgaccgaagcataatgggttgcgaggtgccacaaaaaagaagcatccggctgggcgagtcggaactcaacggtatgattatccagtttgcggacgcttttcacgttatcggcaaattgcaggctgtcgaagtaggggaagttgctgccgttgacgttatgccacgggttgttgcggtcaaaaattcgctggaaggtaaacaccacatcgtcggcattcattttacgagtgggagtaaaccagtcggttttttgaaacggaacatcgcgacgcaggtggaagcgataggtcgcgccgttgtcgagtacttcccagctttcggcaagttccggcatcaggcgataggtatagggatcgacatccagcagtcgatcataaaactgggcggcaagggtatcgacaattaacccactgctcgctttggatgggttaaaggtgttgacttgcccgctgacgcaatagacaaaaccgctgtcgcggatatcagcatgcgggggagattcaggcgcggcgattgcctgaccactcacaagtccagcaatcaccaaaagagacgataatacctggcgcataatattaagggattttatgtaaagaggctatcttactaatatttaatgacatttgccattaccgtttgtgttcaggggtcgtaatgagggccgtgtggttggtcgttgaacaggtgacgtcgccatctgttcaacattcgtacccgtgatttctctataactataactcacagaacaacttagcgaggagcagagcggtacgatcgtgagaaacccattaaagcacgctgcagtgcgtgtcattgttagccagatgcggcgtgaacgctttatccggacaacgatactgaccgatcgtctgcaattaaatcattactcattaccccattgattcaaaaactctgcgatctcatcaatgcgtacgggattaatccccgcttcagcagccatttcatgttgggcttcttcgctgatctcttcattgttcatcaaacgggtgagcagtaactggaagtagtgggccagcggtgtgcgttcagcctctgcgacaggctctgcgcattcggtcgcgtactcatcggcaatatcaaaatattttagcgggatatcgtggttcattatttgcccctggggttaatgcgctaagcataagggcggatgatagcactcgtgatccgggtcatacatctttttatagttaatggcgcggcgcgttaccctcaggcaggataatgcgccgcgcatccgactattacgtttcactcaccggcgttctgtcaccatcatacaacggcactttgcgatagcggcggatcagataccataaatatgcgccgcctaacgaagcccataccagaccgagtgtcagtgacgttgactcgaggttaacccacagcacacccaccgtcagcgcgccaaccagcggcatcagcaaatagtggaagtgatccttccagcttttattcattcctttacgccgccagaaatgattaaacaccgacagattcacgaaggtaaacgccaccagagcaccgaagttaattaacgctgtggcggtaactaaatcgaagaacagcgccgacaacgcgacaatcccgaccataatgacgttgagtgccggagtccgccattttgggtgcacatagccaaacacgcgctccggaaacacattgtcacgccccatcacatacagcagacgcgacacgctggcatgtgaagccaggccagaggctaacgtgttcacaaacgtggtgcagaggaaaatcgactggaagagcttgccgccgacgtacagcgcaatttcaggcagtgcggcatccggatctttaaagcggctgatatcgggaaagaacagctgcataaagaacgacgccgcgataaagataacgccaccgtagaccgccgtcaggaagatggctttcgggatcacgcgtgcggcgtccggcgtctcttccgaaagcgtggtcaccgcatcgaaaccgaggaaggagaaacagacaatcgtcgccccggtaataatcgggatcaggtgcgcgttctcgctgataaacggctgaagtgaccagacggtgccaacgccttctcctttatgcagtccctgaactaccaggaagataaacaccaccatgatggagatttgcaccagtacaaacagggtattgaagttagcgaccaggttgacgctcttcagattcgcggcggttaaaatggcgacgaaggttaccacccacacccacggcggcacttccgggaagagggcggagagatagattttcgccaacaagacgttaatcatcggcaaaaagagataatccagcagcgatgaccagccgaccataaatccgacgtgcgggttaatcgacttttgcgcgtaggtataggccgaaccggcctccggaaactggcgaaccagtttgccgtagctgatagcggtaaacagcacacccgccagcgccagcaaataggacgccggaacgtgaccgtcgctaatgccggagacaataccaaaagtatcaaatacggtcatcggcgtgagataggccagacccatcatcaccacctgccacaatttcagtgattttcgcagacgggttttgccgggttgcgcagcaatattcagtggtgaattaatagccataattgctgcctcccctgcgtaataaggtttgcggtcgtgtcgacctgaaatcaaacctgtttagcaagggaagcaaagggggcggagtccagtcagtagcaggaggggcgcatacgcagcctccctcgccatgcggggatttaatcatcggcatcatctcatttcctcgtcacagtcttaatcgttaacggaagcccgttgccgcccgcgctccataacgcgacatccgggaaatgtctggattaccagcaaatgtcaggcctggctccgctcaggccgatgaaacaaccccgcaaggggtattacgcgtttttcaacatccactcaatttctgtttctgtgatgaggcgctcaaactgcaacagctcatcatttttacaggcgtgatagacatggcagaagcgttcgcctaaatagcggcgcaggtgatcattctcgataaactcacccagggcatcgctctggcgaatcggaaagggtaagccttcctgttccagcccgttgccttcgacttcttcctgcaacggcagctcgttatcaaggccatgcaaaataccggcaaaaatcgctgccatcaccagatatgggttggcatcggcacccgccacgcgatattccacgcggtgattatgacggtcgccgcacggaatacgcagggcgacggtgcggttgttatggccccacgacgcctgcgtcggcacatacattcccggctggaagcggcgatacgagttcacgtttggtgccagcaacgccatcgacgacggcatcaggtcaatcatcccggcgagcatctttttcagcagcggcgaatcttcgccttccgcgtcagaaagcacgttctcgccacgattattttgcatactgatatggatatgcattccgctgcccgcgtgctcttcatacggcttcgccataaaagtggcgtgcatcttatgcttttctgccatcagacgcaccaggcgttttagtgccagcgcatcatcgcaggcttccagcacgttatcagtatggtaaaggttgatttcaaactgacccggcgaggcctcagcgaccgcgccatctgccggaatcagctgtaactgcgccagttcatcaatatcattgagcacgtcggcgaagtggttgaggttatcaacggagtaaacctggctttgtgtattgcggtcatcggtgccaggcgcgcagggcggttgcagatacccttcagcgtcgcgctggcgatccagtaaatagaactccagctctaccgctacgaccgggaacaatccgcgctggcgcagctgctgccacaggcggttaagaacgttccgcggctcaacgtcaaagggagcgccatcttcatcgaccatggtcaggagcatctgaccgataaactctggatcggcggcagaaggagttaaggaaccgagaacaggaacacaggtacgatccggctcgcccatttcctgacccagacctgcttcttctactacgttgcccagaatatccattgcaaataccgaggccgggaaataacaccctttctcgagcttcttcaggcttgaaacaggaatacgctttccacggaagcaaccatttaaatcggtaagtaaaacatcaacatattgcgtattcgggtagcgctccaggtagcgtttcacttcctgcgtaaaggcgctaccccgcctctcttctgactgctgaacaaagttctctacttcaacgatattggtttccatgattcttcgcctttggtttgttttccgctcgttatcaaagcgtaaaatataatgaccaccattcgaatctgtatgcaaactaaatgtttgtcaaatgttaaattgagtttgcaaaaatgaaaacccactgctagattgaaaaaatattgaacataaaggtcatttaaagcgcagtaatggcgataatttagtccactttgtgagattgagcatggaaaatataatgaacaatccggttatcggtgtcgtaatgtgcaggaacaggcttaagggtcatgcgacccagactctgcaagaaaagtacctgaatgccatcatccatgcaggcggcttgcctattgcgctaccacatgcgctggcggaaccgtcattacttgaacaacttttgccgaaactcgatggcatttatcttcctggtagtcccagcaatgtgcagccgcacctatatggtgaaaacggcgatgagcctgacgccgatcccgggcgtgatcttctgagcatggcgataattaatgccgcactcgaaaggcgcatccccattttcgccatctgccggggtttacaagaactggtggtggcaaccggtggttcgttgcatcgcaagctgtgcgaacagcctgaattgctggaacatcgggaagatcccgaactgccggtggaacagcaatatgcaccgtcgcatgaagttcaggttgaagaggggggattactgtctgcgttgttacctgaatgtagcaacttttgggtaaactctctacatggacaaggggcgaaggtcgttagcccacggttgcgtgttgaagctcgctcgccggatggcttagttgaggcggttagcgtcatcaatcatccttttgcgctgggcgtacagtggcacccggaatggaacagtagcgagtacgcgctttcgcgtatattgttcgagggctttatcaccgcttgtcagcaccatatcgctgaaaaacagcgactctgaccactacagtttaaggaaatgcaaatatgagtgatgagggactggcgccaggaaaacgcttgtcggaaatccgccagcagcaggggctttcacaacgtcgtgccgccgaactctccgggctgactcacagtgctatcagtacgatagaacaagataaagtcagccctgccatcagtacgctgcaaaagctgctgaaggtgtatggtctgtcactctcggaattcttttccgagccggaaaaacctgatgagccgcaggtcgtcattaatcaggacgacttaattgagatgggtagtcagggtgtgtcaatgaagctggttcataacggtaacccgaatcgcacgctggcgatgatctttgaaacgtaccagccgggcacaaccactggggaaagaattaagcatcagggtgaggaaataggcactgtactggaaggtgaaattgttctgacgattaatggtcaggattaccacctcgtcgcggggcaaagttatgccattaataccggcatcccgcacagtttcagtaatacgtcggcaggtatttgccgaattatcagcgcccatacgcccaccacgttttaatctttttgttctgtaagccgggtaagcgcaatgcgcccggcaatctatacacaaaatcattcaagttgcatcaaggcggcaagtgagcgaatcccgatgagcttactcaggtaagtgattcgggggagcgaacgcagccaaggcagaggcggcttgaaggatgaagtgtatataaagaatgtcgccagaaataaacgggcatacggcccggggatctctgcgccctgacgttcacaaactgcatatatctgatagacgtgaaacaggagtcataatgaattttcatcatctggcttactggcaggataaagcgttaagtctcgccattgaaaaccgcttatttattaacggtgaatatactgctgcggcggaaaatgaaacctttgaaaccgttgatccggtcacccaggcaccgctggcgaaaattgcccgcggcaagagcgtcgatatcgaccgtgcgatgagcgcagcacgcggcgtatttgaacgcggcgactggtcactctcttctccggctaaacgtaaagcggtactgaataaactcgccgatttaatggaagcccacgccgaagagctggcactgctggaaactctcgacaccggcaaaccgattcgtcacagtctgcgtgatgatattcccggcgcggcgcgcgccattcgctggtacgccgaagcgatcgacaaagtgtatggcgaagtggcgaccaccagtagccatgagctggcgatgatcgtgcgtgaaccggtcggcgtgattgccgccatcgtgccgtggaacttcccgctgttgctgacttgctggaaactcggcccggcgctggcggcgggaaacagcgtgattctaaaaccgtctgaaaaatcaccgctcagtgcgattcgtctcgcggggctggcgaaagaagcaggcttgccggatggtgtgttgaacgtggtgacgggttttggtcatgaagccgggcaggcgctgtcgcgtcataacgatatcgacgccattgcctttaccggttcaacccgtaccgggaaacagctgctgaaagatgcgggcgacagcaacatgaaacgcgtctggctggaagcgggcggcaaaagcgccaacatcgttttcgctgactgcccggatttgcaacaggcggcaagcgccaccgcagcaggcattttctacaaccagggacaggtgtgcatcgccggaacgcgcctgttgctggaagagagcatcgccgatgaattcttagccctgttaaaacagcaggcgcaaaactggcagccgggccatccacttgatcccgcaaccaccatgggcaccttaatcgactgcgcccacgccgactcggtccatagctttattcgggaaggcgaaagcaaagggcaactgttgttggatggccgtaacgccgggctggctgccgccatcggcccgaccatctttgtggatgtggacccgaatgcgtccttaagtcgcgaagagattttcggtccggtgctggtggtcacgcgtttcacatcagaagaacaggcgctacagcttgccaacgacagccagtacggccttggcgcggcggtatggacgcgcgacctctcccgcgcgcaccgcatgagccgacgcctgaaagccggttccgtcttcgtcaataactacaacgacggcgatatgaccgtgccgtttggcggctataagcagagcggcaacggtcgcgacaaatccctgcatgcccttgaaaaattcactgaactgaaaaccatctggataagcctggaggcctgaaatgaccgaacataccagcagttactacgccgccagtgcgaataaatatgcaccattcgacacgctgaatgagtcaatcacctgcgacgtttgcgtggttggcggcggctataccgggctctcctccgcgctgcatctggcggaagcgggctttgacgtagtggttctcgaagcctcacgcatcggctttggcgcaagcgggcgcaatggcggacagcttgtgaactcctacagccgcgacatcgacgtgatcgaaaaaagctacggcatggacaccgcccgtatgctcggcagcatgatgttcgaaggtggtgagatcatccgcgaacgtatcaaacgttatcagattgactgcgactaccgccccggcggcctgtttgtggcgatgaatgataaacagctcgccacacttgaagagcagaaagagaactgggaacgctacggcaataaacagctggaattgctggacgccaacgccattcgccgtgaagtagccagcgatcgctataccggtgcgctgctggatcacagcggtgggcatattcatccgctaaaccttgccattggcgaagcggacgccatccgcctcaacggcgggcgcgtgtatgaactttctgccgtgacgcagatccagcacaccacgccagccgttgtgcgaactgccaaaggtcaggtgacggcgaagtatgtgattgtcgccgggaatgcgtatctgggcgataaagtagagccggaactggcgaaacgcagcatgccgtgcggcacgcaggtgatcaccaccgaacggctgtcggaagatttagcccgttcgctgatcccgaaaaactactgtgtggaagactgtaactatctgcttgattactaccgtcttaccgccgacaaccgcctgctgtacggcggcggcgtggtctacggcgcgcgcgacccggatgacgttgagcgccttgtggtgccgaaactgctgaaaaccttcccgcagctgaagggcgtgaaaattgattaccgctggacgggcaacttcctgctgaccctgtcgcgtatgccgcagtttggtcgcctcgataccaacatctattacatgcagggctacagcggccacggcgtgacctgtactcatctagccggacgtttgattgccgaactgctgcgcggcgacgccgaacgtttcgatgccttcgccaatctgccgcattacccgttccccggcgggcgcacgctgcgtgtgccgtttaccgcgatgggcgcggcgtattacagcctgcgcgatcgtctgggcgtttaatttccgattaaccgtgaagagtcaaaaggtgtgaaacatgagcaacaatgaattccatcagcgtcgtctttctgccactccgcgcggggttggcgtgatgtgtaacttcttcgcccagtcggctgaaaacgccacgctgaaggatgttgagggcaacgagtacatcgatttcgccgcaggcattgcggtgctgaataccggacatcgccaccctgatctggtcgcggcggtggagcagcaactgcaacagtttacccacaccgcgtatcagattgtgccgtatgaaagctacgtcaccctggcggagaaaatcaacgcccttgccccggtgagcgggcaggccaaaaccgcgttcttcaccaccggtgcggaagcggtggaaaacgcggtgaaaattgctcgcgcccataccggacgccctggcgtgattgcgtttagcggcggctttcacggtcgtacgtatatgaccatggcgctgaccggaaaagttgcgccgtacaaaatcggcttcggcccgttccctggttcggtgtatcacgtaccttatccgtcagatttacacggcatttcaacacaggactccctcgacgccatcgaacgcttgtttaaatcagacatcgaagcgaagcaggtggcggcgattattttcgaaccggtgcagggcgagggcggtttcaacgttgcgccaaaagagctggttgccgctattcgccgcctgtgcgacgagcacggtattgtgatgattgctgatgaagtgcaaagcggctttgcgcgtaccggtaagctgtttgccatggatcattacgccgataagccggatttaatgacgatggcgaaaagcctcgcgggcgggatgccgctttcgggcgtggtcggtaacgcgaatattatggacgcacccgcgccgggcgggcttggcggcacctacgccggtaacccgctggcggtggctgccgcgcacgcggtgctcaacattatcgacaaagaatcactctgcgaacgcgcgaatcaactgggccagcgtctcaaaaacacgttgattgatgccaaagaaagcgttccggccattgctgcggtacgcggcctggggtcgatgattgcggtagagtttaacgatccgcaaacgggcgagccgtcagcggcgattgcacagaaaatccagcaacgcgcgctggcgcaggggctgctcctgctgacctgtggcgcatacggcaacgtgattcgcttcctgtatccgctgaccatcccggatgcgcaattcgatgcggcaatgaaaattttgcaggatgcgctgagcgattaatagcccaacgcaataatgtctgatgcgctgcgcttatcaggcctgcaaacgacgtattgattatgtatgccgaataaagcattcacgccgcatccggcaagttgtattgctcaacttcgctaaatctggtgctttttcaacaacgcgcggaactgatgataagttaaccccagtaattcagccgcgcgcttctggttatatttcccttgttgcaaactgagttgcagcaactctttttcctgctgcatctgaaactcacgtaaatccagcggcagtgttggaagcgaggtggtttctgaaacggcgatagcgtcttcaggcggacgccgtttaaagggatcaataatgatgtcatcaagcggataatcgctggtgccgtggcgatacactgaacgttccaccacgtttttcaattcacgaatatttcccggccaacgataattcagcaatgtttctctggcgcgctccgtaaaccccgggaacagaggcagcttgatttcccgacacatctggatggcaaagtattctgccatcaacattatgtcgctttcgcgctcgcgcagtggtggcagttgtacaacatcaaaagccagtcggtcgagcaggtcagcgcgaaaagtgccttcattgaccatcgccgggagatcggcattcgtcgcgcataccaaccgcacattcacctgcaatggttggctgccgccaacgcgctccagttcaccgtactcaatcacgcgcaataatttctcctgcaccatcatcggtgccgtagcgagttcatcaagaaatagcgtaccgccgtcggcacgttcaaatctccctggatgacgtttttgcgcaccggtaaacgcccccgcttcgtgaccaaacagttcggaatccagcagattttcatttaacgccgcgcagttaagggaaataaacggcccttgccaacgggaggagagataatgcaggcggctggcaatcagctctttaccggtgccgcgttcgccgatgatgagcaccggtttgtccagcggtgcgagatgcgaaacctgttccagcacttcgagaaagctgttcgcctcaccaagtaaattatctttgtattctgccatgatgaaattcgccacttgttagtgtaattcgctaactcatcctggcatgttgctgttgattcttcaatcagatctttataaatcaaaaagataaaaaattggcacgcaaattgtattaacagttcagcaggacaatcctgaacgcagaaatcaagaggacaacattatgggtattttttctcgctttgccgacatcgtgaatgccaacatcaacgctctgttagagaaagcggaagatccacagaaactggttcgtctgatgatccaggagatggaagatacactggttgaagtacgttctacttcggcgcgcgcgttggcagaaaagaaacagctgactcgccgtattgaacaagcgtcggcgcgtgaggttgaatggcaggaaaaagccgaactggcgctgctgaaagagagagaggatctggcacgtgcagcgttaattgaaaaacagaaactgaccgatctgattaagtccctggaacatgaagtgacgctggtggacgatacgctggcacgcatgaagaaagagattggcgagctggaaaacaaattgagcgaaacacgcgctcgccagcaggcattgatgttacgtcatcaggcggcaaactcgtcgcgcgatgtgcgtcgtcagctggacagtggcaaactggatgaagcaatggctcgtttcgaatctttcgaacgtcgtattgaccagatggaagcggaagcagaaagccacagcttcggtaaacaaaaatcgctggacgatcagtttgccgaactgaaagccgatgatgcaatcagcgaacaactggcacaattaaaagccaaaatgaagcaagacaatcaataataacatccaggcggcgtccgaacgcgccgccgctcatcgtctaaggagtacttatgagcgcgctatttctggctattccgttaaccatttttgtgctgtttgttttaccgatctggttatggctgcattacagcaatcgttctggtcgcagtgaattgtcgcaaagtgagcagcagcgattagcgcaactggctgatgaagcaaaacggatgcgcgaacgtattcaggcgctggaatctattcttgatgcagaacatccgaactggagggatcgctaatggcgggcattaatctcaataaaaaattatggcgtattccacagcagggcatggtccgcggcgtctgcgccgggattgccaactattttgatgtaccggtaaaactggtgcgtatcctggtggtgctgtcgattttcttcggtctggcgctgtttaccctggttgcttacatcattttgtcatttgcgcttgatccaatgccggacaacatggcctttggtgagcagctaccttccagcagcgaattgctggatgaagtcgaccgtgaactggcggcaagtgaaacgcgtttacgcgagatggaacgttatgtcacttccgatactttcacgttacgtagccgtttccgtcaactgtgaggaaagttatgaatactcgctggcaacaggccgggcaaaaggtaaagcctggtttcaaattagcaggcaagctggtacttcttaccgcactgcgctatggcccggcgggtgtggcgggctgggcgataaaatcagttgctcgccgaccgctgaaaatgttgctggctgtggcgctggaaccgctgttaagtcgggctgctaataaactggcacagcgttataaaaggtgaggggagtttcgcaaaaattgttaaatctcaggcgtataatggatggcaattttcatccatagaaggacgcttacatgtttaaaaaaggcttacttgctctggcactggtgttttcactgcccgttttcgccgctgaacactggatcgatgttcgtgttccagagcagtatcagcaagagcacgttcagggggccatcaatattcccctgaaggaagtgaaagagcgcattgccaccgccgttccggataaaaacgacaccgtgaaagtgtattgcaatgccggacgccagtcagggcaagcaaaagagatccttagcgagatgggatatacccacgttgagaacgccggtggcctgaaagacatcgcaatgccgaaggtcaaaggttaaaagaattcaccatgagcggcgcttatgcgccgtttttttttctgtcacaccttatttacatccccatagattatttgcgtcagctcacaaatacgctttttccctggtaaaaaatgatttcctgcgtgactaaaacccttgtgctcaattgacagtttattttctgcggagtagtctctcgtttcatgggaccgctaccacggaaaggcaacatgaaacagaaaattacggattacctggacgaaatctacggtggaacatttaccgcaactcatttacagaaacttgtaacgcgtcttgagagtgcgaaacgattaattacacagcgacgtaaaaaacactgggatgaaagtgatgtcgtgttaattacctatgccgatcaatttcacagcaatgatttaaaaccattacccacatttaatcagttttaccatcaatggctgcaaagcattttttcacatgttcatttgttgccgttttatccatggtcatctgatgatggcttttcggtaattgattatcatcaggtcgccagtgaagcgggggagtggcaggatattcagcaactcggtgaatgcagtcatttaatgtttgattttgtctgcaaccatatgtcggcaaaaagtgaatggtttaaaaactatttacaacagcatccaggttttgaagatttttttattgccgttgacccgcaaaccgatctcagcgccgtcactcgcccgcgtgcgttaccgttattaacgccattccagatgcgcgatcattcaacgcgccatttatggaccacctttagtgacgatcaaattgacctgaattaccgtagccctgaagtgttgctggcgatggtggatgttttactctgttaccttgcgaaaggtgctgagtatgtccgcctggatgccgttggctttatgtggaaagagccgggaacaagctgcatccatctggaaaaaacacatctgattatcaaactgttacggtcgattattgataacgttgcgccaggtacagtgatcattaccgagaccaatgttccgcataaagacaacattgcttactttggcgcaggcgatgacgaagcacatatggtgtaccagttctcgctgccgccactggtgctgcatgcggtgcaaaaacagaacgttgaggcgctttgtgcgtgggcgcaaaacctgacactaccttccagcaacaccacctggtttaacttcctcgcctctcacgatggcatcgggctaaacccgctacggggcttgttgcctgaaagcgaaatattagagctggtcgaggcgttacagcaggaaggtgcattagtaaactggaaaaataatcccgacggtacacgcagtccgtatgaaataaatgtgacctatatggatgcgttaagccgccgtgagagtagcgatgaagaacgttgcgccaggtttatccttgcccatgcgattttgttaagtttccccggtgtgccagcgatatatattcaaagtattcttggctcgcgtaatgattacgcaggtgtcgaaaaactcggatataaccgtgcgattaaccgtaaaaaatatcacagtaaagagataacccgagaactgaacgatgaagctacattaaggcatgcggtatatcatgagttgtcgcgtttaattacacttcgtcgcagccataacgagtttcatccggataataattttaccattgatacgattaattcatccgtaatgcgtattccaagaagtaacgctgatggtaattgtctgactggattgtttaatgtcagtaaaaatattcagcatgtaaatattactaatctgcatggtcgggatctgattagtgaagttgatatattgggtaatgaaataacgctgcgcccctggcaggttatgtggattaaataaaaaggaacatctcatgattaaatcaaaaatcgtgctgttatcagcactggtttcatgcgccctgatttcaggctgtaaagaagaaaataaaacgaatgtatccatcgaatttatgcattcttcggtggagcaggagcgccaggccgttatcagtaaattgattgcccgttttgaaaaagaaaaccctggcatcaccgttaagcaagtgcccgtggaagaagatgcctataacactaaagtcattactctttcacgtagcggttcgctgccggaagtgatcgaaaccagccatgactacgccaaagtgatggacaaagagcagcttatcgatcgcaaagcggttgccacagtcatcagcaacgttggtgaaggcgcgttttacgatggcgtactgcgtattgtgcgtaccgaagatggtagcgcatggaccggtgttcctgtcagcgcctggattggcggtatctggtatcgcaaagatgtgctggcaaaagcggggcttgaggagccgaaaaactggcaacagctgctggacgttgcacagaaactgaatgacccggcgaataaaaaatacggcattgcgctgcctacagcagaaagcgtgttgacggaacaatccttctcccagtttgcgttatccaaccaggctaacgtctttaacgccgaaggcaaaatcacccttgatacaccagagatgatgcaggcactgacctattaccgcgaccttactgccaacactatgccgggttctaacgacatcatggaagtgaaagacgcctttatgaacggcaccgcgccgatggcgatttactccacctatatccttccggctgtgattaaagaaggcgacccgaaaaacgtcggtttcgtggtgccaaccgagaaaaactctgcggtctacggcatgttgacctcgctgaccattaccgccgggcaaaagaccgaagagacggaagcagcagaaaaatttgtcacctttatggagcaggcagacaacattgccgactgggtgatgatgtcgccaggtgctgcgctgccggtgaataaagcggtggtgactaccgccacctggaaagacaacgacgttattaaggcgctgggtgaactaccgaatcagctaatcggtgaactgccaaatattcaggtttttggcgcagtaggggataaaaactttacccgcatgggtgatgtgacgggttctggcgtggtgagttcaatggtgcataacgtcaccgtgggtaaagccgatctctctactacgctgcaagcgagccagaaaaaactggatgaactgatcgaacagcactaaacccaggacaggaatccgcaatgaacaggcttttttcaggtcgttccgatatgccctttgcgctgctgcttctcgcgcccagcttattactgctgggcggtctggtggcgtggccgatggtgtcgaatatcgaaatcagttttttacgtctgccgctcaatcccaacatcgagtcaacgtttgttggggtgagcaactatgtgcgtatcctctccgatcccggcttctggcattcgctgtggatgacggtctggtataccgcgctggtggtggcgggcagcaccgtgctcgggctggcggtggcgatgtttttcaaccgcgagttccgcctgcgcaaaaccgcgcgttcgctggtgatcctctcctacgtaacgccgtccatttcgctggtgttcgcctggaaatacatgttcaacaacggctacggcattgttaactacctcggcgtcgatcttctgcatctctatgagcaggcaccgctgtggttcgataatccgggcagtagctttgtgctggtggtgctgttcgccatctggcgctacttcccgtatgcctttatctcgtttctggcgattttgcagaccatcgacaaatcgctgtacgaagcggcagagatggatggcgctaatgcctggcaacggtttcgtatcgtcacgctgcccgcaattatgccggtcctggcgacggtggtgacactgcgcaccatctggatgttctacatgttcgcggatgtttatttgctgacgaccaaggtcgatattctcggtgtatatctctacaaaaccgcctttgcctttaatgatttaggaaaagcggcggcgatctcggtggtgctcttcatcattattttcgctgtcattctgctgaccaggaaacgggtgaacctcaatggcaacaaataaacgcacactcagtcgcatcggtttttactgcgggctggcgctgtttctcatcatcacgctgtttccattttttgtgatgctgatgacctcgttcaagggcgcgaaagaggcgatctcactgcatcctacgctgctgccgcagcagtggacgctggagcattacgtcgacatttttaacccgatgattttcccgtttgtcgactacttccgtaacagtctggtggtgtctgtggtttcatccgtggtggcggtattcctcggcattcttggggcttacgcgctttcccgcctgcgctttaaaggtcggatgaccatcaacgccagcttttacacggtgtatatgttctctggcattttgctggtggtgccgcttttcaaaatcatcaccgcgcttggcatttacgacactgagatggcgctgatcatcaccatggtgacgcaaactctgcccaccgccgtgtttatgctgaaaagctacttcgacaccatccccgatgagatcgaagaagcggcgatgatggatggcctcaaccgtctgcaaattatcttccgcatcaccgtgccgttggcgatgtccgggctgatatccgtgttcgtctactgctttatggtggcgtggaacgactatctgtttgcgtcgattttcctctccagcgccagcaatttcaccttaccggtgggcctgaacgcgctgttcagtacgccagattacatctggggacggatgatggcggcctcactggtgaccgcattgccggtggtgattatgtatgcgctttcggaacgttttattaagagtggtttgaccgccggtggcgtgaagggctaaagcggccagtttctttacaaggagttttaaatgaaaaagttagtagccacagcaccgcgtgttgctgcgctggttgagtatgaagatcgggcgattttagctaatgaagtgaagatccgcgtgcgtttcggcgcaccgaaacacggaacggaagtggtcgacttccgcgccgccagcccgtttattgatgaagactttaacggcgaatggcagatgttcactccgcgtccggcagatgcgccgcgcggcattgagtttggcaaattccagcttggcaacatggtggttggcgacattatcgagtgcggcagcgacgttaccgactacgcggtgggcgacagcgtatgcggctacggcccgctctccgagacggtcatcattaacgcagtgaataactacaagctgcgcaaaatgccgcaaggcagctcctggaaaaacgccgtctgctacgacccggcgcagtttgccatgagcggcgtgcgcgatgccaacgtgcgcgtaggggattttgtggtggtggtagggcttggcgcaatcggtcaaattgccatccaactggctaaacgcgctggcgcttctgtggtgattggcgtcgatcctatcgcccatcgctgtgatattgcccgtcgccacggcgcggatttctgccttaaccccatcggcactgatgtaggtaaagagatcaaaacgctgaccggcaagcagggtgccgatgtgattatcgaaaccagcggctacgccgacgcgctgcaatcggcgctccgcggtctggcttatggcggcaccatctcctatgtcgcgtttgccaagccgtttgccgaaggttttaacctcggacgcgaagcgcatttcaataacgccaaaattgtcttctctcgcgcgtgcagcgaaccgaacccggattatccgcgctggagccgcaagcgtattgaagaaacctgttgggaactgctgatgaacggttatctcaattgcgaagatttaatcgacccggtggtgacctttgccaatagcccggaaagctatatgcagtatgtcgaccagcatccggaacagagcatcaaaatgggcgttacgttttaattcaaaggaatgaaaaaaatgaaaatcggcacacagaatcaggcgttctttccggaaaacattctggagaaatttcgttatatcaaagagatgggcttcgatggttttgagattgacggcaaactgctggttaacaacatcgaagaagtcaaagcggcgatcaaagaaaccggtttaccggtgaccaccgcctgcggtggctatgacggatggattggcgactttatcgaagagcgtcgtcttaatggcttaaagcagatcgagcgcattctcgaagcgctggcagaagtgggcggtaaaggcatcgtcgttccggctgcgtggggcatgtttaccttccgcttaccgccgatgacctcgccgcgtagcctggacggcgaccgcaaaatggtgagtgattccctgcgcgtactggaacaggtcgccgcgcgtaccggaaccgtggtgtatctcgaaccgttaaaccgctatcaggatcatatgatcaacaccctcgccgatgcccgccgttacatcgtcgaaaacgatcttaaacatgtacagattatcggcgatttctatcacatgaatatcgaagaagataacctggcgcaggcgctgcatgacaaccgcgacctgctcggtcatgtgcatattgcggataaccatcgctaccagccgggcagcggcaccctggatttccacgcgctgtttgaacagctgcgcgcggataactatcagggctatgtagtgtacgaagggcgtatccgggcggaagatcctgcccaggcgtaccgtgattcgttggcctggttgcgtacctgctaagaggtctttgtgaaaagtgcaatgacaagctctccgctgcgggtcgcgataataggcgcaggccaggtggcggataaggttcatgcttcgtactactgcacccgcaacgatctggaactggtggctgtctgtgacagccgcctttcccaggcgcaggcgctggcagaaaaatacgggaatgcatccgtgtgggacgatccgcaggccatgctgctggcggtgaaacctgatgtggttagcgtctgctcacctaaccgttttcattacgaacataccctgatggcactggaagcgggctgccatgtgatgtgcgaaaaaccgcccgccatgacgccagaacaggcgcgggaaatgtgcgataccgcgcgcaaactgggcaaggtgctggcctacgactttcaccatcgttttgcgctcgatacgcaacagctgcgtgaacaggtgaccaacggcgttttgggagagatttacgttaccaccgcccgcgccctgcgtcgctgcggcgttcccggctggggtgtctttaccaataaagaactgcagggtggtggcccgctgatcgacatcggcattcatatgctggatgctgcgatgtatgtgctgggctttccggcggtgaaaagcgtgaatgcgcatagctttcaaaagatcggcacgcaaaagagctgtggtcaatttggtgagtgggatccggcaacttacagcgtcgaagattcgctgtttggcaccattgaatttcataacggcggcattctgtggctggaaacgtcatttgcactcaacatccgcgaacagtcgattatgaacgtcagcttttgtggtgataaagctggtgcgacgctgtttccagcacatatctacaccgataacaacggtgaattaatgacgctgatgcaacgggaaatagcagacgacaaccgccatttgcgcagcatggaagcctttatcaatcacgtacagggcaagcccgtgatgatagccgacgccgagcaggggtacatcatccagcaactggtggcggcgttgtatcaatccgcagaaacagggacgcgtgtggaattatgaccaggccagtaacgttatcagaaccccatttcagccagcataccctgaacaagtatgcatcgctgatggcgcaggggaacggctatcttgggcttcgcgccagccatgaagaagattacacgcgccagacgcgagggatgtatctggcggggctgtatcatcgggcgggaaaaggtgaaatcaacgaactggtgaacctgcctgatgtcgtggggatggagattgccataaatggtgaggttttctcgttatcccacgaagcctggcagcgtgagcttgactttgccagtggcgaattacgccgcaatgttgtctggcgtaccagcaacggctcaggttacaccatcgccagccgtcgctttgtttcggcagaccaactgccgctcattgcgctggaaatcactattacgccactggacgccgacgcgtcagtgctgatttcaacaggcattgacgccacgcaaaccaatcacggtcgccaacatctcgacgaaacccaggtgcgggtgtttggtcagcatctgatgcaggggagctacaccacccaggatggacgcagtgatgtggccatcagctgttgctgtaaggtgagcggtgatgtgcagcaatgctataccgccaaagagcgccgtttactgcaacataccagtgcgcagcttcatgcaggcgagacaatgacgttgcaaaaactggtgtggatcgactggcgggatgacaggcaagctgctttagacgagtggggcagcgcgtcgcttcgccagcttgaaatgtgcgcgcagcagagttacgaccaacttcttgcagcatcaacagaaaactggcgtcaatggtggcagaaacgtcgtatcacggtaaatggcggcgaagcgcacgatcagcaagcgttagattatgcgctttatcatctgcgcatcatgacgcctgcccacgacgagcgcagcagcattgcggcaaaaggcttaaccggcgaaggctacaaaggccacgttttctgggatacagaagtatttttgttaccgtttcatctgtttagcgatccgacggttgcccgaagtttactgcgttatcgctggcacaacttgccaggcgcgcaggagaaagcgcgacgcaacggctggcagggcgcgctatttccgtgggaaagcgcgcgcagcggcgaagaagagacgccggaatttgccgccattaacattcgcaccgggctgcggcaaaaagtggcctcggcgcaggcggaacatcatctggtggccgatatcgcctgggcggttattcaatactggcagaccacgggggatgaaagtttcattgcgcatgaaggcatggcgctacttctggagacggcaaagttctggattagccgcgcggtgagagttaacgatcgtctggaaattcatgatgttattgggccagacgaatataccgaacatgtcaataataatgcatacaccagctatatggcccgctacaacgttcaacaggcgctgaatattgcccgccagttcggctgtagcgacgatgcgtttatccatcgcgccgaaatgttcctcaaagagctatggatgccagaaattcagcccgacggcgttttgccgcaggatgattcgtttatggctaagccggcgattaatctggcgaaatacaaagcggcggcggggaagcaaaccatactgctggattattcacgcgcagaagtgaacgagatgcagatcctcaaacaagctgatgtggtgatgctcaattacatgctgccggagcagttctcagcggcatcgtgtcttgccaatctgcaattttatgaaccgcgcactattcacgactcgtcattaagtaaagcaatccacggcattgttgccgcacgctgtggcctgctgacccaaagttatcagttctggcgcgaggggactgaaatcgatcttggtgctgatccgcatagttgtgatgatggtatccatgctgccgcaactggcgctatctggctgggggcgattcagggttttgccggggtgagcgtgcgtgacggtgaattgcatctcaatccggcgttacctgagcagtggcaacagttgtctttccctctgttctggcagggctgcgaattacaggtcactcttgacgcgcagcgtattgcgattcgaacttctgcgcccgtttcactgcgtttgaacggtcagcttataaccgtggctgaagaatctgttttctgtttgggtgattttattttgcccttcaatgggaccgctaccaaacatcaggaggatgaatgaaactgcaaggggtaattttcgatctggatggtgtaatcaccgataccgcgcatctgcatttccaggcgtggcagcagattgccgctgaaattggcatcagcattgatgcgcagtttaacgaatccctaaaagggatcagccgcgatgagtctctgcggcgcattctgcaacacgggggcaaagagggcgactttaactcgcaggagagggcgcaactggcgtatcgcaaaaatctgctctatgtccactcactacgcgagttgacggtcaacgctgttctacccggcattcgctctttgctggcagatctccgtgcacagcagatctcggttgggctggcttctgtctccctgaatgcgccgacgattttagcggcgctggagctgcgcgagtttttcaccttctgcgcggatgcttcccaacttaaaaactcgaaaccggacccggaaatctttctcgccgcctgtgcagggctgggcgtgccgccgcaggcatgtatcggcattgaagatgcgcaggcgggcattgacgccattaacgccagcggtatgcgctcggtggggatcggcgcgggcttaaccggggcgcaattactgttgccttcaacggaatcactcacctggccgcggttatcggccttctggcaaaacgtatagcaaaggaatcaacatggctcagctttcgttacaacatattcaaaaaatctacgataaccaggtgcatgtggtgaaggacttcaacctggaaattgccgataaagagttcatcgtgtttgtcggcccgtcgggctgcggtaagtcgaccaccctgcgcatgattgccgggcttgaggagatcagcggcggcgatctgttgatcgacggcaaacgaatgaatgacgttccagccaaagcacgcaatatagcgatggtgttccagaactacgcgttgtatccgcatatgacggtttacgacaacatggcgtttggtctgaagatgcaaaaaatcgccaaagaggtgattgatgagcgggtgaactgggcggcgcaaattctcggcctgcgtgagtacctgaaacgtaagccgggggcgctttccggcgggcaacgtcagcgagtggcgcttgggcgggcgattgtacgcgaagcgggcgtgtttttaatggatgaaccgctctctaaccttgatgccaagctgcgcgtgcaaatgcgcgcagagatcagcaagctgcatcagaaactgaacaccaccatgatctacgtgacccacgatcagaccgaagcgatgaccatggcgacgcggattgtgattatgaaagacgggattgttcagcaagtaggtgcgccgaaaaccgtttataaccaacccgcgaatatgtttgtttccggatttattggatcaccagcgatgaattttattcgcggcacgatcgatggcgataaattcgttacggaaacgcttaaattaaccattcccgaagagaaattagcggttctgaaaacacaggaaagtttgcataagcccatcgtgatgggaatacgaccggaagatattcatccggacgcgcaagaggaaaataacatttccgccaaaattagcgtggcagaattaaccggtgcggaatttatgctctacaccacggttgggggcacgagttagtggtccgtgctggtgcgttaaatgattatcatgcaggagaaaatatcactattcattttgatatgacgaaatgtcatttctttgatgcagaaacggaaatagcaattcgctaaatacagggggaaggcattcccccaggataatacaaggaacaataatgaaaaagttattaccctgtaccgcactggtgatgtgtgcgggaatggcctgcgcacaggccgaggaaaggaacgactggcactttaatatcggcgcgatgtacgaaatagaaaacgtcgagggttatggcgaagatatggatgggctggcggagccttcagtctattttaatgccgccaacgggccgtggagaattgctctggcctattatcaggaagggccggtagattatagcgcgggtaaacgtggaacgtggtttgatcgcccggagctggaggtgcattatcagttcctcgaaaacgatgatttcagtttcggcctgaccggcggtttccgtaattatggttatcactacgttgatgaaccgggtaaagacacggcgaatatgcagcgctggaaaatcgcgccagactgggatgtgaaactgactgacgatttacgtttcaacggttggttgtcgatgtataaatttgccaacgatctgaacactaccggttacgctgatacccgtgtcgaaacggaaacaggtctgcaatataccttcaacgaaacggttgccttgcgagtgaactattatctcgagcgcggcttcaatatggacgacagccgcaataacggtgagttttccacgcaagaaattcgcgcctatttgccgctgacgctcggcaaccactcggtgacgccgtatacgcgcattgggctggatcgctggagtaactgggactggcaggatgatattgaacgtgaaggccatgattttaaccgtgtaggtttattttacggttatgatttccagaacggactttccgtttcgctggaatacgcgtttgagtggcaggatcacgacgaaggcgacagtgataaattccattatgcaggtgtcggcgtaaattactcgttctgataatgggctaaattgccggatgcggcgcgagtactttatccgatctataaatgtaggccggataagatgcgctagcatcgcatctggcattcaggcaaggtagctggtatttatttcagcgtcatatgcgtggcaacggtaatattctgtggtgacggttttccagaaattaagcggaataataactcgcagctttgttgacctaactcctgcgtcggaacatcgatgccgcccggtgcaggcgttaaaataaatgacagcgtttcattgctataacccaccaccgctaactgctgcggaatagcaatatttttctctgctgccgcacgataaatgctcattaatttcaggctgtcagtggcaaacaccgcctcaggcaacggtgactggcttaataattgccgtgctgcttttaatgcagtttcatgggtataaccgccatcaacaatccattcatcacgcactgcaatattatgcgcagccaggctctgcttataaccattaacgcgatcaaccgaaacatggacatcaagcggagcatgcaggcaggcaatattttgatgcccactttcaattaatgcatcggtcaacgcaatgctgtcgccaaaattatcggtatcgacagaataaacatgggcatattgaccttcaactttgccaatcaccaccaccggaatatcatatttatcgagttgggcaaaaaatgactcatccgctggcgaactgagcataataatgcctttaatcattttctgcttaattttgctttcgcatttttgcagatcttctgccggattgtgcgacgtttgtaatatcacgtcgaaaccttcttcttcagctttggcggtgatggcatgcaaaacttcagagaaaaacggattacccgccgtagttttggtcgaacgggtagaaatcaccataatggcatcaaaacccgaagaggtcagcgcgcgggccagcttgtttggctgatactgtaattcttcaatggcccgtaacactttttcgcgcgcttccggggagatattagtttgcttattcagcacgcgtgatacggtggattttgatacgcctgcaaccctggcaatatcataaatagtaggggacataggtcaggaactccgtccgaacgtgaatgctgcacatcttatggagttcgccggtcgatgacaacacgggcagttgataatcaatggcctggcccccacattcatatccttacgaatgattttttttctggtcttcagagcagcacaggacagcaatgaagcgacttaaaaatgaactcaatgcgctggtgaatcggggtgtcgacagacatctgcgcctcgctgtaaccggacttagccgcagcggcaaaacagcgtttatcaccgcgatggttaatcagttgcttaatattcacgccggagcacgtttgccgctgttaagtgcggtgcgtgaagagcgcctgctgggcgtgaaacgcattccccagcgtgactttggcattccgcgcttcacctatgacgaagggctggcgcagttatatggcgatccacccgcctggccaacgccaacgcgcggcgtcagtgaaatccgcctggcgctacgttttaaatcgaatgattcgctgctacgccactttaaggatacctccacgctgtatctggaaattgtggattatcccggcgaatggttgctcgacctgccgatgctggcgcaggactatttaagctggtcgcgccagatgacgggcttactcaatggtcagcgcggagaatggtcggcgaaatggcgaatgatgagcgaagggctggacccgctagcgcctgccgacgaaaaccggctggcggacattgccgccgcgtggaccgattatctccaccactgtaaagagcaggggctgcactttattcagcctgggcgctttgtcttgccgggagatatggcaggtgcgcccgcgctgcaattcttcccgtggccggatgtcgatacctggggcgagtccaaactggcgcaggccgataagcataccaatgccggaatgctgcgcgagcgctttaattattactgcgagaaggtggtgaaggggttctataagaatcattttctgcgctttgaccgccagattgtgctggtggattgcctgcaacctctcaacagtgggccacaggcatttaatgatatgcgtctggcactgacgcagctgatgcaaagttttcactacgggcagcgtaccctgttccggcgtttgttttcgccggttatcgataagctattgtttgctgccactaaagcggaccatgtgaccatcgatcagcacgctaatatggtttcattactgcaacaactgattcaggatgcctggcaaaatgcggcgttcgaagggatcagcatggactgcctggggctggcgtcagttcaggcgaccaccagcggcattattgatgttaacggtgagaaaatcccggcgctgcgtggtaatcgacttagcgatggcgcaccgctcactgtttatcctggcgaagttcccgcacgtttgcctggtcaggcgttctgggataagcaaggcttccagtttgaggcatttcgtccgcaggtgatggatgtcgacaaaccactaccgcatattcgtcttgatgctgcgctggaatttttaataggagataaattgcgatgaccgaaccgttaaaaccacgtattgatttcgacggtcctctggaggtcgatcagaatcctaaattcagggcgcagcagacctttgacgaaaatcaggcgcaaaattttgccccggccacgctcgacgaagcgcaggaagaagaggggcaagtcgaagcggtaatggacgcagcgttacgtccgaaacgcagcctgtggcgcaaaatggtgatgggagggctggctctgtttggcgcaagcgttgtcgggcagggtgtacagtggacaatgaatgcctggcaaacccaggactgggtggcgctgggtggatgtgccgctggggcattgattatcggcgctggcgtaggttctgtggtaacagagtggcggcgcttatggcgcttgcgacagcgcgcccatgaacgcgacgaagcgcgtgatttattgcatagccacggcacgggcaaaggccgcgcattttgcgaaaaactggcgcagcaggcgggtattgatcagtcgcatccggcgctgcaacgctggtatgcctcaatccatgaaacgcaaaacgaccgtgaagtggtcagcctgtatgcgcatttggtccagccagttttagatgcccaggcgcggcgcgaaatcagccgttcggcggcggaatcaacgttgatgattgcggtcagcccgctggcgttggtcgatatggcgtttatcgcctggcgcaatctgcgtttaattaatcgcatcgccacgctgtatggcattgaactggggtattacagccgtttgcgtctgtttaagctggtattgctgaatatcgcttttgccggagccagcgaactggtgcgcgaagtggggatggactggatgtcgcaagatctcgctgctcgtttgtctacccgcgcagctcaggggattggtgcaggacttctgacggcacgactcgggattaaagctatggagctttgccgcccgctgccgtggattgacgatgacaaacctcgcctcggggatttccgtcgtcagcttatcggtcaggtgaaagaaacgctgcaaaaaggcaaaacgcccagcgaaaaataatgcaatatcgggtgctgaccggatatctttacgccgaagtgcccgtttttccgtctttgtgtcaatgattgttgacagaaaccttcctgctatccaaatagtgtcatatcatcatattaattgttcttttttcaggtgaaggttcccatgcgtctggaagtcttttgtgaagaccgactcggtctgacccgcgaattactcgatctactcgtgctaagaggcattgatttacgcggtattgagattgatcccattgggcgaatctacctcaattttgctgaactggagtttgagagtttcagcagtctgatggccgaaatacgccgtattgcgggtgttaccgatgtgcgtactgtcccgtggatgccttccgaacgtgagcatctggcgttgagcgcgttactggaggcgttgcctgaacctgtgctctctgtcgatatgaaaagcaaagtggatatggcgaacccggcgagctgtcagctttttgggcaaaaattggatcgcctgcgcaaccataccgccgcacaattgattaacggctttaattttttacgttggctggaaagcgaaccgcaagattcgcataacgagcatgtcgttattaatgggcagaatttcctgatggagattacgcctgtttatcttcaggatgaaaatgatcaacacgtcctgaccggtgcggtggtgatgttgcgatcaacgattcgtatgggccgccagttgcaaaatgtcgccgcccaggacgtcagcgccttcagtcaaattgtcgccgtcagcccgaaaatgaagcatgttgtcgaacaggcgcagaaactggcgatgctaagcgcgccgctgctgattacgggtgacacaggtacaggtaaagatctctttgcctacgcctgccatcaggcaagccccagagcgggcaaaccttacctggcgctgaactgtgcgtctataccggaagatgcggtcgagagtgaactgtttggtcatgctccggaagggaagaaaggattctttgagcaggcgaacggtggttcggtgctgttggatgaaataggggaaatgtcaccacggatgcaggcgaaattactgcgtttccttaatgatggcactttccgtcgggttggcgaagaccatgaggtgcatgtcgatgtgcgggtgatttgcgctacgcagaagaatctggtcgaactggtgcaaaaaggcatgttccgtgaagatctctattatcgtctgaacgtgttgacgctcaatctgccgccgctacgtgactgtccgcaggacatcatgccgttaactgagctgttcgtcgcccgctttgccgacgagcagggcgtgccgcgtccgaaactggccgctgacctgaatactgtacttacgcgttatgcgtggccgggaaatgtgcggcagttaaagaacgctatctatcgcgcactgacacaactggacggttatgagctgcgtccacaggatattttgttgccggattatgacgccgcaacggtagccgtgggcgaagatgcgatggaaggttcgctggacgaaatcaccagccgttttgaacgctcggtattaacccagctttatcgcaattatcccagcacgcgcaaactggcaaaacgtctcggcgtttcacataccgcgattgccaataagttgcgggaatatggtctgagtcagaagaagaacgaagagtaagcgcgaatatgcctgatggtgcaacaccatcaggcatattaaattatgctttcagtacagccagagctgcttcgtaatccggctcggtggtgatttcatccaccagctggctgaaaatcacattgtcattttcgtcaataaccacaacggcacgcgctgccagacctttcagtgggccatcagcaattgccacaccgtaagcttgcagaaattcagcgttacggaaagtggagagggtgataacgttgttcagaccttctgcgccgcagaaacgagactgggcgaacggcagatcggcagagatacacagcacaacggtgttgtcgatctcagttgccagttggttaaacttacgtactgatgcggcgcaaacaccggtatcaatactcgggaaaatgttcagcactttgcgtttacccgcaaactgaccgagggtgacgtcagacagatcttttgccacgagagtaaaagtctgcgctttgctacccgcctgcgggatggaattggcgactgtaaccgggttgccctggaaatgaacggtttgtgacatgattatctttcctgtttacatatagttaacgtcacacctagtttatgctaactgtcaataacacagcaaacgctatttgcgcttaatccgcagaccaccgcgacaacaaggagtaaagatgagaaccgttaaggtattcgaggaagcctggcccttacataccccgtttgtgattgcccggggaagtcgcagtgaagcgcgcgtggtggtggttgaactggaagaagagggtattaaaggcaccggcgaatgcacgccgtatccgcgttatggggaaagtgatgcctcggtaatggcgcaaattatgagcgtcgtgccgcaactagagaaagggctgacacgggaggagttgcaaaaaattctccctgccggcgcagcacgtaatgcgctggattgtgcattgtgggatctggccgcgcgaagacagcagcaatcgctggctgatttgatcggcataacgcttcccgagacagttatcactgcacagacggttgtcatcggtacgcctgatcagatggccaatagtgcatcaacactctggcaggcaggcgcgaaattactgaaagtgaagctggataaccatcttatcagtgagcggatggtggcaattcgcacagctgtgcccgatgcgacgctgatcgttgatgcaaatgaatcctggcgtgcagaagggttggcggcgcgttgccagctattggcggatttaggcgttgcgatgcttgaacaaccgcttcctgcgcaggacgatgcggcgctggagaattttattcatccgttgccgatttgtgctgatgaaagttgtcatactcgtagcaatttgaaggcgctgaaagggcgctatgagatggttaatattaagctcgataaaaccgggggtctgacggaagcgctggcgctggcgactgaagcgcgtgcacaaggtttcagtctgatgctgggctgcatgttgtgtacctctcgtgccattagcgccgctttaccgctggtgccgcaggtcagtttcgccgatcttgacggaccgacctggctggcggtagatgtggaaccggcgcttcagttcacgacgggcgaattgcatctttaggatgccagcgcagcaagtttgccatcgcaaagagatatttttcgctggcttcgtcggaggagatgggcggaaactctgcggtgatgcaatgcaagttcagatctgcacaccaactgccgaaagagccaggcgtttcataaccgacgctggttaccagaggcaattcaaacgcctgagccagccattcgcctaattcgctgtgtctgggatcttcaatacaggccagtggatcgtggaatgagaccacccaggcaggttgaatgcggtgtataagctggcacagcgcctgggtttcaggttcggagccaggtttgtcacctgtcagtaatacgacatcgcgttcttcagcggcgctgttccagcgataaacggtttcaccttccttccagttcgccgccggaaagtttctgtttaaatccacaccattagcattggcccgtaaccccaactggcagccgtcaggattcacacacagcaccacatgatgacggcgcaaagaaggtgtcaacgtccgcagagcacaggagagcgtgacgaccgaagagttttcatcaccgtgagtgccagccagaatcaaaccactttcgcggctggctgcaggggcaggaaaccagattaacggcgcgcccaataatgaacgtccgtaatgttctgttccgggcggaaatgcgccgcgttcggcgcgtgggcgggttacggtcatgatcgtctctggttcaggaagtattacaggcagtgttgtgcaaattttgcggattatcaaatccttttcttcaacgctatgtcatcgatcttgtatcacttttttgccggaagttgtttgcattttattagttggatagggtttgtggatttttgctggctgacgggcaaataaagtttgtttaatggtttgcttatctgccagttgattaatcacatggcgggctatctgaccgccagcaccaagaatcagtacatttttcatgaaaattatcccagattattggcagcaatatgccagtccatatcactattgcggatttgaatatgtttcattacagagtttcctcaaagaacggagctaatactgaaattgcttcagccacataggctttgccgtcataaagatccatatggtttgcgccttcaacaatgtgatagcgtttatcctggcttgatgctcgatcgtacaggtcgtcactcatccatttgctccctgcctggctgcccgccacaatctgcgtcggctgagtcaggtacacttccgccatatggtaagcatcataggtaataatctggttaaggctgcgcaaagtagcgtaacccggtgctgttggatactgcgcgcgaggggtgtggtaatactcccaggcctgacgcagttcttcgttcggcgcatcggactccttcattggtgccagtggcataatggcgtattctccgctgctaatatcgctggttctggcgtttgaacccgcttcaacgtatggcagggcatcaatagatttcacattgttttcccaaccattacggaatatcgaaccaatattgaccgcactaacggtaccgatggccttgatgcggcgatcctgaattgcagcattggctgtatatcctgcaccggcacaaattcccatcgcaccaattcgggtattgtcgacataagaaagcgttgtcaggtaatcaatcacggcactgatgtcttcagtacgaatgtatgggttttctaactgacgcggctcgccgccactttcaccttgataagatgcgtcataagcaatagtgacaaatcccttttccgccagttttttggcataggttccggccgtttgttctttaacgcccccacctgggtgagataacacaattgcctgatactgacgggtttcatcaaattttggagggaaatagatcactgcagacaaagagatggttggattattgctgttagtgaagctgactttattattcatcattccgttcctcatggagttgtcggttcgttttaacggttggtgatatcactatagatattgatcattaagttgattagacccaaaatcatgattagacctatcatttaaatgattaatagattgcatggagatactgaatgaagcgtgaagaaatcgctgatctgatggcgtttgtcgtcgttgcagaggagcgtagcttcactcgtgcagcagcccgcctgagcatggcgcagtcagctttaagccagatagtgcgtcgtatagaagaacgattgggattgcggcttctgacgcgaaccacgcgcagcgttgttccaactgaagcgggcgagcatcttttgtctgttcttggccctatgttgcatgacatagattcagccatggcatccctgagcgatctgcagaaccgcccatccgggacaatacgtattactactgtagaacatgcagcaaaaacgatattgttaccagcaatgcgcacattcctgaaatcgcatcctgaaattgatattcagctcaccattgattatggtttgaccgatgtcgtttctgaacgttttgatgcaggcgtccgtctgggtggggagatggataaagatatgatcgccattcgaatcgggccagatataccaatggctattgttggctcaccggattatttttctcgccgaagtgttccaacgtcagtgtcacaattaatagatcatcaggcaattaatttgtatcttcccacatcgggtacagcaaatcgctggagattaatacgcggtggacgtgaagttcgtgttcgcatggaaggtcagcttttactgaatacgatagacctgatcattgatgctgcaattgatgggcatggattggcgtatctaccttatgatcaggttgagcgggctattaaagaaaaaaaactgatacgtgttttggataaattcacaccagatttacccggttatcacctgtactatccacaccgtcgacatgctggctcggcattctcattatttatagataggctgaagtataaaggtgctgtttagcactacttgctgatacattaatttaattcttctcttaacgtattctcagttcctttcaacgttttggtcattttttattcttcgtacaatggcgacagatgctgattatgataccgaaaacgggtttgaacgtgcgaagcccgaacgtagtgttcggagttctatgtgctttaccgcattttggagactattatttacactaaatctgatttgatatattgatacttaaaacatttgatgcttcctttgtcacttttttgatggaagttgtttgcatttctttaaggcgaaacaaataattacgcatcaattttaatgtcggttagagggaaacttatgaagcactctgtttcagtcacgtgttgtgcgctgttggtcagcagcatttctctttcgtatgctgcagaagttccgagcggcacagtactggcagagaagcaggagctggtgcgccacattaaagatgagcctgcgtcgctggatcccgctaaagccgtgggcctgccagagattcaggtcattcgcgatctgtttgaaggtctggtgaatcagaacgaaaaaggggagattgtccccggcgttgcgactcagtggaaaagtaatgacaaccgtatctggacttttaccctgcgcgataacgcaaaatgggcggatggcacaccggtaacggcgcaagattttgtctacagctggcaacgtctggtggacccaaaaacattgtcgccatttgcatggtttgccgcgctggcgggaatcaacaacgcacaggcgattattgatggtaaagctacgcctgaccagcttggcgtcaccgcagttgatgcccatactttgaaaattcagcttgataaaccgttgccgtggtttgtgaatttaaccgctaactttgccttcttcccggtgcaaaaagccaacgtagaaagcggtaaagagtggacgaaacccggaaatctgatcggcaatggcgcttatgttcttaaagagcgcgtagtcaatgaaaaactggtcgtggtaccgaatacccattattgggataacgccaaaacggtactgcaaaaagtgaccttcctgccaattaatcaggaatccgcagccactaagcgttacctcgcgggggatattgatatcaccgaatccttcccgaaaaatatgtatcagaagctgttgaaggatattccggggcaggtttatacgccgccgcagctcgggacctattattatgcgtttaacacgcaaaaagggccgacggcagatcagcgcgttcgtctggcattaagtatgacgatagatcgccgcctgatgaccgaaaaagtattagggacgggcgaaaagccagcgtggcattttacaccagatgttaccgcgggatttacgccggaaccttcgccgtttgaacaaatgagtcaggaagaactgaatgcgcaggcaaaaactttgttgagcgcagctggttatggtccgcaaaaaccgctgaagctgacgcttttgtataacacttcagaaaaccatcaaaaaattgcgattgctgtagcatcgatgtggaaaaagaaccttggcgtagatgttaaattgcaaaatcaggaatggaaaacctatatcgatagccgtaacaccggcaattttgatgttatccgcgcctcgtgggtgggggattataatgaaccctccactttcctgacattattaacgtcaacgcattcaggaaatatttcacgctttaacaatccggcatatgacaaagttctggcccaggcatcgacggaaaataccgttaaagcgcgtaatgccgattacaacgcggcagaaaaaatcctcatggagcaagcaccgattgcaccaatttatcaatataccaatggacgattaatcaagccgtggctgaaaggttatcccattaataatcctgaagatgtggcgtacagtcggactatgtatattgtgaagcattgatgtgatgggaactggcgttacccttgtgcataacgccagtgatgtctgatttagcgaccctgttccggcggtgtaatgttatccatatacagcgtctggctggggaaggcaaagtccgcgccgtgtgactgtacaatatcgataatcttcaaataaacgtcttgctgtgcagcaagccattcagcccataccgtggttttggtaaagcaataaaccataatattcaatgaagagtcagcaaactggttgaaataaaccagtaaggtttgtcgctggtcgatggccgggtgatttttcagcatctcacgtacagcttcgacaataacgcccacttttgccgcatcctcataacgtaaaccaatggtcgtggtaatgcggcggttggtcattcgtcctgggttttctacgctgatcgacgaaaacagcgagttcggtacgtacaatggacgattatcaaaggtcgtaattttggtaattcgccagccaatttccgctactgtaccttcgatatttctgtccggtgaacggatccagtcgccaatactgaaaggacggtcgaaatagagcataatcccggaaaagaagttactcagaatatctttaccggccataccgacagccagaccaccaataccaccaaaggtcagcaagccagaaaggctcatgccgaaatgttcgccataaagcagaacaagcaccacaataatggtgattttgatgatacgcgacataatccgcgcactggtgatatcgcgaccttttttaatctgctgtttttcaaactgattaatcagcagaaatagcttaatcgtcagaataaccgcaatcagggacgtacagataaaatcgataacgcctggggtgataaatttgagtttatagttttctataacataattaataatgctaccaacagcactgataattatggtgtagattaaaaattgcaccgcatggaataaaaatccttttcttttacgatttccacggcgaaaccaaaagctcatcagaatcaatgctgcgcagctaccgaaaataatgaccagattaagcgcattatttgtaaacagttcagcgatcattgttttatcaggctcctccagataattgtcgtcatgccggaaacccctggcggggctattttaccgcgacaattcattcagatcatcaatagtcagggaaggaagtagcaacattagctaaggaaggtgcgaacaagtccctgatatgagatcatgtttgtcatctggagccatagaacagggttcatcatgagtcatcaacttaccttcgccgacagtgaattcagcagtaagcgccgtcagaccagaaaagagattttcttgtcccgcatggagcagattctgccatggcaaaacatggtggaagtcatcgagccgttttaccccaaggctggtaatggccggcgaccttatccgctggaaaccatgctacgcattcactgcatgcagcattggtacaacctgagcgatggcgcgatggaagatgctctgtacgaaatcgcctccatgcgtctgtttgcccggttatccctggatagcgccttgccggaccgcaccaccatcatgaatttccgccacctgctggagcagcatcaactggcccgccaattgttcaagaccatcaatcgctggctggccgaagcaggcgtcatgatgactcaaggcaccttggtcgatgccaccatcattgaggcacccagctcgaccaagaacaaagagcagcaacgcgatccggagatgcatcagaccaagaaaggcaatcagtggcactttggcatgaaggcccacattggtgtcgatgccaagagtggcctgacccacagcctggtcaccaccgcggccaacgagcatgacctcaatcagctgggtaatctgctgcatggagaggagcaatttgtctcagccgatgccggctaccaaggggcgccacagcgcgaggagctggccgaggtggatgtggactggctgatcgccgagcgccccggcaaggtaagaaccttgaaacagcatccacgcaagaacaaaacggccatcaacatcgaatacatgaaagccagcatccgggccagggtggagcacccatttcgcatcatcaagcgacagttcggcttcgtgaaagccagatacaaggggttgctgaaaaacgataaccaactggcgatgttattcacgctggccaacctgtttcgggcggaccaaatgatacgtcagtgggagagatctcactaaaaactggggataacgccttaaatggcgaagaaacggtctaaataggctgattcaaggcatttacgggagaaaaaatcggctcaaacatgaagaaatgaaatgactgagtcagccgagaagaatttccccgcttattcgcaccttccctaactaatcaatgcgttgattgtaaatccagctaagaggtgaggttttcagagcagacaacggtgaaatgtcatggtattgttacgtttaggtaacaagaaatttgtctgcacaaggattacatcatgattatggcgaaactgaagtcagcgaaagggaagaaatttctctttggtttgttggcggttttcattattgcggcgtcggttgtgactcgcgcgaccatcggcggcgttatagaacagtacaatattccgctgtctgagtggacgacatcaatgtatgtgattcagtcatcgatgatttttgtttatagcctggtctttactgtgttgctggcaatcccgttgggaatttatttccttggcggcgaagagcagtaagtaaaaaataggcccgataactcgggccttgtcagttattgaagagtcgttaatcgtcttcttcgtcatccagttcaacgggtgtctgatactggtcaggtttaatgaccagcaggtcgcagcgaagatgatcaatcacctgttccgccgtgttgccgaggaatgctgctgaaataccggtgcgtcctaccgtgcccagaaccacaatccccgcctgtaagtgctccgccaaatcaggaatcacctcttctggcagacctttttctacgtgcgtcatgttttcattaatgccgaatttctgccgcagggctttcattgccagcaaatgttgcccacgaatggcatcgttataaacgctcgggtcaaattccggcagttcaatcgcgatattaattggcgttaccggataagcgccaaccagatgaacttcggtatggttgacttgttctgccagttcgatcgtctctttgaccagtttttcattgagcgcattatgatacggctcttcactggcgagattcaccgccaccagcgccttgcctccttccggccacggctggtctttcaccatccacaccgggcttgggcatttgcgtaacagatgccagtccgttggcgtaaaaatcaccgcttccagacggtcatgttggtgcgccatttttagcaccaaatcgtgtccgccgctgatcacttcctgaatgatggcttcgaaaggacggttatgccagaccactttaatttcaatgggaacgccagcattgagataatattttgcctgctcgtggatccaggctgtacgctggctgatgacgccctgacgcatagcggtacgttcgtccggggagagcagggtggtcatttcgtatgagaagtcatagatcggcaaaaaggctttaattttgccaccaatccgttgatgtaaataaacagctcgccgcaatgctggttggtcgtcctggttaggatcgataacaacgagcatgttctgatacatagccatacagggtctccttacaacaactgtcaacgcagtttgtaattaaaagattaacccatatctggtgaatgaaacagtgatgaaccttctgccagatcaataaatcagaaaaatttaatgatatgacagaaggatagtgagttatgcggaaaaatcaggcaacgttacgcgtatgaccagcaagctgggccagcgcatcgttattttcgatggtgatgtatttacctttgactgccagcatgccgcttttctggaagcgacccagcagacggctgatggtttctaccgtcaggcccagatagttaccgatatcgccacgagtcatcgtcaggcggaattcacgaggggagaagccgcgttgggcaaaacgacgggacaggttgtagatgaatgcagccagacgttcctcggcatttttcttcgacaacagcaggatcatgtcctgatcgcctttgatttcaccgctcatcagacgcatcatctgctgacgcagattcggcattttaccggacaaatcgtccagcgtttcgaacgggatttcacataccatcgaggtttccagcgcctgcgcgaagctcgggtgatggccgctgccgatggcgtcaaatcccaccaggtcgcctgctaaatggaaaccagtgatttgctcgtcgccttgctcagtgatggtataacttttaatcgtaccggagcggatggcataaagcgatttaagttcatcaccagccttaaacagcgtctggcctttctgaataggcttcttccgctcaatgatattatcaagctgatcaagctcatgttcgttgagtgtgaacgggatgcaaagctggctgatgctgcaatcctggcaatggatagcacaaccgccagactgaatgcgccgtataattcgcttttccgggatcataggtctgctcaagccgtaattgatatttgtcaattttaacatctttttagggagcaagtaagtctaagcaaaccttaacagcagagaattccgatattagatgtaaatatatgtctatctatttgaaaacccttaagttgttaagggtaactttacataaaagtgtgaacaagctggcacaaattgtttaatgtttacagcaaaagataaccttcatggcgcaataaccactcttttcgctgaactccgcctgcatatccggtcatggtgccgtttcggccaataacccgatggcaaggtacgacgatgctgatgggattcgatccgtttgccgcaccaacggcacgcgccgcgccaggacggcccaattgctcagccagttggccgtaatgcattacctgcccgcaggggatagtgcgtagtgttttccagacttcgcgctgaaatggcgtcccccccgtagcagtgggaagcgtatcaataatgctaagattaccggcaaaatattcacgaagcttgtcgcttaaaccgcctggattggtggcagaaatgcgctcatagccttctttgcgataatggatgtccagcagctgcaccatgcgttcgctgtactcttcccattcaaccgcccgcaggcgaaattgctcatcgcaaatcacccacagtggacccagtggcgtggcaattttttcttcaagtaatctcagcatccgttctctcttaagacaaacgtgggtaaatacccggacctatcggcagaccgacaagataccacgccagcaacatcagcagccataccaccaaaaagataagtggatagggcaagactaacgaatagtaagtacccagtttcgcgtctggtttgtagcgttgcaggaatccaagaaacagtggaacaaaaggagataccggcgctaaaggcaatacggatgagtcggcaatacgaaagaggatttgcgcaaatgccgggtgaaagccaagtagcataaacattggtacgaaaatgggggcgagaatcgaccagattgcggaaccgctggcaataaacatgcataagaaagaggaaagcaacgccagaccgacaaacgccgggatgccgctaagccctgaactttccagtatatcggtcagccccacggcgatgaatttccccatgttgctccagttaaacatggcgacaaattgggcgaggggaaaaaccatcacgataaatcccgccatctctttcatcggttcaatcattaaatgcggtaaatccgcctgacgtcgaattgtgcgggtagcgatgccataagccagcgagacaacaaagaaaaaaagaatgatcagtggcacgatacctttaataaagggtgatggcatcacggtgtgattaatcggatcgcgcaatatcccgttttgcgggatcaccatcagcgcaatcgcagcaataaaaagtagcgatacgacacctgctatgcgtaaaccaaaacgctgactttcggtcaatgtctgcagtttctcatcgctgtttccctgccattgacctaaccgtggctcgatgattttgtcggttatcaggccgccaacaatcgtcagtacgactacggagctggccataaaataccagttatcaattacactgacgtgcatttgcggattgaacgcagctgccgcttccgtgctgatccccgacagcaacacgtcggttgtgacaatcagtaaattagccgtaaagccgcaacctacgcctgcaatggcagccagtaaacctgcaactggatgcctgcccaccgccagaaaaatcagcgcacccatcggtggcatgatcactaacgccgcatcggaagaaatgtggctgaaaaaagcaataaacagcaccatataactggcgtagcgggcattaacatgcgatgccattttaaccattagtgctggcagtaagccgacgcgctccgccagaccggcacctaaaaccagcgccaggatcgcaccaagtggagcaaaaccgctaaagtttttaataacattgggtaaaaaccagtgtaatccttccacactgagcaggtttttcaccacgaccggcgtaccatcggtcgggtttttcgcactgacgccaaaggccgacaaaattgccgtcgtcaccatgagtacgataatcaaatagataaagagcagaaaaggatggggaaccttgttaccaattctttcgacccagccatagagcttcccggattgggaggacgacggtatggatgacatactcatgggcattcctcggttgttgtgtttgcgttgttgttgttattttaaaggtgacggtgtcacgtttttcgggatagggcagtgatacggttgcgtgtccgttacttgctgatgctcttgttggcattcttgcaatagccctgaatcaaggaagagattgactgtggttgctgccatagttttcgccgccagcagcattcctttatgagcaatagatgttcgcccctggctaaccagttgccacgtatgtagcggtgtaccgacggcaaaacaggggctgaaacactgggcaacaggcagtttccaactgacgtcgccgacatcagtcgatgccgcaagcacgttatcggtggcggcatatggagcgacttcattcgccagtaccgtttcacgatgacgtagtgcaaaaaccttgccgttttcgccaccggttgcggcgatattattcagactgttttgccgatcgttggaggtgagcgtagcctgaatttgtttcgcaaaagccagttcttcggagttccattccggggtaccaaaatgggatagggcctggtacatggcattttctaaggtgcgattcgggagataactggaacaggctttgtcgaagcggcattcaaccgtggtttcggtcatcaatgccgcaccttcggcgattttggcgacccgatcataaatatgctgcacgtcggtcatttcgggggcgcggataagataaagcacttctgcctgcgcctggaccacgttgggcgagatcccgccgctatttgtgatggcatagtgtacgcgcgctttttcaataatatgttcgttgaggaagttggtgccagtggtcatcaacgttacggcatcaagggcgctgcgtcccaaatgaggggaattcgcggcatgtgctgcgatccctttaaagcgccatgatgcctgaatgtttgccagcgtgcgggtattgaacataccggcaaaggcttccgggtgccaggtgagtgccgcatccacatcatcaaataccccctcgcgaaccatgaacgttttacccgagccgccttcttcgccaggacaaccataaaagcgcaccgtgccgccttgcccatattgttccagccatttcttgacggctattgcagcggcaaaggcggcggttcccagcaaattgtgtccgcaaccgtgaccattttcaccgggcgtcacggatgtaggttgcgcgcaacctgcttgctgacttaaacctgccagggcgtcatattctcccagcagggcgataaccggtttgccttgaccaaacgaagcaataaaggcatttgggatattgcctacgttgcgggtaacggtgaagcctgcagattccagcgccgaagccagatgctccgctgaccagaactcttcaaaacgtgtttctggatgatcccagatttgatcggcaatatcggtataacgttggcgatcggcttcaatcgcatcgtcgataaaacgatagatttcctgcatcagatacctcgcgtccagggaaaattgagcgcggtgcgcgccagcgtttcgacggcaatagcgagaacctgctcgtcaaaatcgaatttttcgttgtgatgacctgccgccagctgtgtgccaaacaccacgtaggaggcttgcccttgatgttgctgcacgcgggccatcattaatgtggcatcttcggaacccgcaggcgcttcaacacgttcaatggcctgattgacccccgcgacctgagccgcctgactttgcaaccatgcgacccattgcggcgaaggagaactggcggtagctgcacccatcagacgagtttcaacgccgacaccatacatggttgctgcgccctgaatcgcttgttgtgcacggtcaaaaacatattgattaatgacgtcgctggccccgcgtgtttccactttcagcaacgccgaggcaggaacaacgttacgaccgcttcctgcctgcataacgcccacgtttactctggaagctccttcgctgtgcggggcgattgcatgcagtgcaagagtggcttgtgctgccgccaacaaggcattgtgaccgtcttctggttttgcgcctgcgtgagcggcggtaccggtgaagtgcgcgtcaaatttggtggttgccataaaattatcactgccgcacaccacggtgcccgcaggtacgccagtgccaatgtgcacggcagtaaaataatcaacatcatctacgacacctgcatcgaccatcgcccgcgcgccacgcgtaccttcctctgcaggctgaaaaatcagtttgatgacgccatgtagtccggactcgaactgtttaagggtatgcgccagcccaagcccaatggcggtatgtccatcatgaccacaggcatgcatcattccggcgttacatgacgcaaaaccgtcgcggtaggggcgatggctgacatcctgctcttcactgagatccagcgcgtccatatcgacacggaaagccatcaccggaccggggcgaccggtatccagggtggcgacgataccagtgaaaccaccttcaaaagccgcaatccattgtgctagcgcaccctgttgacgagcgcgctcgaattcgcgttgtagagtgaattcatcaggtaatcccatccggctactttcattaactacttcgcgacccagcgccagtgaatagccgagctggtgcaattcttccgcaacaagggtggcagtgcggaattccacccagccagactctgcatagtgatgaaaatcacgtcgccagtgcgataattttggggcaagcgaattaacaaattgattcaaagactccataacctttcccgtcatcagtaaaaagtgtgacccggttcacgtagcgatagtttttacttatcactaactgatttttcacagttttaaccgttcataaattaccctgacacaatcatctgcattaaagtagatgccagtttctttggtctgataaataacggttatcggtggcgtcatggcttttcaggtaaaaattcatcaaattcgggcttttgttgaagtggctcgtcagggcagcattcgcggagcgagccgaatgttgaatatgtcgcaaccggcactgagtaaatctattcaggagctagaagaagggttagcggcgcaactcttttttcgccgtagtaaaggcgtgacgttaactgatgccggtgaaagtttttatcagcacgccagtctaattcttgaagagctgcgcgcagcccaagaggatattcgccaacgacaagggcaactggcagggcagattaatatcggcatgggggccagtatttcccgcagtctgatgccagctgtcatatctcgttttcatcagcagcatccgcaggtaaaagtacgcattatggaagggcaactggtgtcgatgattaatgaattgcgtcagggagaattggatttcaccatcaatacctattatcagggaccgtacgaccacgaatttacttttgagaaattactggaaaagcaattcgcgatcttttgccgcccgggacaccccgccattggtgcccgttcgatcaaacagttactggattacagctggacaatgccgacgccacacggcagctactacaaacagttgagtgaattgcttgacgatcaggcgcaaacgccacaggtcggtgtagtctgcgagacgttctcagcctgtatcagtctggtggcaaaaagcgattttctcagcaaactgcctgaagaaatgggctgcgatcccttgcacggacaggggctggtgatgttgccggttagcgaaattttaccgaaagcggcctattatttgattcagcggcgtgatagtcgccagacaccactgaccgcgtcattaatcacgcaattccggcgagaatgcggctatctgcaaagttaaaactgcataaaaaaatagagtctgtcgacatccgccagactctacagtacacacagcagtgcatccgcgtcttaaatccggcattgtctcctctgcgccggtgactgtgttataacggttttaacctttagttgccaattttcttcagtgacagatttcacgaaaatataagttacattattaatatcgtgaatgaataatcatgcataagtattttgcttaaaatatcggcaatatttggaacttattactggaaatttgggtaatacgttgttggaccgacccggtctggttatcatatcgcgctcttaattgcgggaggatgtaacatgaaccttgacgacaaatcgctgtttcttgacgccatggaagatgtccagccgctgaaacgtgctaccgatgtccactggcatccaacgcgtaaccaacgtgcgccgcagcgtatcgacacgctgcagcttgataatttcctcaccaccggatttctcgacatcatcccactaagtcagccgctggagtttcggcgggaagggttgcaacatggggtgctggataagctgcgcagtggtaaatatccgcaacaggcgagcctgaatcttttgcgccagccggtggaagagtgccgcaaaatggtgttcagttttattcaacaagccctggcggatggtttgcgtaacgtgctgattattcatggtaaagggcgggatgataaatcgcatgccaatattgtccgcagctatgtggcgcgctggctgaccgaatttgatgatgttcaggcatattgcaccgcgctaccgcatcatggcggcagcggggcgtgttacgtcgcactacgtaaaacggcgcaggcgaagcaagaaaactgggagcgccacgctaagcgcagtcgttgatctcgagacgcatccgcggcttatgccgccagcacgcggttgcgtccatcatttttcgcccgatacaaagcatcatcaacgcgtttaaacagttcatcgatgctttcatttccttcgtgatgcgccacaccaatgctgacggtaaagcgtggtaagcccgaaatactcacttttgccacgcttacgcggatagtttcagccagcgaaagcgcggtatccagtggggttcttggtagcaataagacaaactcttcgcctccccaacgaaacaccaaatcgcctttgcgagcgcaactttcgagggtgcgggcgagggcgcataacacctcatcacctttagaatgcccatagagatcgttaatgtgtttaaaacgatcggtgtcgatgagcaacaagctgtaatcctgagcgatggcgagatgctgcatttggcctggttccgtaatgtgataaaactgtcgccgattcagtaatccggtcatcgcgtcatggtgagcagcatgttccagctgctcctccagccgtttttgctcagtaatatcatgcacaatacataacatgagcttgtcgccataaatttcaatcggtccggcataggtctgcacatgacgagtcgaaccatccgccagtttatgaacaaaattcaaaggtttatgaccaccgggtaaatgcgagatttcatgcatgataggcatgacgcgacgcccgagcatatttatttcccaggtatgtttctggcacatcgtttcatggttataaccatagaaattgagcgcggcgaggttagcatcgacgatttgtccatctcgtgacgggtcaatcaacaacattggtgcagagttagtcagaaaaaagcgcgcataaaaaccttgttttttgcgctgataatttgccgagcgactggcttttaaacccagcgttgccggcgcttcgataccttcgaaaataatcaccggttctgtttctgtcagctttcgcaaaacaagccgacagctcaatgctgtttcctcttctttacgctgaacagtgaggatttcgataatatcgtgttggttttgcagatcggagaggtatttcggcagttctttttgtgaggagacggaatagggtccggttcgtagctgactaaacgtgaggtcttgcatcaacagtttcgccgcgctattggcataaattaactgttcctcaaagggcgaaacgatccagacaggactggtgagtaagtccagggtattgaagttgtgcgtaatcattgagatcccgttatttttatcaatttttgttgctatccgatcgcaaaaaagccacgtcatatgatcagataattctgataatgatagacgctatttaacacttcacacggtttgtatacggaaaagcattttgctttttgtattcaatttagacagaattttattaatcatttcagggtaatggggtgatgagatgttgcgtaacagggccagaaggctagactacaaaataatgcgttgatgatggaggcactgtggaagcgattaagggatcggacgttaatgtcccggatgcagtatttgcctggatgctggatggtagaggcggcgttaaaccgctggaaaatacagatgtgattgatgaagcgcatccctgttggctccaccttaattatgtacaccatgatagcgcccaatggctggcgacaacaccgctgcttcccaataacgtacgtgatgcgctggcgggcgagagcacgcgtccccgagtcagccgtctcggtgaaggcacgctgattacattgcgctgtataaacggcagcaccgatgaacgccccgatcaactggtcgccatgcgtgtatatatggacgggcggttaattgtttcgacccgacaacgcaaagtgctggcgctggacgatgtggtgagcgatctggaagagggcacgggtccgaccgattgcgggggatggctggtggatgtgtgcgatgcgttgaccgatcattccagtgaatttatcgagcagctgcacgataaaattatcgaccttgaagataatctccttgatcagcaaattccaccgcgtggattcctggctctgctgcgcaaacaattaattgtgatgcgtcgctatatggcaccgcaacgtgatgtttatgctcgtcttgccagtgaacgtttgccgtggatgagcgatgaccaacgccgtcggatgcaggatattgccgatcgccttgggcgcggccttgacgaaatcgacgcctgtatagcacggactggcgtgatggcggatgaaatcgctcaggtgatgcaggaaaatttagctcgtcgtacctatacaatgtcgttgatggcaatggtctttttacccagtacctttctgaccgggttatttggcgtcaaccttggtgggatccctggcggcgggtggcaattcggattttcaattttttgtattctgttagttgttcttattggtggtgttgctttatggttgcatcgtagtaaatggttgtaacaaaagcaatttttccggctgtctgtatacaaaaacgccgcaaagtttgagcgaagtcaataaactctctacccattcagggcaatatctctcttgcaggtgaatgcaacgtcaagcgatgggcgttgcgctccatattgtcttacttccttttttgaattactgcatagcacaattgattcgtacgacgccgactttgatgagtcggcttttttttgcctgttatttatcagcgtctaccctttaagagtccacccaatgaccagagggaaatatgacgacacttatttatttgcaaattcctgtccctgaaccgattcctggcgatcctgttccagtgcccgatccgatccctcgcccgcaacccatgcctgacccaccacccgatgaagaaccgattaaattgtcgcatcgtgagcgtagatctgcgaggatacgcgcctgctaactttgcgtcgatgaccacgagaatagattgtgaccgctttttctaccctgaatgttttgcctcccgcccaactcacgaaccttaatgagttgggttatttaaccatgacgccggtgcaggccgccgcgcttccggcgatccttgccggaaaagatgttcgcgtgcaggcgaaaaccggcagcggcaaaacggcggcttttggcctcggcttgttacagcaaattgatgcgtcgctatttcaaacccaggctttagtgctgtgtcctacgcgtgaactggcggatcaggtggcaggtgaattgcgtcggctggcgcgttttctgccaaataccaaaattttgacgttgtgcggtggtcaaccgttcggtatgcagcgtgattcgttgcaacatgcgccgcatattatcgtggcaacgccggggcgtttgctggatcacctgcaaaaaggcacggtatcactggatgcgttgaatacgctggtgatggatgaggccgaccgcatgctggatatgggatttagcgatgccattgatgatgtcatccgttttgcgcctgcatctcgacagacgcttctgttttcggcaacctggccggaagccatcgctgcaatcagcggacgagtgcaacgcgatcctttggcgattgaaattgactcaacagatgctttgccacccattgaacaacaattttatgagacatccagcaaaggcaaaattcctctgttgcaacggttattaagcttgcatcagccatcctcttgcgtggtgttttgcaataccaaaaaagattgccaggctgtctgcgacgcgctgaatgaagtagggcaaagtgcattgtcattacacggcgatttggagcaacgcgatcgcgatcagaccctggtacgttttgctaacggtagcgcccgtgtactggtcgcgactgatgttgctgcgcgtggtctggatattaaatcgcttgagctggtggtgaactttgagctggcgtgggaccctgaagttcatgtacatcgcatcggtcgtacagctcgtgcaggaaatagcggtctggcgatcagtttctgtgctccggaagaagcacagcgggccaatatcatttctgacatgttgcagataaaacttaactggcaaacgccgccagctaatagttccattgcgacgctggaagcagaaatggcaacgttgtgtatcgatggcgggaaaaaagccaaaatgcgcccgggtgatgtattaggtgcactgacaggagatatcgggcttgatggcgcagatattggcaaaatcgccgtgcatccggcgcatgtctatgtcgcggtccgtcaggctgttgctcataaagcatggaaacagttacagggcgggaagattaaaggaaaaacgtgccgggtgcggttattaaaataatgaaatgttgaattgccgggtgcaagagtaaacatcttattcgggattgccggatgcgacgctggccgcgtcttatccggcctccataagagtagcccgatacgcttgcgcatcgggcgctatcctggttatttcacttcaaccacattcagccgtaactcatccaactgattttcatcttcttctggctgccagcacgccggttgtagtgggatctcttcgcgatcaaacgccagatcacccccgttaaccacttcagaaccgtgggtgatgcctttgaaatcgaacaggttggtatcgcacagatgcgacggcaccacattctgcatcgcgctgaacatcgtctcgatacgccctggataacgtttatcccagtcacgcaacatgtcagcaatcacctgacgttgcaggttaggctgtgaaccgcacaggttgcacggaataatcgggaacgcttttgcatcggcaaatcgctgaatatctttctcgcggcagtaggccagcggacgaataacgatatgtttgccatcatcgctcatcagtttcggaggcatacctttcatcttaccgccgtagaacatatttaagaacaacgtttgcaggatatcgtcacgatggtgacccaacgcgatcttcgtcgcccccagttccgttgcggtacgataaaggataccgcgacgaaggcgagaacacagtgagcaagtggttttgccctctggaatcttctctttcacgataccgtaagtattctcttcaacaatcttgtactcaacgcccagcttttcaagatactcgggcagaacgtgttccgggaagcccggttgcttttgatcgaggttaacagccaccagcgaaaaattgattggcgcgctttgctgcaaattgcgcagaatctccagcatggtatagctgtctttacccccggagaggcaaaccatgatgcgatcgccttcttcaatcatattgaagtcagcaatggcttcgcccacgttacgacgcagacgtttttgtaatttgttcaggttgtattgttctttctttgtaatttgttgattttcttgcattatttcagttctctggtactaaatggggcaaattgggggcaaactttgcaactacgataaccgcgcattcaacatggctatctgttcgtcgttcatgtcatcaatccacataccgtaaatttcatacaccatctgcgcagtttcatgccccatttggctggctataaatgccgggttcgctcctgccgtcaacagccagcaggcaaaagtatgccgcgtatggtacggattacggcggcgaataccagcacgttttactgctgcattccaccttgcccccaaactgcttaccgagtaataaggtttttgttttccgttacacaccctgggcatgaaaacaaaatgcagtttttgcttttcggttctgccgtactcccgatgataaaaggtgatttcgcttttgcgatgatgcccggtcagtttgtattgctccttcagtgcttcaagagcaggctgcagtagtgttactgttcggatcccggcatttgtttttgggggaccgaacatatcaagtatcgtcaggtttcttctgacattcactattcccttttcgagatccacatcctcccacgccagagctgccagttccccgtgacgaagtcctgagtaaacggcaaatttccacaagttctggctctgtcctttttcactttccattaatgcattgaattctgttttagataacggatcaggctttattctgtttcgctgtaatttttttactccttcaaatggtttggttgatataaatcccgactgatacgcaaaacgcaacagcgaacagagcagggcgatatagttatcaactgtgcgcacggttcttccttttttgttggatcttggattatccaggtaaagcgtttctccatgcagcagttcattccggtagtttaagatatcgctataacgaatatgtgatatcggggtactttcacaaattattattctgagtgtttttaattgtgatttcgttttcttcattgtgtttgttgttaactctgtctctttaatttttgtccagatatcacaaagctctccgaacgtttttatgactctcgttgtcaccatttttgccccagtgctggactggggaaaacgtcttaaatactcaaattcaccggagtttatttcatgaactatcagcgctcttaaatttccggcctttttaatattactgtttgtaatctcccagccttttaatgtttcccgacatcgttttcctcgaaacatgaaccagatgcgaatgtatctacctctaatctcgacacctgttggtaatttagacatatcatgagtctttgataaactgatttatctttggatagttgtaccagataatccctcgtttgctgtctggcttacctaaaggagatactcgtttgaagtggaagccctccacccaacagttctggcggtatgcttcaatttgtctggcccccagaccagtgcgaagcatcaggccgtattcaaccatccactcttcattaaagattacttgtgccatcgcatcacctctggcaggcgccaatgttagactgaaattgacgcccgatgttgattattaataatcagctatgaagttttaatttgaatacaatgcaattctcgaggactgaagtttctcgcaattaaaatttatcagttttactttctgctctctggaaacgcctgcttcttttttacctgagagcattttttcgcattctgatttcgttagtttagattttgaatatcttgtccagttagtaggagtgccaccttccttttcaatagtggcggtaattttatacatgaacacctccattattatttccagtggttcgtttattccatctttcgagtgcttctttttcacttccaccataaccggttcgggattcgcatccgttacacttcgctcggtaatatcctgaaatggctttcaccgttactgatggacaaccacaaaatggacatggtttaacattgtcatatctcataatttttctcataaaaaatatttcaagttggcggtgcattacaccgccaggctgaattattcctctgaattatcgattacactgtattccccggttaatacagaggaatctgcaggatcgattgtcagtggttccttttcatccattgatactgcacgctggatctcaattgatacgggcaaatatttgaacaggcgacgaatagccgttttctttgccatttcttcccagtgagttacccacggcccgttattaccagctttactcaggctgcgcaccagctcaatctgtttgcgcgtcataacttcaaactgagtacctccgtctttcagtcttgcgacagcatagacgtgggtaaccggggcatcttcgttttctcccgggcggtgtattaacttttcatcaaggccaaattcgaagctaaactcgtcaccttcacggacaacacgggctgacaggctggcgatttgaccagaacggcgagccagatcaatcatgccgcgatagccaatgattagctgaacgttctttttaccgctcttttcgtttttattaccaaaaggcagtaaatatgcatgaccgagggcgctacctggctcaagtccgagctgtgaacactgtacgatcgcactgacaaaactcatagtgtcacagtttcctaacgccggaactttacgaatttctgtggtggcgatacggatcatacgttcagccgtcatatggcgtggaagagctgctgccagttgctctttcattgatggctggttaataaaactaatcacgtcgctatttttaactgctgctggtgcacggtttccctgagttttttgcagatcggcttttgcgattggtggttgcttagtcatttgcatattccttagcccagcggggcagtgataatgtcttaatagctggccattcatcggtattcaggcagtcagacagggttcgcagattgcggtgatattcctgttgacctgccagttttgcttcttcgcccatcatgaaaatttcaaccggataacgtccgcattcaatagttgtgctggcaaccagaaaaacgaaagttggctgcactccaaactgtgcttcataaccgtcactgtagaatgcatcctgaacgtgatagcggtagtcgtaataagcggttttgaatcgttgaatatccgccgtagttttcacgtccatgatccagtgaaattcagggataattttgtccggacggcaccgacacaaaattcctgtttcaggatcttcccagtaaattgatgattcagcgtgtccggcgctttcaacaagccattgccccagcggcaaagccataacgctttgatacatgagttcaattttccggccttcttccgcagtgataaccgtttttcctgtgcttgcgcattccatcagaaacgctttctcttcttcttttccggcgtttgtacggcggttaaattcaggtgctacgataaagcggttactgaattcttccggttcaagtacccggcagtggaaagcagttcctaaatcgagcgtttttgtctttgtggtgtccacgggggcatttttacgccacaaatatagtgccggagtatcagcaatgtcatcgagctgagacttactgataccgggacccgcgtggtaattctcattcgaaattccgtaataaatacctggctctatgtcttctacgattacgggatctgcgacttcgccagtttcatcactgcaatcgcgatgcggatcgctgccagcattctcattgtgcggatgttcagcgccttccatttcctccggatcattttccttagcttcaacctgactctcttcatcgaatgtttcctggtatgttgcgtcgcccatcaccgcaccacagtcagggcagttatccccgccagtctggccgcaggcattgcaggctatttccggttcctgttgcactactggctcaggttgattcatatctgggctggttttttccgtttctggctggttctggtacacacaatcgcgagtctggatcccctttacccatttcggatcgttcgggtcgctaattccgtcaacaaattcaccacgtgatgcagcaagcaatttatcgtcatcgacaggattttttgatggaatgtttttccgggcttcatggagttctgcccgcagttcctgatatttcgcatcaacagaatttacctgtgactgagcatccagcggctgcgtgtcctgatgatgttcagttgcgtccggttccattgtttcagcctctccctgttcaactgccgttgttccagatggttgcggtttttcttcatcatcctgttttccttcttctgttactcgctgcggcatcggggcagaggagcgaccgcaggcaatatccacgatttccggatcagggttggcatgatcggtttcagtcagtactttgttcagatattcagtgacgtgcgcggggatgacctcgatcccaattggtgcttcttttacggacgcaaccacgatggcgcgggaataatccagcccgccaggcatggtgatgaatttgtcgcggaaaacagaaaagggcggtttattttcagcgataatttcctcaatgcgtttagcgtgtgccggatgaaggttatagatgtccagatccattgaacgggccagtacgccagtggctacgtcgcgcgccagtgacgtcagatcgtgtacgaaaccttcgccgcgatcggtgaggtttccgccgccagcattagcaccggaagccgtgcgagtgatgtgtgaaacacgattacccttcatccactcttttgtcagcagtcctcgatcggtgtagtcagcgttcaggtatgcttcgaaaaaagcagttatcagtcccaggtttgaattaccaggattagggaaaactttgtcagtgtcacgaaccagtttgtggagttcgcgaatttccagcgggtcgagcaggctggttttgtgggaaacagccagggcagtaacagccggtagttcttcagcccgagcaatgtgtaatgcctggagtccgtcgcgtgaaacgtgcgttaccggtttttcgctgccgtgttgagcaagccaacgaatgggcagttcctggccagaaattgggagtagcatattctcctcaatctcagtcatgtcttcgccgttgacgttggtattgccttgatagtgagcgttgtctggtgctgctcccggttttagttcccatgtcatggagtctttgctgagttgatagcgttcactccaggtaaaatcgatctcaccttcagcgggcaggtcattaacgacaggaaaattcgtggcaacagctttaaaatagctgctcagttttttacctgacttaacgatcaggtagtccagagtggcacaggtcgattcaaaatcgttgcttgcccacaggacgacgtcaggttcaccggatgattttttcgctttccgtaacaggaagagtggttttgtgctcattgttttttaacctcaactcagattaaaattcgttttgttcagtgaatgatcttgccggatacacactgttcatagcctgcgccatacgcaggctatttctttcagatttcaccttttaatttcattgcaattagagttgccagaaattcggcttttttttctgcgggcagattctttccgatatgcaccaggcacatttttttgacaccttcatcaagtgtttttacgttgcctgatggaccatcgatatcaaccacagtgaatggggtttctttattttctgttttaattacgtagccaatgcgctttccttccagattcacctcgtgaacaatgtcatcggtagttacaacagtggcttcataattggtaatcatgtttttctccttaattaaggttgagcgaatacctgccatttctggcataaattcagtttcgaatagtcaattaattaaagttcatgtgccatctggtctttttcggcacaagcttcactgcaatattttctcggttcgtcttttgataaaatcccgtgcatgaagtgaagcattctttcaatagctttgctttcttcaacgtcttttttgcaaaggtggtaagcacattttattttcttagtcatcaccatgactccgcctttacaggtaaaccatcacgaccgaggaagactttaatcatgcggtcagtaatgaatgtttttgtggtcaggttacgaatatatagttttcgctttttaatattgtttgccgaggcaatatatgtccggccttcatgaagaacataatcgccaggagtcacacactgacgtggtatttcatcagttccgaagtgatgtgcaatcataattatctccatttttacaaatgaactttgttgatgcggtgtctggtgcctccaggtgactgcaaccagttaacaattacagtcggctttcccacccaaaccaataaggactaacatgacttttaactgtgccacgtgcgcttagccgcattcaccgcatcacaaaattcactttaaaaagggcggacatcagccgaacttcaagaaaaaaactgatgccgccaggactacacacagcaatgtcgttatttacaaccggaggcgcactcccaccatttaaatttaacagacaagaccgactctttatggatatcggaaatgcgccttcgtgttgtgcccggttttatttcaccacctccgggcttcggtggtctcggctatacccctacagcgagagcttgtgttaacatttcaatacccttacagttgagagttattgatatgttggatgtatttactccattgttgaaactttttgctaacgagccactcgaaagacttatgtatacgattatcatttttggtctcactctctggctgataccgaaagagtttactgtcgcattcaatgcttatactgaaataccttggctctttcagattatcgtttttgccttttctttcgtggtcgccatttccttctcaagattgcgagcacatattcaaaagcattattcattactaccagagcaacgagtattgcttcgtttatctgagaaagaaatcgctgtatttaaagatttccttaaaacaggaaatcttattatcacttctccttgccgtaacccggttatgaaaaaattagaacggaagggcatcattcaacatcagagtgatagcgcaaactgttcttattatctcgtcaccgaaaaatactcccattttatgaagttattctggaacagcaggagtagacgttttaatcgttagcttactgtgtgcttctccaaccatcggcgcgcaccagtttcggttttaaatgttttgcttttggtatacgtcatggcagtgaacgttccatcctggttggggaacacgccgcacaccagggattcgttgttgccgaggtcgattttttgcattttgcgaatctcacatcttgttgctacgtatagcgacttctgcctgccagagatcccagtcgttgctgcgtaaagcctgcacagcctggttgtaagtgataccgcaacaatccatcaaatactgaactacttcgtaatgcaccatcttatctctccccttaacgccgggtggcggaactaactgctgcactgcaaaatttgaatcccgccgtcatgttcatacgcctcgggctggctacttaaccccttaccactgcctggtaactcgaagtattgcccggcgttctgtggggcggggtgggtggtatgctggaactataggtaatgcctaattgattgtcaataggctatgcctaatgttttgagcgtaacctaataggtgatggcgacagcagaaagtgatgggggggttaaataacggaatccaggagttttccgtcagaccatataagtttaagttccagtttttgtgatgttctggcttttccgttcagattcaagagctttcagatacttacccactttcatttccatcgctgctatgtaggcgcgaacatcgtggtcaacccaatctggttctgtagcatttccagataacaggaaagctacaatcgctcttatttcatcagaggctgcttgataaaggttgtttatatctaaaagttcactttttgtatctgaattggtgggggttggtatggggtattcgttaagcccccaatgctctggaccaacaacatcagaaaagaaacgccataattctggaagtttatctttacttatagagcctttcttaatccagtcataaattgatggtggttggactttaaagtggcgtgcgacctccgcctttgatttgacggatcccgatgcgatttttttgttaatggcctgctctatcgctcggcctaagtctttaccactaagcattgcttaatattctcctatgcgcattacattaggcaatccctacccttactgcattaggcacagcctattgacaattgcgttaggcgtcgcctaatatttctgtgtgtttttggagttcattcgatgaaaaaagagaactattcattcaagcaagcttgtgctgttgtcggtgggcaatcagcaatggctaggcttttaggtgtatcacctccaagcgtaaatcaatggatcaaaggggtacgtcaattgcctgccgagagatgtccagcaattgaacgtgcaacaagaggtgaggttctgtgcgaagaacttcgtcctgatattgactggtcatatttacgacgttcggcatgttgttcgcagaatatgtcagtgaagcaactaaatgacagtaacaaatcctcatttgatcatacctgaaacatcaagaggcaaatgattcatgaaaatcaagcatgagcacatcgaatcagtgttgtttgccctagcagccgaaaaagggcaggcatgggtagccaatgcaattactgaagaatatctgcgccaggggggcggcgaattgcccctggttccaggcaaggactggaacaatcagcagaatatctatcaccgttggttgaaaggtgaaacgaaaacgcaaagagaaaaaattcagaagctgatcccagcaattctggcaatccttccgcgcgagctgcgtcaccgactctgcatcttcgataccctggaacgccgtgcattactggcggcgcaggaagcgttaagtacggcaattgatgcgcatgatgatgcagtccaagccgtttaccggaaagcgcatttcagcggcggcggttcttccgacgattctgtcattgttcattaagcaaaagtttccatgctgtttgtgcttattctaagccaccgggcagcatcatacggggcaattatggccgcattaccatacatgcaactgtacatagctgattacctggctgacaccatgcatttgtcagcagaggagcatggtgcgtatttgttgctgatgttcaattactggcaaacaggaaagccaatacctaaaaacaggctggcaaaaattgcccgtctgactaacgagcgatgggctgatgttgaaccatccttgcaggagtttttttgcgataacggcgaggaatgggtgcatcttcggattgaggaagatctggcatcagtcagggaaaaattaaccaaaaaatcagccgcaggaaaagcatctgttcaggccagaagaagcagaaaggaagcagatgttcaaacaaaacaagagagaaatttaacaggtgttcaaacagatgttgaagtggtgtttgaacatgatgtcaacacaaaggcaactaataaagatacagataaagatctaaaaacagatccccccctaaatcccccccgggggaatcgaggtgtcaaaaagtttgaccctctggatattactttgccgaactggatttctgtctcgctttggcgtgagtgggttgaatttcgccaggcattgcgaaaaccgattcgaacggagcagggcgctaacggggcgatacgggagctggaaaaattccgccagcagggtttttcacctgagcaggtgattcgacacagcatcgccaatgaataccagggcttgttcgcgccgaaaggtgttcgacctgagacgttactccgacaggttaacaccgtctcgttaccggatagtgcgatcccgccaggcttcagggggtaactgaccatgaaaaatattgcgacaggcgatgttcttgaacgtatccgcagactggccccgtcacatgtaaccgcgccattcaagacggtagcggagtggcgcgagtggcaactttccgaaggccagaaacgttgtgaggagatcaaccgtcagaatcgtcagttgcgggtggaaaaaattctgaatcgctctggcatccagccattgcaccgcaaatgctcgttttcgaattaccaggtgcagaacgaagggcagcgatacgcgttgagtcaggcgaaatccatcgctgatgaactgatgaccgggtgtacaaattttgcgttcagcggaaaacctggtaccgggaagaaccacttagcggcagctatcgggaatcgcctgctgaaagacggtcagacagtgattgtggttaccgtggctgatgttatgagtgccctgcacgccagctatgacgatgggcagtcaggcgaaaaatttttgcgggaactgtgcgaagtggatctgctggttcttgatgaaattggcattcagcgcgagacgaaaaacgagcaggtggtactgcaccagattgttgatcgccggacagcgtcgatgcgcagcgtggggatgctgacaaacctgaactatgaggccatgaaaacattgctcggcgagcggattatggatcgcatgaccatgaacggcgggcgatgggtgaattttaactgggagagctggcgtccgaatgtcgtccagccaggaattgcgaagtaatttttaccgggagaaaaatttaatggagactgtttttgacgcactgaaagcaatgggaaaagccacatccatagaacttgctgcgcgacttgatatcagtcgtgaagaagtgctgaacgaactatgggaactgaaaaaggctggttttgttgataaaagcgcgtacacctggcgtgtggctgataacaatgttcagcaggaacagccagcgcaggcagaactgccggaagaaatcaccacagcaacagtagcgaaaatctcagagtgcgatttaaccgcgacgattgaacaacgaggaccacaaacggctgatgagctggctacattgtttggtaccacatcacgcaaagtggcttcaacgctggcaatggcaatcagcaaaggtcgtctgattcgcgtaaatcagggcggtaaatttcgttactgcataccgggcgataatttaccagcagagccgaaagcagcatcggtatctccgctctggttatctgcatcgtcgtctgcctgtcatggggtgttaatcattaccgtgataacgccatcgcctacaaagaacagcgcgacaaaaatgccagagaactgaagctggcgaacgcggcaattactgagatgcagatgcgtcagcgtgatgttgctgcgctcgatgcaaaatacacgaaggagttagctgatgcgaaagctgaaaatgatgctctgcgtgatgatgttgccgctggtcgtcgtcggttgcacatcaaagcagtctgtcagtcagtgcgtgaagccaccaccgcctccggcgtggataatgcagcctccccccgactggcagacaccgctgaacgggattatttcaccctccgggaacgactggtaatgatgcaggcccaacttgaaggtgctcagcaatacataaccgagcagtgtttaaagtaaaatcttaactacaatatgattcattttgatgattgtttcataaggaacagtgaagtaagatctaagaggagttaaattttatacagtataatcataatattgcagcaaggtggttataattgaaagaatatttagatatgaatacatctcatgtaagagttgttactcatatgtgtgggttcctggtttggctctatagtctttcaatgttgccaccaatggttgtagcattgttttataaagaaaaaagcctgtttgttttctttataactttcgttatatttttttgcattggtggcggagcgtggtatacaactaagaaatctggcattcaattacgtacccgtgatgggtttattataattgtaatgttttggattttgttttctgttattagtgcattccctttatggattgactcagaacttaatttaacgttcattgatgctctgtttgaaggggtttctggaataacaacaacaggagcaactgtaattgatgatgttagttcattacctcgggcatatttgtactatcggtcacagttaaattttataggtggtttaggagttattgttctggcggttgctgtattgccattattgggtattggtggtgcaaagctttatcagtcagaaatgccggggccatttaaggatgacaaactcactccccgcctggccgatacgtcacggacactgtggataacttattctttattaggtattgcttgtattgtctgttatagacttgcaggaatgcctttgtttgatgctatttgtcacgggatttccacagtttcgcttggtggtttctcaactcatagcgagagtatcggatattttaataactatttggttgagctggtggctggttctttttccctgctatcggctttcaacttcactctttggtatattgttattagcaggaaaacgataaaacctttaatcagagatattgaacttcgtttctttctgttaatagccttaggggtgatcattgttacctctttccaggtctggcatataggtatgtatgacttgcatggaagttttattcattcgttttttcttgccagctccatgctcactgataatggtttagctacgcaggattatgcaagttggcccacgcacacgatagtgtttttgctgttgtcaagtttctttgggggatgtataggttcaacttgtggtggaattaagtcacttcgatttcttatacttttcaaacaaagcaaacacgagataaatcagctttctcatcccagagcgttgttgagtgtaaatgtaggagggaagatagttacagatcgtgtaatgaggtctgtatggagtttcttttttctttatactctcttcacggtgttttttatactggtgttaaatggtatgggatatgattttcttacatcatttgcaacagtggctgcatgtattaataatatgggattaggttttggggctactgcatcgtcattcggagtgcttaatgacattgcaaaatgcttaatgtgcatagctatgattcttggtcgccttgaaatttatcctgttattatattgttttcaggttttttttggcgctcctaatatatggctgatttataattgtgagtttaatattatgttgactcactcattgatccaatacctaactttaccagcaacacctccgtccccagtagcactggctgctggggtgcgttttattcataaagcaaggctgtatgagcgagaaattaaagatagtctatcgcccattacaagaattgtcaccgtatgcgcacaacgccaggacgcacagtactgagcaggtggcacaactggtagaaagtattaagcaattcggctggactaatccggtgctgattgacgaaaagggcgaaattattgcgggtcacggtcgtgttatggcggctgaaatgctcaaaatggattctgttccggtcattgttctgtctggcctgacggatgagcagaagcagcgataacgatcagtatcgctcccgtaatgcattaatccgtcgccacattgagaaaatggatgccagtttgcacgtcggaacgaaggagtttgatatttcaaaggtttccgaggtggattctgttgatgatttactcattgataatgccgctcgttatctgctgaaagactggaaaggggttggtgaactggttaatggtgttgaggttgcactggaatatacggcagaacgagggatcgcgctgcttaagcagaatccagagttgtactggcagatccttgcagaagcagccagcatcgcccagggtaaagagcagcagaagcaggatacgataaaaaagccatagctgcccagcggtggttatcggagttcgggggagaaaggggggaaaaggcaagatggaagcgagaaaaactcaggttgccaccgataccggaaccagaaatagacccggtgcttaaggagttgttgtacgcctattcggtaatatcccgtgcccgacgttatgctggaatggctggggtgcctttgcctttatctctgacagagataaatgaatatttagccactcatccggtattgattgagcgcgatgaatttgaagcagtgatctttgcactggatgaccagtattttcaggagcagtgtgtgtagttgttaattacgtacactctgttacagagatgtgatggtgtctttaattaaatcgatgatgctcctggagaaaagcattgcgtggcctcgtaatcgctatatctactattatgtcgcctgaaacccacttcgcggtgggttttttgttgtcaggagttttaataaatggcagagcaaacctcgcgtctcgcaataattattgatagcactggagcgaaaaataatgctgacaatctgacctcctcattagtcaaaatgacgcaggctggggaaactgctgcaaatagcgcagggaaagtgactaaggcaacagaagatgagaagaacgcgctcgcaaaattaaaagcagctattgatccagttggtgccgcaattgatactgtcggtcgacgctattctgaattaaagaaatttttcgataaagggcttattgataaagaagaatatgaatttcttgtccgtaaacttaatgaaaccacagaggaattgagcggggttgcgcaagcgcagagagaagccgagaaggccggaaaacttgctgccgctcagcaggaagcgcaggctcaggcctttcaaagaatgctggacaagatcgaccctctggctgcggcgctaagaaatcttgaacaacagcatgatgaacttaatgctgcgtttgcatccgggaaaataaatggttctcagtttgagaattatagccgaaaaatacaggaaacacggcgagagcttaccggagaggctcaggcagagcgagaagcagcaaaagcgcatgatgaacaggttgttgctttgcaacgtctgattgctcaacttgatcctgtcggaactgcttttaatcgtctggtagaacaacagaaacagctcaatgaagcaaaagctaaggggatgctttctcctgaaatgtatgaggagctttctggaaaacttcgtgctatgcggagtgagcttgaggttactcaatcacaattaagcaaaaccggaatgtcggcaaaacaaacggcttttgctatgcgcatgttgcctgcacaaatgacggatattgttgttgggttgtccactggtcagtcgccatttatggtgttaatgcagcagggcggccattcagctatgcaggagacaagaatcgccagcttacccgttacagcgatacccgctggcatgaagattccgtgcgtaaccgctggttcagcgtgatggtggggccgtctgtgcgcgtgaatgaatggttcagcgcgtatgcgatggcgggtatggcttacagccgtgtgtcgactttctccggggattatctccgcgtaactgacaacaagggaaggtgcgaataagcaggtcatttcttcccaagctgactcgctgattaaaatttcgcggatctgggccgatttttttcccgcaaacacatcgaatcagcctatttaggctattttttccaccatttctggcgttatttccggtttttactgagatctctcccactgacgtatcatttggtccacccgaaacaggttggccagggtgaataacatcgccagttggttatcgtttttcagcagccccttgtatctggctttcacgaagccgaactgccgcttgatgatgcgaaacgggtgctccaccctggcacggatgctggctttcatgtattcgatgttgatggccgttttgttcttgcgcggattctgcttcaaggtttttaccttgccgggacgctcggcgatcagccagtccacatccacctcggccagctcctcgcgctgtggcgctccttggtagccggcatcggctgagacaaattgctcctctccatgaagcagattacccagctgattgaggtcatgctcgttggccgcggtggtgaccaggctgtgggtcaggccactcttggcatcgacaccaatgtgggccttcatgccaaagtgccactgattgcctttcttggtctgatgcatctccggatcgcgttgctgctctttgttcttggtagagctgggtgcctcaatgatggtggcatccaccaaagtgccttgggtcatcatgacgcctgcttcggccagccagcgattgatggtcttgaacaattgacgggccagttgatgctgctcgagcaggtggcggaaattcatgatggtggtgcgatccggcagggcgctatccagggataatcgggcaaacaggcgcatggaggcgatttcgtacagggcatcttccatggcaccgtcgctcaggttgtaccaatgctgcatgcagtgaatacgcagcatggtctccagcggatagggccgtcggccattgcccgccttgggataaaacggctcgatgacagcggtcatattctgccatggcagaatctgctccatgcgggagaggaaaatctcttttcgggtctgacggcgcttagtgctgaattcactatcggcgaaggtgagttgatggctcatgatgtccctctgggatgcgctccggatgaatatgatgatctcatatcaggaacttgttcgcaccttcccaaggggaaaacgcacgacgtgctgaccggaagtgatgacggtcgccacagcaacacgtctctggcgtggggagctggcgtgcagtttaacccgaccgaatccgtggccattgatattgcttatgaaggccccggcagtggcgactggcgcactgacggtttcatcgtgggtgtcggttataagttctgattagccaggtaacacagtgttatgacagcccgccggttcaggcgggcttttttgtggggtgaatatggcagtaaagatttcaggtgtactgaaagacggcacaggaaaaccggtacagaactgcacaatccagctgaaagcaaaacgtaacagcaccacggtggtggtgaacacgctggcctcagaaaatccggatgaagccgggcgttacagcatggacgttgagtacggtcagtacagcgttattctgttggtggaaggattcccgccgtcacatgccgggaccattaccgtgtatgaagattctcaacccggtacgctgaatgattttctcggtgccatgacggaggatgatgcccgtccggaggcactgcgccgttttgaactgatggtggaagaggtggcgcgtaacgcgtccgcggtggcacagaacacggcagccgcgaagaagtcagccagtgatgccagcacatcagcccgtgaggcggcaacccatgcggctgatgctgcggactcagcacgcgcagccagcacgtcagccggacaggccgcgtcgtcggctcagtcagcgtcttccagcgcaggaacggcatcaacaaaggccactgaagcatcaaaaagtgctgccgctgcagagtcctcaaaaagcgcggcggccaccagtgccggtgcggcgaaaacgtcagaaacgaatgcttcagcgtcactacaatcagcagccacatctgcatccaccgcgaccacgaaggcatcagaagctgcgacctcggcccgggatgcggcggcctcaaaagaagcggcaaaatcatcagaaacgaacgcatcatcaagcgccagtagtgcagcttcctcggcaacggcggcaggaaattccgcgaaggcggcaaaaacgtccgagacgaacgccaggtcttctgaaacggcagcgggacagagcgcctcggctgcggcaggctcaaaaacagcggctgcgtcgtctgccagtgcagcgtcaacaagtgccgggcaggcctcagccagtgccaccgccgccggaaaatcggcagaaagcgccgcatcgtctgcttcaacagccacaacgaaggctggcgaagccactgaacaggccagcgcagcagcgaggtctgcttccgcagcgaagacatccgaaacgaacgcgaaagcgtcggaaacaagcgcagaatcctcaaaaacggctgccgcatcgtcagccagttcggcggcgtcatcggcatcatcggcgtctgcttcaaaagatgaggcgaccagacaagcgtcagcagcgaagagcagcgccacgacggcatccacgaaggcgacagaggctgctggcagtgcgacggcggcagctcagagcaaaagtacggcggaatccgcggcaacgcgcgccgagacagcagctaaacgggcagaggatattgcatccgccgtggcgcttgaggatgcaagtacgacgaaaaaggggatagtacagctcagcagtgcgaccaacagtacgtctgaaacgctggcggcaacgccaaaggcagtaaaatcagcctatgacaatgcagagaaacgtctgcagaaagaccagaacggcgctgatatacccgataagggatgcttcctgaacaacattaacgcggtcagtaaaacagactttgctgataagcgtggtatgcgttatgtgcgggttaacgctcctgcaggtgcaacatctggaaaatattaccctgttgttgttatgcgttctgctggctcagtaagcgaactggcatcaagagtcattatcaccacggcaacgcgaaccgcaggcgatccgatgaataactgcgagtttaacggatttgttatgcctggtggctggactgacagggggcgttatgcttatggcatgttctggcaatatcaaaacaatgaacgagccattcactcaataatgatgagtaataagggcgatgatttgcgctctgtgttctatgttgatggcgctgctttccctgtttttgcgtttattgaagatggcctgtcaatatccgcacctggtgctgatctcgttgttaatgatacgacctataagtttggggcaacaaatccggcgactgaatgtatcgcggcggacgttatccttgattttaagagtgggcgtggtttttatgagtctcattcgttaatcgttaacgataacttgtcgtgcaaaaaactttttgccacagacgaaattgtagcgcgtggtggtaatcagattcgaatgataggtggggagtatggtgcattatggcgtaatgatggcgctaaaacttacctgctgcttaccaatcaaggtgatgtttatggtggctggaatacattaagaccgtttgctattgataacgcaaccggcgaactggttattggaaccaaactgtccgcaagtctgaacggtaatgcattaacagcaacaaagctgcaaacgccaagacgggtttctggtgttgagtttgatggttccaaagatattactttaaccgccgcgcatgtggctgcttttgccagaagggcaacggatacatatgccgatgcggatggtggcgttccatggaatgccgaatctggcgcttacaatgtcacccgctctggcgacagctatattctggttaacttctataccggagtcggaagttgccggaccctgcagatgaaggcgcattacagaaatggtggtctgttctaccgttcttcaagagacggttatggttttgaggaagactgggcagaagtttatacctcgaaaaatcttccaccagaaagctacccagtcggcgcaccaatcccgtggccatcagataccgttccgtctggttatgccctgatgcaggggcaggcttttgacaaatctgcttacccgaaacttgcagccgcttatccgtcaggcgtgatccctgatatgcgtggctggacgattaagggcaaacctgccagtggtcgggccgtattgtctcaggaacaggacggcattaaatcgcatacccacagcgccagcgcatccagtacagatttggggacgaaaaccacatcgtcgtttgattacggcactaaatccacgaataacaccggggcacatacacacagtgtgagcggctctacaaactcggctggagcacacacacactcactagccaacgtgaacacggctagtgctaactccggtgctggtagtgcatcaacaagattgtctgttgtgcataatcaaaactatgcaacatcatctgctggcgcacatacccactcactgtccggcactgctgcaagcgcaggtgcacacgcgcatactgtcggtattggtgctcatacgcactccgttgcgattggttcacatggacacaccatcaccgttaacgctgctggtaacgcggaaaacaccgtcaaaaacatcgcatttaactatattgtgaggcttgcataatggcattcagaatgagtgaacaaccacggaccataaaaatttataatctgctggccggaactaatgaatttattggtgaaggtgatgcatatattccgcctcatacaggtctgccagcaaacagtaccgatattgcaccgccagatattccggctggcttcgtggctgttttcaacagtgatgagtcatcgtggcatctcgttgaagatcatcggggtaaaacggtttatgacgtggcttccggcaacgcgttatttatttctgaactcggtccgttaccggaaaatgttacctggttatcgccggaaggggagtttcagaagtggaacggcacagcctgggtgaaggatacggaagcagaaaaactgttccggatccgggaggcggaagaaacaaaaaacaacctgatgcaggtagccagtgagcatattgcgccgcttcaggatgctgcagatctggaaattgcaacggaggaagaaatctcgttgctggaagcatggaaaaagtatcgggtattgctgaaccgtgttgatacgtcaactgcacaggatattgaatggccagcactgccgtagggtaaaacatataaattctataattagatgtatctttccatttacggcaaggaagggggcttggaagacgtaaagcatctcacaccgagattattttttatatgtcaggtgtctgaagttttgctttggctcttaaaatggtttgccgcgaggttttgaattcccgggcaatggcacttatacttacacctgacttaattcgttcgaataccacctgtttctgttcttcatttaacacaggaggtcgaccaaaacgtttccctgcgccgcgggctcttactatcccggaatgagtgcgttcaagtaaaaggtctcgttcaaattcagcgactgctgaaattacttgcatcatcatttttcctgttggactggtcaggtcaatgccacccaatgctaagcaatgcactctgatacctgtttcggtcagttgttccactgttttcctgatatccattgcattacaaccaaggcgatccagttttgtcacaatcaattgatcaccacatttcaggcgagcaagcaaccggttaaaaccaggacgctcactggttgctgctgagccgctaatgtgttcttcgattatttgctgaggtttgattttaaaacctgcactttcgatttcccggcgttgattttcggtggtctgatccagcgttgatatccgacagtaagcaaaaattcgagacatagtgagactctatacgaaattggtgttcatatcataatgcatctcagaaaataattatgattatttttgtgcatatttgtatgtacacgttcgaaaataaacgaatgcgtatgcaaccccgtaattttggtgagacccaaaatcgattttgtgaaaaatggctttaactcggtttgtttttcgagttccgggcggactcaaggaagaagaatagtgttgcgtgttattttaaccagatttcaagttgtttggtcgtggaaaagtggagcaaaatgttgttaaagtggaaaaatgataaaaaagtaagtttattatattacattttaccatttaaattttggttgtctttaagaactgatatcgctgtttgtaataattctttgttatccagccatgatgttttctttatgtttccttcaatgtaatcaagcaatgttctggtattgataggtcttccctgttttgctacttccactacagcatcccctaggataattcttacttcaggaagctgcgcagggaaccactttagggtgtcttttgatttcatgaagatattccttaaaatattattgattttcattgcgatattgtatgtctgattcaggatatgttgacttatacatcggttttgtctgggttattggatatgccaatccctaattttattagagcatgactaaaaatgctgaatatgataaggagcgaagtgattatcagtatgctgttcatatagcctcgaattagtaatgtgttatatatgatatagttgacaatttttatcctgggtgttcttaaagttcgtagataaacattgtcgtttcaggtatacaggaatgctaacaggtggcggcaaaaatcaggcggtttatggcgcaagctgaagtggcaactgcaaactatcttatgcagagactctacacggattgggtttaaaagtatacatagataacagtttttatctgaagaagaaaaatatcaaggtgatatagcctatatgcctttgatgcggaggaatgaatgtgatgggagtgatgtatctgaatagttgaaaaaccgcagtcacgtcgtatgcaagaacgtgctgcggttggtttgactttgattgagacgttttggaatttttttcggtggcaaaaatggggcaaaacgctgcaaaaggggcaaaaaaggggcaaaaaaagagtggattatcgtagcttattgttgtcgctgatgatatttaacacattgaaaaataagtaaaatacttatgagtcagagagttgtgatttttgcccttacttgttcaggttgtattgttctttcttactaatttcttgattttgcgacatttaaaagcgactcaattcgttatatggcatcagaagagtatgcgtcatgccggaacgcccagcataagaaatctgatataaaaaactgtggcgtgtatggtacggattagaggggaaaatgtcagcacatttgcgaaatgaatcaaaaagcccgcagcaatgtgcgggcgttagtgtcagcgcacaaccagcacggagcactctgcgtgacgcactacagctgcggcgttggaaccgagcagataagtggtgatatccggtcgatgggaagcaatgatgatcatatgagcggggatcttcttcgccaattccagaatgcggtctttgggcgagccttcctcaacatggacatgcactctgtcggttggcagtttaaattttttaatgatctcttccagttgcgatttggcttccgctttcaggtcatccattgccggtaattctgcggaatacgctaaacccagagaggcatagtagggcagtgaaggtattaccgtcaggaaatgaacctctgcatcatcaatctttgcctcttcctcaacgtggctaatcacgcgttgagttaattctgaatcggaaatatcgatagggacaagaatcgttctgttcataaaacctcctgttttagtatccgcataaagtgtaacgccagatgacactttttgtgtaatgacggagttcacatttttaatttagatcaaaggaggaagaataagcagaaaaagcccgccataacagcgggcaggaggatttagaactgataaaccagacctaaagcgacaatatcatcggtagagatgccattggcagcgtagaagctgtcatcttcatccaacaggttgattttatagtcaacgtaggtggacatgtttttattgaaatagtaagtcgcgccaatatcggcgtatttaaccagatctttatcatcaacacctgccgggttgtctgcaccacccgcagcgtgcaggtcacggcctttagacatcaggaaagagactgccggacgcagaccaaaatcaaactggtactgtgcagtgacttcaaaattctgggttttgtttgccacagcataatcgctgtcgccaaacggggtcatattacgcgtttctgaatacatggttgccaggtaaatattgttagcatcgtattttagcccagcagtccacgcgtctgctttatcaccacccgccgcagtatggttaacctggtcattggtgcggtcagaagaggtgtatgccgcaccagcgctaaagcccatgcctaaatcatatgttgtggaaagaccccagccgtcaccgttttcatggcgaacatcacgtccgttgttggtgccttcctgaccattactggctccttcgttgttaccttgatactgcaccgcgaagttcagaccatttaccagaccgaagaaatcagtattacgataagtcgcgacgccattggctcgaccagtcataaagttgtctgcattggtataagagtcaccgccaaattcaggcagcatatcggtccagccttcgatgtcgtacattacgccataattacgtccgtaatcgaaagaaccgtaatctgcaaatttcagcccggcaaatgccagacgggtccatgactggttttttgaagattcagtgttgtttgcctgaatattgtattcccattgaccgtagccagtgagttgatcgttaatttgggtttcgcctttaaaacccagacgcgcatagctctggtcgccatctttcgctgaattatcagaaaaataatgcaggccatcaactttgccatacagatctaatttgttgccgtctttattataaacttcggctgcatgtgcagcacctgcggcgagcagggcaggaattaaaagtgccagtactttgcttttcattgaataaatcctttagttattttatttgccttttatccccatttcggggagtgaaaacatcctaaaggagaagttcagttagccgataaatatcatttgttacgccttaagtaaaaccttaatcaaataattcctctgaaatgataataagtctggtgaatgtatcgaagataatacatacaaaataaaaattatacttttaatttgctatacgttattctgcgcgggttatatgcctttattgtcacagattttattttctgttgggccattgcattgccactgattttccaacatataaaaagacaagcccgaacagtcgtccgggctttttttttagaattggataatccttatccagagcatttaatcggtgttgcttttttccgcttttccggccatttgtgccaggaagtcatagcgtttttgcaaatcagctgcagcatctttccataactgttctgccacttctggctgctgcgaattcagccgacggaaacgttgctcgtgaagtaacgtttcttccggtgcttctgacggcgggcgtgaatccaaggccagcggcagtttgccttcatcggcacgacgcggatcaaagcgatatagcggccagaagccggtagctgtgagttggcgcatctggtcgtggctgagtgccagatcgtaaccatgctcttcacacgggctataagcaatgatcagcgatggccccggatacgcttccgcttcctgaatcgctttcaccgtctggttcagctgcgcgccgagagaaatctgcgccacataaacatgaccgtacatcatcatactgacgccaagatctttacgcgctttacgtttgccgtgctcgccaaatttagttactgcacccagcggtgtcgctttcgacgcctgaccaccggtgttggaatagcattgcgtatccagcaccagaatgttgacgttttccgtcaaactcaatacatgatccagaccgccaaagccgatatcgtaagcccagccatcaccaccaatcagccagattgatttttccaccagtgcatctgcatcacgtagcagttcatgtgcttcggcaacatcgttgagttgctggcgtaaagctgcaacctgttcacgacgaacctctggcgtggcgtctgatttcaacgccgtcagtaattccgccgggattttatcggcaaattgatccagcagacgcagcacgcggacacggtgttgatcgaccgtcaggcggaaaccaaggccaaattcggcattatcttcaaatagagagttcgcccatgccggcccacgaccgttggcatcggtggtatacggtgtagagggcaggttaccgccataaattgaagaacagccagtggcgttagcgatcaacatccggtcgccatagagctgagtcagtaatttaatatacggcgtctcgccacaaccggagcaagcacctgaatattcaaacagcggtgtaatcagctgcgatgtacgaatatcaatacgttccagtttgctacggtcgatttctggcaggttgaggaagaaatcgtaattgattttctcttcttcgacatgttccaggcgagacatcatattgatggctttaatctctggattctgacggtctttcgccgggcaaacttcgacgcacaggttacaaccggtgcaatcttccggtgccacctgcaagacatatttctgcccgcgcatatcacgcgatttcacatccagcgaatgcaggctggcaggggcgttttccatcgcttcaggcggcaccacttttgcgcgaatagctgagtgtgggcaagcggcaacgcagtggttacattgggtacagagttcctctttccagatggggatctcttcggcgatattgcgtttttcccagcgcgtagtgcccatcggccaggtgccgtctggcggcagcgccgaaacggggagggcgtcaccaagcccggcgagcatcgcagcggttacggttttcacgaaatcaggggcggcatcggaaaccactggcggtcgattggcgctgtgcggatttaccggttgcaacggaacttcttctacggattcacgcgccagcgccagagcctgccagttgcgttccaccagatcctggcctttgctactgtaacttttggcaatcgcaccctgcaattctgcgagggcgctatcgccaggcagaatttgcgtcagatggaaaaaagccatctgcatgacggtattaatacgggccgccaggccacattcgcgggcgattttcgccgcgttaatcacatagaagcgcgcttttttctggtttaacacggcctgaacttcttgcggcaagcgcgaccacacttcatctgcgctgtacggcgtgttgagcaggaaaatgccgccaggttttaaacgctcagccatctgatatttatcgataaactgcaactggtggcagccaacaaaatcagcctgggaaatgagataagcggaacgaatcggctgttcgctcactcgaaggtgagaaaccgtcaggccgcccgcctttttggagtcgtaaacaaaatagccctgtgcgtaccacggcgtggaattaccgataatcttgatattgtttttggtcgcggaaacgctgccatcactaccaaggccataaaacaaggcttccagtttcgccgagtttggcagggtgttttccggcaacggcagtgacagattggtcacatcatcgtaaataccaaccgtaaagcgcgctttcggtttagccgcgttgagctcggcaaataccgccagtacacagtctgggccaaattctttggatgaaagaccatagcgcccaccaatgacacggggcagagtttcgcgctcgccattattaaaggcttctgccagtgcggtcattacatccagatagagcggttctgcctgggcaccgggttctttggttctgtccagtaccgccacgctgcgtacggatcccggcagagcttgcagtaaatgtttagcggagaaggggcggtacaggcgaactttcagcacgccaactttttcgccacgggttagcaattcatcaaccacttcttcacaggtgccaatggcagagcccatcaggataatcacccgttccgcttgcggatgcccgtaatattcaaacggctgatactgacgacctgtcgcggcagagaaatcattcatcgcctgttcaacatggtcatagaccgcgttgtaccatgggttggtggcttcgcgagactggaaataagtgtcaggattggcggacgtaccgcggatcaccggatgttccgggttgagtgcccgggcgcgatgagcatcaatttcgacctgcggcatgagatcaagaatcgtgtcatcggccagcgggacaattttattgatttcgtgggacgtgcggaaaccatcaaagaaatgaataaatggcacgcggcttttcagcgtcgcgatttgcgaaatgagagcaaagtcttgcgcttcctggacgtttgctgcacacaacatcgcgcaacccgtctggcgcaccgccataacgtcggaatgatcgccaaaaatagagagtgcatgtgtggcaacggtacgtgccgctacatgcaggacaaacggtgttagttcgcctgccagtttgtacagcgtcgggatcatcagcagcaaaccctgcgatgacgtaaacgatgttgaaagggcacccgtctgcaaagcgccatgcacggtagcgatagcacccgcttccgactgcatttcaaccacgcgtggtgtgtctccccaaacgttctttaagccgtttccggcccaggcatcagcctgttctgccatcgtggaactgggggtaatagggtagatggcgataacttcactggtgcgaaatgcgaccgaagcaaccgcgccattaccgtcaatagtaatcatatgacacccttacattgcgcaaatgaggggcgcacgaaattgctgcgcgcccagtagtaatctttcaattttagcaaatggctttcttctgcattttcgcttttgtgtcccccacatcagcgtaatgaatgttttgatcaaacagagggcaaaaaaatagccataaaaaagtaaaaatgcggggcaacgcgcaggacagctctcgacgccgccctctgtgctgcctattatttatggcggtgtcgtttggcttgaagatcagaggaagaaaagatgcgagcagcgttttgggtagggtgtgccgctttattgttgtcggcgtgtagtagtgaacctgttcagcaggcgactgccgcgcacgtagcgccaggtttaaaagcgtcgatgtccagtagtggagaagcaaattgtgcaatgatcggcggttcgctttctgttgcccgtcaactggatggtacggcgattgggatgtgtgcattacccaacggcaaacgctgtagcgaacagtcacttgccgccgggagctgtggcagctattaattcattaaatccgccagcttataagttaatgtctgttttgcggtcgccagcgttaactggttcgcggtcagatccacttgtgcaccttctttcagcatttcgctaatggtgttatcgagttcattaagctgcgggttagcgcacatcatacgggtcattgccagccctttggctgtcagttcaccattagacagtttgccttcaccgctaaagcggttacacatgctgccggaaatcatcattttttcaccaaagctgatttctggcggatttttatcgctggtcacgggcttaccgtttacgctttccagcacaaagcgatgatgctgtagctgttctggcgtaacagcaattttgtcattacttacacatcccgccatcagcaggcttagcgcaacaaacgcggctactttcttcattgtggttctcaattacagtttctgactcaggactattttaagaatagaggatgaaaggtcattggggattatctgaatcagctcccctggaatgcaggggagcggcaagattaaaccagttcgttcgggcaggtttcgcctttttccagattgcttaagttttgcagcgtagtctgagaaatactggtcagagcttctgctgtcaggaatgcctggtgcccggtaaacagcacgttgtggcaggcagacaggcgacggaatacgtcatcctggatcacgtcgttggatttatcttcaaagaatagatcgcgttcgttctcatacacgtccatacccaacgaaccaattttctgatttttcagcgcttcaattgctgcctgagaatcaatcaatgcaccgcgactggtattgacgatcatcacgccatttttcatctgttcgaaggcggcttcgttcaacagatgatagttttccggtgtcagcgggcagtgcagagagataacgtctgattcagagaacagggttggcagatcgacatactccacaccgagttccagcgccgctgcacttggatacggatcgaacgccagcagacgcataccaaaacctttcagaatgcgcagcatcgccacaccgattttaccggtaccgataacgcctgccgttttgccatacatagtaaagccggtcagaccttccagagagaagttagcatcacgggtacgctgatacgcgcggtgaatacggcggttcagcgtcatcatcataccgatggcgtgttcagcaacggcctctggatcataggctggaacacggactactttcagccccagttcttttgccgcgtcaaggtcgacgttattgaaaccggcacagcgcagggcgatatatttaacgccgtgctttttcagctcttccagcaccgggcggctgccgtcatcgtttacgaaaatacataccgcttcgcagccattggcagttttagcggttttttccgtcagcagaaagtcaaaaaattccagctcaaagccaaaggactcgttcacctgttgcaggtacttcttgtcgtactgttttgtgctataaacggcgagtttcataagactttctccagtgatgttgaatcacatttaagctactaaaaatattttacaaaatttcaaatttaattgaaagctatggcgatattgaaaaattcatcaacaactatgcttagtgtaggcgcaaccttcaactgaacggttaaacatgccacaatacccgtattgaatgcttaatttttcgctaaatcaggatattaactacccatgctgggtaaatataaagccgttctcgcgctgttattactgattattcttgtgccgttgacgctgctgatgacgctcgggctgtgggttcccacgctggcgggcatctggctaccgctcgggacacgtattgcattagatgaaagcccacgcattacgcgtaaaggtttaatcattcccgatctccgttatctggtgggagattgtcagcttgcgcatatcaccaacgccagcctttcacatcccagccgctggttattgaacgtcggcacggtagaacttgattctgcttgtctggcgaaattgccgcagacggagcaatcgccagccgctccaaaaacactcgcgcagtggcaggccatgctgcctaacacctggatcaatatcgataaactgattttttctccctggcaggaatggcagggaaaactctctctcgcattaacctctgatatccagcaactgcgttatcagggcgaaaaagttaaatttcaaggccagctgaaagggcaacaacttacagtcagcgaactggatgtcgtcgcgtttgaaaatcagccgccggtaaaactggtgggggaatttgctatgccgctcgtgccggatggacttcctgtaagtgggcatgctactgcgacgttaaacttgccgcaggaaccgtcactggtggatgccgagctggactggcaggaaaatagcgggcaattgatcgtgctggcacgggataacggcgatccgttgctcgatttgccgtggcaaattactcgtcaacaattgaccgtaagcgatggtcgctggagctggccgtatgcaggttttcctttgagtggccgactgggtgtcaaagtcgacaactggcaggcagggcttgagaacgctctggtcagcggacgactgagtgtgctgacccaggggcaagcgggtaagggcaacgcggtgcttaattttggcccaggaaaattaagcatggataacagtcagctgcctctgcagctgaccggtgaagcgaaacaggcggacctcattttatatgcccgtttacctgcgcagctaagtggaagtctgtctgacccaacgctgacctttgagccaggcgcgttacttcgttcaaagggaagagtcatcgattcgctggacatcgatgaaatccgctggcctttagcgggtgtaaaagtcacccaacgtggtgttgacggacgtttgcaggccatcttgcaggcgcatgaaaatgaactgggcgatttcgtgctgcatatggatgggctggcgaatgattttctccctgacgctggccgctggcagtggcgctactggggaaaagggagttttacaccgatgaatgccacctgggatgtcgcaggaaaaggtgagtggcatgacagcacgattacgctgaccgatctctccaccggtttcgaccagttacaatacggtacgatgacggtagaaaagccgcgattaattctcgacaagcccatcgtctgggtacgtgacgcacagcatccctcctttagcggcgcgctgtcactggacgccgggcaaacgctgttcactggcggcagtgtgttaccgccatcaaccttaaaatttagcgtcgatgggcgcgatcctacctatttcctctttaaaggcgatttacatgctggtgagattggcccggttcgggtaaatggtcgctgggacggtattcgtctgcgcggtaacgcctggtggcctaaacaatcactgaccgtattccagccgctggtgccacccgactggaagatgaacttacgcgatggtgaactgtatgctcaggttgcattttctgctgcgcctgaacaaggattccgcgcgggaggacacggcgtgttgaaaggcggtagtgcctggatgccagataatcaggttaacggtgtcgattttgtcctgcctttccgttttgccgatggagcctggcatctggggactcgcggccccgttacgttgcgaattgccgaagtgattaatctggtgacagcgaaaaatattacggctgatttgcaagggcgttatccgtggactgaagaagaacccttgctgttgactgatgttagcgtcgatgtgttaggcggtaacgtactgatgaaacaattacgtatgccgcaacatgacccggcgctgttgcggctgaataatctctcatccagcgaactggttagcgccgtcaatccgaaacaattcgccatgtccggggcatttagtggtgcactgccgttatggctgaacaatgaaaaatggattgtgaaagatggctggctggcgaatagcgggccgatgacattgcgactggataaagacactgcggatgcggtggtaaaagacaatatgactgcgggttcagcaattaactggttgcgctatatggaaattagccgttcatcgacaaaaattaatttagataatctcggtttattaaccatgcaggccaacattacaggtaccagtcgcgttgatggtaaaagcggtacggtaaaccttaattaccatcatgaagagaatatttttacgctgtggcgcagtttacgctttggcgataatctccaggcatggctggagcagaacgcacgtctgccgggaaatgactgtccgcaaggaaaagagtgtgaggaaaaacaatgaaaattttactggctgcgttgacgtcatcttttatgctggttggctgtacgcctcgcattgaagtcgctgcacctaaggaaccgatcactatcaatatgaacgttaaaattgagcatgagatcatcatcaaggcagacaaagatgtcgaagagctgcttgaaactcgtagcgatcttttctgaggtgatgatgaagaaaacattacttctttgtgcgtttcttgttgggctggtaagcagcaatgtaatggcattgactctggatgaagccagaactcaggggcgggtaggtgaaacattttacggttatctggttgcgctgaaaacggatgctgaaacagagaaattagtagccgacattaatgccgaacgtaaagcgagttaccaacaactggcaaagcaaaataatgtgtcggtagatgatatcgcgaaactcgccgggcaaaagctcgtagctcgggccaaaccgggggaatatgtacaagggataaacggtaaatgggtgcgaaaattttaatagcaaaaccgcaatatcgggataacgctacaggagaaggcgattgatctattttcctgaaacaaggtgaatattcaaaaactcctgtcaaattgccttttgccctgaaaaatgcatagtcaaatatctgttttaactaattggcgttgcagtacatgcaacgccaattagttagcggaatttacgtcgatactcgcctggcgtcatcccaaagcgttgcttaaataccgttgaaaaatgactctggtcagaaaatccccaatgaaagccgatgcctgccagtttttcatcatctgcggcatggcgaatcgcatctgcacaaaaatcgagacgacggttacgaatatattgcgcgactaccaaacctttatcggcaaacattcggtacaaactacgtactgacatacctgtctctccggctatccactccgggcgtaatatctcttcgcgaatattatcgtctatcaacgtaaccactttttgaaactgacgttcacgacgaggttgaacagattcccgctgatgaagtaccgggcgcagcagacacaccatcgcctgtagcgcagcttcactttctgtttcagaaagtgccggattattcatgctctcctgtaacaggcgatgactgagttgcaccatgggtaagtcagcgtccagtctttctgcgcagataggtttttgatggggaaaatattgttccagcagagtgcgtggcaaaagtaatgaaatctgtttagaagactcctgccagtaaagcgaacaggggcgtgaggcatcgagtaacgtaatatcgccagcgccaatctgcacctgacgctcatcctgctccattattgcctgaccactaagctgaaaaacggtgtaaaaccaggcatcgtcgctgccttttacttcctgccaggtgcgggataaattcaccccgctggttgtcacggtactcagctttagtcctttggcaaaatgcgtgtccagtacacccgtgtaacgctcagtcagcaggcgtccggtaaaatttccgcatacctgattgatttgggaaagccattgctgaaactcattatccactgcggggttcatggcacgttttcgctctgtgaaatgtatttttattgttgcatttgtgttgcaataaacgaagctaatgagcctgactataggaaataagtcttgtcaggcatagagacataagcggttattgtcacgatttgcggagcttgtcacagctgacaaagcgaatgtcacagcgaaaaaagtgacttttcttgtcgctgcgtacactgaaatcacactgggtaaataataaggaaaagtgatgacagagccgcatgtagcagtattaagccaggtccaacagtttctcgatcgtcaacacggtctttatattgatggtcgtcctggccccgcacaaagtgaaaaacggttggcgatctttgatccggccaccgggcaagaaattgcgtctactgctgatgccaacgaagcggatgtagataacgcagtcatgtctgcctggcgggcctttgtctcgcgtcgctgggccgggcgattacccgcagagcgtgaacgtattctgctacgttttgctgatctggtggagcagcacagtgaggagctggcgcaactggaaaccctggagcaaggcaagtcaattgccatttcccgtgcttttgaagtgggctgtacgctgaactggatgcgttataccgccgggttaacgaccaaaatcgcgggtaaaacgctggacttgtcgattcccttaccccagggggcgcgttatcaggcctggacgcgtaaagagccggttggcgtagtggcgggaattgtgccatggaactttccgttgatgattggtatgtggaaggtgatgccagcactggcagcaggctgttcaatcgtgattaagccttcggaaaccacgccactgacgatgttgcgcgtggcggaactggccagcgaggctggtatccctgatggcgtttttaatgtcgtcaccgggtcaggtgctgtatgcggcgcggccctgacgtcacatcctcatgttgcgaaaatcagttttaccggttcaaccgcgacgggaaaaggtattgccagaactgctgctgatcacttaacgcgtgtaacgctggaactgggcggtaaaaacccggcaattgtattaaaagatgctgatccgcaatgggttattgaaggcttgatgaccggaagcttcctgaatcaagggcaagtatgcgccgccagttcgcgaatttatattgaagcgccgttgtttgacacgctggttagtggatttgagcaggcggtaaaatcgttgcaagtgggaccggggatgtcacctgttgcacagattaaccctttggtttctcgtgcgcactgcgacaaagtgtgttcattcctcgacgatgcgcaggcacagcaagcagagctgattcgcgggtcgaatggaccagccggagaggggtattatgttgcgccaacgctggtggtaaatcccgatgctaaattgcgcttaactcgtgaagaggtgtttggtccggtggtaaacctggtgcgagtagcggatggagaagaggcgttacaactggcaaacgacacggaatatggcttaactgccagtgtctggacgcaaaatctctcccaggctctggaatatagcgatcgcttacaggcagggacggtgtgggtaaacagccataccttaattgacgctaacttaccgtttggtgggatgaagcagtcaggaacgggccgtgattttggccccgactggctggacggttggtgtgaaactaagtcggtgtgtgtacggtattaatctggttcgctcataagtaaaaaacggcacctggtgccgtttttttgtctgaaacaatcacttatctttcttcagcgcccctagcgttggcgtttcgtcaaagaagttccatggtttcagcagagtatgtacccattcggtcggcataatcggccactcttcggcgcgggccacatgtgtggtgccggtggtcatccagacaacggcgtcggtgttgtccagcgactcgttatccttactgtattgtccaagaccggtgtcatgagtagaacggttcggatatttgccttccgggaaacgctcgccaggatgataacgcgttacccagagctgcttgtccataaagcttaaacgatgatagatccactcgtccggcgcgaactgggcaccttttgctaccgggtgagtaccacctgcataaggaataatttgataggaaaccggattgcccatgcggttctctttgttcgggttactcaacagacgaatcgtgcccggatcaaatttctgtgcggcatcctgttcattgccgatgttgtactgattaacttgcatggtactggtgcgtgggccaccggcagtattcggttttaccactgggtccatcgccaccaggctgttattctcgccatctacatccagatcgaggcggaaattataaatatgttggtgtgtagtacccacgatattgtgatcgataagcgtgccgtagcgcgtgtcatctttcgccgtctcatcgtgcatggttttcgctttaacacctttcaccgcttcgatgcccgtagcaccggcatcgatgccaatagtgccgttttcatggaagatccagtcaaaaatgtagtcatagttacccactgtactgatccagcgcaccactaactcccggcgttcggtactgacgttgggctggcccatttcctgatgcttatactccggcccggcataacgttcaaataccgcgatagcgcgagggatctccatcggcacgccagtgtagtcggcgatggtttcattaaggagcactgcgttagacggggcatctttaccacgagcaattggtgaggttagcgtgcccataccgtagtcaccagagtccagatacgctttaaagtaccagccaatatcaggatcaccgtaaggcacaatcatgccgccgagagaaccttcgtacatgactttgcgtttggtgccattgtcgttataagtcacggtggagatcatcggcccgacgcgagagttcatgctgaggtgaaaatcccagttccgccagtgaatcatatcgccagtaatggtgtaatttttaccttcaggctcaatgatttgcataggcttaactgccggagcaacgcggtcacggccatcaaatgggcgtgcggtcattggcaccggaactaccggaccttcttcaatcttaacgatttttttctgttctaaatcaacgaccgccaccaggttttcgatgggatgtgcccagtagttgccatcaccgacatcaagatagctgatgactttgagcaaccgggcatcttgtttcaggccatctttaccatcgaaataacctacggtcagcggcgtggtaatcacttttttcgcatcagtaataccgcgtttcttcacggcagcggcaaattcttcactgttgttaataatgttctgcacactggcgaaatcatccagcaacaccataccgtgggcgtctttaatgggttgccaggagagcagtttgttgttttgcagatccaccaccgcttcgatgatatgtttgccgtcgagcataatgacgtcggctttgcgcggctggtcaaccggtttgttttccagcgcaaacgcccagacagcttctttatctggcggtagcagggagatctcagtaaaacgggtattgggtttgaagtccgcggaagctttaacaatttcaacggcctgtttaatttcgtccgcagttagcgcattaagtgggtgagggcgcttttctacctgaaaggtttgatccagcccggactggaaaacatcgttaataaaggtgtcagaaacccaggctttattgtctttcatcactaccggtacttgcagtgccagaggctgaccattaacaattgctgtttgcgcaccaggcttcactttcacgtacgcgccatctttaatcagggtaaagagctgggcgtagtcgtcccactgcacatcggcaccaaattctttaagcgttttatccattggcaccatatgcgcttcaccaccgtgggcaaataccggcgcttgccaggcgaaacttaaggcgactgccaacgccagggttgttttacgggcagaatacagagaggggcttcccattattaacctcgtcagatgttgtgttcttgttagcaaccgcgctctgtgggcggtttagtcaggttcacattatcagtactgatgcaaaggggattgcctgcacctgccaggttgtttggcaggtgtgccagcttttcatacagtggatgccctgaaaatagatgtacacatcatgcataatgtgacaacgtcacaaaacttagtgaaataaaagggcaactattcgccgttgcccttcattcaccgattaatcgacaaaatcaccgtgctgcctggccaccagcgtcagaattgaatacagcgccaccggggtttgatgctgattgaatacctctacagcccattccaccacacctgttggtttttcttctgcgctacgctgttttttcagcgtcttgcgcttacaggtgagacgcacctggatggtatcgcctggctttacgggttcgataaaacgcaagctttccagcccgtagttagcaatgaccggaccgacaccggcatcgacaaacagacccgcagccgcagaaagcacaaaatacccatgcaccacccgctcaccgaaaatagattcggcagcagcaatcttatccatatgtgcatagaaatgatcgccgctgaggcaagcaaagttaacaatatcggcctctgtcattgtgcggcggggagtcaacaggctgtcgcctggttgtagctcctcaaaatatttgcggaacggatgaatacgatcttcttcgactttcgcaccgcgcacccactgtttactgatagcggcaagcatcgtcggactaccctgaacagcggttcgctgcatgtaatgtttcaccgctcgtaaaccgcctaattcttcaccgcctcctgcgcgaccaggcccaccatgtaccagttgtggcagtggggagccatgcccggtggattcttttgccgactcttcattgaggatctgaattcgcccatgcgtacgtgccgcgtcggcaataaactgacgcgcaatttgcggatcagccgtcaccagcgttcccgcaaggctaccgccgcctgcacaagccagttgcagagcatgtcgctggttttgtgctggcatcagcgttgcgacagggccaaaggcttctgttgcatgtaccgccggtgtttcatccggctgcggacagtacaataaggttggcgggaagaaggcacccgcagcagataaatccgcctgaccaccgaggcgaatctcgcatcctgcagccagcaatatgttcactttttcctgcacatcggcacgctgctcagcatttaccagtgcgcccattttcacgccttcctgagcaggatcaccgaccacgactttctgtaatcgcgcaaccagagcatcactgacagcattaaccaatgcctgcggcacaataatccgccggattgccgtacatttttgcccggcttttgtggtcatctcacgcacaacttcacgaataaacagcgcaaactccggttgatccggggtgacatcttcgcccagtacgcagcagttcagggaatcagcttccatagtgaaggggatagatttggcgacgatatttggctgaactcgcagcatctgtccggtcgccgctgaccccgtgaaagtcaccacatcctggctgtccagatgatccaacaagtcgccagcactaccgcagatcagactaattgcgccttcgggaacaagaccactatcgacaattgatttcaccatcgcctgagtcagttgggccgtcgcggtagctggtttgatgatggctggcattccgcccagccacgttggtgccagcttttccagcattccccagcaggggaagttaaaggcgttaatatgcactgccacgcctgactttgaggtcagtaaatggcgcgcggcaaatccaccttctttcgataaggggatcaattcatcttccggccacagcgtatcgtcaggcagctcccggctaccgaggctggcgtaagtaaataacgtcccaatgccaccttcaatatcaacccaactgtctgcccgcgttgcgcctgtttgcgcagaaagagcatagaaacgctctttttcactcagcagatgtttagcgaccgctttaagcatcgccgcacgttcgataaaggtcatagcgcgaagggcgggggcacctttttcaatggcaaactggcgggcagccgccatatcaagaccttcactggtcacttcccataacgcctcgccgctaatagcgtggtgaatcaaacggctacggccccggccagactgccaggtaccggataagaaactggctaactgctgcatcgctactctccagatgtttcacatttctgttgctaatagttaaatcgcgaatcataaaaagcaaaggatcttttaacgaaatgttaactatgcgatctgtatagcaactgcggaaaacattaatgcactgataaataatgatttataaaaatagggtgcgaaatccgtcacagttcaaacatacaaaatttgtgattttacttaactattgtgtaactttcataaaacaatgtgattcgtgtttttaattaattcacgaaaactggaatcgtaaaggtgatgacgtgacccaagaagaacgctttgagcaacggatagcccaggaaacggctatcgagccacaggactggatgcccgatgcttaccgaaagacattgatccgccagattgggcagcatgcgcactccgagattgttggtatgttgcctgaaggtaactggatcactcgcgcaccaaccttgcggcgtaaagccattctgttggccaaagtgcaggatgaagccggtcatggtctgtatctctatagcgccgccgaaacactgggctgcgccagagaagacatctaccaaaaaatgctcgacggacggatgaaatattcctccatctttaattatccgacattgagttgggctgatatcggtgttatcggctggctggtggatggcgcagcgatcgtcaatcaggtggcgttatgccgcacttcttatggcccgtatgccagagcaatggtgaaaatctgcaaagaagagagttttcaccagcgtcaggggtttgaagcctgcatggcactggcgcagggcagcgaagctcaaaagcagatgttgcaagacgccattaaccgtttctggtggccagccttaatgatgttcgggccaaacgatgataactcgccaaacagcgccagaagtctcacctggaaaatcaaacgtttcaccaacgacgaactccgccagcgtttcgtggataacaccgttccacaggttgaaatgctcggtatgaccgttcctgacccggatctgcattttgacactgaaagcggtcactaccgctttggtgagatcgactggcaggagtttaacgaagtaattaacggtcgcggaatttgtaatcaggagaggctcgacgccaaacgtaaagcctgggaagaaggtacctgggtacgggaagcagcgctggcccatgcacaaaaacaacatgcccgtaaggtcgcataaggagattcaaaatgagtaatgtttactggccgttatacgaagttttcgtgcgtggcaaacagggcttatcacaccgccatgttggcagtttacatgctgccgatgagcggatggcactggaaaatgcccgtgatgcttacacccgtcgtagcgaaggatgttcaatttgggtggtgaaggcgagtgaaattgttgcctcgcaaccggaagaacgcggtgaattttttgatccggctgaaagcaaggtctatcgccatccaacgttttacaccatccctgatggcattgagcacatgtgaggtcggaaatgaatcagttaacggcttacaccttgcgcctgggcgataactgcctggtgctctcccagcggttgggtgaatggtgcggtcacgcaccggaactggaaatcgatctcgcactggcaaacattggcctcgatttattaggtcaggcacgcaacttcttatcgtatgccgctgaattagcgggagaaggcgatgaagataccctggccttcacccgagacgagcgccagttcagcaacttattgttggttgaacaaccaaacggcaattttgccgacaccattgcacgccagtatttcatcgatgcatggcatgtggcgctctttacccgtctgatggaaagccgtgatccgcaactggcggcgatttctgccaaagcaattaaagaagcgcgctatcacctgcgttttagtcgtggctggctggagcgactgggcaatggtactgacgtatcagggcaaaagatgcagcaggccatcaacaagttgtggcgttttaccgccgaactgttcgatgccgacgagattgatattgcactgagtgaagagggtattgcggttgatccacgcactttacgcgcagcgtgggaagccgaagtttttgccgggatcaacgaagccacattgaacgtaccgcaagagcaggcgtatcgcactggcggtaaaaaaggactgcataccgaacaccttggacccatgctggcagaaatgcagtatctccagcgtgtcttgcccggtcagcaatggtaacagaggagatgggtatgcaacgtctggccaccattgcaccgccacaggttcatgagatatgggcgctactcagccagatcccggacccggagatcccggtgctgaccattactgatttaggcatggtgcgtaatgtgacacagatgggagaaggatgggtgatcggctttacgccgacatattccggttgtccggcaacggaacatttgattggcgcgatacgtgaggcaatgacaaccaacgggtttacccccgttcaggttgtgctgcaactcgacccggcatggaccaccgactggatgacccccgatgcccgtgagcgtctgcgagagtatggcattagcccgcccgccggacacagttgccatgcccatttgccgccagaagtacgttgcccgcgctgcgccagcgtccataccacacttatcagtgaatttggttccacggcctgcaaagcattgtaccgctgcgatagttgccgcgaacctttcgattatttcaaatgtatttgaggatgccatgacaacgtttcattccttaacagtggcaaaagtcgagtcggaaacccgtgatgcggtgaccattacctttgcggtgccccagcctttgcaggaggcgtatcgctttcgccccggtcaacatttgaccttaaaagccagctttgatggtgaagaattacgccgttgttactccatttgccgcagctatctgcctggcgaaattagtgtggcggtgaaagccattgaaggcggacgtttctcccgctatgcccgcgaacacatccgccagggtatgacgctggaggtcatggtgccgcaggggcatttcggctatcagccgcaggccgaacgccaggggcgctatctggcaattgcagcaggatcaggtattacgccaatgctggcgattatcgccaccactttacaaaccgagcctgaaagtcagttcaccctgatctacggtaaccgtaccagccagagcatgatgtttcgccaggcactggcagacctgaaagacaaatatcctcagcgtttacagttgttgtgcattttcagtcaggaaaccctcgacagcgatctgcttcacgggcgtattgacggtgaaaaattacagtcacttggggcctcgctcattaattttcgtctttatgatgaggcatttatttgtggtccggcggcgatgatggatgacgcggaaaccgccttaaaagcactgggaatgccagataaaaccattcatctggagcggtttaatacgcctggcacgcgcgtcaaacgtagcgttaacgtgcaaagtgacggacaaaaagtgactgtacgtcaggatgggcgggatcgggaaatcgtgcttaatgccgacgatgaaagcattctcgatgcggcattgcgccagggggcggatctgccctatgcctgcaaaggcggcgtctgtgcgacctgcaaatgcaaagtgctgcgtggcaaagtggcgatggaaaccaattacagtctggaaccggatgaactggccgcaggttatgtgttgagttgccaggcactgccgctgaccagcgatgtggtggttgactttgacgcgaaggggatggcatgagcgaactgatcgtcagccgtcagcaacgagtattgttgctgacccttaaccgtcccgccgcacgtaatgcgctaaataatgccctgctgatgcaactggtaaatgaactggaagctgcggctaccgataccagcatttcggtctgtgtgattaccggtaatgcacgcttttttgccgctggggccgatctcaacgaaatggcagaaaaagatctcgcggccaccttaaacgatacacgtccgcagctatgggcgcgattgcaggcctttaataaaccacttatcgcagccgtcaatggttacgcgcttggggcgggttgcgaactggcattgttgtgcgatgtggtggttgccggagagaacgcgcgttttgggttgccggaaatcactctcggcatcatgcctggcgcaggcggaacgcaacgtttaatccgtagtgtcggtaaatcgttagccagcaaaatggtgctgagcggagaaagtatcaccgctcagcaagcacagcaggccgggctggttagcgacgtcttccccagcgatttaaccctcgaatacgccttacagctggcatcgaaaatggcacgtcactcgccgctggccttacaagcggcaaagcaagcgctgcgccagtcgcaggaagtggctttgcaagccggacttgcccaggagcgacagttattcaccttgctggcggcaacagaagatcgtcatgaaggcatctccgctttcttacaaaaacgcacgcccgactttaaaggacgctaatgatggaattcatcctcagtcatgtagaaaagggcgtgatgacactaacgctcaaccgcccggaacgcctgaacagttttaatgatgagatgcacgcacaactggcagagtgcctgaaacaggtcgagcgcgacgacactatccgttgcctgttacttacaggtgccgggcgcggattttgtgctggtcaggatcttaacgatcgtaacgttgatcccacaggccccgcaccggatttagggatgtcagttgaacgtttctataacccactggtacgtcgcctggcaaaactgccaaaaccggtgatctgtgcagtcaatggcgtggcggcaggggcaggcgcaacactggcactggggggcgacatcgttattgctgcccgttcagcaaaattcgtcatggcgtttagtaagttaggcttaatacccgattgcggtggaacctggttactgccacgcgttgccggacgagcgcgcgccatggggctggcactgctggggaatcaactgagtgctgaacaggcgcacgaatgggggatgatctggcaggttgttgatgatgaaacgctggcagataccgcgcaacagctggcacggcatctggcgacacaaccgacatttggtcttggacttatcaagcaagcgataaatagcgctgaaaccaatacgctcgatacgcaactggatctggaacgtgactatcagcgacttgccggacggagcgcagattatcgtgaaggtgtcagtgcgttcctggctaaacgctcaccgcagttcacggggaaatagcatgatgataaatgtgcaaactgtggcagtgattgggagcggcaccatgggggcaggcattgctgaagttgctgccagtcatggacaccaggttttactgtatgacatttctgctgaagcgctgacccgcgcaatcgacgggatacacgcgcggctaaattcacgcgtgacgcggggaaaactgactgctgaaacctgtgaacgcacattgaaacgcctgatcccggtgaccgatattcacgcgctggcagctgcggacctggtcattgaagcggcgtctgaacgtctggaagtcaaaaaagcgctctttgcacagctggcggaagtttgcccgccacaaacgctattgaccactaacacttcgtcaatctctataaccgcgattgctgcggagataaaaaatcctgaacgtgttgcggggctgcatttttttaacccggcaccggtgatgaagttggtggaggtggtcagtgggctggcaacggcggcggaagttgttgagcagttgtgtgaactaacgttgagttggggtaagcagcctgtgcgctgtcattcgactcctggatttatcgttaaccgtgttgcgcgtccttattattccgaggcctggcgggcactggaagagcaggttgctgcaccagaagtgattgacgctgcacttcgcgatggcgctggtttcccgatggggccgctggaattaaccgatctgattggtcaggacgtcaattttgctgtcacctgttcggtgtttaacgctttctggcaggagcgtcgttttttaccttcgctggtgcaacaggaactggtgattggtggacggttgggcaagaaaagtgggctgggcgtgtacgactggcgcgcggaacgtgaggcagttgttggcctggaagcggtaagcgacagttttagcccaatgaaagtagaaaagaaaagtgacggtgtcacggaaattgacgatgttttattgattgagacacaaggcgagacggcacaggcgctggcaatacgactggcacgcccggtggtagtgatcgataaaatggcgggcaaggtggtgaccattgctgctgcagcggtgaacccggactcagcgacccgcaaggccatttattacctgcaacagcagggcaaaacagtgctgcaaattgcagattacccaggaatgctgatttggcgaacggtagcaatgatcatcaatgaagcccttgatgcgcttcaaaaaggcgtggcctctgaacaggatatcgataccgccatgcgtcttggggtgaattatccatatggcccacttgcctggggagcgcaacttggctggcagcgaatattaaggctccttgaaaatctacagcatcactatggcgaagaacgctatcgcccatgttcattgctgcgccaacgggcgcttctggagagcggttatgagtcataaggcctggcaaaatgcccatgcaatgtatgagaacgatgcctgcgccaaagcgcttggcatcgacattatctcaatggatgaaggctttgctgtagtgaccatgaccgtcactgcacaaatgcttaacggtcatcaaagttgccacggcgggcagctattttcactggctgatactgcctttgcctacgcctgcaatagccaggggctggcagccgtcgcttctgcctgcacgattgattttttgcgtccaggctttgccggagacaccttaactgctactgcgcaggtacgtcatcagggcaagcaaaccggtgtttacgacatcgaaattgttaaccaacaacaaaaaacggttgcgctgtttcgcggtaaatctcaccgcatcggcggcaccattacaggagaagcctgatgcgtgaagcctttatttgtgacggaattcgtacgccaattggtcgctacggcggggcattatcaagtgttcgggctgatgatctggctgctatccctttgcgggaactgctggtgcgaaacccgcgtctcgatgcggagtgtatcgatgatgtgatcctcggctgtgctaatcaggcgggagaagataaccgtaacgtagcccggatggcgactttactggcggggctgccgcagagtgtttccggcacaaccattaaccgcttgtgtggttccgggctggacgcactggggtttgccgcacgggcgattaaagcgggcgatggcgatttgctgatcgccggtggcgtggagtcaatgtcacgggcaccgtttgttatgggcaaggcagccagtgcattttctcgtcaggctgagatgttcgataccactattggctggcgatttgtgaacccgctcatggctcagcaatttggaactgacagcatgccggaaacggcagagaatgtagctgaactgttaaaaatctcacgagaagatcaagatagttttgcgctacgcagtcagcaacgtacggcaaaagcgcaatcctcaggcattctggctgaggagattgttccggttgtgttgaaaaacaagaaaggtgttgtaacagaaatacaacatgatgagcatctgcgcccggaaacgacgctggaacagttacgtgggttaaaagcaccatttcgtgccaatggggtgattaccgcaggcaatgcttccggggtgaatgacggagccgctgcgttgattattgccagtgaacagatggcagcagcgcaaggactgacaccgcgggcgcgtatcgtagccatggcaaccgccggggtggaaccgcgcctgatggggcttggtccggtgcctgcaactcgccgggtgctggaacgcgcagggctgagtattcacgatatggacgtgattgaactgaacgaagcgttcgcggcccaggcgttgggtgtactacgcgaattggggctgcctgatgatgccccacatgttaaccccaacggaggcgctatcgccttaggccatccgttgggaatgagtggtgcccgcctggcactggctgccagccatgagctgcatcggcgtaacggtcgttacgcattgtgcaccatgtgcatcggtgtcggtcagggcatcgccatgattctggagcgtgtttgagcatatcaacctgcgagtaccctacaatgataaccaatacaaagcttgacccgattgaaaccgcgtctgttgatgagttacaggcgttgcaaacacagcgtctgaaatggacgctcaaacacgcgtatgaaaatgtgccgatgtatcggcgcaaattcgacgcagcaggcgtacatcctgatgatttcagggaactttcagacctgcgtaaatttccctgtaccaccaaacaggatctgcgcgacaactatccctttgacacctttgccgtgccaatggaacaagtggtgcgcattcatgcttcttcgggaaccacaggtaaaccgacagttgtcggctatacgcaaaacgatattgataactgggccaatattgtagcgcgttctttgcgtgcggcagggggctcgcccaaagacaaaattcatgttgcctatggttacggcctgtttactggtgggctgggtgcgcactatggtgccgaacgtctgggcgctacggtgatcccgatgtctggcgggcagacggaaaaacaagcgcaactgatccgtgattttcaaccagatatgatcatggttacgccatcttattgccttaacctgattgaagagctggagcggcagttgggcggtgatgccagcggttgctcgctgcgggttggagtatttggtgctgagccgtggacacaggccatgcgtaaagagattgagcgtcgcctggggatcaccgcactggatatttatggcctgtcagaagtgatggggccgggggtggcgatggagtgtctggaaactaccgacggcccaaccatttgggaagatcatttctatcctgaaattgttaatcctcatgacggcacaccgcttgccgatggtgaacatggcgaactgttattcaccacgctgaccaaagaagcattgccggtcattcgttaccgcacgcgtgatttaacccgactgttaccaggaacggcgcggactatgcgccgcatggatcgcatcagcggacgcagcgatgacatgttgattattcgcggtgtaaatgtctttccgtcacaactggaagaagagattgtcaaattcgaacatttatcgccgcattaccaactggaggtgaaccgccgggggcatcttgattcactttctgtgaaagtggagttgaaagaaagtagcctgacattgacgcatgagcagcgttgccaggtatgccaccagctgcgccatcggattaagtcgatggtggggatctctaccgatgtgatgatcgttaactgtggcagtatcccgcgttcagaaggcaaggcgtgtcgggtgtttgatctgcgcaatattgttggtgcctgacgtatcgtctggccctggtggggtaaagcgccagggccagaagtcgatacgacctgtgctatgattcataaatcacaacaataacaacagactgaagcgaatgagtaaacttgatacttttatccaacatgctgtaaacgctgttccggtcagtggcacatctttgatctcctctctgtatggtgattcgctttcccatcgtggtggtgaaatctggttgggtagtctggctgctttgctggaagggctgggatttggtgagcgtttcgtgcgcaccgctttgtttcgtcttaataaagaaggctggctggatgtttcccgcatcgggcgacgcagtttctatagcctcagtgataaaggcttgcgcctgacgcgacgggcagaaagtaaaatttatcgcgcagagcaacctgcatgggatggtaaatggctcctgttgctctcggaaggtttagataaatcaacgctggctgatgtcaaaaagcagttgatctggcaaggttttggcgcactggcacccagcctgatggcatcgccgtcgcaaaaactggccgatgtacagacacttttgcatgaagcgggtgtggcggataacgtgatttgttttgaagcgcaaataccactggcgctttctcgcgcagcactgcgtgccagagtagaagagtgctggcatttaactgaacaaaatgccatgtacgaaacctttattcagtcattccgcccgctggtgccgcttttaaaagaggcggcagacgagttaaccccggagcgggcatttcatattcagcttttactgatccatttttatcgccgtgtcgtccttaaagacccattgttgccggaggagttgcttccggcacactgggcagggcatacggcgcgtcagctgtgtatcaacatttatcagcgcgtagcgcctgctgctttagcgttcgttagtgaaaaaggtgaaacctcggtcggtgaactgcctgcgccgggaagcctgtattttcaacgttttggcggcttgaatattgaacaggaggcgttatgccaatttatcagatagacggtctgactccggttgtgccagaagagagttttgtccatccgacagcggtattgatcggcgatgttattctcggcaagggcgtttacgttgggccaaatgccagcctgcgtggcgattttggtcgtatcgtggtgaaagatggcgcgaacattcaggataattgcgttatgcacggttttcccgagcaggatactgttgtaggagaagatggacatattggtcatagcgctatccttcacggctgcattatccgccgcaatgcattagtgggaatgaacgcggtagtgatggacggtgcggtgattggcgagaacagcattgttggtgcatccgcatttgtgaaagccaaagcagaaatgccagctaattacctgattgtcggcagcccggcgaaagcgattcgtgaactcagtgagcaggagttggcatggaaaaagcagggtacgcatgagtaccaggtgctggtgacacgctgtaagcagacgttacatcaagtcgagccattgcgggaaattgaacctggcaggaaacgcctggtatttgatgagaatctgcgaccgaaacagtaacagatgtaaaattattttgtccctttaattataaagcagagttatgtttaagctctgctttatttatttgagtattaattcataccgttttttcatcatataattatttataatgagaatgtggttttaatttgtaatttatattatatacacaatttatatatttcatggtctttttttattcacctgaattataattgtgaattataggaaagtatgtttgattagataataatctactggcaatattggatgtcttctatgttttaaataactaattggtcgggttagtgcatccggctttctttatattcgccagaaggatttattatgcaaaggaaaactctattgtcggcctgtattgcattagctctgagtggtcagggttgggcggcagatatcacagaggtagaaaccaccacaggtgaaaagaaaaataccaatgtgacttgtccggcagacccaggaaaactcagtccggaagagcttaaacgcttaccctctgaatgctctcctttagtcgaacaaaacctgatgccatggctttccacaggcgctgctgcgttaatcacggccttagccgtagtggaactaaacgacgatgatgatcatcatcatcgcaacaattctccactcccaccgacaccccctgatgatgaatcagacgacactccagttcccccaactcctggcggagatgagataataccggacgatccggatgatacgcctacacctcccaaaccggtttcgtttaataatgacgttattctcgataaaacagaaaaaacgttaactattcgcgattcagtttttacttataccgagaatgctgacgggactatatctctgcaagatagcaatggtcgtaaggcaacgattaatctttggcagattgatgaagcgaataacactgttgcccttgaaggggtgagcgcagatggcgcaacgaagtggcaatataatcacaacggtgagcttgttattacgggtgataatgccacagtaaacaacaatggcaaaaccaccgttgacggtaaagattccaccggtacggaaatcaacggtaataacgggaaagtgattcaggacggcgatctggatgtcagcggcggcggtcacggtattgatatcaccggtgacagcgcgacggtggataacaagggcaccatgaccgtcaccgatccggagtccatgggtatccagatcgacggtgacaaggccatcgtcaataacgaaggcgagagcaccatcaccaacggtggcaccggcacccagattaatggtgatgacgccacggcaaacaacaacggcaaaaccaccgttgacggcaaggattccaccggtacggaaatcaacggtaataacggaaaagttattcaggacggcgatctggatgtcagcggcggcggtcacggtattgatatcaccggcgacagcgcaacggtggataacaagggcaccatgaccgtcaccgatccggagtccatcggtatccaggttgacggcgaccaggcggttgttaacaacgaaggcgagagcgccatcaccaacggtggcaccggcacgcagattaacggtgatgacgccacggcaaacaacaacggcaaaaccaccgttgacggcaaggattccaccggtacggaaattgctggcaataacgggaaggtgattcaggacggcgatctggatgtcagcggcggcggtcacggtattgatatcaccggcgacagcgcaacggtggataacaagggcaccatgaccgtcaccgatccggagtccatcggtatccagattgacggcgaccaggccatcgtcaataacgaaggcgagagcactatcaccaatggcggcaccggcactcagatcaacggtaacgacgccaccgcgaataacagtggaaaaaccactgttgatggaaaagattccacgggtaccaaaatcgcgggcaatatcggcattgtaaatctggatggtagcctgactgttacaggcggtgcgcatggtgttgagaacattggtgacaacggcacggttaacaacaaaggagatattgttgtttccgatactggatcgattggcgtgctcatcaacggtgagggggcaacagtatccaatacgggtgatgttaacgttagcaatgaagcgacagggttcagcatcacaaccaacagtgggaaggtttcgctggcaggcagtatgcaggttggcgatttctcgaccggggtagatcttaatggcaacaataacagcgtgacgctggcggcaaaagatctaaaagtggtcgggcagaaagcgacgggcataaacgtttctggcgatgcgaatacagtgaatatcactggtaacgttctggttgataaggataaaaccgcagacaatgcggcggaatatttcttcgatccatccgtgggtatcaacgtttacggcagtgataataacgtgacgctggatggaaagttaactgttgtatcagacagtgaggttacttctcgtcagagtaatttatttgatggcagcgcagagaaaacgtcaggtctggttgtgattggcgatggcaataccgttaatatgaatggtggacttgaactgattggagagaaaaacgcgcttgcagatgggtcgcaggttacttccttgcgcacaggatatagttataccagcgttattgtcgttagtggtgagtcgtcggtatatctgaatggagatacgacaatcagcggagaattccctctggggtttgccggggttattcgggtacaggataaagctttgctggaaattggcagtggcgctacgctaacaatgcaggatattgacagttttgaacatcatgggacaagaaccctggatttgcccctatatttccagacatctgttatcacttaacccattacaagcccgctgccgcagatattcccgtggcgagcgataacccagcgcactatgcggatgccattcgttataatgctcgaacgcctctgcaaggttctttgctgccgttaacccgtctggtttgggcatgatactgatgtagtcacgctttatcgttttcacgaagctctctgctattccgttactctccggactccgcaccgccgtgttcttcggttcaagtcccaacatccgggcgaactggcgtgtttcattagcccggtagcatgaaccattatccgtcagccactccactggagacgacggaagatcgttgccgaagcggcgttccaccgctcccagcatgacgtcctgtactgtttcactgttgaagccgccggtagtgaccgcccagtgcagtgcctcacgatcacagcagtccagcgcgaacgtgacacgcagtctctctccgttatcacagcagaactcgaacccgtcagagcaccatcgctgattgctttctttcacggccactctgcctgtatgtgcccgtttcgatggcggtacagcaggttttcgctcaagcaacagcgcattctggcgcatgatccggtaaacacgtttggcattgatcgcaggcataccatcaagttctgcctgtctgcgaagcagcgcccatacccgacgataaccatacgttggcagctctccgataacatggtgtatacggagaagcacatccgtatcatcagtgtgacgactgcggcggccatccatccagtcatcggttcgtctgagaatgacgtgcaactgcgcacgcgacacccggagacaacggctgactaagcttactccccatccccgggcaataagggcgcgtgcgctatccacttttttgcccgtccatattcaacggcttctttgaggagttcattttccatcgttttcttgccgagcaggcgctggagttctttaatctgcttcatggcggcagcaagttcagaggcaggaacaacctgttctccggcggcgacagcagtaagacttccttcctggtattgcttacgccagagaaataactggctggctgctacaccatgttgccgggcaacgagggagaccgtcatccccggttcaaagctctgctgaacaattgcgatcttttcctgtgtggtacgccgtctgcgtttctccggccctaagacatcaatcatctgttctccaatgactagtctaaaaactagtattaagactatcacttatttaagtgatattggttgtctggagattcagggggccagtctaaaccccagaacttacttatgctgattccggtgcgaaaattgttaataaaggtacttgtagattcaattggtcaacgcaacagttatgtgaaaacatggggttgcggaggttttttgaatgagacgaacatttacagcagaggaaaaagcctctgtttttgaactatggaagaacggaacaggcttcagtgaaatagcgaatatcctgggttcaaaacccggaacgatcttcactatgttaagggatactggcggcataaaaccccatgagcgtaagcgggctgtagctcacctgacactgtctgagcgcgaggagatacgagctggtttgtcagccaaaatgagcattcgtgcgatagctactgcgctgaatcgcagtccttcgacgatctcacgtgaagttcagcgtaatcggggcagacgctattacaaagctgttgatgctaataaccgagccaacagaatggcgaaaaggccaaaaccgtgcttactggatcaaaatttaccattgcgaaagcttgttctggaaaagctggagatgaaatggtctccagagcaaatatcaggatggttaaggcgaacaaaaccacgtcaaaaaacgctgcgaatatcacctgagacaatttataaaacgctgtactttcgtagccgtgaagcgctacaccacctgaatatacagcatctgcgacggtcgcatagccttcgccatggcaggcgtcatacccgcaaaggcgaaagaggtacgattaacatagtgaacggaacaccaattcacgaacgttcccgaaatatcgataacagacgctctctagggcattgggagggcgatttagtctcaggtacaaaaaactctcatatagccacacttgtagaccgaaaatcacgttatacgatcatccttagactcaggggcaaagattctgtctcagtaaatcaggctcttaccgacaaattcctgagtttaccgtcagaactcagaaaatcactgacatgggacagaggaatggaactggccagacatctagaatttactgtcagcaccggcgttaaagtttacttctgcgatcctcagagtccttggcagcggggaacaaatgagaacacaaatgggctaattcggcagtactttcctaaaaagacatgtcttgcccaatatactcaacatgaactagatctggttgctgctcagctaaacaacagaccgagaaagacactgaagttcaaaacaccgaaagagataattgaaaggggtgttgcattgacagattgaatctacactgttgaaattcagaatttaggttttgcttttgttactggtgaaaatacaacaggtataaatagtggcacgatctcgttattacaaaatggtaaagatccggcaccgtctcccattgttttactggctactaacggagggagcgccactaatgcaggtacgatcacaggtaaagtgacggaacaacatagcgtatttaacaagtattcaacgggcacatcgaattcatttatttttaataacgatgtcagtagcataacagggttagtcgctcaatcgaatagcacaattatcaatactgacagcggcatcattgatttgtatggtcgtggtagtgtcggcatgcttgctatagcagattcaacagcagaaaatcagggtaaaattacactggattctatgtgggtagatgcaaatgacactaccgcaatgcgagatatagctagcaacagcgccattgacttcggtacaggtgtgggagttggtactgatagttatagtggtgcagggaaaaatgcaacagcaattaaccaattgggcggtgttataactatttataacgccggcgcaggtatggcggcctatggcgccagcaatacagttattaaccaggggacgattaacctcgaaaaaaatggtaattatgacgatagtctggcagcaaatactctggtagggatggctgtttatgagcatggtactgctatcaacgaccagacgggtgttatcaatatcaatgttggtactggtcaggcgttttataacgatggcacaggaacaattgttaactatggtacaatctgcactttcggcgtgtgccaatcggggaatgagtacaataatacagatgatttcacctcactgatctataccggtggcgatacgattacacgaagcggagaaactgtaacgctaaataaatctgctgctgtgactgataagctggctgggaatgttgttaatagcggaacgctttccggtgatcaaattacggtatcaagcggtcttctggaaaataccagcggtggcatcatcaataacttagtaaaacttgacaagggtgccgtcattaaaaatgccggggtgatgacgaataacgtcgatgttagcggtggaatcctcaataatgccggagaaatgactgcgcaaattaccatgaatgctggtgctgatagttcgttagtgaacaacaccggaaccatcaataaaatcgtgcagaacgcgggggtattcaataatagtggcagtgtaacagggcggatgatgtcggctggcggggtctttaataatcaaactgacggggcgattatgagaggtgctgcgctgacaggtactgcagtggcaaataacgaaggaacctggaacctcggaagtagtagtgagggtaacaacaccgggatgctggaagttaataataattcagctttcaataaccgcggcgagtttattcttgataacgacaagaatgctgtgcacatcaaccagtccggtacgctttataataccggtcacatgaacatcagtaattcttcccacaacggagccgttaatatgtggggcggaaatggtcgttttatcaatgacggaacgattgatgtttctgcgaagtcactggtagtcagcgctaataatgccggcgatcagaatgccttcttctggaaccaggataacggggtcatcaacttcgatcacgacagcgccagtgccgtgaaagtcacccacagcaactttattgcccagaatgacggcatcatgaacatcagcggcaccggtgctgtggctatggaaggtgataagaacgcgcagctggttaacaatggcaccatcaacctcggtaccgcaggcactactgacacgggtatgatcggtatgcaactcgatgccaacgccacggcggatgcggtaatcgaaaacaacggcaccatcaatatcttcgccaatgactcgtttgcatttagcgtactgggtacagtaggtcatgtggttaacaacggcacggtggtgattgccgatggggttacgggttctggactgatcaagcagggcgacagcatcaatgttgaaggtatgaacggtaacaacggtaatagcagcgaagtgcattatggcgactatacgttgccggatgtgccgaagcccaatacggttagtgtaacgtcgggaagtgatgaggctggtggcagcatgaacaacctcaacggctatgtcgtcggtaccaacgttaacggcagcgccgggaagctgaaggttaacaatgccagcatgaacggcgtggagattaacacgggctttaccgctggtacggcagacaccactgtgagttttgataacgtagtggaaggtagcaacctgaccgacgctgacgccatcacctcaacgtccgtggtatggactgccaaaggcagcaccgatgccagcggtaacgttgacgtcaccatgagcaaaaatgcctacaccgatgtggcaacagatgcctcggtgaatgacatcgcgaaagcactggatgcgggttacaccaacaacgaactgtttaccagcctgaacgtcggcacgactgctgaactgaacagtgctctgaaacaggtcagcggtagccaggcgaccacggtattccgcgaagcgcgcgtgttaagcaaccgctttagtatgctggcagatgccgcgccgaaagtgggtaacggtctggcgttcaacgttgtcgcgaaaggcgatccgcgtgccgagttaggtaataataccgaatacgacatgctggcattgcgtaaaactatcgacctgagcgaaagccagacgatgagtctggagtacggtatcgctcgtctcgatggtgatggtgcgcagaaagcgggtgataatggcgttacaggcggttatagccagttttttggcctgaaacatcagatgtcgttcgataacggcatgaactggaataacgccttgcgttacgacgttcacaaccttgacagcagccgctcgattgcatttggcaacacgaacaaaacggctgataccgacgtgaaacagcagtacctggagttccgcagcgaaggggcgaagactttcgaaccgagcgaaggactgaaggttacgccatatgcgggtgtaaaactgcgtcacacactggaaggtggctatcaggagcgcaatgccggagactttaacctgaatatgaacagtggcagcgaaacggcggtggacagcatcgtcgggctgaaactggactacgcaggtaaagacggctggagcgctagcgctacgctggaaggcgggccgaacctgagctacgcgaagagccagcgtacggcaagcctggcaggcgcaggcagtcagcactttaacgtcgatgacggtcagaagggcggcggcatcaatagcctgacaagcgtcggcgtgaagtacagcagcaaagaaagttcgctgaatctggatgcgtacaactggaaagaggatggcatcagcgataaaggcgtgatgctgaacttcaagaaaacgttctaatttttagcatgtgatccctaaaccgcaacgctgatacaggttgcggtttttttattgccggatgtggtacgtgacgcgttttgttttgtgtctttcaggacaatagagcaactcatccagtaatcttgtttacaccttcgcattatttatctcttttcgtttctatactgatttttcttaatccgttttattacagggcagggtgcgatgagcagcaatacatttactctcggtacaaaatccgttaaccgtcttggttatggcgcgatgcaactggcaggtcctggagtttttggccccccacgagatcgccacgtcgctataaccgtgctgcgtgaggcgctggcattgggcgtcaatcatattgataccagcgacttttatggtccgcacgtcaccaatcagattatccgcgaagcgctttatccttactctgacgacctgacaattgtcactaaaattggtgcgcggcgtggagaggacgcatcctggttgcccgcattttctccggcagagctgcaaaaagcggtgcacgataatctacgtaatctcgggctggacgtgctggatgtggttaacctgcgcgttatgatgggggatggtcatggcccagcggaaggatcgattgaggccagcctgaccgtgctggcagagatgcaacaacaaggcctggtaaaacatattggcctgagcaacgtcacaccgacgcaggttgcagaggcgcgcaagattgccgaaattgtctgtgtgcaaaacgaatacaacatcgcgcaccgtgctgatgatgcaatgattgatgctttggcccacgatggcattgcctacgtgccgttcttcccgctcgggggctttacaccgctgcaatcgtccacactttccgatgttgctgcgagcctgggtgcaacaccaatgcaggtggcgctggcgtggctgttacagcgttcaccgaatattttgctgatcccagggacgtcttcggttgcgcatttacgggagaatatggctgctgaaaaattgcatctttctgaggaagtgttgtctacgttggatggtatttcgcgagaataacgaatatacaaaagggaaagatgcatttccctttttttcttttttaatggcatggagtgcatatgttgaaggccaggaattgcggctggatacgtttactgcccctgtttatgctgagtctaccagtacaggcggaacttcgatgtgttgcaaatgcagttgatattgaatcatttttttctgcggctaccgctgaagataaacaacaagttgaacaagctatcaacagtagcgtgaatcttgtccccttcggtttatctgcatcgaactggaaagtgcatcgtggcgatttagtggtagaaggtaatatagagagtaatcaaaaattgattgttcttgggaatttgacagtcaaaggtaatatttccactttctctctttctaatccatgggttattctcggtaacgtgacggcaacgaatatagttgcggattcaccactgttaattaccggttcgataaatgcaagtggactggtatttatcgactcatattacgataatccgtctacgattaaggggagtattaatgcgcgtgggatatttatcaatgacataattgcacctgttgttgcgtcttcgacaaatagtgaattcatggtccgtgcgagtgacaaacatgacactgaaaatgtcaaaaaagcgctgatgataataaatcctgatgcatattattgggggctaattaatgatgaagatgctctgaaagaaatttttaagcgaagcaatattcgcatggcagggaatgtctgtaatcagatgaaaaaagaagcgctgtttcgccctaagccttctcctgagttagtgcaagaattgcaaatgctggatgaaggcaaagttgctgcatttgaaggacgagacattgcgacatttgatcttgccgtaatgcgaactctcccaaggcttaaaggaatttcagctaacctacgcaaacaacttattaatagcaatgatgaacaaacgattgaaagtatggcgagatatatgcctgacaatgagattctggagttgaccgatcagcaattgggttaccagcctgttgttctggggttgctcgaccgtgaaccgctctctgtcgaaataatgacgcgaatgagtcgtctacctgatggtgtcggtccgttgaatcttgcgctacgtgaaaatctccctctggatatcgtcatgactctggcgaaaagagattgggatatgatcattcaggagctttataaagatgcgtggttattgcctgaatccattattgatggctatatccgcagtgatgattcctctattcgtcaggtcggtgctggaggacaactcacctacaatcaggcaatgcagttggcgaacgattcatcaaacaatgttgtcacaagcttagcgttcaagctggcagagatgaaacaccatggtcaattgttgcggatgacgccacaagagagtgacaaagttgcaggctatttataccaaaaattcgagaatgacgatgatctaatacgtgtgttatttttagcattgccagataacttacagtttaattttgttaaaaggatggagaaaaaatccccggcctacttttgctgtcgggatatgcaggtaattcactctgacgctgctttacaacggttattgacacgtttcaacgatcctgaagggtggagtaatctggcgaaaaatcagtatctgagcacgtcgatgaaacaaaaaatttggcaacgtgctttatcgcatcggaaaaataatccgaaagcagattcagatgcatatgaaaccagcgctgatatgattttgtctgagctgattagccacggcgaagttgatgaccagatgctattaaatgccaccgccctgatacgttcggacgactgggactttttagagagtgcattaattagttgggataatttacccgctgttgttctcaaggaattacagcaaaacacgccacgcaatgatatttgggcgaagttttttctgaggcaggaaaacagttcccgtgcgcaggttgacgaagcgttacgtgtttattatgcactagaccccgatgcgttagcacaactggatgtactggcaaaacaaccggatcgtatatggtggagtacactggcgaaaagcaatctcacatttttcaagttcggcgcacttaacaaccgccacacaccgcctgcagtactggcggcagaaattgatcccgagtggtggattgtggcgatgaataatccccgttttccagttgatgtattaaaggcgaggctgaaacgtgatcctttgctggcgttagagcttgttaaccctgaactggatttagtccgccagctggcgcttaacggtaagacgcgcgcaatacgggaacaagcgatgagaaaacttgatgagttgtattgatccacaacgtaatgttttttaactatctgattaattggggataatcattcctgacagtgagtccccaataccttgatatattctgaatttttaatgaaacggcgtgttgcgatatctccgtcaggggaattgatgcaccatagcgcaaaccgaattatcaaggattgataatgacgctctaccagataaaaccgctctttcagtcgctgttaaggccgacgatgttttggctttataagcaccacgttacagcgaatcacatcactcttgctgcactggcgctttctcttcttaccggattgctgttgatgttggcggcacaacccatcctctttttgctattgcccatcgtgctttttatccgtatggcgctcaatgcgctggatggcatgttggcgcgtgagtgcaaccagcaaacacgtctgggggcgattttgaatgagactggcgatgttatttccgatattgcgctctatttaccatttttatttttaccggaaagtaacgcatcactcgtgatactcatgttattttgcaccatattgaccgagttttgcggtttactcgcgcagacgattaacggtgttcgcagttatgccggtccatttggcaaaagcgatcgcgcgttaatatttggtctgtggggtctggccgttgccatttatccacagtggatgcagtggaataatcttttatggagcattgcttcaattctgcttctctggactgcgattaatcgttgtcggagtgtgcttcttatgagcgctgaaatataatgctggaaaaatctctggcaacacttttcgcgttgttaattttagcaacgctgataaaccgttttctgctatggcggttaccggagagaaaagggggtgaggttacattacgtattcgtacctggtggggcatcgtcatttgtttttcaatggtgatttcaggtccacgctggatgacgttgacgttttttgcgctgataagttttctggcattgaaagaatattgtacgcttatatctgtacattttccgcgttggttatattggggtattcctcttaactatttgcttatcggttttaattgctttgagctgtttctgttatttatacctttggctgggtttctgatattagccaccgggcaagttttagtgggtgacccctctggttttctgcataccgtgagcgccattttttggggctggataatgaccgttttcgccttgagtcatgccgcctggttattaatgttgccaaccacaaatatccagggcggggcgttactggtgttatttcttttggcattaaccgagtcaaacgatattgcacagtatttatggggaaaatcctgcggcagaagaaaagtggtccctaaagtcagcccgggaaaaacattggaaggtctgatgggcggcgtcatcaccatcatgattgcgtcactgattatcggaccgttactgacaccgctaaatacattacaggcattattagcgggtttgttaattggtattagtggtttttgcggcgatgtcgtgatgtcagccatcaaacgagatattggtgttaaagatagcggaaaactattgccaggacatggcggactccttgacaggattgactcattaattttcaccgctccggtatttttttattttatacgctactgctgttactgaaggaaaatagagaaaatggaaaattcacgcatccctggggaacatttttttaccaccagtgataatacagcgttgttttatcggcactggcccgctttacagcccggggcgaaaaaggtcatcgtcttatttcatcgcgggcatgaacattctggtcgtctacaacatctcgttgatgaactggcgatgccagatactgctttttatgcctgggatgcccgagggcatggaaaaagttcggggccgcgtggttatagcccatctcttgcgcgttcagtgcgggatgtcgatgaatttgtccgttttgctgccagcgacagccaggttggactggaagaggtggtagtgatcgcgcaaagcgtcggcgcagtgctggttgccacatggattcatgattatgcacctgcaattcgcgggctggtgctggcttctccggcctttaaggttaaattgtatgtgccgctggcacgtcctgcgctggcgttatggcatcgtctgcgtggtctgttttttattaattcctatgtgaaaggacgctatttgacccacgatcggcaacggggggcgagtttcaataatgatccgctgatcacacgggcgattgccgttaatatcttgctcgatctctacaaaacgtctgaacgtattattagagatgcggcggcgattacgctccccacgcaacttctgatatcaggcgatgactatgtggtgcatcgccaaccgcagattgatttttatcagagattacgtagccctctgaaagagctgcatctgctgccaggcttttatcacgacacgttgggtgaagagaacagggcgctggcatttgaaaaaatgcaaagctttattagtcgtttatatgctaacaaatcgcaaaaatttgattatcagcatgaagactgcacaggaccatcagcggatcgatggcggctactttctggtggacccgtgccattatcgccggttgatttagcgtatcgctttatgcgaaaggcgatgaaattgttcgggacgcactcttcgggcctgcatctcggaatgagcaccggctttgattcaggcagttcgctggattatgtctatcaaaatcaaccgcaaggtagtaacgcattcgggcgtttagtcgacaaaatctacctgaacagtgttggctggcgcggtattcgccagcgcaaaacccatttacaaatactgattaaacaagccgttgccgatctccacgccaaaggtttagccgtccgcgtggttgacattgccgcagggcatgggcgctatgtactggatgcgctggcaaacgagcctgccgtaagcgatattttgttacgtgattacagcgagttaaatgttgcacaggggcaagagatgattgctcaacggggaatgtctgggcgggtgcgttttgaacagggcgatgcgtttaacccggaggaactcagcgcgttaactccgcggcctacgctggcgattgtctctggcctgtatgagctttttcccgaaaatgagcaggtaaaaaactcactcgcaggtcttgccaatgccatcgaaccgggcggcattctcatctacaccgggcagccgtggcaccctcaactggagatgattgccggggtgttaaccagtcataaagatggtaaaccgtgggtaatgcgcgtgcgttcgcaaggggagatggattcactcgtgcgtgatgccggatttgataaatgcacacaacggattgatgagtggggtatttttacggtttcgatggcggtgcgtcgtgataactgaacgtcggaacgtattgctacaaggcgctggctggttattgttgctggccccgtttttcttcttcacctatggatctcttaatcagttcaccgcggttcaggaccttaacagccatgatatccccagtcaggtattcggttgggaaacggcgatcccttttcttccctggactattgttccttactggagtctggatcttttatatggattttcgctgttcgtttgtagcacgacattcgaacagcgccgacttgtccaccggcttattctggcaacggtaatggcctgctgcggttttttgctctatccgctgaagtttagttttatccgtcctgaagtgagtggggtgacgggatggctattttcgcaacttgaactgtttgatctgccttataaccagtctccttcgctgcatattattctctgctggctactttggcgtcactttcgtcagcatctggctgagaggtggcgtaaagtctgcggcggatggtttttactcatcgccatttcgacgctgacgacctggcagcatcattttattgatgtcatcacagggctggcggtaggtatgttgattgactggatggtgcccgtcgaccgtcgttggaattatcagaaacctgatcaacgtcgaatcaaaatagcactgccctatgtcgtaggcgcgggctcgtgcattgtattgatggagctaatgatgatgattcagttatggtggtcagtctggttatgttggccagtattatcgctactcataattggccgtgggtacggtgggcttggcgcgataacaacagggaaagatagtcaggggaaactaccgcccgccgtttactggctgacattgccctgccgcatcgggatgtggctgtctatgcgttggttttgtcgtcgcctggagccggtgagcaaaatgactgctggtgtttatttaggggcgtttccacgacatattccggcacagaatgcggttctggacgtcacctttgaattccctcgcggacgagccacaaaagatcgactctatttttgtgtaccgatgctggatctggtggttccggaagagggggagctccgacaggccgtggcgatgctggaaacattacgcgaagagcaaggcagcgttctggtccattgtgcattgggattatcgcgcagtgcgctggtggtggcggcatggttgttatgttacggacactgtaaaaccgttaatgaagcgattagctatattcgagccagacgcccgcagattgtgctgacagacgagcacaaagcgatgctgagattatgggaaaacaggtaagtggattgagatgtggactgaatatctacagtccacatcaagaccgtgtccggttatgcagaaacaatgctgtcgatggctgcttttgcgtcagactgtgctttcgctgccatttccggaccgtatgcgatcccttcggcgaagacaaatttcacatcggtaatgccgataaagccgaggaacgtggacagatacggcgtcaccaggtccgttggtccatctttgtggatcccgccgcggctggtaataacgatggcttttttacccgttaccagaccttccggaccgttctcggtatagcggaaagtaacgcctgcgcgggcaaccaggtcaaaatagtttttcaactgagtcgagatgttgaagttatacatcggtgccgcaataacgataacgtcgtgggctttcagctcggcaatcaactcatcggaaagtgccagagcttcctgctgacgcggagtcagcggcgcatcgctcggacgcagagcgccaaccagttcgccatccagtaccggaatcggatttgcagccaggtcgcgaacggtgatttcatcagcggagtgcttttcgcgccattgttcaacaaaataatcggacaactgattagactgagagtaccctgccaggatgctggatttaagaactaataccttgctcatggtgtttccttatagatgtttgaatgggcgatgccccgttgcttgttgacactttattcacaatcctgccacagagatagcgcaataaatcgaagcctatgttcgaatttattgaacaacgcatagaaagccgcgatgtggtactctatatctatcatttaaaagaaaattaatcaggcagactactgcccactaacgttatgacagaacaacaaaaattgacctttacggccttgcagcagcggctggattcgctgatgctgcgtgacagactgcgtttttctcgccgtctgcacggcgtgaagaaggttaaaaatcctgatgcacaacaggccattttccaggagatggcgaaagagattgaccaggcggcagggaaagtcctgctgcgtgaagcggcacgaccggaaattacttatcctgacaatttaccggttagtcagaaaaaacaggacattctcgaagcgattcgtgatcaccaggtggtgatcgtcgccggggaaacgggttctggtaaaacgactcagttaccgaaaatctgtatggagctggggcgcgggattaaaggactgatcggccatacccagccgcgtcgtctggcggcaagaacagtggcgaaccgtattgcggaagagctgaaaacggagccgggcggttgcatcggttacaaagtgcgtttcagcgatcacgtaagtgataacacgatggtcaagctgatgaccgacggtatcctgctggcggagatccagcaagaccgcctgctgatgcagtacgacactatcattattgacgaagcgcacgaacgcagcctgaatatcgattttttgctcggctatttgaaagagttgctgccgcggcgtcctgacctaaaaatcattatcacttccgcgactatcgacccggaacgcttttcgcgccactttaataatgcgccgattattgaagtctccggtcggacctatccggtggaagtgcgctatcgcccgattgttgaagaagccgatgacaccgagcgcgatcagttgcaggcgatttttgacgccgtagacgaactgagtcaggaaagccatggcgacattctgatctttatgagcggcgagcgggaaatccgcgataccgccgatgcgctgaacaagctgaacttacgccataccgaaatcttgccgctttatgcgcggctttcgaacagcgaacaaaatagggtattccagtcgcacagcggacggcgcattgtgctggcgaccaacgtcgcggaaacgtcgctgaccgtaccggggattaaatacgttatcgaccccggtacagcgcgtatcagccgctacagctatcgcaccaaagtgcagcgtttgccgattgagccgatttcccaggcgtctgccaatcagcgtaaaggccgctgtggtcgtgtgtccgaagggatctgtattcgtctctattccgaagacgatttcctctcgcgcccggagtttaccgatccggagattctgcgtaccaacctggcctcggttattttgcagatgaccgcgctggggctgggcgatatcgctgcgttcccgtttgtcgaagcaccggataaacgcaatatccaggatggcgtgcgtctgctcgaagagctgggcgcgatcaccactgatgaacaggccagcgcctataaactgacgccgctcggtcgccagctctcgcagttgcctgtcgacccacgtctggcgcgtatggtgctggaagcgcaaaaacatggctgcgtgcgtgaggcgatgattatcacgtccgcgctctccattcaggatccgcgcgaacgtccgatggacaaacagcaggcatcggacgaaaaacatcgtcgcttccacgacaaagagtctgactttctcgcgtttgtgaatctgtggaattatcttggcgagcagcaaaaggcgctttcttccaacgccttccgtcgcctgtgtcgtaccgattatctcaactatctgcgcgtgcgcgaatggcaggatatctacacccagttgcgtcaggtggtgaaagaacttggcattccggttaacagcgaaccggcggagtatcgcgaaattcacattgcgttgctgaccggtttactttcccatatcggcatgaaagatgccgataaacaagaatataccggcgcacgtaacgcgcgtttctccatcttccccggttctggtttattcaaaaaaccgcctaaatgggtaatggtggcggaactggtagaaaccagccgcctgtgggggcgcattgctgcgcgtatcgacccggaatgggtggagccagttgctcagcatttgattaaacgcacctacagcgaaccgcactgggaacgggcgcagggcgcggtgatggcaacggaaaaagtcactgtttatggtttgccgattgttgccgcgcgcaaggtcaactacagccagatcgatccggcgttatgtcgtgaactctttattcgccacgcgctggtggaaggtgactggcagacgcgtcacgcattcttccgtgaaaacctgaaactacgggcggaagtagaagagctggaacacaaatcacgtcgccgcgatattctggttgatgacgaaacgttgtttgagttctacgaccagcgcatcagccacgatgtaatctccgctcgccacttcgacagctggtggaaaaaagtcagccgcgaaacgcctgatttgctcaactttgaaaaaagcatgttgatcaaagagggcgcagaaaaaatcagcaagctggattacccgaacttctggcatcagggcaatctcaagctgcgtttgagctatcagtttgagcccggcgcggatgctgacggtgtgaccgtacatattccgctgccgttacttaaccaggttgaggaaagcgggtttgaatggcagatccccggtctgcgccgcgaactggtgattgctctgattaaatcgttgccgaaaccggtacgccgtaattttgtacccgcgccaaactatgccgaagcgtttttaggccgcgtcaaaccgctggagttaccgttgctcgacagccttgagcgcgagttacggcggatgaccggcgttaccgttgaccgcgaagactggcactgggatcaggtgcccgatcacctgaaaattaccttccgcgtggtggatgacaaaaacaagaagctaaaagaagggcgctcgctacaagatctgaaagatgcgctgaaaggcaaagtgcaggaaacgctatctgcggtggcggatgacggtatcgagcagagcggcttacatatctggagttttggtcagctgccggaaagctacgaacagaagcgtggcaactacaaagtgaaggcgtggccggcgctggtggatgagcgcgacagtgtggcgatcaaactgtttgataacccgctggagcaaaagcaggcaatgtggaacggtcttcgccgtctactgctgctgaatattccatcgccaatcaaatatttacatgaaaagttaccgaacaaagccaagctgggactgtactttaacccgtatggcaaagtgctggagctgatcgacgactgtatctcctgcggtgtggataaattgatcgacgccaatggtggcccggtctggacggaagaaggctttgctgcgctgcatgaaaaagtgcgtgccgaactgaacgacacggtggtggatattgcgaagcaggtcgagcaaatccttacggcagtgttcaatatcaacaaacgtctgaaagggcgggtggatatgaccatggcgctggggctttctgacattaaagcgcagatgggcgggttggtatatcgcggttttgtcactggtaacggcttcaaacggctgggcgacacgctgcgatatttgcaggcgattgaaaaacggctggaaaaactggcggttgatccacatcgcgaccgtgcgcagatgctgaaagtcgaaaacgtccagcaggcgtggcagcaatggatcaacaaactgccgcccgcacgtcgtgaggatgaagacgtgaaagagatccgttggatgatagaagagttgcgcgttagttacttcgctcaacaacttggtacgccttatccgatttcagataagcgtattttgcaggcgatggagcagattagcggttaaccctgctatttgcctgataaagaaaaaacccggtaagcatttagcgccgggttttttattaattctaaaacggtaagggtaaaaattcaggaattcagaaaaatacaattctctgctgcaagatgaataatgtttatctacagcatttccttaaaagatatgtcaggcttgcggagtggcggttaaggacatacgatttcctcctttcagagtgctccgcttctcactattatctcacgcagtattcttaagggaacgataaggaggaaccatgaacattaccccgtttccgacgctttcgccggcaactatagatgccataaatgttatcggacagtggctggcgcaggatgatttctccggtgaggtgccgtatcaggccgattgcgtgatccttgcaggcaatgcggttatgccgactatcgatgcggcatgtaagattgcccgcgatcagcaaattcctttactgattagtggtggtatcggtcactcgacaacttttttgtatagcgccatcgcacagcatccgcactacaacactatccgcaccactggcagagcagaagcgaccatcctggcggatatcgctcatcagttctggcacattccgcatgaaaaaatctggattgaagaccagtcaacaaactgcggtgaaaacgcacgctttagcatcgcgctattgaatcaggccgtagaacgagttcatacggctatcgttgttcaggaccccaccatgcagcggcgcacgatggcgacgttccgccgtatgactggggacaatcccgatgcaccacgctggttaagttatcccggattcgttcctcagttaggaaataacgcagacagtgtaatctttattaatcagttacaaggattatggccagttgagcgttatctctcactactcactggcgagctgccgcgtttacgcgatgatagcgatggctacggtccccgcgggcgagattttatcgttcacgttgattttccggcagaagtcatccatgcatggcaaacgctgaaacatgatgcggtgctcatcgaggcgatggaaagtcgctcgttacgttaaaaattgcccgtttgtgaaccacttgtttgcaaacgggcatgactcctgacttttatttctgccttttattccttttacacttgtttttatgaagcccttcacagaattgtcctttcacgattccgtctctctgatgattgatgttaattaacaatgtattcaccgaaaacaaacatataaatcacaggagtcgcccatgtcagtacccgttcaacatcctatgtatatcgatggacagtttgttacctggcgtggagacgcatggattgatgtggtaaaccctgctacagaggctgtcatttcccgcatacccgatggtcaggccgaggatgcccgtaaggcaatcgatgcagcagaacgtgcacaaccagaatgggaagcgttgcctgctattgaacgcgccagttggttgcgcaaaatctccgccgggatccgcgaacgcgccagtgaaatcagtgcgctgattgttgaagaagggggcaagatccagcagctggctgaagtcgaagtggcttttactgccgactatatcgattacatggcggagtgggcacggcgttacgagggcgagattattcaaagcgatcgtccaggagaaaatattcttttgtttaaacgtgcgcttggtgtgactaccggcattctgccgtggaacttcccgttcttcctcattgcccgcaaaatggctcccgctcttttgaccggtaataccatcgtcattaaacctagtgaatttacgccaaacaatgcgattgcattcgccaaaatcgtcgatgaaataggccttccgcgcggcgtgtttaaccttgtactggggcgtggtgaaaccgttgggcaagaactggcgggtaacccaaaggtcgcaatggtcagtatgacaggcagcgtctctgcaggtgagaagatcatggcgactgcggcgaaaaacatcaccaaagtgtgtctggaattggggggtaaagcaccagctatcgtaatggacgatgccgatcttgaactggcagtcaaagccatcgttgattcacgcgtcattaatagtgggcaagtgtgtaactgtgcagaacgtgtttatgtacagaaaggcatttatgatcagttcgtcaatcggctgggtgaagcgatgcaggcggttcaatttggtaaccccgctgaacgcaacgacattgcgatggggccgttgattaacgccgcggcgctggaaagggtcgagcaaaaagtggcgcgcgcagtagaagaaggggcgagagtggcgttcggtggcaaagcggtagaggggaaaggatattattatccgccgacattgctgctggatgttcgccaggaaatgtcgattatgcatgaggaaacctttggcccggtgctgccagttgtcgcatttgacacgctggaagatgctatctcaatggctaatgacagtgattacggcctgacctcatcaatctatacccaaaatctgaacgtcgcgatgaaagccattaaagggctgaagtttggtgaaacttacatcaaccgtgaaaacttcgaagctatgcaaggcttccacgccggatggcgtaaatccggtattggcggcgcagatggtaaacatggcttgcatgaatatctgcagacccaggtggtttatttacagtcttaatgagtgaaagaggcggaggttttttcctccgcctgtgcgcgtcagagtttagcgaatttttcgagggtgcgaataagctgtgtgacgaagccatattcgttatcgtaccaggcgaccgttttcaccagttgtaaatcgcccacggcggtaatttccgtttgcgtggcatcaaacaccgaaccgaaatggctgccaatgatatcggaagagactatttcttcatcggtataaccaaatgactcgttattggtggttgcttgtttaagtgcgttattcacctcttcggcagtcacttttttccgagaatcgataccagttcagtgaccgaacctgttttcaccggcacgcgttgcgcatgacctttcagtttgccgctcagttccgggatcaccagaccaatggcttttgccgcccccgtagtgtggggaatgatattttctgccgctgcgcgtgaagcacgtaaatctttaccacgcgggccatccaccagtgactgggtgccagtataggcatgaatggtcgtcatcgtgccgacttctatcccgaaactgtcatgcaaggctttggccatcggcgcaagacagttagtggtgcatgacgccacggaaacaatggtgtcgttgccatccagagtgtcgtcattgacgttataaacgatagttttcatttcaccggcaggggcggaaatcaacaccttcttcgcaccagcatcaagatgcgcctgcgatttctcggcggaggtataaaagccagtacattcgacaatgatttctgcacctttcgctttccacggaatatttttagcctctttttcggcgtaaaccgcgatacttttcccatcaacgataagtgaatcttccgtaaaatcaacgctccaggggaatggtccgtagtttgaatcatgtttcagcaggtaggcgagaatttatggggaagtgagatcattaatagcgacaacgtctatgttgcttttgacttcaagtaatcgacccaacaccagtcgaccgatacgaccaaaaccgttaataccaactttactcatggttttctcctgtcaggaacgttcggatgaaaattgatcctttccaagcttagaccaggatggcgggatgggcaatctccattctcacagtgaaacgtaacgtactgaaaacgggtgaacaatatttaatgaaattttgagaaaagcccgttatgttaacggaaaattatgttaaagcaggaaatgttatggaaaataaatattcaaggttacaaatcagcattcactggctggtctttttactggttatcgcagcgtattgcgcaatggagtttcgtggtttcttcccacgtagcgatcggccactcatcaacatgattcatgtttcctgtggcatctcaattctcgtgctgatggtcgttcgtcttttgttaaggctgaaatacccaaccccgccgattatacctaagccaaaaccgatgatgacgggactggcgcatttgggacatttggtgatttatctcctgtttattgcgctgccagtgattggtttggtgatgatgtataaccggggcaacccgtggtttgcgtttggtttgacgatgccttacgcttcagaggccaatttcgaacgggtagatagcttaaagtcgtggcatgaaacgctggcgaatctgggatattttgtcatcgggttgcacgctgcggctgcactggcacaccactatttctggaaggacaacacacttctacgcatgatgccgcgtaaacgttcctgaaggatatttaaagaaaacgcctgtactaaaaccgacccgtggtacaggcgaagaatacgggtctacatcggaagcgcctattatatttatttgtatgataaataaaaccataatccttgcccatacgtccatctggcttatttttaatcaattcacccgatctttgatctcatcaacggtatcaaaataaaccagcgtataacgttcaaatcgaacataagattcgataaaccatggaggttatatgaaaaaactggcacttattttgtttatgggaacgcttgtttccttttatgccgatgccgggcgcaaaccctgttctggttcgaaaggggggatctcacactgtacggcaggcggcaaatttgtctgtaatgatggttctattagtgcatcgaaaaaaacatgcactaactgaagtgtaaaaggggtgccatgagaaaatgaatctgctagtcaaatgcgcggggaaaatccccgcgcttgcccttacctggacgtgcaggccatgagcgcagcaacctccttatcaccgtcccggaaccgcagttcgtagagcgtttgtcgggtcaggagtgtgaatgtcagaatcgtaatgcagataatgagcagacacaccaccagagggttgtgcttcatagcctttctccttgccggatggcgggtaagaggctaagatctgaattgctaggttcattcgttggcctcggttgatagaaatatcggtcggggccttcgtctttctgattcccggttagcctgaaaacagaaagtctcaggcacccgcaggcatcctatgaggtttccttagggacgaaaataatcacttcacgaaattgcgtgctgttttccagaatttttcgtcattcgggttagccagtttagccattcgttactctcttcattccaatagcattaattttctatgcaataattgttgtaaaaatgtgacgcaaagaggtttttggtcataagtaattaccgtcaagtgccgatgactttctatcaggagtaaacctggacgagagacaacggtaatgaatacaactccctcacagcgattaggttttttgcatcacatcaggttggttccgttatttgcctgcattctaggcggtatcttagttctattcgcattaagttcagccctggctggctatttcctctggcaggccgatcgcgatcagcgtgatgttactgcggagattgagattcggaccgggttagcgaacagttcagattttttgcgttcagcccggatcaatatgattcaggccggggctgcgagtcgtattgcggaaatggaagcaatgaagcgaaatattgcgcaagccgaatcggagattaaacagtcgcagcaaggttatcgtgcttatcagaatcgaccggtgaaaacacctgctgatgaagccctcgacactgaattaaatcaacgctttcaggcttatatcacgggtatgcaacctatgttgaaatatgccaaaaatggcatgtttgaagcgattatcaatcatgaaagtgagcagatccgaccgctggataatgcttataccgatattttgaacaaagccgttaagatacgtagcaccagagccaaccaactggcggaactggcccatcagcgcacccgcctgggtgggatgttcatgattggcgcgtttgtgcttgccctggtcatgacgctgataacatttatggtgctacgtcggatcgtcattcgtccactgcaacatgccgcacaacggattgaaaaaatcgccagtggcgatctgacgatgaatgatgaaccggcgggtcgtaatgaaatcggtcgcttaagtcgtcatttacagcaaatgcagcattcactggggatgacagtagggactgttcgacagggcgcggaagagatttatcgtggcaccagcgaaatttcagctggcaatgcggacctgtcatctcgcaccgaagaacaagcggcggctatcgaacaaactgccgccagcatggagcaactcactgcgacggtgaaacagaatgcggataacgcgcatcatgccagcaaactggcgcaagaggcttctattaaagccagcgatggcgggcagacggtttccggtgtagtaaaaacgatgggcgctatctccacgagttcgaagaaaatttctgagatcaccgccgtcatcaacagtattgctttccagacgaatattctggcactgaatgctgccgttgaagccgcgcgagcgggtgagcaagggcgtggatttgccgttgtcgccagcgaagtacggacactcgcaagtcgcagcgctcaggcggcgaaagagattgaaggcttgatcagtgaatcagtcaggttaattgacctggggtcggatgaggtggcaacggccgggaaaaccatgagcactattgttgatgccgtcgcgagtgtcacacatatcatgcaggaaatcgccgccgcctcggatgaacaaagtagaggcataacgcaggttagccaggcgatttctgaaatggataaggtgacgcaacagaatgcttctctggtagaagaggcctcagcggcggcggtgtcccttgaagaacaggcggcacgattaactgaggcggtggatgtattccgtctgcacaaacattctgtgtcggcagaacctcgcggagcgggtgaaccagttagtttcgctacggtgtgaaaatgttcaaggagggatcgacagatcccttcacctttcagaacggcattgattttcgaatagcgttaatcatcaactggcaaccagaagagaacgtcgcatctacgcgggtcagtattccaatcggttcgcctgcaccatgtcccggaacaggcagggccaccagcgtggcatgacgcaggtcgtcttttacagcgccagaagggacaaaccacacgtaatcgtattcaaccgtaagttgacgagatagcgaagcagacagcgtttcgatacaacccgaaggaattttacagccctggctctgcactaatgcatctgaatgctggcgtggcgcagtgccttctggtgatacaacgaccggccattccagcacccggcttagcgttacgttctcctgaagtagcgggtgattagggcggacaaccagcttcaacgattcaagaaacagcagttcgtaattaagcccggtcatcagttcaggatctgacatccgaccaatgccgatatcgatttccccggtttttaaacccgccagaatcatagggttactcattgtcgcaacttgcaaggtcgtctctttttgttgctgatgaaactgacctataaccgaaggtaatatccccagtgccgcagtaggtagtgcaccaaccctgacgacatcattattaagaccttctttacgatgaagcgaccgtccggcagtgttgatggcgtcaagaactctgactgcatgcgttaaaaattgttcgccgggtaaggtaagttgcgccccctgacgaccacgctcaaacaagcgagcgccagtcagctgctccagttcattcaatgtcttagagagcgcaggttgactcaaattaagggtttcagccgcgcgccccaaagttccttgttgtgcgacagctacgaatgtatgaaggtggcgcaaacggatgcgctgactaaacagactatttttttccataagcgatgttaaaaacgaagcggtgtcgctgacaagtgaagttgtttgattatgataacttgattgcaaaatattattaacaattaaagcaattatgttacagcaaaatggataatattgatgttttcgcggcgagatcacagtttgtaaattcttcccgcaagagtgaatgcggttacctacactccagattactgaccactggaggcagacactatggcgaacagcatcacggcggatgagattcgggaacagttttcgcaggcaatgtcagccatgtaccagcaagaagttccgcaatatggcacgctgctggaactggtagctgatgtgaatctggctgtgctggaaaacaatcctcaactgcacgaaaaaatggtaaatgcagacgagctggcgcgactgaatgttgaacgtcatggggcgattcgcgttgggactgcacaagagcttgctactcttcggcggatgtttgccattatggggatgtacccggtgagctattacgatctctcgcaggcaggggtgccggtacattcgacagcatttcggcccattgatgatgcttctctggcgcgtaatcccttccgcgtttttacctccttactccgccttgagcttatcgagaacgaaattttgcgccagaaagcggcggagattctgcgtcagcgcgatatcttcaccccacgttgtcgacaactgttagaggaatatgagcagcagggcggttttaacgaaacacaggcacaggagtttgtgcaggaagccctggaaacgtttcgctggcaccagtcagcaacggtagatgaagaaacctatcgcgcattgcacaacgaacatcggttgattgctgatgtggtctgttttcctggatgccatatcaaccacctgacgccacgtacgctggatattgaccgggtgcagtcgatgatgcctgaatgcggaattgaacccaaaattctcatcgaggggccgccgcgccgcgaggtaccgattttactacgccagaccagctttaaagcactggaagagacggtgttgtttgcggggcagaaacagggcacgcataccgcgcgctttggtgaaattgagcagcgtggcgtggcattaacgccgaaagggcgacaactgtatgatgatcttctgcgtaacgctggaaccgggcaggataatctcactcaccaaatgcatttacaggaaaccttccgcacttttcctgacagtgagtttttaatgcgtcagcaagggttggcatggttccggtaccgtctgacgccttcgggtgaggcgcatcgtcaggcgattcatcctggagacgatccacagcccttaattgaacgtggttgggtagtggcgcaacccatcacctatgaagatttcttgcccgttagcgcggcggggatcttccagtcaaatctgggtaatgaaacgcagacacgcagtcacggtaatgccagtcgcgaagcatttgagcaggcgttgggttgtccggttttggatgagttccagctttaccaggaagcggaagaacgcagtaaacgtcgctgtggtttgctttaaaatctgaccatccgcctttgcaaaaatttgcctgattttacaaacgaatcaggctcatcccatcgacataaaaaaaatgccgatttatgcatattctctcagttcaacaattggattattaataaatattgtctagagtgagcggtcataaataagcactttcttgccgctgaaaacgaccagcgcgggaccattcacaacaccagaaggactcactttcaggtatggatcgtagacgatttattaaaggttcaatggctatggccgccgtgtgcggtaccagcggcattgcttctcttttttctcaggcggcattcgcggcagattctgatattgccgacgggcaaacccagcgttttgacttctccattctacagtcaatggcgcacgacttagcgcaaacagcgtggcgtggtgcgcctcgtccgttacctgacacgctggcgacaatgacgccgcaggcttataacagtattcaatacgacgccgaaaaatcgctctggcataacgttgagaaccgtcaactggacgctcagttcttccatatgggaatgggattccgtcgccgcgttcgtatgttttctgtagatccagcaacacatctggcgcgtgaaattcactttcgcccggagttgttcaaatacaacgatgcaggtgttgatacaaaacaattagaagggcaaagcgatctcggctttgccggttttcgcgtgtttaaagcccccgaactggcgcgccgtgatgtagtatcatttctcggcgcgagttatttccgcgccgttgatgatacatatcaatacggtttgtcggcccgcggcctggcgatcgacacttacaccgacagtaaagaagagttccccgactttaccgccttctggtttgatacggtaaaaccgggggcaactacctttaccgtttatgcgttgctcgatagcgccagcattactggtgcctataagttcactatccattgtgagaaaagtcaggtgattatggatgtggaaaatcacctgtatgcgcgcaaagacattaaacagctgggcattgcgccgatgaccagtatgttcagctgcggtactaatgaacgtcggatgtgcgatacaattcatccgcaaattcatgactctgatcgtctgtccatgtggcggggcaacggcgagtggatttgccgtccgctgaataatccgcaaaaattgcagttcaatgcttacaccgacaacaacccgaaagggtttggtttattgcaactggatcgtgacttctcccattatcaggacattatgggctggtataacaaacgcccaagtctgtgggtggaaccgcgtaacaagtggggtaagggcaccatcggcctgatggaaatcccaacaacgggcgaaacgctggataacattgtctgcttctggcagccagaaaaagctgtaaaagcaggtgatgagtttgcattccagtatcgtctgtactggagtgcgcaaccgcctgttcattgcccattagcgcgcgttatggcgacgcgtaccggcatgggcggtttctcggaaggttgggcgccaggtgaacactatcccgaaaaatgggcgcgtcgttttgccgtcgatttcgttggtggtgatctgaaagctgccgcgccaaaaggcattgagccggtgattacgctttccagtggggaagcgaagcaaatcgaaattctctatattgaacccatcgatggttatcgtattcagtttgactggtatccgacttcggactccactgatccggtcgatatgcggatgtatctacgttgtcagggggacgctatcagtgaaacatggctgtatcagtatttcccgccagcgccggataaacgtcagtatgttgacgaccgcgtgatgagttaatcgttttttcttcggcaccttcttcgggaggtgccgtctggttaaacacgatcccgctcgcatttttccctaagttaaatgagtaatctgatggtgtgtatttcagatacaccttgtcagccactaacagggagtgcgtatgtttccagaataccgagatttaatatcccgtctgaaaaacgaaaatcctcgctttatgtccttgttcgataaacacaataaacttgatcatgaaattgccagaaaggaaggttccgacggtcgagggtacaatgcggaagtggtccgcatgaaaaaacaaaagctacagttaaaagatgagatgctcaaaatcctgcagcaggagagcgtcaaagaggtgtaaactttcctaagccgccagccaggcggcttttttaacaactgcatggattgactggagataagatgactgaaacgataaaagtaagcgaatcacttgaattacatgctgttgcagaaaatcacgtcaaacctctttatcagttaatctgtaaaaataaaacctggttacagcagtcgctaaactggccgcagtttgttcaaagtgaagaggacacgcgaaaaacggtgcagggtaatgtgatgttgcatcaacgcggctatgccaaaatgttcatgattttcaaagaagatgaacttatcggcgttatctcgtttaatcgtattgaaccactgaataaaaccgctgaaataggctactggctggacgaatctcatcaggggcaggggatcatttctcaggcgctgcaggcattgattcatcattacgcccagtctggtgaacttagacgcttcgtgatcaaatgtcgggtggacaatccgcaaagcaaccaggtcgctttgcgcaatggttttatccttgaaggttgcctgaaacaggctgagttcctgaatgatgcctatgatgatgtgaacttatacgcgcgtattatcgattcacaataaccctgccagcggcgttcgcgtaatgcgctcctcgccgttaatgacttttggaccacggacatgaaccgtgtcgccatcaaaggcttcaacgacggcgtggtcggttaactccacatggttttcaattatcaccgcacctgtaatacggctctcaccttgtatgacaacgtgctcgtcgagcagaatcggtccgccacgtaccacggcatttccgccaaccaagacatgatgttttaacacacaattaccttccacaatggcatattccgccacctgcgaactgtaatgaatcgtcggaatggcatcttcttctatgccagctttcacctgcgcgtgaccgtagactttagcgcaatcgcatagccagacattgttctcttcattaccttcaatactggcaaaatcaaaaacttcggcgcgatgttcaataaaagcataccggacgacggcatcgccataaatttgtgcctggtggacaatacgcgaggcgctaacccttgcgcgatcataaatttggagcaggagttgatggtcgggcgttaagccttgtgcggcgacgatcatagaatgttgatcaattaaggcgtgaccaaatattctacattgcccgtaaactaatgagtcatgaatggtgacgctgtcacttatatatgcaccctggctgatttcactattatcgatccagacgttatccgttgcgtaaacctctccccacagcacgctggtgccggtgatacgcgtattaccggaaatcaccgctccgccgaacgcaatagcattctggtcgtaaatccagcaatttccttcttgtgctaacaccgtttcgcgatcgatccagccgccagcggttcctgctatcacatcgttaaaatcgctaatggcgataatctgccgtaataacacattttttttagtgccatcttcctgataactaaaggctcgctgttcttcacttagacgatatttgcgcatagcgttttcccacaggtgacttactataaccgtagcaaattctgcggctctggctatgctcgagaaaattccataaaatgcatttcaaatatactttataaattaaacaaaatgagtaagaagatgcagagcgataaagtgctcaatttgccggcaggctactttggtattgtgttggggacgatagggatgggatttgcctggcgctatgccagccaggtttggcaggtcagccactggttaggggatgggctggtgattctggcgatgatcatctggggattattgactagcgcatttattgcccgactcatacgctttccgcatagcgtgctggcggaagttcgccatccagtgctgagcagttttgtgagtttgtttccggcaacgacgatgctggtggcgattggttttgttccgtggtttcgcccactggcggtgtgcctgttcagttttggtgtcgtggttcagttggcttatgccgcctggcaaactgcgggattatggcgcggatctcaccctgaagaagctaccacgcctggactgtatctgccgacagttgccaacaactttatcagcgcaatggcctgtggtgcgttgggctacaccgacgccggtctggtgtttttaggcgcaggcgttttctcatggctaagccttgaaccggtgatcttgcagcgtctgcgcagttcgggagaattacccacggcactgcggacatcactcggcattcagctcgctcctgcgctggtggcttgtagtgcctggctgagcgtcaacggcggcgagggtgacacgctggcgaaaatgcttttcggttatggactgctgcaactgctgtttatgctacgtctgatgccatggtatctctcccagccatttaatgcttcattctggagtttctcgttcggcgtatctgcactggcaaccaccggtttgcatctggggagtggcagcgataatggatttttccatacgctggcggtgccgctgtttatctttaccaattttattattgcaatactgctcatccgtacttttgcgcttctgatgcagggaaaattgttagtcagaaccgagcgcgccgttttaatgaaagcagaggacaaagaatgatcattcgtgacgaaaactattttactgataaatatgaattaacccgcacacactctgaagtactggaagcggtgaaagtggttaaaccgggtaaaacgctggatctgggctgtggcaatggtcgtaacagtctttacctggcagccaatggttatgatgttgacgcatgggataaaaatgccatgagtatcgccaacgtcgagcgcattaaatccattgaaaatctggataatttacacacccgagtcgttgatctgaataacctcacatttgatagacagtacgattttattctttcgactgtggtgctgatgttccttgaggctaaaaccatccccgggttgattgccaatatgcaacgttgcactaaacctggtggttacaacctgattgtggcggcgatggataccgctgattatccatgtaccgtcggcttcccgtttgccttcaaagagggagaattacgtcgatattacgaaggctgggagagggtgaaatacaatgaagacgtcggcgagctgcaccgcaccgacgccaacggtaatcgtattaaactgcgtttcgccacgatgctggcacgtaaaaaatgacccggtaagcacaaaacgcgtgaaaattccccacgctgagatgatttactgttcttcttttcggtaagcatattttttatcgaagggatgtgaaattaatcacagtagtcgaagtttttagcagcttaacttactgaaatttaagtactgatgattgacttagcccctttttcggcattgactatgtcgtctgaaaaggggctgaaaaatttattttcaccaacactttttttgccacaacacgaagcggcgctttttgctataacttagaaagtaatataatcatctcaggaaactattcatgcgtaccacatcatttgcgaaagttgcagctttatgcggcttattggctctgtctggttgtgcatctaaaatcacccagccagataaatattctggttttttaaacaattactctgatttaaaagaaacaacctcggctacaggtaaacctgttttacgttgggtagacccgagttttgatcaaagcaaatatgacagcatcgtctggaacccaatcacttattatccggtaccgaaaccgtcgacccaggtagggcagaaagttctggataaaattttgaactataccaacaccgaaatgaaagaagcgatagcgcagcgtaaaccactggttaccaccgctgggccgcgtagtctgattttccgtggggccattaccggtgtagataccagcaaagaagggctgcaattctatgaagtggttcctgttgcattagtggttgcggggacgcaaatggctacaggccaccgtaccatggatactcgcctctattttgaaggtgagctgattgatgcagcgactaataaaccggttatcaaagtcgttcgtcagggcgaaggtaaagacctgaataacgaaagtacgccaatggctttcgaaaatattaaacaagttattgatgacatggcgaccgatgccaccatgtttgacgttaacaaaaagtagttccagacgcgccatcgttagatggcgctttttatccggtgcgccgtaaaaccccatccttcagggcggggatataaggcgcggttttccacctgaccaggtgtttgctgttgttcaatgtattggcggatgacggatattggcgcacctccgcagctactggcaaaatagccaggactccacaaaacgcctttgtagtaatacctgaatgcaatatctggtcgatctcgtcgcagtcacctacccgatacgcctttgaggctgtttaccagactggatatcgccagtttgggaggatagttaattaacaaatggacgtgatctggttcgccatccatttcaaccagttcagcttcaaaatcagcacatacatttgaaaagtaagtgcgtagtttttctgtcgcgtcatggtcaaaaatctggcgtcggtatctggtgacaaagagcaggtgaacatgcatcaggaaaacacaatgccttccacgccggatatcggtttcttttttcacagaccaaagtatcatttgacctgtgaaacgattacaggcatttaaattccagttaagacccggtggtcaacaggagtgtgaaatgaggcgcttcgcaggcgcatgtcgtttcgttttcaatcgtgctctggcacgtcagaatgagaatcatgaggccggtaataaatacatcccttacgggaaaatggcttcctggctggttgagtggaaaaatgccactgaaacgcaatggcttaaagattctccctcacagccattgcaacagtcactgaaagaccttgagcgggcttacaaaaacttcttccggaagcgggctgcttttccccgattcaaaaagcggggacagaatgatgcattccgctacccgcagggcgttaagctcgatcaggaaaacagccgtatttttctgccgaaactgggctggatgcgctaccggaacagccgtcaggtcacgggtgttgtgaaaaatgtcactgtcagccagtcctgcggtaagtggtacatcagtattcagacagaaagtgaagtatcaactccggttcacccttcagcatcaatggtcgggctggatgctggcgtggctaaactcgccacgctgtcagatggcacagtctttgagcctgtaaacagttttcagaaaaaccagaagaagctggcgagacttcagcgacagttaagccgcaaggtcaaattcagcaacaactggcaaaagcagaaacgcaaaatacagcgactgcattcctgtatcgcaaatatccgcagggactaccttcacaaagtcacaacggccgtcagcaaaaaccacgcaatgatagtcattgaggatttgaaggtcagcaacatgtcaaagtcagcagcgggtacggtcagccagccggggcgcaatgtccgggcaaaatcaggtttaaaccgttcgatactggatcagggctggtatgaaatgcgccgccagcttgcgtataagcagctctggcgtggcggtcaggtgcttgctgttccgccagcgtatacaagccagcgttgcgcgtactgtggtcatacagcgaaagagaaccgcctgtcacaaagtaaattcagatgccaggtatgtggatatacagcgaacgccgatgtaaatggcgctcgcaacattttagcggcggggcacgccgttcttgcctgtggagagatggtgcagtcaggccgcccgttgaagcaggaacccaccgaaatgattcaggcgacagcctgaacgtagcagggatccacgtccttcagggcgtggaggatgtcaatatcggtttctgtcagcgattaaattcaacaccacgtaacaaacgcctccggcaattaatccccaaaacgcagaaccaatcccgaccagcgtcaatccacttgccgttaccagaaatgccaccaccgccgcgtctcgctcacgctcattatgcagcgcctgatacaaactgccgccgatggtacttaacagcgccagacctgccagcatctggatccaacttacgggcagggcagccatcatcccggtaatggcactaccaaacagacctgcgagcaaatagaaaatgcctgcaacggcagcggccagccaacgttgatctttatccggatgcgcttccgggctttggcaaatagccgcggtgattgccgcaataccgacggaataaacgccgaaaggggaaaaaaccagtgccagcaatccagtaaatacaattaatggcgaaacaggagccgaatatccagctgctttcattgctgcgatacccggtgcgttttgcgatgccatcgtcaccagaaaaagggggagtgcaacgctcaggctgtgagcaaacgaaaaatcaggggtaatataagtggggagaacgggtttaaagacaacatcagttgtgacaacgtcaccttgcgcgatgacgatcacgatcccaataatcatcgcggcaattaccgcatagcgcggcgcaacggccttggttgccagccataccagcaacatacttccacacaacgtaaattgaccgtccagactggcaaacgcctgtaaaccaaagcgtaataaaatcccggcaagcattgccgccgcaagcgagtgcggaataatgcgcatcagacgagcaaagagtcccgttatgccgcagaggactattagcgcgttggtgacaataaaaacgccgatggcttcgttaagtgttagtccctgcaatccggtgaccaacaaagccgcgccaggcgttgaccatgcggtgagaacaggtacgcgataccataatgtcagagtcagcgtactgacgcccattgccagccccagcgccgtcatccagccagagatttgtgcagtggtggctccggcgacaatcgctgcttgccagattattgccgctgaactggcgtagccaattaataccgccagaaaccccgccagtagcgtgggtggaggaatagaaaacagacgcatagtcacctcgtgcgttatagcgtacaggcaccgtagcatttgtccgttataacgcacaagtgataaacttccgttttgccggaggagtcgcatggaaaatctcgctcgctttttatccaccacacttaaacaactacgccagcagcgcggctggagtctttcgcgactggcagaagcgacgggcgtttctaaagcaatgttagggcagattgagcgtaatgagtccagtccgacggtcgcgacattatggaaaattgccaccgggttgaacgtaccattttcaacatttatttctccgccgcagtccgctacgccttcagtttatgatccacaacagcaggcgatggtgatcacttcgctgtttccttatgatccacaactctgctttgaacacttctcgattcagatggcatctggtgcaataagcgaatcgacgccccatgagaagggggtaatcgaacatgtcgtcgtcattgatggacaacttgatctgtgcgttgatggggaatggcagacccttaattgtggggaaggcgttcgatttgctgcagacgtcacgcatatctatcgtaatggtggggagcaaaccgtacattttcattccctcatccattacccgcgcagttaagcgggaaaactatttcgcaacgtcgcgcttgtggctaaaatagccgccatttttcagctactggataagaatgtgaccgtatcttctcatcgacttgaactgttaagcccggcacgcgatgccgccattgcccgcgaagctattttgcacggtgccgatgctgtttatatcggcggccctggttttggtgcccgtcataatgccagtaatagcttgaaagatattgccgagctggtgccgtttgcccatcgttatggtgcaaaaattttcgtcacgcttaacaccattttgcatgatgatgagctggaacccgcgcaacggctgattactgacctctaccagaccggtgtcgatgcgctgattgttcaggatatggggattctggaacttgatattccgccgattgaactgcacgccagtacgcagtgcgacattcgtacagttgaaaaagcgaagttcctctctgatgttggcttcacgcagattgtgctggcgcgagagctgaatcttgatcagatccgcgcgattcaccaggctacggacgcgaccattgaattctttattcatggggcactgtgcgtggcctattcgggtcagtgctacatttctcatgcgcaaacagggcgtagcgccaaccgtggcgattgctcgcaggcgtgccgtttgccatacacattgaaagacgatcaggggcgggtggtttcctatgaaaaacatctgctgtcgatgaaagataacgatcagactgccaacctcggcgcgctgattgatgctggtgtacgctccttcaagattgaagggcgttacaaagatatgagctacgtgaagaatatcaccgcccattatcgccagatgcttgatgccattattgaagaacgtggcgatctggcgcgcgcttcatcaggtcgtactgaacatttctttgttccatcgacggaaaagactttccaccgtggtagcacagattattttgtgaatgcccgtaaaggcgatattggcgcgttcgattcgccgaaatttatcggcctgccggtaggcgaagtagtgaaagtggcgaaagatcatctcgatgttgccgttaccgagccactggcaaatggcgatggcctgaacgtgttgattaaacgtgaagtcgtcggttttcgtgccaatacggtcgagaaaaccggagaaaatcagtaccgcgtctggcccaatgaaatgccagcagatttgcacaaaattcgtccacatcacccactaaaccgtaatcttgatcataactggcagcaggcactgacaaaaacctccagcgaacgtcgggtggcggtagacattgaactgggcggctggcaggaacaactgattctgaccctcaccagtgaagagggtgtcagcatcacgcatacgctggacgggcagttcgacgaagccaataacgccgaaaaagcaatgaacaatctgaaggatggtctggcaaaactggggcaaaccctctattacgcccgcgatgtgcaaattaatttgccgggggcgctgtttgtaccaaacagtctgttaaaccagttccgccgtgaagctgctgacatgctggatgctgcgcgtcttgccagttaccagcgcggcagccgtaaaccggttgctgatcctgcgccggtttatccgcaaacgcatctgagtttcctcgcgaacgtatacaaccagaaagcgcgtgaattttatcatcgctatggtgtgcagctgattgacgcggcgtatgaagcacatgaagagaagggcgaagtcccggtgatgatcaccaagcattgtctgcgctttgcctttaatctgtgcccgaaacaggcgaaaggcaatatcaaaagctggaaggcgacgccaatgcaactggttaacggcgatgaagtattaacgctaaagtttgattgccgcccatgcgagatgcacgtcattggcaaaatcaaaaatcacatactgaaaatgccgttaccgggaagcgtagtggcatccgtaagtccggatgagctgctgaaaacattgccgaagcgaaaagggtaaaacgccagttttctggttactcacaacttattgaatctgcatgatattgcctgccgggtaaggcgttacgccgcatccggcatcaaatgactcaacgttgtcccgcttctggtttgcgcgatttttgccagtaaaaatgctcgcgcaaaccttccgccgactcttccgccacagcacgcaattcatcgctgtccgcttcatgacgcagctgatgatccacattctttacccacacaaattcatgtcctttgtgccctgccatgagttgtcctgaaaacagagcacacgttaataagacaaccgataacgccttcgtaaacatcctgccacctttttcttaccttttgccgctatgatgccgatcgtttcttgaggttattattcagttttgcaaattagcgcaaagaaattctggaatcttccttcctgattttgcattgcattctgccgttgcggcgatttagtgctattttcgagcaaattacacacggaggtaaacactaatgtttactttgttgatatactcagcggcagggaggcgatgtgaaacaaagcgagttcagacgttggctcgaatctcagggcgtcgatgtagcgaatggcagcaaccatttgaaactcaggtttcatgggaggcgcagtgtcatgccgcgtcacccctgcgatgagattaaagaaccattgcgtaaagcaatcctgaaacaactcggtttgagttaatcgccaattaaaaaggttaatgacatgcgagagacagtcgaaattatgcgttatcccgtcactcttacacccgcgccggaaggcggttatatggtttcttttgtggatatccctgaagcgttgacccagggcgaaactgtcgctgaagcgatggaagcggcaaaagatgctttactgaccgcatttgatttttattttgaagataacgagcttatccctttaccttcgccattaaatagtcacgatcactttattgaagtacctttgagcgtcgcctctaaggtattgctgttaaatgcttttttacagtcagaaatcactcagcaagagttagccaggcgaattggcaaacctaaacaggagattactcgcctatttaacttgcatcatgcgacaaaaatcgacgccgtccagctcgcggcaaaggcgcttggcaaagagttatcgctggtgatggtttaattacagttaacgaaaagttgtcatttttaacaactgatatagactgccgaatcatctgcacataattacgattcgataatgaaaaaataccagcagcttgcagaacaattacgcgagcagattgcgtcgggtatctggcaacccggcgatcgtttgccttcgttgcgtgaccaggtggcgctttcaggcatgagctttatgactgtcagccatgcctatcagttgctcgaaagtcagggatatattatcgcacgaccgcagtcgggttattacgttgcgccacaggcaataaaaatgccgaaagcgccagtcattccagtcactcgagatgaagcagtcgatatcaacacttatatttttgatatgttgcaggccagtcgcgatccgtcggtcgttccgtttgcctcggcctttcccgacccgcgacttttccccctccaacaactaaaccgctcgctggcgcaggtaagcaaaaccgccacagcgatgagcgtgattgaaaacttaccgccaggaaacgcagaactgcgtcaggctattgctcgtcgctatgccttacagggcatcaccatttctcctgatgaaattgtcattactgccggggcgttagaggcattaaacctcagtttgcaagcggtaactgaaccgggcgattgggtgatagtagagaatccttgtttctacggtgcgttgcaggcgctggagcggctacggctgaaggcgttatcggtggcgacggatgttaaagaagggatagatcttcaggcgctggaactggcgttgcaggagtatccggtgaaagcgtgctggctgatgactaatagccagaatccactcggatttaccttaacgccgcaaaaaaaagcacaactggtggcgttgctcaatcagtacaacgtaacgctgattgaagatgacgtttacagcgaactttattttggacgggaaaaaccgctgcctgcgaaagcgtgggatcgccacgatggcgttttgcattgctcttcgttttcgaaatgtctggtgcctggttttcgtattggttgggtcgccgccggaaaacatgcacgtaaaattcaacgcttgcagttgatgagtacgctttccaccagctcaccgatgcaacttgcgctggtggattacctttccacgcgccgatacgacgcccatcttcgtcgcctgcgtcgccagcttgcggaacgtaaacaacgtgcctggcaggcactgctgcgttatctgcctgcggaagtgaaaattcatcataatgacagtggttactttctctggttggagctccccgagccgttagatgccggcgaattaagcctggcggcactgacgcatcatatcagtattgcgccgggtaaaatgttttctaccggtgaaaactggtcacgttttttccgttttaataccgcgtggcagtggggagagcgtgaagaacaggcggtaaaacaattaggcaaacttattcaagaacggctgtaatagcgtttaatttaattcctcttagattgggtaatatgaatttcgaatagcagtcatatttcctaactccttgactatactccagaagataaccttacagacggcataatgcgcggtagctcacaacctgaataaattttctcaggggcgaaggtgtgcctgcaagccgccgtctatggttaaacaaggagatatttttacggcacggcggctgaacaattaattacgacaggagtaagaccttatgagcaagacatttgcccgcagcagcctgtgtgcgctcagcatgacaataatgaccgctcacgccgccgaaccgcctaccaatttagataaaccggaagggcgactggatattatcgcctggccgggatacatcgaacgcggacaaactgataaacaatacgactgggtaacgcagttcgaaaaagagacaggctgcgcggtgaatgtgaaaaccgccgcgacttccgatgaaatggtcagtctgatgaccaaagggggttacgatctggttacggcatccggcgatgcctcgctgcgtttgattatgggtaaacgcgtgcagccgattaataccgcattgattcccaactggaaaacgctcgatccgcgcgtggttaaaggcgactggtttaatgttggcggcaaagtttacggcacaccttaccaatgggggccgaacctgctgatgtacaacactaaaaccttcccgacgccgccggatagctggcaagtggtttttgttgagcaaaatctgccggacggcaagagcaataaaggccgcgttcaggcttatgatggccctatctatattgcggacgctgcgttgttcgttaaagccactcagccgcagttgggcatcagcgatccgtatcaactcaccgaagaacagtaccaggcggtgctgaaagtgctgcgcgctcaacacagtttgatccatcgctactggcatgacactaccgtgcaaatgagcgatttcaaaaacgagggtgtggttgcttccagtgcctggccctatcaggccaacgccctgaaagccgaaggccagcctgttgctaccgttttcccgaaggagggtgttaccggttgggctgataccaccatgctgcatagcgaagcgaaacatccggtttgcgcctacaaatggatgaactggtcattaacgccaaaagtgcagggcgatgtggcggcctggtttggctcgttaccggtagtgccggaagggtgtaaagccagtccgttattaggcgaaaaaggttgtgaaaccaacggttttaactatttcgacaaaatcgccttctggaaaacgcctatagcagaagggggcaagtttgttccctacagtcgctggacgcaggattacattgccattatgggcggtcgctaacttcgctggggtgctttatgacgtacgcagtggagtttgacaacgtctcgcggttgtacggtgacgtgcgcgcagtagatggcgtcagtattgcgataaaagatggtgagttcttctctatgctggggccgtccggctccggcaaaaccacctgcctgcgcctgattgctggcttcgaacagctttccggcggggctatctctatctttggtaaacccgccagcaatctgccaccgtgggagcgggacgtgaatactgtctttcaggactacgcgctatttccgcatatgtcgattcttgacaatgtcgcctatgggctgatggtcaaaggcgtgaataaaaagcagcggcacgcaatggcgcaagaggcgctggagaaagtggcgttggggtttgtacatcaacgtaaaccgtcacaactttctggtggtcagcgccagcgggttgctatcgccagagcattggtgaatgaaccgcgcgtattgctgttggatgaaccgctcggcgcactggatctcaaattgcgtgagcagatgcagctggaactgaaaaaactgcaacagtctctcggtatcacttttatcttcgttacccacgatcagggcgaagcgttatcgatgtccgatcgtgtggcggttttcaataatggacgcattgagcaggtcgattccccgcgcgatctctatatgcgcccgcgcacgccgtttgttgccgggttcgttggtacatcgaatgtttttgatggactgatggcagagaaactttgtggcatgacgggaagcttcgccctgcgaccggaacatatccgcctcaacacccctggtgaactgcaggccaatggcacgatccaggcggtgcaatatcagggcgcggcaactcgttttgaactgaaattgaacggcggtgaaaaactgcttgtgagtcaggccaatatgacaggcgaagaactgcctgccacgctcacgcccggacaacaggtgatggtttcctggtcgcgtgatgtgatggtgccgctggttgaggagaggtgaatggcgatgaatgtattgcaatcaccttcacgtccaggtctgggtaaggtgtccggtttcttctggcataatccggggctggggctgtttttactgctgcttggcccgctaatgtggtttggcattgtctatttcggctcgctgctgacactgttatggcagggattttatacttttgacgatttcaccatgtcggtaacgccggaactgacgctggcgaatatccgtgcgctgtttaatccggcgaattacgacatcattctccgcacgctgactatggctgtggcagtcactatcgccagcgccattctggcttttccaatggcgtggtatatggcgcgctataccagcgggaaaatgaaagcgtttttttatattgcggtaatgttgccgatgtgggcgagctacattgttaaagcctatgcctggacgttattgctggcaaaagatggcgtggctcagtggtttttacaacatcttgggctggaaccactgctgactgcgttccttacattacctgcggtgggcggaaatacgctgtcaacttccgggctggggcgctttctggtgtttctctatatctggttgccgttcatgatcctgcccgttcaggcggcgcttgagcgtttgccgccgtcattgttgcaggcgtcggctgatctcggcgcacgtccacgacaaacctttcgctatgtggtgctgccgctggcaatcccgggtattgccgctggctctatctttaccttctcactcacactgggcgattttatcgtcccgcagctggttggtcctccaggatattttatcggcaatatggtttattcccagcagggggcgattggcaatatgccgatggcggcggcattcaccctggtgccgattattctcatcgcactgtacctggcgttcgtgaaacgtctgggagcgttcgatgcactctgaacgcgcaccgtttttcctcaaactggcggcctggggcggcgttgttttcctacattttcccatcctgataatcgccgcctatgcgtttaacactgaagatgcggcgtttagttttccaccgcagggcctgacgctgcgctggtttagcgtggcagcacagcgtagtgatattcttgatgccgtgacactgtcacttaaagtggcggcgctggcgacattaattgcgctggtgttagggacgctggcagctgccgcgctgtggcgacgagactttttcggcaaaaacgccatttcgctgttactgctgctgcccattgcgctgccgggcattgtcactggtctggcgttattaaccgcctttaaaaccatcaatctggagccgggatttttcaccatcgtggtcggtcatgcgactttttgtgtagttgtggtgtttaacaatgtcatcgcccgttttcgccgcacctcctggagtctggttgaggcgtcaatggatcttggggccaatggctggcaaaccttccgctacgtagtgttgccgaatctcagttcggcgttactggcaggaggaatgctggcgtttgccttgtcgttcgatgaaatcatcgttacgacctttacggcaggtcatgaacgaacgttaccgttgtggttgctcaatcagcttgggcgaccgcgtgatgtaccggtaactaacgtggtggcactgctggttatgttggtaacaaccttgccgatcctgggggcctggtggctaacccgcgaaggcgacaatggtcaataaccactgatacaggaatatgctatgcaacataagttactgattaacggagaactggttagcggcgaaggggaaaaacagcctgtctataatccggcaacgggggacgttttactggaaattgccgaggcatccgcagagcaggtcgatgctgctgtgcgcgcggcagatgcagcatttgccgaatgggggcaaaccacgccgaaagtgcgtgcggaatgtctgctgaaactggctgatgttatcgaagaaaatggtcaggtttttgccgaactggagtcccgtaattgtggcaaaccgctgcatagtgcgttcaatgatgaaatcccggcgattgtcgatgtttttcgctttttcgcgggtgcggcgcgctgtctgaatggtctggcggcaggtgaatatcttgaaggtcatacttcgatgatccgtcgcgatccgttgggggtcgtggcttctatcgcaccgtggaattatccgctgatgatggccgcgtggaaacttgctccggcgctggcggcagggaactgcgtagtgcttaaaccatcagaaattaccccgctgaccgcgttgaagttggcagagctggcgaaagatatcttcccggcaggcgtgattaacatactgtttggcagaggcaaaacggtgggtgatccgctgaccggtcatcccaaagtgcggatggtgtcgctgacgggctctatcgccaccggcgagcacatcatcagccataccgcgtcgtccattaagcgtactcatatggaacttggtggcaaagcgccagtgattgtttttgatgatgcggatattgaagcagtggtcgaaggtgtacgtacatttggctattacaatgctggacaggattgtactgcggcttgtcggatctacgcgcaaaaaggcatttacgatacgctggtggaaaaactgggtgctgcggtggcaacgttaaaatctggtgcgccagatgacgagtctacggagcttggacctttaagctcgctggcgcatctcgaacgcgtcggcaaggcagtagaagaggcgaaagcgacagggcacatcaaagtgatcactggcggtgaaaagcgcaagggtaatggctattactatgcgccgacgctgctggctggcgcattacaggacgatgccatcgtgcaaaaagaggtatttggtccagtagtgagtgttacgcccttcgacaacgaagaacaggtggtgaactgggcgaatgacagccagtacggacttgcatcttcggtatggacgaaagatgtgggcagggcgcatcgcgtcagcgcacggctgcaatatggttgtacctgggtcaatacccatttcatgctggtaagtgaaatgccgcacggtgggcagaaactttctggttacggcaaggatatgtcactttatgggctggaggattacaccgtcgtccgccacgtcatggttaaacattaaggataatattgcagatcgtaagagtatgagatgatcttgcgtactgtcagagcactgatttctctgacagtacgtgctgcgtgcaaaatcactacatcaaataaaccagccaaatctcatagagataagagtaaacaaaccaacagcagcaaagaaatttatcagtactacagttctactggaaacattcatttttgccaccttttatcattgcccctatgtgtatagtacgggttaagaaaatccgcaataatactcattctgaagatggataagggcaagttgctgtttgatgattttttctcaaactggtgaaaaaacttgatgcacgtcaaaaaatgacgcatatttgcgcgcgttttattcatctggctggacgcccgtacatgtctctctatcaacacatgcttgttttttatgcggttatggcagcaatcgcatttcttatcacctggtttctttctcacgataagaaacgcatccgtttcttaagcgcctttctggtgggggcaacatggccgatgagtttcccggtggcgctgttgttttcactgttttaaatcttactcactggcttgacggcaccacgcagacttatatcatttggatgaatcgataaatttcacaagtggctaaggagaaagtatgtcgcatctggatgaagtcatcgcgcgcgtggatgccgcgattgaagagagcgtcattgcccatatgaacgaattattaatcgccctgagcgatgacgcggagttaagtcgggaagatcgctacacccagcagcaacgtctgcgcacagcgatcgcccatcacggtcgcaagcataaagaagatatggaagcgcgccacgaacagttaaccaaaggcggcaccatcctctgattaaaatgagcgtctggctaccaaccaggcgccaaccacaagtaaaattgcgccacaaattgggccgaacaacgcccgtagtggtacgccatgactgcggaagatatccagcatcagaccgccaatcagctgactggcgaccagtacagcaatagttgtcgccgctcccacattctgatatccgctgatactggcgaagacaaaaaacgatcccagcaagccaggtataagtgtccaccagcgcacgctggacaccagttcgccaaaccccgccatgccttgtttaaaccataaaatagaaacaaagagcacaatccccaccagtgagttcagcaacatggcgatgagaatggtagaggaggtctgggtgatgcgcaccatcagcgtgttctggacaaccagaccaattccggcggcaatcaaaaaagcaagggtgagcgactgattcatccaatcgcgtccggttcagtgcgctcgtcgagttgcaactgcataaatgtcagatccagccaacgaccaaatttagtgcctacctgcggcatttgcgcggtgacgacaaatcccagcgactggtggagatgcagcgaggcctgattttgcgattcgatcccggcgaccatgacatgcttcccgcaatcccgcgcttcatcaatcaatcggcttaacaatttacgccccagacctttgccctgatgatcgggatggacataaaccgaatgttccacggtatggcgaaaaccatcgaaactacgccagtcgccaaacgaggcatatcccgtcactacgccgttttcctcgctcaccagcactggataacctgctaaagtccgcgcttcaaaccaggcaatgcggttatcagcatccaccgtttggtcattccagatagccgccgtatacaacacggcgtggttataaatttccgcaatggcagcacagtcggctttgcgggcaaaacggatggacatgtctggcctcaataaaataatgatgatgatgttatcaatactatcgaaaacagcccgaagcaacggattcctcgatgaaattattgcgtgttgcagaggggatgtgacggctgcaaacaaaaccaatcccgtgagcctgctactattgatggattcatgccaaaagcacaggagagcattatggggcaacaaaagcagcgtaatcgacgttgggttctggcctcgcgtccacatggcgcacctgttccggagaatttccgtcttgaagaagatgatgtcgccacaccgggtgaaggacaggtgttactgcgcacagtttatttgtccctggacccgtatatgcgtggacgtatgagcgatgagccatcttattcaccgcctgttgatattggcggcgtgatggtcggcggtacggtgagccgtgtcgtggagtcgaatcatcctgattatcagtctggcgactgggtgctgggctacagtggatggcaagactatgacatatccagtggtgatgatctggtgaaacttggcgatcatccgcaaaatccatcgtggtcgctgggtgtgctagggatgccaggctttaccgcttatatgggcctactggatatcggtcagcctaaagagggcgaaacgttggtggtagctgcggcgacaggaccagtgggggcgacggtggggcaaatcggcaaacttaaaggttgcagagtggtgggggtagccggtggcgcggaaaaatgccgccatgctaccgaggtgttaggcttcgatgtttgtcttgatcaccacgcggatgattttgccgaacaactggcgaaagcgtgcccaaaaggtattgatatctattatgaaaacgtgggcggtaaggtattcgatgcggtgctaccgttacttaatacatctgcgcgcattcccgtctgcggattagtgagcagctataacgctacagagctaccacccggtccggatcgtttacctctgttgatggctacagtgctgaaaaaacgtattcgcttgcaaggttttattatcgctcaggattatggtcaccgcatccatgagtttcagagggagatggggcaatgggtgaaagaggataaaatccactaccgcgaagaaattactgacggtttagagaatgcgccacagacgtttatcggcctgctgaagggtaaaaacttcggcaaagtggtgatccgcgtggcgggtgatgattaaagtttcaacggcggcgtaagccgccataaaaatccaggcaaaaagcttattttcagctttaattaactaaccacatcattgttctgctgctaataacaacaaaggtgagtggtttatgattattcactttaatacaccaggtgaattccttctgccatgcaggcagggttggacagaaaacacgcgaaggaattaaaatgcctggaacgggaaaaatgaaacatgtcagtttgactctgcaggttgagaacgacctgaaacatcagcttagtattggcgcattaaaacctggcgcacgcctgattactaaaaatctggcggagcaattaggtatgagtattacacctgtgcgtgaagcattattacgtctggtttcggtgaatgcgctttctgtcgcacctgcacaagcatttacagttccggaagtggggaaacgtcaattagacgaaatcaatcggatccgctacgaactggaattaatggcagttgctctggctgttgaaaacctcaccccgcaagaccttgcggaactccaggaattgctcgagaaattacagcaggcgcaagaaaagggcgacatggaacaaatcattaatgtaaacaggctatttcgcttagcgatttatcatcgctcaaatatgcccatcctgtgtgagatgattgagcaactgtgggtcaggatggggcctggtttacattatctctatgaagcgattaatccagcggaattacgggagcatatagaaaactatcatctgttactcgctgcgttaaaagcaaaagacaaagagggatgcagacattgtcttgctgaaattatgcaacaaaatattgctattttataccagcaatacaatcgttaaagtaaatgcccggcaaataccgggcatcaaggtaattactcaaatctccacgcaatattcatgccgacaccataatttcgtccgggcgaaggttcgtaatatcgcccgtttgactcattgacaatgacagaaccaacgtattctttatcgaataaattatcgacacgaccaaataaatccacagttaaattgtggtaattgtatttatacccggtgaataagccgacgagagtataagacggcgcttttgccgtattttcatcatctgccataatatcgcccatataacgcgcttccgtgcctgcataccaaccatcttccggtacataacctatcgacgcaaagcccatattacgggcgatccctggcatccgattaccgttacaatcctgttcattgcaaacattgctgcgataggtcgcatcaagccaggtccaggacgcgtttacgcgaaaatctcctgcgaaacgttgatcccatgccagttcagcgccttgacgacgggtctttccggcatttttgtaagtcgtacgcccaccgctactgctatcgacaacaatttcatcatcagtgtcggtctgaaacaatgcgagactaagcagcccatcaccaatacgcgttttactgccgatctcaattgtatcgttggtggatggttttaaacctaagttcataccgctttgcccatcagcacgataagacagctcattaatcgtcggcgtttcaaaacctcgcccggctgccagatagatattccaggcatcggtcattgcatattttaacgaaccggcaggtagccatttatgataactggcatcaccgctgtcatcgccgttacccggagtaacgtaatggtcgttggaatcaaaccacacggagctgtagcgcacgccagcatccagcgacagtttttcgctcagctgccactgcgtctgtaaatagggatcgatgttccacatcagattgcgttcgtcgcgacgcaactcacctttttgcccgtactccggcatgccgctattcaggcggaagttattgtagcccttgcggttttcactcatgttttcgtagttcaggccggtagtgaacgtgaccggaacgcccagttcaccacggtgtgtccagcggctgtctattccctggtaatggcgttgcagggtaatcacgccgcccgcatgtgacgggttaagttgtggtgccatgggtattgactggtactgggtcgtttctcgctctccggcatacatcatcacactcatatcatcccgcgaactcaggctacgctcatagcgcaacccagcctgagtttgcttgatggtttttcgcgtgtcgtactgttctgcacgaggcgcttgttgtggattagccttccattctgctttggttagcccacctgggtcatctgctttgatatccacactattgaaaatcagacttaatttgctggcttcatcaatgcgtacgcccagtttggcattggctaaatttttctgtgcgccactatggtcacgatagccgtgggtcgtaaaacgcgtggttgagacggtgtaatcgacatcgccaggctgtgtgccgtctcccgttgcgcccgttgctttcagcccatagcgccagctgccaaaactgccgtagtaactactggcttcaatggttggtggctgttgtccggtctgggtggtgacattcattaccccaccagacgcgttgccatacagggcagagaaggggccacgcagcacttccacattttgcacactgcttaaatcgatgttggatgtttgcccttgcccgtcgggcatggtggcgggaataccgtccacatacaggcgaataccgcgaataccgtaagtggagcgggagccaaatccgcgaatcgacagctgtaaatcttgcgcatagttctgccggttttgtacctgcaaaccaggcacgccggtcagtgattcggacaagttaatgcgcggtgttgccaggcgcatctcctcgccatccaccacgcttactgctgctggggtatccagttctgaaaccacctgcggtgcggcactgacaatcatagtctgttcatcagcggcaaaaacaacgggggaaaggacaagcagtgcgggcaaaacggtctgtcggacggaaaaaatcttcatgaaaaaagccaggttaagaatgggaaaacgccgtcatggtaatgaaattgtaaatttatggaaaatgaaacggcacaatacgttaagtaattgagaaaattgtagtcgtaacggcaagaaatgctccacatttgagaaaataatgattaccattcccatttataacaagagcgtaacgatgattacgcttagcgaagcattgtgaagcagcaaaaatatcggttcatcaaagggagtcgtcatgcatttacgtcatctgttttcatcgcgcctgcgtggttcattactgttaggttcattgcttgttgtttcatcattcagtacgcaggccgcagaagaaatgctgcgtaaagcggtaggtaaaggtgcctacgaaatggcttatagccagcaagaaaacgcgctgtggctcgccacttcgcaaagccgcaaactggataaaggtggcgtggtttatcgtcttgatccggtcactctggaagtgacgcaggcgatccataacgatctcaagccgtttggtgccaccatcaataacacgactcagacgttgtggtttggtaacaccgtaaacagcgcggtcacggcgatagatgccaaaacgggcgaagtgaaaggccgtctggtgctggatgatcgtaagcgcacggaagaggtgcgcccgctgcaaccgcgtgagctggtagctgacgatgccacgaacaccgtttacatcagtggtattggtaaagagagcgtgatttgggtcgttgatggcgggaatatcaaactgaaaaccgccatccagaacaccggtaaaatgagtaccggtctggcgctggatagcgaaggcaaacgtctttacaccactaacgctgacggcgaattgattaccatcgacaccgccgacaataaaatcctcagccgtaaaaagctgctggatgacggcaaagagcacttctttatcaacattagccttgataccgccaggcagcgtgcatttatcaccgattctaaagccgcagaagtgttagtggtcgatacccgtaatggcaatattctggcgaaggttgcggcaccggaatcactggctgtgctgtttaaccccgcgcgtaatgaagcctacgtaacgcatcgtcaggcaggtaaagtcagtgtgattgacgcgaaaagctataaagtggtgaaaacgttcgatacgccgactcatccaaacagcctggcgctgtctgccgatggcaaaacgctgtatgtcagtgtgaaacaaaaatccactaaacagcaggaagctacccagccagacgatgtgattcgtattgcgctgtaatagatatggcgagggtgaaaacggtgagacttgcctgccttttatcacggcgtatccggcactttcgtcagtaatctgaatttgcccggcacgtagccgggcaattttgcaattaactcgccgtttcaggcttaaacacaatttcctgtttttcttcatcttcctcgacgactggcgcagtgctgtgaatttcagcaacgcgtttgcgcacaccaaaccagcctataaccagcaaaataccgataatcggcagcgccgcgatagtataagtcccgttcgggtaatcgaacgccatcagcacaaggacactcagtaaaaacagtaatgtcagccaggaagtgaagggcgcgccaggcagtttaaaactgacatccgctgctttgccttctttaatcgctttacgcaggcgcatctggcacacgatgataaacgcccatgaagcgatgattcccagcgacgcgaagttcaacacaatctcaaatacgcgcgacggcaccagatagttgaggaatacgccgacgacatacacaactagtgtcgccagaatcccggcatacggcacatgctgacgactcattttcgccataaaactcggtgcggaaccgcccatcgccattgagcgcagaatacgtccggtgcagtacagacctgaattcaggctggagagggcagcggtcagcaccacaatgttcataatgctgccgatatatggcacacccagtttagagaaaaacgtcacgaacggactttgccccgcctgatacgcgctccacggcaataacataaccagcaacaccacggagccgacgtaaaacaggccaatacgccaaatcacactgttaatggctttaggcaccatggtctgcggatctttacattctccggcagctgtacccaccatttcaatggaggcaaaagcaaacactacgccctgaatcaacaccagcgcaggcagcaaaccgtgggggaagaagccgccattatcggtgattaaatgaaagccagtggtgttgccatccagcggctgaccactaccgaggaacactgtacccacgaccaaaaaggtcacaatggcgagcactttaataagcgcaaaccagaactccatctccgcaaaccatttcacaccgatcatattcatggtgccaacgatggtaagtgcagcgagcgcaaagacccactgcggcacgccgccaaacgcaccccagtaatgcatatacagagcgacggcggtaatatcaacaatccccgtcatcgcccagttgatgaagtacatccagccagcaacataagcggctttctcacccaaaaactcacgggcataagaaacaaaactgccactggaagggcggtgtagcaccagctcacccaatgcacgcagaataaaaaacgaaaacaagccacaaattaaataaaccagtgccagtgcgggccccgccatttgcagtcgggctcctgcacctaaaaacaagccggtgccaatcgcgccgccaatggcgatcatctgcacctggcgattgcccatcgctttgtgatacccctcttcgtgggcattaagccagcggcgtttcgcggcgtgttgatctgaagtgtcggtgtcgtgtttactcattgctctccctgattgctttaatgaaaaagtcatataagttgccatgaacaatgtttattcatcctggcgatgatagttatcaccattattctttatgggtataaaactatcggcgcagcatcctacccgttatcgataaacgatgcaaaacatccccttacaatcctgaaggggattaatacaactgacgaaaaaatgacaaatccttttgctggttaacctgtgtactgtcctacacttaatctttaaaagattgtgaggggcatatgattaaggtgtatggcgtacccggatggggctctacaatcagtgagctgatgctaacactggctgatattccttatcagttcgttgatgtcagtggttttgaccacgagggagcttcacgcgagttattgaaaaccctgaacccgttgtgtcaggttccgacactggcattggaaaatgacgagattatgacggagacagcggcgattgcattgatggttctcgatcgtcgcccggaccttgcgccaccggttgggcgcgccgaacgtcagctgtttcaacggctattggtctggctggttgctaatgtctatccaacattcactttcgccgattaccctgagcgttgggctcctgacgcacctgaacagttaaagaagaatgttattgaatatcgaaaatcgctttatatctggttgaattcgcagctcactgctgaaccttatgcgtttggtgagcaactaacgctggtggactgttatctttgcactatgcgcacatgggggcctgggcatgaatggtttcaggataatgccacgaatatcagtgcgattgctgatgctgtatgtcagttaccgaaattacaagaagtattaaaaaggaatgaaattatttgagtgggataccagaagattatgttatttattattcagtaactttatccacaatgatgggcgtaattaattaaattcatggtatgttttttaatttatatcactctccttttcattcagcgtgtctatttcatttcctctgaaaagaaactaactattcacatcgtgcagatgtttcagttgttatcacaggcattctataatctcaaaatgtttttaatgatggatatgctcggagttggagatgcaattaatattaatacaaataaaaatatccggcaggtatgctaaaaggataaatggcgttctctgtatttattcgcaattatctgtaggacaaatatggagagcttgatgagtcagagctaaaacagcaattgattaataaacatgttgatttattcaagaaaatggatgtattttaaatgttgattcttaatataacctaatcaatagattatcaagtgagagctacacattattggaggggcaggggaaaacaccattttgggaacaatgcatcaggtactcttaccactgaagcaagatcatccggcaccaggtggtggtgcagtgctttggaaatggtcccctcgggggagttgtcattattttctatgctatttgcttattatattcatcaggtgaatttaataaattcctaatttgaaatatccactattaagctagtgtttaacgacgttaagatggcaatgtgcagatcatgttatcagggtggggcggtagcgtatattccttatacaaaccatcattcatttcaatgattgttattgaattatttattgttgtgaataaaaagacattatgaatattggtttgactttgcatatcaggttttttattactcgctgtaatgtacgagcctgtcgtgaataacgtcgagaacccatccgttgcgtttgtgattattttgttgactaaacagacacccgtttctctgaagtaaaatcccagactaaatcatcacataaccatgacatttttctgatattccccggtaacgccagatgtcgactcgcttaaccaccctcagccataccagtgaaggccaccgcgtgtcggtccactacggctatgacgataaaggccgcctgaccggcgaacgccagacggtggagaacccggagacgggggaactgctgtggcaccatgagaccggacatgcgtacaacgaacaggggctggcaaaccgcgtcacgccggacagtctgccgccggtggagtggctgacctacggcagcggctatcttgcgggcatgaagctgggcgggacgccgctgctggagttcacgcgcgaccgcctgcaccgtgagacggtgcgcagcttcggcagcatggcaggcagtaatgccgcatataaactgaccagcacatacacccccgcaggccagttacagagccagcacctgaacagcctggtgtatgaccgtgactacgggtggaatgacaacggcgacctggtgcgcatcagcggcccgcgacagacgcgggaatacggctacagcgccacgggcaggctggagagtgtgcgcaccctcgcaccagacctggacatccgcatcccgtatgccacggacccggcgggcaaccggctgccggacccggagctgcacccggacagtacactcacagtgtggccggataaccgcatcgcggaggatgcgcactatgtctaccgccacgatgaatacggcaggctgacggagaagacggaccgcatcccggcgggtgtgatacggacggacgacgagcggacccaccactaccactacgacagccagcaccgcctggtgttctacacgcggatacagcatggcgagccactggtcgagagccgctacctctacgacccgctgggacggcgaatggcaaaacgggtctggcggcgggagcgtgacctgacggggtggatgtcgctgtcgcgtaaaccggaggtgacgtggtatggctgggacggagacaggctgacgacggtgcagactgacaccacacgtatccagacggtatacgagccgggaagcttcacgccgctcatccgggtcgagacagagaacggcgagcgggaaaaagcgcagcggcgcagcctggcagagacgctccagcaggaagggagtgagaacggccacggcgtggtgttcccggctgaactggtgcggctgctggacaggctggaggaagaaatccgggcagaccgcgtgagcagtgaaagccgggcgtggcttgcgcagtgcgggctgacggtggagcaactggccagacaggtggagccggaatacacaccggcgcgaaaagttcatttttaccactgcgaccaccggggcctgccgctggcgctcatcagcgaagacggcaatacggcgtggcgcggggagtatgatgaatggggcaaccagcttaatgaggagaacccgcatcacctgcaccagccgtaccgtctgccagggcagcagcatgatgaggagtcggggctgtactataaccgtcaccggcactacgatccgttgcaggggcggtatatcaccccggacccgattgggttgagaggtggatggaatatgtatcagtatccgttgaatcccatacaagtgatagacccaatggggttagatgcgattgagaatatgacatcaggtggactaatttatgccgtatctggtgtacctggattgattgctgcaaacagcattactaacagtgcttaccagttcggttatgatatggatgctattgttggcggagctcataatggggccgccgatgcaatgagacattgttacttgatgtgtcgaatgactaagacatttggatcaacaatagctgacgtgataggtaaaaatcatgaggcggcaggggatagacaaggtcagccagctaaagaaagaatcatggatcttaaaaataacactgtcggtattgcttgtggcgatttttctgccaaatgtagcgatgcatgtattgaaaaatataacactgggcaactcttcgggttagatggtataaaagcagataatccaataaaagcaaagcaagggagttcagatgcttcaaattattagaggcaaacttgtcatttttttaattaccctttgtttatttgttgtttaccttgggtttgataacaattcaaattctgacatcgtattttatggacataaaacaccaaagagcgttgagatatatctttctgaaaaaaatattatttataaaataattaatgaccaaaaaattagtagagggaatggtcattttataagtataatggttaataattacaggacgcactgtggagtggttgatataaatcttaattttttcaatgatattctttatagcgtgcgattaaaaaacattagtaaactggagaatatggagttctgcgctacaaaacaacgggtgtattttagtgataaaaacaagaaggctagttataaaataattaattatggagactattatgatgttgattattatgataacaatttgaaaaatgaagtttttgactggattggtaaatggtcataatgaacaacaccagaaagagaaaaatataaaatacatacagaaagacatgagagcaagggacggggcagggcaagatcatgaaaattgtgatgtaaatcacgattttcatctttgctttaacgcctacaggtgatcaaaatttaacctttggaataactaaaaagataaaaaaggacgccaggtgagtattcaaagtttgcttgattatatttcagtgacccctgatatacgacaacaaggaaaggttaaacataaattatctgctattttgtttctcaccgtatgtgcagtaattgcaggtgccgatgagtggcaggaaattgaagattttggacatgaaagacttgaatggctaaagaaatatggtgattttgataatggcattccggtcgatgacaccattgcacgcgttgtgagtaacattgacagtttggcctttgaaaagatgtttattgaatggatgcaggagtgccatgaaatcactgatggtgaaattatagcaatagatggaaagaccataagaggctcctttgataagggaaaaagaaaaggagcaatccatatggtgagtgcattctcgaacgaaaatggtgttgtactggggcaggtgaaaacggaagccaaaagtaatgagattacagccattccagagttgcttaacctactgtatttaaagaaaaatttgataaccattgatgctatgggctgtcagaaagatatcgcttcgaagatcaaagataaaaaagcagattatcttctggcagtaaaaggcaatcaggggaaattacatcatgcattcgaggaaaaatttcctgtaaatgtgttttctaattataaaggcgattcgtttagtacgcaggagataagtcatggaagaaaagaaacacgtttgcatattgtcagtaacgtaacgcctgaacttttgtgattttgaattcgaatggaagggattaaaaaagctttgtgtagcattgtcattcaggcagaagaaagaagataaatcagcagaaggtgtaagcatccgatattatatttcatcaaaggatatggatgctaaagaatttgcacatgctatcagagcgcactggctgatcgagcacagtcttcattgggtgttagatgtaaaaatgaatgaagatgccagccggataagaagaggaaacgcagcctaaataatatctggaataaagaagatggcactgaatttattaagagattgcaaagacattaagggtgaagaggaaaagaaagaaggctgcgttaaacacagggaaagatcatcagaagttcactttttgtactaaacaattcgcattttatgtttaaaaattgagatattccttattacctaaagctgttttttattgcttacacatgatcaaatactccttacataattaaggagaacaaaatggaacttaaaaaattgatgggacatatttctattatccccgattacagacaagcctggaaaatggaacataagttatcggatattctactgttgactatttgtgccgttatttctggtgcagaaggctgggaagatatagaggattttggggaaacacatcccgattttttgaagcaatatggtgattttgaaaatggtattcctgttcacgacaccattgccagagttgtatcctgtatcagtcctgcaaaatttcacgagtgctttattaactggatgcgtgactgccattcttcagatgataaagacgtcattgcaattgatggaaaaacgctccggcattcttatgataagagtcgccgcaggggagcgattcatgtcattagtgcgttctcaacaatgcacagtctggtcatcggacagatcaagacggatgagaaatctaatgagattacagctatcccagaacttcttaacatgctggatattaaaggaaaaatcatcacaactgatgcgatgggttgccagaaagatattgcagagaagatacaaaaacagggaggtgattatttattcgcggtaaaaggaaaccaggggcggctaaataaagcctttgaggaaaaatttccgctgaaagaattaaataatccagcgcatgacagttacgcaatgagtgaaaagagtcacggcagagaagaaatccgtcttcatattgtttgcgatgtccctgatgaacttattgatttcacgtttgaatggaaagggctgaagaaattatgcgtggcagtctcctttcggtccataatagcagaacaaaagaaagagctcgaaatgacggtcagatattatatcagttctgctgatttaaccgcagagaagttcgccacagcaatccgaaaccactggcatgtggagaataagctgcactggcgtctggacgtggtaatgaatgaagacgactgcaaaataagaagaggaaatgcagcagaattattttcagggatacggcacattgctattaatattttgacgaatgataaggtattcaaggcagggttaagacgtaagatgcgaaaagcagccatggacagaaactacctggcgtcagtccttacggggagcgggctttcgtaatcttgccctgggcattattgtcgtataaacgctttaccggacacatgacattcacaatgtgtgttaattttactgacatctttcaaaaggagcgtaatcatgccgcacatcgacattaaatgttttccgcgtgaactggacgaacaacaaaaagcagcacttgctgcagatattaccgacgttattattcgtcatctgaacagtaaagacagttcgataagcattgctctacagcagattcaaccagaatcttggcaagctatctgggatgccgaaatcgcgccccaaatggaggctttgataaagaaacctggttatagcatgaatgcttaacccgccgtaacacgcttgccgctggtaacaaacgtcccagcacctaaatgatgcaacgtattgagcttatcatcatcaaactgccagcggccttcgacaaatacccgtgcgtctgccgctgctgatactacttcgccaaacagcgtgtcgtattcttcttgcgcagaagtcgcaggtagcaatcgacactccatccacgccagacatttttcctcgaccagaggcaaaccaaataccgggcctctcacaaccggaatgccatagcaattaaatttatcttcatcacgccccgacacacttcccaccgcccacgtccagttagttgctgcaacgcccgggataacgatgccaaatttaccgttatgttcaatcaactccctggtccatgtcgatttatctaccacaatcgccacgcgtggaggttcaaactccaccggcattgaccaggctgcagccataatgttacgccgctgggattgctcatcgaaactggtgatcaagaccgttgggccatgatttaacagacggctggcatggtgtaattctatggggatgaatcggctcatggtatcgcctcgcgaagaaggtttttttaagcgtagtccgtaacgcaataagtaacgaaattaacgggattggcgatttgcgaacgtgatgcatgtccgcgatcgcacaaaatagccggtgcggcgtctattccaggttataagttgagaaaaccactaagggaaacgcctgatgacgcccattctgaatcactattttgcccgtattaactggtcgggagctgctgcggtcaatattgatacgcttcgtgcattgcacctgaaacacaattgcaccattccgtttgaaaacctcgacgttttgctgccgagggaaatacagcttgataatcaatcgccggaagagaaactggtgatagcccgtcgtggcggttactgttttgagcagaatggcgtgtttgagcgggtgttacgcgagctggggtttaacgttcgcagcttgttagggcgcgtagtgttatcaaatccgccagcattaccgccgcgcacccatcgtttgctgttggtggaactggaagaggaaaaatggattgctgatgtcggtttcggtgggcagacgctaaccgcgccgattcgtttagtttccgatctcgtgcagaccacgccacacggagagtatcggttgttgcaggagggtgatgattgggtgttgcagtttaatcatcatcagcattggcagtcgatgtaccgttttgatctctgcgagcagcaacaaagcgattatgtgatgggcaatttctggtcggcgcactggccgcagtcgcattttcgccatcatttgctgatgtgccgccatttgccggacggcggcaagctgacactgaccaattttcattttacccattatgaaaatgggcacgcggtggagcagcgaaatctaccggatgtggcgtcattatatgctgtgatgcaagaacagtttggtctgggcgtggatgatgcgaaacatggctttaccgtggatgagttagcgctggtgatggcggcgtttgatacgcacccggaggcgggaaaataatttatgtcaggttgccggatgcggcgtaaacgccttatccggcatacattagcccggttgtagacctgacaggcgaagcgcatcagacaacggtttcagagttcaattgcccattcggcatgaaacaaaatcaccgctgtgcctgaaatggtgactttttccggttggttatcacgaattgtcaccgtcacttcaatcataccgtcacgccccaatgcgcgcccctgatggcctttaacacgcaacacgttgccatcgtggggcaatacgttgtgatgtaccaaccatgcacccatcgggccattggcattgccagtcaccggatcttccacaataccaatcgcaggcgagaacatgcgaccatcggtttcgtttttgcctgggcggatctggaacgggaagaaaccattgcagccaatctttttgctgatagcggtcagcgcattaaggtcaggcgaaagggcgtcgatatccacttccggtttcagtgggatcatcacttttgagtgtcctgttgttgccacctgaattggcaagcctggcagaatatcgtcctcagtgagatgaagcgcgttgataatcgccgcacgtgtttcaccttccagcggtggctcaaagcccggcgtaccttgttccagcgaaatacgataatcatcgttgtgcttttcgatagtcacgcgatgttttcctgccagcgatgtttgccagatcgtgcaatttcctaaacctaacaccttcgcacgtacatagtgcgcagctactgtcgcgtgaccgcaaatcggcacttcaaccgttggcgtaaagtagcggatgcgcacatcgctgtcgtcgctgtgcagcagaaaagcagtttccgaatggcctaactcgcgggcgataagctgcatttgcgcttcgctaagattatcggcggggaaaacaacaccggcagaattgccgcgaaacggttgtgaggtaaaagcatcgacgtggtacacctgcggtttcattaacgttctcctgtgactggagaactatcatagcctgcaagtggccggagagcgaagggctatccggccagggtgaaattatcgccgcgaacgcacaatttgatatcgacgagtaaagtactcaaacggcgcgctccacacatgcaccagtcgggtgaacgggaagagcaggaagatggtcattcccaacaccagatgcaggcggaagacgaacgctacgccgttgagcatctctgacgatccaccacggaaagtgacaatgctttgcgcccaacccaccagcttcatcatttcgctaccatcaggatactgtgctgaaaacggtatggtacttagccccaacagacactggatcagcaaaatgctcatgatgatgatatccggcgtagtggaagtggcacgcacgcgctgatttgtcagcctgcgccacagcagtcctgcgccgccaatcaacgtcaacacaccgcaaataccgccgagcaccatcgccatgagttgtttcgctgccactggcaaaaaccacgcgtacatccagtgcggcgttaacatgccgaacaagtgcccgaagaaaatccccaaaatgccgatatggaacagattcgaccatatcaccatcccgcgtttatcgagcatttgacttgaggaggcgcgccaggtgtactgcccgtagtcgtagcgcagccagctgccgaggaaaaacaccgtcgcacaaatgtacgggtagatatcgtaaaaaaagacgttcagatactgaatcatttcccacctcccgcactgatgtcgacatattgcggcgcgacatcctggctaaagcgtcgctgatattgattaagcggcgagctgtcacacgccgtggcgttatcttcaataaacttcacctgttcctcttcccacactgcatcaagcgcctggcgggtgtcatcgcgctcttcgctgtttacttgttttgtgacactgtcacttgaaagggagcttcccgccagttgcagcagagcatcaaacaacgcgtaccacggtgcctcgcgttgttttaagcgaccgccaagcagggcgaggatcggcgcaacattgagcaatccttctttcgcctgatcgtcaggcagtacgcttaaatactccagatacagcggtagataatcgggcagttcccgacaatccagctgcaggccgaccttttcatactccgccagcaggtccaccattgcctggccgcgatcgcgggactcggcatgaacatgttcgaacagcagcagcgacgtggtgcgcccgcggtcaaacacttcgcaccattcggcctgtttatccagcagcggcgcgttaagcaggttgtgggtgaaatccgtaagcatcggcgcgtcgcggcggatcaacgccagcgcgtcctccttgcattcccacaacagctcgtccggatactccatcaacaggccgatcactttgaggatctgcattattcgccctccgctttgtcgcgcacttcggtgatgttgatggcatcgatacggctactgttgaacaggttgaatttactgtccgaaccgtggcaaccgtcgccaaaggtaaaaccgcagccgttgcgttctgcgaaggcatcgcccgccatttcccgatggctggtcgggataacaaaacgatcttcatagttggcaatggcgagatagcgatacatctcttcgacctgggcgacgctcaggcctacttcgtcgatggcacgagtatcagtaacgccttccacggtttgtgaacgcatatagtggcgcatcgccatcatccgtttcagcgcccgcagtaccggaccggtatcgccggcactcaacatattggcgagatattgcaccggaatacgcaggctttcgatggcgggcagcacgccttcgcttttcggcaaaccgcccgcatctgcgtaggactgaatcggtgacagcggaggaacgtaccagaccatcggcagggtgcggtattcagggtgcaacggtagtgccagtttccagtccatcgccattttgtagactggcgaacgctgggcagcgtcaatcacattttgtggaataccttgtttcagggcttcctcgatcactgagggatcgtgtggatcgaggaacacttcgcactggcgttcatagaggtcaacttcgcgctcggtgctcgccgcttcctcgatgcggtcggcgtcgtaaagcagcacgcccagataccggatgcgacccacgcaggtttctgagcacacggtcggttgaccggactcaattcgtgggtaacagaagatgcatttttctgacttgccgcttttccagttgaagtagatttttttgtacggacaaccgcttatgcacaaacgccagccacggcatttatcctgatcaatcagcacaatgccgtcttcttcgcgtttgtagatagcgccgcttgggcaggtcgccacgcagctgggattgaggcagtgttcgcacaggcgcggcaggtacatcatgaaggtgttttcaaactgcccgtacatctccttttgcatggcctcgaagttgcggtcgcgggcacgtttttcgaactcaccgcccagcagttcttcccagtttggcccccagatcactttgtccatccgtttgccgtcaatcagtgaacgcgggcgagcagtaggaatatgtttgccttccggtgcgctatgcaaatgttcgtagtcgaaggtgaaaggttcgtagtaatcatcaatctgcggcaccaccgggttggcgaagattttggttattacgcccatcttgttgcccagacgcgggcgtatcttgccattcacatcacgcacccagccgccttgccactcttcctgatcttcccagtttttcggataaccaatgcccggtttggtttcgacgttgttaaaccatgcgtactccatgccttcgcgcccggtccagacgtttttacaggtcaccgaacaggtatggcagccgatacatttgtcgaggttaagcaccatgccgacttgtgaacggattttcattttttcgcctcctgtacctgatcgcgaccttcatcatccagccagttaacgttcttcatcttgcggatcatgatgaactcatcgcggttcgatccgacggtgccgtagtagttaaagccccaggccagctgcgcgtaaccgccaatcatatgcgttggtttcgggcaaacgcgggtaaccgagttatgaatgccgccgcgcatgccagttacttccgaaccaggaatattcataatgcgttcctgggcgtgatacatcatggtcatgcccggcggtacacgttggctgaccaccgcgcgggcagtcagcgcgccgttggcgttgaatacttccacccagtcgttatcgacaatggtcagttctcgggcatctgtttcgctgatccagacaatcggtccaccgcgagagagcgtcagcattagcaggttttcactgtaggttgagtgaatgccccatttctggtgcggcgtcaggaagttaagtgctttttccgggaagccgtttggcggtatctggcgcatctcactgacgctacgggtgtcgataggcgggcgataagccaccaggctttcaccaaaagcacgcatccacggatgatcctgatagagctgctggcgtcccgacagcgtgcgccacggaattaactcatgaacgttggtgtatcccgcgttataggagacgtgatcgctttccagaccggaccaggtggggctggagataattttacgcggctgcgcctgaatatcgcgaaagcgaatcttctcgtcctctttgtgcagcgccagatgggtatgttcgcgcccggtgatctcgcccagcgcctgccacgctttgactgcaacatgaccgttggtttccggtgccagtgccagaatcacttctgaagcgtcaatggcggtgtcaatcagcggacgcccctgtgccgggccatcacgcttggtgtaattgagtttgccgaggaaatcgatttcatcctgggtattccacgaaatccctttaccgccattgccaagtttgtccatcaatggcccgagcgaggtaaagcgttcatacgtagcagggtagtcgcgctccaccgccacaatattcggcgcggttttgcctggaatcagatcgcattcgcctttgcgccagtcgagcacttcacacggctgtgagagctctgccggagagtcatgcagtaggggttgtaataccacgtcggtttctttgccaagatgacccacgcacacttgcgaaaatgctttggcgatacctttgtagatttcccagtcgctgcgtgattcccacgccggatcgaccgccgcagaaagcggatgaataaacggatgcatatccgaggtgttcatatcgtctttttcgtaccaggtggcggtgggcagaacgatatcggagaacaggcaggtactggacatgcggaagtcgagcgtcaccagcaggtcgagcttgccttcaatcgctgcagtttgccactcgacttcttccggtttgatcccgtcgctggcaccgagttcctcgccctgaatcccgctttcggtccccagcagatacttctgcatatactcgtggcctttgccggaggagccaagcaggttagagcgccagacaaacaaattacgcggatgattgctgctgctatctggttgttcgcaggccatacgtaaatcgcccgatttcagcgcctgggcggtaaattctgtgggggataatccggccttgtcggcttcagctttaatcccgagcgggttacgccccagctgcggcgcagaaggtagccagcccatacgttcggcgcgaacgttgaaatcaatcagatgaccgctgtacttactggcatcggcgagcggtgaaagtaactcctgagcagagactttttcatagcgccattggctggaatgattgtagaaaaacgaggtgctgttcatttggcgcggtggtcggttccagtcgagcgcaaaggccagtggcaaccagccggtttgtgggcgcagtttttcctggccgacatagtgtgcccagccgccaccgctttgcccgacacaaccgcagaagatcagcatattgatcatcccgcggtagttcatgtccatgtgataccagtggttaacacctgcgccgaggataatcatcgagcgcccatgcgttttatgggcggtatcggcaaattcacgggcgatggtttcaatatactggcgcggcacgccggtaatttgctcaccccaggctggggtgtacggtttgatttcagcgtaatctttcgcactgttttcatcttccagcccgcgatcgaggccgtaattcgccagtaccaaatcataaacgctgaccaccggacaggtgttgccatcgactaacgtcaggtttttaacgggcaattggcgcaccagcaccggattgtgttttacgctgcgaaaatgcggattttcaatgccgccaaagtaggggaaggccacgcctgcaacagcgtcatgttgaccgagcagggttaacgacaattcggtttccgtaccggcggcaatggattccagattccatttgcctttttctccccagcggaaaccaatcgaaccgttcggcactaccaattcacctgcggtattaactgctacggttttccactgcggattgttgctttcgcccagtccatccaccaggtcagatgcgcggatcatgcgcccgggaacgtagctaccatcgtcgcgaggctccagcattaccagcatcggcatgtcgctgtagcggcggcagtagttgataaagtagtcgctgggattatcgagatgaaactcttttaaaatcacatggcccattgccatcgccagggcgctatcagtgccttgtttcggtgccagccactggtcgcacaatttggccacttcagagtagtcaggggtaatggcgatggttttagtgcctttgtagcgtacttcggtaaagaagtgggcgtccggcgtacgtgtctgcggtacgttagacccccaggcgatgatgtagctggagttataccagtcggcagattccggtacgtcggtttgctcgccccaggtcatcggcgaggcgggcggcaggtcgcaataccagtcgtagaaacttaaacaggtgccgccaagcagcgacagataacgcgttccggcggcgtaagaaaccatcgacatcgccgggatcggcgagaaaccggcaacgcgatccgggccgtaggttttgatggtccagacgttagcggcggcaatcagctggtttagttcctgccagttggagcggataaacccgccgcgcccacgcacttgtttgtagctcaggcacttttgcggatcgttcataatcgatgcccacgccagtaccggatcgctgtgttgcttgagggcttcgcgccacagttcaatcagtcgtttacgaatgagcgggtatttcaggcggttagcgctgtaaagataccaggagtaacttgcgccacgcgggcagccgcgaggttcatgattgggcaggtcagggcgagtgcgcgggtagtcggtctgttggatttcccaggtcaccagaccatttttaacgtagattttccagctacaggagcctgtacagttaacaccgtgggtggaacgcacgattttgtcgaactgccaacgctggcgatagctgtcctcccagtcgcggttgctatgcatcacctgtccgtgaccatcggcaaaggtttcgcccttttgtttgaagtagcgaaagcgatccaaaagtttactcatgacatgactcctgctccaggaatgaattgggatctgatgccttgtcggatgcgacacggttgtacatcaggcatcgatctcttatttttggctgaacttccgccgaccataaaccagccaggtcagcagcacacaaacgatgtagaagattaaaaacactttcatcgcgccgaccggagagccggtcatattgagcgacatgccaaacgcctgcggaataaaaaagccgcccactgcgccaatggctgagataaagcccagagccgccgccgtttcggtgacggcttctttatgagcttgctcatcactaccgcctttcatctttacccgataaatggttatctggcgaaagatgacggcgatcatctggaaagtagaaccacttcccagacccgcagtcagaaacagccccataaatacggcgtaaaaggcgatgaaattaccggagcctgtgcccggtaaggtaaggaacagcagggcactgaaaatcgccataaaaataaagttgatcaacgtcacccgcacgccgccgaacttatcggaaatagcaccaccaaccgaccgcgcgatggcaccgataaatgggccaaagaacgccaggcgcagaatattcacatccgggaactgggtttttgccagcatggcaaaacccgcagaaaaaccgataaacgaaccgaaggtggcaaggtaaagcaggctcagcagccagagatgcaggcgttgtaagacagggagctggtcggcaattgaggcgcgtgaactggcgatatcattcatccctgaccatgcggcgatcgtggcaatcgccagtagcggtacccaaatccatgcggcattcgccagcgacatcaccgaaccgtcggcctgcggtacgccattgacgccgagaaaggcaaatacaggtacaaaaatgaccagcggtgcaaccagctgcattacacttacacctaagtttcctaatccgccattaatcccaagagcgctcccttgtttggcttttggaaagaagaaactgatattgcccatgctcgaagcaaagtttgcacctgcaaaaccgcatagcaaagcgataacgataaatatcccaaaaggagtattcggattttgcacggcaattccgagccagacgcaaggaataatcaggattgcagtactaaaaaccgtccatcggcgtccaccgaatataggcaccataaaggagtagggaacacgcaataatgcgccagaaacggagggtaatgcggttaataaaaagagttgatcggtagtaaaattaaaaccgattttattgagattaacggtaactgcgctaaatagcatccagacacagaaggcaagaagtagacaactgactgatatccagagatttcttcgagcaatatgttttcctttattttcccagaaggccggattttctggtttccagtcgcgcaaaagataacgactatttttctcattttgcagtgccatattgttcctcacatgcacacattggtaatgaaaaaaagacaaaacacgaggtaaggcgcaatagccagttattagaattaaggatgaattgggtgaagtgctgattgaaagaatagataagaaagcgtaaccgcgggggcagaatggggattaagtagccagatatgtgttactaaatgtaactaacaagctaaccttcaaacggggttaatctttgaacgtatgtcatgtttcaacccttcagatcgtgaatctaaagggttacatattaactatattatcaacaagaccagacacttatagaattagtgatgatttattcactaaaaaggccatgaactggaggaaaacgatctgtccagaaggtctatcggttcctctcttattgcctgattgtaataatcgttattacagtaagtattgtttatttcatctaaggtcatgtttttaacttttatattcatctggtttacaacttcctctgtcttgtaagtgtgtatattatatggggtatatgcttttttaataggatagtgaaacaattcgttatccacatctattccgtcagagtgaacttcaaatgcaccaggcgaaagaattgccaggccagtattaagcttaagtgctggggaaaacaaattaaataacatgagctgcatagtagggcaattgttcttcccagaaacatttaaaaaatttaagttttgctctgttttattatggggaataaagttccaatatcggatgtattattagtatcaatgtgggttattttattattgtccagtcttaaacttttgatagatggaagataagtcaggaaatcaagatttatatatttcaactggttgttagcagcgtttaatgtctgaacattgcagaagttgctatagaatattttaatttcagaaagcaaattgttgttaataagtaacgtattcaagttgggaaataagtcattgtgtaaacttgttagtttattatgggatagatccagcagtaagagttcatttttattacctgcaacaatatcagttaattgattatggctgagattcaggtattgcagccattcgcaagattctaattgcacaaactctagttgattatgtgccgcactaaaataagtaactgatgaaagcctatctatatcaatatttctgagagcattattattcatagatatatgtgtaatacttacatttctgccttgaggaaaatttattgactcaagagcattactattcagacttagctttacgagtctatcgtagttggttgcatcaaaatgtgtgaattggttattatcaagattgatagatgtgaagttttgcagccctggtggttgagtggttaaattaagtcctgataaatcaatggtcacttcattagtgtcatcaattatatttcttactgcagtccagtactgcatttgtgcaagtggatcattgttgatgccgttaactaatacatgccaaagatgttttgatgatattagttgatcaatgtcattggttggcagtaaattgttattgcttaagtttaaatattccagttttgtagtgtttttggcgtttaaatgtgcaatatggttgtcgtttaaagtgattgttttcatcctgggatgattgtgtaatataaggtcagtgatcatattgtgatgggcacttaactcaatcagagattcttgccgcgcgagccgttggcttcatcgttatagcctttaaaatcatattcccagtgaccaaaaccaatcatttgatcattgatttgcgtttctcctttaaagccgagacgggcataagttttatcaccatcgtcacgcttatcatcagtaaaataacgtagagcggtaaccttgccataaaggtcgagtttattaccatccttgttatagacttcggcagcgtgtgctacgttcgcagctaacaaaccagttacaaccaccgcaactatttttaatttcatttaacagaatccttttaattatcgttaaacgtattttctaaacgaattttaaacggcgtcatttataaatgacatactgtttttaaaatagaatggtgattaaaaacaatgagaaaaatagatgaaataatattatttatcgatatgtgatcgaagtcgaaatgagatataaggtgaattactggtatttgaaatttatttttttaatattgtcggaatttatctgattaactaccgggccgtagacccggcagttattttaaccacgacgtgtcgccagccagcagagcagggaaccgccgcagaccatcagcgcgccttgccagaacgagaacgacagcggggcgctgagcagcacggctgcaagcgctgaggaaagtacaggcgtaaaatacgaacctaccgccataatggtgacattgccatgcaatataccgacattccatgcagcataagcaaatcctaaggtaaatgccgcagagatgagtttaatcatgacgggcgtgctaaatatcatttctggttgtggcgtaagaaaatagtaaacccacagacttgctcccgttagcaggacaaaaacggtaattccattaaatccgcgtgcgtatttattcgttactgtgcaataggctgcccagataaacgcaccaatgaacgccaggaaataactcaatgggctggtggtgatattattgatgatttcatcataatgtaacccattgtcaccgcctaacacccaacagacgccgacgagggctaataataatccaggtacaatcaaccagttggttttctgaccattaaacagaatggcaaagagaattgtcaggctgggccacagatagttcaccatacccacttcaatcgcctgatgatgggtcgccgcataccctaaggaaagcgccagacagatttcatagctgacgaataacagactcccggcgagtaaatagcctttcgggatttgccgaatacgcggaaatccaaccgtgaagattaacagcagcccgcttaatgaatagatagcagctgcgccgccgaccgggccgagcccctcactgacaccgcgaatcaatcctaccatcgtgctccacaggacgatcgctatcagccctatgagcgttgctttttgtcgtgtcatgctcgctgttttgtctctcttgccgttaaaaattaagctgaattttatagcatttttttaactggcctgtcaggcagtggtgcgtttttctaccgctattgaggtaggtcaatttgcgaaggcggattattttgtggcaaacagatgttctttttgatttcgcgcaaaaagattcagaattttactgttagtttcctcgcgcagtaatacccctgaaaaaagaggaaagcaatggacgtcagtcgcagacaattttttaaaatctgcgcgggcggtatggctggaacaacagtagcggcattgggctttgccccgaagcaagcactggctcaggcgcgaaactacaaattattacgcgctaaagagatccgtaacacctgcacatactgttccgtaggttgcgggctattgatgtatagcctgggtgatggcgcaaaaaacgccagagaagcgatttatcacattgaaggtgacccggatcatccggtaagccgtggtgcgctgtgcccgaaaggggccggtttgctggattacgtcaacagtgaaaaccgtctgcgctacccggaatatcgtgcgccaggttctgacaaatggcagcgcattagctgggaagaagcattctcccgtattgcgaagctgatgaaagctgaccgtgacgctaactttattgaaaagaacgagcagggcgtaacggtaaaccgttggctttctaccggtatgctgtgtgcctccggtgccagcaacgaaaccgggatgctgacccagaaatttgcccgctccctcgggatgctggcggtagacaaccaggcgcgcgtctgacacggaccaacggtagcaagtcttgctccaacatttggtcgcggtgcgatgaccaaccactgggtggatatcaaaaacgctaacgtcgtgatggtgatgggcggtaacgctgctgaagcgcatcccgtcggtttccgctgggcgatggaagcgaaaaacaacaacgacgcaaccttgatcgttgtcgatccccgttttacgcgtaccgcttctgtggcggatatttacgcgcctattcgttccggtacggacattacgttcctgtctggcgttttgcgctacctgatcgaaaacaacaaaatcaacgccgaatacgttaagcattacaccaacgccagcctgctggtgcgtgatgattttgctttcgaagacggtctgttcagcggctacgacgctgaaaaacgtcaatacgataaatcgtcctggaactatcagctcgatgaaaacggctatgcgaaacgcgatgaaacactgactcatccgcgctgtgtgtggaacctgctgaaagagcacgtttcccgctacacgccggacgtcgttgaaaacatctgcggtacgccaaaagccgacttcctgaaagtgtgtgaagtgctggcctccaccagcgcaccggatcgcacaaccaccttcctgtacgcgctgggctggacgcagcacactgtgggtgcgcagaacatccgtactatggcgatgatccagttgctgctcggtaacatgggtatggccggtggcggcgtgaacgcattgcgtggtcactccaacattcagggcttgactgacttaggcctgctctctaccagcctgccaggttatctgacgctgccgtcagaaaaacaggttgatttgcagtcgtatctggaagcgaacacgccgaaagcgacgctggctgatcaggtgaactactggagcaactatccgaagttcttcgttagcctgatgaaatctttctatggcgatgccgcgcagaaagagaacaactggggctatgactggctgccgaagtgggaccagacctacgacgtcatcaagtatttcaacatgatggatgaaggcaaagtcaccggttatttctgccagggctttaacccggttgcgtccttcccggacaaaaacaaagtggtgagctgcctgagcaagctgaagtacatggtggttatcgatccgctggtgactgaaacctctaccttctggcagaaccacggtgagtcgaacgatgtcgatccggcgtctattcagactgaagtattccgtctgccttcgacctgctttgctgaagaagatggttctatcgctaactccggtcgctggttgcagtggcactggaaaggtcaggacgcgccgggcgaagcgcgtaacgacggtgaaattctggcgggtatctaccatcatctgcgcgagctgtaccagtccgaaggtggtaaaggcgtagaaccgctgatgaagatgagctggaactacaagcagccgcacgaaccgcaatctgacgaagtggctaaagagaacaacggctacgcgctggaagatctctatgacgctaatggcgtgcttattgcgaagaaaggtcagttgctgagtagctttgcgcatctgcgtgatgacggtacaaccgcatcttcttgctggatctacaccggtagctggacagagcagggcaaccagatggctaaccgcgataactccgacccgtccggtctggggaatacgctgggatgggcctgggcgtggccgctcaaccgtcgcgtgctgtacaaccgtgcttcggcggatatcaacggtaaaccgtgggatccgaaacggatgctgatccagtggaacggcagcaagtggacgggtaacgatattcctgacttcggcaatgccgcaccgggtacgccaaccgggccgtttatcatgcagccggaagggatgggacgcctgtttgccatcaacaaaatggcggaaggtccgttcccggaacactacgagccgattgaaacgccgctgggcactaacccgctgcatccgaacgtggtgtctaacccggttgttcgtctgtatgaacaagacgcgctgcggatgggtaaaaaagagcagttcccgtatgtgggtacgacctatcgtctgaccgagcacttccacacctggaccaagcacgcattgctcaacgcaattgctcagccggaacagtttgtggaaatcagcgaaacgctggcggcggcgaaaggcattaataatggcgatcgtgtcactgtctccagcaagcgtggctttatccgcgcggtggctgtggtaacgcgtcgtctgaaaccgctgaatgtaaatggtcagcaggttgaaacggtgggtattccaatccactggggctttgagggtgtcgcgcgtaaaggttatatcgctaacactctgacgccgaatgtcggtgatgcaaactcgcaaacgccggaatataaagcgttcttagtcaacatcgagaaggcgtaagggggcgaacagatggctatggaaacgcaggacattatcaaaaggtccgcaactaactccatcacgccgccttctcaggtgcgtgattacaaagcagaagtcgcaaaacttatcgacgtttccacctgtatcggctgtaaagcctgtcaggtggcgtgttcggagtggaacgacatccgtgatgaagtggggcactgcgtcggggtttacgataaccccgccgatctgagcgccaagtcctggacggtgatgcgctttagcgaaaccgaacagaacggcaagctggagtggctgatccgtaaagacggctgtatgcactgtgaagatcccggctgcctgaaggcgtgcccgtctgctggtgcaatcattcagtacgctaacgggattgtcgatttccagtcggaaaactgcatcggctgtggttactgcattgccgggtgtccgtttaatattccgcgcctcaacaaagaggataaccgggtatataaatgcacgctctgcgtcgatcgcgtcagcgtcggccaggaaccggcttgtgtgaaaacctgtccgaccggggctatccacttcggcaccaagaaggagatgctggagctggcggaacagcgcgtggcgaaactgaaagcgcgtggttacgaacatgctggcgtctacaacccggaaggggtcggtggtacgcacgttatgtacgtgctgcatcacgccgatcagccggagctgtatcacggtctgccgaaagatccgaagatcgacacctcggtaagcctgtggaaaggcgcgttgaaaccgctggcagcggctggctttattgccacttttgccgggttgattttccactacatcggtattggcccgaataaggaagtggacgatgacgaggaggatcatcatgagtaagtcgaaaatgattgtgcgcaccaaatttattgatcgcgcctgtcactggaccgtggtgatttgcttcttcctggtggcgctgtccgggatttcgttcttcttcccgacgctgcaatggctgacgcaaaccttcggtacgccgcagatgggacgcattttgcacccgttcttcggcattgcgattttcgtcgcactgatgtttatgtttgtgcgttttgtgcatcacaacatcccggataagaaagatattccgtggctgttgaacattgtcgaagtattgaaaggcaatgagcataaagtggcggatgtcggtaagtacaacgccgggcaaaagatgatgttctggtcgatcatgagcatgattttcgtgctgctggtgaccggggtgattatctggcgtccgtactttgcgcagtacttcccgatgcaggttgttcgctacagcctgctgatccacgcggctgcgggtatcatcctgatccacgccatcctgatccatatgtatatggcattttgggtgaaaggatcgattaaagggatgatcgaagggaaggtaagtcgtcgctgggcgaagaaacaccatccgcgctggtatcgtgaaatcgagaaggcagaagcgaaaaaagagagtgaagaagggatataatctcttttgaactttaagctgaaaatggcgctgtaaaaggcgccattttcatattgtagacaacgtaggctttgttcatgccggatgcggcgtgaacgccttatccggcatgaaaacccttcaaatccaatagattgcagtgaacgtgtaggcctgataagcgtagcgcatcaggcaatgttgcgtttgtcatcagtttcaaatggcgctgtaaaaggcgtcattttcatattgtagacaacgtaggctttgttcatgccggatgcggcgtgaacgccttatccggcatgaaaacccttcaaatccaatagattgcagtgaacgtgtaggcctgataagcgtagcgcatcaggcaatgttgcgtttgtcatcagttctaaatggcgctttataaagtgccatttttttattgcgtaaccagacggcgtaatcgcgacacatccactgttttttctgcctctgccagactccaggcgttttgcagattcagccacatttgcggcgaactgccgatcaccacggaaagtttaatcgccatttctggcgtcaaagctgcttttcctgtcagcaatcggcttgccgttgagggagcaatttccattgctctggcaaactcgcgcaggctgacattaagttcgtccagtgattcctgaataatgtcccccgggcggggatgattggccattttcattagtgtctttactctcagtagcgttccttcactgggaacactatcattattgttccttcctacgcaacaataatccatttagccatttcatgttggagagtgtgcgatgctgcgacccgaacatggcagtcgcagcaaaggcctcttagtgacggaaatcaatcaccatgcggccacggattttgccttcttccatctcagtaaagatggtgttgatgtccgctaacggacgcagggcgactttcggcaccactttaccttcggcggcaaactggaaggcttcagttaaatcctggcgcgtgccgaccagcgaaccgaccacttcaataccatccagcacaagacgtgggatatccaggctcatagactccggcggtagaccgacagccacaacacgaccgcctgcacggacagcatcaactgccgagttaaacgcagctttagctaccgctgttaccaccgcagcgtgagcgccaccagttttctcctgcacaattttggcggcgtcttcggtgtgtgagttaatcgctaaatctgcgcccatttcggttgccagttttaactgctcatcattgacatcaatggcgatcactttggcgttaaagacattcttcgcgtattgcagggcgaggttacccagaccgccaagaccgtagatagcaatccactgccctggacgaatttttgacagcttaacggctttgtaggtggtgactcccgcacaggtaatgctgctggccgccgccgagtccagaccatctggcacttttaccgcgtaatcggcgaccacgatgcactcttccgccatcccgccatcaacgctgtatccggcatttttaactgaacggcagagcgtttcgttaccactgttacagtattcgcaatgaccgcatccttcgtagaaccacgccacgctggcacgatcgcctggttttaatgaggtgacacctggacccacttctgccaccacaccgatgccttcatggcccagaattacgccggttttgtcaccaaaatcgccattcttaacatgaagatcggtatgacatacaccacaacactccattttcagcagggcttcgccatgtttcagtgagcgcagtgttttatacgtaacgtcaacatgatgatccttcgtaacaactgcagccttcatagttcctccttttcggatgatgttctgcatagcaggtgaggcaaatgagatttattcgccactacccagtatggatgagatctgaaaaagggagagggaaatagcccggtagccttcactaccgggcgcaggcttagatggaggtacggcggtagtcgcggtattcggcttgccagaaattatcgtcaatggcctgttgcagggcttcggcagaggttttcaccgccacgccttgctgctgcgccattttgccaaccgcaaacgcaattgcgcgggagactttctgaatatctttcagttccggcagtaccataccttcgccgttcagcaccaatggtgaatactgcgccagcgtttcacttgccgacatcagcatctcatcggtgatacgtgacgcgccggaagcaataacacccaggccgatgcccgggaaaataaaggcgttgttacactgggcgatagggtagattttatctttccataccactggattaaacgggctgcccgtggcgaccagcgcgttaccttcggtccaggcgataatgtcctgcggtgtggcttccacgcgtgacgtcgggttagacagcggcatcacgatcggacgcggacagtgtttatgcatctcacggatgatctcttccgtaaacagcccggtctgtcctgagacgccaatcagaatatctggttttacattgcgcaccacatccagcagtgacagcacatcgctgtcggtatcccagtcactgaggttttcgcgcttctgcaccagtttggtctggaaaggcagcaggttcggcatcttgtcagtcagcaagccaaagcgatcgaccataaagactttctgccgcgccgcttcctcgcttaatccttcgcgctgggtctgggagatgatcatttcggcaatgccgcatcccgctgaacctgcgccaaggaagacgatttttttctcgcttaactgaccacctgccgcgcggcttgctgcgatcagtgtgccgactgttaccgccgcagtgccctgaatgtcatcgttaaaagaacaaatttcattgcgatagcggttaagtaacggcatcgcatttttttgagcaaagtcttcaaactgcaacagcacgtctggccagcgttgtttcacagcctggataaattcatcaacgaattcatagtattcgtcgtcagtgatacgcggattacgccagcccatatacagcggatcgttaagcagctgttggttgttcgttccgacatccagcaccaccggaagggtatacgccgggctgatgccgccacaggcggtatagagcgacagtttaccgatcggaatgcccatcccgccgatgccctggtcaccaagccccagaatgcgttcaccgtcagtcaccacaatcactttaatattatggttcggcacgttttgcagaatatcgtccatattgtgccggttctggtaagagataaacacgccgcgtgaacggcggtagatctcagaaaaacgctcacaggctgcgccgacggttggggtataaataacaggcatcatctcatcaagatgattgtttaccagacggtagaagagggtttcgttagtgtcctggatgttacgcaggtagatgtgtttgtcgatttcggttttgaatccctgatactggatccatgctcgttccgcttgttcttcgatggtttcgaccacttccggcagtaaccccagcaggttgaagttacggcgttcttccatgctgaaggcactgcctttattcaacaacggaaattccagcagtacagggccagcgtaagggatataaagcgaacgctgtttttttgtttttggttccatgtcactcactcttttttgaatatccatccctggggggcttttatcgtctttgctttaccgccagggcgtcggcctcaagtataaagcagataaaaacaaaaacaccattgcgcaggcaatggtgtttaatcgtcattgaggactgatggttatgaattacttttcagcggggcgttttctgccggttgggttatttactacgctggatttgtcaccttcggtaactattttgcgctggttagaaattttatggtccagtccaagaatatgacgtgcctgacggttcgatttcattttaactcctcaatcctgtagctagttttaaggacaacatcgccgtagcgaagaaacacgtgctaaacccctaaattaggttgccgatcaagcatagcaccttaaagcgtagggtgctggccactgaccacataattgatcgtttgctggtagatatcactgaggatgtcgttatcagaagcttcaacccatttggtcagctccatgagaatgtcatcttcagtgacaacaccatgctgtgcccgaaggccttgctcaatggcattaaccagagcgggttctgctgttgaattttctgcctgataataagtaaacatagtgattctccgtgtctgtgtatttatggtgtctgctacggatcgcagatttataaagcacattcagcatggcaaatatttgccgcttcgttgttaagattagtcctggttgatgatttttatattttaacaccatgatattcatagggattgtgattggtatgatccgattaatattgatacaatatcttttgggttatatattcccggtaatctattgtgggaatttaatttaagtgcagaagtaatattttcgccggattttattcggaatatcctgcttatcctcgtgctgtttctcacgtagtctataatttcctttttaagcccacaggagagcaacaatgacaatccataagaaaggtcaggcacactgggaaggcgatatcaaacgcgggaagggaacagtatccaccgagagtggcgtgctgaaccaacagccgtatggatttaacacgcgttttgaaggcgaaaaaggaaccaaccctgaagaactgattggcgcagcgcatgccgcatgtttctcaatggcgctttcattaatgctgggggaagcgggattcacgccaacatcgattgataccaccgccgatgtgtcgctggataaagtggatgccggttttgcgattacgaaaatcgcactgaagagtgaagttgcggtgccgggtattgatgcctctacctttgacggcataatccagaaagcaaaagcaggatgcccggtctctcaggtactgaaagcggaaattacgctggattaccagttgaaatcgtaaagcattgccggatgacgcgtcaggcgcgtgaatgcctgatgcgttgttagcatctctacagcgcccgccagcaccggagctcacgtccgtcctcccttattgctaatgattgccggacttcacatccgtgggttgccagcgggcaacgttcgtagaaaaaacagccttgcggcaacgtgcggtttcccggcagatccgttttacgtaatgcccattcttcctccagcggtttatcaatggcggggagggaatccagcaataatcgggtgtatggatgtgcaggtgccgtcagcacctgctgcgcgtcgcccagttctacaatctgcccgagatacatcaccgccacccgatcgctcatatgacgtatcaccgagacattgtgtgaaatcagcacataggtcagcccgtgattttcctgtagcgttaccagtaaattgaggatctgcgcctgaacggagatatccagcgcagaggttggctcatcaagcacaatcacgtcaggctgcgaagagagtgctctggcaatggcgatacgttgccgctgcccgccggagaacgcatgaggcaggcggtcgagatactccggacgaatacccacctgcacagccaactcctctgccaacgctcgccgctgttgttcactactacgcttagctatccagagcggttctgtgatgatgcgccacaccggtaagcgcggattaagcgaagagagcgggtcctgaaacaccatctgcataatgcgttgtgagccagaacggatgtactgcccgtggctcggttgcagcatacccattaaaagctgtgcgagggtgcttttgccgcagcctgactcgccgacgatccctaaggtttcaccacggcggatctgtaaatcaataccattaatggcatgaacatgttccgtagttttaccaagccagtttttacgggccgggaaattgatatggacgtcgcgtaacgttaataacgtgtcagacacttataacctcctgctgcggataccaacaggcacagcgctggttgttgtcaccacacgctgtcagcgccgggacgttttcacactgtgcacctgccgcatagcaacgatcgcgaaaagcgcagccgtcaggcaaatgggtgaggtttggtaccgtccctggaatggcgggtaatagctggcgtggtactccatgttctggtgcgcattgcagcaaaccaatggtatacggatgccggggatgatggataacgtctgccgtcacgccgctttcaattacgcttccggcatacatcacgtaaacgctatcgcacagttgcgacaccacggccatatcatggctgatgaacagaaccgcagttccactggcgcgggctttatgtttaagcaaacgcagtacctgcaactgcaccgtgacgtccagcgccgtagtcggttcgtcggcaataatcaattgcggctcgcaggagaatgccagcgcaatcattacccgctggcgcataccacctgaaagctcaaacggatagcgcgacataacttccacggcatccgggatttgcatctcttccagcaggtcaatcgctttagctctggcttcccgacgacttattggttgatgatggcggatcacgtccatcatctgaagacctattcgacgtgtcggattgagggcggtcatcggttcctgaaagatcatcgccactcgtgcgccgcgccactgacgaagctgtttttcccgcgcgttaagaacatcttctcccagcagggaaatctgcccccgatgtacgcaataactgcccgtcggtagcagacgcataatcagcattgcggtgactgatttacctgagccggattctcccaccagaccgacaatttcaccgcggttaatctgcaaggacacattgttgagcgcgtgaacatcaccgttaaaaccggggaaactcaaatgcagttgttgaatgtccagaacgggttgggtcatgactgctttcctcctgctttcgggtcaagcagatcgcgaataccatcaccaaagagattaaacccgacggcggtaagcaaaatcgctgcccccggaaatgcgcaataccaccactgatcgagtacatagttgcgaccatttgctaccatcgcgccccattcagcactcggttgttgagcacccaggccaataaatcccaacgtggcggccattaaaatcgcgctaccgatatccagcgatgcctgcacgatcagcggcggtagggagttacgtaaaatatgccagttgatcagatgccaacgagacgcgccaaaggttttcgccgcctgaacataggtatactggcgtacaactaatgcttgcccccgcgccaggcgcacataaaagggaattcgcacaatagcaatagccagcatggcgttaaacaaactcggcccgagagcggcagccagtgccattgtcagtaccaacgaaggaatcgacagcataatgtccatgatgcgcatgatgatggcgtctgcgcgtccaccaagcacaccggatagacatccgagtagcgaaccaatcatacccgcaatggcaaccacgactaatccggcgagaattgattgctgactgccgaccagtacgcggctaaacagatcgcgtcccacttcatcggtgccaaaccagtgcgccgcagaaggcggcaaaaggcgggcggttaaatcaatggcgttgggatcatgcgtcgccagccacggtgaaaaaatcatcatcaatagcattaatacaatgatgactgcgctggtcacggtgagcggactgcctttcagcatccataccagttttgcaccgttaaatcgcgtttgtttttgtgggcgtacggcggacgtttcctcgcttagcatcattcaccacctccacgtccgatacgcggatcaatccacaaatagagcaaatccaccaccaggttgaccagcacataagcaaatgaaaccacgacggcaaagcccatcactgccgggaagtcgagcgcctgtattgatgttactacccatgcacccattccgggccaggcaaaaacggtttcggtgagcactgcgccatacaacaaatcgcccagcgccaaacccaatacggtaatcgatgggatcaacgcattgggtagcgcataacataaaacgatataccagccgggcaagccgctggcccgggcggtacgaatgtagtcttcactcaattgttccagcatcgctgagcggatctggcgagcgacaattcccaggtgaacgaacgccagcgttaatgccggtaagatgagatgttgcaacgcattgaagaagacttcaccgttgccttcaagcagcgcatcgagcagataaaagccggtaacgtgcgttggtggatccagccagtcatcaagccttccgccgccgggaagaatttgcagatgaccataaaacagcacaatgacgcccagcccaagccagaacgcaggtgtggagattccggtaatggccattattcgcaccagatgatccagccagcgatttcgccagactgcagagagtatgcccagcgggatgccaatcaggagtgccagcagcagggcaccaaaagccagctccagcgtcgccgggaaaaatatacgcaactcttccagcaccggacgcccggtacgaatggatgttcccaggtcaccatgaaacaggtcgctgacgtagcggtaaaactgtacatacagtggctggtccagtcccagttgctggcgaatattttccacgatagcatcgctggcgcggtcacccgccagtaaccgcgccggatcaccagggatcagatgcgagataataaacgtaatcacgcagacgcccgccaccacgagcaccagcccccagcagcgttggcgtaaaatactccagaaggtcacgttatttactcatggtattgatattgaagacctgttccagcatgggattgaacacaaagcctttcacctctttgttcatcgccagttggtagtttttctggaacaggtacacataagcagcgtcatcaatgacgattttctgtgcctgctggtagtcccgggtacgctgcgtctggtcggtggtcgcaagcgcattgcgcagtaacttatcgacctcactgttttcatagaacgagcggttacccggcagaccttttttgtctgactcaaaccagtaattcataaacatatacgggtcggcaaaatccggactccagttgccaatcgcaatgtcgtaatcacctttacccactctgtcgcgcatggtggcgttcgccagcttttccagcttcacaatgatgcccagcttgttgagactggattgtgtcgccagagcaataggctcccagttcggatcgttatcggagtagagaaacgtcaggctggtgggtttgctcgtcactttatcccattcggctttggctttcgtttcgtcatggttgtattgcattgccgtcgcatcgtagccccacatgccttccggaatcgggccgcgcatctgttttccgttaccactcagaatgccgttaaccatgccctgataatcggtagaccaggaaatggcccgacgcagatccgcctgattaagaggcgctttgctgttattcagatacagataggtaacgcgcagtgacggatactctgccacattgactttattttcctgcttcagggcgttgagttgatccaccggcagcgcatcggcaatgtcaatgtcgccacgggagagctgcaggcgacgggaggcactttcaccaataatttttaccgatacccgtttgaagttcggtttattgcctgggtaatgcggatttggcaccagaactaattgctgacctttttgccagcttttcagcataaatggtccggaaccggcggtattttgcgcgaggaagccgcgagcatcatccgctgcatgttcctttaagaccgccggattgataatggatgcaccgtcattcgccagcgtgtagaggaacggtgcgaatggttggctaagggtaaacttcaccgtatgttcgtcgggagcatcaatctttaaatctttgggaaatgcttctgctggcccctggccgatttttagtagccgctcaaaagaaagttttactgcttcggcagtgacaggtgtgccatcggcaaatttagcattatctttcagggtgaacgtccactctttttgatcgtcagacgctttccagctacttgccagatcgccttcaacgtcggttgagcctttatcaccgtccgttttgtactgaaccagccgctgataagacgggtaggtcactgtccagtcgttattatctattgttaccgccgggtcgagggtttgtggatcggcggccttaccaatcaccagcatatcttttggtacggcggcgtgcgcaaccgggaaatttgtggcaaggacgagcgcgagcaatgtgggacgaaacgatatcgatctcttcatgacagtttcctgattaactgacgtgctgtgtgccaggggatataaaacaagagaattgatcagcgagcagagggtaactcgctgcctggggtaattcgaagtgccaccattcgctggagataccgacaaaaccgccaccagtcattatcgcattcagcaacagccgattgcgctgagcggcgggcgggacggaagggtgataggcatgggagcgctcgtgcatttcatcgaaccctgcgcccatatcgaggatgttcccgtgctcatcacgaagcgtcaggtcgatcgccgtgccacggctgtgattagaaccgaccgtcacatcaacaacatattgcgggtctgggcaggcttgccacaacatcgcctgtgcttgttgtgggcgatacgcatcgtaaatcaccagttgtaaccctgacagctgggcgatgctgatacttttcgccagcgcggtaatcgcatccttgtgtaacagacaacgcgcttgctgataaatagctttacctgtgatgttatcagcgcaggcgtatttcaattcgatctccagatcagggaagattacggctaaatcaaccagttcggtggtatccgacataaacggttcctgtataagacaaaaattgctgcgctttccgcttatgcagatctcatgccatgccgggataagcgccagaatgctggcttaaagttatattttttaacttttgatcaacatttgtgcagcgtagtgcagttttggtgcaagaggggaagttaaggaaggaatctcccggaatcgtagctgaaatcacagtatttaagtgacagtgtcacgttaaatgaaaacccgcgagtgcgggcgagaggaatttgtcagattttcagcggtaacacgctgctcatccagcctggaatttcttcggcgggtagggggcgggaaaagaaatatccctgaataacgcgacagtggatcttgcgtagcatctcaaattgctctttggtttcgacgccttccgccacgacggttaaattgaggctttgcccaatgctggtaatggcttcaagtaaggcaaggatgcgtttttcggtcagacaacgatcgacaaaacttttgtcaattttgatttccgttaccggaagactgactaagcgggataatccggaaaagcccgtaccaaaatcatctaccgataagcccacgcccatatcacgcaggatctgaatgcgcttaaagatttcggtatcgtgttccatcatcatgctttccgtgatttctaccgtcagctggtggccgtcaataccccaggcgtgcattgcatcagacacctgattaggcagttgattactgcgaaagtgcagcgccgacaagttcacggataacgccgggatatgaatattctggctacgccattctgctaactgacggcaagcttccgcgatgacccagcgcccaatattttcgatttcaccaatctcttctgcgagaggaataaaccgtgaagggggcacatgaccatgcaggggatcgtgccagcgagcaagggcttcgatgccgtacagttcacccgtttctgcgaagatttgcggctggtaaaccagtttcagttggttattgctaatcgcttctttcagcgctgcgcctaaaaccaaacgctcttttaccatttcgttcatcgccgggctgaagaactgccagccgttaccgccattcttgcgaatataatccattgcattgtgagcagtggagagcaagtaatcgcggtttttacccaggtcgtagctgatgccaatactcaaggtaagcgggaagggtttatcgtcaatcattatcggcttgctgaccacattccgtagctcatcggcgatttgggtaatgttactgacgtcgttttcgaggctcacgaggacaaactgcgtaccttcgatacgacagagatactgatccggtttgagtttttcacgaaagcgattgaccacttccagcaatgcctgatcggcccacgcatagccaaggctatcaatcacatcctgaatatggtcaacaccgatgagatacaccacgggagagacggctttgtcgaccaggtcatcgaggtaattgtgcaggttattgcgatttggcagaccggtcatcggatcaaattggatgagttgttcaatatgctgacggcttttttcctgttccagcgccagcgcggccatatgctggctgatatctgccacgcgttcgataaaggcgctggtttctgctcctgacgaggttttaatttgcaggatccccgcaggcgcgccatcacgctgacgaatggtcgctgaccagctttgcgcattttgaatttctgcaccgtgggaagatgacgcccagtgtatcggcatcccgttgcgcagtgcgaacagcgaaacatgcgattcgttgagtacagattcgatgttacgacaaatgatttcccccatttcatgaaatggcgggctgctgcacatggcggcgagaatattgccttcaagctggcgaatctgccgttcttcggtgatatccgagaaagtcattaccaggttctgcagatgcgcgagcacgtcataaaccgggctgatagaggctttaatccagattttttcaccggtgcgcgtcaacagcagaaattcgtcctgatcgcgggcggttttccatagcaactgttgtaaacgaatgcggttatcggcagggaattcaggaatgttcaggagtgtatcgggctgcataccgctggcttcgctaatgcagtaaccaaacatttcggtaaatgcgcgattgcactgcacaatatggcgttccggatcgaggacaatcaccggtcggtcgagatggtcaacggcaataatcaattgtcgggtctgttctttttgcgccatttctacgctggcatcccgtaccagcgccaggtaataaactttcccctcggcgctcactttcgatagcgcaaaacgggtccagattttactgccgtcttttttctccagctgcagctcccgactcatcccctcaacacgcgctttaccgccttcacggttgtgacgaatgtattcaggatgcgcaggacgcaaatcccgcggaatcagcatatcaatgttattgccaatgacttcttcacgtttgtatccccagagcttctctgcggcggggttgaaaaacatcacttcatcattttcgttaattaacaccgcacccatcatattttgctcaagggcggggaaaaaaatgccatcggcggcattatccgcatcggttagcttcatgattacctctgcatcctggcgcatctaaagactggctttccagagttcaacacggtttctacctcgtcttttggcgatatacagagcttcatcggctatttgaatgaggcgctcatagtcaggatgaccattaaacatggcggcaccgatggaaagtgagagggcaatatcttcgccgtttgcggctttcagtttggttttctccacccgactgcgaatacgttctgcggtacgtaacgtttcgttttcagaagcttcagtcaaaacaatgataaattcatcgcccccgtagcggaaaacataatcactactgcggacgttgtcataaaaggcctgagagactttacgcagaatttcatcaccagtgttatggccccacgtatcgttgatctctttgaatttatcaacgtcaataatcagcactgacagcggtgtaccggtccggttggcatgggcaatttcgcgtttgaagatagtcggtaggaaacggcggttaagtaatttcgtcagtacatccataccgacttcgtggcgcgatacttcttcaaacaattcacgcagcaaggtaataatttgcgatacggtatttcttatctgtaataaaaatttcacccgcagacttctgttattcaaatttctggtgttacgcatggtttgattgaaaataccgtcgaaatcctgaatcagacgggagatatggcctacttcggcaataccactaaaataatgtcgacctttatggttaaaccacaggccaaaatcagcctggcttaaaggcaaactactgcctaaatcagaatccagcaggattttatagataatatctatttcccatgaaagtattgaggctatttgccgttctttttcttcttcggcgttttccagtaacgagaagatacgatagttttcatcttcctttgaggcactactgtcactaaaggtaaacgcgcgagtcatcacttccatcgcgatatcaatactgttaatcgagaaatggtagacctgaagtttttctgcggcggaataatccgaagagaagatcaccggatagaggatttttttcagcacccgaaaccccatctcgacaatttctaccggaattcctatgcgggcatgcacttccgcgacggtatgctggatttgtattagcctttcgacatcgtcaacctgggcagaaagcacgttaataatccagcgttccatcgcactcttcaactgccgctcaacttgttcattactcaagaattcttcggcatgcgggtcgatgcggacaattcgataaaactcgatactcagataatgagcatgcgcaacggcaatttccgcggctttagcacgaatgggcggatctgcctgttcgacaagtccggtccactcatctttcattcttttaaaatacatctccataattcacacccttataaggctgggaaatcagacggaatcaaaatgaaacgcaacgtgcgagatcgactaactgcaccatattctcctgaaatatgaagatatactgaaaagaaataagcgatttaggacagtttcaatctacgctactgttcttcagaagagtatagcccatcgtaattatttttcggtgacagcgaatatcgtatggtttttcatattcatacatttttattagggatttatggctgtttaactaagtgtggttaatttgacttaagtaagcatgattattagtgggatagtttaagagggtaacaagccggtgggtaaagcaccggcttgttacaaagtaagaatgggagtttaactgccccagcgactttgcagatagctgaccgcttgttgagtctgcggtttattcagatagtcctcacggaacaagatggtgccgctaatttcgggcacagcatcgttaagatcgagctgctttttcagttccggtacgccgccgttaatcatccagtctggctctatctttgaaggttcacccactttatagaaggcgataccgatatacaggcgggtcctggtcggtttaacgacatccgcccaccattttgccaacacgtcataacgcgcggcactccgtgagaacggccagtaaatttggggagcaatgtaatccagcaatccttgttccacccatcgacgggtgtcagcgtaggattcgtcataggctgccgcgcctcgggtatcggaaccgagcggatcgtgtgatcggttacgccacacgcctgccgggctaacaccaaattcgactcccggcttaatgcttttaatggtgtgcgatacctttgcaattaactgctgagtattgttgcgccgccagtctgcttttgacgcaaatgcgcctccgtatttacggtacgtttcgttatcatttagccgtgaacccggtgactccgtatagaaatagtcgtcaaactgcacgccatctacgggatagcgggaaaccacttctgcgactattgatgtgatccagtcctgaacctcagggatgcccgggtcgaggacaaagcgatcgccagacgttctgatccagtcgcggtgttgcacatagacgctcgccggttgttgagacagagtgctattcagttccctgatagtaccgggcttcgtattaaccgatacgcgataggggttaaaccaggcgtgtactttcatcccacgcttgtgggcttcgtcgagcataaattgcagcggatcgtaacccggattttcaccaatcttaccggtcataagatcggaccacggcaaaattttcgatggccacagggcggtaccgtccggcttgacctggaaaaagaccgtgtttatgccgagacgttgcagatgatccagtttgtcgatcatcgcctgttgttgtacacgggcccggctggtggggttactaatgttaaccgaggaaaccggtggccagtcgagccgagaaaccgtggccagccagatgccacgcatcggttgtgacgattgttgcgtcgtggctggtggctttgaacctgctggtggtgtcaccatggactctggaggcgtgcttttacaactacacagtaaaagtgccagtgcaactagtatcgctggtcttctaatcgttaatttcttgtttcgggagcagatatccatatgtgctggtttccggtaaacagatgtgcgctcattctcgtacttatccccgttaagtcaatacgacagcaagcacgaaaaagggagcgatgaattatcgctcccttgtcttataaccattcagacatggttagtgtttcttgtcattcatcacaatatagtgtggtgaacgtgcacgcgggtgcaggaagaagtgaccttttggtgcgttctgactgttgattggctccagagtgacgccggtatttgctttgcctttacgatcatgaacagcatagagaataaagggcagggcaagtaccaccaggaaactaacaaccagtaattcaacatacatatcggtagaatcaccctggatgttatccggcggcaggaaggaaacaataaacgccataattgaagtcagcagaccgacaattgccacgaccagtttcacccctttaccaccagggatattaaatgtgcgttttaagtcaggatgtttaagaaccaacacaatgtagccaataaacagcatgaaataagcacacagataaatcaccaccgtcagcgccagtgcgatcaggaaggacatgttgttaccgccaccggtattggtgaggatgatcaacgcgatagacgtaatcaccagctgcgaaatgaccagcgttaccggtacgccatttttgttcattttagcgaatgccgctggcagcaggtttttctgcgctgttacatacatcccgcgagaaggaccaacaatccaggaggcgatttccgccagaacacccagcaacagcagtgcggagatcacgcgaaccgtccactcaatttctggtgccacatgggacatcagaacggtaaaggtttgcattacccctgcggagaggttgatttcattacccggaatgaccatcgcaatagacaaaccaccaacagagcttaagcagattgccgccaccatcagcagtaacatagccaacggatagtcgcgccctgggttgctcatttcattgacgtgggttgcggatgcttctacgcccatataactcaaaatgaaggcaacaaatactaccagggtgcccactttagagaagtcagggaagaaggtcttcgaatccatttcgatagcaacgggggcaccggagtgcagataaatagccgctaatgcgatcaaaataaatgcaggtaacaggataccggcgaagaagccaactttagcaattcgcgccgtgtatttcgtgccaccaaactgcgttaatgccagcgcccaaagaatgatgagtgctgcaatagttttggtaatggggtcttcattcagcgctggccatttcaggatgtaggagagtgcccctaacacgaaatagagcatcggaataaaaccaatggcgatttgcagatagccaaatgagatcgctgcaaatccccatctcggccccagagtatttgatacccaggcgaagacaccaccttcttcccagccgtcgacggtggccatttccgcagcacaaagtcccacgggaataaaccataaaatcccgcctaatagcaggaagaagactaatgaaaagcccgatgttgcgaaggtagggtattcataaacagccattaccatcgatgccgttatggcaaagaatccaagtaatgtgagctgcttagctttacctgtctgtactgatgtagccatattatccccctaaaacggtattcctgtcggaaccgcacctgttttgttctgaagcgtattcagaacaatattttccgttgctaatgccagtgaacagactttggaaattgtcccgaaacgggttcgtttcgggacaccgttaccgttaaacgttatcaggtatgtttaaagctgttctgttgggcaataccctgcagtttcgggtgatcgctgagatatttcagggaggctttgtagtcttccagcaacagttcagcaaagtccatttcgaagccgcgacgacacataatgcgcatcaccacgatgtcggtggcttcaccgccgagagtgaaggccggaacctgccagccgcgcagacgcagacgttcagagaggtcatacagggtgtatcccggatcttcaccatctttcagtttgaagcaaaccgccgggatgccttcgtccgggcgacccgtacagatgaactcatacggccccagtttggcgatttcatccgccagataagcggcaacctggtaagaggcgttctgtactttggtatagccttcacgaccgaggcgcaggaattcatagtactgtgcaattacctgacccgccgggcgggagaagttgatggcaaaagtaccaatttgaccacccaggtagtcaacgttgaacaccagttcctgcggcagcgcttcttcgtcacgccagataacccagccgcagcccagcggagccagaccgaatttatggcctgaagcactgatcgatttcacacgcggcaggcggaagtcccagacgatatccggggcgacgaacggtgccaggaagccaccgctggcagcgtcgatgtgcatgtcgatgtcgataccggtatcggcctggaatttatccagcgcatcgtgcagcggttgtgggaactcatagttaccagtgtaggtcacgccgaaagtcggcaccacgccgatggtgttttcgtcacaggcttcaatcatgcgtttcgggtccataaacaactgaccggggcgcatagggatctcacgcagctccacatcccagtagcgggcgaatttatgccagcagatttgtaccggaccgcacaccaggtttggtttatccgttggtttgcctgcagcttccatacgcttgcgccaacgccatttcatcgccatcccgccgagcatacaggcctcggaagaaccaatggtgttggtgccaacggcctgaccatttttcggcgcaggcgcatgccacagatcggcaaccatatttacgcaacgcaggtcgatggctgcggattgcggatattcttctttgtcgatccagtttttgttaatggataaatccatcaatttgtggacattttcgtcgtcccaggtctggcagaaagtggccaggttctgacgagcgttgccatcaagatataattcgtcattgataatctggaatgcgacatcgtcgcgcatttcgtgcagcggaaaacgttttgattctgcgatagtggaaatagacttcgcaccaaaacgtgaatcgagtagttccgaccttaaatccgttacttgcttcttatccattttaaactccttaaaatgattggatcgcattaaaaaagtaggatttatcgataaagtaagcaagtgcaaaggactcgtgtttaaataacaaaatcctaatgttatttatcgtgagatattacgcgaataatattttttcattgaaaaacaatacaatatgaaattcttgggtggtggtaaggtgttttatgctgttatttttatgcgcattctgtgtctcctgaattatcacgtaaaaatcagaccttaaaatatcactattagtacttgattattattttgaacgcatttataaaattattacataaaaatagcgaatattgctaaaatccccgccaacgatgtgttgacggggctgttattattttggcaataatactccggtataagtatttaccggatgagaaagatattgtttaacggcagtgttaacattctctaccgtcatttgtttcaacaattgctcctgctcagtccatgctgcaggatcgtcatattgaataagactatttacaatagtgttcgctaattgttgaacgctacgctgttggatatcgaggctgcgctgaacgttttgctggtattcattcagttcttgctcactgatccctttagccagacgcttaaccatcacttcattcgctaacgttaacagttcatcatgtcgttctggttgacaagtaaaagccagcaaatgactgatatctttggcctgaggatcaaccgagaggcgagaagaaacgctgtatgctccagatgcctgttcacgaatattaacacgtagatcttttgccagtgcgacgttaaaagcatcgagcgccatacgcgtcggcagattaacaggtgtccgggaatcataacgcttccactgtgaaacctgtgccacaggttcattttgttcttttacagtaaccgatgcgttgtccgtcgcgcgagttaatggtttacctgcggctaatggcgaatcagagtgtttgattgatcctaagtaacgcgtaattaacgccacgagtttgtcttctgcgacattaccgacaatgacaaacgtgatatccgctggagatgaaaacaattggcgatcggcagccagcgcatctgcggcagtaaactgtgcaatctgattttcttgcagtaatttcgtgcggtcatcagcatagcgcgtctcatacatctgctgggcgaatttctccgctggacgctggtcgagcgttttcaacgcctgaatttgagcattttgtagcgatgcccaaatattatcgttaatcgtgctgtgggtgattcgctggttaatcaactgaaaaccaggttcagggttattagtccgcgcgctaacggagagcaacgtattcatgccactgactttactgctcatggttaccgaattttccgcactccagcgtttcaggctggaagaggagagttcgccaacgccgcttccgctaactgctttatttgccagcgcgataagtgatttttgctgcgcagggaaacttaaatcgcctttattcgatacggcaataatttgtagcttttgctcttcacccgcggattttgccagaataaccctggcaccattggaaagtgttaatgatgtcagattctccgccagcgtttctttgctgctaatttccgcctgtgggtctgcgtctactgttaacgataaatttctgcctgggaagacgtaagccgccagctttttgttggcgtactccttttccagcgccaggatagccgcaggagacaatgcttttttggcggcaacctcattgtttaccatttgctcccaaaatgcgtcctggttctttcttaactgctgccatttttccgccagactttgcacggtaatttgctgccacagacgtttcgaaagttgatatgtctcttccggcgacaagaacggcgtattatttaatgagctggatgccaggcgactggtcagcatacgtaaatcacgttcagcttgctgatcaaccgcatttttcagccaggtgaggcgggtagatttgacatcatcgagttcttcagcagaaaaaccatgctgatcaatggttgccaactctgccattaatgcattcgcagcatcctgcatattatcgtctcgtgcatttacacggaaaaacagcgactgataatcgggtgcaattttaacgctgcgcgcagtgccgccagaaatagtcttcaactcgcccgactgtatgcgttcctgcagacgttgattgaacagctgaactaacatgctccattcagcttgttcgataaagctttgctcatcgttcacttgtaccattggcaggcgataatagagtgcgatgccgttcacccggttttctttatcattaatgatattaaagcgcaggtggttttcggcttttgtcggccagacgcgattttcagctgctttgttagccggaagcttacttaaattatcctttatcagcgccagcgcttctttactgtcgatatcgccgaccacgataaaggtcatattatttggttgataccagcgttgataaaattggcgcaattgtgccggtgtgaccgtggcgacagtatccatcaggccgataggttcacggtctaaattacgggtatttgccagcaggaaagggcggcgcgcctgagaggtgcgccatttcgcatcctgatgggcacgccattcctcagtaattacgccacgttcagcgtctacttcgagtttttcaaaggttgcggcattactccattcactgaagattgccatcacttgttgcagattttgtttctgcgtagtcggcaaactcacctgatacaccgtttcgtcatagctggtataggcattaacatcgcgaccaaaacgcaggcccattgactcaaatgtttcgatgactttattacccggccatgtttttgtgccgttaaacatcatatgttctacaaaatgagccacgccgagctcattgtcttcttcctgcaatgaaccggtatgaatttgcagccataaatttacctgatcctttggatgagcatgcggataaatcatatatcgcaagccattgtccagttgcccggtaattaacttttcatcctgcggtaaggcggcggcaatcagccgcccggggagcaacagagttgccactaacgtcagtaagaaacagaggtttctcataattatctccatgcgaaaaccgggcgaatttacccggttaagtaaaatccgaactattaaaatttcatgctgacatcaagccagaaagtacggccactggcgtaggtcgccacaccggtgttcgttgtatcaacagcggttttgctatccagtacattgagaatatcggcactgatcgtcaggttttgttgttgcagaaattgtggcgtccaggacaagcgggtgtcccaggtcaggctgctatccagtttttcgtcaacatactgcttgtaatctgaatattcgctgatgtattgcgcatttgtcttaccaaggataatgcgagctttacgcgcttcttgccaggccagcgtattcgcccacactaacccgctcggttgatgcgtgaaatccatgtttaaggagatctttaatgggttattaaaatctgccactggaacgctatcgtaagagaccagattaccgttataaaccacctggttatcaccggtattgctctcctcataaccattgtttaacgacaagttgcccttgctcttgatatagctaaagacaatttgtgggttaatatctacctggcggatatgcaggggttcggccagttcaaaactgaggctgaacgaatgcgttttggttttgccatcgttgttatattcagtaatggtggttttagtcgcgctgtcggtacgactgcttttgctgatttgatcatgcgcttcacggtaaacatagtttgcacgcgcaataacgttcttaccgattttctgctgcaatcccattgccagttcatcgttataaggcgttttcaaatcctgataacgcgtcagagttttattacctgataccgattccgtccagctattgcggatatcacgtaatcccatatcaagaatattcccgccatagtaacggttataacctgctgtaatcattgaggtttgattagcaaaaatatcccattccgtcataaagcgcggggagatattgtggtttgacagatagttgtcatagtcataccgcacgccgggcattaatgacacattacgccagctaatgcgatccgccatatacagcgtgtagttgtcaattcccaggcggcctttacctttatggtaaatggtatggttagttttctttccggcagcattaatcacataggattcagactggttatggcgttcagtccacgcatcggaatagatgtattccgcgccgaagtagggttgatgcgaaacattacccacggcgaatttttgccagtccaggcgtgttttgaaggtgtaattatctacagcctgggaaatgtgtcctaatccgccacgggtgcaacgccctgtaatatcaccatatgtacatgaaagttcggtgtaccagatgtcatgatcgtgacgggtataatcactaatatgatcccaaccaacggtggtacgcagtttggcccatgcgagctgcgtatccatatcccatgccagaccataggatttattacccatttcgcgatcagactgcgggaaggtgctggtattataatcacggctggagccggtatattttaaggttaaatcgtgggtaaagcggtcgctggcaaaccaggtaaatttgcttaatgcagtatcgataacgtttttatactgtgcccgaccggcgacaatgccgtcattcgaaacataatccgcgcgggtgatatcagactggcggcgcgataaaccggcggtaacgccgaagttatcagcgagttcctgattaaacgacaaggtataaaagttctttttaaaatctggggagtaataagtacttcctgaagagccttgattaaatgcgctcttgttattctcatcgatatgcgatgttaaccagtccgaacgcgtagtgcgataacccaatttcaccttgctatcatcagcgttgaagcgtttgatctttgcatcaattaccccgccattgaagcgaccaaattcaaccggcacaaaactgtcataaagcgtcacattgtccagtaagctgacatcaagataatacccctgtgacatcccgctaatattggttgcactactggcatcggactcattcgctgggttcaggttattagttgcactaataccgtcaatcaaataggcattctggtagggcgacgcaccgtgaatagagattttctcagggcgaatatctccctggttcaacgaggtactttgcgttgaatccatgcgtaccgcagggttggttctcagcagatcgctgatattgccattcccggtcggtaaacgctcgatgctttcactggtgtaatgcgtgttgccgtttacgggtacagggacaggagcatagaccgtcatctcttcaaaaaaatgcatgtacatgtttttgtcatcgacggcctgcgccacatcagcgccacataaaatgacgccaggaataagaactcgcttcatttatttatatctccgtacagcagggcttttattgtttttataaaaccgcgctaatgtcacaaatatcatcggccaggttccagacaccgggttgatgtgtaaccataatgacgccgcttgtgggtagtttttcacgcactaaacgcagtaagcggatagcctcttgttcctcaagatgagaggtagtttcgtcaagaaatatccatttcggacgtcgtaaaattaatcgtgccagggcgatacgttgtttttcgccgctggaaagaatatctccccagcgatcgtggtcatgaatacgcgcagccaatttcccaagaccaacctgatgcagtacttcgctcaacgatttatcgtctacgggcaggggaagtgctttacaaataatctctttcagtaagccggttttgattaacggtgtttgtgacacataccaactgtcagcaggagaagaaatatcacctttaaaccacggccagcagtgggataatgttttaagcagtgtggtttttcccgcgccagagtagcctttcagtaatagccatttgcctggcgaaacatgaaagttcaggttctctaatatgatcttattatcaggcgtacgaatactcgcatcagccacttgtaccgcatgttggcaatttttaggcttattcgtagggcgctgttcagtgagttgatggaactcatacaagcgatcgataaccgcagccagttcagcaagttcgtcatatttataaataaaccagcttaaattgttcgataccagcataaatgcctggcgcgatttcatcagtccgcccagattgatctgcccgctaataaactgcggcaataacagaaagtagggaagaacgctaagcgagcgcgaataaatattctgccagtaatcaagccaccgctgacgattcattaaacgatgccagttctctttaatggtatgaaaattgtcgctcaactcctggcgttgtagagactcagcattgcttagcgcaatcagttctgcctgcttattatgctgcacaagatttgttcgaaatgtcgcttcgctacgttgtttttccacattaagcggacgaatacgtttacccaccttatgggtaaataaagttccaccgatcacaatgagcacgacggtatagaccatatacccctggatattccattctgttccaccaacagtgaatgagagcgtacccgcgctttcccaaagaataacggtaaaggtgatcagcatgctaagtgactggatgaagccaaatgaaagactgagcgttttgctgatcagtaagagaatgtcttcagcgatacgttggtcagggttatctgtatttttatgctcgccgtagatctgcgtgaagtagtagtttttatctgcaaaccaccgattaaggtagtaatctgttaaccattcgcgccagcgaatagtcagtagtttaattaaccatgttttgtttacggatattaatacaaagatccccagcagggcagggaaccaaaggacaagctgccaaagcttatcggtttctttctggcttagcgcattgaaaaaatcattattccagtcgtttaaccagacctgaattttaaccacgccaaggatcatggcgaggataataatgattaacaacactgaagttttattattcttacgcagccaaaagggcttcaacagacagagatactttgctatcaacatacgaagcgtaatgggaatggttatcattagcgaaaattgattgtgccatccaatgattatctatggcaatgatttactgatgaaatttatttaagtatcatttaacaatatgaaatataaaggaatatttcattttcagtggttatggttatgctattgataatcaaggatattgctaatgccctgatgcataccacgtaagccaggattttcgcaagggaagatgatgatgacgaaacacccgacaggaatttatgtcgggtgccttgttaaggtcataagaaggaggctaagaatggagttaaaagagagcgttattaattattctccatttgttttgcaacatccataatgtggtaaagcggtactctgttcttagctaactctaccatggcgttcatataaggtaccatggttgaaaaaaggattttataaccttcgcaaaaataagaaacagtctcattgtttactttagtaatacgatgcttaggacaaccgccattgcagataggtttatatgcacattgctgacatttcgctggaatccgttttttttgcgctgtcagttgtacactgttcatcgttttgagttcagatttattaatgtttccaattttgtactgtggatagacaaaatggtcgcattcgtaaatgtctccattactttcaacaaccagattatccttgcaggactcctggaaaatacaactggtatgcccattccccaaaaaacggctgacaaagctttcaaactgacggatgaaaatttcacccacatcgtttttaacccattgcataaaaatggttgacataaacttgccataagccgtgggaggcacagaaaaatcaatgatacggaatgtgttctcactatgaccactgaaatcaatattcggcgtcccggtttctagcaattcgataaattgcatatgtttactgccgatagattttaaaaaatgataaacctcaagagggtaatggacattaacgttattaatgacggttaacgtattaaactctacttgatatgatttcagacgctcgatggctgctatcacttttgcaaaagtaccgttacctgaattactgcgtctgtaacggtcatgtaactcctgggggccatcgatcgagataccaaccagaaattcatgttctttgagaaaggcacaccattcattattcaataaaatgccattcgtttgtaatgcattaaaaatacgtttttggcctgcatagcgttgttgatagtgaataactttacggaaaaaatccaggccagccagagtgggttcaccgccttgccaggtaaaatagacctgattgccagacgctgcgatatattgtttgatgaactctttcagagtgctgtcatccatccatttttcatgagtaaactgcgactctttttcaaggtaaaaacagtaatcacatttgagattacattgaaaactggagggcttggctgtaacgtgcatcgctatctcgctcaataaggcggcggaaaaatccgccgcatgaaggtttagttatttcgcttcgcttagtgctttcttgatattgttaaacttctcctgatttacctcgctaagcggtggctggctgctgtcgataaactctcttaccacgccttgcatctctttaacgacctgcggattggcggcggcaaggttatctttttgctgtagatccgtcagtttgtagagacctaactgattgttttctactgtatagacaagcgaataatcgttatttctcaccgtataagagaattggcttaagtcctcagtgttggggttatgcgggtaatcgtctgactgatggcgaacaaatttgtggtaattatcccagaatggaatattttcctcgtcaaaccagtgagaataagaggttatccaggtcagatttttatgtggctcgccttgtttcttatcttgcaaccagggcagcaaggaaacgccatccagcttaaggtcttttggaatgctgatatcggctgcatcaagagctgtcgggtagaaatccattgcggaaatcagcttgtcataattaccgggttgaagttttcctttccaccacataaacattggggtgtgagtaccgccaggataggtctgactcttatagcctttttgcgccccgttcagcggcagaggaccatcgataaccgcaccattatcggaggtaaagagaataattgtattgtcatactgtccgtttttcttcagttgttcgagaatgcgttttacaccctgatcaacagaataaacggaagcgtagtagttatctgctgtttgactaccggtattaaattgcttctgatattgatccggtgcaggattatcatttggcaggtgcggagcattataagccaggtaaagcataaaaggctggtcaagtgttttggcacgatcaacaacgccaattgcctcatcggttaactgatcgctgatataaccttttgcggggacacgttcacgatttttgaacagtgaaggggagttgtaatatgccgttcctgcagcgtggaatcccataaagtaatcaaagccacggttttgaggttgccattcttccgcagaaaatgtggtgaagttgtcatgatagtcacgcgtttgtttatcttccggtaccggcacattactgatttttgacaagtgccatttacctactgctgcagtgtaataaccatgattctggaataattcaggcaagaaagtttctgttagcggaataccatcctgagcatcggtattggaatagacaccaaagcgggcgggagctcgaccggtcattattgcggcgcgggaggggccggaaacaccgtgtgccacatagccgttagtaaaacgtacgccttcatccattaatgaaaggagcgtcggcgttgatttttgtgcagcttcaatggctttatctatccctattttgtaggtatcgacaacttcacgattttccattgtttttgggtcaaaagatcccttatcaaaaggaagttgtccataaccaagatcatccatggtcagtacgataatatttggctttcctttggtactgtattctgtcggcgtaaagtctgagaaagcaacgtttgttttggttgctttcagctttacatcatctgccgcatgagcagcaaatgcagccataccagatgccagtatcaaagatatcgaggtacttacgacacttttctttaatgcagacttcataaatgttcctcttcttattgtacttaattccaaagtaattttacgaagagaaataagtggatgtaagtgaagttagtcacataaagagatagcagatttagctaaaaaaagggaaaaaacagtccataaagcgttgacattactttctgttctattaagtaatttctcgccgataaacaactaatttattgatatttaataaattattgcattttactgacaaaatgcagaattgagatcataaataatcatgcaacaggttatgcaagtgcataaatatgtgatggatgtcacttatttatttcaataaatatatcgcctaaaaacaacgcggggcagggaatggctgccccatttaattcttacgcagcgtgtgtggttgactactcgttagcaaataatcaaatagctaaagcattcatcgtgttgcccgtattcatacccgtgtgactttgacaacggtactccttagaaactctcttcggactgttgccgaaatgtttgcggaacgcataaataaaataagatgtactggcataaccacattgttcggcaattttattgactgaaccttctacgcgtatcaaattttttgcgtgctgcattcttgcatctaaaagaatctgtgagaatgtcgtttgctcttgcttaagttttttcttcaacaggctttcactgatgtacaggcagtcacaaatatctttcagcttccatgggtgcgccggcttcatgttgacaatatttctcactttcccagaaacggatagcacaccgttagttaatagtgtaatgaaacctttgcatgcggcaaaaatagacaggcaagaaaaaagcaaaagttctgaaaaattatgatgattgcgttcttccgagttgagataagcaatcatttcattaagcaatccagtcggtacatttgaagcacgtaaaaacttcgcaggaacaggcaccgtcactgtctggatgttagtgcattgtagatattttttaatggtattttcagtaaatccgatctctttaaaatgccgctcataaggttcaaaatgcgtacgaacagcgttatctaccatcaggatctcgccgtcagagaaggcgtaatctttatctaaaatgttagcgttgaaggcatgatgaataaatataacagaacaaacgagcgacattttatctccttaaaacaataaagtttttatcgatacttttttaacatttcatatttataatttgctgtttgttttcagccttgcaaactattgataatgaaatgtgtaagatctcttgcaatgcgacccatttctgaaatactcagctgatcaattgccgaaaaaatggctatcaacgtaagtgtcagtaataagacaaccacaattgcagacatgatttctttatagttgtctctttgcgtgattttgtttttcactgtggtcgcatgcatttcaaatatgtttatttagcggataacgttaaaaatcgttaatcagtatgcttaatataacaggctggagaaaagaggaaataggactggtgcttcagtactgagcggagtttcttacagctgtaggcagaagtttatatcttatagtatgtagtttaatttaatccatgtgagcaaattgcgaaataatagtcaatgaggaattcttctgctgtgcggatgacagcagaagaaatgagaagaggcattaatttgatggttctaattcaaccggaatacttttatagccaggaatgccacttaatggatcgtggttatcaagtgttagcatgtgattcgattctggaaaataggtcaccagtgagcggtcagccatagggtaaatgaccacttttaatctatccatgcggcgtgagctgcgcttaccgtctggcgtaagcgcaataagattaactctttcgccgttttttacacggcaaattttagcttgtttagcactcataaagaccacatctcgttgaccgaatacccctcgatagcgatcatccataccataaatcgtcgtgttgtactgatcgtggctgcgtactgtcgccatgaccagcttactgttaaacgctgaagagggatcttctaacagccctttgctggtaatgaaattagccttacctgacggcgtcatccagcgcctttcagcagctgcatttatcaggtgaaaaccaccgggatgacggatgcgctggttatagtcggcgaactctggcagcacagcttcaatgtcattgcgaatgcgatcataatcttccaccagatactcccaggctaccacgctctggggtagtgctgcctgcgcgattcccgcgaccactgcacactctgatttcagcattacaccggcgggttttaacacgccacgcgaggcatgaatcatcgacattgaatcctcaacggttaccgcctgcgcaccgtttttttgcatgtcaatctcgctacgtcccaggaccggcagaatatagctatgccgtgcggtcaacagatgagagcggttaagcttagtggctacgtgtaccgccaaatctaattgcgttaacggtacagcgctcgcttcccgatctggcattgccagcgcaaaattgccccccatgcagatcaatgctcgagcctgccccgtacatattgcttgcatgctggcaattgcagcatgtccaggtgcatgaggtggggtgaagccatagcgctcacccagacgagccagaaactctgcagacggtttctcggtgataccgacggttcggtcgccctgtacattagagtgtccacgtagtgggcagatacccgcaccaggcttgccaatgttacctttcatcaacagcagattgaccagttgctgtacgttctgggtaccatgttcgtgctgagtgatccccattccgtaacagataatggtgcgttcggcagcggcatatgcgtcagccagttcggcgatttgtgtctgacttagtccagaaatacgttcgatatctttccactcggaattgagaacgtcacggcgtagctcgtcaaagccgacggtatgcgtttgaataaactcgtcatcaagcaatgaaggccgacctgcggcgcttgcagcatcatcgcgctcaattaacaggcgcatcatccccttgagcaacgccatatcgccaccaatgcgcacgttatagtaggcactggccaactgagtctcagagttcgtcagcatttcaaacgggttttgcggtgcggtaaatcgctccaggccacgttcctgtagaggattgatggcgatcattttcgctccccgtttcactaaagcgcgcaacgaagtcagcatgcgagggtggtttgtaccagggttatgcccaatgcaaatgactaaatcgcacttctcaaagtcttccagcaacacggtccctttacctacaccgatactcgctgccaaacccacgcttgtcggttcatggcacatgttggagcagtcgggaaagttattgctcccgtattcacgggcaaaaagctgataaagaaaggcagcttcattggaagtgcggcccgaagtatagaattcaacctgattgggatcactatagctttgaaggcgtgcgccaatttcgtcgaaagcttgttgccagcttaatggcttgtaacagtcgctgacggcatcatatttcaaaggctgagtgagtcgccccgcagcctcaagctcgtggtctccccaggtaagtaatgattgaaccgtattctcagcaaagaaagaggcgtttacctgcttatccgtgacttcccaggcgattgcttttgcgccgttttcacaaatgtcgaatgacgcactgtgcttaggatctggccatgcacaacccggacagtcaaagccctctggcttattcatgtcaaacatggcaataacatcctggcgtatatccatctgcttacgtactgcattcgctacggatttaacagcaccccaaccacctgcagcaccctggtaggattcaatttttttcttcatctacttatcctgtgtggaaatgaattattaggatttgtaatagcgatgatgcacagtacatacaaagggattatcgccaacatggatatataagagtaggggactactctctttctatttttaatctattatcgttaaacaatagattaaatacgataagttaagcatcatctctcatagtgtttaaattaacatatttttcaatataaaaaataagactctggcttcaattgtgcgcggattttcttacaggtgtaggctaatagccttcacaaaataattatccgcgcaattttcgtgaatggagcgcatagactaaggtcaaaatcacaattattcatagataaaagtgacaccaatgactgactggacggttccggctgaaaccttgtttcctgtttgtccataggttgcgcttaaacccagaggtactttgcttttatttactgtccccagggagacattttctcccgtagccagtatttttccattacgcattagagtgacacccactcccgatgcttttgttgcatcaggtgctgtgttagcaaacacttgtcggctactgtcagtggtggcacccgaaagataaaatgagagcttttgttcgcttgagcaatatacgccaaggggtatttctgcgcttccaggaaagtccgggagatccacggtgacatttcgactatcaacggtgcagccgcctgttggcataacaacattgttatttgaaataatattccacgtaaaattacgcggatttccgcttcctaatgttgcaattttatacatatgaatacgggcaatgacttcccccgcttttatgacaactccaccggccgccccaactggggtaatatagagttttaacggtaatggcatcggtgtcttatcaccaatatccaatacgttggtatttgtcgtcaacgggaaggggtaggtcacattattccagtacagcgatcctttatatgactgtagggagcctgcgaaagctgagccttgtaccaggtttatatgatcagtgtcgtaccagccgccgtaatcattccagcaacttatatgctgagacaagtctacaaccagattctggcccggctgtattacagggtcgagattaacataaacagaggttgtacctgctccaatacttgacccgccatcgacattacaactgaaggcaaaaactttgcctgccattaatagaagataaataccgaacaggacctttatactgattgttttacccatgatatatcctaaggttaaaaattgatttaaaaagaaggctaagaaaatcgaatcgacgttattgccaggtgtagatcacattgattagcgcctcgatcgttccctggcttgcgtttccattcaccgtgatagctcttgccttaagtggaaactgtgcattacgagtgatctcatcaacaataaccgttttgctatcgccattttttaacgcagcatcctggtcatccctcagctctatctgaatattttcggcagtaccttcatttttgtaataacccgtattgtcagttgaacctgtcacgattgccgtcactgcacttgtttcaaccggacaatcggttaatgacaaagtaatattgtgccagccagatgcagaaccaggttgttgcagattgcgcgtataaagatccccgagattaacgttagcttctttggtttgaatagtgcagggtttagcgactacccgaccattaacagtgatagtgacatcggcggcctggagagttgctgtgaataacgcgcaaaacgtagctaacaggaacctcttgtgaagtcttttcatatctgactctgattattgaaattcaagggtaaaggttgccgaagccctcaccagtcccggattgacggacttctgagttgacttcagacgagcggagtaaggcaaaatattgttctgttctggtaccagtgggatccactgcatcccggcatgaagatcattcagtttcaccggacgcatatttgcgtccaatatttctatacccaaaccggaggccgtattgcttccttcatccagtttcaacaaagtattattttctgcatcctcaataccgttaaatgcaacccgaacccccgttgtccctttgctgcattcacttaacgtaatctgaaaagggacggctggacttgtgctaccggtcgttggaaattgtctggcactgtttttttggagatctacggtaaaattaagcgaatccgatgagactgtgcagccataatcgaggacgcgcccgctaattttaataacgctatctgcggataaagcagaataggtggttaaccccagacataaaccgaggaaaataatgttattgtatttcataatctattgttccttagcgacagattgctgtctgctggttcagtaaggtaccaggagaaacttcaggaagcttgtactcgacaatacagtttgagtttttatctttgccccatgaaacctgtaattgccctgactgtggaagtccagtcagataaacctgaccattttccgcgacaatgctgccatttttattctctccgtgtgtgacaattgcaccgaatggaacgctcttattaccgtacttcaacgtcattaatactttcccgccgatttgtgcattaaatgttgctctggcaatagcaccgtgagttgggatgacagtgaccacggtttcatccagttcaacattatctgcaagggaattcgcgttaagagcaacacggttttctctatattctgtcgcaaatggtaatatggcatagccacgccagtcggtatgaattccggtctggttctctattttgacattatcagcaccaggagccttaaccagaaccattgtgtcgcccagcggctgtccaaaggtgatgccatcagcatgagcaataatcccaccactcattccgtaataaatctggctgctgtcaccactccgactgtaaccgacattagtattaccataagctccacgataattaagagaactgtaaccactggtgccagacgatgtattacctccgtgggtgttaccgacctgaacgctataattcaggttattatccggcagcagagtgccataaacccccgatagattggtcatgccgcctttcaaatcgtttgacatactgtaactggcgtttgaattacgaaatgccgactgactgtctgtacgcatccaatgactgaagggaacattaagcgtaaaagcgagtaaatgatcccgatcgttttgccatatattattggaatagctgtaattcagcgaagtcgtaatatcaccaaacggcacatttaatccaaatgatatttgctggtcgctgcgtgacgtgttccagtaactttggcgactggcactgaaaaatgtcgtaccgtaatttccaagctgctgagagatgcttatttgttcctgaccacgcttactgtagaacagattaaaataatcaataaattgtgtctgctcattggtgtctccggtaggaggcttgacggtgtaaccactcattcgactgtaggcactgtcggataagttataaaaaccttgcgtagaatagcgatatcctgcgacctggatattggttccacaacaagtttattgctgcacttgttgaagagagtatttgcaaaaacattttatgtcgctaaataacatgacgatttcattatgcatgttatttataaaccgtgactaaacagaatattattgcgaacaagggaagtgtcaggaaaggtcaagagctaccaatggttaatatggctataaatcattagctatggttaatgtttgcttgctgaaactaacaccgaattgctctaaacagataagtgcagggtttattaaagctgtccgacagactttcttaacctggtaatatctctcttgggtgactctccaaacatccgcgaatattcccgactgaaatgggatagctttcgtaaccgacagcataggctgctgtggtgacatcgtaatgttcattcagcatctgtcgcctgacttcattgagacgtagccatttctgataccggagtggactcattcccgcttgatccgtccttaaataagtaacagcaccctctggtgttttcgtatgcagtgtctatgcgacagacactgcgctcttagcatggggcagggaataaccaggctatttctccatgcacaggccaattatgaaagaggagaggcttaagttcttgaaccctgaacgaataacgactaccagaaaagcacttcgcatcactcagacatgatttaacataatatacattatgcgcaccaatataaaccaaggaagaatccagtcgttggcggtcatgattgtcatgctcattaacaatgaccaaaccccatatctcacttactaccgtattctcggcttaaccgtccatgcaacctcaacacattgctttcaactgccgtcaccacgttctccggaaaatctgtcggtaatgaagtcttcacgttatccagtgctgctggaatcattctggcaaagtcactcaggatttcatgcatctgcacttccgggaatctcagcacctttgctgtcgccaaaaaatgtcgcggataaattttatcgattgccgtttttttgcctttggatgcgttaagccccattgccagtttgagatcgctgatgtgtattcccgtaccgccaaggaccggaaatgctgaaatgatgtcgtaaaatggcgtgagtcgataactgccgccagcctgaataaatacggagaagttttttgcatgaccgtccgttgcgccaatcaaccactggaagacctggaatttcataaaatcatagcgatctttcagcgcctcgctggaccccatcaaaaaagccatgatccgcgcgatgcctgggcctccatctgattcatatttcaccgatgaaggtaaaccgaatgtctgacacatatcctcctgtggcaagcgaagtaaaaccgttcgctcagcattccaacgcctgtcaaaacgttcgaccgctaacgcgcgcacatttcccgctttaatgatttctgcgtccggaacattcaacccaagttctttcgccagcagcagacagtaatactcattatcaacgctttggctgagatcgagcgtcgcattgggctgcctgatttcgccaatcggtaatttaatgatgtgcgtcgtcggcgttattcctttcggaatgcaccagtcattgcctattctgagcagtgctgtcttctcctgtgcgccagcaaccgagatgcgaaagtcattttcttctctaatcatgcctagcgggatatctgctttataagccgttaatacttcttcaagtctggcttcagtaagcttttcccatgccattatcggatgcgttacggtttcgtcttcgggtattaacgtcacggcaccaacgctgtctcgccctatttctgacaataaatcaaacggttgtctggatttggcatgataacgtttaacgatccggtcacgtacaatcgggctatcgggtaacaggttatcgaagaagttaaatacggcatcagaggtgatattccccctctgcaatggcagcgaaagtgacaacggtctggcataacggcttgctaaccactccggtgcatacttaaaggtgtgcgcgccgttggctaacttcgttaactcgcctacccgctggttgttcatccaagtgacaagtttaggcattaccactccagattttgctgttctgttgattctggcgaggcatttttcgcgtcgcatagcgtcattgagagttcaagcgactgtaaaatcttaaaaaatgtcgtgagcgtggtattgtcagggttgttttcgaaattggaaatcgtcgcctgcttaataccaatttttttcgccagctcgctctgcgtccagccattttgctggcgaaccagtttcattgcattcgccaattgcgttgggctatagatcttctgaaagctcatcatgtcatacgtccacagcaagtttatccgcttaaggggatattataagttttatcctttagtgaggataagtcaatctggaaacacatcttatccgctctacgggataaacgctgcgatatccgcgatcgcggataaaaaggaggatttaaataaggcgttgatgcgccgtttgaagtcggcaatattaagccgcatgccatctcgacatgcggcttatacggtttaccagctatatttcactcccagcatgccctgagtatcgctatagcctttatcacctagttgcacaccgacattcccccacaggctaaggttgttatttactttcgcctcaaccccggtacgtacttcaccgagattacgcgcaccttcacggcctacggtttgaccattcatcttcacggcgtagactttgctattgttgatccagttcgcttcaatgtaaggctggaactcacgctgtttaccatcgtcacgctggtgatggctgttcaggtaggttttcaccccaagtcgcgtttgcacatttccgtcgccttccgtttcaatgcgcgttccgtctttccgggtatggtcggaatctttcacacccatccaggtgatttgcgcctgtggctggacgtaccaggtattcagcgtcccttcgctgccgctaaatgttcccgcttcaaaggtatacccaccctcaacagaggccgtcacaccgcgagaatcatagtcgtcagcagaacggttatcggaactgacgctgttatcaaaccagttatacagcgcccagctgtcaacataagcgccggtcttattcgcatcgttctgataccaggtcgcgtacagcccagcgctgtaaccgctgatgcgcccatccgatttataacccacacgattactctgagtattactgtgctgattggcgtagcctgccatcacgccaagatgccagcgatcctgcgcgttgctactccactgcgccaaatcgccgcctagctgcaatacatagcggttagcctgagtatttagctgaccgtcaccggcccttgaacgttcgtgccctccgacatgacgcatccacatactgcttgccgacccctgagaatgcagtgaatctgtatactgcggctcacccagacggtcgtgtaaacgatggctaaacagcgagttggctgcggcaatgttgctgatatagcttccggcctccgggcgataaactgatgggccttccggatccacaacagggggattattgatgggatcgggtgtatccgctggcgttacgccgtcccatttactggtcagataccagtttttctcgtcattccccttccctttagccagcgtgtagacgtaagccccagcttcgacagttccggtggtcagcgcgaagttacctgcagaattaccgccaacctcaatgagttcaataccgttgaccgtttgtgcaccgacgccgccaatgttatcaacccgaacgcgagtgttcccttgggtatcgcctttcacgttcatcttatcggtgggcgaattatcgccgcccagcgtcgcgttgaacgtcatcaggccattgtttccggtatagttgccgttaacggtcagtacattccccggtttccccccttcgctattcatttgaaccgtgccgccattctccaggttgccgccgatagtggttttagcgacacgcagtgccccccccaggcataacgttcatatcacctgcagtggtgacatttcccgacatcacaccgctgttatggatattaatgtgttgacttgccatattaatggcagagtcggaaccgaaagcaatttccccccccacgatatccgtcgtaccctgatacgccgcggaatcgttgttaagagtcaggatcccggtacccagttttgtcacatcaccgctaccgctgatactgtgcgtcatcgcccagctacgctcagtggagatggtgagcaggccattattgataacggaagcatcacccaggtttttctgctcgttgacgctgagcgcgctgcctgtatcaatgttgaattgccccacaaagcggctattatcgccatccaactctacatctgtcctggcggttgcgctcacgatacccttcccgcttatgctattacgcagttcgccagtcacgttttttagcgttaacagaccgtcattggcaatatttcctctgcctaacccctgagtattatcgaggctgacttccgcatttgggctaatgctggttaacgcattgtagcgtgcattaagcccctcgatagccagcgttccccctgtaacattcaggtttccgccacctgtcagttcaccctgactgatcccacctttatttaccgtcagcgccccctctttgaacaaaacagtcgaacccatctgcccggtgaatgtctctaccgtctgcgtcgatccattaagatcgacgatggccgcgttgctgatgttcagttcccgggtgttgccaagtgcaccatccgcatcggtacgtaatgtccccatctgaacgtaggttgccccctgatagtcgttctgaccgttggaaagcgaaacctgtcgcaccgtattgattgccagatccccttcaccaccgatttttgccgacatatcggccgttgcgccataggctccgccatgttcggctaacgtcagcttttgcccaccatggatgttcagcgctttcagcccatagttaacgtacaaaccattacctggtgcggtcgtgaggcggaatccataatcaccctcggcgaccaccgttccgttttgcgcaatgtgtaacgttttgtccgcttccacctcgtcgccctgtaaatcacgtaacgttaatgagccacccgacccaataaccgtttgcgccttcaccagttgaacgccgacatggctatcgtcgtgttccagcaaattgagcgtcgtcagagggttattcgccatgggatcattccacggtttaggcacgtcgataagcacgtcgcccgtcccgtttacctgatagttacggcctttccaggtgtagtcacccgcgccgacaaccagcgtatcgacgctgatatatccctccgcgagcgtcgcagcaggaatatccgtatcgaaaatgatggtacctccattcatggccagtccaccaatggattgctctccaacttttaccgatgtggtattttcactgtcagactgcaacatcgcgtgagtaagcgcagcggtgttgtcgcgttccagagtgaaggtactgtctttcagttgggcaacaccggcgaattcagtccctgttgcatgggtaaagccaaacatcttgtcggaggatgacagctgcactcgcatcaagccatcgcctttgagcgcattggtcagcgtgtaatctcctgcactgttcgttgatgcgagaatgtcgagcgtaccggggtttgcaatggttacttcactcgaccccatgcccgttaccccatctgccgtatgagacgcaatggtcaggaggccgtcattgaccagcgttttaccgctataagtattccctgcattgaacaccgtatggcctgcatcatggatcacttttccgtctttatcgtcacctgtaatcagcatatcgacctggtagccggcatcactgttattggtatgattaaagacaaaaacgccttcgccaagaccaaactccactttcgtcgcattggtgataaatccggcatctgccgccgcctcaccgtgagcagcaccaatgtttagcgttcctacagcaggctcaaaaacacctaagtaaacttctccaccttcgacattcagcgtaccgttattcgtcagggttaacgtacccgtaccagatgtccctacgtacatattgaatgtttcaagaagagagttctgcccatccaccctcacgtcgcccttacttttgtcattgagagctatctgtgtatcacgcgctttaactatacctccggtggtaatattcagttcacccgtgcctaatacaccgacctgtagcaattgtgcgttagtagatgatgtctttaaattccagagactgtccgttgaaatattaactatccccttaccggaggcatttcctccgataaatccatagcccgttgaattaagggtggcaccattactgacatttacgataccgctaccaaaattaccgacattgatacccacagtatcgaacgatgatgtcgcatccatcaggttcagtgtgccgataccgcttgctttatcgcccaaaaaagtaatattttgcgatacgaacttaccgccatcgctaatattgaggtttccgacgcccgcaacaccaatggtggtatagacattcttattgacctcccacattccccccgtggtgatgctgacattcccgacgccggtttctccataaccgagtgaacttcctccgttgctgacaacaagcccctgattactgatattcatttcgccgtggccgtcataaccaagattagttccgagattagtgataacggagttcttatccttaacagtaatgttgcctgtgcctgtttctttcatccccgcagtgataattcccgaatctactttgccttcactcgagacattaagttcaccgtcgccagcatcaccgatatagatatagcggaaagcttcgcccgttccgaggaaattccaatgccctttatcggtcacgttgacgacaccgtgggaaccgtcctgaacgcccaccaatgaatattctttgttattaatcagtccattattggaaatattgactgtgccattaccgaaatatccattatagagtctgcgtaccgtgatgacagagtcttgatcctgcacattcagggttccgataccggtggcattgccaccgataatcgtattttcagccgtaaccaaccccccctcgcgaatagtcgcctccccagttccttgattaccaatttgaaattcaattgaggaatcattattttttattagccactcgccacccttttcaacgacaacctggccattactgcccgcctgatagcctaaaatggcgacgattgaactcgtgacgtaacccttatccgtaatatttaatgaacctgtgccatagctacctatttcgaataattcggtcgtcagaacagagtcctctccctcaacattgaccgtcccgacgcctcctgtcgaagaacctaatcttaaatagcctccatcgacgtgacccttctgtttaatattcagcgtccccgttccggattgacccacatttaaaggccttgcattatttccgctatcatacaatcgccaggtgccacccaaaacattaacggtgccctctgagtcctcattagcgccaatgacgctggtagtaatagtggttaaggaggcattaccgccagccaaaatattaagcactccagtgccataccagccaaccaggtaggcatcataagcaacatcagtatcaatattggtaatctgatcattatcaacttccagacttgcaccagacgctgaaccgcttagtgccagcaaaacacccagcgtcaatctactgaatttcgttgtcagtccagaggatttacgcaaattaaccgtcgatgttttacctgccctgcgagttaattccgagcaggcctgaaatacctgtagagtgcaattccatatcacgcgatagattctattcatataaacgctccatatacaaacaatacagccacgaaagagatgagtcgtcagacattaaaaatgaaacttattaaattgtcagaggtctgtattgagtgttagttggaggtgggaaggtgtcaatttggctaatttgctaatgctttcgaattgatagattaaaaattgcatagttcttattttatttaaatatgaactatgagttattgttgcttaataagaaaactgtttctttcaataggaaaattatcatcatcatatttaacaaagaatagcactaattgctaaaaatcgaagtttattaaaccccttttgcatccattagtgtctttaggaatattcgctataaaataagggttgtgcttaatgctttaagaaaaatagcaattttcccttgaatatcgtactggtgatggaacgatgaatctgcaagctggcttttaacaagccagctctaaaagaagggaaataagaataactatactcaaaaactaacagccacggtcatcatgatgtggctgtcaatgaaactataacccaggcgctttccataacgacgtcgtcagtccatgatcaaccagccccagctgatcctgataaactgcctgccacttatcgcgtgaatcctgataaagttcatgcttttccgggtctggtgtgtgcgtccgttcccagcgaaccaggcgttctccggtttctgccattgatgaaaaaattccggcaccgacgccagctgcaatggcacatcctaatgcagtggcttctttgaccaccggaatattgacgggtaatcccgagacatcagcgagaatttgactccataatttcccttttgaacctccgcctgcaaagactaacgatgaaggatgaatattcgagaaatcagcaatttgctgcaagttacacgctgatacaatcgccgcattttcttccagcgcacggaacaatgtcgctttgttacatttatccgggtcaatggacaagttaataaaggaaggcgcagcgtgataccaggttttaaagcgcattctgtcggagaagatcggcattacgccccacgacccaggcggcacccgactggccatctcttccagcagcgtataggtgtcgatgcctaaacgttcggcaatcagtttttcttcggcacagaaagcatcgcggaaccagcgcatggtgagtccggtaaaaaagcttatagattcagcttgtaccatgccaggaataacatgaggattaacgcgcacgttcatttctgggtctgtcaccggcgcggctaaatttacaacttgctgccagaatgtgccgccaagaaccgcggtttgtgccggacgcacaacgcctaacccaaggcaaccaagctgcacgtcgcctcctccaacgaccaccggagtgcccgccttcagaccgcagagttccgccgcttgtgaacttaccacgcccagcaatgtgccggtttctttgacaggagaaagaatatcggcacgtaggccagccatatccagcaatgcaggtttccagtcacgggtggttagatcaagaagtcccgtggtgccagcgttagagggatccaccgccagttcgccgctgagcatataggccagccagtcgctgatcatggtgatggttgatgcctgacggtaaatatcggaacgatggtgcgccagccaaagtaatctggggatggcacttaaagccagtgtttgtccggtcgcgcgataaacttcgttttcaaaggtattgttgtgcagttctttaagttcgctaacttcgcgtgccgctctggcatccacattggcgcaggcccagatcggggctccttcattattatataaaacaatgccttcacgcatcgaacatgccgaaacggcagcgatatactccggggctatgccggcgttgtgcagcgcctggcgcatacactcacacgccagttgccagtttttgttgagatcaaattccatagaaccaggaacgtccggtactgccagatgccgccactccgcctgtcccactgctatttgattgccttccaggtcgaatatcacagcccgaatacttccggtgcctgcatccagcgccatcaggtagtactttgattctgaaagggtaaagagtcgagccattagattatcctcggcttatgcgttctgtctgttcctctatacgttctccatcattcccggtaataaggtcatgcaaatttaactacgtaaaatcgccgctgctgtgtcctgatcggtaaccagtgcgttgatataaccgcctttcattgcagcggcaattgcttcggctttattttctccccctgccacgccaacccggacgggtatggtcttcagcgcgcttaaaggtaagccaatcagttcgttatgtattttgatattcgtgacaacgtcaccttttgcatcaaaaaagtagcctaaaatgtcgccaaccgccccttttcggccaatcattaactgttcgccctggctgatataaccggagcgaatgattgtcgcatcgtcctgttgactcacagcaccaatgccgacaatcgccacatccgctgcttgcgcggctaacagaacatctttgacgcaattttcattttttagcgtacgggcaatgtcagcggaggatgcccgcaacggagccggaataatattcacactgcacgccgcgttaagctgcccgattcccgtcatataagaaccgacgccaccggagagcgtgaccaggcgaatttgctgtgacgaaataaaaccacttaagcgttgcagcgtattcatggttgcctcgccaaaaccaatcgccagcatctgttgtggttgaagtaaactcatcaacatatgcgccgcgcctatccccagtcgcccaccgacatcagcatccgcaagcccagggatcacccggacatgttgcagcgaaaactgacgacgtaattgagtttcatattccagacagccttcaaagcgagaattaatctgtacgcgaataatgccggactgatgccctttctccagcaatcgcgacactttcaaacgtgtcaggccgagacgatcgctgatctcgctctgggtcagcccgtcgtgatagtaaaaccacgcgatccgcgcgacctgttcttcttcacacattccctgttctgaaattgccgaatcgttgattgtcataattcattcttcactttgaacatatttaaatctttaatgcaattgttcagttcttgctcatttatatctgtgatggcaaccacagtttgactctacgagcatgaacaaacgcaaccgtgaaaatcaaaatagcataaattgtgatctattcgtcggaaatatgtgcaatgtccacctaaggttatgaacaaattaaaagcagaaatacatttgttcaaaactcacctgcaaaactgaacgggggaaatatgcaaacgagtgatacccgcgcgttaccgctactttgcgcccgctcggtttataaacagtattcaggggtcaatgtcctgaaaggcatcgattttacgttgcatcagggggaggtccacgccctgctcggcggcaatggtgccggtaaatcgacgttaatgaagattattgccggtattacccctgctgatagcggtacgctggagattgagggcaacaactacgtcagattaacgccagttcatgctcatcagctgggtatttatctcgttccccaggaaccgctgcttttcccaagcctgtcgataaaagaaaacatcctgtttgggctggcaaaaaaacagctctccatgcagaaaatgaagaacttgctggcggcgctgggctgccagtttgatctgcatagtctggcaggatcgctggatgtcgccgatcgccaaatggtggaaatcctccgcgggctgatgcgcgactcgcggattctgatcctcgatgaacctaccgcctcgcttacccctgcggaaaccgaacgcttgtttagtcgcttgcaagagctgcttgctactggcgtgggtattgtttttatctcgcataagctgccggaaattcgccagattgccgatcgaattagcgtgatgcgcgacggaaccatcgccttaagcggcaaaaccagcgaactgtctaccgacgacattattcaggccatcaccccagcggtacgggaaaaatcgctctctgccagccaaaaattatggctggagttacctggtaaccgcccacaacatgccgccggaacgccggtgctgacactggaaaatctgaccggcgaaggtttcaggaatgtcagcctgacgctcaatgccggagaaattctgggcctggctgggctggtgggggccggacgcacagaactggccgagacgctctatggtctgcgtactttgcgtggcggacgcattatgctgaatggtaaagagatcaataaattatccactggagaacgtttactgcgcggtctggtttatctgccggaagatcgccagtcatccggactgaatctcgatgcttcgctggcctggaacgtctgcgcccttactcataaccttcgtggattctgggcgaaaaccgcgaaagataatgccaccctggaacgttatcgtcgggcgctgaatattaaattcaaccaaccggaacaagctgcacggacattatccggtggcaaccagcaaaaaatcctcattgccaaatgcttggaagcttcgccgcaagtattgattgtcgatgagccgacgcgcggcgtggatgtctcggcccgtaatgatatctaccagctgttgcgcagcatcgccgcacaaaatgtggctgtgctgcttatctcctccgacctggaagagatcgaactgatggcagatcgtgtgtatgtgatgcatcagggcgaaattacccactctgcactgaccgagcgcgatattaatgtcgagactattatgcgcgttgccttcggcgatagtcagcgtcaggaggcgtcatgctgaagtttattcagaacaaccgtgaaatcacggcactgctggcggtggtgctgctgtttgtattacccggttttctcgaccgccagtatttaagtgtgcaaacgctgaccatggtttatagcagcgcgcaaatcctgatcctgctggcaatgggcgcgacgctggtaatgcttacgcgcaatattgatgtttcagtgggttcgattaccggaatgtgcgcggtgctgttggggatgttactgaacgcaggatattcactacctgttgcttgtgtcgcgactttactgcttggtttgctcgcgggatttttcaacggtgtcctggtcgcgtggctaaagatccctgccattgttgccacccttggcacgttagggttgtacagaggcatcatgttgctgtggactggcggcaaatggattgaagggttacccgccgaactgaaacagctctccgccccgctgctgcttggcgtttcagcaattggttggttgacgataattctggtggcatttatggcctggctgctggcaaagacggcgtttggacgcagtttttatgccacgggcgataatttacagggcgctcgtcaactgggcgttcgtactgaagccattcgcattgtggcattttcgttgaacggctgcatggcggcactggcgggaattgtgtttgcttcgcagattggttttatccccaaccagaccggtaccgggctggagatgaaagcaattgcagcctgcgtgctgggcggcattagtttgctcggtggttccggtgcgatcattggtgcggtactcggcgcatggttcctgacgcagatcgatagcgtactggtgctgttgcgcattccggcatggtggaatgattttatcgcgggtctggttctgctggcggtgctggtgtttgatggacgcctgcgttgtgcgctggaacgtaatctacggcggcaaaaatatgcccgctttatgacgccaccgccatccgttaaacccgcttcgtcaggtaaaaaacgggaggccgcataatgcgtattcgctacggttgggaactggctcttgccgcactgctcgttattgagattgtcgcatttggtgcaattaacccgcgaatgttagatctcaatatgttgctgttcagcaccagtgactttatctgcattggcattgtcgccctaccgctaacgatggtgattgtcagtggcgggatcgatatttcgtttggttcgaccatcggcctctgcgccattgcattgggcgtactgtttcaaagtggtgtgccgatgccgctggcgatactcctgaccttactgctcggcgcattgtgcgggctgatcaacgccggattaattatctataccaaagttaacccgctggtgattacgcttggcacgctgtatctgtttgccggaagcgctctgctgctttccggtatggccggagcgacggggtacgaaggtattggtggattcccgatggcgtttacagatttcgctaacctggatgtgctgggactccccgttccgctgattatcttcctgatatgtctcctcgttttctggctctggctgcataaaacccatgccggacgtaatgtgtttttgattgggcaaagcccgcgcgtggcgctttatagcgcgattccagttaaccgtaccttatgtgcgctctatgccatgacggggctggcgtctgcggtcgccgctgtgctgctggtatcgtattttggttcagcacgttccgatctcggtgcgtcgtttctgatgcccgccatcaccgccgtggtgcttggcggggccaatatttatggtggttccggttccattatcggcaccgccattgcggttttattagtgggatatttgcaacaaggtttgcaaatggcaggagtgccaaatcaggtgtccagcgccctttccggtgcgctacttatcgtcgttgtcgtaggtcgttccgttagcctgcatcgccagcaaattaaagagtggctggcgcgtcgggccaataacccattgccataaaggatatcttcatgacacttcatcgctttaagaaaatcgccttacttagcgctcttggcattgccgcaatctctatgaatgtgcaggccgcagagcgtattgcatttattcccaaactggttggcgtgggattttttaccagcggtggcaacggcgcacaacaagcgggtaaagagctgggcgttgatgtgacctacgacgggccgacagaacccagtgtttctggtcaggtacagttgattaataacttcgtcaatcaaggttataacgccattatcgtttctgcggtttcgcctgatggcttgtgtccggcactgaaacgcgccatgcaacgtggtgtgagagtgctgacctgggactctgatactaaaccggagtgccgctcttactacattaatcagggaacgcccgcccagttaggaggtatgttggtggatatggcggcgcgtcaggtgaataaagacaaagccaaagtcgcgtttttctactcaagccccaccgttacggaccaaaaccagtgggtgaaagaagcgaaagcgaaaatcgccaaagagcatccaggctgggaaattgtcactacgcagtttggctataacgatgccactaaatcgttacaaaccgcagaaggaatattaaaagcgtatagcgatctcgacgccattatcgcccccgatgccaacgccctgcccgctgccgcacaagccgcagaaaacttgaaaaatgacaaagtagcgattgtcggattcagtacgccaaatgtgatgcgcccgtatgtagagcgcggcacggtgaaagaatttggcctgtgggatgtggttcagcaaggcaaaatttcagtgtatgtcgcggatgcattattgaaaaaaggatcaatgaaaacgggcgacaagctggatatcaagggcgtaggtcaggttgaagtctcgccaaacagcgttcagggctatgactacgaagcggatggtaatggcatcgtactgttaccggagcgcgtgatattcaacaaagagaatatcggcaaatacgatttctgatgtgcattacttaaccggagtaagttatggcagatttagacgatattaaagatggtaaagattttcgtaccgatcaaccgcaaaaaaatatcccttttaccctgaaaggttgcggtgcgctggattggggaatgcagtcacgcttatcgcggatatttaatccgaaaacgggtaaaaccgtgatgctggcttttgaccatggttattttcagggaccgactaccggacttgaacgcattgatataaatatcgccccgctgtttgaacatgccgatgtattaatgtgtacgcgcggcattttgcgcagcgtagttccccctgcgaccaataggccggtggtactgcgggcgtcaggtgcgaactctattctggcggaattaagtaatgaagccgtggcgttatcgatggatgacgccgtgcgcctgaacagttgcgcggtggcggcgcaggtttatatcggcagcgaatatgaacatcagtcgatcaaaaatattattcagctggttgatgccggaatgaaagtgggaatgccgaccatggccgtgactggcgtgggcaaagatatggtgcgcgatcagcgttatttctcgctcgcgactcgaatcgccgctgaaatgggggcgcaaattatcaaaacctattatgtcgaaaaaggttttgaacggattgttgccggatgtccggtacccattgttattgctggcggtaaaaaattaccggagcgcgaggcgctggaaatgtgctggcaggctatcgatcagggcgcttctggtgtggatatggggcgtaatattttccagtctgaccatccggtggcgatgatgaaagccgtacaggcggtggttcaccataacgaaacggctgatcgggcatatgaactctatctgagtgaaaaacagtaactgcggatctaaggagaagaattatgcacgtcacactggttgaaattaacgttcatgaagacaaggttgacgagtttatcgaagtttttcgccagaaccacctgggctctgtacaggaagaaggcaatttgcgcttcgatgtcttacaggacccggaagtgaattcgcgcttttatatctacgaagcctataaagatgaagacgcagtggcgttccataaaaccacgccccactacaaaacctgtgtcgcgaaactggaatctttaatgaccgggccgcgtaaaaaacgtctgttcaatggtttgatgccgtgaggcgaatttatcaattttatctacaattggggtaacgcgctgacgggagtaaaaaaatgtctgactggaacccctctttatatctacacttttccgctgaacgatcgcgtccggcggtggagctgcttgccagagtgccgctggaaaatgtcgaatatgttgccgatcttggctgtggcccaggtaacagcaccgcccttctacaacaacgttggcctgcggccaggataacaggcatcgactcgtctccggcgatgattgctgaagcgcgcagtgctttgccagactgccagttcgtggaagcagacatccgcaactggcaaccggtacaggcactcgatctgatttttgctaatgcctcactgcaatggctgcccgaccactacgaattgtttcctcatctggtttctttacttaatccgcagggcgtgctggcagtacagatgccagataactggctggagccgacccatgtgctcatgcgcgaagttgcctgggaacaaaactacccggatcgcgggcgtgagccgttggctggcgttcatgcttactacgatattttgagcgaagccggatgtgaggtcgatatctggcgaaccacctactatcaccagatgccgtcacaccaggcgattatcgattgggtgactgccactggattacgtccgtggttacaggatctgaccgagagcgaacagcagctttttcttaagcgctaccatcagatgctggaagagcagtatccactgcaagagaacggacagatactgctggcatttccgcgtctgtttattgttgcccggcgtatggagtaaatatcacgtcagctggtaatgacgatcgggaagaatttttgctggaatttcggcttcatcgttcatctgtaacaggtcaatttcaatagcgttgcagatggcatccagtggtaaatcattgttttcagtaccgaacggatcttccagttcttccgccagacaatccagcgaaataaaagtgtaggaaatcagcacagagataaaaggcgtcatgtaatgcaggtccacgaccagcgcgaacggcagcatgatacaaaacagataaacggtacgatgcaaaatcagggtgtaggcaaagggaattggcgtataggcaatgcgctcgcatcctgccaggaccgctgaaatatcattaagccgatcgttgaggctaataaacaggatatctgaaagctgtccattgcggcgctgaaccgccaaccattctcccattattaacaagatacggttagctggagagttcgaagccagtacacgctgaagatcttcagtcttgagataatgagccagcacttccgcctgtggctgtttgcgtaatgtcatgcgtaaacagtgggcgaaagcgatttgcagccgggcaaactcccttacacttgccgaatccggcaatgtcgtttttacctcgcgcagtaacgaccgtgaggcaatcatcaactgcccccaaagttttcgcgcttcaacgtaacgggcgtacccggcattattacgaaaaccaagaaaaatggcgatggcgacaccgagaatgctgaacggtgcgagggtgaatttgatgcccagatgcgtgtaccagggcagcatgaaaataacagcgatagaaaagagaaaattgagtagtaagcgcgaggatatcttggataatactgagccgtgccagacaaaaatacggcgcagccagtgttgttgtggacgaacaatcatggttatcttcaggcgtggaaaagtcgccctattaaacgtgattacgatcacattctcaagacgctacttacaaattacctacaagcttacaacattagcaggcgctgcatgtggcacctgttaatgataaaggcatataggatgttgtaactaatatggtgaaataagaaacccggtcgaaaccgggttcagaagtaacggtgttattagcacaacggacgtacagcttcgcgcatccctttttcgagaatcgcatccaggtcattagcaacctgctcgaccagaccaggcacttgcgtcaggtcctgctcccagtggtctttttctgccaaaacaatcgctaccagttcctgggtgccgataacacggtcacgatgctggctccagagttgctgataacgttccagccagtgtgcatcgtcctgtaccggatatgtttcgccgttacgctcaccacgatagaacgcaatcaatgccgctaatgcgaaagtaaggcgcgccggaagtgtgccgtttgccttctgccctgccagcagctgtggcaggatgcgggtgcggaacttggtcataccgttgagcgcgatagacagcagctgatgcttaatgtacgggttacggaaacgcccggtgactgcactggcgaaagattccagttcatcacgaggcaaatccagtaccggaataatttcttcgtagatagctttttcaacgaatgcgcaaatttcagcatcgttcatcgcttcacctacggtatccagccctgcctggaacgccaccggcaccagcgcggtgtgcgcaccgttgaggattgccactttgcgttctttgtacggtttaatatcgtcaacaatcagcacgttgagcggatatttgtccagacgcagttcagtcgctaaggatttcggtccctgaatcacaaacaggtaaaagtgttcagcggtgtcgagaaaaccatcgtgataacccagttcttcttccagtttagccacttcatcgcgcggataaccggtaacgatacggtccaccagcgtagaacagaagctgttagcctgatccagccattgaataaatgcttctggcagtgcccactcttgcgcatagcgcagcaccagttcacgcaacgcgtcgccattgtagtcaatcaactcacacggaatgatgatccaacctttatccagcgcaccgttgaaatggctaaagcgttcgaacagcagacgggtcagttttgccggatagcttaccgctggcgcgtcatcgaatttatcgcccgcatggtagctgatacccgcttcggtggtgttagagaaaacaaagcgcatttccgggttgtgcgccagtttcaggaattcatcgtattcactgtagacgctgatttcacgattaaccgagcgaatcagacgcgcgtcgctgaccgcttcccccttctcattcaggccacggataatggtggtgtacagaccatcctgcgtgctcagtgacggcgggaatgaagtttcaatcggacgaacaacgaccacgccagaattcagatcggtgtgctcattcaggagatcgatttgccagtcaacaaaggcgcgcaggaagttaccttcaccaaactgaatgatacgttctggatactgtgcaccgggaaaatcgcgacgatttagtgttttcacaatgggttcccttctgattagtcatacaacctgtttgaattggtacgacaggttagcaaactttaatacgccgaacccctgttttgatcaactcctgatgattaatgagcagttttatgagaaaagtgtggcgcggatcatggtttaatcgaggaaaaacgccttttcctggatcataaagtggtagaacacattgcattcaaatcgcgcgtaatgaataaagatgtcagacaacttcctcaccgtaacgcatagtgctggtacggttgcgcccatctttcttcgagcgatacagacacgtatcggcttcgaccatcaatttattaaagtcatcggtcagcgttaggtacgatgcgcgaccactaccgacgccaatacttaccgtgagataaagcgttttttgttgccaggtgaatggttgcagttcaacgcctttacggattttttccgccattagcagaccatcgacaggattcaccgacggcactgcaacagcaaattcttcgccgcccattcgcgccaccagccccttatcaccgacaatcttctgaatatgccgggcaaacacgcttaacactttatcgccacattcatgtccatagttatcgttaatgcttttgaaatagtcgatatcaagcagcatgacagtcagatgttgtgtctgtttcagcgatggacttttcagcgcctcataaagaccggaccgtgagtaaacctgagtcagaaaatcaaagtcggctcgcagcgcaacttgcttcattagcgaattgatcgctgccacgctaaaagaaaccataattgggcatatcgccatcgtggcaataccgagacgtgcggagaacatttgcggaatggagaacggcgaaccgaccgagatatcaatcaccgaatttgccaccagtacgatttccaccgcaccggtgacaaaggtcaacagacatgttacctgcggcgtatagcgcactgcacaccagattaatgcaggcagcgggaacgccagactccccgctccgccaatgactaccgaggcaataaccgacacaataagcgcgatggcgggcatcatctgttctgctttaaagcgcggcagcactccaggaatagccaacgtcagcatacaaggcacgatcaacacgcccgttgagaattgctcactgaaccagtccgcaagcaaaggccagaaatccagactatcaatactgaccgaaccaagatagcatgttcgctgacagcggcggcaaataaaggtaccctgggaatgctattttgtcgttttccgcaattctcatggctgattcatctgtacaaccagccagtgatagattaccgccacgatataacgttgttgttcttcgcttaacgaaacaccctgcggaatgttatgccacttagccagacaaccgcgacagcaggtcgcggtggcgtgctgagcgataaacaccggatgcccgcgcatgggggtttgcttaccgtcattagccggtaatgccggagcaagacgtttagcgacaaaatccgccgcatgttgttcgatgactggcgcgcctttctccaggcaatactgacgctctttcatgcccagacgaaagcgagagcgaaattttgaacgggataaacgcgcgaagagtggatcgagagactgcattaataaaccgaacgccctaactgtttcgtcaattgttcaagaacggcaatacccgcaagcgagttacctgcatcatccagttccggactccagacagcgatggccatttcatgcggaacaatcgccacaataccgccaccaacgccagatttcgccggtagccccacccgccaggcaaactcccccgcgttctggtacataccactggtcgccatcagcgcgttaatttgccgcgcctgcattggcgtcaccactggttcatcaatatgaatagctttcccctgattagccagaaagacaaacgtccgggccagctctacacagctcattttcagagcgcagtaatgaaagtagttttgcagaacggttgtcacgtcatgatggaaattgccaaacgacttcatcagccaggcgatagccgcatttcgcgcggaatgttcaaattcggaacgcgctaccaccgtatcgtaggaaatatcagacacaccgcttaagccgcgcacgacttccagcatacgttgccgtggtgcgcttaatcgcccttgcaacatatcgcagaccaccagcgcaccggcattaatgaacggattacgcggtataccctgctccatttccagttgcactaaggaattgaacggtgatccagacggatctttgccgacgcgttgccagatttcctcttcggagtaatgacgcatggcgacaacgagactcagcactttggaaatagactgaatggaaaaacgttcttgcgcgtctccggcctgaaaaagctgtccgtcaacggtacagatagcaatccccaatcgggaaccgtctactgtagccagcgccggaatataatccgcgactttaccctgaccaatgagcggccgcacttgccgcaagatgttttctaaaattgcattatccatggcgactgccactttctactcctggaccgcaggtctgaaaagacctgcgagtatatcagagctgaatatgtcgcgtcagatccggtctttccacaccgtctggatattacagaattcgtgtaagccgaaatgggaaagctcacgaccaaagccactctttttcacgccaccaaaggccactcgcgcgtcgctggcacaataaccattgataaacaccccaccgcattccagacgtgccgccatctgtctggcctgtgtttcgtcagtggtaaaaatggtcgctgaaaggccgaactcactatcattagccagttccagtgcatgttctgcatctttcgcaatggtgattgccgcaacggggccaaacatttcttcccgaaacgcggtcatttctggggtaacattcgccagaaccgttggcggatagtagttacctgccccagccatcttttccccgcccagtaacaaacgcgcaccctgcgccagggttttctccacctgatgatgcagctcatcacgtaaatcaaaacgagccattggtccgagagcgttctcttcgtcacggggatcgcccattttcaaggctgccgcagctgccacaaaacgttcggtaaatgccgaagcaattccctcttcgataataaagcgttttgccgctgcacatacctgtccggtattctgataacgtccggctaccgccgctttcaccgccagttccagatcggcatcgttaagcacaataaacggatccgaaccgcccagttccagtacgcattttttcagtgccgctccagcctgtgcgccaatagccgctcccgcacgaacacttccggtcaccgtgacagcagcaatgcgcgagtctttaatcatctgactgacaccgtcgttgtcggcattcagccagccatatacgccttgtgggatacccgcatctttaaacacctgggcaatgagctgtgcacagcccatcacattcggcgcatgtttaagtaagtagccgttacctgcaagaatgatgggaacagcgccacgcatcacctgccataacggaaaattccacggcataatcgccagaatcgtccccaacggtcgatactcaataaccgcctgctgattttccaccagcgtaggttccgccttcagcattgccggaccatgttctgcataccagtcacacaaattcgccgatttcgccacttcagcgcgcgcctggttgattggtttgcccatttcgcgggtgatcatttgcgccatttcttcgctacgagcgcgcagagccttaccgatatcacgcagtttttcagcacgataatctatatttgtctcgcgccagtcgcgaaagcctgctgccgccagctgaagtgcgttttcgatatcgtcagcgccagcccacggcagcacagaaagttgttcacccgtggcaggatttatcgaaattgcatgagttgccggagtaatggtcatcggggtatctcctttatgagtcatggtatgaagatacgcagatttactcttgctttaaaatgaataatattaagccacttattcacgaatcgagaatgctatggatctgacccaactggagatgttcaacgcggttgccgaagctggcagcataacccaggctgcagcaaaagtgcatcgcgtgccgtcgaatctcactacccgtctgcgccagctggaaacagaactgggggttgatctgtttattcgcgagaatcagcgtttacgtctctctcctgccgggcataactttttacgctatagccaacaaattctcgcgttagtggatgaagcgcggagcgttgtcgctggcgatgagccgcaaggtttattttctcttggttcgctggaaagcaccgctgcagtgcgcattccagccacgctggcggaattcaaccgtcgttatcccaaaattcagttttcactttccaccggcccttccggcactatgctggatggtgtactggagggaaaactgaatgcggcgtttattgatggacccattaaccatactgccatcgacgggataccggtataccgcgaggaactgatgatcgtcacgccacaaggatatgcgccagtaacccgtgccagtcaggttaatggcagtaacatttatgccttccgcgccaattgttcgtatcgtcgccacttcgagagctggtttcatgctgacggtgccgctccgggaactatccatgagatggagtcttatcacggaatgttggcctgtgtgatcgcaggagcaggcattgcgcttattccgcgctctatgctggaaagtatgccggggcatcaccaggttgaagcgtggccgttagctgagcaatggcgttggttaacaacctggctggtctggcgtcgtggtgcgaaaacacgtccgctcgaggcatttattcaactgctggatgtgcctgactcggcaagacagggatatcaatgagctatttttgatagttcttgcggttaatatgctctatatagtgatgttccgatgacttatgactatatggggcaaatatggttacgccagtaagcatcagcaattacatatctcttcctgatgattttcccgtacgtaatattgcaccgcaggtaaaagaagttttaaaggattttattgatgcacttagtacaataatatgtaatgaagagtggcgcacgtctttaaacatcaactcagccacaaaaaagatatttaataaccttgacaacttatcatatattcagaggacttcttttcggggtaacgacacgctatacaatgaaaaggttcagtttaaactcacttatcccgccaggaatggaagacacaaagaaaatattgaatttcaggtagtaataaatttaagccctatttatttagataattttcgccatgatggagaaattaatattttttgcgctcccaacccaaagcctgtcactatggggcgcgtatttcagaccggcgtcgagcgtgtactctttctgtttctgaatgattttattgaacaatttccaatgatcaaccctggtgttcccatcaaaagagcgcatacaccacatattgaacccctgccttcggatcaccataccgctgcagattacttacgccagtttgatttgcttgtcctgaattttatctctcgcggtaattttgtcatactcccccgattatggaataactctgaggttcacagatggttcgtcaataaagatcctaacttgatcaccgccattctcgacataacggacagcgaattaaaagaggatttgttgcaaagcctgatggattcattaggttctaacaaacatgtactacccgaagtctgcatctgctttttatcccttttagcagaacaagaatctcctcattttcagaacttgtttttatttttcgccaatatgttattgcactatcaccaatttatgaatcccaatgaaagtgatttgaatgacgtgttgatgccagcatcattaagtgatgataaaattatcaaacatatggcgcgcaggaccctcaaactgtttgtaaaaaatgaaacaccgccaaaagttactcacgaagacctggtgaaaaacaggcctcgctcccctgtcagaccacctatacccgcaaccgccaaaacgccagacctccctgaacgtcattaaaccgtgatgttaccgactctctgacgcgtgaaagaatcagcgtcagagaaacggaaaacgcgatccagatcacaaatgcattgtattcacatcattaaccgttttaagatcatttcatcactttttcgcaactcacccgataatctgttatgacaacaaacactgtttcccgcaaagtggcgtggctacgggtcgttacgctggcagtcgccgccttcatcttcaacaccaccgaatttgtccctgttggcctgctctctgacattgcgcaaagttttcacatgcaaaccgctcaggtcggcatcatgttgaccatttacgcatgggtagtagcgctaatgtcattgccttttatgttaatgaccagtcaggttgaacggcgcaaattactgatctgcctgtttgtggtgtttattgccagccacgtactgtcgtttttgtcgtggagctttaccgttctggtgatcagtcgcattggtgtggcttttgcacatgcgattttctggtcgattacggcgtctctggcgatccgtatggctccggccgggaagcgagcacaggcattgagtttaattgccaccggtacagcactggcgatggtcttaggtttacctctcgggcgcattgtgggccagtatttcggttggcgaatgaccttcttcgcgattggtattggggcgcttatcacccttttgtgcctgattaagttacttcccttactgcccagtgagcattccggttcactgaaaagcctcccgctattgttccgccgcccggcattgatgagcatttatttgttaactgtggtggttgtcaccgcccattacacggcatacagctatatcgagccttttgtacaaaacattgcgggattcagcgccaactttgccacggcattactgttattactcggtggtgcgggcattattggcagcgtgattttcggtaaactgggtaatcagtatgcgtctgcgttggtgagtacggcgattgcgctgttgctggtgtgcctggcattgctgttacctgcggcgaacagtgaaatacacctcggggtgctgagtattttctgggggatcgcgatgatgatcatcgggcttggtatgcaggttaaagtgctggcgctggcaccagatgctaccgacgtcgcgatggcgctattctccggcatatttaatattggaatcggggcgggtgcgttggtaggtaatcaggtgagtttgcactggtcaatgtcgatgattggttatgtgggcgcggtgcctgcttttgccgcgttaatttggtcaatcattatatttcgccgctggccagtgacactcgaagaacagacgcaatagttgaaaggcccattcgggccttttttaatggtacgttttaatgatttccaggatgccgttaataataaactgcacacccatacataccagcaggaatcccatcagacgggagatcgcttcaatgccacccttgcccaccagccgcataattgcgccggagctgcgtaggcttccccacaaaataaccgccaccaggaaaaagatcagcggcggcgcaaccatcagtacccaatcagcgaaggttgaactctgacgcactgtggacgccgagctaataatcatcgctatggttcccggaccggcagtacttggcattgccagcggcacaaaggcaatattggcactgggttcatcttccagctcttccgacttgcttttcgcctccggtgaatcaatcgctttctgttgcggaaagagcatccgaaaaccgataaacgcgacgattaagccgcctgcaattcgcagaccgggaatcgaaatgccaaatgtatccatcaccagttgcccggcgtaatacgccaccatcatgatggcaaatacgtacaccgaggccatcaacgactgacgattacgttcggcactgttcatgttgcctgccaggccaagaaataacgcgacagttgttaatgggttagctaacggcagcaacaccaccagccccaggccaattgctttaaacaaatctaacattggtggttgttatcctgtgtatctgggttatcagcgaaaagtataaggggtaaacaaggataaagtgtcactctttagctagccttgcatcgcattgaacaaaacttgaaccgatttagcaaaacgtggcatcggtcaattcattcatttgacttatacttgcctgggcaatattatcccctgcaactaattacttgccagggcaactaatgtgaaaagtaccagcgatctgttcaatgaaattattccattgggtcgcttaatccatatggttaatcagaagaaagatcgcctgcttaacgagtatctgtctccgctggatattaccgcggcacagtttaaggtgctctgctctatccgctgcgcggcgtgtattactccggttgaactgaaaaaggtattgtcggtcgacctgggagcactgacccgtatgctggatcgcctggtctgtaaaggctgggtggaaaggttgccgaacccgaatgacaagcgcggcgtactggtaaaacttaccaccggcggcgcggcaatatgtgaacaatgccatcaattagttggccaggacctgcaccaagaattaacaaaaaacctgacggcggacgaagtggcaacacttgagtatttgcttaagaaagtcctgccgtaaacaaaaaagaggtatgacgatgtccagacgcaatactgacgctattaccattcatagcattttggactggatcgaggacaacctggaatcgccactgtcactggagaaagtgtcagagcgttcgggttactccaaatggcacctgcaacggatgtttaaaaaagaaaccggtcattcattaggccaatacatccgcagccgtaagatgacggaaatcgcgcaaaagctgaaggaaagtaacgagccgatactctatctggcagaacgatatggcttcgagtcgcaacaaactctgacccgaaccttcaaaaattactttgatgttccgccgcataaataccggatgaccaatatgcagggcgaatcgcgctttttacatccattaaatcattacaacagctagttgaaaacgtgacaacgtcactgaggcaatcatgaaaccactttcatccgcaatagcagctgcgcttattctcttttccgcgcagggcgttgcggaacaaaccacgcagccagttgttacttcttgtgccaatgtcgtggttgttcccccatcgcaggaacacccaccgtttgatttaaatcacatgggtactggcagtgataagtcggatgcgctcggcgtgccctattataatcaacacgctatgtagtttgttctggccccgacatctcggggcttattaacttcccacctttaccgctttacgccaccgcaagccaaatacattgatatacagcccggtcataatgagcaccgcacctaaaaattgcagacccgttaagcgttcatccaacaatagtgccgcacttgccagtcctactacgggcaccagtaacgataacggtgcaacccgccaggtttcatagcgtcccagtaacgtcccccagatcccataaccaacaattgtcgccacaaacgccagatacatcagagacaagatggtggtcatatcgatagtaaccagactgtgaatcatggttgcggaaccatcgagaatcagcgaggcaacaaagaagggaatgattgggattaaagcgctccagattaccagcgacatcaccgccggacgcgttgagtgcgacatgatctttttattgaagatgttgccacacgcccaactaaatgctgccgccagggtcaacataaagccgagcatcgccacatgctgaccgttcagactatcttcgattaacaccagtacgccaaaaatcgctaaggcgatccccgccaattgtttgccatgcagtcgctccccgaaagtaaacgcgccaagcatgatagtaaaaaacgcctgtgcctgtaacaccagcgaagccagtccagcaggcataccgaagttaatggcacaaaaaagaaaagcaaactgcgcaaaactgatggttaatccataccccagcagcaaattcagtggtactttcggtcgtgcgacaaaaaagatagccggaaaagcgaccagcataaagcgcaaaccggccagcatcagcggtggcatgttatgaagccccactttgatgaccacaaaatttagcccccatacgaccactaccagtagcgccaacaccccatcttttcgcgacattctaccgcctctgaatttcatcttttgtaagcaatcaacttagctgaatttacttttctttaacagttgattcgttagtcgccggttacgacggcattaatgcgcaaataagtcgctatacttcggatttttgccatgctatttctttacatctctaaaacaaaacataacgaaacgcactgccggacagacaaatgaacttatccctacgacgctctaccagcgcccttcttgcctcgtcgttgttattaaccatcggacgcggcgctacgctgccatttatgaccatttacttgagtcgccagtacagcctgagtgtcgatctaatcggttatgcgatgacaattgcgctcactattggcgtcgtttttagcctcggttttggtatcctggcggataagttcgacaagaaacgctatatgttactggcaattaccgccttcgccagcggttttattgccattactttagtgaataacgtgacgctggttgtgctcttttttgccctcattaactgcgcctattctgtttttgctaccgtgctgaaagcctggtttgccgacaatctttcgtccaccagcaaaacgaaaatcttctcaatcaactacaccatgctaaacattggctggaccatcggtccgccgctcggcacgctgttggtaatgcagagcatcaatctgcccttctggctggcagctatctgttccgcgtttcccatgcttttcattcaaatttgggtaaagcgcagcgagaaaatcatcgccacggaaacaggcagtgtctggtcgccgaaagttttattacaagataaagcactgttgtggtttacctgctctggttttctggcttcttttgtaagcggcgcatttgcttcatgcatttcacaatatgtgatggtgattgctgatggggattttgccgaaaaggtggtcgcggttgttcttccggtgaatgctgccatggtggttacgttgcaatattccgtgggccgccgacttaacccggctaacatccgcgcgctgatgacagcaggcaccctctgtttcgtcatcggtctggtcggttttattttttccggcaacagcctgctattgtggggtatgtcagctgcggtatttactgtcggtgaaatcatttatgcgccgggcgagtatatgttgattgaccatattgcgccgccagaaatgaaagccagctatttttccgcccagtctttaggctggcttggtgccgcgattaacccattagtgagtggcgtagtgctaaccagcctgccgccttcctcgctgtttgtcatcttagcgttggtgatcattgctgcgtgggtgctgatgttaaaagggattcgagcaagaccgtgggggcagcccgcgctttgttgatttaagtcgaacacaataaagatttaattcagccttcgtttaggttacctctgctaatatctttctcattgagatgaaaattaaggtaagcgaggaaacacaccacaccataaacggaggcaaataatgctgggtaatatgaatgtttttatggccgtactgggaataattttattttctggttttctggccgcgtatttcagccacaaatgggatgactaatgaacggagataatccctcacctaaccggccccttgttacagttgtgtacaaggggcctgatttttatgacggcgaaaaaaaaccgccagtaaaccggcggtgaatgcttgcatggatagatttgtgttttgcttttacgctaacaggcattttcctgcactgataacgaatcgttgacacagtagcatcagttttctcaatgaatgttaaacggagcttaaactcggttaatcacattttgttcgtcaataaacatgcagcgatttcttccggtttgcttaccctcatacattgcccggtccgctcttccaatgaccacatccagaggctcttcaggaaatgcgcgactcacacctgctgtcacggtaatgttgatatgcccttcagaatgtgtgatggcatggttatcgactaactggcaaattctgacacctgcacgacatgcttcttcatcattagccgctttgacaataatgataaattcttcgcccccgtagcgataaaccgtttcgtaatcacgcgtccaactggctaagtaagttgccagggtgcgtaatactacatcgccgattaaatgcccgtaggtatcattaaccaatttaaatcggtcaatatccaacaacattaaataaagattcagaggctcagcgttgcgtaactgatgatcaaaggattcatcaagaacccgacgacccggcaatcccgtcaaaacatccatattgctacggatcgtcagcaaataaattttgtaatcggttaatgccgcagtaaaagaaagcaacccctcctgaaaggcgtcgaaatgcgcgtcctgccagtgattttcaacaatagccagcattaattcccgaccacagttatgcatatgttgatgggcagaatccattagccgaacgtaaggtaattcatcgttatcgagtggccccagatgatcaatccaccgaccaaactggcacagtccataagaatggttatccgttatttctggcttactggcatctctcgcgaccacgctgtgaaacatactcaccagccactggtagtgggcatcgatagccttattgagatttaacaagatggcatcaatttccgttgtcttcttgatcattgccactcctttttcacagttccttgtgcgcgctattctaacgagagaaaagcaaaattacgtcaatattttcatagaaatccgaagttatgagtcatctctgagataacattgtgatttaaaacaaaatcagcggataaaaaagtgtttaattctgtaaattacctctgcattatcgtaaataaaaggatgacaaatagcataacccaataccctaatggcccagtagttcaggccatcaggctaatttatttttatttctgcaaatgagtgacccgaacgacggccggcgcgcttttcttatccagactgccactaatgttgatcatctggtccggctgaacttctcgtccatcaaagacggccgcaggaataacgacattaatttcaccgctcttatcgcgaaaaacgtaacggtcctctcctttgtgagaaatcaaattaccgcgtagtgaaaccgaagcgccatcgtgcatggtttttgcgaaatcaacggtcattttttttgcatcatcggttccgcgatagccatcttctattgcatgaggcggcggtggcgctgcatcctgttttaaaccgccctggtcatctgccaacgcataaggcatgacaagaaaacttgctaatacaatggcctgaaatttcatactaactccttaattgcgtttggtttgacttattaagtctggttgctatttttataattgccaaataagaatattgccaattgttataaggcatttaaaatcagccaactagctgtcaaatatacagagaatttaactcactaaagttaagaagattgaaaagtcttaaacatattttcagaataatcggatttatatgtttgaaaattattatattggacgagcatacagaaaaagcaaatcacctttacatataaaagcgtggacaaaaaacagtgaacattaatagagataaaattgtacaacttgtagataccgatactattgaaaacctgacatccgcgttgagtcaaagacttatcgcggatcaattacgcttaactaccgccgaatcatgcaccggcggtaagttggctagcgccctgtgtgcagctgaagatacacccaaattttacggtgcaggctttgttactttcaccgatcaggcaaagatgaaaatcctcagcgtaagccagcaatctcttgaacgatattctgcggtgagtgagaaagtggcagcagaaatggcaaccggtgccatagagcgtgcggatgctgatgtcagtattgccattaccggctacggcggaccggagggcggtgaagatggtacgccagcgggtaccgtctggtttgcgtggcatattaaaggccagaactacactgcggttatgcattttgctggcgactgcgaaacggtattagctttagcggtgaggtttgccctcgcccagctgctgcaattactgctataaccaggctggcctggcgatatctcaggccagccattggtggtgtttatatgttcaagccacgatgttgcagcatcggcataatcttaggtgccttaccgcgccattgtcgatacaggcgttccagatcttcgctgttacctctggaaaggatcgcctcgcgaaaacgcagcccattttcacgcgttaatccgccctgctcaacaaaccactgataaccatcatcggccaacatttgcgtccacagataagcgtaataacctgcagcatatccgccaccaaaaatatgggcgaaataactgctgcgatagcgtggcggtatagcaggaagatccatattttccgccaccagcgcccgcaattcaaaatcatcgacatcctgcattgcttcgttttcttccaggcaatgccagcgcatatcgagaagtgcggcgctaagcagttcgctcatctcataccctttgttgaacaggctggcattacgcattttctgttgcagttcgtcaggcattgctgccccgctctgataatgccgggcgtagcgagcgaatacctgcggatgcgttgcccagtgttcgttgatttgcgacggaaattcgacaaaatcacgcggcgtgttggtgccggaaagcgtggcataacgctggcgggcaaaaaggccgtgcagcgtatgaccaaattcatggaataaggttatgacatcatcccagagtaacaacgcaggctcaccggcagcgggtttctgataattgcagacgttataaattaccggatgtgttttattaagcgttgattgctcaacaaaattgcccatccatgcaccgccgctttttgaatcacgggcgaagaaatcaccgtaaaataacgccagccccacgccattatgatcaaaaatttcccacacacgaacgtcaggatggtagacaggaatatcaaaacgttcgacaaacttaataccgaagagctgattcgcggtccagaatacaccttcatttaacaccgtgtttaattcaaaatatggcttgagctgcgcctcatcaagatcaaatttctcccgccgtacctgttccgcataaaatgcccagtcccacggctgcgcgctaaacccgccctgctgcttatcgataaccgcctgtatggaggctaattcatcgctcgcacgttgacgcgccgctggaacaatttcccgcataaagttaagtgctgcttcaggtgtttttgccatctgatcggcgattttccatgcggcataatgaggaaaaccaagtagtgttgcctgttgtgcacggatctccaccagacgttgaatgatagcgcgggtatcattggcatcatttttttccgctcgcgtccagcccgcaataaacagtttttcacgcgtcgcacgatcgcgcatttcggcaagcgccggttgttgggtggtattcagcagcggaatcagccatttgttatccagacctttctcgcgagccgcctctgccgccagcgcaatctcttgctcactcattcctgccagctgcgcgatatcgttcacaaccagaccgccggatttatttgctgccagtaatcgctggttaaactggctggtcagggtcgcagcttctgtattcagtacttttaattttgctttatcagcttgcgcaagtttggctccggcaaggacaaaacgttgatgaatcacctccaccaggcggatggattcactatcaagccccagggattcacggcgctgccagacagcatctacccgcgcgaataattcaccgttcagatagatatcattagccagttccgccagttcagcggaaaactgctcgtcaagacgctgtaattcatcattggtatgcgccgcagtcatcgcaaaaaagacgctggtaacgcgggtaagtaattctccgctttgttccagtgccagaatagtattgttgaaatcaggcatttgcgggttaagcgcgatggcagcaatttctgcccgcttttgctgcattccctcatcgaatgccgggcgatagtgatgattggcaatttgatcaaaatggggagccagatacggcagtgtgctttgcacaaggaaaggattcattgttgtcattttcttctcctgaacgcgaggtgttccatagcgtaggcttactgataacggagtgcaatcttgcaatccagtattacccgctcttaagcatcccgtgctatgttattgacacacaaaagcgttgaggaacagtgagatgatcgttttagtaactggagcaacggcaggttttggtgaatgcattactcgtcgttttattcaacaagggcataaagttatcgccactggccgtcgccaggaacggttgcaggagttaaaagacgaactgggagataatctgtatatcgcccaactggacgttcgcaaccgcgccgctattgaagagatgctggcatcgcttcctgccgagtggtgcaatattgatatcctggtaaataatgccggcctggcgttgggcatggagcctgcgcataaagccagcgttgaagactgggaaacgatgattgataccaacaacaaaggcctggtatatatgacgcgcgccgtcttaccgggtatggttgaacgtaatcatggtcatattattaacattggctcaacggcaggtagctggccgtatgccggtggtaacgtttacggtgcgacgaaagcgtttgttcgtcagtttagcctgaatctgcgtacggatctgcatggtacggcggtgcgcgtcaccgacatcgaaccgggtctggtgggtggtaccgagttttccaatgtccgctttaaaggcgatgacggtaaagcagaaaaaacctatcaaaataccgttgcattgacgccagaagatgtcagcgaagccgtctggtgggtgtcaacgctgcctgctcacgtcaatatcaataccctggaaatgatgccggttacccaaagctatgccggactgaatgtccaccgtcagtaatttttatacccggcgtaactgccgggttattgcttgtcacaaaaaagtggtagactcatgcagttaactcactcacaagcaagaacgaatgaccgtcgaaacgcaacttaatcccacacagcctgtcaatcagcagatttatcgtattcttcgtcgcgacattgtccattgcctgattgctccaggcacaccgttgtcggaaaaagaagtttctgttcgtttcaatgtgtcacgccagccggttcgtgaagcctttattaaactggcggaaaacggcctgattcaaattcgtccgcaacgtggcagctacgtcaacaaaatttccatggcccaggtgcgcaacggcagttttatccgtcaggccattgagtgcgcggtggcgcgtcgggcggcgagcatgattaccgaaagccagtgctatcaactggaacaaaatcttcaccagcaacgcattgccattgagcgcaagcaactggatgatttttttgaacttgatgacaacttccatcaactcctgacgcagattgccgactgtcaactggcgtgggataccattgagaacctgaaagcgaccgttgatcgcgtgcgctatatgagtttcgaccacgtttctccaccagaaatgctgttacgccagcatcttgatattttctctgccctgcaaaaacgtgatggcgatgcggtagaacgtgcaatgacgcaacatttgcaggaaatcagcgaatccgtgcgccagatccgccaggaaaacagcgactggtttagcgaagagtaattcatttcctctcatcccatccggggtgagagtcttttcccccgccttatggctcatgcatgcatcaaaaaagatgtgagcttgatcaaaaacaaaaaatatttcactcgacaggagtatttatattgcgcccgttacgtgggcttcgactgtaaatcagaaaggagaaaacacctatgacgacctacgatcgtaaccgtaacgcaatcaccactggcagccgtgttatggttagcggcaccggtcacactggcaagatcctgtcgattgatactgaaggtctgaccgctgagcaaatccgccgcggaaaaaccgtagttgttgaaggttgtgaagagaaactggcaccactggacctgattcgtctcggcatgaactaagcgtgtgaatgccgccgatggcggcattgcttttttacttcacggaatattttgccacggtcgctttcgcgccatgcgctaataaagacaagtacgtttccgtcactcttgcagtaaacaaactattgtctggcaaatcatcaccaaagatcgccttaatcgccagcaatgactggacgcgcgctttcccttcggcactactttgtacagccttctgaataacaggtaacagtgggtcactgatttctatcggatttccctgttcatcaacaccaccgacataacgcatccaacccgcgacgcccagcgccagcagatcgaacttgctgtcatgcgccagatgccagcgaacagaatccaacatccgctgtggcaatttctggctaccatccatcgcaatctgccaggttcgatgacgtaacgccgggttgctatagcgtgcaattaatcggttagcgtaatcttgcaaatcaacgccctgcactttcaacgtcggcgcttgttcctgcaacatcaagccatacgccgcataacgataatgttcatcttccatacagtcattaatgtgctgatatcctgcaagataccccagatacgccaggaatgaatgactgccgttgagcatgcgcaacttcatctcttcataaggcagcacatcgctaaccagttcggctcccgctttttcccattccggacgtccggcaacaaagttatcttctattacccactggcggaaaggttcacaggcaacgcccgcaggatcgcgcacaccggtaagttgttcgattttcgccagcgtatcctctgtcactgcgggcacaatacggtccaccattgttgatgggaaagtcacgttatcttcgatccattgtgccagttttacatcaacggcttgtgcgtaggaagtgacaacgtcacgcataacatgaccgttttctggcatgttgtcacatgacatgacggtaaatgcgggaagtcctgccgctttacggcgagccagcgcctcaacaatcacccctgttgctgttttcggctggtggggattttgcacgtcggcagctaccatcgggtgatcgagcattaactgtccggtcgccggagagtggaaataccctttttcggtgattgtcagagagacaatcgcgatttgcggttcacacatcgctgccaacacggtttctaagccatctatctgtacgtgcaaggcttttttaacgacgccaacgacgcgagccgtccacacatcggccgacatttccgcaacggtataaagattatcttgctgttgtaaatcggcaatttgctgttcgccgccgattaagttgacctcataatatccccagtcactgaaatgttccgtagcaagaatatcggcatacacaccctgatgcgcacggtgaaatgcaccaaagcctaaatgaacaattcttggagccaggttattaagatcataaacagggagtgtcgcttttgctgataacaaattatttcccataacaattccttaaatataaatatggcaagctatatgttttgttatatgaataaaaatcccctctccggtaagagaagggattaagggtttacagacttctggaaggttgcgcagctcttacaacacgcggttgatcttccgcagcgtcttccagcgcacttaaatcacggtctttcacctctggcattttcagcgcagagattaaaccaatcactgaatatgccatgatcataatggcgatcggataccaggattccgtcatggtgcagaaaatacccgccaggataggaccaaaaccggaagcgataagaccaccaatttctttagaaatagccatccgggtaaagcggtttttacagccgaacatttctgccatggtaatgttttccagagcaaataatcccagcaccgcacagttatgaatcacaatcagtgcaaccataatggtgctcggggcatagcttttatctacaatgatagaaagcattggccatgccagcacaatcgcggaggtattcataataatatacgggatccggcgaccaattttatcggataaccaaccaaggaacggaatggtcataaagccgagaatcgaactgatcatcaatgcatctgttggaattgctttgttaaacaataacgtctgcactaaatagcctgcaaggaaagtctgaattaacccggagttacccgcctgaccaaaacgcagccctgttgccagccagaaggatttgctctggaacatgctaccagcaggtgcaggttttgctgtcggttggttactgtcgttaaccttctcaaagaccgggctttctttcagattcatacgcaaccagatagcaaagaccatcacgacaacactcgccaggaacggtatacgccatccccacgccagcagttcctctttactgagaatgaagaacataaaggcccagattgccgttgcgctcaaggttccgcagttagttcccatagccacaaatgaggagataattccgcgcttaccttttggcgcatattccgccagcatcgtaccggcaccggaaatttccgcacctgcacccaacccctgaataatacgcaacgtcaccagcaagatgggtgcaaaaacaccaatctgtgcataggtcggtaacacaccaattaaggtggtacagatccccatcatggtgatggtaataaagagcacttttttacgccctattctgtcgcccattttgccgaaaataaatgctccgacaatacgcgccacataacctgcaccgtaggttcccattgccagaattaacgccattgccgttgatgattcaggaaaaaatatttcatgaaacactaacgctgcgccgagcgaatataactggaaatccataattcacaggtgttttttcccatcctgtggtttccttggcgttttctaggttttttcagatagttgcatttttttaaaaagcatcctaagttcgatctcagtgtctatctggggcctatttctgtcccatatatgccccaaaaaaactccccaacagataagtagttttttcatggatttatgcgtaaaatcaagaacggctggaaatcattcaatactcacactatcgaaaaatttaccagccaatcgcagcacgttcttgcataaggtgtgtctgcggtttttcaactattcagatacatcactcccatcacattcattcctccgcatcaaaggcatataggctatatcaccttgatatttttctttttcagataaaaactgttatctatgtatacttttaaacccaatccgtgtagagtctctacataagatagtttgcagttgccgcttcagcttgcgccataaaccgcctgatttttgctgccacctgttagcattcctgtatacctgaaacgacaatgtttatctacgaactttaagaacacccaagataaaaattgtcaactatatcatatataacacattactaattcgaggctatatgaacagcatactgataatcacatctctccttatcatattcagcatttttagtcatgccctaataaaattagggattggcatatccaataacccagacaaaaccgatgtataagtcaacatatcctgaatcagacatacaatatcgcaatgaaaatcaataatattttaaggaatatcttcatgaaatcaaaagacaccctaaagtggttccctgcgcagcttcctgaagtaagaattatcctaggggatgctgtagtggaagtagcaaaacagggaagacctatcaataccagaacattgcttgattacattgaaggaaacataaagaaaaaatcatggctggataacaaagaattattacaaacagcgatatcagttcttaaagacaaccaaaatttaaatggtaaaatgtaatataataaacttacttttttatcatttttccactttaacaacattttgctccacttttccacgaccaaacaacttgaaatctggttaaaataacacgcaacactattcttcttccttgagtccgcccggaactcgaaaaacaaaccgagttaaagccatttttcacaaaatcgattttgggtctcaccaaaattacggggttgcatacgcattcgtttattttcgaacgtgtacatacaaatatgcacaaaaataatcataattattttctgagatgcattatgatatgaacaccaatttcgtatagagtctcactatgtctcaaatttttgcttactgtcggatatcaacgctggatcagaccaccgaaaatcaacgccgggaaatcgaaagtgcaggttttaaaatcaaacctcagcaaataatcgaagaacacattagcggctcagcagcaaccagtgagcgtcctggttttaaccggttgcttgctcgcctgaaatgtggtgatcaattgattgtgacaaaactggatcgccttggttgtaatgcaatggatatcaggaaaacagtggaacaactgaccgaaacaggtatcagagtgcattgcttagcattggggggcattgacctgaccagtccaacaggaaaaatgatgatgcaagtaatttcagcagtcgctgaatttgaacgagaccttttacttgaacgcactcattccgggatagtaagagcccgcggcgcagggaaacgttttggtcgaccacctgtgttaaatgaagaacagaaacaggcggtattcgaacgaattaagtcaggtgtaagtataagtgccattgcccgggaattcaaaacctcgcggcaaaccattttaagagccaaagcaaaacttcagacacctgacatataaaaaataatctcggtgtgagatgctttacgtcttccaagcccccttccttgccgtaaatggaaagatacatctaattatagaatttatatgttttaccctacggcagtgctggccattcaatatcctgtgcagttgacgtatcaacacggttcagcaatacccgatactttttccatgcttccagcaacgagatttcttcctccgttgcaatttccagatctgcagcatcctgaagcggcgcaatatgctcactggctacctgcatcaggttgttttttgtttcttccgcctcccggatccggaacagtttttctgcttccgtatccttcacccaggctgtgccgttccacttctgaaactccccttccggcgataaccaggtaacattttccggtaacggaccgagttcagaaataaataacgcgtcgccggaagccacgtcataaaccgttttaccccgatgatcttcaacgagatgccacgatgactcatcactgttgaaaacagccacgaagccagccggaatatctggcggtgcaatatcggtactgtttgctggcagacctgtatgaggcggaatatatgcatcaccttcaccaataaattcattagttccggccagcagattataaatttttatggtccgtggttgttcactcattctgaatgccattatgcaagcctcacaatatagttaaatgcgatgtttttgacggtgttttccgcgttaccagcagcgttaacggtgatggtgtgtccatgtgaaccaatcgcaacggagtgcgtatgagcaccaataccgacagtatgtgcatgcgcgcctgcgcttgcagcagtgccggacagcgagtgggtatgagcaccatctgatgatgtcttccctgcattacgagtctggccactaccgcttgttgtgctcataatccccgcgcttagatttgaaatcgcggtataaccattagggaaaatgctcgtgttcgtgccaccaaatgcaccggaactcttgtgttggtgcgcaccggcactatttgcggtcccgctaatactatgggtatgcgccccggtgttattcgtggatttggttccgtaatcaaacgacgatgtggtttccgtccccaaatccgtactggatgcgctggcgctgtgggtgtgcgatttaatgccgtcctgttcctgagataatacggcccgaccactggcgggcttgcccttaatcgtccagccacgcatatcagggatcacgcctgacggataagcaactgcaagtttcgggtatgcagatttgtcaaaagtctgcccctgcatcagggcataaccagacggaacggtatctgatggccacgggattggtgcaccgactggataaaactctgcaggaggatgagccgaggtgtaaagctgcgcccacggcgaccagtttgcgtcggtcgtatcccgtcgtgaacgaataaatgccggagcatgagcaccgcttgtaccactccagccgatgagtaactcaccttcgccaacggctgtcatccctttcaggtgaatgatatttccatacgctgttggatatccgttgttatacacctcgtataactcaagacctgctgccccctgcgtattgtctgtcagcgcggttatattcactcagcaaccccggtatcagttcatccagcgcggctgctttgttcatggctttgatgatatcccgtttcaggaaatcaacatgtcggttttccagttccggaaaacgccgctgcaccgacagggggatcccgtcgagaatactggcaatttcacctgcgatccgcgacagcacgaaagtacagaatgcggtttccaccacttcagcggagtctctggcatttttcagctcctgtgcgtcggcctgcgcacgcgtaagtcgatggcgttcgtactcaatagtccctggctggagatctgtctcgctggcctgccgcagttcttcaacttcccggcgcagcttttcgttctcaatttcagcatccctttcggcataccatcttataacggcggcagagtcataaagcacctcattacccttgccaccgcctcgcagaacgggcattccctgttcctgccagttctgaatggtacggatactcgcaccgaaaatgtcagccagctgctttttgttgacttccattgttcattccacggccaaaaacagagaaaggaaacgacagaggcccaaaagctcgttttcagcacctgtcgtttcctttcttttcagggggtattttaaataaaaacattaagttacgacgaagaagaacggaaatgccttaaaccggaaaattttcataaatagcgaaaacccgcgaggtcgccgccccgtaacctgtcggatcaccggaaaggacccgtaaagtgataatgattatcatctacatatcacaacgtgcgtggaggccatcaaaccacgtcaaataatcaattatgacgcaggtatcgtattaattgatctgcatcaacttaacgtaaaaacaacttcagacaatacaaatcagcgacactgaatacggggcaacctcatgtcaacgaagaacagaacccgcagaacaacaacccgcaacatccgctttcctaaccaaatgattgaacaaattaacatcgctcttgagcaaaaagggtccgggaatttctcagcctgggtcattgaagcctgccgccggagactgtgctcagaaaaaagagtttcttctgaagcaaacaaagaaaagagtgacattactgaattgctcagaaaacaggtcagaccagattgaagcaatttagataatcgtgcagactacgccccctcatatcacatggaaggtttatctatggatcaggtagtcatttttaaacaaatatttgataaagttcgaaacgatttaaactatcaatggttttattctgagctaaaacgtcacaatgtctcacattacatttactatttagccacagagaatgttcatattgtattaaaaaatgataatacagtgttattaaagggcctaaaaaacattgtgtctgtcaaattttcaaaggataggcatcttatagaaacgacctctaataagctgaaatccagagagatcacatttcaggaatacagaagaaaccttgctaaagcaggagtttttcggtgggttacaaatatccacgaacaaaaaagatattactatacctttgataattcattactatttactgaaagcatccagaaaactacacagatcttaccacgctaaaccataacgtccggcttctctcactcctgagccggactgcattggtttaataaaaaccatcaacaattgtgatttagatattcggaaccattcaaatataacaaaaccccgtaaaaacgaggtttatggataaattttattattgaatacatcagattaaattaatcttgacatcatagctttcaagacccgtcattttttcccgtgcggtaaactgaatactggtaacttctttcccggtctttttcttaagttcaataattttttttgttatatattcagaaatatctgcttctgcttttgtttttaagttttcaatattcatcatttcctcttttagtctgttatgactttccagttacacagtaagtcgattatatggtgcaaacgtgtaaaagataagatgaaacatcgcaataatcaacatacgatagtctaaattttacacaaacagacaaagagaattttcctgaattatcaatgcaatagcatcaaatcaactcaagagccttattgctgcttccagaatttcttctgaagtaacatgtcgatccgcggctacataaatgactttatgatctccggtcagagatggaaaccctgcggccattacagtaaggtgtgttttttcgccatttggatattcacgcatgatggtgttaactccagtcatcgctggcactaccactgctggttcagagttaaaaaaactatgatttttttcatgatgttaccgtagtatgtgagtatccatcgaatagacaccaagcaaaaaagctcccgaaggagccttcattttcacttttttaaatccaacgacagacggctggcatttaagtattgtgaaatattatcaaatgtaatcatcattgatttacaaaagatacattttgccccgaaaggattcatgtcagaaacatcaaaagatgatgttctatactgggaaccatgacaacacgggcatctaaagtgaatatggtttgtaatattgtctacctcaaagcgccactacatgaacagcggcaggacctttaggtccgttctcaataccaaattcaacttcctgattctcagttaatgttttgaaatcgttgctctgaattgctgagaaatggacaaacacatctttgctgccatctttcggcgtgatgaaaccaaaacctttttcagggttaaaccatttcactaaaccagtcattttgttagacataattattaccttttgaagaaattagcccttgggcagaatggtccgaaaaaaaatatcagagagaaaaaccaacaaggaaatctcaagaggtacaaataataaaattataacaatgactgcttcagataaatttgtaacaaaccagaacaccattaacgcatgattaaccacccatagcaaggattacttttgtaaagaaaaacacagcaatgaaagaatagctttatttattaataaaacgtgtcattctgattaagaccttttatcttacccttaagatttcaggaattttggctcatggaagagtcctttttatttaaattttacattccgcgatgtaaatgttccgatttaatattaccctacatttgatgctttttatctcttaaagattcatagatctgttgacaagtcactcctgcgatgtagcgttcgtcagcaatttcagcataaagctgagcttctgctgcaatatctccgagcatgttggtgagcattccttcggcggttttggttgttttgcctctgacggcagcggcaagatctgcggtatgcttcgctgcgtcaaggcgtatggcatatttttttgcttcggcacgcaactggttaacactatcagacagataagcagccctggcagaaatttcagcagatttctgttgcgcatctttaacagcctcatcacgggctatagttcgcccctgttcaattattcgagcagcaaattgagcatttacctcttgtgataatgcggcagcatcacgttccgcccattttttttgccatcctcggtcgctccagacatttccgacgataaatcctgacaacacgagaaaaatcaccatgaatatctgattcactgttctatcccccagcaggttaatgcgctctcctggtcacgacgaataacctgaccgtaacagttatttgaacgaatgcggcaatcgcgtccgccatccttaatccaccagcgaatcgcttcgcatgcacctttacgatcaccagcattcagccgcttataaaacgtcgacgggaaacacttaccggggccaatgttatagggacaaaatgacgcgatacccgctttttgtggttcggtcagtggtactttaatattgcgctccacccatgccagcgccttatcacgctcaatggcgttgacctggtcgcatttttccttcgacagtttcatattgggaaaaacggtttttccatccaccactgtggcaccccgacagatggtccatatgccagaaccatcgcggtatgccattgtgtggttaccttctttttcgtccagaaactggtcaagtatctgaggagcagatgcgccagcaccaatcagcgccagaacggcagccgacaggccgtatctgatttttgtgttcatagatatttatgatgaggacgctcgtgcttattggcaggattttcaatcttaaaggagtactgatgctgcagataagactcaactttttctgacaatttttctgctacttccaggaagacttgccggacgctccttctggctgctgcctcataaaactccagcgcagctccttcaacacggtccatggcgacatccaggtcaaaaatttcaccgtcaaagcgttctttgtcctgtaaggctacagttaccgtaactttattctcaaaattacggactcctttcacaaccagttcatagtcttgagtcattggattactctcctctcgcagccttacgcctgtcttctttaatcttgaaataaagatttgtcagatacgtcagcaggccaaaaaccaggctacccagcacaccgattgcagcccactgtgacggagttactttatcgagtaactgcaatgcccagaaaccagcattacccgccgatgtgccataggcaacacctgttgttaacttatccattgatttcatatcctcaccccgatgtacacggatggtgcaatatgtttgaaaagatcggagtctacggggtagttttgacagcacacgttgttctcaacggcgctaaaaaaacatacacattaaaaatgtgggtaattattttgaaagaaagtcatatataaaataataatacgagaaatgttttcatatttagtgtactgtatacggccatttatacaggaaaagcctatgtcagaacgtaaaaactcaaaatcacgccgtaattatctcgttaaatgttcctgcccaaactgcacccaagagtcagaacacagtttttcaagagtacaaaaaggtgcccttttgatctgccctcattgcaacaaagtattccagacaaatcttaaagctgtagcctgattgattttattagtaacaagtattttttatattttaataatatatttaaagcagataataaaaaacccgcctgagcgggtttgagattgtggtgctttttgtgggagtcatccacttacgcactttgttttgccatgccagcagttagcttctgctgtaaaactattcatgcagcaaacctgcacttcaccacaatggttagcatacttttcctgattaagattttgccaaatatgctagccattgtttcatgtattggacctccttactttttattaaagagatccaatattcactactctgtccgtatctctactcaggcatcagccttcttcgttatcgtatacagacgagcgatgaattttaatcagtaatgatgacatttgctgctgcaggacctttagcaccactctctatagagaaggtaaccttttgaccttcaaataaggttcgataattatcattctgaatcgcagaaaaatgcacaaacacatctttactaccatcaacaggagaaataaagccgaaacctttatcagcgttaaaccattttactaaaccagtcattttatttgacattctacattccttaacttgagcctttcggcataaatggtttgcataacagaaacgacttcgtacttaattggagagactcaaagaaggaataagtgaataacacctgaaatgagaactgctttagtaaactacttcgtatatcgtctgttcttcaaaccgacgcaatcattaacgcatagttgaacatatgaagcaatgtttattttagacatccagccatcttcaaccccatcaaaaaactatagctttcttcaggaacgtgtgtatagtgcgccaagttatcagtattaaggaatttttttgtcccgtaaaatgacaggaattgtcaaaacctttgacggcaaaagcggcaagggtcttatcaccccatccgatggtcgtatcgatgtccagcttcatgtttcagcgctcaatctccgcgatgcagaagaaattaccaccggattacgcgtggaattttgccggataaatggtctgcgtggcccttcagctgccaatgtttacctttcatgagctatattaaagctttaatttcaggccccatcggatcacacatggagagtttttatgaataaccccgtctgtcttgatgactggttgattggctttaaaagcttatgctgtactttggccgtaatagctctgctaataatataataagcagactcattgtgtttagggacattgtactggaagaaaacattttaaacatcaggcaaataaccaagtcaccagctaaataataagttaacagacatgagtcccgggatgagattcaacattaccattgccccatttaaagcacaaaacccgctcatcagcgggttttctactttttcttaacgtcgggtatacaaagcccatcgttgaaaaaattttatccatattttttgaaaaatgcaaacatcatgtcgccatcttcagcaaaaatcatttatctcgtcaccttcctcaattgcgcttccgcgtatgcttcttcctgccagcactttgttaccagtttaccaatgacgtccgcataccccttataccactgataatcggtcaggtctggtaccagcttctggacatgacgtcgtgccagcgtggtcggtaaacgactaaaccggtttccattacaacgcccacaaatcttatataccggtacgccatgaaaccgggttcttttttcatccagaacaatccctttacccttacaccctctgcacgctgtgctggcttcgcccttaccatggcaatgctgacatagttccttcacccattcttccttgattacagattccccgcgtctgtagtgtttcaccacttcgcgcaatacattataaaatcccgtacctgaacaatgctcacagcgagccttacttgccgcagacctggagtaatcagcaaaggcaaaactcacgaggtaaggaataatctgtaaccggatttcttcactcaatttgttcaatgtcgggttatccagtgccatcgcgtaatttagcaggccttcaatcgcaaactgagggtcctgaacaccaacttttgccagaaataaggccaacccaagtggtgctttcgactgcaccatcccctgcgctgccattacatccgtaattgttaaacaaccggtgcctgtcgctggagcgtcatcgctcaattttggagattttggggagtaatattttggtaaggcttcaaggttcatgctcgttctccacttacgccagtacgccaattgccagcgcgcgatcgataaaacgaaatatcagctccagttgggagccatacttatcttcaaatgccactgtatccgtatgcagctcgttgtgatgctttctgcacaaaggcaacacaaagagatcatgtgcttttgttcccattccgccctgcccgtgaccaatcagatgatgcggatcgtcggctggcataccgcagcaagcacacggctgtgtcttaacccaacgtgtgtatttctccttaacccagcggcgacgtttaggcagcttcatgaaagattccggagactctggatcaacggtgatgcttaccaccgtcttttcctgtggtgatttttgttgctggtgggcgtaaggcaacggtgcaagattttttgtgcgttgtttcaatatgctggtggcggtcagctctcccggtacgatgtcgctttcgcggtacaccgagcagattttttccgctggtaatcccagcgaacgacgcgatacagcctcaggtagtgcatccaccacctgattgcagaccgcccaccaggataattcagccaaagataattcccgctcctgcgtaccgcttattgcgtgacggatgacgtcaatcacccatgctgtcagattttgttgagcaagcagctccagtgattccgatgtctggtcacgcagttggttgtcgcagtgccagcacaacaccattgcgccggtaccataacggtgaatgactgtttcagtgtgatggtaatcgccattaggccactggcaggatgtaacatgacgtaatagccagtcggacaatgcgccaacgccgccagcagcacgaatcacccgttcgttactaaaaaacggcagcaatgttttgtcttccgccagcggctggcgaacggcaggaacgactccggatggcagattacgcatgctttttggttccggttccaccagcactcgaggattatgaaatatctgtatggattcacggcccggcttaaggaccaccagcccaagctcaggcaccagaacaggtctaagtaatacccgcacgttacctccagatccgttgctggaaagtgcgggacgcacgtggtgggcgttcggaataaggcagcctgacagagattatccagtgccgatagtcgagactgagagctttcttaacctcgaacccgcgcctgcggtaagaatgaatcagccattcggcctgttctgcagtgcatggagggtgctggaaccattcagacttgaatgcgtgagaataccgcccgtgcgtgcaggcaagaacgggcgaattatcagaattgtaatattttgcgttgcgtgccatcggttttctccggtggcacggtgttactcagcgggagttcagccccgcgcaagattgtagatgagtttattctcctgaaaaagcagaaaagccagcttttattccgatctctttcaatgcctgtaatgaagtgacaaactcaccttcgcgcaagataaatccgtccgtgacccgagcatccacaaaattaattaacgcagccccattctttcgcaaacacataatgcggtaatgactaacaagatttccattttcaacgcacacagcatagaggccatcttcacaaaaaattttacgcagttcttcgatgttcatcatcagaatccttccggataattagctctcccctttaagggaccatccctcttatccctgcgcgctacttaagtatttttgattctattccggcaccgtccagaacttcaaacgcgttgaaaataaaaacaaaaacccgccgaagcgggttaagtgcgggtgcgttgaggatgcctgccacatcagaggtggcgagggatttctcccccgccgggtctcttactcctcaggttcgtaagctgtgaagacagcgacctccgtctggccggttcggattcgtacctcgcagaggtctttcctcgttaccagtgccgtcactatgacggttaaacagatgacgatcagggcgattaacatcgccttttgctgcttcatagcctgcttctcctgtcaacgcaaagcagaagtgtcaccttcggtgcgaaacagagatgtcatgctttggttcagagaatgcgtttgaccgcctcgctatatacttccgagcgttctcttttcccaacagaaatcacgaaaacgacaactttctcgtctataacctggtatacaaggcgatagcctgaagaccggagcttaatcttgtaacaatcaggcataccacggagcttgtttgcttcaatccggggtgactcaagtacttcaaccagcttctttttcaactgttcacgtaccgtcgagcccagctttcgccattcctttagtgcccgctcgtcaaaatccagaaaatacgccatcagagttcatccagcgtcacacgtactggcttaggattacgaagccgttctttcactatctccacaagttcagcatcttcatcactcaggagtgtctgtttgaacggcaagcgttcattgtcagcgatatactcgagcatgagacgaagcgcttcagaaggagttacacccattttttcaagcgcggcgtaagaacgcgctttaagttcatcgtcaatacgcaggttaatgctacccatgtcttacacctcttgtaattacaaatgtcattacaagtatcgcactacaacatgcttagggcaagtcacgaaggaagtcagaaagtagtcgtaagaacggtgatcactgtccgctttgtgccaggagcagccattgctaagtccatcctgtattgtgcaggtcagctcgtttttaaagagtccggccatcatcttactggtacagacaccatatactttgtgacggtcaggctacatatgcacaactcaacttattcatctattttttgctttagcatgtcagtgttgctttctcgtcggcgggtgagcggtgacctgacctgtcgataaaggaacgtaacacgttttatgcaacacccgcatgcggcagaaaattattgccgaacgtttacccctgtcaacaagctttactttctgaggcgcgccagcccgcgaggaaaacaatctgaacatcaaacaattaatgacacaagaaatacgattaaagatttttttgtgcatgccgatagtgcttttttaaaaggagaaatctatgtctgtcacaattcagggaaatacctcaaccgttatttcaaacaactccgccccggaaggaacatcagaaatagccaaaatcacaagacaaattcaggtgctgactgaaaagcttgggaaaatctcatcggaagaggggatgacgacacagcagaaaaaagaaatggctgcattggtacagaagcaaattgaaagcctctgggctcaactggagcagttgttaaggcagcaggcagagaaaaagaatgaagacgcgacagttcagcctgataaaaaagaagagaaaaaagacgatacaaataccgctggcaccattgatatttacgtctaagtgacagccgtattgtggccctcatcgggccacttttcgccatcagccttttctttaaagacatattatctttgtatcatttctgatagttaacattacaagatataagtaatggacgcactcccaattagtctatttaaatcgccacgagtttaactgacaacccatgatcaattatgaattgcaactatttctgtagtcacttttgtggggacagtccacaaaactgccaacttccgcttcttgctcttagcggacattagcataggctatttaccataacgcctcattacgcgcaccgcccagactgactcagcgcgtttctggcatatccccggtaaaacaagtaacaaaccacccgaaaatgaacaccagaaacgcgacttaagaatctaccctatgaatggatatgcactcaaccgaatcgatcttggtttcaatcttttttatcgggatcaggcttctttttaggtaacttcgggggcttaacttgctgatgactttgcgttcggcgcgtaagccagggatggtcagctttaggtttaacatagtattttgagcgtaaatcaatacgggcattatccactcgttcatggacactcttttcatcatccagtggtagcctccataattgcaggcactagcgccgtgaacttttcacgcttatccctggtgtcgatagccttccagcgttcaaatatcttcactcgattaacgccaagcgctcgctgatcaatcgcgccaccttcatatgtgacacgctgaacatcgatgttcgggcgctctttcaaagcccagaatgcttcagtgattaatatcgtcgcctgctcctgtgtcattcctggtcgacatatccaggcatccagagcctcacgagcctgttcaggagtgattttcattgttcaaccgccccgcccgcttcgtcttacgatattcatcataaactttgggatcatactgaagctccccgccagatgcctcctgtagacgcatcgcgcgaccttcgggaactaaatcccctttccagctataaagcgaagccaaacgaatacctgctgcttgtgcaagttttgtttttgaaccgaaatacaaaagagcgtcagttttaagcatttaaaacacctttattgttagtcataactaacaagatagatgttaacaaaaacatagtcaatacgatttagcattagctaactatggaaacaaaaaatttaactatcggcgaacgcatcaggtatcgtcggaaaaacctcaaacacacccaaaggtctcttgctaaagccctgaaaatctcccatgtgtctgtatcacaatgggaacggggtgatagtgaacctacagggaagaacctttttgccctcagtaaagtattgcaatgctcaccaacatggattctatttggcgatgaagacaagcaaccaacaccacctgttgagaagccagttgccttatcccccaaagaactagagctccttgagctgtttaatgcactgccagaatcagaacaggatacccagctcgccgaaatgcgagctcgagtaaaaaacttcaataaactctttgaagaattactaaaagcccgtcagcggacaaataaaagataacatcatcaatgagttatcttttaccacatcaattatgttagctatagcatacaaaatcacttgaccgatatgttagtcatggctaatcttgtttgcatcaacacaccgcacggtgttctcagcaaacagttccgctaccccagcgttaaggggaaatgaggtcagcatggatactatcgatcttggcaacaacgaatctctggtgtacggcgtgtttccaaaccaggacggcacgttcaccgcaatgacgtataccaaaagcaaaacgtttaaaaccgaaaatggtgcccgtcgctggctggaaagaaactcaggtgagtgatatggatttcgacacaatcatggaaaaggcttacgaagaatacttcgaaggccttgccgaaggcgaagaagctctcagcttcagtgagtttaaacaggcgctttccagttcggcaaaatctaacggctgataagcgaaacagcaccgcgaggaatcagtatgcagaaacgagaacccgtcatcatcgcgccagactataccgatgatgaactttatgagtggatgcgccagaaaattaatgcagcgcaggatctgaaatgggctaatgaagccagggctaagcaggctgaaaatctgtccgctctggagcaggatatcaccaatctggaaaaagcagcggcattaagcattgccagaatgattacatacccgcgttagtagctaatcaacaaagctaaggttagtaattaaggagttctccacgggtgaggtggagtgcgtgcgccggacacgggtgcgcatccggaactgacagtttactgaaaggatatttccctgaaaagtcagaccataacgcgaaagcgcatggcgaggtagctggttcatagatagcctgtcgttaaattttcgtcgaccgtgcgcttccggttgtggcaacccgcgaaatggcgcggcggtaagtatggcggggttattccttccccgttgaggacaccgggttgtcaggttgaccatacgcttaagtgacaaccccgctgcaacgccctctgttatcaattttctggtgacgtttggcggtatcagttttactccgtgactgctctgccgccctttttaaagtgaattttgtgatgtggtgaatgcggctgagcgcacgcggaacagttaaaaccaaaaacagtgttatgggtggattctctgtatccggcgttaattgttaactggttaacgtcacctggaggcaccaggcactgcatcacaaaattcattgttgaggacgcgataatgaaaacgttattaccaaacgttaatacgtctgaaggttgttttgaaattggtgtcactatcagtaacccagtatttactgaagatgccattaacaagagaaaacaagaacgggagctattaaataaaatatgcattgtttcaatgctggctcgtttacgtctgatgccaaaaggatgtgcacaatgaattcagcatttgtgcttgttctgacagtttttcttgtttccggagagccagttgatattgcagtcagtgttcacaggacaatgcaggagtgtatgactgcagcaaccgaacagaaaattcccggtaactgttacccggtcgataaagttattcaccaggataatatcgaaatcccggcaggtctttaaaacagttccgtaataaatatccggtttcattcttatatgccagcaatggcagggatttgttcatccttaaatctgtcatgaggttaaaacaaatgagtaaagtctttatttgcgccgctattcctgacgaactggcaacaagggaagaaggcgctgtggctgtagccacagccattgaagctggcgacgaacgccgtgctcgagcaaaatttcactggcaattcctggaacattatccggctgctcaggactgcgcttataaatttattgtctgcgaggataaacctggcataccccgccctgccctcgattcatgggatgctgaatatatgcaggaaaaccgctgggatgaggagtctgcttcttttgtcccggttgagactgaatccgatccgatgaacgtcacttttgacaagctggcccctgaagtacagaacgctgtcatggttaagttcgacacatgtgaaaacatcaccgttgatatggttattagcgcacaggaattgttgcaggaagacatggcaacattcgacggacatatcgttgaagcgttgatgaaaatgccagaagttaacgccatgtatccggagcttaagttgcacgccattgggtgggttaagcataaatgtattcctggtgctaaatggcccgaaattcaggcagagatgcgcatctggaaaaaacgtcgcgaaggtgaacgcaaggaaaccggaaaatacacgtctgttgttgatctcgcccgcgccagagccaatcaacagtacactgaaaattcaacaggaaaaatcagcccggtcattgctgccattcatcgcgaatacaagcagacatggaaaacactggatgacgaactggcctatgggcgctgcttcgcagacaggcagaacttgatggtatgcctgcgatcaatgccaaacgtgtttaccggatcatgcgccagaatgcgctgttgcttgagcgaaaacctgctgtaccgccatcgaaacgggcacatacaggcagagtggccgtgaaagaaagcaatcagcgatggtgctctgacgggttcgagttctgctgtgataacggagagagactgcgtgtcacgttcgcgctggactgctgtgatcgtgaggcactgcactgggcggtcactaccggcggcttcaacagtgaaacagtacaggacgtcatgctgggagcggtggaacgccgcttcggcaacgatcttccgtcgtctccagtggagtggctgacggataatggttcatgctaccgggctaatgaaacacgccagttcgcccggatgttgggacttgaaccgaagaacacggcggtgcggagtccggagagtaacggaatagcagagagcttcgtgaaaacgataaagcgtgactacatcagtatcatgcccaaaccagacgggttaacggcagcaaagaaccttgcagaggcgttcgagcattataacgaatggcatccgcatagtgcgctgggttatcgctcgccacgggaatatctgcggcagcgggcttgtaatgggttaagtgataacagatgtctggaaatataggggcaaatccacaggtgaactacgctcctctgtttgttacgcaataaaaactggtgttttcgactatgcaaaacagtttccctcctcacgcaatctggaaaaatttggtgaggcccgacaagatttaaccataaaagaactggctgaaaaatttctggcactgaaagaaactgaagtcgccaaaacatcactcaacacataccgtgccgtcatcaaaaatatcctgagcataatcggtgaaaaaaatcttgcctcatcgattaataaagaaaaattactggaggttcgtaaagagttactgactggataccagatccccaaaagtaactatattgttacacaaccagggagatcggctgtaactgtaaataattacatgacaaatcttaacgccgtgttccagtttggtgttgataacggttacctggcagataatccgtttaaggggatctcgccattaaaggaatcaagaaccattccggatcctctttcgcgggaagaatttatccgtcttatcgatgcgtgcagaaatcagcaagcaaaaaatttatggtgtgtttctgtttatactggagttcgccctggtgagctgtgtgcacttggatgggaggacatagatctgaaaaatggaacaatgatgatcaggagaaatttagcaaaagaccgtttcacggtaccaaaaacacaggcgggaaccaatcgggtcattcatcttattaagccagcaatcgacgctctccggagtcagatgacattaacgagactgagcaaagagcatatcattgatgttcacttcagagagtatggcagaacagaaaaacaaaaatgcacctttgtttttcaacctgaagtgtcagcgagagtaaaaaattatggtgaccattttaccgttgactcaataaggcagatgtgggacgcagcgataaaacgtgccggactccgccatcgaaaatcatatcagtcgagacatacttatgcctgctggtcgctgacagctggtgctaacccggcatttatagcaaaccagatgggccatgcagatgcgcaaatggtatttcaggtatacggaaaatggatgtctgaaaacaataatgcacaggtagctttgttaaatacacagttaagcgagtttgccccaaccatgccccataacgaagcaatgaaaaattaatttaatatttatcaaatagttaacacgcatgactcttgaaatccataaattcaagcgcagtgcccagccatcccgatactgctgctttcaccaaatccttagtgcttctttcgtgtttttctattgtcataatggttatctctaaaaaagaggtaagatgcgtactacttactcgccgttattggtattattcagaaaaagtgagtaagactttgcagcaatgtttttgatcctgttcaaataaactaatggcatcagcaacatgctggaaatcaaacgtatgggtaattaatttttctggtttaattaaccctttacttaaccagtcgataacgatcgggaatttatttgcatttaagcgtgaagagaaaatagagagttcttttccggtaattccttgctgaatcacttcagacggttcactggagaaccccatcaatacaatacgtgccgctggagaagccagcgttacggcctctttcaggatagaaggatgacaagccgcatcgataattaatgtcggcttgatgcctttttcagtgaaaatctcgccaagcggtgtctggctgttattaatcgcccagtcagccccgctctctttcgctttttccagtcgttcatcaatgcgatcggcaacaatcacatttttaacgttatagacgccttttaatacctgaacgatcgtcaggccgattggaccggcaccataaaccagaacggtatcattttcagtcggttgaccatgtccggttacgttagccgcaatggtaaaaggttcgatcattaccgcatattgatcggccactgcttcaggaattttccacgcattttttgccggaaccacggcatattcactgaaaccaccgtcagcgtgcacacctaatacagccagtgtcgtacaaacgttcggtttacctatagagcacggatagcaatgcccacagctgaccaccggatcgacagcaacacgttcaccgactctggcgctttccacgccttcacccactgcatcaatgacgccaaagaattcatgaccaatgacgcgcggatatttcgcaaaaggattatgcccacgataaatatggctatctgaaccacaaattccggcaagtttcacttttactcgtacttcacccgctgacggggtgggtatttcacgttcgacaatcgccagttgattcggtttttcaattaatatgcttttcattatcttactccttaccagttccacagcgtgccatcttccagacgtgcgactggtagataagcaggttcatagggatatttcgccgccagcttttcatcgaattcgataccaagacccggtttgtctcccggatgcatatagccgttatcgaaagtccagttgtgcgggaagacttcgagcatttgttcggaataacccatgtattcctggacaccgaaattggggacccacagatcaaagtgcagcgccgcagccatgcagactggtgacaaatcggaaggaccgtgtgagccagtacgtacctgatacagcgaagcaaaatcggcaatccggcgcataccggtaattccgcctgcatgggtcagcgtggtgcggatataatcgatgagttgctcttcaatcagttgtttgcagtcccagatgctgttgaagacttcacccactgcgatgggtgtgacggtatgttggcgaatgagacggaagcattcctggttttccgcaggcgtcgggtcttccatccagaacatgcgataatcttcaatgcttttaccaaagcgcgccgcttcaataggcgttaagcgatggtgcatgtcatgcagcaaatgttcattaaaaccaaacttgttacgtaccgcgtcaaacaatttcggcatgaaatcgaggtatttctccgtcgaccacagctgctcttccggccactgtcctttggttgcgggttcataagccagacctttacctttcgacatgccgtaggtggttttcataccagggattccgcactgcacgcggatggctttgaatccaagctcttgatgacgggcataatcatccagagcttcatcaatactgtgaccggtggtatggcaataaaccatcaccccttcacgagacgcgccgccgagtaactggtaaagcggcatgttggcagctttggctttaatatcccacagcgccatatcaaccgctgaaatggccgacatcgtaaccggaccgcgacgccagtaagcacctttatagaaaaactgccagatatcttcgatacggtgcgcatcgcgaccaataagctgcggacaaaggtgatcctgcaaataagaggccacggaaagctcacgtccattgagggtggcatccccaaggcccgtaataccgtcctcagtggtgatttttaatgtgacgaaattacgccccggacaggtaacaaaaacttcagcctttacgatcttcatgttcgattccttgcatcgcttgtcgtgatgcatgaaatctacgcaactgagctactaccatacaagtataaagatcgaaaaaagccggagtgatcacaaaaaaaggcgtatatttgcgctgtgaatggttgacaaaagatgaaatagaataccttttgtcagctgacacttcctcttatcttattgataaaatggatttatgttcctacgtgcgcccccagcccgcaacaatgatcaacatgccgcaaagcgcaatcaacgcacccgtccagtcataaagagtcagtttcacgccatccacaacgcgcagccacatcaacgccgtgcagacataaacgccaccataagccgcgtaaacacgcccactcgccgctggatgcaacgttaacaaccagacaaacagcgccagtgaaatccccgccggaagcaacagccagatactggcgtttcgttttaaccacaaccagggcagaaagcatccaataatttcacacagcgcagtagcaaaaaatagtaacgttgttttaatcatctttgtctcttattgacatcatgtatagttatagggcgacataatatcatcaatataaacaccctcctggtacgttttgcgtccgcagtggatggtgtagaatcacctttaatcattcatacagggaatgaattatgaaaatcactctcagcaaacgaatcggcctgctcgctattctgctgccttgcgcactggcattgagcacaactgttcatgccgaaactaacaaactggtgattgagtctggcgacagtgcacaaagccgccagcacgccgctatggaaaaagagcaatggaatgacacgcgcaatctgcgccagaaagtgaataaacgcactgaaaaagagtgggataaagccgacgccgcttttgataaccgcgataaatgtgagcaaagcgccaacatcaatgcctactgggagcccaatactttgcgctgcctggaccgtcgaactggccgcgttattaccccctaacctgttattgatttaaggaatgtaaggacacgttatgccaagcgcccacagtgttaagctacgcccgctggagcgtgaagatttacgctatgtacatcaactcgacaataacgccagtgtgatgcgttactggtttgaggaaccctacgaagcctttgttgaactctctgatctgtatgataagcatattcacgatcagagcgaacggcgctttgtggtggaatgtgacggcgaaaaagccggtctggtggagctggtggaaattaaccatgttcatcgccgcgcagaatttcagataattatctccccggagtatcaggggaaaggtctggcaacccgtgccgccaaattagcaatggactatggctttaccgttctcaatctctataagctgtatctgatcgttgataaagagaatgaaaaagcgattcacatttaccgcaagcttggcttttcggttgaaggtgaattgatgcacgagttctttattaatggtcaatatcgtaatgccattcgcatgtgtatattccagcatcagtatctggcagagcacaaaacaccgggtcagactctcctgaagccgaccgcacaatagcattaataataatcgatcgtatttttgatggtgtaaacccgttcgacggcgggttttactccttcatcaacaatgattagctgacagtccaccggattagcgtgactgtcatattcacagctctgttttacattaccaacccgttgattattcagtaaagtaaccgctgtgtaatctaattttttgatcggatccgttgatggcgtggcgctgacagataatgttttgtcgttacttttcgtggttttacccagcggataaccctgatcatcatagcgatattccatctgcatttgtttgctgctggctttaatcacgaagccattatcatcggtttcccaactcaccccggcagaaggtaattctgctagctggcattttccctgtaaacgtactctcttctccagcgtctcggcatcacggtaataattggcgtccagtaccagagcgaccacggtattattttccagatccagtaattcgagtgaatcaaaacagccttcttccgacaaagtcccagaaacacgtttcgtcacttcaccttgctcatccattaatgtctgagtgaaatcttttaccggaccacgcagcggatcaaaatcgaattcattagagaaactggccatctcaggggtaaatgaaagtgttacctctgtgcggtcacatcctgtgaggaatatcgcgagtaagcatggtagtaatttgtatttcacaacagtcaccagagagtagagatgattctcaatcatagtagcaaatacagtactttacacgttaaatgctatgcttaaagaagttatcttcgcgtaaggagcttatgatgaaactctcaacctgctgtgccgcgcttctgctcgccctcgcctcacccgcggtactcgccgcgccgggatcctgtgagcgcatacagagcgatatatcacagcgcattatcaataatggcgtacccgaaagcagcttcacgttaagtattgtacccaatgaccaggttgatcagcctgattcccaggtcgtcggccattgcgctaatgatacgcataaaattctctatacccgcaccaccagcggtaacgtctctgctcccgcgcagtctagccaggatggcgcgcctgccgaaccgcagtaacacattatcgactgaacgccggatatgacaaatccggcgatttgaacatacaacataatcccaccttattactcatacccttctattgatatggattaataattcttaacccaaaatgggtagactccctctattgttagcgcgctaaatattcaatatataaacttttatataacgataaagaacagggagtgagttatgtccaaaaatgaacgaatggtgggcatcagccgcagaacactcgttaaatctaccgcgataggttctctggcgctggctgcaggcggtttttctttgccgtttaccctgcgcaatgcagcagcagcggtacaacaggcccgcgaaaaagtggtctggggtgcctgttccgtcaactgtggtagccgctgtgcacttcgtctacatgttaaagataatgaagtgacctgggtggaaactgacaataccggcagcgatgagtacggcaaccatcaggtacgcgcctgtttgcgcggtcgctccatccgccggcgtattaatcatcccgatcgcttgaattacccaatgaaacgcgtgggcaaacgcggcgaaggcaaattcgaacggattagctgggatgaagccctggatactatcgccagtagcctgaagaaaaccgtcgaacaatatggcaatgaggctgtatatattcagtactcttcggggatcgttggcggcaatatgacccgctcttcgccatcagcctcggcggtcaaacgcctgatgaactgctacggcggttcactcaaccagtatggctcctacagcactgcgcaaatttcctgtgccatgccctacacctacggcagtaatgatggcaacagcaccacggatattgaaaacagcaagctggtcgtgatgtttggtaacaacccggcagaaacccgcatgagcggtggtggcatcacttatcttcttgaaaaagcgcgcgagaaatcgaacgccaaaatgattgttatcgatccgcgatataccgatacggctgccggtcgtgaagacgaatggctccctattcgcccgggcaccgatgccgcgctggttgcgggtattgcctgggtattgattaacgaaaatctcgttgatcaaccttttctcgataaatactgcgtcggctatgacgaaaaaaccttacccgcagatgcacccaaaaatggtcactataaagcctatattcttggtgaaggtgacgataaaacagcgaaaacgccgcagtgggcttcgcaaattaccggtatcccggaggaccgtatcatcaaactggcgcgtgaaattggcacagcaaaacccgcttatatctgccagggctgggggccacaacgccaggcaaacggcgaactgactgcacgcgctattgctatgttacctattttgacgggcaatgtcggcatcagcggcggaaatagtggcgcgcgtgaatcgacctataccattaccatagaacgcctgccggtgctggataatccggtcaaaacgtcaatctcctgcttcagctggacagatgctatcgatcatggtccgcaaatgacggcaatccgcgacggcgtccgcggcaaagataaactggatgtgcccattaagttcatctggaactacgcgggaaataccctcgttaatcagcattctgacatcaacaaaacgcatgaaattctgcaggacgaatcgaaatgcgaaatgattgtggtcatcgaaaactttatgacctcatcggcaaaatatgccgacattctgctgccagacctgatgaccgttgagcaggaagatattattcctaacgactacgccggtaacatgggatatctcattttcctccagcctgtcaccagcgaaaaattcgaacgcaaaccgatttactggatcctgagtgaagtcgcgaaacgtcttggacctgacgtctatcaaaagttcacagaaggtcgcacgcaggaacaatggttacaacatctgtacgccaaaatgcttgccaaagatccggcgttaccgtcttacgacgaactgaaaaaaatgggtatctataagcgtaaagatcccaatggccattttgtcgcctacaaagcatttcgtgacgaccccgaggcaaatccacttaaaacgccttccggtaagattgaaatttattccagcaggctggcggaaattgcccgtacctgggaactggaaaaagatgaagtgataagcccattgccagtttatgcctcaacctttgaaggctggaactcccctgaacgtagaaccttcccactgcaactgtttggtttccattacaaatcccgtactcactcgacctacggcaatattgatctcctgaaggctgcctgccgtcaggaggtgtggatcaaccctatagatgcgcagaaacgtgggattgccaacggcgatatggtgcgggtgtttaaccatcgtggcgaagttcggctaccagccaaagtaacaccacgtattctccctggagttagcgctatgggccagggagcctggcacgaggccaatatgtctggcgataaaatcgaccatggcggctgtgtgaatacgctaaccactctgcgcccttcaccactggcgaagggaaacccgcagcacactaatctggtcgagatcgaaaaaatataacccacgacaaccataaattctggcatgacattttgtttgaaaagcaataagtgagtaatgatgaaaatccataccacagaggcgctcatgaaggctgaaatcagccgtagaagtctgatgaaaacctccgcacttggcagtcttgcgctggcaagcagtgctttcactctgccattttcccaaatggtccgggcggcagaggctccggtagaagagaaagcggtctggagttcctgcaccgttaactgcgggagccgctgtctgttacgtttgcatgtgaaagatgacaccgtgtactgggtggagtctgatacgacaggtgacgacgtctacggtaatcatcaggttcgagcgtgtttacgcgggcgctctatccgccgacggatgaatcatcctgataggttgaaatatcccatgaagcgcgtcggcaagcgcggtgaaggtaaatttgaacggataagttgggacgaagccctggataccatcagtgataatcttcggcggatcctgaaagattacggcaatgaggctgtacatgtcctgtacggaacaggcgtagatggcggaaacatcaccaactcaaacgtcccgtaccgtctgatgaactcttgcggtggttttctcagtcgctatggcagctacagtaccgcacagatcagtgccgcaatgagttatatgttcggtgccaatgatggcaacagcccggatgatatcgccaatacgaaactggtcgttatgttcggaaataacccggcagaaacgcggatgagcggcggtggtgtcacttactacgtcgagcaagcccgcgaacgttcaaacgcacgcatgatcgtcatcgatccacgttataacgacactgctgccgggcgtgaagatgaatggctgcccattcgccctggcaccgatggcgcactggcctgtgcgattgcctgggtactgattactgaaaacatggtcgatcagccatttctcgacaaatattgtgttggttacgatgaaaaaacgctgcccgccaacgcaccacgtaacgcgcattataaagcctatattctgggcgaagggcctgacggcatagctaaaacgccggaatgggcagcaaaaatcaccagcatcccggcagaaaaaattatccagttggcacgagagatcggttcagcaaaacctgcttatatttgtcagggttgggggccacaacgacattccaacggcgagcaaacatcccgcgctattgccatgctttccgttctcaccggcaacgtcggcataaacggcggcaactcaggcgtacgcgaaggtagctgggatctgggggtagaatggttcccgatgctcgagaatcctgttaaaacgcagatttccgtctttacatggacagatgccatcgaccatggtacggaaatgaccgcgacccgtgatggtgttcgtggaaaagaaaaactggatgtccccatcaagtttttatggtgctacgccagtaacacattgatcaatcaacatggcgacatcaatcacacccatgaggtgcttcaggatgacagcaagtgcgagatgattgttggcattgaccacttcatgacggcctcggctaagtattgcgatatcctgttgcccgacctgatgccaacagagcaagaagaccttatctctcatgaatctgcagggaatatgggctatgtgatcctcgcccaacccgcaacctcagcaaaatttgaacgcaaacccatctactggatgctgagtgaagtcgccaaacgcttaggaccagacgtttatcaaacctttactgaaggtcgcagtcagcatgaatggatcaaatatctccatgcgaaaacgaaggaacgtaaccctgagatgcccgactacgaggagatgaaaacgaccgggatctttaagaaaaaatgcccggaagaacactacgtcgctttccgcgcattccgtgaagatccacaggcaaacccgttgaaaacaccttcggggaaaatcgaaatttattctgaacgactggcgaagattgcagatacctgggaattgaaaaaagatgaaattattcatccccttcctgcgtataccccaggttttgatggctgggacgatcccctgcggaaaacctatccactgcagttaacgggcttccattacaaagcgcgtacccactccagctacggcaatattgatgtgttacagcaggcctgcccacaagaggtgtggatcaaccccattgatgctcaggcacgcggtatccgtcatggcgataccgtgcgggtatttaacaataatggagaaatgctgattgccgcaaaagtgactccgcgtattctgcctggcgttaccgccatcgggcaaggtgcgtggcttaaagcggatatgtttggtgaccgggtcgatcacggcggcagtatcaatattctgacctctcaccgcccttcaccgctggcaaagggaaacccgtcgcacagcaatcttgtccagatcgaaaaggtttaaggagtagcccatgaccacacaatatggattttttatcgattccagccgctgtactggctgtaaaacctgcgaactggcgtgcaaagattttaaagatcttggcccggaagtcagtttccgccgtatttatgaatacgctggcggcgactggcaggaagataatggcgtctggcaccagaacgtgttcgcttattatctctccatctcctgtaaccattgcgatgaccccgcatgtacaaaagtctgccccagcggcgcaatgcataagcgtgaagatggctttgtggtggttgatgaagatgtttgtatcggctgccgctactgccacatggcttgtccgtacggcgcgccacagtacaatgctgaaaaagggcacatgacgaagtgcgatggttgttattcgcgcgtcgccgaggggaaacaacccatatgtgtcgaatcctgcccgctgcgtgcacttgagttcggtccaattgaagagctgcgccagaagcacggcactcttgctgccgtcgcgccactgccgcgcgcgcatttcacaaaacccaatatcgttatcaaacctaacgccaacagccgcccgaccggcgataccactggttatctggctaatccggaggaagtgtaaaatgggaaatggatggcatgagtggccactggttatctttaccgtattgggtcaatgcgtagtaggcgcgctgattgttagcggaattggctggttcgccgccaaaaatgacgcagaccgtcagcgtattgtccgtggcatgtttttcctctggctgttgatgggcgtcgggtttattgcctctgtcatgcacctgggatcgccactgcgggcgtttaactccctgaatcgaatcggagcttctggtctgagtaacgagattgctgccggttccatattttttgccgttggcggattatggtggctggtggcagtcatcggtaaaatgccgcaagcgttggggaaactctggttacttttcagcatggcgctcggcgtcattttcgtctggatgatgacctgcgtgtatcaaatcgacaccgtgccaacctggcataacggttacactacgctggctttcttcctgacggtattgttgagcggtccaatacttgctgccgcaattctgcgggcagctcgcgttacatttaataccacaccatttgccatcattagcgttctggcgctgatcgcttgtgccggggtgattgtgctgcaaggtttgtctctggcgtctattcactcatccgtgcaacaagccagcgcactggtaccagattacgcctccttacaggtctggcgtgtggtattgttatgcgcaggtcttggatgctggctttgcccgctcattcgtcgccgtgaacctcacgttgccggacttattctggggctaatcctcatacttggcggtgagatgatcgggcgtgtgctcttttatggcctgcacatgacagtaggaatggctattgcaggttaacaaattggtgcggggcaacccgcacatttcaggatgttaggaatgacccatttttcacagcaagataatttttctgtcgcggcgcgcgtgttgggcgcgctgttttattacgctccagagagtgcggaagccgcacctctggttgcggtactcaccagtgacggctgggaaactcagtggcctctaccagaagcgtcattagcgccgctggtgacggcttttcagacacagtgtgaagagactcacgcccaggcctggcagcgtttgtttgtcggcccgtgggcactgccgtctccgccgtgggggtcggtctggctggatcgcgaatctgtgctgtttggcgattcaacattggcacttcgtcagtggatgcgcgagaaaggcattcagtttgaaatgaagcaaaacgaaccggaagatcattttggttcactgctgttgatggctgcgtggttggcggagaatggtcgccagacagaatgcgaagaattgctggcatggcacctttttccgtggtcaacacgttttcttgatgtttttatcgaaaaagcagaacaccctttctaccgtgcactgggtgaactggctcgcttaacgctggcgcaatggcaatcacaactgttaattcctgtcgcggttaaaccgctgtttcgataggatcaccgtaatattgccggatggtgacgattacgcgcaatccggcaataataggttacagtgtcacgtttttttatctcttaaagcacgcactgcttttgcggctggcctcttttgccgcaaaatagtcgcccgtgtttcattgcccatttctgctcatgcatcatctacacatctatccggatctgcgcactatgttccaccgtctgcttatcgcaacagtcgtcggtattctcgcggcctttgccgttgccgggtttcgtcatgcgatgctgctactggagtggttgttcctcaataatgactccggcagtctggtcaatgcagcgacaaacctttccccctggcgacggttgctaactccggcgctcggcggactggcggcgggtttgttgctgatgggctggcagaaatttacccaacaacgccctcatgcgccgaccgattatatggaagcgttgcaaaccgatggacagttcgattacgcagcaagcctggttaaatcgcttgcctctctgctggtagtaaccagcggcagtgcaattggtcgcgaaggtgcgatgattcttttagctgcccttgccgcctcctgttttgcccaacgttttacgccacgccaggagtggaaattatggatcgcctgtggggccgcggcgggaatggctgcggcctatcgtgccccgcttgctggcagtttatttatagccgaagtgctgtttggcactatgatgttggcctctctcggcccggtgattatttccgccgtcgtggcattgctggttagcaatctgattaatcatagcgacgcgttactctacaacgtacaactctcagtgacggttcaggctcgtgactatgcgctgattatcagtacaggtgtgctggcaggtctgtgcggaccactgttgttaacgttaatgaacgcctgtcatcgtggatttgtgagtctcaaacttgcgccgccctggcaactggcactaggcgggttgatcgtgggtctgctttccctgttcacacctgcagtgtggggcaacggctatagcaccgtacaatcctttttaaccgccccaccactgttaatgatcattgccgggatcttcctttgtaaactgtgtgccgtgctggcgagtagcggttccggcgcacccggtggggtctttacaccgacgctatttatcggtcttgccattggcatgttgtatggtcgtagcctgggattatggttccctgatggcgaagaaattacacttttactcggattgaccgggatggcgacactgttggcggcgaccacgcacgcgccgattatgtcgacgttgatgatatgtgaaatgaccggggagtatcagctactccccggtttattgattgcctgcgtaattgcgtcggtaatttcgcggacgttacaccgtgactctatctaccgccagcacactgcgcagcatagctaagcggatgtattgccccagttcacgctgttcggcgcgcggcagataaggcagttcaccaatgagcggtgccggaagttttttacccagcacatcaatgatttccgcataatgcgccagtcctgggttgattcggttagccacccagccaatgagcggcagcccgtcgttggcgatcgcctgagctgttagcagtgcatggttaatgcaaccttcctgaataccgacaaccatcaacaccggcagttgttcctgcactacccattcagagagtggacgcaaatcattcatcagactgcgccagccgccagtcccttctaccacgacatgatcgactttttcggtcaggtttgccaggccgtttgaaatgagggtgtaattgattgggcaactgtgcgccacgctactttcttcttcgcttaacgcgataggattaactgcttcataaggcagttcgatggttgaaacactctgcaacaccagggcatctttattacgcagcccttcgggtgtctctttgctccccttcgctacgggtttatatcccgcaaccgtttttccctgggaggctaacgcttgtagcaatgcgcgggaaaccaccgttttccctacagaagtgtctgtaccggtaataaagaaacgcttcagcatcactaactccaccgttatgcttcacaaatataaaccaggaaaataattaaccttgaaagtctaagttatgctttcctggcccaaattgagatagcgcaaattttggtagaacagttaaaaaatgttaaccctgcaacagacgaatcaacaaagaaccgttatacatcgcgtcttttaccagtgcagcgcctgccatcgtgccctggttagaaaactgagtactctcaacgctgatgtgctgactatacgcaggaagggcctgctgacggatgctgtctgagatgaccgggaagaggatatctgccgctttacttaacggtgagccaatcagtattttttgtgggttaaataaattcaccatgatggcaagaatgcgcccgacatgcgcgcccaccccggtaatgatgtcttttgccagtagatcgccgcgcaatgccgcctgacacaatgagtccacggttaacggttgtccatgtaacatcgagctcatggattgattaagacgcagctgtgccagctcaagaatactgtccacgctggcgatggtttcgaggcagccgtgattcccgcaataacagcgtttcccatacgggtcgacctgtgtgtggcctatttccacgagactactgctgcctgcgtgtagcagatgaccatcggtaatgacgcccgcccccacgttgtgatcgataaccacctgaatcacatcgcgcgccccgcgtgaggcaccaaacaaggcctctgccatcgtccatgcgctgatatcatgctgaatataaaccggaacgccggtatgctgctccagcgcctcgccgagcggcatctcttttacatcctcgtagaacggcatgcgatgtacaataccattttccgtatcaataattcccggcaaggttatggcaatcgaagttagacgctcaagttttttctggtggcggataaaaaactgatcgatatgggaaataatacgatccagcaatggcaagtcatcttttaacgccagttcctgcgactcttccaccaccagtttgctgctcagatcgcgcagagcaaggaaaatctccccgcgactaatgcgcagagaaagatagtgccaggcttcagtttcaaccaccagccccaccgccggacggccacggttccccgcttctttgatttccagctcttgcaccaggtgtgcttcgagcatctcacggacaattttagtgatactggcaggagccagttgcgccagacgggaaagatcgatacgcgagactggaccaagctgatcaatcaggcgataaaccgcgcccgcgttggtctgctttatttgatcaatgtgcccaggctggttttcagcaaccaccgcatactccctatattttcgcgctccgaaataatctgtaggctatggtgaagcacttcaatacgtgtcgtcaaatttttacttaggcatgtgattaacagcacatttttcgggctttttcgctgaaatttccctcacctgagagcattcagcagatgaatacgaaagttacgcgcagccggactttgttcatgatgtttcggccagaccaaccacatttcagaaaccgcatcctcttcagcaatcggcacccagcgcatttcgttgagctgaacacgtttaaatgacgcaggcaaaattgaaacacccagaccggcggaaaccagaccgatgatggtcattgcctcgcccacctcctgagtgatgacgggcgtcaaatggtaacgtcgcatcagcccgagaatatcgtcatacagccctgtcccgacgtgcggatcaaaaaagacaaagggttctttcgccagttcagccagcgttacattcgggttatttgccaggggatgatcgtgcgggatcatcgccataagcggttcatggacgatgactgcgtgttcaagcgactccggtaacgctgtgttacgcagcaatcccatatccagcgttccttcaatgagcggagcgatttgctcgcgagtgttcatttcgcgggtttgtaaatggacatcaggataatcacggcgaaacagcgataacgtatcggacaccgcccgaataaaaggagccgacgaagtaaaaccaatgcgcaactcccccgcttcaccctgatgcagcctttcagcgcgagcggcagcgtcatccaccatagacaggatttgccgactatctgcaagaaactgttttcctgctgccgtcagcaatacactgcgattggttcgtgccagcagtcgggcaccaatttgttgctccagcgcctgaatctgctgacttagcggcggttgcgaaatattcaggcgggcagcggcgcgcccgaaatgcagctcttccgcaacagcaacaaagtaacgcagatgacgaagttcaatattcatatttaaaacatcttatttgagattattaatatattagacagaacaattcgattttcctaccctatgtataagcctgatctacaggcatatttagcaaggatttcaagtgagccgtactacaactgttgatggcgctccggcaagcgacactgacaagcaaagcatttctcagccaaatcaatttattaaacgcggtacgccgcaatttatgcgcgtcaccctggcgctgttctctgccggactggcaacatttgcacttctctattgtgtgcagcctatccttccggtgctttcgcaggagtttggcttaacccccgcgaacagtagtatttcactgtccatttccacggcgatgttggctattggtttgctgtttactggcccgctatccgatgccattggtcgcaaaccagtgatggtcacggcgctactgttggcctccatttgtacgttactttcgacaatgatgaccagctggcacggcattttgattatgcgcgccttgattgggctttcgttaagtggcgtggcagctgttggcatgacttatcttagcgaggaaatccatcccagtttcgtggccttttcaatggggttgtatatcagcggcaactcaattggcggcatgagcggacgcttaattagcggtgtcttcacggactttttcaactggcgaattgctctggcggcaatcggttgtttcgcgctggcctcggcgttgatgttctggaaaatcctccctgaatcacgccattttcgcccgacttcgctgcgccctaagacgttgtttatcaactttcgtctgcactggcgtgaccggggattaccgttattgttcgcagaaggctttttgctgatggggtcgttcgtcacgctgtttaattacatcggctatcggttgatgctctccccctggcatgtcagtcaggccgtggttggcttattatcgctggcttatttgaccggtacatggagctcacccaaagccggaaccatgaccacccgctatgggcgtggtccagtgatgttgttttcgacgggggttatgctgtttggtttactgatgaccttattcagctcgctgtggctgatctttgccggaatgttactcttctcagcaggattcttcgcagcccactcagtagccagcagctggatcggcccccgcgcaaaacgcgctaaaggccaggcctcctcgctgtatctgttcagttactatctggggtcgagtattgccgggacgctgggtggtgttttctggcataactatggctggaacggcgtcggcgcatttattgctctgatgctggtcattgctctgctggtcgggacgcgtttgcatcgtcgtctgcacgcctgaaaaataagtccggactgcggtaaatacccgtccggacttattgccagctcaaaccaacgttaatagccatcctaaaatagacgaagcgccagccaattcccgcagcgcgtctagcgtcatcaggattataagtacccaaataaacggattcattttgctgtgtgtcatttattactgatgcgcagttattctactgctttgtaagtagtaaaatagttaacccgatcaagactactattattggtagctaaatttcccttaagtcacaatacgttattatcaacgctgtaatttattcagcgtttgtacatatcgttacacgctgaaaccaaccactcacggaagtctgccattcccagggatatagttatttcaacggccccgcagtggggttaaatgaaaaaacaaattgagggtatgacaatgaaaaaagtattagctctggttgttgccgctgctatgggtctgtcttctgccgcctttgctgcagagactacgaccacacctgctccgactgcgacgaccaccaaagcagcgccggcgaaaactacacatcataaaaaacagcataaagcagcacctgcccagaaagcgcaggcggctaaaaagcatcataaaaatacgaaagctgaacagaaagcccctgaacaaaaagcgcaggcagcgaagaaacacgccaagaaacacagccatcagcaaccggcaaaacctgctgcacaacccgcagcgtaagttttcaacagtaatgctggcgcgccccctcgcgcctgaaaattacggtgctaagcgggtaacgtttagcaccgcctttagcggagggtagtatggtgggccgttatcgctttgagttcattctgatcatccttattttatgcgcactgattaccgcccgtttttatctttcctgattgtagttatctgattttactcccactttcatcccgtcccgtctatagtatttatgagggtttgcttttaataatcataattacccaccagagtgtgatatgcgtacaaccattgctgtagtgttgggtgcaattagtttgacgtctgcttttgtgtttgcagataaaccagacgttgccagatcggcaaacgatgaggtcagcaccctgttttttggtcatgatgatcgtgtgccagtgaatgacacgacccaatcaccgtgggatgcggttgggcaactggaaacggccagcggcaatttatgtacggcgacgctgattgcacccaatctggcattaacggcaggacactgtttattgacacctccaaagggtaaagccgataaagcagtggcgctgcgttttgtgtcaaataaaggtctttggcgctatgagatccacgacatagaaggccgcgttgatccgacactgggaaagcggttaaaagcagatggggatggttggattgtacctcccgcagccgcgccgtgggacttcggattgattgtgctacgtaatcccccttctggcattacgccgttgccgttatttgagggagataaagccgcgcttaccgccgcattaaaagcggcaggtcgtaaagtgactcaggcaggctaccctgaagatcatctcgatacgttgtacagtcatcaaaactgtgaagtgactggctgggcgcaaacgtcggtgatgtcacatcagtgcgataccttgccgggtgacagcggttcgcctctgatgttgcataccgatgacggctggcaattaattggggtgcaaagttcggctcctgccgcgaaagatcgctggcgcgccgataaccgggccatttctgttaccggttttcgcgacaagctggatcaactgtcgcaaaaataatgttcaaacgctgcccgacagcgcgggcagcgtcttcatcaggcaagtttcaccatgatcattccagccaacagcaagaccaggccaatccagcctttacgatttaaccgttgaccaaacaagatccaacctgcggctaacgtggcggcaataccaaacccgccccacaatgcataagcgacagacaagtcgatccctttaacggcttgagaaagcgcactaaaggcagccagcaccgccgccagggagagcaagccaaatattttgcgacgaaagccgtcagaaaatttcaaaaagacgttagcaacgatttccagcacgattgccaatgccagccaggcggcgtgaacccattcaaactgcgccatggttcacctccagttcaggtttacgcgctttacgggtacctgattttatcaacacaatcccggcgaccagggtggttaacccggcaattttcatcagcgataaactttcgtcgaataacaaaacgctaaacaaggtaataaataaaataccgataccttcccacagcgcataagctacgcctaaggcgatttttttaacggcgaaagagagaaatatatacgacagagaaatcatcaccagcattaaaataaagccgccatttccctcactgacgctcgcccatttcattgacagcgtaccggtaatttctgtagcaatagccagacctaataaaatccaataaatatacattgtccttctcctgcaagagaattattttaattttcgcttaattcagcgaaaccaaagtaaagtggtcaagccccgcgcatagcgcaagctttggcagaagaaaggactaaagcgcgttgcgccagtgctgctcacctacgagcaagatagtggatgaggtacgaagatgggtaaatgtagaaaataacgtcctgaacaaattgtccataatattacaattatccgcagtgttgcttctcgtcatcgcggatgataattgtcctcggtagttgaacacgcctgatttgtatcatagcttaagaattaactcaaaatattttcacttctttacctgagcggtttgattttcgttatgatgacggagcgaaaaagacattattattagcaaaggaagaaaaaacggggacaagcatggcaaagccgatcatcacgctcaatggcctaaaaatcgtcattatgttgggaatgctggtcattattctctgcggtatccgttttgccgccgagatcatcgtgccgtttattctcgcattatttattgctgttattcttaacccgctggtgcaacacatggtccgctggcgtgtgccgcgtgtactggcggtgtcgattttgatgaccatcatcgtgatggcgatggtgttgctattagcttatctgggttccgcgctcaacgagttgacgcggacgttaccgcaatatcgcaactctattatgacgccgctgcaagcgcttgaaccgttgttgcaacgcgtagggattgacgtctcagttgaccagctggcgcattatattgatccgaacgcggcgatgacgttgctcaccaacttattgacgcagttatctaatgccatgtcatcaatatttttattgctgctgacggtgctgtttatgctgctcgaagtgccacaattgcccggaaaatttcagcaaatgatggcgcgtccggttgaagggatggcggcgattcaacgtgcgattgacagtgtttctcattatctggtgctgaaaacagccatcagcatcatcaccggcctggtcgcctgggcgatgctcgccgcactcgatgttcgcttcgcttttgtctggggattgctggcctttgcgcttaattacatcccgaatattggttcagtcctcgcggcaatcccccctatcgctcaggtactggtgtttaatggcttctacgaagcgttgctggtgctggcgggatatctgctgattaatctggtcttcggcaatattctggagccgcgtatcatggggcgtgggctggggctttccacattggtggtatttttgtcgttgattttttggggatggttgttaggaccggtgggtatgctgctttccgtgccgttgacaattattgtcaaaattgcgcttgaacaaacagcgggaggtcaaagcatcgccgttctgttaagcgatctcaataaagagtgacggcctcagcagaggccgtcagggttacagagctttcaggattgcatccacgctggctttggcgtcaccaaacagcatgtgggtgttttccttgaagaacagcgggttttgcacaccagcatagccagtgttcatcgaacgtttaaagacaatcacgttctgcgctttccacacttccagcacaggcataccagcaatcggactcttcggatcatcctgcgccgccgggttaaccgtatcgttagcaccaatcaccagtacggtatcggtatcagcaaagtcatcattgatctcgtccatttccagcacgatgtcatacggtacttttgcttcagccagcaatacgttcatatgtccaggcaaacgccccgcgaccgggtggataccgaaacgcacattaataccacgagcgcgcaatttctcagtaatttcagcgacaggatattgcgcctgcgcgactgccatgccgtaccccggagtaatgatcactgaatgggagtttttcagcagttccgctgtctcttctgcggtgatttcgcggtgctcacccacttcctgatcatcgccagtagaagagccgtcggtgccgaaaccacccgcaataacgctgataaaggaacggttcatcgccttacacataatgtaagaaaggatagcccccgaagaaccgaccagcgcaccggtcacaatcagcaggtcgttgctgagcataaagcccgcagccgcagccgcccagccggagtacgagttcagcatcgacaccaccactggcatatctgcaccaccgatggaggcgactaaatgccagccgaataccagcgcaattgcggtcattatcagcaatgccagcacttgcaggccgacgctgtccgtgcgaacaaatacaatcagcagcaggaaggaaacgaccagagccgccaggttcattttgtgacggtttggcagcatcaatggtttagacgaaatcttgccacacagtttgccgaacgccaccaccgaacccgtgaacgttaccgccccgatgaagataccgaggaacacttccgtcaggtgaatattgaccagaatcggtgccattcccgcgtcatgatgcagatagctgttaaagccaaccagcactgccgccagacccacgaagctatgcaggatcgccaccagttctggcatttcggtcatttcaactttcttcgccagacggataccaattgccccaccaatgaccatcgccagcaagatccagccaacattacccgtatccggtccaaaaatggttgcgattaacgcaatcgccatcccggcgataccgaagttgttaccctggcgagacgtttcatgtttcgaaagaccggccagactgaagataaacaggatcgcggcaacaatgtatgcagctgtaactaatcctccagacatatgttaccccttaatttttgcggaacattttcagcatgcgctgagtcacggtgaagccaccgaaaatattaatgctggctataagcaccgcgataaaactaaggaagctaacccagccgccctggccaatctgcaacagtgctccgacaacaataatccctgaaatcgcgttggtgaccgacatcaacggtgtatgcagcgcgtgcgatacattccacaccacgtaataaccgacaacgcaggccagcgcgaaaacggtgaagtgcccaaggaattctttcggcgcaacgcttgccatccagccaaaaagaatgattgccagcgccatcaacgcgtatttacgccacggtgagcaggtacatttttcctcagttttcacttccggtgccgctttttgtgccgcctgcggctgagctgatacctgaatcggcggtgccggccaggtaatttcgcccgcacggatcacggtcacgccgcgaatcaccacatcatcaaaatcaacagtgatattgccgtctttctctttgcacaacagtttcagcagattaacgaggtttgtgccgtaaagctgtgaggattgcgtcggcagacggcccggaagatcggtataaccaatcactttgacaccattttccgtagtgaagatttcacccggcacggtgtattcacagttgccgccgttttgggctgccaggtcgacaatcacactgcccgccttcatggagtcaaccatttcacgggtaattagcttcggcgctggtttgcctggaataagcgcggtggtgacaatgatatcgacctcttttgcctgggcggcaaagagttccatttccgctttgatgaacgcgtccgacatcactttggcatagccatcgccgctgccagcttcctctttaaaatccagctcgaggaattccgcgcccatactttgaacttgttctttcacttccgggcgggtgtcgaatgcacgcacaatcgcgccgagactgtttgctgcgccaatggcggccagacctgcaacacccgcaccaatcaccatcacttttgccggtggcactttcccggccgcagtaatttgcccggtaaagaagcgcccaaattcatgtgccgcttcaacaatggcgcgataaccggcgatgttcgccatcgagcttagtgcgtccagcgattgtgcgcgtgagatacgcggcacagagtccatcgccatcacggtcacgttacgttccgcaagtttttgcattaattccggattctgcgcaggccagataaaactcaccagcgttgtcccaggattcagtaacgcaatttcatcatctaacggcgcattgaccttcagaatgatctctgactgccagacgctattcccttctacaatttcagcgcccgcttgcacaaacgctttatcgtcaaaacttgccagttgacccgcgccgctctctaccgcgacggtaaaacccagtttcagcagctgttccactgtttttggcgttgctgcaacacgggtttcattggttaaccgttctcttggtatgccaattcgcatgatattcccttccatcggttttattgatgatggtttgcctgtgtcaggagccacacaagctgctcatgtacgagctaaatgttactccgttaaaataaattagtaacaaacgccctataacgtactgaaaattatgcctgtgatctagcgccaaaaatcagtatttcggcgtgaactcgcaaaatattaacgattcagccgtgatagtgggataaacaccttagaacgccggataaagactgataattgtcttcgacggtcgggtaaaacgagacatcgccccggcacgaatcactacttaacattaaattaacttatacaattcagttgcttcagtagtaatgatgctgatacggctgttttttaagcatagacggtcatttgagcaggattaaaattggcttaaggaatgtgatatgaaaaatgacgcagacagttacaccgtttaaatgcaataatcagccacgtttctcgttaataacaataccagtacctggtttgcgcaaggcgaaggattatttttatgaagcttaagaacaccctcctggcgtcggcactgctttctgctatggcattctccgttaacgcagcaacagaactgacaccggagcaagcggcagcggttaaaccttttgaccgtgtagtggttaccggtcgttttaatgctattggcgaagcggtgaaagccgtttctcgtcgcgcagataaagaaggtgccgcctctttttatgttgtcgacacttctgattttggtaacagcggtaactggcgtgtggtcgctgacctctataaagccgatgctgaaaaagcagaagaaacaagtaatcgcgtaattaacggtgttgtcgaactgccgaaagatcaggctgttctgattgaaccgtttgacacggtcaccgtccagggcttctatcgtagccagccagaagtcaatgatgccatcaccaaagcggcaaaagcgaaaggtgcctactctttctacatcgttcgtcaaatcgatgccaaccagggcggcaaccagcgtattactgcattcatctataaaaaagatgctaagaaacgtatcgtccagagcccggatgtgatcccggcagattccgaagcaggacgtgcagctctggctgccggtggcgaagccgcgaagaaagttgagatcccgggtgttgcgactaccgcatcaccaagttctgaagtcggtcgcttctttgaaacccagtcatcaaaaggcgggcgttacaccgtcacgctcccggatggcactaaagtcgaagaactgaacaaagcgaccgcagcgatgatggtcccgttcgacagcatcaaattctctggcaactacggcaacatgaccgaagtctcctatcaggttgcgaaacgtgccgcgaagaaaggtgctaagtattaccacatcacccgccagtggcaggaacgtggtaataacctgaccgtcagcgcagatctgtataaataactattcagttactcctataaggcggcttgatgccgcctttcgcatttttagtcacaaatttccccgcgaccattgcatgcagacacatctcttcgtaaaatcccgcgcttcagtggcaaactccatttttatgcgttttgccctaatatttattcttcttatcacgttttaatcactggatatcgatggaaaagaaactgggactgagcgcactcaccgcgctggtattaagctcaatgctgggcgcgggtgttttcagtctgccgcaaaatatggcggcagttgccagcccggcagcactgctcatcggctggggtattactggcgctggcattttattgctggcctttgccatgctgatcctcacgcgcattcgtcccgaacttgacggcggtatctttacctatgcccgcgaagggtttggcgagctaatcggcttttgttccgcatggggatactggctgtgcgcagtcatcgccaacgtctcctatctggtgatcgttttttccgcgttaagcttttttacggacacgccggaattgcgcctgtttggcgatggtaatacctggcaatcgatagtcggtgcatcggctttattgtggattgttcactttttgatcctgcgcggggtgcaaaccgctgccagcattaacctggtggcgacactggcaaaattgttgccgctgggtctgtttgttgtgctggcgatgatgatgttcaaactggataccttcaagctcgacttcaccggacttgcacttggcgtacccgtttgggaacaggtgaaaaacaccatgctgatcaccctgtgggttttcattggtgtggaaggtgccgtggttgtttctgcgcgtgcgcgtaataaacgtgatgttggcaaagcgacactgctggcggttctctccgctctgggcgtttacttgctggtaacgctgctttcgctgggtgtggtggcacgtcctgaactggctgaaattcgtaacccgtcaatggccggtctgatggtggaaatgatgggaccatggggcgaaatcatcatcgctgccggtttgatcgtttccgtttgcggcgcgtacttaagctggaccatcatggcagcagaagtaccgttcctggccgccactcataaagcattcccgcgcatttttgcgcgccagaacgcacaagctgcgccatccgcctcactgtggttgaccaacatctgcgtgcaaatttgtctggtactcatctggctgaccggttccgattacaacacgttgctgaccatcgcctcagaaatgattctggtgccctatttcctggtcggcgcgttcttgctgaaaatcgcaacccgtccactgcataaagcggtaggtgtcggtgcctgcatttatggcttatggttattgtacgcctctggtccaatgcacttgctgttatccgttgttctgtatgcaccggggctgctggttttcctgtacgcgcgcaaaacgcatacccatgataatgtactgaaccgtcaggaaatggtgctgattggcatgctgttaattgcctcagttccggcgacctggatgctggtgggataacgttcatcccatcgttggatagcaaaggagataacgatgggtaaaacccagcccttgccaatattaattactggcggaggtcgtcgcatcggcctcgccctcgcatggcatttcattaatcaaaagcaaccggtgattgtcagctatcggacacactatccagccattgatggactgattaatgcaggtgcgcagtgtattcaggctgatttttcgaccaacgacggtgtgatggcgtttgccgatgaagtactaaaaagcacccatggtctgcgtgctattttgcataacgccagtgcgtggatggcggaaaaaccgggtgcgccactggccgacgtactggcttgcatgatgcagatccacgttaataccccatacctgctcaaccatgcgctggaaagattactgcgtgggcacggacacgccgccagcgatatcattcactttaccgattatgtggtggagcgcggtagcgacaaacatattgcgtatgctgcaagcaaagcggcactggataatatgacccgctcgtttgcccgcaagctggcaccggaagtgaaagtgaattctattgcgccatcgctgatcctgtttaatgaacatgatgatgccgaatatcgacaacaggcgctgaataaatcactgatgaaaaccgcgcctggcgagaaagaagtgatcgacctggtcgattacttacttaccagttgctttgtcaccggacgcagtttcccacttgatggcggtcgtcatctgcgttaatgcagctttatccagcatataatcaacacccatgcgcttatcccccaacacgcaacagaaccaacaaaagcggcgggcaagcgcatcattccggtgaaataccacagcgacaccaggtaaacaaaatagggaataatcgaccacatactaaaaatgatggttgcgcgtaaggcttcaatgccgcgttcgctggcaacaatataatgcgcgataagcgcaaaggtcgggaaaagtggaatcagcccggcgatataataatttttcgtttttgctaaaacaccaatcaacagcactaccagcgcaccgagcgcggctttgattaccagccccatctttttaccttaacacttccataacaagtcatcagtagaatacctgatgaaaacttgtttagaaacgattgatagtaagtaaaaacagcgcggtgtattgtgacgtttttatatctaccgtgaatgttatgaacactatcgtatttgtggaagatgatgcggaagtcggttcactgattgccgcgtacctggcaaaacatgatatgcaggttaccgtagagccgcgcggcgaccaggccgaagaaaccattttgcgagaaaatccggatttggtgttactcgacatcatgctaccaggcaaggacggcatgaccatttgtcgtgatttacgcgcaaagtggtctggaccgattgttcttctaacctctctcgatagcgatatgaaccacatcctggcactggaaatgggtgcctgcgactatattctcaaaacgacgccccctgctgttttgctagcgcgtttacgtttgcatttgcgtcagaatgagcaagccacactgaccaaaggtcttcaggaaacgtctctgactccctacaaagccctgcatttcggcacgttgaccatcgatcccatcaaccgcgtagtcaccctggctaacactgaaatctcgctctcgacagctgatttcgaattattgtgggaattagctacccatgccgggcaaatcatggaccgcgatgcattgctgaaaaatttacgcggcgtcagttatgacggactggatcgtagcgtggacgtggctatttcgcggttaagaaaaaaactgctcgataacgccgcagaaccttatcgcattaaaactgtgcgtaacaaaggctatctttttgcgcctcatgcatgggaataagcgatgaaaaaactgtttatccagttttacctgttattgtttgtctgcttccttgtgatgtctctgctggttgggctggtgtacaaatttaccgccgaacgcgcgggcaaacagtcgctggatgatttgatgaacagttcgctgtatctgatgcgcagcgaattgcgtgagatccccccacacgactggggtaaaactctgaaagagatggatttaaatctctctttcgatctgcgtgtcgagccactgagtaaataccatcttgatgatatttccatgcaccgactgcgtggcggcgaaattgtcgccctggacgatcagtacacgtttttgcagcgtatcccgcgcagccactacgtgctggcagttggtcctgttccttatctttattatctccatcagatgcgattgctggatatcgccctgatcgcttttattgctatttccctcgcctttccggtgtttatctggatgcgtccgcactggcaggatatgttaaaactggaagcagcggcgcaacgatttggcgatgggcatctcaatgaacgtatccactttgatgagggttcgagctttgaacgacttggcgtcgcatttaaccagatggcggacaatatcaacgccttaattgccagcaaaaaacagcttattgacggtatcgctcacgaactgcgaacaccgttagtgcgcctgcgttatcgactggagatgagcgataacctgagcgccgccgaatcccaggcgttgaatcgtgatatcagtcaacttgaagctttaattgaagagctgctgacttatgcccgactcgatcgcccacaaaacgagcttcatcttagcgaaccagacctgccgttgtggctgtcaacgcatctggcagatattcaggcagtaacgcccgataaaacggtacggataaaaacgctcgtgcaaggccattatgcggcgttggatatgcgcttaatggagcgcgtgctggataatttgctcaataacgccctgcggtactgccattcaacggttgaaaccagcctgctactgtcggggaatagagcgacattaattgttgaggatgatggcccagggattgccccagaaaaccgcgaacatatctttgaaccttttgttcgcctcgatcccagccgggatcgctcaaccggcggctgcgggctggggctggcaattgtccactctatagcactggcaatgggcggtacggttaattgtgacaccagcgaactgggtggtgcccgcttctcgtttagctggccgttatggcataacatcccgcaatttacctctgcctgacactacgcgcacgatggtcaagtcaccacgactgtgctataaaataagtatgttgtaactaaagtggttaatattatggcgcgttacgatctcgtagaccgactcaacactacctttcgccagatggaacaagagctggctatatttgccgctcatcttgagcaacacaagctattggttgcccgcgtgttctctttgccggaggtaaaaaaagaggatgagcataatccgcttaatcgtattgaggtaaaacaacatctcggcaacgacgcgcagtcgctggcgttgcgtcatttccgccatttatttattcaacaacagtccgaaaatcgcagcagcaaggccgctgtccgtctgcctggcgtgttgtgttaccaggtcgataacctttcgcaagcagcgttggtcagtcatattcagcacatcaataaactcaagaccacgttcgagcatatcgtcacggttgaatcagaactccccaccgcggcacgttttgaatgggtgcatcgtcatttgccggggctgatcacccttaatgcttaccgcacgctcaccgttctgcacgaccccgccactttacgctttggttgggctaataaacatatcattaagaatttacatcgtgatgaagtcctggcacagctggaaaaaagcctgaaatcaccacgcagtgtcgcaccgtggacgcgcgaggagtggcaaagaaaactggagcgagagtatcaggatatcgctgccctgccacagaacgcgaagttaaaaatcaaacgtccggtgaaggtgcagccgattgcccgcgtctggtacaaaggagatcaaaaacaagtccaacacgcctgccctacaccactgattgcactgattaatcgggataatggcgcgggcgtgccggacgttggtgagttgttaaattacgatgccgacaatgtgcagcaccgttataaacctcaggcgcagccgcttcgtttgatcattccacggctgcacctgtatgttgcagattaacgcccggctttcatactgccgaccatctgttctggccgtacccagctgtcaaactcggcttcgctaagataccccagcgcaagggccgcagcttttaaggtcagcccttctttatgcgcttttttggcgatctcggcggctttgtcataaccaatgtgggtgttaagcgcagtcaccagcatcagcgattcattgagtaattgattgattcgctcacgattcggttcaatacccactgcgcagtgtttgttaaaactttccatgccatctgccagcaagcgcaccgattgcaggaaattgtggatcaccattggacggaagacgttcagttcaaagttaccggaagcgccccccatgttgatcgccacgtcgttccccatcacctgacagcagagcatggttaatgcctcacactgtgttgggttcactttccccggcatgattgagctgcccggctcattttccgggattgagatttcaccaattccgcagcgcgggccagaggccagccagcggacatcattggcgattttcatcagtgacgcagccaaccctttcaacgcgccgtgcgcctgaaccagggcatcacaggtcgccagcgcttcaaatttgttcggcgcggtaacaaacggtgcacaggtaatgactgccagttcatctgctacgcgacgcgcatactccggatgggtatttagtccagtacccaccgctgtaccgccaagagccagttccgctacgtgaggcaggctgtattcgatatgtttgagattatgctcgagcatcgctacccagccggaaatctcctgccccagcgttaacggcgtggcatcctgcaagtgagtacgaccaattttgacgatatcggcaaaagcacgggatttctcattcagtgtctgtgtcagggttttaagctgaggaatgagttgcttgcgcagcgccagcagcgccgcaacgtgcatcgccgtcggaaagacatcgttggaactttggcttttgttcacgtcgtcgttagggtgaactttacgttccatcccgcgcacaccgccgagtaattcactggcccggttagccagcacttcgttcatgttcatgttactttgcgtgccggagccggtctgccagatagccagcgggaattcgtcgtcatgctgtcctgccagtacttcatccgccgcctgacgaatggcgctcgctttctcttcagacaacaagcctaaatcttcattaacttttgccgctgcacgcttggttagcgccagcgcatgaatcagtgaggtgggcattttctccgtcgaaatgcggaaatgctccagcgagcgttgagtttgtgcgccccacagcttatctgccgggacatcaatcgcccccatcgaatctttttcgctgcgtactgtattcatgacctgctcctcacctgattaattttttctttctgttttgctttcgttaagcaacttttagctcacttattatttaccatttgataacaaatgtttggtctttcgtgccatgtaaaaaaaccgccccgaagggcggctctgtttatttcacacagcgggtgcattgtgtgagttgtatctgctggaagaagtcatttcctttatcatccacaaggataaacgccgggaaatcttccacttcaattttccagatggcttccattcccagttccggatattcaacacattccaggctcttaatacttccctgcgccaatacagcggccggaccaccgatactgccaaggtagaagccgccgtgttttttacaggcatccgtcacctgctggctgcggttgcctttcgccagcatgatcatacttccgccctgcgcttgcagttgatcgacataagaatccatccgtccggcggtcgttgggccaagagaaccggaggcataaccttccggcgttttggccggacccgcgtagtaaatcggatgatctttgatgtactgcggcagcccttcaccgttatccatccgctctttcagtttggcgtgagcaatatcacgaccgacgataatcgtgccgttaagcgataagcgtgtagaaacgggatactgcgacaactgtgcgaggatctctttcatcggacggttaaggtcaacgcgcaccgcttcgccttctcccgctttgcgcagctcttccgggatatatttgcctggattatgttccagtttttcgatccagatcccctgacggttgatcttcgctttgatattacggtcagcagagcaggagacgcccataccgaccgggcaggatgcgccgtgacgtggcaggcgaatcacgcggatgtcgtgagcgaagtatttaccaccaaactgcgcacccagaccaagattttgcgcttcgatcagcaattctttttccagttccacatcgcggaacgcctgaccgtgctcattcccttccgttggcagttcatcatagtatttcgcggaagccagtttcaccgttttaaggttcgtttctgcagaagttccaccaataacgaacgcaatatgatacggaggacaggccgccgtacccagcgtgcgcatcttctcaaccaggtaatttttcagtttccccggcgtcagtaacgctttggtttcctgatagagatacgtcttgtttgccgaaccaccacctttggcgatacagaggaatttgtattcgtcgccatcaacggcataaagatcgatctgcgctggcagattggtgccggtattcacttctttatacatatccagcggcgcgttttgcgagtagcgcagattatcttcgatataagtgttatagacaccgcgcgccagcgccgcttcatcaccaccaccggtccatacacgctgcccttttttaccaacaataatcgcggtgccggtatcctgacaggttggcagaacgcctttcgccgcgatgtcggagttacgcaggaattgcagcgccacatatttatcattttcgctggcctccgggtcacgcagaatgtcggccacctgttgttggtgcgccggacgcagcatgaacgacgcatcatgaaacgcctggcgcgccaacagagttaacgcttcgggtgcgactttcaaaatctcctgcccttcaaattcagatacgctaacgtgttcgctggttagcaggtaatactcagtatcatcttttttgagtggaaaaggagcctgataatgaaagggtttgtttgacattgttctctcacttactgcctggtttggttatgctctgggcgggtgttccgttgccctgttaaaagcgagtaacaatatcctacacacttttttaacaaaaactgagactagtacgactttttgcggctccaggttacttcccgtaggattcttgctttaatagtgggattaatttccacattaaaacagggattgatcatgcaaaaactcattaactcagtgcaaaactatgcctggggcagcaaaacggcgttgactgaactttatggtatggaaaatccgtccagccagccgatggccgagctgtggatgggcgcacatccgaaaagcagttcacgagtgcagaatgccgccggagatatcgtttcactgcgtgatgtgattgagagtgataaatcgactctgctcggagaggccgttgccaaacgctttggcgaactgcctttcctgttcaaagtattatgcgcagcacagccactctccattcaggttcatccaaacaaacacaattctgaaatcggttttgccaaagaaaatgccgcaggtatcccgatggatgccgccgagcgtaactataaagatcctaaccacaagccggagctggtttttgcgctgacgcctttccttgcgatgaacgcgtttcgtgaattttccgagattgtctccctactccagccggtcgcaggtgcacatccggcgattgctcactttttacaacagcctgatgccgaacgtttaagcgaactgttcgccagcctgttgaatatgcagggtgaagaaaaatcccgcgcgctggcgattttaaaatcggccctcgatagccagcagggtgaaccgtggcaaacgattcgtttaatttctgaattttacccggaagacagcggtctgttctccccgctattgctgaatgtggtgaaattgaaccctggcgaagcgatgttcctgttcgctgaaacaccgcacgcttacctgcaaggcgtggcgctggaagtgatggcaaactccgataacgtgctgcgtgcgggtctgacgcctaaatacattgatattccggaactggttgccaatgtgaaattcgaagccaaaccggctaaccagttgttgacccagccggtgaaacaaggtgcagaactggacttcccgattccagtggatgattttgccttctcgctgcatgaccttagtgataaagaaaccaccattagccagcagagtgccgccattttgttctgcgtcgaaggcgatgcaacgttgtggaaaggttctcagcagttacagcttaaaccgggtgaatcagcgtttattgccgccaacgaatcaccggtgactgtcaaaggccacggccgtttagcgcgtgtttacaacaagctgtaagagcttactgaaaaaattaacatctcttgctaagcttattaaaggcttataacaccttcaggcggccagtccgcctgatttcattttatggataatcattatgaataaatcgctggtagcggtaggcgtcattgttgcgctaggcgtagtctggacaggcggcgcatggtatacaggcaagaagattgaaacccatctcgaagacatggtcgcgcaggcgaacgcgcaactcaaactgacagctcctgaatccaacctggaagtgagttatcaaaactatcatcgcggcgtattcagcagccagttgcaactgttggtgaaacccattgccgggaaagaaaatccgtggattaaaagcggtcagagcgtcatcttcaacgaatcggttgatcatggtcccttcccgcttgcccagcttaaaaaactgaacctgatcccgtcgatggcatcaattcaaaccacgctggttaataacgaagtaagcaaaccactgtttgatatggcaaaaggtgaaacgccttttgagattaactcgcgcattggttacagcggtgattccagttccgatatttcgctcaagccactgaattacgagcaaaaggatgaaaaagtcgcctttagcggcggcgagttccagttaaatgctgacagagacggcaaagccatctccctttccggggaggcgcaaagtggtcggatagacgcagttaacgaatacaaccagaaagtgcagttgacctttaataatctgaaaaccgacggttccagcacgctggcaagttttggtgagcgtgtaggaaatcaaaaactgtcactggaaaaaatgaccatttcagtggaaggcaaagaactggcactgctggaaggcatggagatcagcggtaaatcggatctggtcaatgacggtaaaacgatcaatagccaactggattactcgctaaacagcctgaaggtacagaatcaggatctgggcagcggcaagctgactttaaaagtcggccagattgatggtgaagcctggcatcagtttagccagcaatataacgcgcaaactcaggcgctgctggcacagccagaaattgccaacaaccccgaactttatcaggagaaagtgacggaagccttctttagcgccctgccgctgatgctgaaaggcgatccggtgattactatcgcgccgctaagctggaaaaacagtcagggtgaaagtgccctgaatctgtcgctgttcctgaaagatccggcaacgactaaagaagcgccgcaaacgctggcgcaggaagtagatcgttcggttaaatctctggatgcgaaactgaccattccggtggatatggcaactgagtttatgactcaggtagcgaagctggaaggttatcaggaagatcaagcgaaaaaactggcgaaacagcaagttgaaggtgcatcagcaatggggcagatgttccgtctgaccaccttgcaggacaataccatcaccaccagcctgcaatatgctaacggtcagataacgttaaatgggcagaaaatgtcgttagaagattttgttggcatgtttgcgatgccagctcttaacgttccggctgtaccggcaattccgcagcagtaattcacggccaaaacgccggagaattttcactccggcgttttcatctgaaaacaaaccagagattgcctgatgcgctacgcttatcaggcctaccttttcctgcaacactttgaatttatgagtttttgtaggctggataaggcgtttacgccgcatccggcataaaaaacgcgcactttgtcaacaatctgaaacgccggagatttttctctccggcgttattttttacttcagcataaagtcatactgaatactcattttcacatcccagtaattcaggcgatcgcccagcgtactgccatcgcgcttttcccgccctttatcggcagcaagaaagaaattcatcccttgtaacggcccttcgctgacccgatagttcataccacctaagatacccgtgccttcaatccgcacatctcgtttactggattcatagccgcgagtcacaatcggtgcaaatgtcagcgtaaattgcggcgttaaacgatagttgacgcccaattgccaggactgcattccttcacggttacgatcaagacttaatgaaaagggatagccaatgtcggtatccaccacggcaccattcattgcatggcgcaaataaccaccactgccaaatacacttccccacggcgcattccaggtcaattgtccactaaccaacgccgtttcattgggctggctggtattacgacttaaaccttcgagctgcgcgtaaaagccgagcaactcccctttcaacgtataattcgggtcgagcggtatgcttttctcgagaatactttgtatctgattggaaacatctttctgtaccgatgcccccagagaatagcgactggtatcatcatgccaactggcggctaaaaaagaacgtgcgcgatgtttatcgtattttcccgtctggctgttatacaccccttcatcacgaataccggttgttgaatcagtccataaaaatactcgtgaacgccacattccccacagatcaatatttggtgttaaagcccaataacctaatgctccttcagaaactgtcggtaatgtacgttgcgaactgccagccattaacggaatacgataaggtaagctaccataactataatccgtcccgaagcgacctaatttaagcaggctattttcactgggttttatttttactgcccccagggcaaagccaaaacttttatcaccatcaagataccaccgggtactcatatcagcacgagcacctaatttataaacataatacgccccgccttcaacgccaataatattggaataataaccactattgaaatcgagcaatcctccctgtacccatgcgtaaatatctcttcccgcgccagcactgggcttatccgccctgcgcaattcgtttttcagtctgatgcgtagtcccgcttcatcgtcagccagttgcgccgcataagcagaggtaaggccagaggcagccgtcaggcaaataacggccatggccactatttttctcatagttgcacctttgatgttctgattatttttattgaatattaattagtgatatcgctgattaattgctgctgcacttttttacgattatcaatttcaaccacgatttctttgaattttttatccgtgagcggataaaaccagataataacgaatgccagtagcataaatccgcaaggtactaaggcaattgatgtgcggatgcccataataacttccggcgtttgcacctgattggcgatatatccgcttaaccccaaaataaaggcaggaattgaacctccgattgcctgaccgcatttacgggtaaatgagaatagtgaataggtgagcccttcaattcgcacgccggtcaggtattcaccgtattctacggtatcagcttccagcgcccacatcacggtcatggtaacgccctgaccaattgaagcgatggccaacgcaaccaacgccaccggcagtgaccagacggaaacccagaagaacagcagataaccgcaggttcccagcaaagcgccaatcaggaaggtattctttttaccgatcctcgcgaccatccccggcaccagcggtgccgatgccacagtaccaaccaggttttgcaccagtaccagcacagtgaacagcccggtatcatttaacacatagcgcacgtagaacaacgacgaggcgctgaccgcaaaggtcgaaatcagcacacacagcgcaccgatgcacaacataaacagcgggcgattccgtttcagggtttgcagactgatattcaatgacggctgcgcaacgatacgtaccacattctcacgcgtcgatttgaagcagatgaagtaaagcaccattccggcaatcgccagcacaattgtccagaaatggtataccgacaccatctcttccgggctggagttcttaatgctcggtcctatcagaaatgccaggcagacaaaggtcaatgaagcggcaatcccacgagccgcgcccagacgggcgcgggattgtggttgttgggtcatcgcggtagcaagtgaaccataaggaatattcaccaggctgtagcaaagcccgaggcccatgtaggtcaaatatgcatacaccactttgctaccatggctccagtcggtcagcacccagaataccagcacgctgaagatcattaacggcgcagtaccgaagagtaaaaacgggcggaattttccccagcgggtattcacactgtccaccactcgtccggcaaagacgtcggcgaaggcatcgaatacccgcaccagtaacagcatggtgcccgccgcagcggcaccgacgccagcgacgtcggtgtagtaactcaacaggaagagcgcccccattgcgaaggcgaagttattggcgacgtcaccgaggctgtagccgacgatggtgcgccaggagagttgttgattcattgtttgcctccctgctgcggtttttcaccgaagttcatgccagtccagcgtttttgcagcagaaaagccgccgacttcggtttgcggtcgcgagtgaagatccctttcttgttaccgccaacgcgcaatatgccttgcgaggtcgcaaaatcggcgaaattccatacctgttcaccgacgacggcgctgacgcgatcaaagacgcggtgatacatatccagccatgcacactgatactcttcactccacatgtcggtgtacattgagtgcagcccggctaacgtatccacgccgtattcggtgatgataatcggctgatgcagtttctcctgccaggccagaagttctttttccagtaccttctctgccgtttccaaatcgccgctttggacataccatccgtaataacggttcaggcacagcacatcaaagagatcgctgatggtatcggtgtgagcgtcgcagaacattacattgacgcaggtgatcggacgcgtcgggtcgagtttacgcgttgcttccgccagtggcgcgaaatattcccgtgcaccttgcggacgggtatccggttcgttggcaatactccacatcaccacgcttgggtggtttttgtcacgcgctatcagctctttaatcgcctgtaagtgcgcttgctgagtttccccgttgactgcctcttcgctgtacagttctttcggcttgttgcccgcttcgaaaccaatgcctaaagagaggttaaagccgacagcagcagtttcatcaatcaccacgatgccatgttcatctgcccagtcgagcatctcttcagcgtaagggtaatgcgaggtacggtaggagttggccccaatccagtccattaatgcgtggtcgtgcaccatcagcacgttatcgaatcctttgccacgcaagtccgcatcttcatgacgaccaaagccagtaaagtagaacggtttgtggttaatcaggaactgttcgcccttcactgccactgaccggatgccgacgcgaagcgggtagatatcacactctgtctggcttttggctgtgacgcacagttcatagagataaccttcacccggttgccagaggtgcggattcaccacttgcaaagtcccgctagtgccttgtccagttgcaaccacctgttgatccgcatcacgcagttcaacgctgacatcaccattggccaccacctgccagtcaacagacgcgtggttacagtcttgcgcgacatgcgtcaccacggtgatatcgtccacccaggtgttcggcgtggtgtagagcattacgctgcgatggatcccggcatagttaaagaaatcatggaagtaagactgctttttcttgccgttttcgtcggtaatcaccattcccggcgggatagtctgccagttcagttcgttgttcacacaaacggtgatacgtacacttttcccggcaataacatacggcgtgacatcggcttcaaatggcgtatagccgccctgatgctccatcacttcctgattattgacccacactttgccgtaatgagtgaccgcatcgaaacgcagcacgatacgctggcctgcccaacctttcggtataaagacttcgcgctgataccagacgttgcccgcataattacgaatatctgcatcggcgaactgatcgttaaaactgcctggcacagcaattgcccggctttcttgtaacgcgctttcccaccaacgctgatcaattccacagttttcgcgatccagactgaatgcccacaggccgtcgagttttttgatttcacgggttggggtttctacaggacgtaacataagggactcctcattaagataataatactggtcaacctttaatctgattagttaaccaattctgtgttgcacacagttatctgtgagaaacccatggaagagaaatggaaataaaaagaactgacaccgcgatcaaaaaaccaaaaactgcaatacccacagcgtgatatagatcgcattaatctttaaaacagcgttgacagaagccataaaataagcaaccgaacgttcgttcgagcgtattgggaacgataaactctcatgacatatggctacagtgaatattttggggggaattctccgaagccgggaaggataatttttgcacagagaaattacgatatgaaacgcgggcacagttatcaccagcccgccgaaaaagagagagaatcaggatgcggttaagataccgccaatcatcgcgcgtaatccctgagcaaacgacgcttcacgcgccaggtcttccgcttcgatatcggccagtacaccgtaggtcagatccagcagtaaacgtgaagtcattgccgtgttgatgtctgggcttatctcgcctttttgctgggcatcacgcatccgctgggcaacaaattccgtgatcgtcatatgcttatttttaagcatggcggcgacctgtgggttacgcatcccttccgccataatttcaaccaccagcgcccgttgtccaaaggcttcatgggtgagagagacaatggactcgaccatatagtcaacgaaatgaatcccttcaatcggttcccggaaacgggccagcgccctctcctggtcctgtaagataatcgcctgaatcaaggcttctttggagatgaaatggtgatagagcgtcccgggactaatggcgcaagatttacagatggctttcatcgaggcactgtgaaatccattttctgaaaaaatctctctggcagcattgaggatccgggtccgtgtcggttgtgcttcagtctgcatgttatccatcattaaaccattatagttagcgtgaataactagtttaccgcgttgtcaggtgagcgcctatcattgctgttgaatagtgcgaaggcacactctattcgtatacttttcactctgaaattggttaaccaatagccgtgatttggctgccagttatttagcagagacgttgatgagtttatcccggtaaacaacacgcacggttgtttaccggtccgttagtgtattaattgagctcctgtaccccaccaccggagacggtgagaatttgtccgcttacccagctcgcagcaggcgagcaaaggaacagcgctgcgttagcaatatcttgcggttggcccagacgtctgatcggcgtgtgctgtaacattttttgttcaatttctggtgtaataacggatttcagggcatcggttaatattgcccccggcgcaatgccatttacccgaatatttttttcacccaggtcaaacgccatatttctgaccagatgactggccgcagctttagatgatgcataggaagtcatgtttatatttttattttctgccgccatagaagtgatggtcagaataacgccaccgccatttttttccatttctggcgcaacaagttgtgacagatggaaaaaagaaaacacattcagttcataagcacggcgaaaatccgccattggcatatcaaacggtttaggtccaccgccaccggcgttgttaaccagaatatcaactttacccagcttactgatagcaaagtctgccagtgcagagagttcctgttcggaagtaatatcacaacggcaggcaaatgcctgaccacccagttgttgaatttcgtctacaacatggttagctgcgtcggcgttaatatcactgaccaccacagatgcgccagctgtcgcgaatgtaatggcgatttctttaccaatacctgcacccgcacctgtgatgatggcgcattttccgtcgagtctcaggttgtcagaattaaacacataaacctcctgtgaacttcagtaaaaataaaaggcaccgcctgtgtgccacattttttatcattaaccttgaggaaaggacactaccaggtatagcagataaagagaggattatttcgctgcaatgagccgggcgggaataataagattgcgtgaatgcgtctcttcatgggtgattttttgcatcatgcgatccgcaagtgtgataccaagttcccgcgctggcgtgctggcccaggtaacaggtatatcatcaagtgtggttggtgtcgcatcggtaaatgccgccagcgaaacctgttgctcaaagtaacgatcgactccgctttccccgctttgccgccctgctttgagcaaaccaaaccatgcccccatcgcaatagtttcgttatagcaaaccacggcactgatggtcgggttatgacgtaaaagcgccgtgatagcttccgcggcttgcttctggctggaagtgcactccaacacccaatcgctatgaaacggcaggccaaattttagtagagttgcacaatagcccccaacccgttctgcacgggttaatgaggaactttgccctcccagccaggcgatccgctgatgcccattgcgaatgagatgctccgtcaacaactgtgcagcctgcatgttgtccgggcgaaccgtatcaacatcatcaagataactggcacgggaagcgaaaatcaccgggatagctttttcttctgccatccgtcgcaggtcatcgctacttcctgcagctccggcaattaccacaccatcgacaccctgattcagtaacagtgaaaaccgctgtgccagctgctcaccgtctttaccgccgtgaagcaaaaaaaccatccgtccctgcgcttccagagcttccgtcaatccggccgtcaattcggcgtaaaacggcgcagataaatcacggacgatcaaaccaatgacgccgctttgcccgccgcgcagcgccgacgcctggcgattgcgcacaaatcccagctcttcaatggcggcgttaacgcgttctcctgtggcggtagagattcgccctttgccactaagcaccagcgaaacggtacttaccgacacgcccgcagccagcgcaacatcatgaatggttatttttttggcggtagccatgcagatgacctactccctgattatgtgacagataaaacgttttaccttttatttatcttatacccgctattatcgttgcgtaatgtgatttatgcctcactaaaatttgataaaacgttttatcttctcgcgcaatttactgaatccagattgttctctacgaggagtcgttttatgacggcgaaaacagcaccgaaagtcacgctgtgggagttcttccagcagttaggcaaaaccttcatgttacccgtggcattattgtcgttctgcggcattatgctcggcattggtagttctcttagcagccatgatgtcataaccctgatcccggtcctgggcaaccccgtgttgcaggctatctttacctggatgagtaagattggctcgtttgcttttagtttcctgcctgtcatgttctgtatcgccatcccgctgggcctggcacgcgaaaataaaggcgtagcggcattcgctggcttcatcggttatgcggtaatgaacctcgcggtaaacttctggttgaccaataaaggcattctgccaaccacggatgccgcggttctgaaagccaataacatccagagcattcttgggatccagtcgatcgataccgggatcctcggtgcggtgatcgccggtattatcgtctggatgctgcatgagcgtttccataatatccgcctgccggatgcgctggcattcttcggcggtacgcgcttcgtaccaattatctcctcgctggtgatgggccttgtcggcctggtgattccattagtctggccgattttcgccatgggtattagcggcttgggccatatgataaacagcgcgggtgatttcggaccgatgctgtttggtaccggtgaacgtctgctgttgccgtttggtctgcatcacattctggtggcattaattcgctttaccgacgcaggcggcacgcaggaagtctgcggtcaaaccgtcagcggcgcactgaccatcttccaggcgcaattgagttgcccgaccactcacggtttttctgaaagcgccacgcgtttcctttcgcaaggtaaaatgcctgcgtttctcggcggtctgccaggtgcagcgttagctatgtatcactgcgcgcgcccggaaaatcgccataaaattaaaggtctgctgatttctggcctgatcgcctgcgtcgttggcggcactaccgaaccgctggaattcctgttcctgttcgtagcgccagttctgtatgtcatccacgcgctgttaaccggcctcggcttcaccgtcatgtctgtgctcggcgtcaccatcggtaataccgacggcaatatcatcgacttcgtggtgttcggtattttgcatggtctgtcaaccaagtggtacatggtgccagtggtggcggcaatctggtttgtcgtttactacgtcatcttccgtttcgctatcacccgcttcaatctgaaaaccccggggcgcgatagcgaagttgccagctcaatcgaaaaagccgttgccggtgcgccgggtaaatcaggttacaacgttcctgcaatcctcgaagcattaggcggtgccgacaatattgtcagcctcgataactgcattacccgtctgcgtttgtctgtgaaagatatgtcgcttgttaatgtgcaggcactgaaggacaatcgggcaattggcgtagtacaacttaatcaacataacctgcaggttgttatcgggccacaagttcagtcagtaaaagatgaaatggccggtctgatgcatactgtccaggcataaggataagatatgttcgatttttcaaaggtcgtggatcgtcatggcacatggtgtacacagtgggattatgtcgctgaccgtttcggcactgctgacctgttaccgttcacgatttcagacatggattttgccactgccccctgcattatcgaggcgctgaatcagcgcctgatgcacggcgtatttggctacagccgctggaaaaacgatgagtttctcgcggctattgcccactggttttccacccagcattacaccgccatcgattctcagacggtggtgtatggcccttctgtcatctatatggtttcagaactgattcgtcagtggtctgaaacaggtgaaggcgtggtgatccacacacccgcctatgacgcattttacaaggccattgaaggtaaccagcgcacagtaatgcccgttgctttagagaagcaggctgatggttggttttgcgatatgggcaagttggaagccgtgttggcgaaaccagaatgtaaaattatgctcctgtgtagcccacagaatcctaccgggaaagtgtggacgtgcgatgagctggagatcatggctgacctgtgcgagcgtcatggtgtgcgggttatttccgatgaaatccatatggatatggtttggggcgagcagccgcatattccctggagtaatgtggctcgcggagactgggcgttgctaacgtcgggctcgaaaagtttcaatattcccgccctgaccggtgcttacgggattatagaaaatagcagtagccgcgatgcctatttatcggcactgaaaggccgtgatgggctttcttccccttcggtactggcgttaactgcccatatcgccgcctatcagcaaggcgcgccgtggctggatgccttacgcatctatctgaaagataacctgacgtatatcgcagataaaatgaacgccgcgtttcctgaactcaactggcagatcccacaatccacttatctggcatggcttgatttacgtccgttgaatattgacgacaacgcgttgcaaaaagcacttatcgaacaagaaaaagtcgcgatcatgccggggtatacctacggtgaagaaggtcgtggttttgtccgtctcaatgccggctgcccacgttcgaaactggaaaaaggtgtggctggattaattaacgccatccgcgctgttcgttaaccccaattgcgcaacgtaaaaaatcgttgcgcaatcgtggatttttaccctgctttgtttttataatggtgcgcacttttatatccagaaaaagagtgcgaccatgattgataccaccctgccattaactgatatccatcgccaccttgatggcaacattcgtccccagaccattcttgaacttggccgccagtataatatctcgcttcctgcacaatccctggaaacactgattccccacgttcaggtcattgccaacgaacccgatctggtgagctttctgaccaaacttgactggggcgttaaagttctcgcctctcttgatgcctgtcgccgcgtggcatttgaaaacattgaagatgcagcccgtcacggcctgcactatgtcgagctgcgtttttcaccaggctacatggcaatggcacatcagctgcctgtagcgggtgttgtcgaagcggtgatcgatggcgtacgtgaaggttgccgcacctttggtgtgcaggcgaagcttatcggcattatgagccggaccttcggcgaagccgcctgtcagcaagagctggaggcctttttagcccaccgtgaccagattaccgcacttgatttagccggtgatgaacttggtttcccgggaagtctgttcctttctcacttcaaccgcgcgcgtgatgcgggctggcatattaccgtccatgcaggcgaagctgccgggccggaaagcatctggcaggcgattcgtgaactgggtgcggagcgtattggacatggcgtaaaagccattgaagatcgggcgctgatggattttctcgccgagcaacaaattggtattgaatcctgtctgacctccaatattcagaccagcaccgtagcagagctggctgcacatccgctgaaaacgttccttgagcatggcattcgtgccagcattaacactgacgatcccggcgtacagggagtggatatcattcacgaatataccgttgccgcgccagctgctgggttatcccgcgagcaaatccgccaggcacagattaatggtctggaaatggctttcctcagcgctgaggaaaaacgcgcactgcgagaaaaagtcgccgcgaagtaacaaaatggatggtgcaaatgcaccatccatttttcatgcaaggcacaaagtcgcgcgatgtttggcggattcgatgcccagctcaatcaactccattacctggattgcctggcttgccggaaccggattttcaccatcgccatttaacgcatcacgaatagccgcatagtaagccggataattcccaggcaccgtcaacagcgtttcttcgacacgttcctcaccttccacgcgggtaagtacgccatcacgcatatcgtagccccagtcttcctgcggtagacgctcgccatttttcagacgttcttcctgtggatcgaggccatatttcacataactgcctcgggatccatgcacgatataccgtgctgactcagcggctgccagcatggtaccgtgtaaaatgactcgccgctgtggataggacaagatggcgtggaaataatcggtcgactgcgctccgggccgtaactgtgccaaatctaccgtcatgctgaccggtaaaccaaaaagcgtaatggcctgatcaagaagatgtggtgctaaatcgtaccagataccgctgcctgggccgccctgttcacgccaacgatcgcgcacctgcggacggaagcggtcaaaatgagactcaaagtaagcaacttcacccagcacgccttccgcgagtaaaccttttagcgtcaagaaatcgctatcccagcgacggttatggaatacagacagcacacgccccaggctttttgccagcgcatccagctctcgcgcttgtgacagtgtcacggtaaagggtttatcaacgaccacatgtttacccgcctcaagcgccgctttggctaacgggaaatgggtatcgttgggtgtaggaatgacaatcaggtctatgttgggatcgttaaacagatgcttcggctcagagacaaccgtaaccgttggccagtcggcttttacttttgtttcatcactgctggagattaccgccagttcctgcccgggcgtgcccgcaatcaggggcgcatggaaggttttgctcgcataaccatacccaatcaacccaacacggatgttgtcgctcatgtcattgcctctcattgaagtatgatggctatttgacactatcctttacccacgctcaacagtttaataacctgccagcaataagggatgttgtttaacttaagtcaaaaaaatagcgaattttccaacgacaaaagctaaatatcgcaaaaacctcagtaaaaatcttgctggagctattattgctaagtaacatttaccccctgaagttaatggatcaatcaagagagatgtgggctgtaatgaatcgtcttattgaattaacaggttggatcgttcttgtcgtttcagtcattcttcttggcgtggcgagtcacattgacaactatcagccacctgaacagagtgcttcggtacaacacaagtaagctctgcacttgtggagcgacatgctgcccgtccgggtgcatgttttcacttgtcggatattaaaccaggaatttattatcttgttcgatgttgttggtgattgtcagggatagtaaagcgcgttactcttttcagagcagtttttcatccctgaatatttgccatcagcgcattcttattattgtaataacacaagcgttcacttttggtgaaattttatcatcactaataatacctacccctttggtattaattattttatggaccttttatgactgttcaggactacttattaaaatttcgcaaaatcagttcactcgaaagtctggaaaaactctacgaccatcttaattacaccctgacggacgatcaggaactgatcaatatgtatcgtgctgccgatcaccgtcgcgcagagctggtttctggcgggcgtttgtttgacctcggccaggtaccgaagtccgtctggcactatgtccaataaagaaagtagcgatcggttataaaagccttataataacgcccctaaaattagatttgcctgtttgcgtcgctattctggagaacctatgaccaccacaacgccacaacgtattggaggctggttgcttggcccgttggcctggcttttagtcgctctgttgagtacgacgctggcgttgttgctgtataccgctgcgttatcttctccgcaaacatttcaaacgctcggcggacaagcactgacgacacaaatcttatggggcgtttcttttattaccgctatcgccttgtggtattacacactgtggttgaccatcgctttctttaaacgtcggcgttgtgttcctaaacactatattatctggctgcttatttccgtattgctggcagtaaaagcattcgctttttcacccgtggaagatggcatagccgttcgccagttgctgtttactttgttggcaaccgcattgatcgtcccctatttcaaacgctcgtcgcgggtaaaagcgacgtttgtgaatccgtaataaccttacagttaacctgttgtcgcctgctctggattaacggataataggcggcttttttatttcaggccgaaaaatgactgactacctgttactgtttgtcggaactgtactggtcaataactttgtactggtcaagtttctcggtctctgtccgtttatgggggtttccaaaaaactggaaaccgcgatgggcatggggctggcaacaacgtttgtgatgacgctggcgtctatttgcgcctggcttatcgatacgtggattttgatcccacttaatctgatttacctgcgcaccctggcatttattctggtgattgctgtggtcgtgcagttcaccgagatggtggtgcgcaaaaccagcccggtgctttaccgtctgctggggatttttttgccgcttatcaccaccaactgtgcagtgctcggcgtggcgttgctgaatatcaatctcgggcacaatttcttgcagtcggcgctgtacggtttttccgccgctgtcggtttctcgctggtgatggtgctcttcgccgccatccgcgaacgccttgctgtggctgatgtcccggcaccttttcgcggtaatgccattgcgttaattaccgcaggtcttatgtctctggcctttatgggctttagtggtttggtgaagttgtaatgaatgctatctggattgccgttgccgccgtgagcctgctgggcctggcgtttggcgccattctgggttatgcctcccgccgttttgcggtggaagacgatccggtcgttgagaaaattgacgaaatcttaccgcagagccagtgtggtcagtgcggttatcccggctgtcgcccctacgcggaagccatcagctgtaacggtgaaaaaatcaaccgttgcgccccaggtggcgaagctgtgatgctaaaaattgccgagttgcttaatgtcgagccgcagccgctggatggcgaagcgcaagagataacgcctgcgcggatggtggcggttattgatgaaaataactgtattggctgcactaaatgtattcaggcgtgtccggtagacgccatcgttggcgctacccgtgccatgcatacggtaatgagtgatctctgtacgggctgcaatttatgtgttgatccgtgcccgacgcactgcatctcgttgcaaccggtcgcagaaacacctgactcctggaaatgggatctgaacaccattcccgtgcgtatcattcccgtggaacaccatgcttaagttattctctgcattcagaaaaaataaaatctgggatttcaacggcggcatccatccaccggagatgaaaacccagtccaacggtacacccctgcgccaggtacccctggcgcagcgttttgttattccactgaaacagcatattggcgctgaaggtgagttgtgcgttagcgtcggcgataaagtattgcgcggccagccgcttacccgtggtcgcggcaaaatgctgcctgttcacgcgcccacctcgggtaccgttacggctattgcgccccactctacggctcatccttcagctttagctgaattaagcgtgattattgatgccgatggtgaagactgctggatcccgcgcgacggctgggccgattatcgcactcgcagtcgcgaagagttaatcgagcgcatacatcagtttggtgttgccgggctgggcggtgcaggattcccgacaggcgttaaattgcagggtggcggagataagattgaaacgttgattatcaacgcggctgagtgcgagccgtacattaccgccgatgaccgtttgatgcaggattgcgcggctcaggtcgtagagggtattcgcattcttgcgcatattctgcagccacgcgaaattcttatcggcattgaagataacaaaccgcaggcgatttccatgctgcgcgcggtgctggcggactctaacgatatttctctgcgggtgattccaaccaaatatccttctggcggtgctaaacaattaacctacattctgaccgggaagcaggttccacatggcgggcgttcatccgatatcggcgtattaatgcaaaacgtcggcactgcttatgcagtgaaacgtgccgttattgatggcgagccgattaccgagcgtgttgtaaccctgactggcgaagcaatcgctcgcccgggcaacgtctgggcacggctggggacgccagtgcgtcatttattgaatgatgccggattctgcccctctgccgatcaaatggtgattatgggtggcccgctaatgggctttaccttgccatggctggatgtcccggtcgtaaagattaccaactgtctgttggctccctctgccaatgaacttggcgaaccacaggaagaacaaagctgcatccggtgtagcgcctgtgctgacgcctgccctgcggatcttttgccgcaacagttgtactggttcagcaaaggtcagcaacacgataaagctaccacgcataacattgctgattgcattgaatgtggggcttgcgcgtgggtttgcccgagcaatattcccctggtgcaatatttccgtcaggaaaaagctgaaattgcggctattcgtcaggaagaaaagcgcgccgcagaagccaaagcgcgtttcgaagcgcgccaggctcgtctggagcgcgaaaaagcggctcgccttgaacgacataagagcgcagccgttcaacctgcagccaaagataaagatgcgattgctgccgctctggcgcgggtgaaagagaaacaggcccaggctacacagcctattgtgattaaagcgggcgaacgcccggataacagtgcaattattgcagcacgggaagcccgtaaagcgcaagccagagcgaaacaggcagaactgcagcaaactaacgacgcagcaaccgttgctgatccacgtaaaactgccgttgaagcagctatcgcccgcgccaaagcgcgcaagctggaacagcaacaggctaatgcggaaccagaacaacaggtcgatccgcgcaaagccgccgtcgaagccgctattgcccgtgccaaagcgcgcaagctggaacagcaacaggctaatgcggaaccagaagaacaggtcgatccgcgcaaagccgccgtcgaagccgctattgcccgtgccaaagcacgcaagctggaacagcaacaggctaatgccgagccagaacaacaggtcgatccgcgcaaagccgccgtcgaagccgctattgcccgagccaaagcgcgcaaacgggaacagcaaccggctaatgcggagccagaagaacaggttgatccgcgcaaagctgccgtcgaagcggctattgcacgcgccaaagcacgcaagctggaacagcaacaggctaatgcggtaccagaagaacaggttgatccgcgcaaagcggcagttgccgcggctattgcccgcgctcaggccaaaaaagccgcccagcagaaggttgtaaacgaggactaaatggtattcagaatagctagctccccttatacccataaccagcgccagacatcgcgcattatgctgttggtgttgctcgcagccgtgccaggaatcgcagcgcaactgtggttttttggttggggtactctcgttcagatcctgttggcatcggttagtgctctgttagccgaagctctcgtactcaaactacgcaagcagtcggtagccgcaacgttgaaagataactcagcattgctgacaggcttattgctggcggtaagtattccccccctcgcgccatggtggatggtcgtgctgggtacggtgtttgcggtgatcatcgctaaacagttgtatggcggtctgggacaaaacccgtttaatccggcaatgattggttatgtggtcttactgatctccttccccgtgcagatgaccagctggttaccgccacatgaaattgcggtcaacatccctggttttatcgacgccatccaggttatttttagcggtcataccgccagtggtggtgatatgaacacactacgcttaggtattgatggcattagtcaggcgacaccgctggatacatttaaaacctctgtccgtgccggtcattcggttgaacagattatgcaatatccgatctacagcggtattctggcgggcgctggttggcaatgggtaaatctcgcctggctggctggcggcgtatggttgctatggcagaaagcgattcgctggcatattcccctcagcttcttagtaacgctggcgttatgcgcaatgttgggctggttgttctcaccagaaacactggcagcaccgcaaattcatctgctgtctggagcgaccatgctcggcgcattctttattttgactgacccggttaccgcttctacgaccaatcgtggtcgtcttattttcggcgcgcttgcgggcttattagtctggttgatccgcagtttcggcggctatcctgacggcgtggcttttgccgtcctgctggcgaacatcacggttcctctgatcgattactacacgcgtccgcgcgtctacggccatcgcaaagggtaaaccatgctgaaaactatccgaaaacacggcattacgttggcgctatttgcagcgggttcaacagggttaactgcggccatcaaccagatgaccaaaacgacgattgctgaacaggccagtctgcaacaaaaggcgttatttgatcaggtgctgccagccgaacgctataacaatgcgctggcacagagttgctatctggtaactgcgccagagttaggtaaaggtgagcatcgggtttacatcgccaaacaggatgacaaaccggtagccgccgttctggaagcaaccgcgccagatggctattccggtgcgattcagctgctggtgggagccgattttaacggcacggtacttggcacgcgcgtgacagagcaccacgaaacgccagggcttggcgataaaatcgaactgcgcctttctgactggatcacccattttgcgggtaaaaaaatcagtggtgcagatgatgcgcactgggcggtgaagaaagatggtggtgatttcgaccagttcaccggcgcgacgattactccccgcgcggtggttaatgcggtaaaacgcgccggattgtacgctcagacgttaccggcacaactttctcaacttcctgcctgtggagaataaagcgtgagcgaaattaaagacgttattgttcaggggttgtggaaaaacaactctgcgctggtccagttgctcggcctttgtcctctgttggcggtcacgtccactgccactaacgctctgggtttaggacttgcgactacgctggtactgacgctgaccaacctgaccatttcgacgctgcgtcactggacgccagccgagatccgcattcccatttacgtgatgatcatcgcctcggtggtcagcgctgtacagatgctgatcaacgcctacgcctttggcctgtatcaatcattagggatttttattccgctgattgtcactaactgtatcgttgtgggccgcgctgaagccttcgccgccaaaaaaggtccggcgctttcggcactggacggcttttcaattggtatgggcgcaacctgcgccatgttcgtgctgggttcactacgcgaaattatcggcaatggcacattgtttgacggtgcagatgcgctgttaggtagctgggcaaaagtattacgcgtggagattttccacaccgactcccctttcctgctggcgatgctgccaccaggtgcatttattggcctgggactgatgctggcaggaaaatacctgattgatgaaagaatgaaaaagcgccgtgctgaagcagctgcagaacgtgcattgccaaacggtgaaacagggaatgtctgatgaataaagcaaaacgcctggagatcctcactcgcctgcgtgagaacaatcctcatcccaccaccgagcttaatttcagttcgccttttgaattgctgattgccgtactgctttccgctcaggcgaccgatgtcagtgttaataaggcgacggcgaaactctacccggtggcgaatacgcctgcagcgatgcttgaactgggcgttgaaggggtgaaaacctatatcaaaacgattgggctttataacagcaaagcagaaaatatcatcaaaacctgccgtatcttgctggagcagcataatggcgaggttccggaagatcgtgctgcgcttgaagccctgcccggcgtaggtcgtaaaacagccaacgtcgtattaaacactgcattcggctggccgactattgctgtcgacacgcacattttccgcgtttgtaatcgtactcaatttgcgccggggaaaaacgtcgaacaggtagaagaaaagctactgaaagtggttccagcagagtttaaagtcgactgccaccattggttgatcctgcacgggcgttatacctgcattgcccgcaagccccgctgtggctcttgtattattgaagatctttgtgaatacaaagagaaagttgacatctgaagaaaaggggtaacaccgattaccccattgataacctttctttatcctcttttaaaacatctttttaacgtcaatgatgccattgcttagcgttatcatcaggtaatccgtttgcggataaccaaaaatgcaggttaattgtttttttaatagcgaaattttctattcattcgtgatcaagatcacgatgctgtcgcaatgtaaaaacattgcaagaatcaggttaaaatcatttaaatttacacacgcaacaaatattgacctacaaaacattacactggctatttttcagaaactggactatctcactagtaaaaacgctaaatagcagaacatatcgccgttaagccatcacccccctctcagtgcagtgaaaaaatctgccgttacgttttttgaaaaatttaacgctggataacatttcccggaatggttgaattccccgcctcagttatatgtaacagattattacaaaggacttgtctgaaagtgcaagatagtgaacattacctgccgtttcccctcccactataacaattgcgcgtatgttttttatacataacgcgagaaagcacccccgttaatatgggatgtaaaaaaagaggtaaaagtgtccactgcaaaccaaaaaccaactgaaagcgtcagtttgaacgctttcaaacaaccgaaggcgttctatctcatcttctcgattgagttatgggaacgttttggttattacggcctacaaggaattatggctgtttacctggttaaacaactgggtatgtctgaagcggattcaatcacccttttctcttcctttagtgccctggtttatggtctggtcgctatcggcggctggttaggtgacaaggtactgggtactaaacgcgtaattatgctcggcgctattgtgctggcgattggttatgctctggttgcctggtctggtcacgacgccggtatcgtttatatgggtatggcggctattgcggtcggtaacggcctgtttaaagctaacccgtcttctctgctttctacatgctatgagaaaaacgacccgcgtctggacggtgcattcaccatgtactacatgtccgtcaacatcggctctttcttctctatgattgctacgccgtggctggccgcgaaatacggctggagtgttgcgtttgcgttgagcgttgtaggcctgctgatcactatcgttaacttcgccttctgccaacgctgggttaaacagtacggttcaaaaccagacttcgagcctatcaactaccgtaacctgctgctgaccattattggtgttgtggcactgatcgctatcgccacctggctgctgcacaatcaggaagttgcgcgtatggcgctgggcgttgttgccttcggtatcgtggttatcttcggtaaagaagccttcgcgatgaaaggtgctgcgcgtcgtaaaatgatcgttgccttcatcctgatgctcgaagccattatcttcttcgtgctgtacagccagatgccaacgtcactgaacttctttgcgattcgtaacgttgagcactccattctgggtctggccgtagaacctgagcagtatcaggcactgaacccgttctggatcatcatcggtagtccgattctggccgctatctataacaagatgggcgataccctgccgatgccaaccaagtttgcaatcggcatggtgatgtgttctggtgcgttcctgattctgccgctgggtgcgaaattcgcgtctgacgctggtatcgtgtctgtaagctggctggtcgcaagctatggcctgcagagcatcggggaactgatgatctctggtctgggtctggcaatggttgctcaactcgttccgcagcgtctgatgggcttcattatgggtagctggttcctgaccactgccggtgcaaacctgattggtggttatgttgcgggtatgatggctgtgccggataacgttaccgatccgctgatgtcactggaagtctatggtcgcgtattcttgcagattggtgtcgctactgccgttattgcagtactgatgctgctgaccgcgccgaaactgcaccgcatgacgcaggatgacgctgcagacaaagcggcgaaagcagccgtagcgtaaaattcagggaaactcttttacaagccgctaacttttcgttagcggctttttttttgttcagcaacgcactaccatactttaaaccacagacaaaaggagttaccgatgaaattgttctacaaaccgggtgcctgctctctcgcttcccatatcaccctgcgtgagagcggaaaggattttaccctcgtcagtgtggatttaatgaaaaaacgtctcgaaaacggtgacgattactttgccgttaaccctaaggggcaggtgcctgcattgctgctggatgacggtactttgctgacggaaggcgtagcgattatgcagtatcttgccgacagcgtccccgaccgccagttgctggcaccggtaaacagtatttcccgctataaaaccatcgaatggctgaattacatcgccaccgagctgcataaaggtttcacacctctgtttcgccctgatacaccggaagagtacaaaccgacagttcgcgcgcagctggagaagaagctgcaatatgtgaacgaggcactgaaggatgagcactggatctgcgggcaaagatttacaattgctgatgcctatctgtttacggttctgcgctgggcatacgcggtgaaactgaatctggaagggttagagcacattgcagcatttatgcaacgtatggctgaacgtccggaagtacaagacgcgctgtcagcggaaggcttaaagtaatagccatcggcccacaggtcgttgtgggccgaaatgagatatttcagagctttgttgcgctgaagtaatgttctggtttggcaatacgatcctgagcagccaccacttgcagctcatattcctgcattgctttggtggtcaccatgatttcgtagactgcagcggtcacatgttccagcgcctcctgcagcgttgccccctgaagcagtttcaccagcagtaaaccgctcgtcacatcaccaacacctaccggctggcgcataccaaaatccaccagcggacggctgatatgccaggcttcatcggcggtgaccagcagcatttcaaaacggtcacggctgtagccagctcgcgccaggtgtttaaccaacacaatttgtggcccttgcgcaatgagttcgcgcgctgccagaaccgcttcttcgacgttatttaccgcatgctcacagagtatttccagctcaaccagatttggcgcaatgatatcgctggcaggcaaaccgtgccgcacatgaaactctgcgacacccggtgcaacgatacagcctttttccggatgacccattaccggatcgcaaaaatatttcgcctgcggattcgcggctttcacctgacggacgataccgaggatatgttcaccctgctccgccgatcccagatagccacttaatacggcatcacaggtgtgtaatttatcaatggcggcaatgccttgcacaatttcggttaaatggctgggcggcatcacgcagccagtccatttgccgtattgggtgtgattagaaaattgaacggtgttcagcggccagacgttcgcgcccaggcggcgcatcggaaactctgccgcactgttacccgcatgaccataaacaacgtgagactggatagcgagaatatttttcatcatgttccctgtataaaaaccagggggagtgatttctcactccccctttccacttaatgcattatttccagcaaatcagacagtaattctttttaccgcgacgcagtaaggtaaaacgaccaaacagacgatcttcttctttaaagaagtattcaggatcggactgtttttcaccgttaatggtgatggcattggaggcgatagttttacgtgcctgaccacgggaaggttgcagttcagaatcgaccagtgcctgcatcaggtctgcgcccttttccatctcaaccatcggtacgccgtcctgcgccagctgttcgaagtccgcttcactcagcgcactcaaagaaccgctgaacaggcattcggtaatacgttttgccgcctgtaaaccttcttcaccgtgaaccagacgagtcacctgctccgccagtacatactgggcgcgcggtgctttaccgctgtttttatcttcttcttccagggcgttgatctcttcaatgctcataaaggtgaagaacttcaggaagcggtaaacgtcggcatccgcagtgttgatccagaactggtagaatttgtacgggctggttttcttcggatccaaccagactgcgccgccttcagttttaccaaatttggtgccatctgctttagtgatcagcggaacggtcaggccaaacacctgattctgatgcagacgacgggtcaggtcgataccagaagtgatgttaccccactggtcagaaccaccaatttgcagcaccacaccgtactgtttgttcagacaggcgaagtcataaccctgcaacaggttgtaggaaaactcagtgaacgaaatcccctgatcttcacggttgagacgctgcttaaccgcttctttgttgatcatctggttaacggagaagtgtttgccaatatcgcgcaggaaggtcagcacattcatattgccgaaccagtcatagttgttcgccgcgatagcagagttttctccacagtcgaaatcgaggaacggggcaacctgcttacggattttgtccacccactcctgaacagtttcttcggtgttcagcttacgctcggcagctttgaagctcgggtcgccaatcagacccgtcgcgccgcctaccagcgcaaccggcttgtggcccgcctgctggaagcgtttcaggcataacaatggaacaagatgccccaaatgcaagctgtcagcggtaggatcgaagccgcaatagagcgcgatcgggccttgcgccagtcgctctgctaacgcttcctcgtccgtcacctgggctaccagcccccgctcttgcaattgtttaatcaagttactgcttgccatcaaaatctccatgtatataacgactgcacctttgccggtacacgacttttcgccagatgcgaaagagacatagaataaagtgccagaatcaggagtaccagcgattaaagcaagatttttgcatcttttcagggtgcaagacgatcaatcttccacgcatcattttcacgctggtacaaaaagcggtcatgcaggcgatgctcaccaccctgccagaactcaatctgttcaaggctgacgcgaaaaccgccccaaaagctcggcaatggcacttcgccctgttgaaacttctgcttcagctccaggaatttactttcaaggataccgcgggcagaaatgcgactggactgcttcgaaacccatgcaccaatctggctatcacgcgggcggctatgaaaatatttcatcacttcgagagtcgaaagtcgttctgctttaccgatcaccatcacctggcgctcaagggtatgccacgggaacagcaggctaacgcgcggattattttcgatttgatgtgctttacggctgccgaggttggtgtaaaacaccatgcctttttcgtcgtaatgtttgagtaaaacgatgcgctgataaggctgaccatgttcatccacggtagcgaccaccatcgcggtagggtccgccagtttggcttcacaagcctgagagagccaacgttcaaaaagggttaatggatcggcgggaagatcgcggcggcgtaacccgcctttggtgtattcacggcgcagatgcgcgatttgctgcaattcgtcgttatcagacatggttttctttacggattgtcagtgggtgacgctattgtgcgccgcccctggaaaaatctcaacgctgtggattttgtaactgacagttattcaagacgatgcggtcgcgtttatagacagtcgcttcatcgcctttcgaccagaaaacatagattccgtcagtgtaacgcgcgccagaggctgaaatgccctgtttgagatgcagtagttgattatcgtaaacaaaactgacctcctggcgcggattattcagtttgaccgtcaacggtttttcatcacactggtattccagcgtatcggtttgcatgcgctcaaccagctgattaaaggcgctacagccggagagaaggaccggcaaaatgataattaacagttttttcatagtcatatcccgaagactttcctggtctggagggcaatacgccctccctaacgttccaagtgtaacggcagacgcggtaagaaaaattcagttaactctgatatcacgggttagcggggaaaatagcccccagtaccgtctcctggcttgcgccagtgacggaaggcagatttcctggtaatcccgccagcgtccgccaggcaagccaggcgaaagccaatgcttccatgtcatcgccactaatgccaacggcatcggtggtggtgacttctgtgcctggcagtaatgccgccagacgcgccatgagtagcggattacgactacctccaccacataccatcaatcgttcgcagccaccgctcaacaaaacttgttcagaaatggtcacggcggtgagttctgccagtgtcgcctgcacatctcggggatcaacacccggaaaatggcgcaaatggcgctccagccaaccatagttaaagtattcgcgtccggtgcttttcggtgcaggttgcgagaaatacgggtcgctgagcatattttgcagcagtgggagaataactttacccgcccgtgcccactcggcatctttatcgtaaggtttaccggcctgacgccagatccaggcatccatcagcatgttaccaggaccggtatcgtagcccccaaccggctgcccaggaatgagcagtgacagattggcgatgccgccaatattgagcaccattcgtcgctcggttgggtgagccagcagcgcatgatggaacgcaggtaccagcggtgcgccttgtcctcccaaggcaatatcgcgacggcgaaaatcaccgacaaccgtaattccggtgcgtgccacaatttgattgttatcgccaatctgtaaagtgtgtggtgccacgcccgtcggttcatgccagacggtttgaccgtgacaaccgatcgcaactatatctcttgcctgcagattttgttccttaagcaaggcattgaccgcatcagcaaaaagttgcccgagttgagtatcaagctgtccaaactgcgaaagtgtaagctgctggccctggcaaatatccagtacagcctgtttcagagataccgggatcggccaactcaaacttgccagctgtgcgacccggtgttcatcaattgtcgccaacacaacatcaacaccatcaaggctggtgcctgacataacgccaataaagcggcccgatttcatagttcatcctttttcaatctgacgtttgcgcaccactcaaacataaacttttcgtgaataccatgcggaatgaccgatttttaccgttggtagtaaaacattatcttcaaatcaataatcatcatgaatgttttgtttataattggttgatcctactttcattatgatttgctcatatttggtagaacatgtaaccatggattcacatatgccatatactttgaccatgagggatgcttgcgtggcgtttcatggtgaacaggagatttttcaatgattaaacgcgtattggttgtttcaatggtaggtctgtctcttgtcggttgtgttaataacgacaccctgtcaggggatgtttataccgcttctgaagcgaaacaagtacagaatgtcagctatggcaccatcgttaacgtacgtccggtacagattcagggcggtgatgattccaacgttatcggtgcaattggcggtgctgttcttggtggtttcctggggaatactgttggtggcggaaccgggcgttctctggctactgcagcaggcgctgttgcaggtggcgtagctggtcagggcgtacagagtgcaatgaacaaaacgcagggtgtcgagctggaaattcgtaaagacgatggtaataccatcatggtggtacagaaacaaggcaacactcgtttctctccgggccaacgtgtcgtactggccagcaatggcagtcaggtgaccgtttctccgcgctaaataagtttgcgtgtggtcaggttactgaccacacgcccccttcatttcaccctttggcctgtaactcaatgatattatgctcaagttttgcgatgagcgtaatcagttgctccagttcctctgcggagatgccatgtaatatttccgcgcgggttttgttaataacagcttccatttcgctgatcagcggctctgccttttccgtcagtttaatacgtttagcccgacgatcgctggcacaagtttgacgcgaaattaaccctttttcttccagttggtccagagtacggaccagtgatggctgctcgatgccaatcgcttttgccagttgaatttgcgactggtctggaggtaactgatggatattgtgtaacgtaacccaatgggtttgtgttaactccagcggtttcaggcgatggtctatcagagcacgccatatgcgcaccaaccgtgccagatcagaacctagtggcgattccaatttcatctccttataattagcttgctaagatattatgcggcttttagaatagtgtgcagcaattgtattgctaaaacaaatgtattgctgcatttggttaccgtcagacatatttttcagaaattgcgcgtaaatttttcgcacttaaagaatatttattaatctaacgcaatatattcggtcgtaaaggaatctactttgtgaagtttatgctcaatgcaacaggattgcccttacaagatctggtgttcggtgcgtccgtctactttcctccgtttttcaaagcattcgcgtttggattcgtcatctggcttgtcgtacaccgcctgcttcgtggctggatctacgccggtgacatctggcatcccttgttaatggatttatcgctgtttgcgatttgcgtttgccttgctctggcaatactgattgcgtggtaactatgtcaattaaaacaattaagtatttctcaacaatcattgtagcggtagttgcggttcttgccggatggtggctgtggaattattacatgcaatctccgtggacacgcgacgggaaaatacgcgcagaacaggtttctatcaccccacaggtgtcgggacgtattgttgagctgaatataaaagacaaccagctggttaacgcgggggatcttctgctcacgatcgataaaacgccctttcagatcgccgagctgaacgcacaggctcagctggcgaaagcgcaatctgacctcgcaaaagccaataacgaagcgaatcgtcgtcgtcatctctcacaaaattttatttctgccgaagaactcgataccgctaacctcaatgttaaagcgatgcaggccagtgttgatgccgcacaggcgacgctgaaacaggcacaatggcaactggcgcaaacggaaattcgcgccccggtgagtggatgggtgactaaccttactacccgcatcggcgattacgctgataccgggaaaccgctgtttgcccttgtcgacagccactcgttttacgtcattggttattttgaagaaaccaagttgcgccatatccgcgaaggtgcaccagcacaaattaccctctatagtgataacaaaacgttacagggtcacgtttccagtatcggtcgggcgatttatgatcagagcgttgaaagtgactcaagccttattccggatgttaaacctaacgtcccctgggttcgactcgcccaacgcgttcccgtccgctttgcgctggataaagtcccaggcgatgtcacgttggtgtcgggcaccacctgtagcattgccgtaggtcaataatgaacgcatcgtcatggtccttgcgcaatttgccctggttcagggccacgctggcgcaatggcgttatgcgttacgcaataccattgccatgtgtctggcgctgacggttgcctattatttaaatctggatgaaccctattgggcgatgacctcggctgcagtggttagctttcccaccgttggcggtgttatcagcaaaagcctcggacgcatcgctggcagtttgctcggagccattgcggcactgcttcttgccgggcatacgctcaatgagccgtggttttttctattgagcatgtcggcgtggcttggcttttgtacctgggcctgtgcgcacttcacgaataacgtcgcgtatgcatttcaactggcgggctacacggctgccatcatcgcctttccgatggttaatattactgaggccagccagctgtgggatatcgctcaggcgcgcgtttgcgaggtaatagtcggtattttgtgcggcggcatgatgatgatgatcctgccgagcagttccgatgctactgcccttttaaccgcattgaaaaacatgcacgcccgattactggaacatgccagtttactctggcagcctgaaacaaccgatgccattcgtgcagcacatgaaggggtgattgggcagatactgaccatgaatttgctgcgtatccaggctttctggagccactatcgttttcgccagcaaaacgcgcgccttaatgcgctgctccaccagcaattacgtatgaccagtgtcatctccagcctgcgacgtatgttgctcaactggccctcaccgccaggtgccacacgagaaattctcgaacagttgctgacggcgctcgccagttcgcaaacagatgtttacaccgtcgcacgtattatcgccccgctacgcccgaccaacgtcgccgactatcggcacgtcgccttctggcagcgactacgttatttttgccgcctttatctgcaaagtagtcaggaattacatcgtctgcaaagcggtgtagatgatcataccagactcccacggacatccggcctggctcgtcataccgataacgccgaagctatgtggagcgggctgcgtacattttgtacgttgatgatgattggcgcatggagtattgcttcgcaatgggatgccggtgccaatgcattaacgctggcagcaattagctgcgtactctactccgccgtcgcagcaccgtttaagtcgttgtcacttctgatgcgcacgctggtgttactttcgctattcagctttgtggtcaaatttggtctgatggtccagattagcgatctgtggcaatttttactgtttctctttccactgctggcgacaatgcagcttcttaaattgcagatgccaaaatttgccgcattgtgggggcaactgattgtttttatgggttcttttatcgctgtcactaatcccccggtgtatgattttgctgattttcttaacgataatctggcaaaaatcgttggcgtcgcgttggcgtggttagcgttcgccattctgcgtccaggatcggatgctcgtaaaagccgccgccatattcgcgcgctgcgccgggattttgtcgatcagctaagccgccatccaacactgagtgaaagcgaatttgaatcgctcacttatcatcacgtcagtcagttgagtaacagccaggatgcgctggctcgccgttggttattacgctggggtgtagtgctgctgaactgttctcatgttgtctggcaattgcgcgactgggaatcgcgttccgatccgttatcgcgagtacgggataactgtatttcactgttgcggggagtgatgagtgagcgtggcgttcagcaaaaatcactggcggccacacttgaagaattacagcggatttgcgacagccttgcccgtcatcatcaacctgccgcccgtgagctggcggcaattgtctggcggctgtactgctcgctttcgcaacttgagcaagcaccaccgcaaggtacgctggcctcttaattacttaattacaccacaggcatagcgttcaccgccaccgcccagcggtttaggttgatcggacatattatcgccgccaacgtggaccatcagcgctttgtctttgatttcatccagtgatttcagacgaggcgcgatgacggcatcggtagctttgccgtcattattgacgaccagtgcaggcagatcgcctaaatgcccggcaccttctggcccttcatgtttaccggtattttgtggatcaagatgcccgcctgcggattccgcggcgctggctttgccatctttggtggctggctggcagcttcctttggcatgaatatggaagccatgttcaccggggggtaatgctttcagatcgggcgaaaactccagacctttatcggtttcagtaatggtgacgctaccaattgactgccctaccccttgcgacgtgacgaggttcatctcgactttttcactggcagcttgtgcgccggttgcaacaaccagcgccagaatagccagactaaaacgtttcataggacctccgttcattgtgcattcctgaataagtgtaaaccagtgacacatttttgaacggcggctattcctaaaagtgcttacggtacgtcgtaccccagtgccgctttacggatacgaaaccattgttgacgggtcattttcagtgtttctgcttcgacagctgcccgtacgcgctcaattttacctgaaccgataattggcagcggctgcgatggtaaacgtaatacccaggcgtaaaccacctgttcaatcgagcccgcgtttaactcctctgccaccacagccagttcatcacgcagcggctggaaataatcatcattaaacagacgaccaccaccaaggcaggaccacgccatcggacgaacacgcagttgttgtagttggtcgagcgtgccatccagcagtaacggctgatgcaccggggatatttccacctgattagtggcaagggtaaacggcagacgtgattgcaacagggcaaattgcgcaggcgtaaagttcgatacgccaaaatgacgcactttgccgctctgatgcagatgtttgaacgcgtccgccacttcatcggcatccattaacgggtctggtcggtggattaacagcaaatccagatgatcggtcgcgagattaattagcgactgttcggcgctcttaatgatgtgatcgcggtcagtgatgtaatgaccaatgacgttttcttcacgcgcggtcgtcgcgataccgcatttactgacgatttccatccgttcacgcaggtgaggtgccagtttcagtgcctcgccaaacgccgcttcgcactgatagccaccataaatatcagcatggtccacggtggtcacgccgagatccagatgctcttcaataaaactgaccagctggcgggcggacatattccagtccatcaatcgccagtagcccatcacaaaacgggaaaactccgggccttgcggcgcaatagtaatacgctgaaccataatcgcttcctcttatcagatatgagaggagtatacgcaagattaggttcaaaagagtgatggttgctccggttcgtctgatgacgctggcttatttgcgcgtaatttgcgcattaatcgctgccgacaaaggcgcagcacctcttgtttttcgccatcgctcattttattccagttaaaacgctcatcacgactacgaaaacagccgcgacaaaacccgcgttcgtcagactggcaaattccccggcacgggctctggacgggaaagaactctaattgctccgccacttcgccctcctcagataagattattaccattattgaagctgttaatgtccaaagtagcaactttgcttgcactagaccgactggtctactacactccaacgcatgaacaaacacaccgaacatgatactcgcgaacatctcctggcgacgggcgagcaactttgcctgcaacgtggattcaccgggatggggctaagcgaattactaaaaaccgctgaagtgccgaaagggtccttctatcactactttcgctctaaagaagcgtttggcgttgccatgcttgagcgtcattacgccgcatatcaccagcgactgactgagttgctgcaatccggcgaaggtaactaccgcgaccgcatactggcttattaccagcaaacactgaaccagttttgccaacatggaaccatcagtggttgcctgacagtaaaactctctgccgaagtgtgcgatctgtcagaagatatgcgcagcgcgatggataaaggtgctcgcggcgtgatcgccctgctctctcaggcgctggaaaatggccgtgagaaccattgtttaaccttttgtggcgaaccgctgcaacaggcacaagtgctttacgcactgtggcttggcgcgaatctgcaggccaaaatttcgcgcagtttcgagccactggaaaacgcgctggcccatgtaaaaaacattattgcgacgcctgccgtttagcaggcattttttatcaccagacgaccgggagcctttatgtcatctgaaaaactgtattccccactgaaagtgggcgcgatcacggcggcaaaccgtatttttatggcaccgctgacgcgtctgcgcagtattgaaccgggtgacattcctaccccgttgatggcggaatactatcgccaacgtgccagtgccggtttgattattagtgaagccacgcaaatttctgcccaggcaaaaggatatgcaggtgcgcctggcatccatagtccggagcaaattgccgcatggaaaaaaatcaccgctggcgttcatgctgaaaatggtcatatggccgtgcagctgtggcacaccggacgcatttctcacgccagcctgcaacctggcggtcaggcaccggtagcgccttcagcacttagcgcgggaacacgtacttctctgcgcgatgaaaatggtcaggcgatccgtgttgaaacatccatgccgcgtgcgcttgaactggaagagattccaggtatcgtcaatgatttccgtcaggccattgctaacgcgcgtgaagccggttttgatctggtagagctccactctgctcacggttatttgctgcatcagttcctttctccttcttcaaaccatcgtaccgatcagtacggcggcagcgtggaaaatcgcgcacgtttggtactggaagtggtcgatgccgggattgaagaatggggtgccgatcgcattggcattcgcgtttcaccaatcggtactttccagaacacagataacggcccgaatgaagaagccgatgcactgtatctgattgaacaactgggtaaacgcggcattgcttatctgcatatgtcagaaccagattgggcggggggtgaaccgtatactgatgcgttccgcgaaaaagtacgcgcccgtttccacggtccgattatcggcgcaggtgcatacacagtagaaaaagctgaaacgctgatcggcaaagggttaattgatgcggtggcatttggtcgtgactggattgcgaacccggatctggtcgcccgcttgcagcgcaaagctgagcttaacccacagcgtgccgaaagtttctacggtggcggcgcggaaggctataccgattacccgacgttgtaatccaacattgcgagcggcgtaaagccgccgctatactaaaacaacattttgaatctgttagccattttgaggataaaaagatgcgtcttcttcataccatgctgcgcgttggcgatttgcaacgctccatcgatttttataccaaagtgctgggcatgaaactgctgcgtaccagcgaaaacccggaatacaaatactcactggcgtttgttggctacggcccggaaaccgaagaagcggtgattgaactgacctacaactggggcgtggataaatacgaactcggcactgcttatggtcacatcgcgcttagcgtagataacgccgctgaagcgtgcgaaaaaatccgtcaaaacgggggtaacgtgacccgtgaagcgggtccggtaaaaggcggtactacggttatcgcgtttgtggaagatccggacggttacaaaattgagttaatcgaagagaaagacgccggtcgcggtctgggcaactaatctcctgccgggcgtgaactcatcgcgcccgcatctttactgcatcgacaagtaatatttgtcataatgcgcgctgcaatttatccgtattaagagaatcagatgtccgataacgctcaacttaccggtctgtgcgaccgttttcgtggtttttatcctgttgtgatcgatgttgaaacagccggatttaacgccaaaaccgatgcgctgcttgagattgccgccatcaccctgaaaatggatgaacaaggctggctgatgccggacaccacattacatttccacgtcgaaccatttgtcggcgcaaatttgcaaccagaagccctcgccttcaacggcattgacccgaacgatcccgatcgcggcgcggtcagcgaatacgaggcgctgcacgaaatttttaaagttgtacgtaaaggtattaaagcgagcggctgtaaccgcgccattatggtggcgcacaatgccaattttgatcacagctttatgatggccgccgcagaacgcgcctcactgaaacgtaacccgttccaccctttcgccacttttgacactgctgcactggccgggctggcactcggacaaaccgtattgtcaaaggcttgccagaccgctggcatggacttcgacagcacccaggcgcactccgcgctgtacgacaccgaacgcactgctgtgctgttttgtgaaatcgtcaaccgctggaaacgtctgggaggctggccgctatctgccgccgaagaggtgtaatcgagtcgatgcctgatgacatgcaatgattcaggcatctatagtgaggctattccacgcatcctgcatgatattcacggggaatagcgttaatggcagataatccagacccttcatcgctcctgccggacgtgttttcaccggcgacccgcgactggtttcttcgcgcctttaaacagccgaccgctgtccagccgcaaacctggcatgtggcggcgcgaagcgaacatgcgctggtgattgcaccgaccggctccgggaaaacgctggcagcatttctctacgccctcgatcggctcttccgcgaaggcggcgaagatacccgcgaggcgcataagcgtaaaacctcacgcatcctctatatttcaccgataaaagccctgggcaccgacgttcagcgcaacttgcagatcccgttgaagggtattgccgatgaacggcggcggcgcggcgaaacggaagtcaatcttcgcgtagggatccgtactggcgatacgcctgcacaggaacgcagcaaactcacccgtaatccgccggatattctgatcaccacacccgaatcactctatctgatgctgacctcccgcgcgcgcgaaacgctacgcggcgtcgaaacggtaattattgatgaagtccacgcggtagcgggcagtaaacgtggtgcgcatctggcgttaagtctggagcggctcgatgcgctgctccacacctcagcacagcgaattggcctttctgccactgtgcgctcagccagcgatgtggcagcatttcttggtggcgatcgcccggttacggtagtcaacccgcccgcaatgcgccatccgcagatacgaattgtcgtaccggtcgccaatatggatgatgtctcatcggtcgccagcggcaccggcgaagacagccatgccggccgggaaggctccatctggccatatattgaaacgggtatccttgatgaagtgttgcgccatcgctcgaccattgtctttactaattcgcgggggctggcggaaaaactgacggcacgattaaatgagctttacgccgcacgcttacagcgttccccgtctatcgccgttgatgcggcccatttcgagtcgacctccggcgcaacctctaaccgtgtacaaagtagcgacgtttttattgcccgctcacaccacggctccgtctctaaagaacaacgagcaatcaccgaacaggcgctgaaatcgggtgaattacgctgcgtggtcgcaacctccagtcttgaactggggattgatatgggcgcggtggatctggtgattcaggtggcaacgccgctttctgttgccagtgggttacaacgcattggtcgcgccggacatcaggttggcggtgtatctaaagggctgtttttcccccgtacccggcgtgatttagtcgattccgcagtcattgtagagtgtatgttcgcaggcaggctggaaaacctgacaccaccgcataatcctctcgacgtccttgcgcagcaaaccgttgccgccgcggcgatggatgcattacaggtagacgaatggtactcccgcgtacgccgtgccgcaccgtggaaagatctgccaagacgtgtttttgacgccacgctggatatgctttccgggcgctatccctctggcgatttttctgcttttcgccccaaactggtctggaacagggagaccgggatattgaccgcccgacctggcgctcaattgttggcggttaccagcggcggcaccattccggatcgtggcatgtatagcgtgttattacccgaaggtgaagaaaaggccggttcgcggcgggtgggtgaactggatgaggagatggtatatgagtcgcgggtgaacgacattatcactctcggcgctacctcatggcggatccagcaaatcacccgcgatcaggtgattgtgactcctgctccgggtcgttctgcccggctccccttctggcgtggtgaaggtaacggacgtccggctgaattaggcgagatgatcggcgattttcttcatttgctggcggatggcgcgttcttttccgggactattcccccgtggctggcagaagaaaatacgatcgccaatattcaggggttgattgaggagcagcgcaacgcgacgggcatcgttccggggagtcgccatctggtcctcgaacggtgccgtgatgaaattggtgactggcgtattattttgcactctccctatggaagacgggtgcatgaaccctgggcggtggcgattgccgggcgaatacatgcgctatggggcgctgacgcgtcggtggtcgccagtgatgacggcattgttgcacgtattcctgacaccgatggtaaattgcccgatgccgcgatttttttgtttgaaccagaaaagttgctgcaaattgtccgcgaggcggtaggcagctcggcacttttcgccgcccgttttcgcgaatgcgccgcgcgggcattattaatgccggggcgcactccgggccatcgcaccccgctttggcaacaacggctgcgcgccagtcagttgctggaaatcgctcagggatatccggattttccggtcattctcgaaaccctacgcgaatgtctgcaagatgtttatgatcttcccgcactggaacgtttgatgcgtcgcctgaacggtggcgaaattcaaatatccgatgtaacgaccactacgccctcgcctttcgccacaagtttattgttcggctatgtcgcggaatttatgtaccagagcgacgccccgctggcagagcgccgggcatccgtactgtcgctggacagcgagttactgcgcaatctactcggacaggtcgatccgggggaattactcgacccgcaggtcattcgccaggtggaagaagagttgcaacgactggctcctggcagaagagcgaaaggtgaagaaggattgttcgacctgctgcgcgaactggggccaatgaccgttgaagacctggcgcaacggcatacaggcagcagtgaagaggttgcgtcgtatctggaaaatcttcttgcagtaaaacgaatcttcccagcgatgattagcggacaggagcgtcttgcctgtatggatgatgccgccaggctgcgtgatgccctcggcgtacgactaccagagtcattgccagagatttatttacatagagtcagttacccgcttcgcgacctctttctgcgctatctccgggctcatgctctggtcacggctgaacaactggctcatgagtttagtctcggtattgccattgtcgaagagcagcttcagcaactgcgtgaacagggtctggtgatgaatctgcaacaagacatctgggtgagcgatgaagtatttcgtcgtctgcgtttgcgctcgctgcaagccgccagagaagcgacgcgtcccgttgcagccacgacctatgcgcgattgctgctggaacgtcagggcgtattacccgccaccgatggtagcccggcgctctttgcctcaacatcgccaggcgtttatgagggcgtagatggcgtgatgcgggtgatcgaacagcttgccggagtcggtttacccgcctcactctgggaaagccagatcctgcctgcccgcgtacgcgactattcgtcagaaatgctcgatgaattactggcaaccggtgcggttatctggtcggggcaaaaaaaactgggtgaagatgacggcctggtggcactgcatctacaggaatatgctgcagaatcgttcactcccgccgaagcggatcaggcgaatcgttcggcgctgcaacaagcgatagtcgctgttctggctgacggaggagcctggtttgcacaacaaatcagccaacggatacgcgacaaaatcggcgaatcggttgatctctctgccctgcaagaggcgttatgggcgctggtctggcaaggcgtcatcaccagcgacatttgggcaccgttacgcgccctcacccgcagcagttccaacgcacgcacctcaactcgccgcagtcaccgggctcgtcgtggacgtcctgtctatgcgcaacccgtctcgccgcgggtatcttacaacacaccaaatctggctggacgctggtcgttattgcaggtggagccactaaacgataccgaaaggatgctggcgctggcggaaaatatgctcgaccgctacggcatcatcagtcgtcaggcggtgatagccgaaaatatccctggcgggtttccatcgatgcaaacgctttgtcgaagtatggaagactccgggcgaattatgcgaggtcgttttgtagaaggtctgggtggcgcgcaattcgctgaacgtctgactattgaccgattgcgcgatctggcgacacaagccacgcaaacgcgccactatacaccagtggcgctctctgccaacgatccggctaatgtgtggggaaatcttctgccctggcctgcacatccggcaacgctggttccaacgcgtcgggcgggtgcgctggtggtcgtttctggcggcaaattgttactctatctggcgcaaggtggcaaaaaaatgctggtctggcaggaaaaagaggaattactcgccccagaggttttccacgcgctgactaccgcactgcgtcgcgaaccacggctgcgctttacgctaacagaagtgaatgatctaccggtccggcaaacgccgatgtttacgctgctgcgtgaggcgggattttcaagttcgccacaagggctggattggggatagagaaaggactgacggatgcccgttcgcatccgtcagtattgcaggacggattattccgcgtccggctcttcagacttgtatttagcggcagtttctttgatcagctgctgcagttcgccacgctgatacatttcgatcacgatatcacaaccgccgaccagctcgccgtcaacccacagttgcgggaaggtcggccagttagcatatttcggcagttccgcacgaatgtccggattctgcagaatatcaacataggcaaaacgttcgccacatgcggcaagcgcctggactgcctgggcagagaaaccgcagctcggcagtttcggtgaacctttcatgtacagcaggatcgggttttcagcaatctggcgttggattttttcgatagtggtgctcattgtcttgcttcctcaaacttctttacggcagtaatctgacattgtagcgggtcagtgcggcatcggaaaataacattttcatcacgcttttgctattttatccctttgctctatttgttgcatttcaaatattcgtttcttctctgatgccggcaaactggcgtatttataaccatttttagctttcactgctgcatttttttgcgctcgccaacgaaacgtattttttaacaataaaagctattaactttctcttcttctatgcattagaatcatcaagttttgtaaatcagacgcaggcatgatagacctgcctttacagagggacgctcagtggcgcggataaaccgtatttcgatcacgctctgtgctttactttttaccaccctgcctttaacgcctatggcccatgcttcaaagcaagccagggagagttctgctaccactcatatcaccaaaaaagcagataaaaagaaaagcacggcaaccaccaaaaagacccagaaaacagcgaaaaaagccgccagtaaaagtacgaccaaaagcaaaaccgcttcttccgttaaaaaatcttccattaccgcttctaaaaacgccaaaactcgcagcaaacacgccgtcaataaaacggcctcagccagctttaccgaaaagtgtaccaaacgtaagggctataaatcgcattgtgtgaaagtcaaaaatgccgcgtcaggaactcttgccgacgcgcacaaagcgaaggtgcaaaaagctacgaaagtggcaatgaataaactgatgcagcaaattggtaagccatatcgttggggtggcagctcaccgcgtaccggttttgattgcagcggcctggtttattacgcttataaagatttggtgaaaattcgtattccgcgtacggcgaatgaaatgtatcacctgcgtgatgcagcgccaatcgaacgtagtgaactgaaaaacggcgacctggtctttttccgtactcagggacgcggcacagccgatcatgtcggcgtgtatgtcggcaacggcaaatttattcagtcaccgcgcacaggtcaggaaattcaaatcacttctctcagtgaagactactggcagcgccactatgttggcgctcgtcgggtaatgaccccaaaaacacttcgctaaaactttaccctgttgttacggcaacagggtaagttcatcttttgtctcaccttttaatttgctaccctatccatacgcacaataaggctattgtacgtatgcaaattaataataaaggagagtagcaatgtcattcgaattacctgcactaccatatgctaaagatgctctggcaccgcacatttctgcggaaaccatcgagtatcactacggcaagcaccatcagacttatgtcactaacctgaacaacctgattaaaggtaccgcgtttgaaggtaaatcactggaagagattattcgcagctctgaaggtggcgtattcaacaacgcagctcaggtctggaaccatactttctactggaactgcctggcaccgaacgccggtggcgaaccgactggaaaagtcgctgaagctatcgccgcatcttttggcagctttgccgatttcaaagcgcagtttactgatgcagcgatcaaaaactttggttctggctggacctggctggtgaaaaacagcgatggcaaactggctatcgtttcaacctctaacgcgggtactccgctgaccaccgatgcgactccgctgctgaccgttgatgtctgggaacacgcttattacatcgactatcgcaatgcacgtcctggctatctggagcacttctgggcgctggtgaactgggaattcgtagcgaaaaatctcgctgcataataactgatggcaaatgcagcattgcctgaagcgctacgcttatcaggcctacgcggatcatcgatgtaggtcggataaggcactcgccgcatccggcaagataaatcgcacgttgtcagcaactgtaacgcagaaggttatccttctgcgtttttgtttaattagctgttagcaacgcaaactgtttcaggttgttttctggctgacataaacaccagcaataatgccagtcccgcgacaatcgctcccatcaccggcacaaagctgtatcccagcccagcggaaattaccgcaccaccagcagctgctcccagcgcatttccaagattaaaggcaccaatattgactgatgaagacagacctggcgcttcactggcgacacgcatcacgcgcatctgtaacggcggtacgaccgcaaaggttgctgcgccccacaccaccatgctaatagctgcgccgaactcattgcgggccaggaacgggattgccagcataatcaccatcaacaacaacaaaaagcctttcaacgtgccgttaactgaacgatctgccagtttgccgccgagatagttaccgatagagaatccgacaccaatcagcaccagcattgccgtgacgaacaccggtgttgcgtgggtaatactttgcagtaccggagagatataggtgtagagagtaaacattgcaccagctcccagtaccgtcgtcagcaatgcagacagcacctgcggacgcattaataccgccagctcttttttcacttcaggtcgtgcccctgcaccacctttaggtaatgagaagaacagacttaccattgaaatcactcccagccccgccgttgccagaaatgacatccgccagccgatggtttcacccaaccaggtcgccgccggcacgccaccgatatttgccagggttaaccccataaacatagtggcaactgcgctggcctgtttatgttttggcaccacgcttgcggccacgactgaacccaaaccaaaaaatgctccgtgattcaggctggtcaaaatgcgtgaaagcatcagggtcatataatccggcgcgatggcggaaagtacgttgccgagcgtgaaaattgccatcaggaaaatcaacgcactgcggcgggcacgatgagaaagtagaagcgtcatcagcggcgcgccaaccattacgccaactgcataggcactgattaacattccggcagcgggaatcgagacatccacaccgcgcgcaatgacgggcaacaagcccattggcgagaactccgttgtcccgataccaaacgcgccaatcgccagcgccagcaacggatagttaattttcatgccttatctccacctcttcgcgtcattacgcgatattcattaaagtggcgaaagcatgacagcaatcacaaaaaaatgaaaataacaaaaagagaaaacacttttgccattttgctaacaaacaggaaggagatgcgagggagaacgcgctccctcgagaggaaatcagtgcagcgcggcagtcaaacccacggctacgatcaaaccgaggacgataatcgttgttaccagtgaaaatttaaggtcggtgctcatcaagttttctccttttttattaccacacaaaaagtgatattacgcatttttacacactgtgatgaaaaaatctcccgtcatttataatgataagtgtttttaccacttccccttttcgtcaagatcggccaaaattccacgcttacactatttgcgtactggccattgaccccttcctgacgctccgtgtcgtttttccggcgtaccgcaacacttttgttgtgcgtaaggtgtgtaaaggcaaacgtttaccttgcgattttgcaggagctgaagttagggtctggagtgaaatggaatggcaacaataaaagatgtagcgaaacgagcaaacgtttccactacaactgtgtcacacgtgatcaacaaaacacgtttcgtcgctgaagaaacgcgcaacgccgtgtgggcagcgattaaagaattacactactcccctagcgcggtggcgcgtagcctgaaggttaaccacaccaagtctatcggtttgctggcgaccagcagcgaagcggcctattttgccgagatcattgaagcagttgaaaaaaattgcttccagaaaggttacaccctgattctgggcaatgcgtggaacaatcttgagaaacagcgggcttatctgtcgatgatggcgcaaaaacgcgtcgatggtctgctggtgatgtgttctgagtacccagagccgttgctggcgatgctggaagagtatcgccatatcccaatggtggtcatggactggggtgaagcaaaagctgacttcaccgatgcggtcattgataacgcgttcgaaggcggctacatggccgggcgttatctgattgaacgcggtcaccgcgaaatcggcgtcatccccggcccgctggaacgtaacaccggcgcaggccgccttgccggttttatgaaggcgatggaagaagcgatgatcaaggtgccggaaagctggattgtgcagggtgactttgaacctgaatccggttatcgcgccatgcagcaaatcctgtcgcagccgcatcgccctactgccgtcttctgtggtggcgatatcatggcaatgggcgcactttgtgctgctgatgaaatgggcctgcgcgtcccgcaggatgtttcgctgatcggttatgataacgtgcgcaacgcgcgctattttacgccggcgctgaccacgatccatcagccaaaagattcgctgggtgaaacagcgttcaacatgctgttggatcgtatcgtcaacaaacgtgaagaaccgcagtctattgaagtgcatccgcgcttgattgaacgccgctccgtggctgacggcccgttccgcgactatcgtcgttaatcacccgttgcgggagtctcttccggctcccgcagccactccttattcagcgtctcactatcgccgagatactcaagcaaccaggttaacgcaggcgacatatcattttgctgccatgtcagacaacatgccgaatccggaaaggggttttccagttctaatgctacccacttcccctcattaagccacggtttggcgaaatgtgttggcaccatccctatgcataatcctgccgagatacaggttgccgatgattcccagtcaggcacgacaactcttttttggttatccagcaaccaggtaatacgtttaggtagcgttcgcgaggtgtcttcgcgcaccaacgacggccagttgcgcaacgtatcatcgctgaacgggccatccatcaacgccagcgggtggtgactggcaacaacgcaactccagcttagcatccccatatcccggaaggcataacgaccgcctaccggaatcgcgcgtgttgcgccaatcgccagttccacgcgcccgtcggaaagcgcatcccagacaccgttgaacacttcctgaaagacaagaagttcgacatcatcaaaatggcgataaaaatcaacgatcatctgccgtgtacgttctggcctgacaatattatccactgcgatagctaactgaccgcgccagccgttcgctatctgctgacattgctggcgggtgatctgcatttttttgacaacagagcgcccttctttgagaaaccacgctccagcagcggtcagctccacatcacggtgccgtcgttcaaagagcggcaccgccagccactcttccagctgacgcacggtatagctgaccgcagaaggaacgcgatgcagctcctgtgccgcagcgctaaaactaccattacgcgctaccgcatcaacaacttcgagtgaatattctgaccacatagtctgcctgcaaaatttttgaaaccagtcatcaaatattaccgtttcacaacactaatttcactccctacactttgcggcggtgtttaattgagagatttagagaatatacatgcaacctgggaaaagatttttagtctggctggcgggtttgagcgtactcggttttctggcaaccgatatgtatctgcctgctttcgccgccatacaggccgacctgcaaacgcctgcgtctgctgtcagtgccagccttagtctgttccttgccggttttgccgcagcccagcttctgtgggggccgctctccgaccgttatggtcgtaaaccggtattattaatcggcctgacaatttttgcgttaggtagtctggggatgctgtgggtagaaaacgccgctacgctgctggtattgcgttttgtacaggctgtgggtgtctgcgccgcggcggttatctggcaagcattagtgacagattattatccttcacagaaagttaaccgtatttttgcggccatcatgccgctggtgggtctatctccggcactggctcctctgttaggaagctggctgctggtccatttttcctggcaggcgattttcgccaccctgtttgccattaccgtggtgctgattctgcctattttctggctcaaacccacgacgaaggcccgtaacaatagtcaggatggtctgacctttaccgacctgctacgttctaaaacctatcgcggcaacgtgctgatatacgcagcctgttcagccagtttttttgcatggctgaccggttcaccgttcatccttagtgaaatgggctacagcccggcagttattggtttaagttatgtcccgcaaactatcgcgtttctgattggtggttatggctgtcgcgccgcgctgcagaaatggcaaggcaagcagttattaccgtggttgctggtgctgtttgctgtcagcgtcattgcgacctgggctgcgggcttcattagccatgtgtcgctggtcgaaatcctgatcccattctgtgtgatggcgattgccaatggcgcgatctaccctattgttgtcgcccaggcgctgcgtcccttcccacacgcaactggtcgcgccgcagcgttgcagaacactcttcaactgggtctgtgcttcctcgcaagtctggtagtttcctggctgatcagtatcagcacgccattgctcaccaccaccagcgtgatgttatcaacagtagtgctggtcgcgctgggttacatgatgcaacgttgtgaagaagttggctgccagaatcatggcaatgccgaagtcgctcatagcgaatcacactgatctatatcgatatacttatacttaggctgctaacaaaattttgttgtatgattgaaattagcggcctatactaatttcgagttgttaaagctacgataaatattatgtttttacggggacaggatcgttcccgactcactatggatagtcatttcggcaagggttcctcctttccctctgttctacgtcggattatagactcgcggttttttctgcgagatttctcacaaagcccaaaaagcgtctacgctgttttaaggttctgatcaccgaccagtgatggagaaactatgagttcatcgtgtatagaagaagtcagtgtaccggatgacaactggtaccgtatcgccaacgaattacttagccgtgccggtatagccattaacggttctgccccggcggatattcgtgtgaaaaaccccgatttttttaaacgcgttctgcaagaaggctctttggggttaggcgaaagttatatggatggctggtgggaatgtgaccgactggatatgttttttagcaaagtcttacgcgcaggtctcgagaaccaactcccccatcatttcaaagacacgctgcgtattgccggcgctcgtctcttcaatctgcagagtaaaaaacgtgcctggatagtcggcaaagagcattacgatttgggtaatgacttgttcagccgcatgcttgatcccttcatgcaatattcctgcgcttactggaaagatgccgataatctggaatctgcccagcaggcgaagctcaaaatgatttgtgaaaaattgcagttaaaaccagggatgcgcgtactggatattggctgcggctggggcggactggcacactacatggcatctaattatgacgtaagcgtggtgggcgtcaccatttctgccgaacagcaaaaaatggctcaggaacgctgtgaaggcctggatgtcaccattttgctgcaagattatcgtgacctgaacgaccagtttgatcgtattgtttctgtggggatgttcgagcacgtcggaccgaaaaattacgatacctattttgcggtggtggatcgtaatttgaaaccggaaggcatattcctgctccatactatcggttcgaaaaaaaccgatctgaatgttgatccctggattaataaatatatttttccgaacggttgcctgccctctgtacgccagattgctcagtccagcgaaccccactttgtgatggaagactggcataacttcggtgctgattacgatactacgttgatggcgtggtatgaacgattcctcgccgcatggccagaaattgcggataactatagtgaacgctttaaacgaatgtttacctattatctgaatgcctgtgcaggtgctttccgcgcccgtgatattcagctctggcaggtcgtgttctcacgcggtgttgaaaacggccttcgagtggctcgctaaaggctattctatcgccccctctccgggggcgatttcagatcaggcttctgtgcctggttgattcatggcattttctcgtgccgccagcacacgttctaccgtatctaccactgcctgagtttgtggatcgatttcaatgttgacgcgtgcgccaagttttttcttcccaagagtcgtgcgttccagtgtttccggaattaaatggacgcaaaaacgcgttggcgtgacttcgccgacggtcaggctaataccgtcgatgccaataaatcctttgtacagaatatatttcatcaactgactatcctggactttaaaccagatctggcgattattttctgaggttaatattttcgccacttcagcagtggtcataatatgacctgacattaagtgtccgccaatttcatcactgaatttcgccgcacgctcaacgtttacccaatcccccacttttaaatcgccaagattggtaatgcgtaacgtttctttcatcaggtcaaaactgacatggttgccgttaatttccgtcacggtcaggcagcaaccgttatgcgccacggaagcaccggtttccaggccgtccagcatgtggtcgggtaactccaccacatgcgtacgaaaatttggtttctcgtcaatcgacaccagttttgcggtgccctgtacaatccccgtaaacatacttacaactcctgaaatcagttaagacattctgttcagcacaatagcaggtggaaaacgcccttaccagtgaaggggtaagaatggctattttttcactggagaattaataaatcctcgctacaatagactgaatttcccctgcttcttctttttgctgcccattcaggcggctttttagtctctcatataactacaaataaaaggtgttcacgtgcagaagtatatcagtgaagcgcgtctgttattagcattagcaatcccggtgattctcgcgcaaatcgcccaaactgcgatgggttttgtcgataccgtgatggcgggcggctatagtgccaccgacatggcggcggtcgctatcggtacttctatctggcttccggcgatcctctttggtcacggactgctgctggcattaacgccggttatcgcgcaattaaatggttccggtcgacgtgagcgcattgcgcatcaggtgcgacaaggtttctggctggcaggttttgtttccgttctcattatgctggtgctgtggaatgcaggttacattatccgctccatggaaaacatcgatccggctctggcggacaaagccgtgggttatctgcgtgcgttgttgtggggcgcgccgggatatctgttcttccaggttgcccgtaaccagtgtgaaggtctggcaaaaaccaagccgggtatggtaatgggctttatcggcctgctggtgaacatcccggtgaactatatctttatttatggtcatttcggtatgcctgagctcggtggcgttggttgtggcgtggctactgcggcggtgtattgggtcatgttccttgccatggtttcttacattaaacgcgcccgctccatgcgcgatattcgtaacgaaaaaggcaccgcaaaacccgatcctgcggttatgaaacgactgattcaactcggtttgccgattgcgctggcactgttctttgaagtgacactgtttgccgtcgtggctctgttagtgtctccgctcggtattgttgatgtcgcaggacaccagattgccctgaactttagttcactaatgttcgtgcttccaatgtcgctggcggcagcggtaactatccgcgtaggttatcgtctgggtcagggctcaacgctggatgcgcaaaccgctgcgcggaccgggcttatggtgggtgtctgtatggcaaccctgacggccattttcacggtttcactgcgggagcaaatcgccctgttgtacaacgacaatcccgaggttgtaacgctggctgcgcatttgatgttgctggcggcggtatatcagatttctgactcaatccaggtgattggcagtgggattttgcgtggttataaagatacgcgttccattttctatattacctttacggcttactgggtgctgggcttgccaagcggctatattctggcactgaccgatctggtcgttgaacctatggggccagcaggcttctggataggctttattattggcctgacgtcggcagccattatgatgatgttgcgtatgcggttcctgcaacgtctgccgtcagccatcattctgcaacgagcatcccgctaataaagacaaggcgcaaccttcacgggttgcgcctgtatttttacgcaggctggagcgttgcgccaatcccgtcttcgtctggctgtaatttcagagcgttacacagagtttgccgactggcatctgttatctcaacgtgtatatccccggtaacttcccctttcacattgatgaagtcaggtgaaatttcttttgcactggtttgcaggcaaatcgctccctctccgcgcaggcgtttcactttcagttgcacatgcgttgccgcatcagtgatcagccacagttttccaccattcagattgatgttaccaacaatgaaagtgacactgtcaccttttaccgtactgccgtctagaatcaacacaccgccctgctgtacagtaatcgttgattgttgcagctctgcgccataaccaataatcattgaagcgccgtccagtaatgcaacactcccggtcagttcaaccggtgcgcgatcttcctctacgacaaaattttcgtccgcgctggtgggtgacaacaggatcactgtcccaccttgtattaccgcgttttccagcgtaccggcatgcacttcagcccgaccacccacattcacggacaggttttgcgtcttaccggaactgtagagctgaaggccatccgtccccagacgataaatggatccattctcaacaatagtgtcagagtcttcaccaccgagattattcatggtgccaccagcaagcaacgtatcactggctttcccggccagcataaaaacgccgccctgattaatctcacaattgctggcttccccacctggatacaccaacaattcaccaccttcatctaccacgaccgctgaggttgtcccattaaccaacaggccgccctcttgatcgagaatgattttttccgcgcgatgtccttccagtacacgcaggttaccgccattttccagcaacaaaccgcaggcataacctttatcaacgctgaattcaccttcgggatggcggccattaaccgtagcgagcgtagagagactaattgcgcctccctcggactgaacaatatctgtggcaatggcaccatcgctgaccgatagcgtgccattgttaccgtactgtgtgcatttggcgatcccaccggttgccactttcaaccagccagcccccgtgaccacggtattttcggctcttccgccagcttcaacaatcaactcgccttcagtaagttgcgtcgcgccaatgacctcgccggtcttaacaatttgcacgttcccgtcgctcatcaagtttttcgcatcagatcccatgatttattcctttgctgcatctgtgtgcctttattgctacctaagtgtaaaggctacggaggatttatccacgacagatttgagatggtggcaaacaactctgtttaaactctgatacacgaattattgggttgtatcagatgtaaatgcgatcctgaataaaaatcacccttgcaaatcaacaaaatatagccaatttgcttaaaagctctgcaaacggtcgaaatagcgcagaaaattacgttttgcctcttgccaccttcccactctgccgctaatattcgtccccgttgtcacctacaacgttgcgttcatagctcagttggttagagcaccaccttgacatggtgggggtcgttggttcgagtccaattgaacgcaccatcctgcgtccgtagctcagttggttagagcaccaccttgacatggtgggggtcggtggttcgagtccactcggacgcaccagattttcttaatctggtcttctcctttttccctctgtttcttctctgtatccaatacgttaaaagatttacactgtcttcgtatgcgttatcagaaggagaatcgctatggcaactttgttacaacttcattttgcttttaatggcccatttggcgacgcaatggctgagcagcttaaaccacttgctgagtcgattaatcaggaacctggttttctgtggaaggtatggacagaaagtgaaaagaaccacgaagccggtgggatctaccttttcactgatgaaaaaagcgcccttgcctatctggaaaaacatactgcccgactgaaaaatctcggcgttgaggaagttgtcgccaaagttttcgatgtcaatgagccacttagtcaaatcaatcaggcaaaactcgcctgacagaatttaatcaagggcggttagcgcccttttcatccctgtctgaaatttctcaaattctaaaaatctcaaccaaacttatctgataacactaaattcgaaagaatgcgtacaggtaagtaacaatgaaaaaaattgctattgtgggtgccgggcctacggggatctacaccttattctcgcttctacagcaacaaactccactttctatttctatcttcgagcaggctgacgaggccggtgtcgggatgccatacagtgatgaggaaaactcaaaaatgatgctggcaaatattgccagtattgaaataccgccgatttattgtacgtatctcgaatggctacaaaagcaagaagacagccatctccagcgttatggcgttaaaaaagaaaccttgcacgatcgtcagtttttaccgcgaattctgctgggcgaatatttccgcgatcaatttttacgactagtagaccaggcacgacagcaaaaatttgcagtggctgtttatgaatcatgccaggttaccgatctgcaaattacaaatgctggcgtcatgctcgctacaaatcaggatttacccagcgagacgtttgatttagcggtgatcgccacgggtcacgtctggcctgatgaagaagaagcaacccgaacgtattttcccagcccgtggtcaggcctgatggaagcaaaggtcgatgcgtgtaacgtgggtattatgggaacatccttgagcggactggatgcggcaatggcagtggctattcagcatggttcgttcattgaagatgataaacaacacgtcgtttttcaccgcgataacgcaagtgaaaagctaaatatcacgttgttgtcgcgcacgggtattttacccgaagccgatttctattgccctattccctacgagcccttacacatcgtcaccgatcaggcattaaatgctgagattcaaaaaggcgaagagggccttttggatcgggtatttagattgatagtagaggaaatcaagtttgctgatccagactggagtcaacgcatagccttagagagcctgaatgtcgattcctttgctcaagcctggtttgccgagcgcaaacaacgcgacccatttgactgggcagaaaaaaatctccaggaagtcgaacgcaataaacgagaaaaacatactgttccctggcgttatgtcattctgcgcctgcatgaagccgtacaggaaattgttccacatctgaatgaacacgaccataaacggttcagtaaaggccttgcccgggttttcatcgataattatgcggcaatcccttcagagtctattcgtcgcctacttgccttacgtgaagcgggaatcattcatattctcgccctcggtgaagactacaaaatggaaattaatgagtcgcgcaccgtcctgaaaacggaagacaacagctactcgtttgacgtttttattgatgcccgcggacaacgtccgcttaaagtgaaagatatccctttccctgggctacgcgagcaattacagaaaacaggggatgaaatccctgatgttggcgaagattatacgttacagcaacccgaagatattcgtgggcgcgtagcgttcggcgcgttgccctggttgatgcacgaccagcctttcgttcagggacttacggcatgtgcagaaattggtgaggcgatggctcgggcggtcgtaaagcctgcatcccgtgctcgtcggcgtctttcgtttgattaaaggtaaagctatcagcactcaacaaactgatgctgttcattaagacgatagcggactccggctcgaatattgttttcaccttcaatggcgacggcgaagcgaactctttcgccgtcatgatatgccagtgcggcgcttcctcctggcccgagaataattgagtcgaccacgcccgtgctcactaccgttgaattttcaccgctggcaatgatgtgtacattgtcgccgctgttggcaattctggcgtttgcgccaaagctggcgatttgcaccaggtcaccattactggcgacatgacaccgttcacccaatgtacaaacgcgtactcgcattccggtattcgcaatccgactgctatctccagcgctgcttatccgcgaagaattaccggttacagcaacccgtgcgcgttcaccggagctgccaatgtgactgttaaagccgacacttccaatccgcacgctataacccatactggcaatttgcgcggcatacccagcggttgcgattctggcgttatcctcacaacagccgatgcgagcatgatcgtcgctgcgggcaaactgactgcaaaatggtctctctccggggtctgtggccagtttttgcatagaggaaacttcctgatgcgcgaagttttcatccgccagccattttttccacgcatactcaaccagactctccgcccagtccgtatatccttcctcaatcagtgcatgatgaatatcggcataactaccgccgcgtgggaaatggcgcaggaaccagcgatacatcaccgctccgatacgccattctcgcaggtctgcttgtgtaatgatcattcgttagtgccggtgatagccatcgaccatgcttttaaaggtttcgtgtggcgtacgccccgtggtgcaaagataaagatgaccgaagataaaaaagaggcttataaatgccagagcaaaatgtgtctgcaataaccagtatcttacgccaggaaacacatctcccacggcttgcggatagagacacagcagccccgtcaatagtaacaacggcagcaatccatacatgacaccaacataggcgacctgctgtaagggattaaatttagactgggttgttgccgggaaaggatgttcttccccctgcataatgccaaacaaataaaatcgcgtttgttttgccgctcgttccagccacccctgacgacgaatgcgatagtggtgaccattatccccaacggcattgatcagcacaaagccgagccagcatgccagtaacaaaaatccgcaaacttcatgcaccgcaaccagacttttaaccgcagttgcgcccaccatcgcaaagtgatttatcagcccactggccagcaacaatacaaagagtaacgcattcgaccagtgccataatctgaccgctttgctgtaaagataaatcttctcaccatgatcggtggctgatttcttcacgccacgagcacgaagcaaggcatgcagccccagcaccaaccacatcccaaccagcaatactccggcaatgatcaaccacaccggccaaaattcgggagtgaactgtggcacatagttcgctaactggctctgaaactgttcagcatgttgcgacgggttcatacattttcctttttaatcaaatgttgaccgaaccggcgatacagatgcggtttcccggcaccaggtagctgatattgatagtatttattttgctgcaaccacgcctgaatttctgggctatcttcgcgaccaaagatcaatgcgtgttccgggcaggcgctgacgcaaatgggcggaaagccttttgccagtcgggactcagcgcagaaatcacatttatctgccactttagtgacagggttaaggtagcgaacctggtacggacaagcgccaatgcaataactgcagccgatgcactgcgatttttctacccgcacgatcccctgctcatcacgccacgacgcccccgtcgggcaaacgtcgatgcacggagcatcttcgcagtgctgacatgactggcgaaaaaagtgatactgcgtttcgttgtcgttatcggtgactggaatgtgtgctatcgataaacggcttccctgagcggggacgtggttagttttacggcatgcgcgggcgcaaatattacagccattgcaccgtgactcgtcatgaatcatggcataccgaacttccttttcttgcctcgtgttcgctaacagagaagacgcagaaccagtaaaaaagattactgttcccatccccagaacaaatttgcgtcgagtgaaggacatctgattatcccctaatgcagtggctgcaactgtccaccctatccatgacatctccctgaaatttcaggggttctgaaactgctctacctcgaaccattcgcataagccataagccttgccataggtcataaatcgctcgctaaacaagtacaacaccgccgtcgatgactccacctgccgtatatcggcatattcaggtgcaacatccatcgcggcgatcgcggcttcaatctgcgcttcctggaagtaatatggcgcttgcatcagcatggcgactttgtaaggacgaggatacgtctggcactcaaaacgaacggcgtgtgcaatggcgcgacaaatgtcctgctccacaacttgcaaagacatcgccgcgtagttttcactcatggcctgcgttgagtaatagtaatcatccttgcttcccgtcaaacaagcgatatccgcgtagtctccgttctgcttaatgctttccagcaaaactgacagttcctcttctgcaaccaaatagggtggcgagagaaacacggcgcgcgccaccagctgcccagccgcagaatgctggcgaatgaactcagccaggatttcagcaggttctggttcggttaccgtatcaacggggtgacgcatcccctgcaaccattgccgcttcgcctcgtcaacttcgctgactttcgctaacggcaattcatcctgatggttcatcttacccattccttacgcaggcagtagattgtgtgctgccagatcggcggcaatatcttccagccccagacgctgcaatgtttcgcgggttggacaaccaagctgtgggtcccagcccatttctttgtagaacatcgtgagcgaagcatgcatatcgtcacgatccattttgtcagtaccttcagtaaagaccgggatctgcggatccttgtcgaatacccaggaacagataagatcgtgttcattacgcatatctttggtttgcatcagttttaccgtgtaggcacgatgcaacgtaaaaatacgctctgcagctaaatctaatttttcctgagtcatctcttcgccggtgatcgctttgaagaatttggcttcaagcgccagatcgccccggtaattacggcttttcagcggcgaaacggtcattggccagacccagttgcacagggtgacggcgttatgcaaacagacccgcaacagcgaccactttgcatatttaatttttgcgtcattgattggcgtgtagtttttggtttcatcgtaagcatcttcagaaccaaaaagttctttcgccacttcacgttgcagtttcaatggcaagccggaaccaataaagttgatatgggtatgcgtcatgcagtcacggttgaacatacagttaacaatggaaccgacctgcgctgacgcttcattggcatggtgaaccggatagccaaacggcgaccagagtttatttttcgcgtagccccagtactcttcacccaaattccagcgttctgcgatggcatatgaaccatcagccaggtgactcagctcacccacacgatgcgccagacggtagtaaaaatctttaatgaagttaacgtcacccgcttccagttgatcccagcgaatttctgcatactcttcagctggcagaacacgcttgaacacacctttgctgtaacaataagtaaagtcgcgatgcaactgcccgtagttacaccataggccgtagtcatcgaacaaattcagacccaccaggttaccaatcacacgaccatcgtctttatcttcaaaatctttcggcccgttcgggaagatggtggtatggacaaagtttgctacacaagtgttaccacctgtgctgggcacgccaaactctttcacccgaggaatattcatttgggtcatacaacggatcgggcaagagtggcagccgctcatttttactgtgtatttctctgccgccggtcctaagtcaaaaacggatttataggtacgaaagccgaccgtattctgattgcctggcggaatttcacccgtttcaatcggaccaccttcagccgcgccccaaaacagccctttacgtgctgtccagcgtgacttgggatctgaatactctgcccacgattgtggcgtacttggcacgacatggttgttattcgcaccaataagttcagtcatcatgtaatcattgagacgcttcatctcctgacgatcggcaatgttgacccctttcgtcccttcaaccgcaatcgctttcaggtttttcgaacccattattgcgccagttcccgcaccgccgctgtggttacggctattcaacatgccagagagaggaacaaggttttccccagcctgaccaatagccgccacacaggtttccggactggtcaatcgacaaatttcttccgtcgttgcgcgcgtcccttttccccataagaaatcggctttttccaggctaactttgtcatctttaatcttcagccataccggtgatttcgccttcccttcgataataatgacgtcgtatccagcgaatttcatttgcgctgcaaaaaagccacccatatgggcatcgacgactaaatttcctttggtaaaagtagaaagtgaggtgatatttacgcgagaactacagggggcaccagatccagttaatgggccggtagcaaagactaatttattcgcttcatcgaaaggtttcgtgcctggcggtacttcgtcatacataattttgtagccgaagcccatgccaccgacaaaacttttaaacttactggaatcttcgagggtaatatttcctgtcgtgagattgactcttaatatattacctgtccaaccgttagccatgattttttcctttgcaagattcacacagtaatatctttccactcgataatttttaacgcccctgttgggcaggcgtttgcgcattcaccgcataacacacatttcgaggattttttactttcggtatttacggtggccatcatccacgggcatgccgtagtacaggcgctacagccaatacagcgtttatgatcgacggtaatacagccttctttctgctgccaggtaatcgcaccaatcgggcagacgttcatgcattgcggctctttgcattgacggcaggtgtccgcggtatagttgagatcgccatacaggccgccgccagagccaaccccgttgtcgccaaagaaataattgcgatggattttgatacgggagaagaatgtccctactgagccatcgttgaagttggtacaagagatttcacagcggtggcaacccgtgcatcgcgctcgctgggtcaccagcacccctttgggggtatttatcaaccctactgtgccgctatcaatatcttcctgtttgcaacccaaaagtgacagtaacgcaggggcaattgttagaccagcaaggccttttcctgatatacgcaagaattctaatcgcgttaagccaatatctaatagtggacgatcaaccgggttcatttatttcgcatcctcttcgcaaacacagtgctgacaattcagcagcctgatattaagcattcaactaatacgctgctgactctgtccccaacaccagatattttccctaacccgatagtgtatgagaaaagattaacgccgataaactaatcctttatggttaggagaaaaaataatgtgattattctgagcccttaacattgatcgttatcaattaaaattacaaagcaagaaattataagtgaactgatatttattatcatttgaaataaatttaacttaagcgacaattatttgtgactttcattgcagaaaataaaaataacattatcgctataaattaaaatacataccgaaattcgtataatttcagcagttgttatttagaatgattaactggaccgcaactgaagcaagaatatcaggatgaagcttaccgcctcatcctgaatggtcattttaccagtgcgttaatgacggtttccatcgcctgcttttccagctcactgcgctgaatgcgtttattggctaatgctgtacgtaatacgcctgcgataacaatatgctttggttcctgccccagatcgcgcatttccagcacaactttaccgacaactctgcacatttctcggtacagttcatcctcttttgtccgatttcccattctttatacctatttatcatgccaactatcagcatatatcaatctaaccaattaaacaaaaatcaaacaaaatcagacaaataacgcgataaattattttaactgtagcaattgagcgatgatatatttatacaccggatgaactttcacttatcctcacactgacaacttcggcaccagacgttgcgcaaacagtgaagtttttgcgtaaccttttccctggaacgttaaatctttgataacaatttattgtctaacaagttgtatattttttgaaacgctgtttttgttttccttttggattaatttcagcgtataatgcgcgccaattgactcttgaatggtttcagcactttggactgtagaactcaacgactcaaaaacaggcactcacgttgggctgagacacaagcacacattcctctgcacgctttttcgatgtcacctatccttagagcgaggcaccaccactttcgtaataccggattcgctttccggcagtgcgcccagaaagcaagtttctcccatccttctcaacttaaagactaagactgtcatgaaaaagaccaaaattgtttgcaccatcggaccgaaaaccgaatctgaagagatgttagctaaaatgctggacgctggcatgaacgttatgcgtctgaacttctctcatggtgactatgcagaacacggtcagcgcattcagaatctgcgcaacgtgatgagcaaaactggtaaaaccgccgctatcctgcttgataccaaaggtccggaaatccgcaccatgaaactggaaggcggtaacgacgtttctctgaaagctggtcagacctttactttcaccactgataaatctgttatcggcaacagcgaaatggttgcggtaacgtatgaaggtttcactactgacctgtctgttggcaacaccgtactggttgacgatggtctgatcggtatggaagttaccgccattgaaggtaacaaagttatctgtaaagtgctgaacaacggtgacctgggcgaaaacaaaggtgtgaacctgcctggcgtttccattgctctgccagcactggctgaaaaagacaaacaggacctgatctttggttgcgaacaaggcgtagactttgttgctgcttcctttattcgtaagcgttctgacgttatcgaaatccgtgagcacctgaaagcgcacggcggcgaaaacatccacatcatctccaaaatcgaaaaccaggaaggcctcaacaacttcgacgaaatcctcgaagcctctgacggcatcatggttgcgcgtggcgacctgggtgtagaaatcccggtagaagaagttatcttcgcccagaagatgatgatcgaaaaatgtatccgtgcacgtaaagtcgttatcactgcgacccagatgctggattccatgatcaaaaacccacgcccgactcgcgcagaagccggtgacgttgcaaacgccatcctcgacggtactgacgcagtgatgctgtctggtgaatccgcaaaaggtaaatacccgctggaagcggtttctatcatggcgaccatctgcgaacgtaccgaccgcgtgatgaacagccgtctcgagttcaacaatgacaaccgtaaactgcgcattaccgaagcggtatgccgtggtgccgttgaaactgctgaaaaactggatgctccgctgatcgtggttgctactcagggcggtaaatctgctcgcgcagtacgtaaatacttcccggatgccaccatcctggcactgaccaccaacgaaaaaacggctcatcagttggtactgagcaaaggcgttgtgccgcagcttgttaaagagatcacttctactgatgatttctaccgtctgggtaaagaactggctctgcagagcggtctggcacacaaaggtgacgttgtagttatggtttctggtgcactggtaccgagcggcactactaacaccgcatctgttcacgtcctgtaatattgcttttgtgaattaatttgtatatcgaagcgccctgatgggcgctttttttatttaatcgataaccagaagcaataaaaaatcaaatcggatttcactatataatctcactttatctaagatgaatccgatggaagcatcctgttttctctcaatttttttatctaaaacccagcgttcgatgcttctttgagcgaacgatcaaaaataagtgccttcccatcaaaaaaatattctcaacataaaaaactttgtgtaatacttgtaacgctacatggagattaactcaatctagagggtattaataatgaaagctactaaactggtactgggcgcggtaatcctgggttctactctgctggcaggttgctccagcaacgctaaaatcgatcagctgtcttctgacgttcagactctgaacgctaaagttgaccagctgagcaacgacgtgaacgcaatgcgttccgacgttcaggctgctaaagatgacgcagctcgtgctaaccagcgtctggacaacatggctactaaataccgcaagtaatagtacctgtgaagtgaaaaatggcgcacattgtgcgccattttttttgtctgccgtttaccgctactgcgtcacgcgtaacatattcccttgctctggttcaccattctgcgctgactctactgaaggcgcattgctggctgcgggagttgctccactgctcaccgaaaccggataccctgcccgacgatacaacgctttatcgactaacttctgatctacagccttattgtctttaaattgcgtaaagcctgctggcagtgtgtatggcattgtctgaacgttctgctgttcttctgccgatagtggtcgatgtacttcaacataacgcatcccgttaggctccacggaatatttcaccggttcgttgatcactttcaccggcgttcccgtccgcacgctggagaacaaggctttaatatccggtgcattcatgcgaatacaccctgaactgacgcgcaaaccgacgctgtccggcgcactggtaccatgaatgaggtattcgccattaccatgcgcgaggcgcagtgcgtaacgtcctagcgggttatttggtccggcaggaacgactggcggtaatttaatgccacgctccagcgaacgctgacgaatgcctgccgtaggcgtccaggttgggttagggattttctgcccaacacgcgtttccatcaccggcgtttccagcccctgcaatccaatacctattggataaacctgcacaatattttctcccggcggataataataaaggcgcagctctgcaaggttaacgataatcccctgacgcggtgcatcaggtaataacagttgtgaaggaatagttatcgtcgtaccaggttttggcaccggggcgatagtgttattggcttcaaggatcaacattgccgcagtatcaaaacgtcgggcaatagcctgaaggtttttatccccttcttgcaccgtatacgtttgattttgcccaaccagtcggcttccggttggtggtagcggataatcaaccgcccaggcagcctggatggcgctaaaagcgccgataagcgtgagtgtaagcaaagacgcgcgtttcattgtaaacctcctgtatttgccggagactcacgctgaaacgtcggatggcgcttatgttcacctgaaaccaaaacactcctgtgcaggtcagtgtaaacattgaccatccggcaatgtgagccaaccggatgaaagctgtccttttagtttagctaagtgcagcggctttggcgcgaattgcgcgaatcatcgcttccagaccttgtgaacgagatggggtgagatgttgggtgagcgccattttttcaaaccacggacgcacatcgaaattgacaatatcctgcggcgtcatctgatcgtagagaataaagacgaccgcaataagccctttcacaatcgccgcatcgctgtcgccctgtaattcaataattccctgggcattctggcgcatgacaatccacacctgactctgacagccctgaatgctattttgtggacttctgtcttcgtcgcgtaattctggcagacgctggcccagctcaataatgtagagatatttctcttcccagttggcgcagcgtaaaaaattacgcagcaacttttctttatccggcaataaagccatagtgcctccctgttatcccagcaaacggtgaatacgttgcaggccggtcaccagacgatccacttcttcatgggtgttatacatggccagcgacgcccgacacatcgcagggacgttgtaataggccatcaatggcattgcgcagtgatgtccggtacgcacagcaatgccgtaattatcgagaaaactgccaacatcataggcgtggtgtttaccgagattaaaagcaataacgccaagcctgttttgtgggccatagagagtgagatccggtacagattccagctgtgatagcgcataatgcatcagattctgttcatactcggctatgttattaagccccagcgccgaaacatactccagcgccgcgccaagaccaatgatgcccccggtattgggtgtaccggcttcaaaccgccatggtgctttggtccaggtagtgccttcactcaggctgacggtggcgatcatagaaccgcccccttcccacggcggcatctcctgcaacaaggcttctttcacataaagaatgccaattccggtggggccatacagtttatgcccggagaacacgtaaaagtcgcaatccagcgcctgaacatccaccggatgatgcatcaccgcctgagcgccatccaccagcacttttgcgccatgctggtgcgcaagcgtgatcatttccgccagtggattttctgtgccaagcacgttggagacatgagtaattgccagcaggcgagttttctcatcaaacagcgtaggcagcgtctccagttgcaacgtaccatcgggattgagcgggatcacacgcagctctgcgccaacgcgtgcgcaaagcatctgccagggaacaatgttagcgtggtgctccatctgactgatgatgatgttatcgcccgcccgcacgttgctgttgccccagctattggcgaccagattgatcccttccgtcgtgccgcggacgaacaccagctcttccgccgaacgggcattaataaacagcgatgcccgcttgcgcacgttctccattttctcggtcgcctgggcgcttaaggtatgaataccacgatgcaccgccgcgtagccatgacgataaaactcggcctcggcgtcaatcacctggctcggtttctgcgcactggcggcgctgtcgagataagccagcggcaaaccgtttacctcacgcgaaagcaccggaaagtcggcccgcactttgtcgacggaaaaaatcatcttgcacctcctggcagccgttgaccgattcgggccagcacctgctgtttaagcccctcatcacgcagtgcttccgtcagttcggcagcgaaggcgtaaatgatcatctgctgggcatcctgctgattgatcccgcgcgagcgcagatagaatatctgttcatcatcaatacgccccaccgtcgcgccgtggctgcatttcacatcatctgcatagatttccagctgcggtttcgtatccacttccgccagtttgcccatcagcagattgttgttggtcatctgaccatccgttttgatggcgtgctgcgcgacgttgatcaaaccgttaaataccgcgcggcctttgtcgctgacgatagttttgtgcaactgtcggctgttacaaaaacctttattgtgttccagccaggtacgggtatcacacacctcgtttttcaccggcatcgccaggctattgatccgcagcgtgctgttttcgccattgagttgcgtactggtgttgtgtcgtaacactgcgccacccagcaggaaactgtggctaaatgcggtggcatcctcagccagcaacaaatcgttatgagcaaagtggtgactgagcgggttttcaaacgccagcttgatatgctgcaagtgggcattcgctgcgacgttgatagtgaaccgtgccccggtaaaatgacgagcatcattcaggctgacaaaatgttcgatcaccgttgcttcggcaccttccgccagatccagatgatgtcggtaatgggcagtgttcacctcttcacctgccacgccctgggtgatatgcattaacagcaatggctttgccggccgttgaccgcgcttcacggcgatatgcgtcacgctttgtgccaggctttccgtcaaatgcagaaacacttccgcctgaatagcgtcgggtaaaccctgacggtcgtcgttaatgctcacttcatatccgctgccttcagttgcatcgctcagtgcgggcacgtaacgcccatcgacaaacaccagccgcacggagtctaacgttaacgctaaggcatcacgctgctgtggggatatctctcccgcaatgctgacaaactggctattgatcagcccttccagcggcgtatatttccagttttcatgtttacgtgtcggcagtccggtacgcagcaattgttgtaaatgctgctgtgcttgcggggagcgttttgtcccttcagcttcaaacaagtgatgccactgttgcagcgcgttactgctgttcggtaagccagccataaccctgctcctccagttgtttgaccaacgtgaaatcgccggatttcacaattcgtccctgatatagcacatgaacgtaatcaggcttgatgtagtcgagaatgcgttggtagtgcgtaacaatgatgaatgagcgcttgccatcacgcagcgagttcacgccatcggcgaccacttttaatgcgtcaatatccagcccggagtccgactcatcaagaatgcataactccggttccagcaccgccatttgcaaaatatcgttgcgctttttctcgccgccggaaaaaccaacgtttaccgaacgggttaataaatcttccggcatcttcaggagagcgattttctcttccatcaaatcctgaaaatcaaagcggtcgagcgtttcctggccgcgatagctgcgcaccgcattaagtgccgtttgcaggaaaaactggttactgacacctggaatctccaccggatactggaaggccataaagatgccttcgcccgcgcgatcttccggcgacagcgcaagcaaatctttgcctttgaactcaaccgtgccgcccgtcacttcataatcttctcgcccggcaagcgttgccgataaggtacttttgcccgaaccgtttggccccataatggcgtgaacttcgccgggatgaacgtcgaggcttaatccgcgcaggatagctttatcttccacgctgacgtgtaaatctttaatacttaacatgtttattccttatccgacgctgtgttcaagactgatggcgaggagtttttgtgcttcaacggcaaattccaacggcagctccgagaacacgtctttgcagaaaccgttaacaatcatcgagatggcgtcttcttcgctgatcccgcgttgcaggcagtaaaacagttgatcttcaccaatacgtgatgtcgttgcctcgtgttccagttgcgcactattgttacgacactcaacatacgggaaggtatgcgccccacaattagcgccaatcagcattgagtcgcactgagtgaaattgcgcgcattggttgccgtcggcatgattttcactaagccgcgataactgttctgactatgtccggcagagatccctttcgagataatggtcgatttggtgtttttaccgatgtggatcatcttggtgccggtatccgcttgctgatgaccgctggtcagcgccactgagtaaaactcaccaatggagttatcgccgcgcaaaatgcagctgggatatttccacgtaatcgctgacccggtttctgattgcgtccatgacattttgctgttttcgccttcgcacaaagcacgcttggtgacgaagttgagaataccgccggtgttgttatcgccaggaaaccagttttgtaccgtggaatatttcacctcggcgtttttatggatgatgacttccaccactgccgcgtgtaactgatagctgtcacgcaccggagcggaacagccttcaatgtagctgacgtagctgtcttcgtcggccaccagaatggtgcgctcaaactgcccggttttttctgcgttaatgcgaaaataggtggaaagttccatcgggcagcgcacgcctttaggcacataaataaacgtaccatcagaggctaccgccgcattaagcgcggcaaagaagttgtcattccccggcaccacggtgccgagatatttacgcaccagttccgggtgatcgtggatcgcctcaccaaaggaacagaaaataattccctgctccgccagtttttcgcgataagtagtggcaaccgaaactgagtcgaaaatggcatccaccgccacctctttgccttcccgcacgggaacgcccaactgctcaaacgccgcctccacctctttacttaaaaaggcgttcgcgccagtttgctgcaccgcgccaggttcagacgcgcaagtgtcgtcacaattaccgcacgatggtgctgagtagtagctgtaatcctgataattcagcttgtcgtagtgcgctttcaaccagtgcggttcttccatctccagccatgcgcgataggcgtttagacgaaactccagcatccactccggctcattacgcttcgccgaaattgcgcgcaccacctcttcgtttatcccctttgccagctcatcggtggctaactgggtgaagaatccttctttataattcagcgggccgccggtccaggttttgacatcgtcagttgcttcagtattacgagacatagtaccgcctataccccaaagctttcgccacagccacattcattctgggctttagggttgtgaaatttgaatatctgattaagtccttcacgaacgaaatcgacttccgtgccatcaataaacggcatcgcttgcagcgggacaaacagcttcgcgccgtcgtgttcaaacagcagatcgtctttgtccggctcgctaacactgtcgagcacatagccaaagcccgcgcagcccgtttgcttcacgcctaagcgcacgccgaccatacccggctgctttgccaccagctcacggatgtgtatcgccgctgcgggtgtcagcgttaagccttgccaggcgaaatcttgtgggttaaaggttcctgaatgcatgtccatcgatttacctcacttcatcgctttcagcgtataacagcatgttagtgataatgattatcagttcaacccagcaaacgcaggggctttaccgtaaaacatgctttttgcctgcttttaataagcatagaccctgatgtgtgggttaacaggcacgctaagaattaggtatctcattgttagataatggttattatctaaggagcattaaggctgtgatgaaaaagaaaaagttgtattgaaaatgactatttaagagataggtaaaaaagtgcagcgttcagaaataagaaaacccttaagtctgtgcgacacaggcttaagggtttctaccccatccggcgcttatctccggcactctcagtggcttagctcttgaaggggcgataagaataatctcataaagctaacccgccgttttaacacaaactgcgattagtattatttttgaacaatatcaggcggtagataagcagtattaagaaggtcatcgaacctggacggaggttaatccaggtcgatttggcgaacttgcggcattaagtcaggatcaatgcacgcccagacgccaggcaaagtagatttcttcttttaattcagcagaagagagagtaagcaggtcagcaaattcaagttctagttgtttcagacgtttgagatattgggcaggtgaaagattgctctggtcacggcgtaaaaattcaatggccagctgggtgggatcaagttgagtagacatagcatcctcgcttttagacaagacctgcacagtataccaccgtttactgtgcagataatgaccaaaagcaatatgcgtcacacttttctggtgacaacgtcacaaaatggcggtcgtcaatcgtgacgaacagcacaaacgccctttctcatcgaagatttcaatctgccagacctggtgacgcgaaccgagatgcaacggtttgcatacgccgcgcacccgcccttctcgtgccgagcggacgtggttagcattgatttccagaccaaccactttttgctcaccttcggtacataaataaccggcaacggaaccgatactttcggccagtaccacggatgctcctccatgcagcaacccgaaaggctgctttgtccgcgagtctactggcattgtcgcttcaagggtgtcatcaccaatatgttcaaagcgaatatccaggaaccccaccatgtttccttcacccatagcattcagtgcttccagggtgattttccgtttccatatcatttaataatctccagtaaagcctgcacaggatggcgtacccccgtgccttcaacccgttttacctggctacggcaggaatatccggtcgccagacagcggttacgcggcagtcgctgcatagcctgatgccaggataactcatagatcccgagcgaattttcatggtttttcgcttcatgtccgtaagtccctgccatgccgcagcaacccacgctgacattttccagtttcgcgccaaaacgggcaaatatcgcggcccattgtgctggcgcacccggcaaggcggtaacttcggtacagtgaccaaagaaataccatgattcaccgctgactgtagccactggctgtgactcaagtgcgcttgccagccattcattcgccagtaagacgttaaactcgccacgctcctcgcccagcgccagtttatattcatcgcgataacaaagtaccagcgccggatcgacgcccaccattggcatacccagcttcgccatacggttgaggaaatccgccgtctttttcgccgtcttcgcaaaacgattaagaaaacctttaatatgctgggctttgccatttggcgaaaatggcagtaacacaggctggaaacctaatttttcgaccagacggacaaaatccgccaccacttgcgcatcgtaatagctggtaaaggggtcctgcaccaccaacactgtgcgcgctttctgctctgcattgagagattcaagctgttccagcgtcatgtttgccgagcgatgccccaccatttgttgttgtagcgaggggaccgacagcagcggcaaatcaaccatgccgatatgtttttccgagagtttgcgcaccagcggctggttaatgaagaagttaaaggttttcggcgcgcgtgccatcagcggcgcgtagctctcgaccgtagcgacgaggtggtcgcgcagcgggcgtaaataacgggtgtgatagagctgcagaaaacgagagcgaaactccggcacatcaattttgatggggcactgggtcgaacacgctttacaggccagacagcccgacatcgcctctttgacttcgtgtgagaagtcatattcgcctttattcgcatgccagctattgcgcgtgcgggcaattaacgtccgcaaactgacgccggattcaggcagttcttgttccagtttgagtggatcaacgccgcgatccgccaacaaacgcagccattcacgcaccagcgttgcgcgccctttcggtgaatgaatccggttctgggtgatcttcatcgacggacacatcggactacgggcatcaaagttgaagcataaaccgttgccgttacactccatcgcaccgcgccactgctggcgtaccgcaatggggatctgccgatcgaatgtaccgcgcttcaccgcgtccactttcatcatcggcgcatcgagaccttctggcgggcaaatcttccctgggttgagtcggttatgcgggtcaaatgccgctttcactttgcgcagttctgcaaaaagttcctcaccgaaaaacgccgggctgtattcagcgcgaaaacctttgccgtgctcgccccacaacaaaccaccgtatttcgcagtcagcgccaccacgtcatcagagatttgcttcatcaaaatctcttgttgaggatcgcacatatccagcgctggacggacgtgcaagacacctgcgtcgacgtgaccgaacataccgtagcttaagccgtggctgtcgagcagcgcgcgaaattcagcaatataatccgccaggtgttccggcggtacgcaggtatcctcagcaaacggaattggcttagcggcacctttggcattgccaagcagaccaacggcttttttgcgcattgcatagatacgttcaacccccgccagctcacggcacacctgccagccgatgacacctgcttgatgactggcgatcagctcatccaaccgcgcacagagtgcatttacccgctcatcaatcagcgcctcatcatcaccagcaaattccacaatgttcagcccgagcatctcttggtcaggcacatcggtaatcaactcgctgacggaatgccagacaatatcttcccgcgccagattcagcacttttgagtccaccgtctctaccgaaagcgcccgcgcctcaaccataaacggcgcgttacgcagcgcagagtcaaaagagtcatatttgacgttcaccagacggcgcactttaggcaagcgtgtaatatccagccgcgcttcggtaataaaggccagcgtcccttctgaacccgtcagaatgcgcgtcaggtcgaactcggtcatctcatcgttaaagacatgacgcagatcgtaaccggtaagaaagcggttaagtttggggaagttgtcgataattaactggcgttgctgacggcaacgttgataaaccgtgttataaattcgcccgattgtggtattggatttacccagcgtttccgccaattcgacgggtaaaggttgcgtatcgagaatatcgccccccaacaacaccgcgcgtacgccaagtacgtgatctgacgttttgccatagaccagcgatccctgaccggatgcatcggtattgatcatcccaccgagcgttgcccggttgctggtcgaaagttccggcgcaaaaaagtagccgaacggtttcaggtactgattgagttgatcttttatcaccccggcctcaacgcgcacccagccctcttcagggttaatttcgatgatgcggttcatatggcgggacatatcaacaataatcccctggttgagcgcctgaccgttagtgccggtgccgccgccgcggggggtaaagatcagcgatgaatagcgttcctgcgcggcaagacgggcgatcagcgccacatctgcggttgaacgcggaaataccaccgcatcggggagaagttggtaaatactgttgtcggtcgacattgtcagacgatcggcataacttgtcgccgtatcgccggtaaaaccttgttgctccagctcttgcaaaaaattaagcaccagttgaacgacgccgggtgcctgggaaatctgtggaatcattatattgaccctttcctgcggtctgtgatgtaggtcgatacactattctttcaggctgctgcaatagcgcactgaaaggtgatgtttgtttactctatggatttcgtgttgcaggaaggcggcaagcgagtgaactccaggagcttacaatagtaagtgactggggtgaacgaacgtagccgcagcacatgcaacttgaaatacgacgagtaaatcgtttgcgtgttgcctgagttgttgtaccacatttttttctaacacgcccatcagaattaagggcagaatcggcctgttaaaaaccgctgaaattgctcatcattatgcaggtgagtttcgcgtgttcacgtcgcgtcgacgatttgacgcacaaaaaaggtgaaaagtagttatggtaaatgttcgtcagcccagggatgtcgcacaaattctgctttcggtgctgtttttagccatcatgattgtggcatgtctgtggattgttcaaccctttattctcggctttgcatgggccggtacggtggttatcgccacctggccggtattgttacgtttgcaaaagatcatgtttggccgccgctctctcgccgttctggtgatgacgctgttattagtgatggtgtttatcatccctattgctttgctggttaacagtatcgtcgacggcagcggcccgctaattaaagccatttccagcggtgacatgacgttacccgatctggcgtggcttaataccattccggtgattggcgcgaagctgtatgcaggctggcacaacttgctggatatgggggggacggcgatcatggcgaaagtccgcccttatattggcaccaccaccacctggttcgttgggcaggcggcgcatatcgggcgctttatggtgcattgtgcgctgatgcttctcttcagtgccctgctgtactggcgcggtgaacaggtggcacaaggcattcgccattttgcaacccgtctggcaggcgttcgcggagatgccgccgtgctgctggcggcacaggctatccgcgcggtggcgctgggtgtggtggtgacggcgttagtacaggcagtgcttggcggtatcggcctcgccgtatccggcgtaccttatgcaacgttgctaacggtgttaatgatcctctcctgccttgtccagcttggcccgttgccggtactgattccggcgattatctggctctactggactggcgataccacctggggaacggtattgttagtgtggagcggtgtggttggcacgctggataacgtcatccgcccaatgttaattcgcatgggtgccgatttaccgctgatcctgattctctctggcgttattggtggtttgattgctttcgggatgatcggtctgtttattggtccggttctgttagccgtttcctggcgtctgtttgccgcgtgggtggaagaagtcccgccgccgacggaccaaccggaagaaattctcgaagaacttggcgaaatcgagaaaccgaataagtaatttctcatcaggcggctctgccgcctgattgttaaccaccgctaattgatatttgcttgctcttccccatattttcctgcttaccgccattcagctggtagtacctgtcgcaaattctttacagtttttaaactaatgagacgaatctgatcgacgcaaaaagtccgtatgcctactattagctcacggttataaatcaacatattgatttataagcatggaaatcccctgagtgaaacaacgaattgctgtgtgtagtctttgcccatctcccacgatgggcttttttttaacatttttccgcttcgctacctcgcccctcactctttccaataatgttgcacaagatactgtgactctcttcaagccgtcagcaggctgataatgttatttatattttattgtttatttcatgcagccattacacgatgaacgcttatgaactccaggcactccgccatatttttgccatgactattgatgaatgcgcgacctggattgcccagaccggtgacagtgaaagctggcgtcagtgggaaaatggcaagtgtgccattcctgatcgtgtagtcgagcaactgttggctatgcgtcagcaaagaaaaaaacatcttcatgccatcatagagaaaataaataaccgcatcggcaacaacaccatgcgttttttccccgacttaaccgcatttcaacgagtctaccctgatggcaattttattgactggaagatctatcaatcggtagctgctgaattatatgcacacgatctggagcggctttgttaatttttccacagaaaggaattgtcgttgttacaacaataatgaacggatgctgacacaacatcgcttcactttttaaagcacctttgctaagtagaacctatgaaaaatccctatttccctaccgcacttgggttgtattttaattacctggtgcatggtatgggcgtccttttgatgagcctgaatatggcctcgctggagacactttggcagactaatgccgcgggtgtctcgatagttatctcatcgctgggcattggtcgattaagtgtcttgctttttgcaggattattatccgatcgctttggtcgccgcccttttatcatgctcgggatgtgctgctatatggccttcttttttggcatcctgcagaccaataacatcattatcgcttatgtttttggctttctggcgggaatggcaaacagttttctcgatgcaggcacttatcccagtttgatggaagcttttccacgctcacctgggacagccaatattttaattaaagcatttgtttccagcggacaatttttattaccgctaatcattagcctgttagtgtgggctgaactgtggttcggttggtcctttatgattgctgcaggcattatgtttattaacgctctgtttttataccgttgtacgttcccaccccatccgggtcgtcgcttacctgtcataaagaaaaccaccagctctacggaacatcgctgttcaattatcgatttagccagttataccttatatggctatatctcaatggcaacgttttatctggttagccagtggctggcacagtacggacaatttgttgcaggcatgtcatacactatgtcgatcaaactactcagtatctacaccgtgggttcgctgctttgtgtatttattaccgctccactcattcgtaataccgttcgcccaacaacattactgatgctgtacacctttatctcatttattgctctgtttaccgtctgcctgcatcccacattttatgtggtgataatatttgcttttgtcattggttttacctctgctggaggtgttgtgcaaattggcctgacgttaatggctgaacgtttcccttacgctaaaggtaaagctacagggatctattacagtgcgggcagtattgcgacctttactattccgttgattacggctcatctgtcccaaagaagtattgccgatattatgtggttcgataccgccatcgctgccatcggttttttactggcactgtttatcggcttacgcagccgcaaaaaaacgcggcatcactcgctaaaggaaaatgtcgctccgggtgggtaatgcaatattcttttcaggtcatgcaagatcttacggataaataactctttctgcgctaactaaggaaaatcgcgatcaaaaacaaactatgacatgcaatattcctggaaacataaactttatgccatgtacccagggaaaatcatcttcagtatagtaattatgtaaaccgtcggagaacaatacgtacggtaacgaaattatctttcagcaaggagctgtgaaaatgtctcaaaataaggctttcagcacgccatttatcctggctgttctttgtatttacttcagctacttcctgcacggcattagtgttattacgcttgcccaaaatatgtcatctctggcggaaaagttttccactgacaacgcgggcattgcctacttaatttccggtatcggtttggggcgattgatcagtattttattcttcggtgtgatctccgataagtttggtcgtcgggcggtgatattaatggcagtaataatgtatctgctattcttctttggtattcccgcttgcccgaatttaactctcgcctacggtctggcagtgtgcgtaggtatcgctaactcagcgctggatacgggtggctaccccgcgctcatggaatgctttccgaaagcctctggttcggcggtcatactggttaaagcgatggtgtcatttgggcaaatgttctacccaatgctggtgagctatatgttgctcaataatatctggtacggctatgggctgattattccgggtattctatttgtactgatcacgctgatgctgttgaaaagcaaattccccagccagttggtggacgccagcgtaactaatgaattaccgcaaatgaacagcaaaccgttagtctggctggaaggtgtttcatcggtactgttcggtgtagccgcattctcgaccttttatgtgattgtggtgtggatgcccaaatatgcgatggcttttgctggtatgtcagaagctgaggcattaaaaaccatctcttattacagtatgggctcgttggtctgtgtctttatttttgccgcactactgaaaaaaatggtccggcccatctgggctaatgtatttaactctgcactggcaacaataacagcagccattatctacctgtacccttctccactggtgtgcaatgccggagcctttgttatcggtttctcagcagctggcggcattttacagctcggcgtttcggtcatgtcagagttttttcccaaaagcaaagccaaagtcaccagtatttatatgatgatgggtggactggctaactttgttattccactgattaccggttatctgtcgaacatcggcctgcaatatatcattgttctcgattttactttcgcgctgctggccctgattaccgcaattattgtttttatccgctattaccgcgttttcattattcctgaaaatgatgtgcggtttggcgagcgtaaattttgcacccggttaaacacaattaagcatagaggttaaaggagttaattatggatgttaccgcaaaatacgaattgattgggttgatggcctatcctatccgccacagtttatcgcccgaaatgcagaataaagccttagaaaaagcgggattgccatttacctatatggccttcgaagtggataacgatagctttcctggagcaattgaaggattaaaagccctcaaaatgcgcggaactggtgtatcgatgccgaacaaacaactggcgtgtgaatatgttgatgaattaacaccagctgccaaactggtgggggccatcaacaccatcgttaatgatgatggctatctgcgtggctataacaccgacggcacgggccatattcgcgccattaaagagagcggttttgatatcaaaggcaaaacgatggtgctgttaggggccggtggtgcctcaacggcaattggcgcgcagggggcaattgaaggtttaaaagaaattaaactctttaaccgtcgggatgagttcttcgataaagccctcgccttcgcgcagcgggttaatgaaaacaccgattgtgtcgtcacggtcaccgatctcgccgatcagcaagcctttgctgaagccctggcttccgccgacattttaaccaatggcacaaaagtgggtatgaaaccccttgagaatgaatcattggttaatgatatcagtctgttacatccgggacttctggtcactgaatgcgtgtataacccgcatatgacgaagttattgcagcaggcgcaacaagctggttgcaaaacgattgatggatacggcatgttgttgtggcaaggggctgaacagttcacattatggactggcaaagatttccctctggaatatgttaaacaggtcatggggttcggtgcctgacaggctgaccgcgtgcagaaagggtaaaaaatgaaaaccgtaactgtaaaagatctcgtcattggtacgggcgcacctaaaatcatcgtctcgctgatggcgaaagatatcgccagcgtgaaatccgaagctctcgcctatcgtgaagcggactttgatattctggaatggcgtgtggaccactatgccgacctctccaatgtggagtctgtcatggcggcagcaaaaattctccgtgagaccatgccagaaaaaccgctgctgtttaccttccgcagtgccaaagaaggcggcgagcaggcgatttccaccgaggcttatattgcactcaatcgtgcagccatcgacagcggcctggttgatatgatcgatctggagttatttaccggtgatgatcaggttaaagaaaccgtcgcctacgcccacgcgcatgatgtgaaagtagtcatgtccaaccatgacttccataaaacgccggaagccgaagaaatcattgcccgtctgcgcaaaatgcaatccttcgacgccgatattcctaagattgcgctgatgccgcaaagtaccagcgatgtgctgacgttgcttgccgcgaccctggagatgcaggagcagtatgccgatcgtccaattatcacgatgtcgatggcaaaaactggcgtaatttctcgtctggctggtgaagtatttggctcggcggcaacttttggtgcggtaaaaaaagcgtctgcgccagggcaaatctcggtaaatgatttgcgcacggtattaactattttacaccaggcataagcaataatatttcggcgggaacaccctccccgccgaactaaaaaatatattcaatcgtatttaataaaaatatttcgtgagtctctgtgcgctaattctccatttggcgtagggaaaatcacatctgaatcaggaattaacaatgaaacctgtaaaaccacctcgtattaatggacgagtgccggtcctgtcggcacaggaagcggtgaattatattcccgacgaagcaacactttgtgtgttaggcgctggcggcggtattctggaagccaccacgttaattactgctcttgctgataaatataaacagactcaaacaccacgtaatttatcgattattagtccaacagggcttggcgatcgcgccgaccgtggtattagtcctctggcgcaagaaggtctggtgaaatgggcattatgtggtcactggggacaatcgccgcgtatttctgaactcgcagaacaaaataaaattattgcttataactacccacaaggtgtacttacacaaaccttacgcgccgccgcagcccaccagcctggtattattagtgatattggcatcgggacatttgtcgatccacgccagcaaggcggcaaactgaatgaagtcactaaagaagacctgattaaactggtcgagtttgataacaaagaatatctctattacaaagcgattgcgccagatattgccttcattcgcgctaccacctgcgacagtgaaggctacgccacttttgaagatgaggtgatgtatctcgacgcattggttattgcccaggcggtgcacaataacggcggtattgtgatgatgcaggtgcagaaaatggttaagaaagccacgctgcatcctaaatctgtccgtattccgggttatctggtggatattgtggtggtcgatccggatcaaacccaactgtatggcggtgcaccggttaaccgctttatttctggtgacttcacccttgatgacagtaccaaacttagcctgcccctaaaccaacgtaaattagttgcgcggcgcgcattattcgaaatgcgtaaaggcgcggtggggaatgtcggcgtcggtattgctgacggcattggcctggtcgcccgagaagaaggttgtgctgatgactttattctgacggtagaaacaggtccgattggcggaattacttcacaggggatcgcctttggcgcgaacgtgaatacccgtgccattctggatatgacgtcccagtttgatttttatcacggtggcggtctggatgtttgttatttgagttttgctgaagtcgaccagcacggtaacgtcggcgtgcataaattcaatggtaaaatcatgggcaccggtggatttattgatatcagtgccacttcgaagaaaatcattttctgcggcacattaactgcgggcagtttaaaaacagaaattaccgacggcaaattaaatatcgtccaggaaggacgggtgaagaaatttattcgggaactaccggaaattactttcagcggaaaaatcgctctcgagcgagggctggatgttcgttatatcactgagcgcgcagtattcacgctgaaagaagacggcctgcatttaatcgaaatcgcccctggcgtcgatttacaaaaagatattctcgacaaaatggatttcaccccagtgatttcgccagaactcaaactgatggacgaaagattatttatcgatgcggcgatgggttttgtcctgcctgaagcggctcattaacaggagtataatgatggatttttctttaactgaagaacaagaactgctgctggccagtattcgcgaactgattacgactaactttccggaagagtatttccgcacctgcgatcaaaacgggacatatccgcgtgagtttatgcgggcgctggcggataacggtatttccatgcttggcgtgccggaagaatttggtggtatccctgcggattacgtcacccaaatgctggcgctgatggaagtgtcaaaatgcggtgctccggcatttttaattaccaacggtcaatgtattcacagtatgcgccgtttcggttctgcagagcagctacgtaaaacggcagagagcaccctggaaacgggtgatcccgcctatgccctggcgttgacggaaccaggtgctggctcagataacaacagtgccactaccacttacacgcgtaaaaacggcaaggtctacatcaacggacaaaaaacctttattaccggtgcgaaagagtacccgtatatgctggtgctggcgcgcgatccgcaaccgaaagatcccaaaaaagccttcaccctgtggtgggtcgactccagtaagcccggcattaagattaacccgctgcataaaatcggctggcatatgctcagcacctgcgaagtctatctcgacaacgtggaggttgaagagagcgacatggtgggcgaagaaggaatgggtttcctcaatgtgatgtacaactttgagatggagcgcctgatcaacgccgcgcgcagcaccggctttgccgaatgcgcctttgaagatgccgcccgctatgccaaccaacgtatcgcttttggtaagcccattggtcataaccagatgatccaggaaaaactggcgctgatggcgattaagatcgacaacatgcgcaacatggtgctgaaagtggcatggcaagccgatcagcatcagtcactgcgcaccagcgcggcgctggcaaaactgtactgtgcacgtaccgcaatggaagtcattgatgatgcgattcaaatcatgggcggtctgggctataccgatgaggcgcgcgtctcccgcttctggcgtgatgtccgttgtgaacgtatcggcggcggtacagacgaaattatgatttacgtagcaggtcggcagatcctgaaagactatcagaacaaataatctgcaggcggcgcagcttcttaacaaactgcgccgccagatttatccaacaagacttaccggttgaggaaattcagataggatttcttgttccgcaaaacagtttttaaattgtctacggtaatcgctgggcgaacaaccgacatggcgcaaaaacagtttggcaaagtgatcgacattttcataacccacacgccaggagatctctgcctgtgataattcagtattagtgagtgaccattttgcttccgtcatacgccgttgaataacatagttaataggggaaatacgatactctttggtaaattcatggcaaatataactgacgctggcacgaaattttttcgataactgttctaaagtgattttttcgcgataattattattcagatagaaaagaatatcttttatcagaacatcttttttaatatacccctgctccgaacgataagcatttttaaaattttcgtagtaaagaatggctaacgtataggcaaatgcatcccataacgaagatgtttggctatttttactttgcggcaaaatcacacttagctcattaaataaggtttttatgacttcttttccctgccccgcggcaattaccggacaagaatgcggttgcagtagctgattttcctcagccccctgaaactgaaagccgtacagcgcacaggtacacgtcgttgccggatcgttaacgtcagaggccaccgcatgcagcctgccgcgttctatcaccacaatgtcatccgcatgtgcgacatataacgaagaatcgatggtaaaccttgcaacccctttcttgacgtaaatcaactcggtttcattgtcatgaacgtgatgtccggactcccattttggatcatcgctaaatgcaaaacgtgaaagccgtggcgttttaccggcgacaaacagcgtttcactggcgttatcaaaacagcgttgatacatgacaacctccctattccatgagcaagcaaaaacaatatatgccggataaaatacggcgtgtattgcggttatacaaccgcgtttagcgagagctaaacaagattatttacactgaatgcaagattgtacggtcatggaataactatattgccgcaaattgcacttttgttttagcgatcgcattttttttgcaagattgttggcaaggaaaacagcttgctccgtcgaaaaccccgcaccgctatcgcacactattttcaggccatttttaccttccatcggagatggttccgtatgcgactcacaggagaaatcatgaaaataataacctgctttaagctggtgcctgaagaacaggacattgttgtcactccagaatacaccctgaatttcgacaatgccgacgccaaaatcagccagttcgatctcaatgccattgaagctgcaagccagctcgcaacagatgacgatgagatagccgcgctgaccgttggcggctcattgttgcagaactcgaaagtgcgcaaagacgtgctatcccgcgggccgcacagcctgtatttggtgcaggatgcgcaacttgaacatgcactgcctctcgataccgcaaaagcgctggcggcagcaattgaaaagatcggcttcgatttactgatctttggtgaaggttccggcgacctttatgcccagcaggttggcttgctggtcggagaaattctgcaacttccggtgattaatgcagtgagtgctattcagcgtcagggcaatacactggtgattgaacgcacgcttgaagatgatgttgaagttattgaactctctgttccagccgtgctctgcgtcacctccgatattaacgtgccacgcattccttcgatgaaagccattctcggcgcgggtaaaaaaccggtaaatcagtggcaggcaagtgatattgactggagccagagcgcgccacttgctgaactggtcggcattcgcgtaccgccgcaaacagaacgtaagcacatcattatcgataacgattcgccggaggccattgccgagctggcggaacatctgaagaaagccctgaactgaagcctacggagaagaaacgatgagtcaattaaacagcgtctgggtctttagcgataatcctgaacgttatgctgaactgtttggcggcgctcagcaatggggccaacaggtgtatgccattgtacaaaataccgaccaggcgcaggcagttatgccttatggtccaaaatgtctttatgttcttgcgcaaaacgacgcgctgcaacgcactgaaaattacgccgaaagcattgctgccctgctgaaagataaacaccccgctatgttgctgttggccgcgacgaaacgtggtaaagcgctggcagcacggttaagtgtgcaactgaatgcggcgctggtgaacgatgccacggcggtggatattgtcgatggtcacatttgcgccgaacaccggatgtatggcgggttagcgttcgctcaggaaaagatcaacagcccgctggcgatcattacccttgcacccggtgttcaggaaccgtgcaccagtgatacctctcatcagtgcccgacagaaacggtaccttatgttgctccgcgtcatgaaattctctgtcgcgaacgccgtgcgaaagccgcaagcagcgtggacctgagcaaagcaaaacgtgtggttggcgtcggtcgtggactggcggcgcaggatgacctaaaaatggtccacgaactggcggcggtgctgaatgctgaagtcggctgttcacgtccaattgccgaaggcgagaactggatggagcgtgaacgttatatcggtgtctccggcgtgttgctgaaatccgatctctacctgacgctggggatctccgggcagatccagcatatggttggcggcaacggcgcaaaagtgattgtcgccatcaataaagataaaaatgcgccaatcttcaactatgccgactacggtctggtgggcgatatctacaaagtcgtccctgccctgattagccagttgagccgctaattcccctttcaaccacatctcccgctgtaaacgcagcgggaagggagcataacgcatgtcggatgacaaatttgatgccattgtggtcggtgcgggcgttgctggtagcgttgccgcactggtcatggcacgagccgggctggatgtcctggtgatagaacgcggcgacagtgccggatgtaaaaacatgaccggcgggcgtctttatgcccacacacttgaagcaatcattccaggctttgcagtatcagcgccggtagaacgcaaggtcacacgcgagaaaatctccttcttaaccgaagaaagcgccgttaccctcgattttcaccgcgagcagccagatgttccgcaacacgcatcttataccgtattgcgtaatcgtctggacccgtggttgatggaacaagccgagcaggcgggcgcgcagtttatcccaggcgttcgcgtcgacgcgctggttcgtgaaggaaacaaggtcactggcgtgcaggctggggatgatattctcgaagcgaatgtggtgattctggctgatggcgttaactcgatgcttggccgctcgctgggaatggttcccgcttccgatccgcatcattacgctgttggtgttaaagaggttattggcctcacaccagaacagatcaacgatcgctttaatattacgggcgaggaaggtgccgcctggctgtttgccggttccccttctgacggcctgatgggcgggggatttctctataccaacaaggattccatatccttggggctggtttgtggattgggtgatatcgcccatgcgcaaaaaagcgtgccgcaaatgctggaagattttaaacaacaccccgccattcgcccgctgattagcggcggcaaactgcttgaatattccgcgcatatggtgccggaaggcggtctggcaatggtgccgcaactggttaacgagggcgtgatgatcgttggtgacgccgcaggcttctgcctgaatttgggttttacggtccgcggcatggatttagccattgcatcggctcaggctgccgccacaacggtgatcgccgccaaagaacgcgcggatttctccgccagcagtctggcgcaatacaaacgtgagctggaacaaagctgcgtcatgcgtgatatgcagcattttcgcaagatcccggcgctgatggaaaacccgcgcctgtttagccaatacccacgaatggtagccgacatcatgaacgagatgttcaccatcgacggcaaaccaaaccagccggtacgaaaaatgatcatgggacatgcgaagaaaattgggctgatcaacttgctgaaagatggcattaagggagcaaccgcgctatgagccagaacgctacggttaacgtcgacatcaaattaggcgtcaataaattccatgttgatgagggccacccgcatatcattctggcggaaaatcccgatatcaatgaattccataaattaatgaaagcctgccctgccggactttataagcaggatgacgcaggaaacattcattttgattccgccggttgtctggagtgcggcacctgtcgggtgctgtgcggtaacactattctcgaacagtggcaatatcccgcaggcaccttcggtattgattttcgctacggctaatcatgcatcccacaggcccgcatctcgggcctgatgttctgtttcgagagtccaacatgaaagtgacattaacgtttaacgaacaacgtcgtgcggcgtatcgtcagcaagggttatggggcgatgcttcgctggccgattactggcagcagaccgctcgtgcgatgccagacaaaattgccgtggtcgataatcatggtgcatcgtacacctatagcgcgctcgatcacgccgcgagctgtctggcaaactggatgttagcgaagggtattgaatcaggcgatcgcatcgcatttcaactgcctggctggtgtgaatttaccgttatctatcttgcctgcctgaaaatcggtgcagtttccgtgccgctgttgccttcctggcgggaagcagaactggtgtgggtgctcaataagtgtcaggcaaaaatgttctttgcaccgacgttgtttaaacaaacgcgtccggtagatttaatcctgccgctgcaaaatcagcttccacaactacaacaaattgtcggcgtggacaaactggctcccgccacctcttccctctcattaagtcagattatcgccgacaatacctcactgaccacggcgataacgacccacggcgatgaattagctgcggtgctgtttacctccggaaccgagggtctgccaaagggcgtgatgctaacgcataacaatattctcgccagtgagcgggcttattgcgcgcgactgaatctgacctggcaggatgtctttatgatgcctgcgccacttggtcacgcaacgggctttctgcatggcgtaacggcaccattcttaattggcgctcgcagcgtgttgttagatattttcactcctgatgcgtgtctcgcgctgcttgagcagcagcgttgcacctgtatgctcggcgcaacgccgtttgtctatgatcttttgaatgtactagagaaacaacccgcggacctttcagcgctgcgtttctttctttgcggcggaaccacaatccccaaaaaagtggcgcgtgaatgccagcagcgcggcattaaattattaagtgtttatggttccacagaaagttcgccgcatgcggtggtgaatctcgatgatcctttgtcgcgctttatgcacaccgatggttacgctgccgcaggtgtagagattaaagtggtcgatgacgcacgcaagaccttaccgccaggttgcgaaggtgaagaagcctcgcgtggccccaatgtgtttatggggtattttgatgaacctgaattaaccgcccgtgccctggatgaagaaggctggtattacagcggcgatctctgccgtatggatgaggctggctatataaaaattaccggacgcaaaaaagatattattgtccgcggcggcgaaaatattagcagccgtgaagtggaagatattttattgcagcatcctaaaattcacgatgcctgtgtggttgcaatgtccgatgaacgtttaggtgaacgatcatgcgcttatgtcgtgctgaaagcgccgcatcattcattatcgctggaagaggtagtggctttttttagccgtaaacgggtcgcaaaatataaatatcctgaacatatcgtggtaatcgaaaaactaccgcgaactacctcaggtaaaatacaaaagtttttgttaagaaaagatattatgcggcgtttaacgcaggatgtctgtgaagagattgaataagtttcatcttcggggatcacataaccccggcgactaaacgccgccggggatttattttatttcttcagttcagccaggcttaaccaggtttgcaccacggtgtccgggttcagagacaggctatcgatcccctcttccatcaaccatgcggcaaagtcttcgtggtcggacggaccctgaccgcaaatcccgacatatttgccctgtttcttcgcggcacggatagccatcgacagcagtgctttcaccgcatcgttgcgctcatcgaacaattcagacaccacgccggagtcacggtccagaccgagcgccagctgcgtcatatcgtttgagccaattgagaagccgtcgaaatattcgaggaactgctcggccagcaaggcgttggacgggatttcacacatcatgatgattttcagcccgttctcgccacgtttcagcccctgacgcgccagttcttcaaccaccgctttcgcctgatctacggtacgcacgaacgggatcatgatctcaacgttggtcagtcccatgtcgttgcgcacacgtttcactgcttcacactccagcgcgaaacagtcgcggaagctgtcggaaacatagcggcccgcgccacggaagccgagcatcgggttctcttcatctggctcgtaacgctcaccaccgaccaggttggcatattcgttcgatttaaaatcagagagacggacaatgacgcgcttcggataaaacgcggcacccagcgtcgcgatcccttcagtcagacgaccaacgtaaaattcacgcggagaatcaaaacctttcatcatctcgcggatttcgttttgcaactgcggttcctgatcgtcaaactcaagcagtgcgcgtgggtggacgccaatcatacggttgatgataaattccagacgcgcaaggcccacgccttcgttcggtaggcaggcgaagtcgaaagcacggtccgggttaccgacgttcatcatcactttcaacggcagatccggcatcgtttctacgctggagcttttcacgctaaattccagcaactccgcatagacgtaaccggtatcaccttcggcacaagaaacagtgacgttctcaccgtctttcatccgttctgttgcatctccacagcccactaccgccggaatgcccagttcacgagcgatgatcgccgcgtgacaggtacgaccgccacggttggtgacgatggcagatgctttcttcatgatcggttcccagtccgggtcggtcatgtcagtaaccagcacgtcgccaggttcgatgcggttcatttcgctgatgtcatggatgactttcaccggacccgcaccgatgcgatgaccgatagcacggccttcggcgataatcttaccctgtgaatgcagcgtataacgctccatgacctgaccgcgtgagcgcacggtttccggacgcgcctgcacaatgaacagtttaccggtgtggccatctttcgcccactcaatatccatcgggcgaccgtagtgtttctcaatttgtacggcctgttttgccagttcctgcacttcttcgttggtcagcgagaagatgtcacgctgttcctgcggtacgtcttcgattttaacctgcttgccgtgctcctgggtcggcgcgtaaaccatgcggatttttttcgaccccatggtgcggcgcacgatagccgggcgattcgccgccagtgtcggtttatgcacgtaaaactcatccgggttaaccgcaccctgcacgaccatctcaccaaggccccatgcggaagtgataaacaccacctggtcaaagccggattcggtatcaatggagaacatcacgccagatgatgcgaggtcagagcgcaccatccgttgaacaccggcggagagcgccacaccacggtgatcgtaaccctggtgcacacgataagagatggcgcgatcgttaaacagagaagcaaatacatgtttcactgccacgagaacggcgtcaaaaccctgaacgttgaggaaggtttcctgctgaccggcaaaagaagcgtccggcatatcttctgcggtggcggaggagcgcaccgcaaaagaggcgttttcgtcatcggcggaaagctgtgcataggcttcgcggatggcgttttccagctcaggctggaagggagtgtcgataatccactggcggatttgcgcgcccgctttcgcaagctgagtaacatcgtcaatatccgttttatccagcagttcataaatgcgctggtttacgccgctttggtccagaaactggttaaacgcgtcggcggttgtggcgaaaccattcggaacggaaacacccattccggaaagattagtaatcatttcacccagggaggcatttttgcccccaaccctgtctacatcattcatgccgagttggttataccaaagcaccagcggtgacgagccattgttggacatcgaacaatccttttgtgataaatgaacggtttgagaaacacatttctgcgcatttatctttgcatatttaaccggatgaaaaaaacggtgaatcgttcaagcaaatatatttttttactttttaagactgatcccagcgttgcgcaaatctgctctcttcgacaatttccacataaaccatcggtataaacgaaaccataaaaatgaaatgctgttttcataaaaaataaaattgaaggttcattttataaaccagacataacgttctacgcttctgtgcgtttttaatttatgctttcatagaattatgtctgcatcacgggaagaacaaaatggataatgctgttgatcgccacgttttttatatttctgatggtacggcaataactgcggaggtattaggacacgcagtaatgtcacaatttcccgtcactatcagcagcatcacgctgccgtttgtcgaaaatgagagccgtgcacgggcagtgaaggatcagattgacgcaatttatcaccagacaggcgtgcgcccgctggtcttctactccatcgtgttgccggagattcgcgccatcatcttgcaaagtgaaggcttttgccaggatatcgttcaggcgctggttgccccgctacaacaagagatgaaactggatccaacgccgattgctcatcgtacccatggccttaaccctaataatctcaataaatatgatgcgcgcattgcggcgattgattacaccctcgcccacgatgacggcatttcgttgcgcaatctggaccaggctcaggtgatcctgctcggtgtttctcgctgtggtaaaacccccaccagtctgtatctggcaatgcagtttggtatccgcgcggcaaactacccctttattgccgacgatatggataatctggtgctacccgcgtcgctcaaaccgcttcagcataaattgttcggcctgactatcgacccggaacgtctggcggcgattcgcgaggaacgtcgggagaacagtcgctatgcctcgcttcgtcagtgcaggatggaagtcgcggaagtggaagccttgtaccgtaaaaatcagatcccgtggattaacagtaccaattattcggtagaagagattgccaccaagatcctcgatatcatgggccttagtcgccgaatgtactagagaactagtgcattagcttatttttttgttatcatgctaaccacccggcgaggtgtgacacacctcgcacttgaaatcagcagcgattggtttatcgtgatgcgcatcacttcccggcagtcctgccgtagaagcaacaaatttctgagacttgtaatgaacagaactgacgaactccgtactgcgcgtattgagagcctggtaacgcccgccgaactcgcgctacggtatcccgtaacgcctggcgtcgccacccatgtcaccgactcccgccgcagaattgaaaaaatactgaatggtgaagataagcgactgttggtcattattggcccctgctcgatccacgatctcaccgctgcaatggagtacgccacccgtctgcagtcgctgcgcaaccagtaccagtcacggctggaaatcgtaatgcgcacctattttgaaaaaccacgaactgttgtcggctggaaaggactaatctccgatccagatttaaacggcagctatcgggtaaatcacggtctggagctggcgcgcaaattacttttacaggtaaatgagctgggcgtcccaaccgcgaccgagttcctcgatatggtgaccggtcagtttattgctgatttaatcagttggggcgcgattggcgcacgtactaccgaaagtcagatccaccgcgaaatggcttcggcactctcctgtccggtaggttttaaaaatggtaccgatggcaatacgcggattgctgtggatgctatccgcgcagcccgcgccagccatatgttcctctcgccagacaaaaatggtcagatgaccatctatcagaccagcggcaacccgtatggccacattattatgcgtggcggcaaaaaaccgaattatcatgccgatgatatcgccgcagcctgcgatacgctgcacgagtttgatttacctgaacatctggtggtggatttcagccacggtaactgccagaagcagcaccgtcgccagttagaagtttgtgaggatatttgtcagcaaatccgcaatggctctacggcgattgctggaattatggcggaaagtttcctgcgcgaaggaacgcaaaaaatcgtcggcagtcagccgctcacttacggtcaatccattaccgacccgtgtctgggctgggaggataccgaacgcctggtcgaaaaactcgcctctgcggtagatacccgcttctgaatgcgtgcccattcctgacggaatgggcatttctgcgcaacttgttgtcttctcaacaaattactgcttgctctggtcagccataatattgataataagaatcattgttatatcaattattattaatttttatgcgttatacggatagcagaaaactcacgcctgaaacggatgccaatcacaagaccgcttccccgcagcctattcggcgaatttccagccagacactgttaggtccggatggcaaactgattatcgatcatgacgggcaagaatatctgctccgtaaaactcaggctggcaagctgctgttgaccaagtagcctttaactcgagcagctgacttccagccgtttaccccagtcaggtggacgactgacatagtcatcatctctgtcgctgaaaggatttcgcaacgcctcatgcaggcggtgcaattccgtcatatcacccttttctgccgcttcaatcgcccgttgcgccaaccagttgcgcaataccagagcggggttaacgctttgcatcagttgctgacgctcactatcgctaacctcgtcttgttgcaaacgcccccgataacgggcaaaccagtcatcaaatgccgcacgatcaataaactcatcacgtagcggtgacgccgcgctgtgctgctcggtcagactcagcatgcggaatgtgcgggtataatcgctgcgctctcgcgccatcagactgaataattcattcagtagcgcgttatcctctttttgctccgtcatgaagcccagtttctgccgcatccgttctccataatgcgtcaacaaaacctgctgatagctgtccagggcctcattcagggcatctacggcaacaaatggcgacaatgtctgcgccagacgctgtaaattccacaacgcgacggcaggttgattatcaaagctgtaacgcccttgatgatccgagtgattacaaataaaaccgggttcgtaatcatcaagaaaaccaaacggcccgtaatcaagcgtcagccccagcagcgacatgttgtcggtattcatcaccccatgagcaaagccgaccgtctgccattgggcaattaacgacgcggtacgtgcgacaacatcgctaaaccagagacggtatttgtcctcatcatctgcaagatgtgaccagtaatgacgaatagcaaagtcagctaactgacgaaccttttccgactcgcggcggtagtaaaaatgttcgaaatgaccaaagcgcagatgacttggtgccacacgcatcagcatcgcgcctggctccgccgtttcccgatacactggcgaatcgctggtgacgatacttaacgcgcgggtcgtcggaatgcccagataatgcatcgcctcactggcgagactttctcgtatcgtcgaacgtaaaaccgcccgtccatcacccattcgcgaataaggcgtcaggccagcacctttcagatgccagtccattgtagtgccatcagcaagcagttgttcgccgagtaaaatgccgcgcccatcacccagttggcccgcccagacgccgaactgatgaccactgtaaacctgcgccagtggtgacataccaggcagtagggcttcgccgccccagacacctgcgccatttttaaacagcgacgatggaatactcagcgtgttagccagttcggtattatgccaaatcagccgggcattatttaaaggcgtaggggaaagtgctgtataggtttctggcaattcatcgcgccagcgggtaacaaaagacagggtcatagatcctcctgtttgatagtgtagacggttactctcgtcttaaacaccagcaaacagaagggttatcgctgaaccaacgtcgttatctgatttatgggaacggcaggccacaggcatccctggagagcatggaaatcgaagggggtaatctgtgccaatatttctgccgtatcaatgcctcccgcaatgatgcaattgcaacaaggggaaatttgcgcctggatcgcacgaataaacggttcgaaggagcggtgcgtgatttgttgctgaataaaacttttatccagcatgacgcgggtgaaaagaccatcaaaaaccgctttcattgtgctattgcctgctcccaaattacctaacacaaggggatacacttgcgataaggataaaagaccgcgattatcttttccttcattgagatgcgggtaattctcattaatcaacagttcaataaacggatattttaatagttcgcctgcgtaattatccctctctaataataatgtagccacttgtggcgttaaattaagccaggcaaagagtttatgttgaataaaaaaatgttggcatgattttagtaattccaactgctctgaaaataattgccaatgttgctcctcggtaagttgcgctataacccgactcgtcgggatacgaaccgtaccatcttcactggagaaatgggtaattaactcaacgccgacaaggacttgctggttgtctcttatcggcaggaaatagcaatcagaatgataaagattctccaaaaaaatcttcatggtaaccgtccctctcgaaggatgtttttcagtatccggctaaaagggatgaggccataagacataacaattacagaaggagtaactttcatttgttccatgttaaccactttttcaggggtcctttttttagattatcctgattataaacgaataatccatttacggaatttttgtctgcaaaatactactgtattcaggagtaaatggacggcgatgtatcatcgccgtccatttttcgacatactagattcgtctcgcctgccagaaatttttctgccaatagacattatcaagtgaggaacgcatcactcccttgctggtagaggcgtggataaattggttgttggtatcgtaaatacctacatgcaaaccattttgtccggaccccgttttgaaaaagaccaggtcacctggcagcaactcgtctttatcaatttgcgtgccaatagaggcttgttgtttggtttcacggggcagctgcaaatcgaaacgatcgcgcatcgtcacaaccacaaatcccgaacagtccacaccgcgccgcgtcatgccaccataacgatacggcgtgccatgccagctttgtagctggtcgttcaaaccggcaataacggtaatcgaatcagaaagtctggcatttggcggcggtgctttatggtggctacacccggccagaagcagtgctgtgatcaaaataaggcagaaacgcattccgtacggttcctctgttttttattcttgcattaatttagcgtcgtaattacccgattttcaagatactaatgaaatcagatggtcgaaatcagcattctgtgaccttcgatatccagacggcgaaaattcatcccataggcctgcgccagatttggcggcgtgagcacctcttccctgcgtccactggccagcatttttccaccttttagcaaccacgcccgatgcgcatgacgcaatgtgtggttgagatcgtgactgctcatcacaatcgccagtccttgctgacacagcgcgctcagaattttgtctaacgcactttgttgcgcaacatcaagactgttcatcggctcatcaagaagcagcaattggcctgcgggattggcttgtggtgtgatttgcaacaccaccgcagcaagacgtacgcgttgccattcaccgccggaaagttgattggtgctacgtccgagtttgtcatcaagagccagcgcccctgcgacatcattcagtagttcggtacgcgttttatcgtgctgatgcagtgtcaggtagtgccagaccggcgttgcaaacggcggcgtctgctgttgtgaaagataggcgcgatgcagcgcgagttttgttgcggaccatgcttccagtggttgccccgcgaactgaatgcttcccttaccgctggtcattccggccattcgcgccagtaaggtactcttacccgcgccattcggccccaccaggtgcaggatctccccagcccgaacctcgccagaaagcggccccaggcgggtagattccgcaacatcttgtaactgcatcacaatagacattattttgccaacgccagtttaatgctttccatcacaatgggatcttccggcgtcatatccggggaaaaacgctggatgacttttccgtccctgccaaccaggaatttttcaaaattccataaaatatcatccgggtacagcggtgcacggcctttgctgaccatacgggcatagaatccgctctcttccggcgcgactgcggtcggcgctgcggcaatcaatttttgatacagcggatggcgtccttcgccattaacttcaatcttactgaacatcgggaacgtcaccccccatgtggtggtacagtaagttttaatctcttcatcgctgcccggttcttgttccagaaactggttgcacgggaatcccagcaccataaaacctcgatcgacccaggctttctgaatattctccaactgctcatattgcggcgttaagccacactttgaggcgacattgacaatcaacagcacattaccggcgaacttctccagcgtggtcacttcaccgtcgatatctttcactacggtcgtcagaatggaatcttgcatcgtttctcctgggtgtggtcagtaaaaatcttagcttttaatcatagaccgtctttttgcggctaacgtcctgcttttaacaataaccagataaacaccggcgcacctaacgttgcggtgaccacgccaataggcagctctgcggcagctaatgccaggcgcgctacaatatcggccagcagcaatgcgctcgcccctgccagcgcgcagccgggaagtaatacgcgatgatcggttaaaccacacaaccggagaatatgggggatcaccagaccaataaagccgatagcacccgccagcgccacactgacgccaaccatccagccggtcgctgccaccagcacattgcgccagaaccacaggggtaaacccagttgccgcgccgagatctcgccaagtgctaacatattcatcggcctggactgacaacagatccacaacaacacggggatcaatgccagcatcagccagctttgccgccagtctacgccgccaaaaccgcccatcatccagtacatcagctgacgcaaatcaactgaggtggaaaagtagatagcccacgtcattagtgcgctacagataatccctaatgcaacgccagccagcaataaccgactggtcgaaagatgacgacgggcgaaacgtaagagtattaaagtgatgataagcgcgccagcaatcgcacacagccctagcgcccagttggggagttgcccttgcccaagcaataccgcggcgataagccccacgcctgcgccgttagagacgccaagtagtccaggttctgccagaggattttcaaacaacgcctgcattacagcgccggatatagccagcgccgcaccaaccagcaatacagccagcgtacgtggcaggcgaatttgccagacgaacagttcgccacgaggagtaaaccagtcacctggcgagatccattgttcaccggcgcaaaggcttaagagaagcgccagcagcatcaaaactgacaggcataataaccagcgaatattttgtcgctgttgttggcgggcaagtgtcagcatggtatccgttctgctgaagtgtcatggcgttgattttacggtgactcttcgacagtgaaaagaaaaaaggccgcagagcggcctttttagttagatcagattactcgtctttgggcgaagcgttttcgacccggctttttaacttctgcccgggtctgaaggtcaccacgcgccgtgctgtaatgggaatatcctcgcccgttttcgggttacgtcccgggcgttgattcttatcacgcagatcgaagttaccaaaaccagagagtttcacctgttcgccgttttccagagcgcgacggatctcttcgaaaaacagttcaaccagttctttggcatcccgcttgctaagcccaagcttatcaaacagatattctgacatttcagcttttgtaagcgccataggttcaatccctcaatgatgcctggaatcgctcttttaatgcctctacacatttggcgacggtagcggcaatctcctcttcttcgagtgtacggctggtatcttgcaggatcaggcttatggcgaggctcttatacccctccgcaacacccttaccgcggtacacgtcaaataagtttacgccaactacctgatttacgccaactttcttacattcggataaaatatccgctgcgggaacgttttctgcgaccaccaccgcgatgtcacgacggttcgccgggaagcgagaaatctcgcgcgcctgaggcaccacgcggtctgcgagcttgttccactccagttcgaacaccagagtgcgaccgttaagatccagtttacgttccagttcaggatgaacaaccccaacaaaaccaatacgttcacctttcagataaatcgctgcggattgccccggatgcagtgccggattcgcttctgcacggaactcaacctcattcagtttaccggtcaggtcgagaacggattcaagatcgcctttcaaatcatagaaatcaacggtctcttttgccaggttccagtgctcttcgtaacggttaccgcaaatcacaccggctaacatcagatcctgacgaatgcccaacggtgcctgagtatctggtacgaaacgcagaccgctttcgaaaatgcgcacacggttctgctgacggttctggttgtacaccacggttgccagcaggccagtccacagagaaagacgcattgctgacatttcaacagagatcgggcttggcagcagtaaggcttcaacgcctggatggatcatctgctgcactttcggatcaacgaagctgtaggtgatcacttcctgatagcctttgtcgttgagcagcgttttcacgcgcttgagcgacaggtcagcttcacggtgagtacccataatcaggcttgcctgtaccggctcatccgggatgttgttgtagccgtaaacacgcgcgacttcttcaaccagatcttcttcaatctccatatcgaaacgccagctcggcgcaactgcctgccattcgtctttgccttcggtcacttcgcagccgagacgacgcagaatgtcagttacctgctcatccgcaatatgatggccgatcaggcgatccagtttgctacgacgtagagtgatggttgcacgcttcggcagcgttgcttcgttggtgatatcaattaccgggccagcctcaccaccgcagatgtcgatcagcagacgggtcgcacgttccatcgctttgtgctgcagtgccggatcaacgccacgctcataacggtgagacgcatcggtatgcaggccatgacgacgagcacgaccggtgatagacagcgggctaaagaacgcgcattccagcagcacgttttgtgtttcgtcattcacgccagagtgttcgccaccgaagatgccgcccatcgccagcgccttgttgtggtcggcgatgaccagagtgtcagcattcagcttcgcttcagtaccgtcgagcagcaccagcgtttcgccctctttcgccatccgcaccacaatgccgccttcaatgcgatctttatcgaaagcgtgcatcggctggcccagttcgagcagcacatagttggtgacgtcaacaactgcatcgatagaacggatcccgcaacgacgcagtttttctttcatccacagcggagttggcgctttaacgttaatgccttttaccacacggccaagataacgcgggcaggcttccggcgcttcgactgtaatcggcagcgtgtcgtcgatggtcgcaccaaccggaacgatttccggttgaaccagcggcagctggttcagcacggcaacgtcacgcgcaacaccaatgatgcctaagcagtcggcacggtttggcgtcacgctgatttcgatggtgttgtcatcaagtttcaggtattcacggatatcggtgccaatcggcgcatccgcaggcagttcgataatgccgctgtgatcgtcagaaatgcccagttcagagaaggagcacagcatcccttcagacggttcgccacgcagtttcgccgctttaattttgaaatcacccggcagaacagcaccaatggtcgctaccgctacacgcaggccctgacggcagtttggcgcaccgcagacgatgtccagcaggcgatcgccgccgacattcacttttgtcacacgcagtttgtcagcgttcggatgctgcgcacactcaaccacttcaccaacgaccacgccgtggaagctgccggcaaccggttctacaccgtcaacttccaggcccgccatagtgatttgatttgccagcgcatcgctatcaatcgccgggttcacccattcgcgtaaccacagttcactgaatttcataatctattcctgccttatttaaactgtttgaggaaacgcagatcgttttcgaagaatgaacgcaggtcggtgacgccgtaacgcaacatagtcagacgctccatccccatcccgaaggcgaaaccagagtaaacttccgggtcgatgccaacgttacgcaacacgttcggatgcaccatcccgcagcccagcacttccagccatttaccgtttttacccatgacgtccacttctgcagaaggttcggtaaacgggaagtaggaaggacggaagcgaatctgcaaatcttcctcaaagaagttacgcaggaagtcgtgcagcgtgcctttcaggttggtaaagctgatgttggtatcaacaatcagaccttccatctgatggaacatcggcgtgtgagtctggtcgtagtcgttacgataaacacggccaggcgcgatgatacgaatcggtggctgctgggctttcatggtgcggatctgtacgccagaggtctgggtacgcagcaggcgggtagtgtcaaaccagaaagtgtcgtggtcagcgcgcgccgggtggtgaccaggaatgttcagagcatcgaagttatgataatcgtcttcgatttccggcccggttgccacggtaaagccaagctcaccgaagaaactttcgatacggtcgatggtacgggtaaccggatgcagaccgccgttttcaatgcgacgacctggcagagagacatcaatcgtttccgccgccagacgcgcattcagtgcagcgctttccagttccgctttacgcgcattcagcgcctgctgaacctgctctttcgcttcgttgataaccgcaccagctgccggacgctcttctggcggcagctcacgcagggtcgtcatctgaagggttaagtgcccttttttacccaaatattcgacgcgcacattatctaacgcggcaacatctgacgcctggctaatggccgccttcgcactggcaaccagttctgcgagatgtgacatggttttcctcattgtgtcagtggtgacactggttcgttggacttagagcctatcccatcaggctattttacttgccattttggtcccgggctgtgctcgaaattctcacgtacttaaatacgctccggtttctccgcgctggccgtgtccagtctggctgcgacaattacacctgatgagacaggctttttatttttcaaaacgcgcatacaaaaaaagcctccactgggaggctttcaggcgctgttttccgtttctcttctcacgcgctagcctcctggattcaggtgctaaagtaaaaaaagaagcggaaaatagcagcattcattgcttgcgttaccttttggtactcttcaaaagacctttattgaaaaggctacggcgataaaagtcaatgttttgatggcgttgaaacgaaaagagggagactagctccctctttcaactggcttatgccagagctgctttcgctttttcaaccagagcggtgaacgctactttgtcgaatactgcgatatcagccaggatcttacggtcgatttcaacagaggcttttttcaggccattgatgaatttgctgtaagaaataccgttctgacgtgctgctgcgttgatacgcgcaatccacagttgacggaactgacgcttacgttgacgacggtcacggtaagcatactgaccagctttgataacagcctggaaggcaacgcggtatacgcgagaacgcgcaccgtagtagcctttagcttgtttcaaaattttcttgtgacgtgcacgtgcaataacaccacgttttacgcgagccatatgtgctctcctgtatctatattctaattaaaaagttaaaaacgttaacggcttatgcgtacggcaggcacgcgattaccaggcccagatcgcctttggaaaccatggctttcggacgcaggtgacgtttacgtttggtcgcttttttggtcagaatgtgacgcaggttagcgtgcttgtgcttaaaaccacctttaccggtttttttgaagcgcttagcagcaccgcgtacggtcttaatttttggcattttaataacttccacttcgcattgttaataaacgaaacaaaggcgaacaaagcctgtgaagcccgaaggctccacagacagtgctacttgaaggccttactgtttcttcttaggagcgagcaccatgatcatctggcggccttcgatcttcgttgggaaggattcgaccactgccagttcttgcaaatcgtctttcacgcgattaagcacttccataccgatttgctggtgcgccatctcacgaccgcggaaacgcagcgtgattttggctttatcaccctcttcgagaaagcgaatcaggctgcggagttttacctgatagtcgccttcatctgtaccaggacggaatttaatttccttaacctggataactttttgctttttcttctgttccttagaagacttgctcttttcatagaggaatttgccgtaatccattatacgacaaaccggcggctcggcgttagggctgatctcgactaagtctactccggcttcttctgctttctccagagcttctctcagactcacaataccaagctgctcgccttccagacctgttaagcgaacttcctgggcgcgaatttcgccattgatacggttagggcgcgccgtttgaactcgttttccgcctttaataccttattcctccaattgtttaagactgcggctgcgaatctcttgttgcagcttctcgatcacttcatttacgtccatgcttcccaggtctttaccacggcgggtgcgaacggcaactttgcctgattccacctctttatcaccacagaccagcatatatgggacgcgacgcaaagtgtgctcgcggattttaaagccaatcttctcatttctcaagtctgctttaacacgaatgcccgcatttgatagtttttgcgtcaattcgttaacgtattcagactgtgaatcggtaatattcatgataacaacctgaaccggcgcaagccaggtcgggaagaaaccagcgaactcttcggtcaggataccgatgaaacgttccatcgaccccagaattgcgcggtgaatcattaccggtactttacgttcattgtcttcgcctacataagaagcgctcagacgagacggcaaagagaagtccagctgtactgtaccgcactgccatgcacgatcgaggcagtcatacagggtaaattcaattttcggaccgtagaaagcgccttcacccagttgatattcaaacgggatgttgttttcttccagcgcaaccgccaggtccgcctcagcacgatcccacatttcgtcgctgccaatacgtttttcaggacgagtggagagtttgacgacgatcttctcgaagccaaaagtgctgtacatatcatagactaaacggatacatccgttaacttcatcgcgaatttgttcttcagtacagaagatatgcgcgtcatcctgggtaaatccacgcacgcgcatcaggccatgcagcgaacctgacggctcgttacggtggcagctaccaaactcggccatacgcagcggcagatcgcgataagacttcagcccctggttgaaaatttgtacgtgacccgggcagttcatcggcttaatgcagtattcacggttctcagaagatgtggtgaacattgcatctttgtagttgtcccagtgaccggttttttcccacaggacacggtccatcatgaacggacctttaacttcctgatactggtactctttcagtttagaacgaacaaacacttccagttcacggaagatggtccagccgtcgttgtgccagaataccatacccggcgcttcttcctgcatatggtacaggtcgagctgtttaccgattttacggtggtcgcgtttcgcggcttcttccaggcgctgcaggtaagcgttaagtgcttttttgtctgcccacgccgtaccgtaaatacgttgcaacattttgttgttgctgtcgccacgccagtaagcccctgccgttttcattagtttgaaatgatggcagaaacgcatgttcggtacgtgcggaccgcggcacatatcgacatattcttcatggaagtacagacctggcttgtcatcatgggcgatgttttcgtcaagaatggagactttgtagctctccccacggttggcgaaagtttcacgcgcttcgtgccagctgactttcttcttaatgacgtcgtagtttttctcagcaagctcatgcatccgcttctcgagtgcttcgacatcttcctgggttaacgtgcggtcaagatcaacgtcgtaataaaaaccgttgtcaataaccgggccgattgccattttggtatgcggccaaagttgtttaatcgcgtgccctaacaggtgcgcacaggagtgacgaatgatctccagaccttcttcgtctttggcggtaatgatcgacagttgtgcgtcgttttcaatcagatcgcaagcatcaaccagttcgccattaacgcgccctgcgatacaggctttcgccagacctggaccaatgtccagcgcaacatccatggggcttacagcgtgatcgtaatggcgttggctgccatcaggaagagttataacaggcattttatatccttatttgcagtggtgacccacacgaaagatcacatacaaagaaaaatttgtttattaacagttcattgcgaaaccatctagccaacaaatgctaaattggttcgcaatcaggtacacaaatgaaagacattaacctctcaccttccacccggttgagcgatgttaacactaaaaaaagggagattgtacctttccgtttcacattgattcgattcgcaattcgtttgtagtgagtacaccagcaaaacgcttaaagaacaactgataacatcacggtgcgtctgaaaggtttactgcgagcggatttacagcagcataaactgaatccagcaaagttcgttgcgtgatttggcggtagtattttaaacgctcatgagattaatgacgaagtggtcatatcacaatgataaaagtgacacaattcttataacaatttttcgtgcacatttcgttctggcgataataattaatcatcatcctcaaaacctccagatatatataaggcgaacagattatgagtcaaaacgatatcattatcagaactcattataagtctcctcatagattgcacatcgatagcgacataccaacaccttcatcagagcctattaatcaatttgcgcgccagctcatcaccctacttgatacctctgacttaagttcgatgctgtcatactgtgttactcaggaatttaccgcaaactgtcgaaaaatatcacaaaattgttattccactgccctttttaccattaactttgccacttcacccatccatacagaaaatatactcattacattacactataaaaaagaaatcatttccttattactggaaaccacgcctattaaagctaaccatttgcgaagcatactggattatattgaacaggaacagttaactgctgaagatcgtaaccattgtatgaaactgtctaaaaaaatccatagagaaaaaaactatacacccaacagtaaatctcaatggtagtgcatgttttttgcaatctccttctgacgctattttttgtcgccatctgtcattgcaatacgcccttgattcattgagaaatggaaaaggcaaagtcaacctgattaaacattactcctccgttgaatccatacagcagcatgtccccttagtccgggacgcggagttcagagcattacttcgccatcctcctgcagggagtcgcgttatcgcgagtaaggattttggcttcgctttagatattttcttttgtcgaatgatggcaaacaatgtcagtcatatgtccgcgattttatatatagacaatcatactttgtcagtaaggctacgaataaagcagtcagtgtatggacaattaaattatgttgtgtccgtttacgacccgaacgataccaacgttgccgtcagagacacccacaggacagcacggggctttctttcgcttgataagttcatcagttcaggtcccgatgctcagacctgggctgatagatatgttcgcaactgtgcaattgctattctgcccctattacctgtgggagttccaggggctattttcgcgggtattgcatcacgaatgccatttgcccctatacatccatcggcaatgttgttaataatggctacaggccagtctcaacagcttattacattattcaaacagttgcccatactccctgaaaaagaaatcattgaaataataactgcgcagaatagcgttggtacacctgctttatttttggctatgatgaacggacatactgacaacgtgaaaatatttatgcaagaaattcagtcactggtagataatcacatcattcatgaagataatctggttaaattactgcaaactaaaagtgctaacgaaacacctggactttatatctccatgttgtatggattcgatgaaataatcgatatctttctgaatgcattaaccactccaatagcacaagagcttttaaacaaaaaactggtgatgagtattttagccatgaaaatacatgatggtgagccaggattatacgccgcaatggaaaataatcaccctttgtgtgtcacacggttcctctctaaaattaatggcatcgcctttaaatacaagttgagcaaagctaacatcatggatttattaaaaggagctacagcacagggaacccctgcattatacatcgccatgagcaagggtaatgaagacgtcgtgttatcttatatatcgacgctgggtgcttttgcaaaaaaacattcttttagtcaacatcagttatttacactattggccgctaaaaatcatgacaacatgtcagctgttcatatagccattcatcataagcattataaaactgtagaaacatattatgctgctattaatgcaatcagccaaagcctgagttttagtgctgatgaaataaagacgtatttataaccagctatttacgatatatatcgatacataattttatttttttcataaaacgcagaaacagtgaccatgtgcacaacgccacccgacggctgtaataacaaaaaatcccttgatgcctgtcccttttgttacactccgttatcacgcacaagagatatgcaggacactggtatgccgactaaacgctttgataaaaaacactggaagatggtggtggtgctactggcaatctgtggcgctatgttgttgctacgttgggcagcaatgatttggggctgagcagtgacaaacgaagacagccagaccgcataacacggtccggcagataattttacatgctgtagcccagcgataaggttgtccgacggtcggtatgttccggtgcagactctggaggttcagagttccatgtgacgttgtaagccaccttcagtccaaaatgttcattaatagcaacatttaatgcgctttcggagttcagcgttgtgtcttccgcgccaaagaccgaaacaccctgcgtaaatttagcgttgtcagtcaactgccatgcataagccccggaggcatagcccagcggctgggtttcactggcattgtcggtatatttgtcgtaacgcacacctggaccgaattcaaagcggaaactgtgtaccgggccattcaaaaactgacgaccataacccgcggtcaacacatcgcgctctcgatagccgttataacggtctgtcagccagcttgcctgaccaaataaatagtcataatcagttaaattaaaacggctacgcccgcccgccgcatatttttctgaagaacgctcatcattagaagaagtattactggcgttcccccacagcgaccaggcagtggtgtgtccataccaggtcatggtggtgtcagccgtaagtgaggagcttttcgtattgcctgattgtgcaagatatcctgcgttcagattaccttcgaaaggttttttagcgctggcaggatcatccatgacagtaaaaacggaatcatcggcagctgcattcagtgacgcaaacatgccccccgccaacataacgatggcaggaactgtcttcaaaagcttcatttatcaagagtccgtacaacaaaaaaagagaccatcgcggtcccggaaactttcttaaggatcaaagattagcgtccctggaaaggtaacgaattataaaaaggcgcgaataacttagcaatgtattcttatttcattttttgaataagcatgtggcgaaaacagatttttatttatatatatttatctgcaaaattttaaataaagctccaataaatcatattgttaatttcttcactttccgctgattcggtgccagactgaaatcagcctataggaggaaatgatggtacgtatctatacgttgacacttgcgccctctctcgatagcgcaacaattaccccgcaaatttatcccgaaggaaaactgcgctgtaccgcaccggtgttcgaacccgggggcggcggcatcaacgtcgcccgcgccattgcccatcttggaggcagtgccacagcgatcttcccggcgggtggcgcgaccggcgaacacctggtttcactgttggcggatgaaaatgtccccgtcgctactgtagaagccaaagactggacccggcagaatttacacgtacatgtggaagcaagcggtgagcagtatcgttttgttatgccaggcgcggcattaaatgaagatgagtttcgccagcttgaagagcaagttctggaaattgaatccggggccatcctggtcataagcggaagcctgccgccaggtgtgaagctggaaaaattaacccaactgatttccgctgcgcaaaaacaagggatccgctgcatcgtcgacagttctggcgaagcgttaagtgcagcactggcaattggtaacatcgagttggttaagcctaaccaaaaagaactcagtgcgctggtgaatcgcgaactcacccagccggacgatgtccgcaaagccgcgcaggaaatcgttaatagcggcaaggccaaacgggttgtcgtttccctgggtccacaaggagcgctgggtgttgatagtgaaaactgtattcaggtggtgccaccaccggtgaaaagccagagtaccgttggcgctggtgacagcatggtcggcgcgatgacactgaaactggcagaaaatgcctctcttgaagagatggttcgttttggcgtagctgcggggagtgcagccacactcaatcagggaacacgtctgtgctcccatgacgatacgcaaaaaatttacgcttacctttcccgctaacaaaaacattcccccagcattgggggaatcatcaccaacctgtcggcaacgcgtttctccgactatgctcaaaagtcatgtgataacaaaggggtgaactatggccagtggcgatcttgtccgttatgtcataaccgtcatgttgcatgaggatacattgactgaaattaacgagttgaataattacctgactcgcgacggttttttgctcactatgacggatgatgagggaaatatccatgagctgggaactaacacttttggacttatcagtacccaaagtgaagaagaaattagagaactggtttcggggcttacccaaagtgcaaccggcaaagatcctgaaatcaccatcacgacctgggaggaatggaatagcaacagaaaataaatggtttttgggcaataatcagtctgtggtgtgcgttagctcgtgtttttacaccgcattcttgcgctaaccttatgatctggcagacaacatgggagagacatcatgtggcaggcaatcagtcgtcttttgagcgagcagttaggtgaaggcgaaatcgaactgcgtaatgaactgcctggcggagaagtccatgccgcatggcatttgcgctatgcaggacatgattttttcgtcaaatgtgatgaaagggaactgcttcccggttttaccgccgaagccgaccaactggagttactgtcgcgtagtaaaaccgtcaccgtgcctaaggtttgggcagttggcgctgaccgtgactacagttttctggtgatggattatctcccacctcgtccgctggatgcgcatagcgcatttattcttggtcagcaaattgcgcgtttacatcaatggagcgaccaaccacaatttggccttgatttcgataacgcgctctccacaactccacagcccaacacctggcaacgtcgctggtcaacgttttttgctgaacaacggattggctggcagttggaactggctgcagaaaaagggatcgctttcggcaatatcgacgccatcgtcgagcatattcagcagcgtctggcctcacatcaaccgcagccttctctgttgcacggcgatttatggtccggcaactgtgcactgggtccggatggcccgtacattttcgacccggcctgctactggggtgaccgagagtgcgacctggcgatgttaccgctgcatactgaacagccgccacaaatctatgacggctatcagtcagtatccccgctacctgccgatttccttgaacgtcaaccggtttaccaactctacacgctgttaaatcgtgcaaggttatttggcggtcagcatttggttattgctcagcagtcattggatagattattagcagcatgatatgggttgaggataatggccgctccgtgcggccttttgattaaataaacccaagcagagaaaagaacacataacctgcagcaatacaaataaccggcaggatatacagtgagaaaaactgcaggaaaatagtatggtgcggaacaacaatacgggactcaatttgttcacgcgttagcccctcttcccctttggctttttccagaatgagttgatcttcaacaccttcccgcaagaagcgcgcctggcgactcatccgggcaccggaatcctgcaacgccagtccgacaaaaatcaggatgaaaatcacccagaacataacgttcacgccaccattaaaattgggcgtcggggagttataccagaatagattcaaaaaaggcgtattcgcctgcatcatatcgatcatgacatgagtaaagtcgagcatgaccgcattaatgccttccttgttttcctgccgggtattcataaatttcagcaaagaaatcaatgtagagatcaatgcaggtataaaaatcacccaacccaaaatccttttcaaaacagcaatgcgtccagcttgttgatacgtcatgagttctccttgattaagacgcgtcgtttcacttagtttacctgtagatatctgttttcgcccattctttaaaggcgatatgataggcgcttaatcataagcacggcttaataccttacacataatgctctaaaggagaggttgtaatgtcaaccccgcgtcagattcttgctgcaatttttgatatggatggattacttatcgactcagaacctttatgggatcgagccgaactggatgtgatggcaagcctgggggtggatatctcccgtcgtaacgagctgccggacaccttaggtttacgcatcgatatggtggtcgatctttggtacgcccggcaaccgtggaatgggccaagccgtcaggaagtagtagaacgggttattgcccgtgccatttcactggttgaagagacacgtccattattaccaggcgtgcgcgaagccgttgcgttatgcaaagaacaaggtttattggtgggactggcctccgcgtcaccactacatatgctggaaaaagtgttgaccatgtttgacttacgcgacagtttcgatgccctcgcctcggccgaaaaactgccttacagcaagccgcatccgcaagtatatctcgactgcgcagcaaaactgggcgttgaccctctgacctgcgtagcgctggaagattcggtaaatggcatgatcgcctctaaagcagcccgcatgcgttccatcgtcgttcctgcgccagaagcgcaaaatgatccacgttttgtattagcagacgtcaaactttcatcgctgacagaactcaccgcaaaagaccttctcggttaatgaccaggggcagtgatctcgctgcccctggttctttatctgaaattgcattcaactgacggattaatcgtcaatttaagagaaagagttacaccgtcaccacttccgtgcactgtataaaaatcctatactgtacgtatcgacagtttagtgagttttatcatgacggcggaaggtcaccttctcttttctattgcttgtgcggtatttgccaaaaatgccgagctgacgcccgtgctggcacagggtgactggtggcatattgtcccttccgcaatcctgacgtgtttgttaccggacatcgatcacccaaagtcgtttcttgggcagcgattaaaatggatatcaaaaccgatcgcccgcgcttttgggcatcgtggttttacccacagtctgctggcggtatttgcgctgctggcaaccttttaccttaaggttccggaaggctggttcattccggctgatgcgctacaaggaatggtgctgggttatttgagccacatacttgccgatatgctgacacccgccggtgttcccctgctctggccatgccgctggcgtttccgcttgcctatcctggttccccaaaagggcaaccaactggaacgttttatctgcatggcattatttgtctggtcggtatggatgccccattcattacccgagaacagcgctgttcgttggtcatcgcaaatgatcaataccttgcagatccagtttcatcggcttattaagcatcaggttgaatactaaaaaggcaaaaatcacctttctggaataagcaattccatttgaatataagagccagctcacagttctgttaatcttgcgccaacactatgactgctacgcagtgatagaaataataagatcaggagaacggggatgaactttccattaattgcgaacatcgtggtgttcgttgtactgctgtttgcgctggctcagacccgccataaacagtggagtctggcgaaaaaagtgctggtgggtctggtgatgggtgtggtttttggccttgccctgcataccatttatggttctgacagccaggtacttaaagattctgtacagtggtttaacatcgttggtaacggctatgttcaactgctgcaaatgatcgttatgccgttagtcttcgcctctattctgagcgcggttgcccgtctgcataacgcatctcagttaggcaaaatcagttttctgaccatcggtacgcttttgtttaccacgctgattgcggcgctggtcggtgtgctggtcaccaacctgtttggtttgacggctgaaggtctggttcagggtggtgcagaaactgcacgtctgaacgccattgaaagtaactatgttggtaaagtctctgatctgagcgttccgcagctggtcttgtcctttatcccgaaaaacccgtttgccgatcttaccggagccaatccgacgtcaattatcagcgtggtaatttttgccgcattcctcggcgtagctgcattgaaactgctgaaggatgatgcgccgaaaggtgaacgcgtcttagccgctatcgataccctacaaagctgggtgatgaaactggttcgcctggtcatgcagttgaccccttacggcgttctggctctaatgaccaaagtggttgcaggttctaacttgcaagacatcatcaaactgggaagtttcgttgtcgcgtcctacctcggtctgctgattatgtttgcagtgcatggcattctgctgggcattaatggcgtgagtccgctgaagtacttccgtaaggtatggcctgtgctgacgtttgcctttaccagccgttccagtgctgcgtctatcccactgaatgtggaagcacaaacgcgtcgtctgggcgttcctgaatccatcgccagtttcgccgcctctttcggtgcaaccattggtcagaacggctgcgccggtttgtatccggcaatgctggcggtgatggttgcgcctacggttggcattaacccgctggacccgatgtggattgcgacgctggtcggtattgttaccgttagttccgcaggcgttgccggtgtcggtggtggtgcaactttcgccgcactgattgtactgcctgcgatgggcctgccagtaaccctggtggcgctgttaatctccgttgaaccgcttatcgacatgggccgtacggcgttaaacgttagtggctcgatgacagctggcacgctgaccagccagtggctgaagcaaaccgataaagccattctggatagcgaagacgacgccgaactggcacaccattaattcttatgctggcaacggtccgttttgtataggggccgttgccttactttttaaatgttccatcgcggcgatgcatactgactcatatttaaacagatcgtcagcgaaaaaaatgtccaacttatcaatacattcctggctcaatgaatgtgcctgtagcgagaagcttaaaacctcatacccgagacgttttctaagtgaactatctggaatactcataatatcttcaagcacaccacttcccattcccggaagatttagtggattaaaaagaagattgatattaagcattgatattatcgaaggaaactttaggagactctcatttttttgaatcgcagcaaaaatgctcccgacaggatgtatataattttgttcatagtatatagtccttaaatagtgaataaccaacctgttttttatactgatcaaattggtcattttttctgggcgaaatacagaagtgacatccattccaataaaatctttatttatacctcttatccgaatttcactaccataaagattattaattattactctatatttaacattgtcctgcagatatgtatcaaaactaagtgctggcgctcctggctttgaggcatcatagttaatgttagacatataggcaatcatataattaaagtttgattctgctatttcatcgcagtcacattgacccgttgatataaagaaagtgagtgctgtcatagtagactgcagcctttctttaaaagagtcgaaagccaggcttttaatatttaaatcaccataattactctgtattaagtttgtagaaaacatctcccgcctcatattgttaacaaaattattatctcatttaaatctaagtcatttacaatataagtttaagagcgacgccacaggatgaactatcaaaaatagctcatcatgattagcaaaacttaaccattttaaaataaataaacaattaaagaaaaaagatcacttatttatagcaatagatcgtcaaaggcagctttttgttacaggtggtttgaatgaatgtagcaacgaaatacagaatttcaggtcatgtaactcccggcaaaaccgggaggtatgtaatccttactcagtcacttccccttcctggcggatctgatttgcccaacgttgggcagattcaggcacagtaaacgccggtgagcgcagaaatgactctcccatcagtacaaacgcaacatatttgccacgcagcatccagacatcacgaaacgaatccatctttatcgcatgttctggcggcgcgggttccgtgcgtgggacatagctaataatctggcggttttgctggcggagcggtttcttcattactggcttcactaaacgcatattaaaaatcagaaaaactgtagtttagccgatttagcccctgtacgtcccgctttgcgtgtatttcataacaccgtttccagaatagtctccgaagcgggatctggctggtggtctatagttagagagttttttgaccaaaacagcggccctttcagtaataaattaaggagacgagttcaatgtcgcaacataacgaaaagaacccacatcagcaccagtcaccactacacgattccagcgaagcgaaaccggggatggactcactggcacctgaggacggctctcatcgtccagcggctgaaccaacaccgccaggtgcacaacctaccgccccagggagcctgaaagcccctgatacgcgtaacgaaaaacttaattctctggaagacgtacgcaaaggcagtgaaaattatgcgctgaccactaatcagggcgtgcgcatcgccgacgatcaaaactcactgcgtgccggtagccgtggtccaacgctgctggaagattttattctgcgcgagaaaatcacccactttgaccatgagcgcattccggaacgtattgttcatgcacgcggatcagccgctcacggttatttccagccatataaaagcttaagcgatattaccaaagcggatttcctctcagatccgaacaaaatcaccccagtatttgtacgtttctctaccgttcagggtggtgctggctctgctgataccgtgcgtgatatccgtggctttgccaccaagttctataccgaagagggtatttttgacctcgttggcaataacacgccaatcttctttatccaggatgcgcataaattccccgattttgttcatgcggtaaaaccagaaccgcactgggcaattccacaagggcaaagtgcccacgatactttctgggattatgtttctctgcaacctgaaactctgcacaacgtgatgtgggcgatgtcggatcgcggcatcccccgcagttaccgcaccatggaaggcttcggtattcacaccttccgcctgattaatgccgaagggaaggcaacgtttgtacgtttccactggaaaccactggcaggtaaagcctcactcgtttgggatgaagcacaaaaactcaccggacgtgacccggacttccaccgccgcgagttgtgggaagccattgaagcaggcgattttccggaatacgaactgggcttccagttgattcctgaagaagatgaattcaagttcgacttcgatcttctcgatccaaccaaacttatcccggaagaactggtgcccgttcagcgtgtcggcaaaatggtgctcaatcgcaacccggataacttctttgctgaaaacgaacaggcggctttccatcctgggcatatcgtgccgggactggacttcaccaacgatccgctgttgcagggacgtttgttctcctataccgatacacaaatcagtcgtcttggtgggccgaatttccatgagattccgattaaccgtccgacctgcccttaccataatttccagcgtgacggcatgcatcgcatggggatcgacactaacccggcgaattacgaaccgaactcgattaacgataactggccgcgcgaaacaccgccggggccgaaacgcggcggttttgaatcataccaggagcgcgtggaaggcaataaagttcgcgagcgcagcccatcgtttggcgaatattattcccatccgcgtctgttctggctaagtcagacgccatttgagcagcgccatattgtcgatggtttcagttttgagttaagcaaagtcgttcgtccgtatattcgtgagcgcgttgttgaccagctggcgcatattgatctcactctggcccaggcggtggcgaaaaatctcggtatcgaactgactgacgaccagctgaatatcaccccacctccggacgtcaacggtctgaaaaaggatccatccttaagtttgtacgccattcctgacggtgatgtgaaaggtcgcgtggtagcgattttacttaatgatgaagtgagatcggcagaccttctggccattctcaaggcgctgaaggccaaaggcgttcatgccaaactgctctactcccgaatgggtgaagtgactgcggatgacggtacggtgttgcctatagccgctacctttgccggtgcaccttcgctgacggtcgatgcggtcattgtcccttgcggcaatatcgcggatatcgctgacaacggcgatgccaactactacctgatggaagcctacaaacaccttaaaccgattgcgctggcgggtgacgcgcgcaagtttaaagcaacaatcaagatcgctgaccagggtgaagaagggattgtggaagctgacagcgctgacggtagttttatggatgaactgctaacgctgatggcagcacaccgcgtgtggtcacgcattcctaagattgacaaaattcctgcctgatgggaggcggcgcaattgcgccgcctcaaatgatttacatagtgcgctttgtttatgccggatgcggcgtgaacgccttatccggcctacaaaactgtgcaaattcaatatattgcaggaaacacgtaggcctgataagcgaagcgcatcaggcagttttgcgtttgtcagcagtctcaagcggcgcagttacgccgcctttgtaggaattaatcgccggatgcaaggttcacgccgcatctggcaaacatcctcacttacacatcccgataactccccaaccgataaccacgctgagcgatagcacctttcaacgacgctgatgtcaacacatccagctccgttaagcgtgggaaacagtaagcactctgacggatagtattatcgataaacgccggatgacacatcacctccagcgaacgatcaccccgatggcctgcgtcatccagcacttgcaggaacagcgactcactgatctcttcaccgtagaatgcactgctgaatccctgggtagtgcgcaggttgaccggcaaatcaaacgccatctgacgatccgcccgcaacgcaatgccctgctctgccgcaaacctggcaacaatcgggaaaatctgcgggaacatatgcacatgatgatggctatcaagatgcgtaggtttgcgtccaaatagctcaatgaaacgcaaatactgactgacaagctcctgagtaatttcttccagcggtaaagcatcttcttctgccaactgccagatccattttcccagcacaccatcgcgggttaaccccggcatagctgtcagtggcttacccatagtaaggacaaagtgcatccctatggccagactcggttcatcacgactcaactgcaccgcatggtcaatagcctgcccattcaccagcgccgtcgtcgacgtgacaatcccattgcgacaggcctcgataatgccgtagttctgacctttgcttaagccaaaatcatcggcattaacaatcagtaagcgttccataatcagcctcggttaatgtgcttttttaagctctgcgatgcagtcggcaaagtttggcagccatttctcgtgcgccagaatcatctcgcgtgccagcagctcagcatcgcgatcggaatgcaccaacggactaaggtttagcgccagtaacacatcgttaaattctccgctaagtgcggcgttactggcagcaatctcgaagcctttaatggtgtgaatcagccccattactttatcatcgaaatgcgtaatgcgcggatgtggcgtcgcgccatcgcgccccagcttacaggtcatttctactgcccagtctgccggaatattatcaatctgcccatgatgcgggatattaacgtaatgttctgcttgcttgtcgttgtagatagcgttgatcacttcgcatgctgcatcagagtaataagccccaccgcgctgttccagttctttcggcttaactttcagctcaggatttttatacagctcaaaaagttgtttctcgactttctgtactacctgcgctcgtgcgccgcctttgtagtattcgcccatttcaatagccagcatctctttctgcttgaagtaatacagcagataagaacatggcagcagattcaacgaacgaattaagccctcactaaatggcagatcgaaaatattttttacagaggacgcttttaactgccctgacgccacaccatcaagcaattcggcaaagcgcgacttgccatttatcagcacatccttaatgaacaccatatggttgaggccgaacaaatcgatagataaatcatcgctgtctttcagcatcagaacatcgcgaataaacatcttcatgccgatcggaatattacacacgccgataaagcgtttaaatccggtatgacgataaacggcttcagtgaccattcccgccgggttagtgaagttaatcacccatgcattcggacaaagttcttcgacatcttttacgatgtcaaaaatcaccggaatggtacgcagacctttaaacaaaccgcccgcgccgttggtttcctgaccaagataaccatgacttaatggaatacgttcatccagttcacgcgccggtaattggccaacgcgcagttgggtagtaacgaaatcagcatctttcaatgcttcgcggcgatccagcgttttataaagcttcatcgggacgccagcgttatcaatcatccgttggcagagatcgaaaataatatccagtttcggtttaccaccttcgacatccaccagccataattcgctgaccggcaattcgtgataacgcttaataaatccttccagtaactccggggtatagctgctcccgccaccaatagtgacgacttttaatttctggctcataatttctcccttcagtacagaatactgatatctggcatatctgcccccccggacataaataatccagcaacaggacagatatgtgaattgtcaggtataacgacttactgattaaattcagtcaatttcttacgatagctcttaggcgtaaaggacgttaatttcttaaacgttttaataaacaaactcgggctactataaccggcctcaaacgcaatatccgtcactgaatagttggtcatttccagttgttttttggcaaaattaatacggatttcattaataatctgcattggcgttttgccataatatcgttgagtcgctcgcgtcaaatattcctgtgatttggctgacaacgccaccatattctccagcgccgattcactaaactgctctttatcatgcatcttttctaccgtacttttcagccactgcggtacatcatcaatcacctgttcttcgcggtaatgacgtaaacggttaatgacataaaaagtaaccatctcaacaaactcttccagccctgtttcgcggaaattcaatgaagaaatcactgtttccacataggtgagaaaagcgttattggtccggtatacctgcgaagcgacaaagcaataaggcaacaatggcaggtaatgctgctcaaaaaagcgtttactgatcccaacgttcaatatgcgcgtggcaccaaactcataaaaactttgatggtgcgaacctaacggaataaaaacaaaatcgccccgttccagtaacacgcgcttaccgttaatctcctggaaataacgcccggttaataccagagtaaattcataatagtcgtgctgatgcagtccgctgatactctcagttttgttatagataaacacatggaagtttttgccattaaacaactgctgttctcgggcagtggcaatttccggcgcgttaatcactggctgcatcatcgactccttatgccttcagtttttcatgaagctcaattaattcagtaatcagttcacgcgcaagcatggacgtcattaaatgatcctgagcgtggaccagcaccagactcactttcatcttaccttcgcccgcatcgccttcaatcagtttcgtctgtaccagatgcgcttcattcaatgccatccgtgactgatccatcatggcttttgctgcggcaaaatcgccctgcttcgcctgtttcagtgccgcatacgccaggctgcgcgcttgtccggagttgatgatcagccccatcaccacttcttccagctcttcagcttccgtttgcgtatcgggaatgttatcgagatccatcatacatcgttcctctcttttcttaccggcacgattacccgtaccggcatcgattaaaatttcagggcgttagcgatatcttcttcgctctcttctttatcaatcgcattttgtgctttgttagccaccacaacaaagggcagataaattaacgttgcgatgccaaggttgaagagtgcgaccagcaatgcggcgacgctaccgttggtgttaaagaaggctcccagaccggttggcatggtccacggtgcaatattggtcaccggaggaataatgcccatgtagtacgctgcgagggtgattgccgccagaatcggttgtaccagtacaaacgggataaacatcaccgggttcatgataattggcagaccaaacagaatcggttcgttaatctggaagatgccggacggcagcgccagttttgccacctgacgataatcagcacggcgagaggcgataaagatagccaggatcaggcctaaagtcgcaccactgcccccaaggaaaataaaggagtccagcatcggcttggcccagatatggaaggtcttaccggctgccagcgccgcttcgacggaaccatattgctgataggtcgcgatattttccagtgcccacggcgtcataatgccgttgtccagtgcggtcagcgccagcgcgccatgaataccgaagaaccagagcagtggaacaaagatcacataggcccagcccaccacgctacccaacgatgccagtggggttgagatggtatccataatgatctgatggaagttggtgccccaggtattcaacgcccaggcaataatccccatcacggaaagaataataaagccgggaattaatgccgagaaggaacgcgatactgaagcaggtacgctgtcgggcagtttaatgacccaattgcggcggacaataaaggtaaacatttctgccaccaccaggccaataataatcccggagatgatattcgccccacctaaccagtttgcaccaaccgcataggcctcaccgacactatatggggtgacggtcataaatgctgcaacggataacaacccagccgccagcgcatcgactttacgctcttctgccagcgccatgccaataaagaacggtgccattaaagacattattcctaatgttccgttatatacgttgccgccaatacctttcagaccattaagtgtttcaatggttgaggcgtcgaggcgaatacctaaggaataaaaaaacgacccctccccaaagcttagaaaaacgttgttaattaatacaaacatggcccccgcaagggttaacggcattaagcgaataaagccatttttgattgcattaacgtgtggctgctttcctattttaactgcaaaagggaggagtaccttttcaagcgatgcaataacattactcatagaaaaatacccttaaaaaccgcaatttaaatattgcggtattgatttatgaaataactctttgacgggaaaatttaaaataaattaatttgctgcggcttttttaatcgctgcaaccgcagccttaagcacgcctaaaccatcgactttgccataaagcagcgagtcaattacttcaaccggtttgttgggtaacaaacgctggatttcgggcaacatataagcaatctgcggccctaataacacgacatcggcattctgacctttttcaccagccagtgtttccggaaatgcttcaataatgaccggaacttcatatttttctgcctgtgcgcgcatttttgataccagtaaagaggtagacatgcccgcagaacaaaacagataaatgtgtttcttttccataaaactgccctcatcgacgattatctgtcagccagacactccgcaagccttaacctgcttccatgctctgggtaacttgcgaaaccaacatgactttttttgtggctgaaaggagtatacggtatagacctgagcaatagtatttctttgaccttataaattgtttctccttgacctgtggttatgaccctcttcacatttcgggcaaataattcgcgaagataattaagaactcaggccaaaaaaaaccggcgcaatggccggtttccgttgttactcaagctttcagacgaattgattacttcgcagcctgtggatcagtgtcgtattcagcacaggtctgataaccggagttgatgacatgtccggtatcatctaacgcgacaaagtaggtttctgctttaccatcacgttgacccaggatgtaggtctggcaagtaccgcgagcatggatcatgctcacttcagacgaaggtttacccgcaatttgtgcaacctgcgcccggctcatgccttttttgacgtctttcaccacaggctgtacaaactggtctttggtacgatcataagccgtacaacccgccagcatggttaataccgccgctgcactcagaattcctgccatattcttgttcatattccgtcctcttgtttatcagcgtgttagataagcctggaatacattgggcgctttttcaagcccgtgaacgaaacggctccgctttcagaggattcctgtatgacgttttaaccaccattcagcccgctgtcgcttgtcgtttcagtagcaacgggttagctttaaggaagttttgtcttttctgtctggaggggttcaatgacattgcaacaacaaataataaaggcgctgggcgcaaaaccgcagattaatgctgaagaggaaattcgtcgtagtgtcgattttctgaaaagctacctgcaaacttatccgttcattaaatcactggtgctcgggatcagcggcggtcaggactccacgcttgccggaaagctgtgccagatggcgattaatgagctgcgcctggaaaccggcaacgaatcactgcaatttattgccgtacgcctgccctatggtgttcaggccgacgaacaagattgccaggatgccattgcctttattcaaccggatcgcgtattaaccgttaatatcaagggcgcggtattggccagcgaacaggcattgcgggaagcaggcattgaactgagcgattttgtccgtggcaatgaaaaagcgcgtgagcggatgaaagcacaatatagcattgcgggtatgaccagcggtgtcgtggtgggcaccgatcatgcagcagaagccattaccggattcttcactaaatatggtgacggcggtacggacattaatccgctgtatcgtctcaacaaacgtcagggtaaacagttactggcggcattagcttgcccggaacacctttataagaaagcgccaacggccgatctggaagatgatcgcccttctctgccagatgaagtggcactcggcgtgacctatgacaatatcgacgactatctggaagggaaaaacgtacctcaacaggtcgccagaacaatagagaactggtatctgaaaaccgaacataaacgccgtccgccaattaccgttttcgatgatttctggaaaaagtaataatttgcacatattggattgtgcgaaaaagagtaatttgttcacgccggatgcggcgtgaacgccttattcgacctataaaactatgcaaattcaatacattgcaggagtcgaataggcctgacaggcgtagcacgtcagacggtgtaacctttgtcatcgacccgcctcttttttaatcgcttcccgcctgttacactggatagataaccagcattcggagtcaacagtggtacggcgtttaacttctccgcggctcgaatttgaagctgcggcaatttatgaatatcccgaacatttacgttcattccttaatgacttacccacccgaccaggggtgtatctgtttcatggtgaaagtgacaccatgccgctctatatcggcaaaagcgttaacatccgcagccgcgtcctttctcatttacgtaccccggatgaagccgccatgctacggcaatcccgacggatcagctggatatgtaccgccggtgaaatcggcgctctgctccttgaagcgcgattaatcaaagaacaacagccgctgtttaataaacggttgcgccgcaatcgccagctctgtgccctgcaattaaatgaaaagcgcgtcgatgtggtgtatgccaaagaggtggatttttcacgagcccccaacctgtttggcctgtttgccaataggcgcgcagctttgcaagcattgcagaccatcgctgatgaacaaaaactttgttatggcctgctgggactggaaccgttaagtcgcggtcgtgcatgttttcgttcagcgctaaaacgttgcgccggagcatgctgcggtaaagagagccatgaggaacatgcgctacgcttgcgccagtctctggagcgtttgcgggtggtgtgttggccttggcaaggggcggtggcgctgaaagaacagcacccggaaatgactcaatatcatattattcaaaactggctgtggctgggggcggttaattcgctggaagaagcgacaacgttaattcggacacccgccgggtttgatcacgacggttataaaattctttgtaagccgctgctttccggtaactatgaaattactgaacttgatccggcgaatgaccagcgagccagttgatttcactgaacaacagtttaccttgcggttgtaaaagccgcagggtgtgcctgccatcgaaccagcacgcgccctggtcggtagtgagcaatttatcgcccagttgccacgccccgttaatcacaaacaccaccccgccgcgtgagccaaaggtagtaaacgtacgttcggcaattctgactttcgccttacagacatccaggcgtgtcatgatgttgaaatccatcgacatctgccctgccgtcagtttcgcttttaccacctggtccgctgcaaaggcaaaaggctggaacggttttaaggtatggttaaagcggtctgcgctttcaaggagcatctcgccgccttccagcaacgtcactatcctttccatgccgggaaacaaagaaaactccccattcgccgcgatggatgcaatgctggcacgccagtaaaaatcacgttttgccggtgggaacgtgcaaatttcgcgcgtttcaccggcagcatttcgccacagattcaccgacattttacgcatatcaaagtattccatactcgctcccggcccgttcttttcattgttatcgttcaggtaaccgtggatggttatcggcaactcgggtgatttacgttagtggtgatcaggctttttttacaactgtttgagaagagaaaagaaaaccgccgatcctgtccaccgcattactgcaaggtagtggacaagaccggcggtcttaagttttttggctgaaagattattcagcagttgcaggcattttaccttttgccgctggacgttctgtcagacgcttctcaaaattagcattaaattgctttttctgttccggcgtcaggatgttgtaaattttgttctgggtttccatgtgcgccagcatgttagctttgcgctgttcttccatttttgcgatctgcgcttcagcttttactttatcgaaggtatcgctggcaatgatgtcatgcattgcgcggcgttcttccagcggcggacgtttcatctggtcacgctggcctttcatgatttcgcggatctgctgtttctgcgcgtcggtcaggttcaggtctttgaacatcatgtcctgatgcggaccgaacttgcctttgtggtgcatcatcggcttcgcgtcagccggtgctgcggtagtggtgtctgcggcatgggccaggttagccgcgccaagagccagggtagaggcaacaaacagtgcagttaatttacgcatattctatatccttcctttcagttatttattacggctttcttaagtagcgtgccgtgttgacgagattaactttactgactttagcgtcaattaatcagagcaacggtaaaacaatgaaagtgtaaaaaacacttttgcgccaattatggagaaaaaaagaaaatttgatggagagtgatgagagaatattacaacacgatgattttgcagagattatgaagaactataccggatgactggtgataaataaagcaaataaccaggattaatctgtattaatttataagaaagcaacttaatacccgcagaatgatttctgcgggtaagtattagcttattttttcgagcattaatcccgcgcgtaatcccaacgctaccaacggattagggaataacacatactctacatcatgggttacggtaaaacgttcctctccgtcctgcgccagcaatgttcctttctcaaacggcataaaattcagcgtgtcacttgccatatgcatttcgaaggacggcgagtggcgagtaatttgcgaaaccacccgataacggagcggcggtgttctcacgataccgacactctcaccagatagcagcgcagcaattgcgctggcagttactgcaaactggcgaagatcgttttgcccaaagggcaacgctttgccaagttccagcgtacaggccagcgcgccaaaatgtctggcgctgaaatgggtaaacgtaccaccaggttcctgatggaacaccagcgcctccagccccgccgcacccagccacgtcagaaatttctcgtcccagggaatgtcgcgttgcggtaatacaccgaactgcggatgcaaggagccacgaattgcggtatgtagatcaaggtgccagcgcacagattctttgccctggtcataaaaatcttccaggcactgttccagttcgcgcgcccgacaggtttctccgctttcagcaaatagctgccaacgaccgccaaacattcgattcatatcgctatggcaataacgtttcccttgcttcagcgcaggaggattcccgaggatcaccagcaaccgccaacgtaacgggatctcgccgtgagatatcgcgccaagcaacgcgtccagcatctccacaggtgccgtctcattaccgtgtattcccgctgaaatcaccagtgcgccttgcggtggcgttaatggcgtcagttccagcacaccatcgcccagccagcgccagcgaacgccgttgatttctcgctcggtgataaccggttttttacccgttaaggtcagagcaagaaaattatccattgccccctccctcgcgctggaacggataaaccgaaccgagattcagtaattggctcaatacatccagtgcttcccgcccttcgcgcagcaattgcgggtcggccagatcggcagcagtaaggcgatcgcggtagtaacgatccacccagtcattgagcgcattaaacagcgtatcgttcatcatcaccgccggattcaccgcccggcgttcttcttctgtcaataccacccgcaaccgcaggcacgccgggccgccgccattcgccatgctttcacgtaaatcaaagacttttagttcgctaatcgggttgtcagcggcaaggagttcattgagataaccccatactccggcgtgttcccgacactcctgaggcagcaccaacatcatggaaccatcatcgcggctcagcagttggctgttaaacagataggtagacaccgtatcagacacggaaacctgagttgccggaacttctatcgccataaaaccattgacccgcgcacgcaggtttgccagtaactgtgactggcgagcgaacgcctgttggtggcaaaacagcacctggcggttactcacggcaatcacgtcattatgaaaaacgccctggtcgataacgtccgggttttgctgggcgaaaatcacctgttggggattcacctgattcagccttgccaccgcctcgctggcttcgcgagtctgtcgcgccggataacgggaaggccgggtatcattgccttcttctcgcccgtagacaaaaagttgcatacccggttcaccgtaatgaccgccgagacgattgtggtttgccgccccctcatcaccgagcaacgctacctgtggcaacgccgaatggacgctaaatttctcttcgtcgttaaaaatcgcttttaacagcgattcagtgacgggcgcttccagcgaacggtgaaatttattgttcaggttggcaacggtgagatgcactttgccatccagcgtatcggcagatggcgcgatcgttgccgcattggctacccacattggcgaagcggaactgacgctggaaagccagtgcggtgcctggcgtgcaactttttccagtacctgctcatcgctaccactgaatcccaactgacgcagcaccggaataaacggacgctcgtgcggcgggatcacggcctgggggaatcccgcatcggcaagggctttcattttcagtaagccctgcttcgccgccagtcgcgggttagacacctgaaaacggtgacgggtagaggcttcattaccaaacgacaggcccgcgtaatgatgcgtcagccctaccagcccgtcgaaattgacttcccaggcgttcatcgcaccacctcatcggaaaaatccagcccggggttaagcgtggcgggcaatgttaacgagtccgactccaggctcgccatcggccatgcgcagtaatctgcggcataccaggcgctggggcgatggttaccggaagcaccaatgccgccgaatggcgcggtactggcagcaccggtaagcggtttgttccagttaacaatccccgcccgcgcctccagcaacagttgatcgaacttttcccgctcgggggaaaccagaccgcaagagagtccgaagcgagtgttattcgccattcgaatcgcttcatcgaaagtatcataacgccagacgcgcaataacggtccgaacacctcttcatctggtacgccagcaacgcctgtcatttcaatgatccccggcgtcagcaacgatgtccctgcttgtaataagcgcggcgcaagcaggggtcgtccgcccatcgcttccagttgctgccatgcagtaaccacctgctgtgcggcctgttcagaaatcagcccgccaataaacggctgcggttcgtcatcccagttgcccggcgttaatcgctggctgacggcaaccagacgagcaagaaacgcatcgccctgcgccccgcttttcagcaataaacggcgggcgcaggtgcagcgttgaccggctgtgacaaacgccgactgaatggtcagatggacagccgcgtcgatatccgccacctcatcgataattagcggattattaccgcccatctcaagggcgagaattttctccggctgaccggagagctggcgatgcaactggtagcctgtattggcgctaccggtaaacagcaaaccgtcgagatcctccagcgcactcagcgcctgacccgtttcacgcccgccctgcaccaggttcagcacgcctggcggcaagccagcctgctgccataaacgcattaccgcttcgccactccacggtgtcagttcgctgggtttaaagataatggtgttacctgccagcaatgccggaacgatatgtccgttcggcaaatgaccagggaaattatacggcccaaacaccgccagcacgccgtgcgggcgatgtcgcaggctcgccgcgccgtccggcatttcactacgctgctcgccggtacgaacgtgatacgccttaattgatatcgcgattttattgatcatcgccgtcacttcggttgccgcttcccagcgcggcttacccgtttctctggcaataatcgcggttaattcggctttattgctttccagcagtgcggcaaagcgttcgacaacggcatgacgttcagcaaatgaaagccgcgcccagcgcggaaacgccgcacgggctgcccgacaagcctgctcgacctgagcggcatcggcatcattgccttgccataacacctcgcccgataccggattacgcttcacacgcgatgcgccctggcccgttatccagtcaccgttaatccataaagtcatgctgttttctcctctgcgcacaggcgcaccagacgaacgcgatccccggcgtggcatttgagggcatccagttgtgcggcggttaaaatcaaacgctcggttgccggatcggtacgcaccagcaccacgcggaaatggtgataattttcattggcgaccaggcaggctgggaaatcgccctgcgcaggctgcccttctgccacttccaccagccgacttttacggatggcgcgcacgcggtcgatgtcacactcaagcgtcggcccaccgtcaaagatgtcgatatagttacggtagcgaaaaccttctttctccagcaccgcgcgggcaggcgcggtttgcggatgtacctgaccgatgacgtcctgggcttcctgggataaaaagtgggtatagatcggatgtttcggcatcagttctgcaataaatgccttttgcccggtgccgcagagaaaatcggcgcggctaaaatccatcgaaaagaagcgtttaccgaggctttgccagaacggtgaatagccgtgttcgtcaatcaccccgcgcatttcagcaaccactttgtcattaaacttgtcgcgaaaagccgccataaacataaagcgcgatttcgacagcaaatagccgttgccctctttgcgccagtccgggtcgagaaacagcgtgcacagctcgctgctgccggtgtgatcgttactgagaaacagcgtcggcaatgcgttatagacattcagctcttttgaggcgtgaaccaacgtgccgacgcgatagttgtaccagggatcgttcagcccaaccgccacctcaatggcacaaatccccgccacggtgcctgtctcgctatcttccagcacgaacacatagccctgctcacttttgggcagttcgccttgccaggttttgattgccctttcgatacgcgccgaaagcgtggcttcattggcgggaagcgacgtcaggccgccgcccgttttgctggcaagctgcatcagcgccgagacatctgatcgctcaacgggacggatgaccatcatgatgaacctcggctaacaaagtgttcgcaagcagctgcaaagcgatccagtccggtcgtcacctcttcttcgctgacattgagcgcaggcgcaaaacgcaccacgttgccacccgcaatcagtaccatcacgcctgctttcgccgcttcctgagagatctgtttcgcttgcccggcgtaatcggcattcagtacacagccaatcagcaaacctaagccgcgaacttcactgaacaaaccatagcggtgattaatagtattaagacgctcaacaaaccagtcgtgacgctgtttaacgccattaagcatctctggtgtgttgatgagctccagcactttgcctgccaccgccgaggccagcggattaccgccataggtggtgccatgagtgccaacggtcatcacgcgggcgcactcttcggttgccaacaacgcaccgaccgggaaaccgccgcccagcgctttggcggtagttaacagatcaggcgtcacgccgtagtgcatataggcatacagttccccggtgcgcccgacgccggtttgtacttcatcaaaaatcaacagcgcattgtggcggttacacaattcacgcagaccttgtaaaaacgcgttgctggctggcaccacaccgccttccccctggatgggttcgacaatcaccgcacaggtagagtcgtcaatcagcgcgctggcagagttaatatcgttatatgcagcatgacgaatatccgccggcagtggcgcaaaatcctgtgaataggctggctgcccacccgcactgacagtaaacagcgtgcgaccatgaaacgcatttttgaacgccacgatgccgctcttatggctgccgtagcggtcgtgagcgaatttacgcgccagttttagcgccgcttcgttggcttccgcaccggagttacaaaagaagacgcgatcggcaaacgtggcgtcgatcaattttttcgccagtcgcagtaccggctcgttggtgtaaccgttgccggtatgccagaacttactcgcctgttcgttcagcgcttcacgcagttccggatgcgcatggcccagcgcgttcaccgcaatgccacccgcgaagtcgatatactctttcccctgctgatcccacaagcgcgaaccttcgccacgtaccggtataaagggtgccggagcgtaaacaggtatcatccattcatcaaagttttcacgcgtaattggctgagacatagcgacctctacagtaaataattcgttatttatatgttaataataagtaatgtttgcgctgtaaatgtagattgcagggttcgtgccagccagtgataaaagtgcataaacggcggaggctaactggaaatcaaggagttataaccaaaccatatgcatttaaagtgcatataaagtgaatacgtttgcgatgtgggtgaataaaaagaataaaaaacgcaatgttatgcagaagtaaaatataattctggaattgtgatcattgacgaaatttactggaaattactgcgccattctgacgcagcgcgcaccaaaagcgggcattttttgcgccatcgttgacatcattaacaaccatcgatcaaatcacttaacaacaggcggtaagcaacgcgaaattctgctaccatccacgcactctttatctgaataaatggcagcgactatgaaatttgtctcttttaatatcaacggcctgcgcgccagacctcaccagcttgaagccatcgtcgaaaagcaccaaccggatgtgattggcctgcaggagacaaaagttcatgacgatatgtttccgctcgaagaggtggcgaagctcggctacaacgtgttttatcacgggcagaaaggccattatggcgtggcgctgctgaccaaagagacgccgattgccgtgcgtcgcggctttcccggtgacgacgaagaggcgcagcggcggattattatggcggaaatcccctcactgctgggtaatgtcaccgtgatcaacggttacttcccgcagggtgaaagccgcgaccatccgataaaattcccggcaaaagcgcagttttatcagaatctgcaaaactacctggaaaccgaactcaaacgtgataatccggtactgattatgggcgatatgaatatcagccctacagatctggatatcggcattggcgaagaaaaccgtaagcgctggctgcgtaccggtaaatgctctttcctgccggaagagcgcgaatggatggacaggctgatgagctgggggttggtcgataccttccgccatgcgaatccgcaaacagcagatcgtttctcatggtttgattaccgctcaaaaggttttgacgataaccgtggtctgcgcatcgacctgctgctcgccagccaaccgctggcagaatgttgcgtagaaaccggcatcgactatgaaatccgcagcatggaaaaaccgtccgatcacgcccccgtctgggcgaccttccgccgctaatttagcagctctcctggctcaaactgggtcaggagaattaaccttgagaaaaatcaacaaactgtcagtaatgatttgttgcctgccgtcctttgttataccgtctctgcgtttttagttgtctgaccacttctctattatcaagtttgatataggaaactccacgatgaacgctgagcgtaaatttctttttgcctgtcttatttttgcgctggtcatttacgctatccacgctttcggtttattcgatctgctcaccgatttaccccacttacagacactcatccgccagagcggatttttcggctatagcctctatattctgttattcatcattgccaccctcttgctgttaccaggaagcatactggtgatcgcgggaggaatagtttttggcccgctcttagggacactactctcattaattgccgccacgctggcctcctcgtgctcattcctgctggcgcgctggctgggacgtgatttactgctgaaatacgttggccatagcaataccttccaggccattgaaaaaggcattgcgcgtaacggtattgattttcttattctgacccgcttaatcccgttgtttccttacaatattcaaaattacgcttacggattaaccacaatcgccttctggccttatacccttatttcggcactcacgaccctacccggtattgttatttataccgtgatggcaagcgatctcgccaatgaaggcattacgctgcgctttattttacaactctgtctggcgggcctggcgctgtttattctcgtccagctcgcaaaactctacgcccgacacaaacatgtggatctgtctgcttcgcgccgcagcccacttactcacccaaaaaatgaaggatagaacgatgttgcaacattattcagtgtcatggaaaaaaggactggctgcactctgtttactggctgttgctgggcttagcggctgcgatcaacaagagaatgcggcggcaaaagtggaatacgacggactttcgaacagccaaccgctgcgtgtcgatgccaataaccatacggtaaccatgctggtgcaaattaatggtcgtttcctcaccgacgacactcgtcacggtattgtgtttaaagatggctccaacggacataaatcgctgtttatgggttatgcgaccccgaaagcattttatgaagccctgaaagaggcaggtggtacgccgggcgaaaacatgacgatggataataaagaaacgactcatgtcacaggcagcaaactggatatttcggtcaactggcaaggggcggcaaaagcgtattccttcgatgaagtgattgttgacagtaatggcaagaaactggacatgcgctttggcggtaatttaacggcagcagaagagaagaaaacgggttgcctggtgtgtctggatagctgcccggtcggcatcgtcagcaatgcaacatacacttatggtgcggttgaaaaacgtggtgaagttaaattcaaaggcaatgcctcagttctcccggcggataacacgctggcaacggttacctttaaaatcgccgaataaagccaggataaaggatgatgatgatgcaatcgcgaaaaatctggtactaccgtataaccctcatcatcctgttgttcgctatgctgctggcatgggcgctgcttcccggcgtccatgagtttatcaatcgcagcgttgcggcgtttgccgccgtggaccaacagggtatagaacgctttattcagtcttacggcgcactggcggcagttgtctcgttcttgttgatgattttgcaggccattgctgcaccgctacctgcgtttttgatcacctttgccaatgcgtcgctgtttggcgcgttctggggcggcttgctgtcgtggaccagttcgatggccggcgcggcgctgtgcttttttatcgccagagtgatgggccgcgaagtggtggaaaaattaaccggcaaaaccgtgcttgacagtatggacggctttttcactcgctacggcaaacacaccattctggtctgtcggttattgccttttgtccctttcgatccaatcagctatgctgccggtttgacttcaatacgttttcgctcgttttttatcgccaccgggcttggtcagttaccggcaactattgtttattcctgggcgggcagcatgttaacaggcggtactttctggtttgtcaccggactgtttattctgtttgccctgaccgtggtgatttttatggcgaagaaaatatggcttgaacgccagaagaggaatgcctgatgggtttaccgccgcttagcaaaattcctttaattttacgtccacaggcgtggctgcatcgtcgccattacggcgaggtgctaagccccattcgctggtgggggcggatcccgtttatcttttatctggtgtcgatgtttgttggctggctggagcgcaaacgctcaccgctcgatccggtagtacgatcgcttgtcagcgcgcgcattgcgcaaatgtgcctgtgtgagttttgtgtggatatcaccagtatgaaagtcgccgagcgcaccggcagcagcgataaactgctggcagtggctgactggcggcaaagcccgctctttagcgatgaagaacggctggcgctggagtacgccgaagccgcaagcgtaacgccgccaacggtcgatgatgccctgcgtacccgactggctgcgcattttgacgctcaggcgctcaccgaactgacggcattgatcggcctgcaaaatctgtcagcccgttttaattctgccatggacattcccgctcaggggctgtgccgtattcctgaaaaacgttcttaaggagagatgatgcgccattgtgggtggttgctgggattgttatcgctgttttctctggcaacacatgccagtgactggcaagaaattaaaaatgaggccaaagggcaaaccgtctggtttaacgcctggggcggcgataccgcaattaaccgctatctcgactgggtgagcggcgagatgaaaacccattacgctataaacctgaagattgtccgtctggcggatgccgcagacgcggtgaagcgcattcagaccgaagccgcagccggacgtaaaacgggcggctcggtggatctgctctgggtgaacggcgaaaacttccgcaccttaaaagaggccaatttattacaaacgggctgggcggagactctgcccaactggcgctatgtcgacacacagctgccggtgcgggaagatttttctgtgccgacacaaggtgcggaatcgccctggggcggcgcacaactgacgtttatcgcccgccgcgatgttacgccacagccaccacaaacgccgcaagccttactggagtttgctaaagccaatcccggcacggttacctatccgcgcccaccggactttaccggcacggcgtttcttgaacagttgctgattatgctgacgcccgatcccgccgcattaaaagaagcgccggacgatgcgactttcgcccgtgtcactgctcccttgtggcaatatcttgatgtgctgcatccgtatttgtggcgcgaaggaaaggatttcccgccttcacccgcgcggatggatgctctgctgaaagccggcacattgcgcctgtcgctgacctttaaccccgcgcatgcgcagcaaaaaatcgccagcggcgatttgcctgcaagcagttacagttttggctttcgcgaggggatgattggcaacgtgcatttcgtcaccattcctgccaacgcgaatgccagtgctgcggcgaaggtagttgccaatttcctgctctcacccgatgcgcaactgcgtaaagcagatcccgctgtctggggcgatccttctgttctcgatccgcaaaaactgcctgacgggcagcgcgaatcattgcaatcaagaatgccgcaggatctgccgccggtactggctgaaccgcacgcaggttgggtaaatgcgctggaacaagaatggctacaccgttacggtacgcattaatctttttgctgtgggcgatggtggcggtgatttatgcaccgctgatcccggcagctctcacgctgatatcgcctgctttgtcgttgacacactggcaggcgttatttgccgatccacagttaccgcaggcattactggcaacgctggtgtcgacaaccatcgcggcggtcggggcattgttgattgccctgctggtgattgtggcgctgtggcctgggccgaaatggcagcgtatgtgcgcccgtctgccgtggctgctcgccattccccatgtggcttttgccaccagcgcccttctgctctttgctgacggagggctgctttatgactatttcccgtatttcactccgccaatggaccgatttggcatcggtctgggcctcacccttgcagtgaaagaaagcgcatttctgctgtggatcttagcagcagtattgagcgaaaaatggctgttgcagcaggtcattgtgctggattcgctgggctacagccgctggcaatgcctgaactggctgctgttgccctccgtcgcgcctgcgctggcaatggcgatgctggcgattgttgcctggtcgctgtcggtcgtggatgtggcaattattctcgggccaggtaatcccccgacgctggcggtaattagctggcagtggttaacccagggcgacattgaccaacaaacaaaaggcgcgcttgccagcctgctgttgatgctgttactcgccgcctacgttttgctgagctatctgctatggcgcagctggcggcgcactattccccgcgtagatggcgttcgcaagcctgccacgcctttattgccgggcaatacgctggcgatttttttacccttaaccggtgtgctgtgtgtggttctgctggcgatcctcgcggatcagtcgacgatcaatagtgaagcgctcatcaacagcctgacaatggggctggtggcgacattcatcgctttgctcctgttactgctgtggctggaatgggggccacagcgtcgccagttgtggctatggttgcccattttattacctgctctgccactggtggcgggccagtacacgctggcgctatggctgaaactggatggaagctggacggcggtggtctgggggcatctgctgtgggtgatgccgtggatgctgtttatcctgcaacccgcctggcagcgcattgattcacggttaattttgattgcgcaaacactgggctggtcgcgggccaaaatcttcttttacgtgaaatgcccactcatgttgcgccctgtgctgattgccttcgcggtgggatttgcagtcggtattgcgcagtatatgccaacgctgtggctgggcgcggggcgttttccgacgctcaccactgaggcggtggcattaagcagcggcggcagcaacggtattctcgccgcccaggctttatggcaactgctattaccgcttattatttttgccctgaccgcgttagtcgcaaaatgggtaggttatgtcagacaaggactccgctaatgctctgcgtgaaaaatgtttcgctacgtttaccagaaagccgcttgctgacaaacgttaactttacggtggataaaggtgacattgtcacgttaatggggccgtctggctgtggaaaatccactctgttttcatggatgattggtgcactggccgaacagttttcttgtacaggtgagctatggctcaatgagcaacggattgacatcctacccaccgcacagcgtcagattggcattctttttcaggatgcactgttatttgaccagttcagtgtcgggcaaaatttactgctggcgctaccggcgacacttaaagggaatgcccgacgtaatgccgtgaatgatgcacttgagcgttcaggccttgagggagctttccatcaggatcctgccactttgtctggcggtcagcgagcgcgcgttgctctactacgcgcccttctcgcccaaccaaaagcgttactcctggatgagccattcagccgtcttgatgtggctctgcgcgataattttcgccagtgggtgttcagcgaagttcgcgccctggcgatccccgtcgttcaggtaacgcacgatctccaggatgttcctgctgatagttctgttctggatatggcgcagtggtcagaaaattacaacaaactgcgataacgcaaagtttttctcaatgcgtcagttcagaatggcgcactcaaaactacaatgtcgggattttcgatgaaacgtgtttctcaaatgaccgcgctggcaatggctttagggctggcttgcgcttcttcgtgggccgctgaactggcgaagcctcttacacttgaccagcttcaacaacaaaatggcaaagcgatagatactcgccccagcgcgttttataacggctggccacaaaccttaaatggcccttctggtcatgaacttgccgccttaaacctctctgccagctggcttgacaaaatgagcaccgaacagctcaacgcgtggatcaagcaacataacctgaaaaccgatgctccggtggcgctgtacggtaatgacaaagatgtcgacgccgtcaaaacgcgactgcaaaaagcaggtttaacgcatatctccatcctgagtgacgcgctaagcgaaccttcccgtctgcaaaaactgccgcattttgagcagctggtttatccgcaatggctgcacgacctgcaacaaggtaaagaggttacggcgaaacctgccggtgactggaaagtcattgaagcggcctggggcgctcctaagctttaccttatcagccatattcccggcgctgactacatcgataccaacgaagtggaaagtgaaccgctgtggaacaaagtttctgatgaacaactaaaagcgatgctggcaaaacacggcattcgccatgacaccacggtcattctgtatgggcgtgacgtatacgctgcagcgcgtgtggcgcagattatgctttatgctggcgtgaaagatgtgcgcctgctggatggcggctggcaaacctggtccgacgcgggactgcctgttgagcgcggaacgccaccgaaagtgaaagcggaaccggatttcggcgtgaagatcccggcacaaccgcagttgatgctcgatatggaacaggcccgtggactgctgcatcgccaggatgcatcgctggtgagcattcgttcgtggccagaatttatcggtacgaccagcggttacagctatattaaaccaaaaggtgaaatagccggcgcacgttggggacacgctggtagcgactcgacgcatatggaagattttcataacccggatggcaccatgcgcagcgccgatgatattaccgctatgtggaaagcgtggaatatcaaaccagagcagcaagtttcattctactgcggcaccggctggcgcgcgtccgaaacctttatgtacgcacgcgccatgggttggaagaatgtttccgtgtatgacggcggctggtacgaatggagcagcgatccaaaaaatccggtagcaaccggtgaacgcggcccggacagtagcaaataacattgcaattactgacgctggagcgacttcagcgtcagatacccactccacacccgcgtaaaggtcgtcatccagcacaacgcaccgaagatccacgcaaaccacgcaaaccatgcagggaataaacatcccagcacaaacagtaagatcgtttctgtgccttcggttaatccccccagatagtaaaacgacttatgtgcataaccggggttatcaatctgatgttttgctgccagtgcagcaaaggcgagaaaactgctgcccgtgccgataaacgcaaacaacaaccagccgcctgccagcgcattttgctccggtgcagcaagaataaagccaaacggcaccagcgcgtaaaagagaaaatcgagagaaatatcaagaaagccgcccgcgtcggtaagctctctgcgccgcgccagcgcaccgtccagaccatcaagcagcctgttcaacaaaatgacgactagcgccgccagataccagcccagcgccagaaacggcagagccagcacgccgatggcaaatcccactaatgttaaaccatctggcgtaatgcccggtttatcaagaacccgcacgcactgatgcaacaacggtttaatccggggatgaagatggcggtctagcacaggcactccttaaatataaagcctttctgattgagcaacagtgcggatattatggcatttttcgcttatctgcccgtgtgtaatttatgaaaatgattgaagttgttgccgccatcattgaacgtgatggcaaaattttactcgcgcaacgccccgcccagagcgatcaggcgggattatgggagtttgccggtggtaaagtcgagccggatgaaagtcagcggcaggcgctggtgcgtgagttacgcgaagaactgggcatcgaagcaactgtgggtgaatatgttgccagccatcagcgagaagtttcggggcggattatccatcttcatgcctggcacgtacccgacttccacgggacgttacaggcacatgaacatcaggcgctggtctggtgctcacctgaagaggcgctgcaatatccgctggcccctgctgacattccattattagaggcgtttatggctttacgcgccgccagaccagcggattagtgctaagggttttgtcatcacgctggcattgcagcagtattccttcggctttaattaccgccccttcagaataattttgatcctgataaacgcagcactgagtacagggctgcgctgactgcccgcctgaactgaacacttctggcggtacgtttacctccacgtccggacgataatgcgggttagccagtgcaattaatggaaatgctaatactacggcgaacaatgctcgactcacagggaactccttaacgttattgtctctgctactgataacggtagccgggtggcaaaactttagcgtctgagttatcgcatttggttatgagattactctcgttattaatttgctttcctgggtcatttttttcttgcttaccgtcacattcttgatggtatagtcgaaaactgcaaaagcacatgacataaacaacataagcacaatcgtattaatatataagggttttatatctatggatcagacatattctctggagtcattcctcaaccatgtccaaaagcgcgacccgaatcaaaccgagttcgcgcaagccgttcgtgaagtaatgaccacactctggccttttcttgaacaaaatccaaaatatcgccagatgtcattactggagcgtctggttgaaccggagcgcgtgatccagtttcgcgtggtatgggttgatgatcgcaaccagatacaggtcaaccgtgcatggcgtgtgcagttcagctctgccatcggcccgtacaaaggcggtatgcgcttccatccgtcagttaacctttccattctcaaattcctcggctttgaacaaaccttcaaaaatgccctgactactctgccgatgggcggtggtaaaggcggcagcgatttcgatccgaaaggaaaaagcgaaggtgaagtgatgcgtttttgccaggcgctgatgactgaactgtatcgccacctgggcgcggataccgacgttccggcaggtgatatcggggttggtggtcgtgaagtcggctttatggcggggatgatgaaaaagctctccaacaataccgcctgcgtcttcaccggtaagggcctttcatttggcggcagtcttattcgcccggaagctaccggctacggtctggtttatttcacagaagcaatgctaaaacgccacggtatgggttttgaagggatgcgcgtttccgtttctggctccggcaacgtcgcccagtacgctatcgaaaaagcgatggaatttggtgctcgtgtgatcactgcgtcagactccagcggcactgtagttgatgaaagcggattcacgaaagagaaactggcacgtcttatcgaaatcaaagccagccgcgatggtcgagtggcagattacgccaaagaatttggtctggtctatctcgaaggccaacagccgtggtctctaccggttgatatcgccctgccttgcgccacccagaatgaactggatgttgacgccgcgcatcagcttatcgctaatggcgttaaagccgtcgccgaaggggcaaatatgccgaccaccatcgaagcgactgaactgttccagcaggcaggcgtactatttgcaccgggtaaagcggctaatgctggtggcgtcgctacatcgggcctggaaatggcacaaaacgctgcgcgcctgggctggaaagccgagaaagttgacgcacgtttgcatcacatcatgctggatatccaccatgcctgtgttgagcatggtggtgaaggtgagcaaaccaactacgtgcagggcgcgaacattgccggttttgtgaaggttgccgatgcgatgctggcgcagggtgtgatttaagttgtaaatgcctgatggcgctacgcttatcaggcctacaaatgggcacaattcattgcagttacgctctaatgtaggccgggcaagcgcagcgcccccggcaaaatttcaggcgtttatgagtatttaacggatgatgctccccacggaacatttcttatgggccaacggcatttcttactgtagtgctcccaaaactgcttgtcgtaacgataacacgcttcaagttcagcatccgttaactttctgcgatagcagcagatatgccagtaaagaaatcccatttgactatttttttgataatcttcttcgctttcgaacaactcgtgcgcctttcgagaagcaagcattatataatgccaggccagttcttcttcaattgtcccgttttgaaaagctgtgcttgatatcgagatcatccatgataattccgccgcccatattagcttcgccgaggatttaccggagctatgattagcgcaatcagagatatagtctgagggaaaaacagcaaatttattcaacaaggcgataacctgctctggggcttcctccatgtttgctttaaaggtattggctccatggtcgccagaaagaaaatgctccattaaggcacaataactttcgctatcttcgataccccattgatcctctaaagactcgcgtcttttacttatgatatcgatcgagtcaaaaggaagcacatgatattggaaggtatctttgccaggttcaggctttcgcggccagaactccagcgtttcagaccattgcttatgatagaatcgataaggtgcgatcaattgtagcgcctgtaacttctcgatactgagcggctcaatacctttagcctgataataatgcagttgttctttttttgctttaaaaccggcccgaacaataagccccatcataattaatagataaagaaaagagcatcccgcggtaatcaggcctctttcattcaaaccgttggatgttatcgctgcgaacacaaacattacagcgacaacacatgttaaataaaacccccacttacaaagcagcatggccttattttctttaatcatccgttcaaaattactattaaatatttcccagccattaaaagaatacttctcgctcccaggatggttttgtaataaaacttttttcatcacattccctgttattacatactttagaggcgataattttatccatgcaaaaaaaatatccaacgaattttcttgatccgctggatatttcagaatatgactcgaatagcacgaaagattcactcgcttacgctatcgccccgcttccgacttcatctgctggcggactttttttcgcactacgtttacgcggtgcagcctttttcttatcagcactgccaccactgcccggagccacaatgccgcgaaactgccgcaccggcgtacgtttggcttgatcaataagctgatatagcgtccccaccagcggctgcataaagtcctgatagcgacactgcttttcgctgatttgcgtcagcaccgattcccagtgcgcggtcatgtccggtcgcgtcgccatctccggcagcgaatggaatagcgcttttccggcgtcggtggagtggatatagcgcccttttttggtcaggaaaccacgcttgaacaacagttcaataatcccggcacgcgttgcctctgtccccagaccatcggtcgcacggaggatctttttcagatctttatcctgcacaaagcgcgcgatcccggtcatcgccgaaagcagtgttgcatcggtaaaatggcgcggcggctgggtttgccgctctaccacttcacctttttcacacagcaactcatcgcctttcgccaccacaggcagtggcgtgccgtcgttttcttcatcgcgctctttgctgcctaacagcgtgcgccagcctgcttcagcaagaaaacgcgctttagcgacaaatttgcctttggcaatgtccagttcgataacacacttgcggaacaccgcatccgggcagaattgcatcagatactgacgggcaatcaggttatagaccttcgcttcgttctccgtcaggttgatcgcagaactccgtgcggtcggaatgatggcgtggtgcgcatcgacctttttgtcatcccaacagcggttgcgtatatctggatctaccactggctgcggcaacagatccggtgcatgaacactgatggcattcatcaccgcgtggcgtccggcaaaatgttcttctggcaaatagcgacaatcagaacgcggataagtgattagcttgtgcgtttcgtacagtttctggcagatatcaagcacgttctgcgcactcagaccaaaacgttttgccgcttcaatctgcaacgctgaaagcgaaaaaggcagcggcgcggattctgattcccgtttatcgttatagctggtgacaatagccggttgaccactaatgcggttaaccacatgctccgccagtggacgatgtaacaagcgcccttcttcatcctggtacggttcacacgcttcgctcggttgccagatagcggtaaaccgctcatcggcaggtgtcacgatatgtgctttgacttcaaagaagtctttcgccacgaagttttcaatctcttcatcgcggcgcaccaccagcccaagcacgggcgtctgcacgcgtcccacggaaagtacgccctgataaccggcattgcgaccgagaatggtatacgcacgggtcatattgatgccgtacagccagtcggcacgcgctcgcgccagcgcagaaacgcacagcggtacaaactcactgttggaacgaagacggtcgatcgcccgctcaaccgcctgcgggttcaggtcgtttatcaagcaacgctgtacctgctggcgcttttccggtgccagttgcagatagtccagcacttcatccaccagcaattgcccttcacgatccgggtccccggcgtgaacgatttcgctggcttcatgcaggaaccgtttgatgacgttaagttgtttggtcacggagggtcggggctgtaattgccacttttccgggacaatcggcaaatccgcaagattccagcgcgcatagcggctgtcgtaggcgtctggctgcgcctgctcaagcaggtgaccgatacaccaggtcaccacctgaccattaccgcactcgataaagccatcgcctttccggtgcggtttgggcaggacatcagcaatggcgcgcgccagactcggtttttcggcaataaacaaccgcattgaattaacgaatctcaaccatggcacgaccgccgcgcgctggcaccagttcgccaattgccgtcagttcaatgccaaactcggcggctgtagctttgacctcattttctgcttccggcatgaccgccagcagcaaaccgccagaagtttgcggatcacacagcagatcgcgcacttcacgcggcatttcacccatcagatgaccgtagctggcaaagttacgttcagtgccgccaggtactgcgcccaacttaatgtactcttcaacaccggggagtttcgggatcgcttcatagtcgacgcgtgcctgcacaccagccccctgacacatttcgctcaagtggcccagcagaccaaagcccgtaacgtcggtcatcgcttttacgccttcgatgttggcaaaggacgcgcctgcgatgttcatccggcacatcacttccgtcgccagtccctgatgttctggtttcaacagtgattttttctcagccgtggtaagaacgccgatccccagcggtttcgtcaggaacagtttgcatccggcttgtgcggtactgtttttcttcacccgctcggtcggtacgatccccgttaccgccagaccaaaaatcggctccggcgcatcgatggagtgaccgccagccagcgcaatacccgcctgacgacatgcatagcgtccaccttcggtcacttcgcgggcaatttctggggaaagtttgttaatcggccagccgaggatcgcaatcgccataatcggtttgccccccatcgcgaagatatcgctgatggcgttagtcgccgcaatgcggccaaaatcgaaaggattatcaacgatcggcataaagaagtcggtggtactgataacgctggtgccattgcccagatcgtacaccgccgcatcgtcgcgggtttcattacccacaagcaaattcggatcaacaaacttcgcctgctcactatgcaggatggtttccaacacttttggggaaattttacagccgcaaccagctccgtggctgtattgggtcaaacgaatcgagttctcgctcatggacatctcctgtcaatgcaatccgggtatggtaaccctcattccgtgaagtgataagtgagagtgtctgaattcctgcgcctttgctcacaatccagacagtttcgcgacaattatcagaaataagttacaaacggcgtcgggtccgggacgttaatcgacgtagatgctttcagctgcggcgtaccgaggtagagaaaaccgacaattttatcctgctcacggcaaccgaatgcttcacgcactaccggactttcagttaatgcgccactgcgccagatgccgccaaacccctgggcaactgctgccatttgcatcgccatgaccgcgcatccggcagacatttcctgttcccagcgcgggactttatgattctcttcgcatttcgccaccaccgtgatgatgagcggtgcgcggaacggcgcattacgggctttgtcgatagctttgtcatcactaccggcagcaatcgccccctgttccagtacggcgctgaaacgctcgcgcccttccccttcaatcacaaaaaaatgccacggttgcatggacttatggtccggcgcacgcatacccgcacgcaggatgttttgcagttgttcacccgttggcgcgggttcagccaagcgggaggcgctacggcgattgatcaatagttcgagtgcatccatttgattaactcctgtcgtgatatttattcacaaaattaacacgagagtggattttgttacagcacagtccgcaattcctgctgacaagtaccggttgggtcattacgataaccacatctattgcgcctgtgacaggtgtgaccttaagttgggagaatacatgcgaaccctttggcgatttattgccggattttttaaatggacgtggcgtctgctgaatttcgtccgtgaaatggtacttaacctgttctttattttcctcgtactggttggtgtggggatttggatgcaggtcagtggtggtgattcgaaagaaacggccagtcgtggcgcactgctgctggacatttctggtgtgatcgtcgataaacccgacagttctcagcggtttagtaaattaagccgccagctgcttggtgccagttccgatcgtctgcaggaaaactcactgtttgatatcgtcaacactattcgccaggcgaaggacgaccgcaatatcaccggtattgtgatggatctgaaaaacttcgcaggcggcgaccaaccgtctatgcagtacatcggcaaagctctgaaagagtttcgtgacagcgggaaaccggtttatgccgttggcgagaactacagccaggggcaatattatctcgccagtttcgccaataaaatttggctgtctccgcaaggcgtggttgatctgcacggctttgccaccaacggtctgtactacaaatcgttgctggataagctgaaagtttccacccatgtgttccgcgtgggtacgtataaatctgccgttgaaccgtttattcgtgatgatatgtcaccggcagcccgcgaagctgacagccgctggattggtgagctgtggcaaaactatctgaatactgttgccgctaaccggcagatccctgctgagcaggtattccctggcgcgcaagggttgcttgagggtttaaccaaaaccggtggcgataccgcgaaatatgcactggaaaacaagctggtcgatgcactggcatcgagtgcggaaatcgaaaaagcactgaccaaagaattcggctggagtaagactgataaaaattatcgcgccatcagttattacgattacgcattgaaaacgccggcagataccggtgacagcatcggtgtcgtctttgctaatggcgcaattatggatggcgaggaaactcaggggaatgttggcggtgataccactgcggcacaaatccgcgacgctcgccttgacccgaaagtgaaagcgattgtcctgcgtgttaatagcccaggcggcagcgttaccgcgtctgaagtgattcgcgctgaactggcagcagcccgggcagcgggtaagcctgtggttgtatcgatgggcggcatggcggcatctggtggttactggatttccacgccagctaattacattgtggctaaccccagcaccctgaccggttctatcggtatcttcggcgtgatcaccaccgtagaaaatagtctggattcgattggtgttcatactgatggtgtctcaacttcaccgctggcggatgtttctatcaccagggcactgccgccggaagcgcagctgatgatgcagttaagcattgagaatggctataaacgctttatcacgctggttgctgatgcgcgtcattcgacgccggagcagattgataaaattgcccagggccacgtctggaccggtcaggatgcaaaagctaacgggctggtcgatagtctcggggatttcgatgatgcggtcgccaaagcagcagagctggcaaaagtgaaacagtggcatctggaatattacgttgatgaaccgaccttcttcgacaaagtgatggacaacatgtctggttctgtccgggcaatgttgccagatgcgttccaggccatgttacctgcaccgctggcctcggtagcctctaccgttaaaagtgaaagtgacaagctggccgcgtttaatgacccacaaaaccgttatgcgttttgcctgacctgcgccaacatgcgttaagtcttgtactgagtggccgacagatcgtcggccacattattttttacgtcgacgaatcctcttcccgctgtttcgccccatatttccttatccgcatagtatcaggtgcgctccccctgcctcacgtatatacttttgctctttcgatatcattcatatcaatatcatgcaaaagaaatcaatttacgttgcctacacgggcgggaccatcgggatgcagcgttccgagcagggttatataccggtgtcaggtcatctacaacgccaactggcgctgatgccggaattccatcgcccggagatgccagatttcaccattcatgaatatacgccgctgatggattcttcagatatgacgccggaagactggcagcatattgctgaagatattaaagcgcactatgacgactatgatggttttgtcattctgcacggcaccgacacgatggcgtataccgcctctgcgctgtcgttcatgctcgagaatctcggtaaaccggtcattgtgacagggtcacaaatcccgctggctgagttacgctctgacggacaaattaatctgctgaatgcgttgtacgttgcggcgaattatccgatcaacgaagtaacgctctttttcaataaccgattgtatcgcggcaaccgcactaccaaagcccatgccgatggttttgatgcgtttgcctctccaaaccttcctccgttactggaagcaggtatccatattcgtcgtttgaatacgccacccgccccgcacggtgaaggggaattaatcgttcatccaatcaccccacaaccaattggcgtagtgacgatttatccagggatttctgctgacgtcgtgcgcaattttctgcgccaaccggtgaaagcattgattctgcgctcctatggcgtgggtaatgcgccacaaaacaaagccttcctgcaggaattacaagaagccagcgatcgcggtattgtggtggtcaacctgacacaatgtatgtccggtaaagtgaacatgggtggttatgccaccggtaacgccctcgcccatgccggcgtaattggcggtgcagatatgactgtagaagccacgctaaccaaactgcattacctgcttagccaggaactggatactgaaaccattcgcaaggccatgagccaaaacctgcgcggcgaactgacgccggatgattaaggagactgtaatgccccctcgcgccctgttactggtcgatttacaaaatgatttctgtgctggtggcgcgctcgccgtgccggaaggtgacagtacggtggatgtcgctaaccgcctgattgactggtgccagtcgcgcggtgaagcggttatcgccagtcaggactggcacccggcgaatcacggcagttttgccagtcagcacggtgtagagccttatacgccaggccaactcgacggtttgccacaaaccttctggccagatcactgtgtgcagaacagtgaaggcgcacaattacatccgttactgcaccaaaaagcgatcgcagcggtgttccataaaggcgaaaatcctttagttgacagttacagtgccttttttgataacggccgtcggcagaaaacctctctcgatgactggttacgcgatcatgaaatcgatgaattgatcgttatgggcctggctactgactattgcgtgaagtttaccgtgctggacgcgttacagttaggttataaggtaaacgtgattaccgatggttgtcgtggcgtgaatatccagccccaggacagtgcgcacgcgtttatggagatgtcagcagctggggcaacgctatatacgctggcagactgggaagagacacaggggtaattttacgctggcctacaattctgtactggcattgtaggccaaataaaacacgtcagtggcacatctggcaattgatgccatcaacgaaagatttaattcacctcagaaatctcttccaacgacaccttccgcgtttcgatgccaaaaatggagagaaccagcgcacagagcaataacataacaccaagtaccataaacaccgtgatcgacccataatgtgttaataatgccgcaacgccatagggcgtgaagactgcgacgatccgtccgacggcattaacgaaacccgaaccgcgcaggcgtaaatgcgttggccaaagctccgggatataaaccgccgacgcgaagcaaacatacatgtataaaaagaagatcatcaccagtccatagattaaaatcgcccactctgtagtctgaattgaatagatatagcctaacacggcaataataataagtaaggtggagccaaataaccgacgaggaaaatgatcaataattaatgccgcaataaatattcctaccggagcgccaatcataataacagcggtcattaatattgatttatcgacatcaatgccggagttaacaaatatggtcggtatccatacggtgatggtataaagcgaaatgttcattgcaattaaaacagtaatcgcgactaatgtacgtcgtaacatttcacctttaaacaggagccagaaagtacccttgattactttaaccttgctgttgctctgatacgaagtaagcgggggtaaacgaatactcttctctctttcaatttgctgctctacttcacgaagttggcattctgcacctgcgatttgccctttccctgccagccatcgtggcgactcgataaagtatttacctgagagaaaccaggctaacagtatgccaataccacccagcagaaacattattcgccaactaaaaaaagcgataaccaccacgcctatcgccgcagacagcatgggcgaccagttaccaacaaatgagagccgcgcggaccattttccacgcaccgtcgcggggataaactccgtaaatgaggcatagccaaccataatcagcgcccccattcctgttcccatcaggaagcgaaagaagatgagccagtacatatcagggacaaaagcggcccctgttgcagcaataccgacgatgagaagatttatgcgaaacgccctgcgccgcccaaagtagtcaccaataaacccaccagtaagtgagccgatgaaataaccaaacattaatgccgaggtaaaggcggcattgaggaaattatttgaccatccattgcttaccagctttgctaagacgacattaccggagtaactcaaaaaccctgttaataacagactaaagcttataataccaaatatacgataatgaaaccgggccaaaggcaagcggtccagtcttgcgccaatttgatcatattgttccattaggtgcctcggatttgctaaaaaggtagcaattgcggcaaattcacttgccgcatctttatcatcattttatttcaaggcgcaggaacaaataatattgacaacgtgtgcttaaattaccacaccagctggatattattgtctttgcaaaatgctatccactctgcacccggtgatttatcagttattatgtaattaatatgactaaaatcagctaactggacaaaagctttgcgatcaaacttagagtgatcaaccaataacgcaacttctgtcgcctgacggatcattgtctttttgatttcagcttccgcttcattagagtccagcgcgccgctgttaatatcaagacctttacaactcattaccatgatatcgacatgatagcgcctgatgatctctttagtaattcttccttgcagtgaaagtgtatttttgtttagttccccacccgttgaaacgactttaatttctgactgagccagaacatgaatcgcttccgccgagttggttagcaacgtcaggccactacggtcctgtaacaatttgagcaattccattacggtactactggaatcggctgccatggtggttttattgtcgataaagggtagtgccttgcgtgcaataagctgcttctcttcataaaacgatgaagcgcgcttataaaaatggatattctccgtcaacatcgctgtatttaaaacagcaccaccataggttctggtcaaaaagccttcatcttccagcttctcaagatcgcggcgaatggtttcttcggttacctgaaaaatcccactcaaatttgagactgtcacctttttatcgttggcaaccatttgcttaattgcctgaatcctgtcttttgccgccacgattacacccctgtatctttttacatcacattagcgcgattatcgcataaccgatgtttactttcaaaataacctgtttgaatcacagattttcatcacagttttcacagaaacagaggtgaatcgtgttgagtatttaacgctccagggcctctgccatttccctcatcaatgttgcgtctgcatccgataagttgatattcagtgccgcgacattttcgcgtacctgttccggtgcagtagccccactaagaatggagattaaatcactctgttttaatatccacgccagtgccagagtgggaattgtgcactgataacgagcacaaagtggctgccactgttcaagcatatcaatcactttcagcatgttttcacgctggaaccagactttatttgcccgagcgccgcccggaacgtaatcacgagtgatggtgccggtcaacaatccctgctctagcggggaataaacctgaaccacaatgccattatcacgacatagtggcagcagttcgttttccattgcccggtcgaggatactgtatttcgcctgaataatatccagttcaccatattgcagatactcgcggatatggtcagcatcgacgttagcagcgcctatagcgcgaattttcccttcagactttaactcattaagcactgcgacagtttcagcgatcggcgtaaaaaatggcggcaccgactgccagtgcgtcatgtagatatcgatgtaatcaatacccagacgttgcaagctcgctgctacctcttcgcggatagattccggggaaaggtttttatacaactgccgatcgccaactttgttgaataaacttccttttcgttcccagacaatgccgcatttggtttctactacaacctgttcacggggcagtttttttaacgcctgaccgacgataacttcactattgccaaagttatatcctggcgcagtatcaatcagattaatgccacaacgatgggcttcaagaatcgtatcaatacatatttgccgatcgagatcgccattccatgcaggaccgccgccaatggcccatgtccccaaccccattcgcgaaagcgtaatatccgttgtgcctaaaggtatctttttcatttgccttcattatccttcgtattcttccagcaattgttcgaccagctttctgttttttacgccggtggtggcaccgacgcttagaaccgagatagccgccgttgcattggcaaagcgtgcgcattcacgcagatttttgccttctaacagtgccgcaataaaacctgaagcaaagttatcgcccgcgccaatggtgtcgatggcggttattcctgcgaccgccggcaccttcatcgtcatgtcaccacgcttgataaagcagccgtctttacccgttttaatcaccaccgtttttacgccgcacgcaagaaagcagtcagcaatttcatccagtgtctctttcccggtgagtaattttgcctcggcaaaattaggaaacagataatcgacataactcaatgcttcgcaaatatcatccagcgtttcattcaaccgcggtttgatcatatcggcacagataatcatctgccgggctttagcttgcgtaaaaatttctgttagcgctttaccatccaatagtggactgttgaaaatactggccagtgataataatttcgcctgagaaaaccgcgcaaaatcaacatcgtcaatattcaatttccacagactgccattacggtttgtgacaaacgtccgctcgccatcctccgtcaccagtccaacgttaatagaggtatctatgctgacgtcctgcttcaggctttgaatatcaatattctctttgcggcaatggtcgagaataaattgccctgcggcatctttaccaatacgactcattaatgctgtgcgatggcccagacgagaaataattgttgcttcatttattgcatcacccccggtggtcattgcgattctttcaagaggataagaatccacatcaaagatatttttactgaccggttgcaatggaatatcaacaatagcggcacctatacaaataacgtcgagattatccatatcattattccgctttgccatcagaaccgaacagtttaattttttccaatgcccgttcttttacagctttacgtacttcacgttctaaatgcaggaaaggctgatcctggttttctttcactgcaaccattgcggcctgacagagctccgtatgaatgttgattttcgcgatacccaacgaaattgcagttttaatgtcggcatcactgatccccgatgcaccgtgcaaaaccagcggaacagaaacggcatcgcgtacgcgtttgacgacctcaaagttcaattgtggctctgacgtataaaccccatgctggttgccgatggcgacagccaatgaatcacagcccgtacgttcaacaaattcagccgcctggtcaggatcggtatagtgatagcccgccagcgcttcctcataaacggtttcattaccgacatgccctaattccgcctctaccggaatacccagcggatggaagaaatcgacagcctctttggttaaacgaatattttcttcgaaatcaaacgcggaagcatcacgcattaatgaattcataccatgagtccaggcgttatgaataatctccatactccgaccatgatcccaatgagttattaccggcaccgttgctttttgtgccattgataccatcatgtgagagaaatcttcaaatgaggtgttaccgacaaaacctgtaccaaaagaaataataaccggggatttcgcttcttcggctgcgtcgataacgcccatcaacatttctgcattccatacgttaaaatgggcaattgcataatgtttatttgtggcatcgttttcccaatatctgatatctgcgagcatgttctgttctcccgtattaattaatcgctaattttaataacgcctttaataatgtcgcgtttgttgttaactgactcttcaaatgcctgttgtacatcccgataatcgtaaatatgcgtcaccatcgatttcacatcgaatcgccctgaagaaatagcttcaatcgtgaccggataacgattggcatagcggaataccgtctggatagtgacttcgcgattgattttgaggaaattgattgccgaatcgccgggtacagtaccaacaatcataattttaccgccgcgcattaccagataaggtgcctgtttaacggtgaccgcagaacccgctgtttcgaaaacaatatctgcgcccatgtcttcggtaaattgctgacagcgtgcaatagtgtcttcttttgcgccgttaataaccactgtcgcaccaagctgttccgccattgccagacgtttttccagcacatcaacgacggcaatttccgttgctcccaggcatttgcacgcttgcaacgtcatcaaaccaatacaacctgctcccagaataattatcttcttacccggtttaacatctgccagcatcgcggcatgcatcccgactgcggcaggctccaccagcgccccttccatcgtgtccatattgtcgggcagtttgtaagtaaagctctccggatgacacagatagtgcgttaatgcgccgcggtagttgggttgtgtcgccataaaatcaacgtccgggcagatgttatatttgccttccagacagtaacgacagtgaccgcaaggaacgccaggttcgatatttacccgatcccccggtttaaatttgcgcacgcggcttcccacagccacaaccgtcccggcgcattcatgacccaggccaatttcttgatttgggtctttaggcggaataaacgggcctgattcaaaaccatgtacatctgaaccacaaataccgacatattctactttaatcaaaacttcatcttctttaggcactggtatttctgctgaaataattttcattgtgcccggcacctgcaatattgcttttgaatttttcattttgaatccacccgtattatttattggctactgcatcaatacttaaactttcaacggagacacctttggtttcgattccaatggtggcgatagcaattgcgacaataattgaaaccgcccccagaagaataaagactcccgtaacgccataactactgagcagcactgcaacggcataaggtgcggcaataccactgattcgccctaccgcattcgccagaccggagccacggagtttggcctctgtcggccagatttcagggacatacactgccgaggcatagcaaacgtacatatagacgaaagtaatcaggaagaaaccaatcaacgttatgagcaacatactggtttgcagtgaatagatatatccgagcaccgcaatcaggattaatagccccacacccattgttttacgcggaattttatccatcaccagcatggcaataaaaataccaaatggcgcgccaaacatactcatggtatttaaaacaatcgagtcttttaaattaatcccctgggtcatgaatattgttggcaaccagttaattagtgtgtactgcacaacgttcatggcaatcagcacacaagagcctaatatcacgcgtttcagtaatactcctgtcagtaaggctgaatacggcaccgcttgtggcgctttaccgtcatcagcaataaccacaggcggcaaaggtttacccgtctggcgtatgacgccttcttctatactccgcatgactttctcggcttcctgataccgtccgcgcgattccagccagcgcggggattcaggaaagtagcgccaggccagcgccgtagcgataagcgacaatattgcagggataagcagttgtacccgccagttccactctgcactaatcagcggcgtgagtcccatcgctatcaatgaacagagcggatatgaccagttgccaataaaggaaacccgacttgaccacgttccacgatttctaccgggcatatattcggtgaaaccagcaaacagcgtaaccagtaaagctcccagcccaactcccatcacaaaacggcaggcaataaggaaatccatattcggtgagaaagcaccgacaaccatcgaggcaatatgaatggcctcatagaggatgaacgcatttctgcgaccggttttgtcgccaatgatgccgcccaccagcgcaccgagaaacattccggcggtcgtgattgctgagaatgtggctgtggtggaattatctgtccagcccaacgctttcagctgcgcgaggatcaagccaccaacggcattactccagcagacaagcaagccaaacgcgacgatggcaaacattgatgaatgccagcggcaatccggtaagcgatccagccgtgcaccacaatgcggttttgttatctgttccatgcgataacgttccttcaggagagtggttattcatcaaagtcgtaagtcatgatcactttgattgcggttttatcgaccatcgcatcaaacccttcgcgccattgcgacaggccgatacgatgcgtgatcatcggtttgactttgatagcgccgctggctaatagcctgatagcgttacgccatgaggtggagtcataggccatatgcccaatgatgcttttgttccaggcggtaatgtcattaatcgagaaatcaagaggtttgaagcccattccaacgcgtaccacttccccgttcgggcggagcatttcgatggcttgtttcagtgcgatattggcaccggagcattcaatcaccagtcccagattgtctttgccacaaatttgctggcagcgcgccaccacatcttcggtagaaccatttactactgccgtcgcacccagttcttttgcaaccgggaagcggaccgccacatcttcttgcagaccaacgacgacgatatttaccgcccccataattcgcgccatttgtacggagaacagcccgagtgggccagtgccgatgacgaccacatcctgaccaggaaggaatttcgattgctgcgcgatggatttgtaggcattacagatagggtcaagtacggctgcgtcctcataatcaacaccatcagggatttcccacaacgcatgacgatgaattttgagaatttcaccaggaaccagacaatatttggaaaaaccaccgccccaggtattattatccagaccaaggtttactttttctgtacaacacagaaaatcaccttgttcacaggccggacaaacaccgcaaacgtgaccgctgttatccgatacgacgcgttgccccactttccagtctttgactttttcaccaacctgcgcaatacaacctgcgaactcatggccgcggatagagttaaactcatcagaaccgctatcgacattgtagtgcttcatgtctgcgccgcagattgccgcggctttaatttcaatcactacatcttccgggccacacatgggttgtgggacatcaatcatcttgtagccgccaaaggccttgccaaaccgagccagtgctttcattgcgtcatcctctgtgtttagttttgcttagatggccatcatacttacccacatgatttttgaggtcaacattaaatctgtaaaacacagataatgatctgcgttttacaactcagatcacaattacgcagaaaatggctgggtctgttacaggttgatggaaggcggggcgcaaaaagagcaaattcgagagggattaccggccaaataggtctgagacttaagttcaggagaagtcattcaggtgtgaacgggacggcaagagatcggactgggacttagccaggtcatggcgagataattgagatgagtcgtggggtcattgttggctatccccttcatagccgaggcaaaaaggggatgaaccacttacttaaacatggcaataggctttgctgagataccaaaatcttcttttaactgctgtttgctcttcatgaccatctgaccatttgtgtcaattgtcatatgctgtgcttcgatattatggcgggcttgccacagcatcaccagttgcaggcagttctctttttgttcctcggtcaacgcaacgccatcaggccatttccccagttcaacggcggtcgacaaacgctggtatacctcaggcatcatgctgttgataatgtcatcaagattcataatttttccgctcctgtggaataagttgctgaatcgttttttcaaccgttgatttcttcgccgttttcgccatcggtaaagcgtaaagaggcagagttaacacaataacgttcgcccgttggctgcggcccgtcggggaagacatgccccagatgggcatcacagttaccgcaacgaatttctatgcgctgcattccatgtgacaagtctttgatataacgaatggattcttcacttaccggttcgtagaaactgggccagccacagccggaatcatacttggtttgggaatgaaacagcggggcatcgcagatcaaacagtgatatacgccgtcacgcttgttatgcagtaaacgacccgtaaatggcggctctgtcccatgattctgcgtcacgtaaaactgcatctcggacaaattttttttcagttcttctgccgaaggtttattagccatttgctcacatctcactttaatcgtgctcacattacgtgactgattctaacaaaacattaacaccaactggcaaaattttgtcctaaacttgatctcgacgaaatggctgcacctaaatcgtgatgaaaatcacatttttatcgtaattgccctttaaaattcggggcgccgaccccatgtggtctcaagcccaaaggaagagtgaggcgagtcagtcgcgtaatgcttaggcacaggattgatttgtcgcaatgattgacacgattccgcttgacgctgcgtaaggtttttgtaattttacaggcaaccttttattcactaacaaatagctggtggaatatatgactatcaaagtaggtatcaacggttttggccgtatcggtcgcattgttttccgtgctgctcagaaacgttctgacatcgagatcgttgcaatcaacgacctgttagacgctgattacatggcatacatgctgaaatatgactccactcacggccgtttcgacggtaccgttgaagtgaaagacggtcatctgatcgttaacggtaaaaaaatccgtgttaccgctgaacgtgatccggctaacctgaaatgggacgaagttggtgttgacgttgtcgctgaagcaactggtctgttcctgactgacgaaactgctcgtaaacacatcaccgctggtgcgaagaaagtggttatgactggtccgtctaaagacaacactccgatgttcgttaaaggcgctaacttcgacaaatatgctggccaggacatcgtttccaacgcttcctgcaccaccaactgcctggctccgctggctaaagttatcaacgataacttcggcatcatcgaaggtctgatgaccaccgttcacgctactaccgctactcagaaaaccgttgatggcccgtctcacaaagactggcgcggcggccgcggcgcttcccagaacatcatcccgtcctctaccggtgctgctaaagctgtaggtaaagtactgccagaactgaatggcaaactgactggtatggcgttccgcgttccgaccccgaacgtatctgtagttgacctgaccgttcgtctggaaaaagctgcaacttacgagcagatcaaagctgccgttaaagctgctgctgaaggcgaaatgaaaggcgttctgggctacaccgaagatgacgtagtatctaccgatttcaacggcgaagtttgcacttccgtgttcgatgctaaagctggtatcgctctgaacgacaacttcgtgaaactggtatcctggtacgacaacgaaaccggttactccaacaaagttctggacctgatcgctcacatctccaaataagttgagatgacactgtgatctaaaaagagcgacttcggtcgctcttttttttacctgataaaatgaagttaaaggactgcgtcatgattaagaaaatttttgcccttccggtcatcgaacaaatctcccctgtcctctcccgtcgtaaactggatgaactggacctcattgtggtcgatcatccccaggtaaaagcctcttttgcattacagggcgcacaccttctctcgtggaaacctgcgggtgaagaagaagttctgtggttgagcaacaacacaccgttcaaaaatggcgtcgctattcgcggtggcgtaccggtttgctggccgtggtttggtccggcggcacaacaaggtctgcctgcgcacggttttgcccgcaacctgccgtggacgctgaaatcacatcatgaagatgctgatggcgtagcgctgacttttgaattgacgcaaagcgaagagacgaaaaaattctggccgcacgactttacgctgttagcgcatttccgcgtgggtaaaacttgtgaaatcgatcttgaatcacatggcgaatttgaaaccacctctgccctgcatacctactttaacgtgggtgatatcgctaaggtaagcgtcagtgggctgggcgatcgcttcattgataaagtgaatgacgcgaaagaaaatgtactgaccgatggtattcagaccttccctgaccgtaccgatcgcgtgtatctgaatccacaagattgcagcgtgattaatgatgaagcgctgaatcgtattatcgccgtaggccaccagcatcatctgaacgttgtcggctggaacccgggaccggcgctttcaattagcatgggcgatatgccggatgatggctacaaaacatttgtttgtgtagaaacggcttacgcttcagaaacgcaaaaagtgaccaaagagaaacctgcacatctggcgcaatccattcgcgttgcgaaacgttaatttacgttaatgttgtgtgccgggtgcaatgcatccggcacacaacatcacaccatatccagcgcagtttttccttttggtgccggatatgccttatccagcatagctaattccgctgaagaaagttcgacctcaagcacagccgcattttgttggacatgggcaatcgtggccgcttttggaatcgccatcacaccctgatgactgatcacccacgccaacaatacttgtgccgcgctgatattgtgagcatgtgcaatttcgttgactaccgcgttttttaacagtccattgcgcaaccgcccggcctgggctaacggactgtaagccatcaccggcatctgctgttgctggcaccaggggagtagatcgtactcaattcctcgtgaaccgagatggtaaagcacctgattagtggcacactgatttccccccggcagctgccagagttcctgcatatcagcataatcaaggttagaaacgccccagcggcggatttttccctgggcgatcaatttttccatcgctgcgacagtctcttcaaaagcgaaactgccagaccagtgtaataagtaaagatcgagataatcagtattgagacggcgtaaactggcttcgcatgcatttatcgctttttgcccgccagcattccacggatagactttagagacgagaaagaccttctctcgcagaccggttaatgcttccccaaccaccttttcggcaccgccatcggcatacatttcggcggtatcaatgagggttaaaccgagttcaatgcccgcgcgtagtgcagcaacttctgttttgcgctgactggcatcttcgcccatataccatgttccctgccctacggctggcagtgagacatcgccactaaattgaatcattttttgttgcattgtttcctcccaggtattgcaccaccgtaatgcaaaacagggcgtgacgccctgtttttatgcacaaaatgccctggaaagatgcattatcagaatttgtaggtgatcccggtagaaatcaggccagtccaggatttatccaccatcgggctgtcagtaacttcatcagacagacgggtgtagcgtgcggtaccgtaaacactccagtcgccgaggaagttgtagctggcgctcagctccaggtaagggctccagctgtcgttcgggttatagccacgcagaccgctgcgagcggactctttgcgcgatacgccataatagtattcgttctggttttcgctgttccactgcacaccaatacccggagtcacggtcaggccaccgttggtgtaacgatacaaccaggccatatcccagacgatgccgttgctgttatccagggtatcgccagccagggtggtacgcaggtaaccgtactgggtaaagtgagcataagacagaccagccatcatggtgctcttacggtcatccaggtgacgcatttggtgatcgccactgtctttcgctttgaagtaaagcggcgaccagtaagcggtaattgaaagtttatccgttgcgtcattccacaggtagtaaccaccacctaagccacggaaccagaagttatcgccttcatagttgattaccggtactgggtaaacatcggtatcgtaatctttatatgggtgttcaacgacacctacgcctgcgcccagggaaaatttaccttcagcgtgcgctacgcctgcagacgttgcgataagcactccaagtgccagaagtttgagtttggtcacaattaatcattccttaaacaaatgtttagcgggcgacaaagtttacccgtcaatacatcgaaacccaacctttttacgttttcattttttaaagtaactgtttaattttcctgacgcggatgacaccgcgcttacagccaaatgaatttagcgttactggcgagcctggtctttacattaattatgcaaaatttatggatgagttgttgatatgccattgaaattaagaaagccgtgcaggcaagttttccatttgccatctacgcttaattttgaaggtgtatcaccgggcacgttgttctcatcgtcgataaaatggcatgagagttgctgtgttttagcaagagacgtcgttcagtttacctcttccgggagcctctactattcatatgaacggctcttaacctgtgctaaaaaacgaaaggacggcataccatgaatatattcgatcactatcgccagcgatatgaagctgccaaggacgaagagttcacactgcaggagtttcttaccacttgtcggcaagatcgcagtgcttatgccaacgcggctgagcggctattgatggctatcggtgagcctgtcatggtcgatacagcccaggaacccagactttctcgactcttttctaaccgggtcattgcacgttatccggcgtttgaagagttttacggcatggaagacgcgattgaacagattgtctcttatctgaaacacgcggctcaggggctggaagagaagaaacaaatcctgtatctgctggggcctgtgggtgggggtaaatcatcgcttgctgagcgactgaaatcattaatgcagctcgtaccgatttatgtattgagcgcgaacggtgagcgtagcccggtcaacgatcatccgttctgtcttttcaatccgcaggaagatgcgcagattctggaaaaagagtatggcattcctcgccgttatctcggcaccatcatgtcgccgtgggcggcaaaacgcctgcatgaatttggtggcgatatcactaagttccgggtagtgaaggtctggccgtcaattctgcaacaaattgctatcgccaaaacggaacccggcgatgagaacaaccaggacatctccgcgctggttgggaaagtcgatattcgtaaactcgaacactacgcgcagaatgacccggacgcctacggctattccggtgcgctgtgccgcgccaatcaggggatcatggaattcgttgagatgtttaaagcaccgattaaagtgctgcatcccttgttaaccgccactcaggaaggtaactacaacgggacggaaggtatctccgccctgccgttcaacgggattattctcgcacactcgaacgagtccgaatgggtcactttccgtaataacaaaaacaacgaagccttcctcgatcgtgtttacatcgtgaaggtgccgtattgcttgcgcatttccgaagagatcaaaatctacgagaaattgcttaatcacagtgaattgactcacgccccatgcgcccctggcacgctcgaaacactgtcacgtttttccattctttcgcgcctgaaagagccagaaaactccagcatttattcaaagatgcgggtttatgatggcgaaagtctgaaagacaccgatcccaaagccaagtcgtatcaggaatatcgtgactacgccggtgtcgatgaagggatgaacggtctgtcgacgcgttttgcgtttaagatcctctcccgcgtgttcaacttcgatcatgtagaagtggcagcaaacccggtccatctgttctacgtcctggaacagcagattgagcgcgagcagttcccacaagagcaggcagaacgctatctggagttcctgaaaggttatctgatcccgaaatatgccgagtttatcggcaaagagatccagacggcctaccttgaatcctattccgaatatgggcaaaacattttcgaccgttatgttacctacgcggatttctggattcaggatcaggagtatcgcgatccggataccgggcagctgtttgaccgcgagtctcttaacgccgagctggagaaaatcgagaaaccggcggggatcagtaatccaaaagatttccgcaacgagattgttaacttcgtactgcgcgccagagcgaataacagcggacgcaatccgaactggaccagctatgaaaaactgcgcacggtcatcgagaagaaaatgttctccaataccgaggagctgttgccggttatctcgtttaacgccaaaacgtcaaccgacgagcagaagaaacacgacgactttgtcgaccgtatgatggaaaaaggctacacccgtaaacaggtgcgtttactgtgcgaatggtatttgcgcgtacgtaaatcgtcttaacaaccctggcccggtacacatgttaccgggcctacaacgacagcgaaccgtgggcctgagaagcggcaacacaggcgtagcatacagttggcaaatgtagtacggggggcatatgacctggtttattgaccggcgtctgaacggcaaaaacaaaagcatggtgaatcgccagcgttttttacgccgttataaagcgcaaattaaacagtcgatctccgaggccattaataagcgttcggtgactgacgtcgacagcggcgaatccgtatccattcccacggaagatattagcgaaccgatgtttcatcaggggcgtggcggtctgcgccaccgcgtgcatccgggcaatgaccatttcgtccagaacgaccgaattgaacgtccccagggtggcggcggaggttccggcagtggtcagggccaggccagccaggatggtgaaggtcaggatgaatttgtctttcagatttcgaaagatgagtatcttgatctgctctttgaagatttggccttaccgaatctgaaacaaaaccaacaacgccagctgaccgaatataaaacgcatcgggcgggttataccgctaacggcgttccggccaatatcagcgttgtgcgttcattgcagaactcactggcgcgacgcacagccatgacggcaggcaagcggcgggaacttcatgcactggaagagaatttggccatcatcagcaacagtgaacctgcgcaactgctggaagaggaacgtctgcgcaaagaaattgcagaattacgtgccaaaattgaacgcgtcccttttattgacaccttcgatttacgttacaagaactacgagaagcggcccgatccctccagccaggcagtgatgttttgcctgatggacgtttccggttcaatggatcaatccactaaagatatggctaagcgtttttatattctgctgtatctgttcctcagcagaacgtataagaacgtggaagtcgtatacatccgccatcatacccaggcgaaagaagtcgatgaacatgagtttttctactcgcaggaaacaggcggcaccattgtttccagcgccctgaaactgatggatgaggtagtgaaagagcgttataacccggcacagtggaatatttacgctgcacaagcatcggacggcgataactgggccgatgactctccgctttgccatgaaatcctggcgaaaaaattattacctgttgttcgttattacagctatatcgaaattacccgtcgtgcacatcagacattgtggcgagaatatgagcatctgcaatctactttcgacaactttgcgatgcagcacatccgcgaccaggatgatatttatccggtgttccgtgaactgtttcataaacaaaatgcaacagctaaaggctaaaactatcagccaggtcattatcgcctggctgatttttagcttactgtaaattatctcatttattacatacattagcttacaatcgctttaaatatgacagcataacctttacataatttagttccagaaaacaatcattcggaaaaatgattcagtcaacacgtatttccatggggttattctttaaatattttttatcgttaacgaaaattgatcctggtcaaaactatatatctctgccatcaataaaatccagcactcacattgctctcctttttatggtttctatgggtacacaaaaattaaaagctcaaagcttttttattttcagtttattgctgacgttaattttattttgcattactaccttatataacgaaaacacaaatgtaaaactcatcccacagatgaattacctgatggttgttgtggctttgtttttccttaacgccgtcatttttcttttcatgttaatgaaatatttcactaacaaacaaattttaccaacactcattttaagccttgcatttttaagtggccttatctatttagttgaaaccattgtaattatccataaaccaattaacggcagtacactgatccagacaaagtcgaatgatgtttctattttctatattttccgccaactcagttttatttgtttaacctcgctggcgctcttttgttatggaaaagacaacatccttgacaacaataagaaaaaaacgggaatcctgttgctggcgctgatcccttttttagtttttccccttctggcacacaatctgagcagttataacgctgactattctttgtatgtcgtcgattactgtccggacaaccatactgcgacctggggaatcaactatacaaaaatattggtttgtctgtgggcatttttactgttctttattatcatgcgcacacgattagccagcgaactatggccgttaatagcattattatgtctggcatcgctatgctgcaacttacttctactgactctggatgagtataattatactatctggtatatcagtcgcgggattgaagtttccagtaaactgtttgttgtgtcttttctgatttataacatttttcaggagctgcaactctccagcaaactggcagttcatgatgtgctgaccaatatttataatcggcgctactttttcaacagcgtagagtcattattgtcgcgacctgttgttaaggacttctgtgtcatgctggttgatattaatcagttcaaacgcatcaatgcccaatggggacatcgtgtgggtgataaagtgctggtttcaattgtcgatattatccagcaaagcatccgccccgatgatattttagcgcgactggagggtgaggtgtttggcttgctatttaccgaactcaatagtgcccaggcaaaaatcattgcggaacgtatgcgtaaaaatgtcgaactcctgaccggctttagtaacagatatgatgttcctgaacaaatgaccatcagtattggcacggttttttcaacgggtgacacgcgtaatatctcgcttgtcatgacggaagcagataaagccttacgcgaagcgaaaagcgaggggggcaacaaagtgattattcatcatatttaagtgcaaaaatattcagagccatgctttttgcgtggcttttgcatacaatttattactattacccctaaatttcccctccccagcggcgcagagatgagtataattagcgcccctgtgccaggccgcaatcgaactttatctggttttctcgtttcactaaccgaaggagtgccatttatcatgaaattgcaccatagaatgctccggcattttatcgccgcaagtgtcattgtgctgacatcttccttccttatttttgaacttgtcgccagcgacagagcaatgagtgcctatctgcgctatatcgtgcagaaagcagactcctcctttctttatgataagtatcagaatcagagtattgccgcgcatgtgatgcgcgctctcgctgctgagcagtcggaagtgtcgccagaacagcggcgcgccatctgcgaggcttttgagtctgccaataacacccatggcttaaacctgactgcccataaatacccgggcttacgcggcacactacaaaccgcatccactgactgcgacacaattgtggaagctgcagcactattacccgcttttgatcaggcagtggaaggcaaccgccaccaggatgattacggttcaggtcttgggatggccgaagagaaatttcactattatctcgatctcaatgaccgctatgtctatttttatgagccggttaatgttgaatactttgcgatgaataactggtccttcctgcagtcaggaagtattggcatcgatcgcaaagatattgaaaaggtatttaccgggcgtaccgtattgtcgagcatttaccaggatcagcgtactaaacagaacgtgatgagtttgctgacgccggtatatgtcgcagggcagctaaaagggattgtgctgctggatattaacaaaaacaatctgcggaatatcttttatactcatgaccgccctctcctctggcgttttctcaatgtcacgctaaccgataccgattcggggcgcgacattatcatcaaccagagcgaagataatctgttccagtatgtcagttacgtccatgacttaccgggcggcattcgtgtctcgttatccattgatattctttactttatcacgtcttcgtggaaaagcgttctgttctggattttgacggcgttaattttgctgaatatggtgcggatgcacttccgtttataccaaaatgtgtcgcgagaaaatattagtgatgcgatgactggactgtataatcgcaaaattttaacccctgaactggagcagcggttgcagaaactggtgcaatccggttcttcggtgatgtttattgctattgacatggacaagttaaagcaaataaatgacaccctcggtcatcaggagggggatttagcgattacgttattagctcaggcgattaaacagtcgattcgtaaaagtgattatgccatccgactcggtggcgatgaattctgcatcattcttgtcgattcgacgccgcaaattgcagcacaactgcctgaacgtatcgaaaaacgtctgcaacatatcgcgccgcagaaagagatcggcttctcttccggtatttacgcgatgaaagaaaacgatacgttacatgatgcgtataaagcttccgatgagcgtttatatgtcaataagcagaacaaaaacagccgttcatgataaccttctgtggttgtttgcttgtaatctcaggagcgtgaaatgactgaaatggctaaaggaagcgtgacgcatcagcggttaatcgctttattatcacaagaaggtgctgacttccgcgtcgttacccatgaagcggtaggtaaatgtgaagcggtgtcagaaattcgtggcaccgctctaggccagggtgctaaggcactggtatgtaaagtcaaaggcaatggcgtaaatcaacatgttctggcgatcctcgcagccgatcaacaggccgatctgagccaactcgccagccatataggcggattacgcgcttcgttggccagcccggcggaagtcgatgaactcacaggctgtgtcttcggcgcgatcccccctttcagcttccatccaaaactcaaactggttgccgaccctctactcttcgaacgatttgatgaaatcgccttcaatgcaggcatgctggataaatccgttattttgaaaaccgcggattatttgcgcattgcgcaaccagaactggtcaatttccgccgcactgcgtaactagccggtccgttcgataagaagaacggacaaaaccagtacaacagcaatggcaaaaaacgatgacgtgataatcagtgtctcgacaaacatttgatcgttcatagcatgcccccgggagatagctgttttcacgttattgttagcgtgcacaaatggcagtttgatgacagttcgcctgattttttatgcaaaaaacgtaaagattttctacttccttcctgcagcaagcgtaaagtaagcaggcttattattttttggcaaggaaaccacgatgtttgatgtcactttgctgatcctgctcgggttagctgcgctgggctttatcagtcataacaccactgtcgccgtttcaattctggtgttaatcattgtccgcgtcacaccgttaagcaccttttttccgtggattgaaaaacaggggctaagtatcgggataatcattctgacgattggcgttatggcccccatcgccagcgggacgctaccgccctcaaccttgattcactcgtttctgaactggaaatcactggtggcgattgcagtaggcgtgattgtctcctggctgggtgggcgcggcgtgacgttaatgggcagccagccgcaactggtcgccgggctgctggtaggcactgttttaggcgtagcgctgtttcgcggcgtaccggttgggccgcttattgccgcgggtctggtttcgctgattgtggggaaacagtagttaatctcgcaatatatcggcctggcgtttgccccaggcctttcttaaacatagtaataaaggccgttgttgaatcataccccagcgtatgagcaactttctgtacagtatcgcctttcactaatccctgaagcgccataatcagctgtaactgctgacgccactggcgaaaactcaaccccgtctcttttactatcagtcgggcaagattgcgttcactcatcgcaaaaaagccagcccattgccccaatgccccccactcgacaggccctttcgccatcatctccaccatcgtgcggattttaggatgagaagaaacgggcaggtgcagctgttgttgtggctgctgagggagttcatcaaacaggacctgaattaatctgcgggtcattggctcagcacgctgagtcgtcgtcctgtttgccagggttaaaattaattcccggcataagggcgatattttcaatgtgcaacatgttgtcggcattgtcactgcgctgggttcgataaacagaaaacagagttcagcattagctgttacttgattgctatgttccaccccgcccggtatccaaaccgcatattgtggcggcaccatccacaaagcattttccaccgtacaggtaattgcaccatgtagcgccagtatcagctgtcctttgcggtgctgatgtacaggactggttaactcatccgttccggcgtgaatacaaaatgcgaccgcggcttcatggtgtcggtcgggttcatagccattgagattcaacctgtgcatcattttgtccgaacttagcgataatttgtcattttagcttgattcaacataacaataaaaacggtaaggtacagcctcgtttgtaacaatgagaagcatatgacctgttcaacttcattaagcggcaaaaacaggattgtccttatcgctggcattctgatgattgccacaacattacgcgtcacctttaccggcgcagcaccgttactggatacgattcgttccgcttactcgctgacgacagcgcaaaccggcttattgaccaccctgccattattggcctttgcgctaatctcacctttggctgccccggtagcgcgacgttttggtatggaacgtagcctgtttgccgcgttacttttgatctgtgctggtatcgcaattcgctctctcccttcgccttacttattatttggcggtacagcggtcattggcggtgggattgcattaggcaatgtcttactgccaggattaattaaacgcgatttccctcattccgtcgccagacttaccggcgcatattccctgacaatgggagctgcagcggcactgggatcggctatggtcgtgccgctggctttgaacggttttggctggcaaggcgcgttgctcatgctgatgtgttttcctctgctggctctttttttatggctgccacagtggcgaagtcaacaacatgcaaatttgagtacctcgcgcgccttacatactcggggtatctggcgttcaccgcttgcctggcaggtcacattgtttcttgggatcaactcactggtctattacgtgattattggctggcttccggcgatcctcatcagtcacggctatagcgaagcacaggcgggttcactgcatggtttgctgcaactagccacagcagcacccggtttgctgatcccacttttcttacatcatgtgaaagatcagcgtggtattgcagcgttcgttgccttgatgtgcgcagtgggcgcggttgggctctgctttatgccagcgcacgcgatcacctggactctgcttttcggttttggttccggcgcaacaatgatactggggttgacgttcattggtctgcgggctagttctgcgcatcaggcggcggcactctcggggatggcacaatccgtcgggtatttgttggcagcctgtgggccgccgctgatgggtaaaatacacgatgctaacggtaactggtctgtaccacttatgggtgttgccatactttcactactgatggcgattttcggactttgcgccgggagagacaaagaaattcgctaatatccggtgctatagtgacgtaacaaatcatgcgtgaaagggagaacaaacacgatgaatattcagtgcaaacgcgtttatgatccggctgaacagagcgatggttatcgcatactggtcgaccgcctctggccgcgcggtatcaaaaaaaccgatttagcccttgatgagtgggataaagaaatcacgccgtcaacggaactgcgcaaagcctttcacggcgaagtcgtcgattatgcaacctttcgcgagcaatatcttgcagaactggcgcaacacgagcaagaaggaaagcggctggcggacatcgccaaaaaacagccgctgaccctgctctactcagcaaaaaacaccacgcagaaccatgcgctggtgctggccgactggctacgtagcttgtgattttagtacagcatccggcggttatttttcaccagccggatggtcacgccgccacaatgcccattcatcaatcgtttcaccgcccggtaatttgcaattgttgctgaccccttgcgctgtctgcactggaatgagcgtcccgcccttctgctggcaatagaccgacgccggatttgccataccaatctgcggcggtttaggtgcttctggctgagaaggggttgaacaaccagccaggaccagcaagcaaggcagaacaaaactgataattttcatttattgatctcacatatttatccaagattagagtatcgcggtatcgttttgttttgcagcactatttttattacattcactcaaaacatattacgtcttgtttcatctttgttgatgatgttttatcatgcctgcaaagattaaataatcagcatttacccgccgtatcctggagttgttccgtgtcagatcagattatcgcccgcgtctcgcaatcccttgccaaagaacagtcactggaaagtctggtccgacagcttctggagatgctggaaatggtcactgatatggaatcaacctacctgaccaaagtggatgtcgaagcgcgcctgcagcatattatgtttgcccgtaacagccagaaaatgtacatcccggagaattttaccgtctcgtgggattactcgttatgcaaacgcgccattgatgaaaactgctttttcagcgatgaagtccccgaccgttggggtgactgtattgcggcacgcaatcttggcatcaccacatttctgagcacgccaattcacttaccggatggatcattctatggcacgctttgcgccgccagcagtgagaagcgccagtggagtgaacgcgcggaacaggttttacagttattcgccggactgattgcacaatatattcaaaaagaggcactggttgaacagctgcgcgaagccaatgctgcgctgattgcgcaatcgtataccgactcgttaaccgggctaccgaatcggcgggcgatttttgaaaatctgacgacactgttttccctcgcccggcatcttaaccataagataatgatcgcgtttatcgatctggataacttcaaattaatcaatgatcgttttggtcataatagtggcgatctgtttctcattcaggttggcgagcgccttaatacgctccagcaaaatggcgaagttattggtcgtctcggcggtgatgagtttttagttgtttcactaaacaacgagaatgcggatatttcgtcgctgcgagaacgcattcagcagcaaatacgtggagaatatcacttaggtgatgttgatttgtattatcccggtgccagtcttggcatagtagaagtcgatcctgaaacaaccgatgcagacagtgccctgcatgctgccgatattgcgatgtatcaggagaaaaaacacaaacagaaaacaccttttgtcgcgcatccagcgctacattcctgaggcgtattcacatccttttgattggtgataacatgcgaatcggtattatttttccggttgtaatcttcattacagcggtcgtatttttagcatggttttttattggcggctatgctgccccgggagcataaagatgaaaaaaacaacgattattatgatgggtgtggcgattattgtcgtactcggcactgagctgggatggtggtaacgtcacctctaaaaaatagcaaaggctgcctgtgtgcagcctttgtgcaatttaagcgttaacttttaatcttcctgtagataaatagcacgacaatcgcaccaataacggcaaccacgaagctgccaaaattgaagccatcgactttaccaaagccaaacagcgtgctgatccatccgccgactacggcaccgactatccccagcaggatagtcataaagaatccacctccatctttacctggcatgatccacttcgccagaataccggcaataagcccaaaaataatccatgacagaatgcccattgtttcctcacttatctgttttgcattagcgggttagtcgctgataaaaagcatagcacaacatcgggagggcaagatttgtgacgagcatcacggaggttttttttgcgatggcgcagaaattgcgccatcaacgatcagtgataattaccaaccacaaacatcatgttcgttttccgtgtcataagaacgtacggtattcaccagatcttttatcacttcagccgccacttctggcaccagcaaagtcatcggcgtctctgtttcataatcgacagaaacgccattgctgttattggtgacggtcacggtatacgttgctttgcccatgattcatttcccgttatgaatgactttccgttgttgcgcaccttccatcaggacttcaggagccacgaagaagtcaatgttgaaataagtatcgtcagtcatggcttcaatgttgtgccacttttctggagggaacaccgcaaactgccccgcttcgataaggatcacctgatcaggctctgcactgtgttcatcagcgtagccgagatatttgaccgccccatgcataacggaaaggcgtgggtaaacccccgggcgcgttcctttatcaagatgacgttcgaatattccggcaggtgcagtttgtttattccagaaaggcgttgagcgcgtatgaatataattctgtgggatttgaagcatccttttccctccttcggtgaatgcgctgaaaacggtttattccagccgtttcagggtacgcctgataatttgcattttaaataccatttattggttactttttagcaccatatcagcgaagaatcagggaggattatagatgggaagcccgcgacaacgcgggctgaaagcatcaggattgcagcgtcgccagtcgggcagcgaaacccacgaacatcaaaccaatcagtgagttgccaactttagccagtttctttttggtacgtatgtactgcgtgacaaaagcaccagatataatcaggaagctcaaatagcagaaactcaccagttccagcgtcgccgccagaataaagaatgaaattcccgtatgtggggcattaacatcgataaactgtacgaaaaacgacacatagaacaaaatggctttcggattagtcaggctcaaaattaacgcgcgtttaaaaatagcaccgtattggggctcatcggatttggcctcgctatttttacccttcagggtcgcgtaaagaattttactccccagatagagcaaataaaacgcaccaagataacgtacaatgttgaataatatcggggtggtcttaattaatgtcgccactccagcccatgccagaaacatcaataccgcatcgccaataaatacaccgcaggccgcaagataaccgcctttcataccgctactgacgctatttttgagtacaaacagggtatttggccctggcaccaacacaataaaaatggccccaaccagataggtccagtaattcagaaccccgtattcagcgaacacattaacctctttaattatctttcgatcatgcgcgattaaaggtgaatatgctaaccaatctgtagcggcttagaaaggagaaaatcaggttttaacctgatatcaacccgataattgaatcattaatcaggcatgctccagtgaaaaattcgggtagtgctcggcaaaatactggcgtaaaaattctaccgttatccgcactttcgctgacgtcgccagccttgaaacataaacggcccagacgttcgctggctggtaatattccggtagcacttgcactaaatgaccactggcaatgttttcgctaacatcccaccaggaacgcagagcaatcccctgcccatcgagacaccactgatggacaatttctccatgattagacgacagtgggccggtgactttaatcgcatgggggccttctttattgcgtaattgccagacaccaaaaggatgatcgcgctctttaatgaccaggcacggcaatgcagaaagatcggttaaatgtttcggcgcgccatgttgcgcaataaattccggcgacgcgcagagaatacggtaattggtcgccagtttgcgggcgattaaattaggggcgatgtcatcgccaatgcgaatatcgagatcgacaccttcattgaccaaatcgaccagtcggtcttccacatcaaaacgtaattccagttgcggatacgccttcgccagcgctaataacgccggagccaccacctgtcgtccaaaaccaaagctgctgataatacgcagcatcccctgcggcacctgacgcacgtcagaaagttcgtccatcatctgaccgacatcctgcaaaatccgctgcgcccattcataaatccgctctccttcttcggtaatggtgacgcggcgggtggtgcggtgtaacaacaccacgtttagcgtttgctccagcaaggcgatgcgcttgctgacgaacgccggtgaaacgcccagttcttccgccacggcggcaaaaccagcccggcgagccaccagcataaagacgcgcaaatcattcagcagcggtaaattattcatgattcgtgttttatgtttcaccagttacggggattaattccttttcagtcaattataggatggtgatgttgtcaattttgatggtcaggaagtgagaacccaatgatgaaaacgatgcgtattgctgcgatcccgggagacgggattggcaaagaagtccttcctgaagggattcgcgtgttacaggctgccgctgagcgctggggcttcgccttgagttttgagcaaatggagtgggcgagctgcgagtattacagccatcacggtaaaatgatgccggacgactggcatgagcaacttagccgtttcgacgccatctattttggtgccgtcggctggccggataccgttccggaccatatttcgttgtggggttcgctgctgaaatttcgtcgtgaattcgaccagtacgtcaacctgcgcccggttcgtctctttcctggcgttccctgcccgctggcgggaaaacagcctggcgacatcgatttttacgtggtcagggaaaacaccgaaggcgaatattcctcgctcggcggtagagtgaatgaaggtacagagcatgaagtcgtcattcaggaatcggtatttacccgccgtggtgtcgatcgcattttgcgttatgccttcgaacttgcgcaaagccgtccacgtaagacactaacttctgccactaaatcgaacggtttagccatcagcatgccgtactgggatgagcgagtggaagcaatggccgagaattacccggagatccgctgggacaagcagcatattgatattctctgcgcgcgttttgtgatgcagccggaacgattcgatgtggtggtggcgtccaatttgtttggcgatatcctttccgatcttggcccggcctgcaccggcaccattggcattgccccatccgccaacctgaatccggaacgcactttcccgtcgctcttcgagcctgtccacggttccgcgccggatatctacgggaaaaatattgctaaccctatcgccacgatttgggccggggcaatgatgctcgattttctcggcaatggcgatgagcgtttccagcaagcgcataacggtattctggcagcaattgaagaagtgattgctcacgggccgaaaacacctgatatgaaaggcaatgccaccacgccacaggttgccgacgcgatttgcaaaattattttgcgttaaggtcaaaccagtttatttgaaccgcgtcactgacgcggtttttttattcgttctttgcagtaaataacctgcgtcatttcaccttttattgtttccgtttcgtgttttatggctttccgtattcttaattgtttaatttatgtaacatgcaaattttgttacgcgtacgttaggttccgccgtacaggtattggttttgctggcaatgggactggtgatttatttagccaccagtaaatacggcaatattcgtcttggcgaaggaaaaccggaatacagcacgctctcctggctgtttatgtttatttgtgccggtttaggttcttctacgctttattggggggttgctgaatgggcctattattatcaaacacctggattaaatatcgcaccgcgttcacaacaggcactcgaatttagcgttccctactctttcttccactggggcatcagcgcctgggcaacttatacgctggcctcattaatcatggcttatcactttcatgtgcggaaaaacaaaggtctgagcctttccggcattattgctgctattaccggcgttcgcccgcaaggcccatggggaaaactggtcgatttgatgttcctgatcgccactgtcggcgcactgaccatttcccttgttgttaccgcagcaacctttacccgtgggctttccgcgctgaccggtttacccgataacttcaccgtgcaggcatttgtgatcctgctttccggcggcattttttgcctaagctcgtggattggtatcaacaacggtttgcaacgtctgagcaaaatggttggctggggcgcgttcctgctgccattactggtgctgattgtcggcccaaccgaatttattaccaacagcatcatcaatgccatcggcctgaccacgcaaaacttcctgcaaatgagcttattcaccgatccgcttggcgatggttcatttacccgcaactggaccgttttctactggctgtggtggatctcatacacccctggcgtagcaatgtttgtcacccgcgtttcccgcggtcgtaagattaaagaagttatctggggactgatcctcggcagcaccgtcggttgctggttcttctttggcgtaatggaaagctatgccattcatcagtttatcaatggcgtaatcaacgtcccacaggtgctggaaacactgggcggcgaaacagctgtacagcaagttctgatgtcgttgccagccggtaaattgttcctcgccgcatacctgggcgtgatgattattttccttgcctcgcatatggatgcagtggcctacaccatggcggcgaccagtacgcgtaatctccaggaaggtgacgatcctgaccgtgggctgcgtcttttctggtgcgtggtgatcactctgatcccgctttccatcttgtttaccggtgcttcgctggaaacgatgaaaaccaccgtcgtgctcacagcccttcccttcctcgtcattttactggtgaaagtcggcgggtttattcgctggctgaaacaggattacgccgacattccggctcatcaagttgaacattatctcccgcagacaccggttgaagccctggaaaaaacgccagtgctccctgcgggaaccgtattcaaaggcgacaactgagcgccatcatcctaacgataaaggtatccctatgagcaatctgagccctgactttgtactacccgaaaatttttgcgctaacccgcaagaggcgtggaccattcctgcccgtttttataccgatcagaacgcgtttgaacacgaaaaagagaacgtcttcgccaaaagctggatttgcgtcgctcacagcagcgaactggcgaatgccaatgattatgtgacgcgtgagatcattggcgaaagcatcgtgctggtacgcggtcgtgataaggttttgcgcgcgttctataacgtgtgtccgcaccgtggtcatcagttgttgagcggtgaaggaaaagcaaaaaatgtgattacctgcccgtatcacgcatgggcattcaaactcgatggcaacctggcccatgcacgtaactgcgaaaacgtcgccaatttcgatagcgacaaagcgcaactggttccggtgcgtctggaagaatatgccggattcgtcttcatcaacatggaccccaacgccaccagcgtagaagatcaattacccggcctgggcgcgaaagtgctggaagcctgcccggaagtccacgatctgaaactggcggcccgctttaccacccgcacgcctgccaactggaagaacattgtcgataactatctcgagtgctatcactgtggtccggcgcatccaggtttctccgactccgtacaggttgatcgttactggcacaccatgcacggtaactggacgctgcaatacggtttcgccaaaccgtccgaacagtcgtttaaatttgaagagggtacggatgcggcattccacggtttctggctgtggccgtgcacgatgctgaacgtcaccccgatcaaagggatgatgacggtcatttatgaattcccggtggattctgaaactaccctgcaaaactacgatatttacttcaccaatgaagagttaaccgacgagcaaaaatcgctgattgagtggtatcgcgatgtgttccgtccggaagatttacgtctggttgaaagcgtacagaaagggctgaaatcgcgtggctatcgtggtcaggggcgcatcatggccgacagtagcggtagtggcatttccgaacatggtatcgcccatttccataatctgctggcgcaggtgtttaaggactaatgacatcggcggcggtattttccgccgctgggctgatttttgatggagtacagcaatgtcagactatcaaatgtttgaagtacaggtgagccaggttgaaccccttaccgaacaggtgaaacgcttcacgctggtggcaaccgatggcaaaccattacctgcgtttaccggaggaagtcacgtcattgtgcagatgagcgatggtgataaccagtacagcaatgcgtattcactactgagttcgccgcatgacacctcttgttatcagattgccgttcggctggaggaaaactcgcgcggcggttcccgctttttgcatcagcaggtaaaagtgggcgatcggttaacgatttcaacgcctaataacctgtttgcgctaattccctcagccagaaagcatctgtttatcgcgggcggtattggtatcacccctttcctgtcgcacatggcagagctgcaacacagcgacgtcgactggcagctacattactgctcgcgaaatccagaaagttgcgcatttcgtgatgagctagtccagcatccgcaggctgagaaagtccatttgcatcattcatcaaccggaacacgactggaattagcgcgattattggcggatatcgaacctggcacacacgtttatacctgtggccccgaggcgctaattgaagcggtaagaagtgaagctgcgcgtctggacatcgccgccgatacgctgcactttgagcaatttgctatcgaagacaaaaccggcgatgcatttaccctggtgcttgcccgttccggaaaagagtttgtggtgccggaagagatgactattttgcaggttattgaaaataataaagccgcgaaagtggaatgtttatgtcgtgaaggggtatgcggaacctgcgaaacagcaatactggaaggtgaagctgaccatcgggatcaatattttagcgatgaagagcgtgccagccagcaaagtatgttgatctgttgttcgcgtgcgaagggtaaacgcctggtgttggatttgtagtttgccgaagccggatgtggcgctgagcgcgcccagtccggcttcggaagattttactgcggatattcctgcaataaattgtgtaatgcttccgccatcagctcaccacgccagccggaaatcagctccggcaaattgttctgcggtttcagtttccagtgccagttcagcagttggttgatttgccgacgcgatgccagcaattcggcgctgatcttatgcgtttcgctcacgtcagtaatcagcgacttaatcgctttaaacgctttacgataacccggcatgtccatcaggttaagcatcggctgcggtaaggcatcttccggcaatgtctgcgctttttccaccagcgctagcagcgttttaccgtgaaagcggatttcgctaccggataaacccaggctgtccagttcgcctaaacttcccggcatataacgcgctaccgaccacaaatgctcttcacgcacgacaaagttcaccgccagatcgcgctctcgcgccttgcgcagtcgccagtcggctaacagttgcagacaggccagttggcgtgtgcgtaattgccaggcattggtgatatcacgccaggcatcttccggcgcaacgacttcctgacgacgcatttgcatcaggcggcattcatccagcgccgcaggtagccagccggaggcctccgtttctaccataagcttggcggtgatcggtaacagataccagacatccgccgctgcgtattcacactgacgttcggtcagcggtctggccagccagtcggtgcgcgattcactcttgtccagcgtaacgccggaatactcttccaccatggaagcgaaaccccatgacatcgggcgtccgcagaaggcagcaaggatttgcgtgtcaatcaagggttgtggtaattcgccaaagacattgaggaacacttccagatcttcactgcctgcatggagaaattttgtgatggacggatcgcgcaggatcgctttcagcggtgaccagtcggtgatcccgagtggatcgattagcgccagatgctcgccatcgaaaagttgaatcaaccccagctgcgggtaataagtgcgcgtacgaacaaattcagtatccagggctatcgccggaaaggcacggacggcttcacacaaagaagccagcgcatcgtccgtggtaatcatttggtaattcaaattgttttctctttagtgggcgtcaaaaaaaacgccggattaaccggcgtctgacgactgacttaacgctcaggctttattgtccactttgccgcgcgcttcgtcacgtaattctcgtcgcaaaatttttccgacgttagatttcggtaactcatcacgaaactccaccagcttcggtactttgtatcccgtgagctgacggcggcaaaaagtcaccagtgactcttcggtaagcgatggatcttttttcactacgaagattttcaccgcttcaccactggagccggaaggtacgccaacagccgcgacttcctgtacgccaggatgctgcatgacgacatcttcaatctcgttgggatagacgttaaaaccggaaaccagaatcatgtcttttttacgatcgacaatgcgcaggaatccttcttcatccattaccgcgatgtcgccggtgtgtaaccagccatttttgatgatttcatcggtagcatcgggacgctgccagtaacccagcatcacctgcggtcctttgacacaaagctcacccggttgacctggtggtacttcattatcatcatcatccaccagtttggcttccgtcgacggcaccggcaaaccgatgctaccactatgataatcaatatcatatgggttaacgctgaccagcggcgcacactcggtaaggccatagccttccagcagatactgtccggtcagtttcacccaacgctctgccaccacttgctgcactggcatcccaccgcctgcggaaagatgcagactggagaaatccagctgctggaactctttattgttcagcaacgcattgaacaaggtgttaacgcccgtgatagcggtaaacggatatttcgctaactcttttaccaaccctggaatatcgcgcgggttagtgataagcaggttctgcccacccagttcgataaacagcaggcagttaatggtcagggcaaaaatgtgatacagcggcagcgccgtcaccaccagctctttgcccggatgcaacagcggaccataggtcgcgttaacctgttccaggttcgccagcatattgcggtgagtcagcatcgcgcctttcgccacaccagtggtgccgccggtgtattgcagaaaagctaaatcttccggcaccagttcgggtttgacgtactgcatccggtagccgttatgcagtgcgctacgaaatgaaatggcatctggcagatggtatttcggcaccaaacgcttgatgtatttaacaacgaaattgactaccgtgccttttgccgtagatagctgatcgcccatacgggtcagaattacgtgctgaacggcggttttatcaaccactttttccagtgtgtgagcaaagttagacacgataacaatcgccgatgcgccgctatcgttaagctgatgctcaagctcacgcggggtatacaacgggttaacgtttacgacgatcatcccggcacgcaaaatgccaaacagcgccaccggatattgcaataaattaggcatcatcaacgcaacgcgatcgcctttcttcagccccaacccttgttgcaaataagcggcaaacgcgcgactgcgttcttccagcttgcggaaggtcattacctcccccatattcacaaacgcaggttgatcggcgtagcgcgcgaccgactgctcaaacatatctaccagagattgataacggtcagggttgatctccgtcggaacgtccgcgggataacggttaagccaaaccttcttcaattcttcacctctaaaatgcgtgttcgtcgtcatcgcaaccccaaatgatatacatgccgttaacataatattaactcatcataccagcttgataattacccaacgaaaaggttgcgaagcgcgtcactatttatttttatctttaccgtaagaatgcagaaacagcggaccagccgctgtttctttttctttaaaaacaagcaattattcagttacaactgtttgtactctcgcggggccgggattataccagccccatccgccgtagccatagggccagccacgaccgccataaaaccatggatcaatcggctgaggcggcataatcacctgctgggttaaatgccaacgtttgtaacccgttacttgcatcaccataaatttatagggcgtattgccgattttgccgtcaaccgcaccagtgattggcccgactaccgtaaccagttgtccacggaaatccaccgggtccagaaaaccgttcacatcggcataaatgcgaccgcgagaaggttctcccagcgtcggtctggctccgctgtccagcggtacggtagcaatttccaggcgagttttcccttgctggttttgtaccgcaaccactttgccaccaaagcgtgcctcctgaccaacgtacagctgcggcgcactcatcacccgaactaaatcttgttgcggcgtgggactgctgcctttaatggcgtccggcacagtgacacaaccgctcagcattagcgcaaacgtacctgccagtatgcctttgataacattcttttgaaccgccatggtgcgactcctttttttctcagggcatactcttaagattcattctttgcccggaagtttcttccatgcgacgttgttacgtaaataaaccggttcggcatgttccaccgccaccgttttaccctcagcaaacatctgacacgcaatcggcagcatatcttcagcagcaggcagtaacacttcgccatcgcgcaaaaccagcccgctctctttaccgagatccggccaagcttgccagcccgtccctaccgtcacccattcgccggaaagctgttgcattcgttcatggacgatttcgggtttgagtacggcttcggtttcttcaccgtgccagataccgttttcatcacgctgatattcggcccagtaaacttcgcccattcgcgcgtcaatggctgccagcacgcgggttgcgccgtttttgcgccacgccccttgcgccatcgtcattagcgtggagacgccaatcatcggtaattccgcgccaagcgccagcccttgcgcgatgccaataccaatgcgcacgccagtaaagctaccggggccgcgcccgtaagccagagcgttaatatcagtcagggaagttccgctggtggtcaggatatcctgcaccatcggtaagattcgttgagtatgttcacgagggcaaagctcaaaatgagcgttgacagtaccgtcgttccacagggcgacagagcaggcctctgtcgcggtatcgatagccagaattcgcatgggtcttcgtgcttagatcaataaaaaggcgcgcatcataccatactccgtaacaaattacctggaggatggtatcgcaaggaaacgaaccgcacgggcaatgtcacgggtgcgtggcgcgggcggcagactggcgagaaacgtcgcgccgtaaggacgcatcaccagccgattgtcacaaatcaccagcacgccacgatcgtcggcgtcgcgaatcagtcgccctaccccctgtttgagagtaatgacggcatctggtagttgcacttcatcgaacgggtcgccaccgcgcaaacgacaatcttccatgcgcgcttttaacagtggatcatccggcgaggtaaacggcaatttgtcgataattaccaatgacaatgtatcgccacgcacgtccaccccttcccagaaactgctggttgccacaagaagcgcattaccggcgctgacaaattgctgcaacagttgccctttgctggtttccccctgcaacaatacaggaagcgtcatggtagcgcggaactgctcggccagatcgcgcatcatggcgtgcgaggtacaaagcataaaacaacgaccgttgttagcttcgatgatcggtcgcagcattgccgctaactggcgagcagaacctggctggttggtttgcggcagattgcgcagcacacagagtaacgcctggcggctgtaatcaaatgggctgggcaacagcaacgactcggcctgttcgatgccaagccgcgaggtgaaatgatgcagatcgtcgttcaccgacagcgttgctgaggtgaagatccagctaccgggtttttgcgccattaactctttgaatttatccgccacgctgagcggcgtgagagccagagtaaaatggcgcgaagtgcattcgtaccagtagctgtagcccggctgattgatctcttttagccgcttcagccgtgtgcgatacaacgtggcgcgctcaaatgccgcatccagcaaggcggaacgccccagtgacagtttcgccacgtcataacaaagttccagggtgtcatcgagcagtaaaaatgcccgctgaatttgcggattagctaacagctcacgcaggttaccgcgataacctggctcaccgagttgcagacgaaaatcctgcgcactctgggcaagacgatcagcgcacttttgtaactgctgggtgtcttttaattcggtgcggtaggcgatggtgatgtcttttgccaggtcgagcagttgtcgactggagagtgactgaccaaaatactggctggcaatgtccggtagctggtgggcttcgtcgaagatcatgacgtccgcttccgggatcagttcgccaaatccactctctttaaccaccatatccgccagaaagagatgatggtttaccaccaccacatcggcgtccatcgcttttttacgtgctttgaccacaaagcaatctttatacatcgggcagtcgctgccaagacagttgtcgttggtgctggtgaccagcggccacgcctgtgaatcttccgccacgctgacgcaggtgctgatatcaccatcgactgtttgattagaccaggagcgcagcaggatcacatcgcttaagatttgtaccggcagatcgccccccgccagcgcctgctgttcgagacgttcgaggcagaggtagtttgagcgccctttcagcagcgccacgttgcccgtatatttcaatgcctttgagactgttggcaaatcgcggctgtagagctgatcctgcaacgcttttgagccggtcgagataatgactttctttttcgcccgcagcgcaggagccaggtaagcgtaggttttgcccgtaccggttcctgcttccaccaccagcggctggcctttttctatcgcctgggtgacggctaccgccatctgtcgctgtggttctcgcggcttaaagcctggtatcgctttcgccagctgaccgtctggtgcaaaatcgtccgtcacactaccccctgttgatttgaacagggattatgtcaggatgagggcgctttcgccagttgaagtggtgacggcgacctcacattgtggcagtctttgcagcacgaaaatggaagtataatgaggacaaaatgatgactatcgttcgtatcgatgctgaagcccgctggtctgatgtagtaatccacaacaacacgctctactacactggtgtaccggaaaacctcgacgccgatgcctttgagcaaaccgccaacacgctggcacagattgacgccgtgctggaaaaacagggcagcaataaatcgagcattctggatgccaccattttcctggccgataaaaacgacttcgcggcgatgaataaagcgtgggatgcttgggttgtcgcgggtcatgcgccggtgcgctgcacggtacaagcgggtttgatgaacccgaagtataaagttgaaattaagattgtggctgcggtgtaagctttatcgaagcaaaataagtcagacgataatttatcgataatactggtcggttttacataaatcgaccagagaataagatattactgttgatgcttctgctaattcattatttatatttataatttcaattttatctataaaactaactatataaataaacataaacatgccgttgtgttcgccctttgattagcaactctggttttctttcttagctgaacaatctggttatagcgtgcggactgaccgttaaatttctccatcttactggataacacaccatgagctgctacctttaaaacacctgaatgtcaacaggttaactcgtgccatatcgttataatccctttgatattagatgcaaattaaggtcatatatagccttatcgataacatggttaattttaaggataagaatatgcctgctgtaatagataaagccctggatttcattggtgccatggatgtatcagcgccaacaccaagttcgatgaatgaaagcacggcgaagggaatctttaaatatttaaaagaactgggagtacccgcgagtgccgctgatattacggcgcgagctgaccaggaaggctggaaccctgggttcacggaaaaaatggttggatgggcaaaaaaaatggagacaggtgaacgttctgtgattaaaaatcctgaatacttttcaacatatatgcaggaagaactaaaagcactggtctgagttaaatttatatcagcataaatgggtcaggacgcttttaatcacatataaaaagcgtcctttttctcacaatcaaatgatcatcggcttctataacgaaatcgatacggattagtgtgttactcgtcttcatcctcaaaacgcgccacgattcgctcgccggagtggttggcacgcagctcttctgccaccagcgcgattgcctggccgctgctcatcccttgtgccatcagttcctggatccgctcgacagctttttgctgctgttcatgggtgagtgaaggtaaacctgcaaacattgttaactcctgctaaattgttggcgctaattatttcatgctacccggcacatagccagtagagtcaggactgatgaagacgttatctcccgctgtgattactttactctggcgtcaggacgccgctgaattttatttctcccgcttaagccacctgccgtgggcgatgcttttacactccggctatgccgatcatccgtatagccgctttgatattgtggtcgccgagccgatttgcactttaaccactttcggtaaagaaaccgttgttagtgaaagcgaaaaacgcacaacgaccactgatgacccgctacaggtgctccagcaggtgctggatcgcgcagacattcgcccaacgcataacgaagatttgccatttcagggcggcgcactggggttgtttggctacgatctgggccgccgttttgagtcactgccagaaattgcggaacaagatatcgttctgccggatatggcagtgggtatctacgattgggcgctcattgtcgaccaccagcgtcatacagtttctttgctgagtcataatgatgtcaatgcccgtcgggcctggctggaaagccagcaattctcgccgcaggaagatttcacgctcacttccgactggcaatccaatatgacccgcgagcagtacggcgaaaaatttcgccaggtacaggaatatctgcacagcggtgattgctatcaggtgaatctcgcccaacgttttcatgcgacctattctggcgatgaatggcaggcattccttcagcttaatcaggccaaccgcgcgccatttagcgcttttttacgtcttgaacagggtgcaattttaagcctttcgccagagcggtttattctttgtgataatagtgaaatccagacccgcccgattaaaggcacgctaccacgcctgcccgatcctcaggaagatagcaaacaagcagtaaaactggcgaactcagcgaaagatcgtgccgaaaatctgatgattgtcgatttaatgcgtaatgatatcggtcgtgttgccgtagcaggttcggtaaaagtaccagagctgttcgtggtggaacccttccctgccgtgcatcatctggtcagcaccataacggcgcaactaccagaacagttacacgccagcgatctgctgcgcgcagcttttcctggtggctcaataaccggggctccgaaagtacgggctatggaaattatcgacgaactggaaccgcagcgacgcaatgcctggtgcggcagcattggctatttgagcttttgcggcaacatggataccagtattactatccgcacgctgactgccattaacggacaaattttctgctctgcgggcggtggaattgtcgccgatagccaggaagaagcggaatatcaggaaacttttgataaagttaatcgtatcctgaagcaactggagaagtaagacgtggaataccgtagcctgacgcttgatgattttttatcgcgctttcaacttttgcgcccgcaaattaaccgggaaaccctaaatcatcgtcaggctgctgtgttaatccccatcgtccgtcgaccgcaaccggggttgttgctgactcagcgttcgattcatctgcgtaaacacgctggacaagtggcattccctggaggtgcagtcgatgacacggacgcatcagctatcgccgccgcgctgcgcgaagctgaagaagaggtcgctataccgccttccgccgttgaagttatcggcgtgctgccgcccgtcgatagcgtcactggctaccaggtaaccccagtggtcggcattatcccgcccgatctgccgtatcgcgccagtgaagatgaagtctcggcggtgtttgaaatgccgctcgcccaggcattacatctgggtcgttatcaccctttagatatctaccgccgtggtgattcacatcgggtatggctgtcctggtacgaacagtattttgtatggggaatgaccgcaggcataattcgtgagctggcgctgcaaattggtgtgaaaccctgactatacttatctttacatctacaaaacactacttgagacaatcatcgcaatattagttaaatcgcggtttttgattagtttaattcatgtgaatagttaagccagtcgccgcgttccctcttacactatgcgctgttattagttcgttactggaagtccagtcaccttgtcaggagtattatcgtgattagtctattcgacatgtttaaggtggggattggtccctcatcttcccataccgtagggcctatgaaggcaggtaaacagttcgtcgatgatctggtcgaaaaaggcttactggatagcgttactcgcgttgccgtggacgtttatggttcactgtcgctgacgggtaaaggccaccacaccgatatcgccattattatgggtcttgcaggtaacgaacctgccaccgtggatatcgacagtattcccggttttattcgcgacgtagaagagcgcgaacgtctgctgctggcacagggacggcatgaagtggatttcccgcgcgacaacgggatgcgttttcataacggcaacctgccgctgcatgaaaacggtatgcaaatccacgcctataacggcgatgaagtcgtctacagcaaaacttattattccatcggcggcggttttatcgtcgatgaagaacactttggtcaggatgctgccaacgaagtaagcgtgccgtatccgttcaaatctgccaccgaactgctcgcgtactgtaatgaaaccggctattcgctgtctggtctcgctatgcagaacgaactggcgctgcacagcaagaaagagatcgacgagtatttcgcgcatgtctggcaaaccatgcaggcatgtatcgatcgcgggatgaacaccgaaggtgtactgccaggcccgctgcgcgtgccacgtcgtgcgtctgccctgcgccggatgctggtttccagcgataaactgtctaacgatccgatgaatgtcattgactgggtaaacatgtttgcgctggcagttaacgaagaaaacgccgccggtggtcgtgtggtaactgcgccaaccaacggtgcctgcggtatcgttccggcagtgctggcttactatgaccactttattgaatcggtcagcccggacatctatacccgttactttatggcagcgggcgcgattggtgcattgtataaaatgaacgcctctatttccggtgcggaagttggttgccagggcgaagtgggtgttgcctgttcaatggctgctgcgggtcttgcagaactgctgggcggtagcccggaacaggtttgcgtggcggcggaaattggcatggaacacaaccttggtttaacctgcgacccggttgcagggcaggttcaggtgccgtgcattgagcgtaatgccattgcctctgtgaaggcgattaacgccgcgcggatggctctgcgccgcaccagtgcaccgcgcgtctcgctggataaggtcatcgaaacgatgtacgaaaccggtaaggacatgaacgccaaataccgcgaaacctcacgcggtggtctggcaatcaaagtccagtgtgactaatacttcttactcgcccatctgcaacggatgggcgaatttatacccgctttctcgtctgctgtaatattccccactacacttccactgttgcgtcaggcgtttgtcgccatacgcttacagggtggcccgcatgcaaaaagcacaacggatcattaaaacctatcgtcgtaatcgaatgattgtttgtacgatttgcgcactcgttacgctcgcttcgaccctgagcgtgcgatttatttcacagcgtaacttaaatcaacaacgggtagtacaattcgccaatcacgctgtagaggaattagataaagtactgcttcccctacaggcaggtagcgaagtcttgcttccgctgattggtctgccctgctctgtcgcccatttgccattacgtaaacaggcggcaaaactccaaactgtgcgatccattggcctggtgcaagacggcacactttattgctccagcatttttggttatcgcaatgtgcccgtcgtggacattctggctgaacttcctgcaccgcaaccacttttacgcctgacgatcgaccgtgccctgattaaaggcagtccggttttgattcaatggacgcctgcagcgggcagtagcaatgctggggtcatggagatgattaacatcgacttactgacggcaatgctgcttgagccacaactgccgcaaatcagtagcgccagcctgacggtggacaaacggcatttgctctatggtaatgggctggtagattcccttccgcaacctgaagacaatgaaaactatcaggtttcttcgcaacgctttccttttaccattaacgttaatggtccgggggctacggcgctggcatggcactatcttccaacacaattaccgctggcggtgctgctaagtttactggtgggctacatcgcctggctggcgaccgcttaccgaatgagcttttcccgcgaaatcaatctgggcctggcgcaacatgagttcgaattgttctgtcagcctttgcttaatgcgcgcagccagcaatgtattggtgtagagattttgctgcgctggaacaatccgcgtcagggctggatttcaccggatgtgtttattcctatcgcggaagaacatcatttaattgtgccactgacccgctatgtgatggcagaaaccattcgtcagcgccatgttttcccgatgagtagtcagtttcatgttggcattaacgtcgcacccagccattttcgccgtggtgtgctgataaaagatctcaatcagtactggtttagcgctcacccgattcagcaactgatcctcgaaatcaccgaacgcgatgccttactggatgttgattatcggattgcccgcgagctgcatcgtaaaaacgtcaaactggcgattgatgacttcggcaccggcaacagctcgttttcctggcttgaaacattacgtcctgacgtgctgaaaattgataagtcatttaccgcagctataggttctgacgcggttaactcgacggtgaccgatatcatcatcgcgctggggcaaagactgaatattgaactggtggcggagggcgtggaaacgcaagaacaggcgaagtatttgcgccgtcatggcgtgcatattttgcaagggtatttgtacgcacagccgatgccgctacgtgattttcccaaatggctggcgggcagccaaccgccgcccgcccggcataatggacatatcacgcccattatgccgttacgttaacgcttactcatcttcatcgtgcgccggttgctctttaacaatgcgaaccagatcaacacgataatcattggcttcaatgatggtgatatgcagtggccctacatcaatcacatcgcccacacggggaatgtgaccatttgccgagatcacgaggcccgcgaccgtcgcgatatcatcgtcatcggcaaggtgctcaacatcaagcgcctgctgcaaggcatgcaaatctgtaccgccttttaccagccagccgtcaccatcagtaatgatttccggcgtttcgtcagcgtccgggaattcacccgcaatggcttccagcacatccagcggcgtgaccagaccttgtaccacaccaaactcgttggtcacgataacaaagctcccgcgagcacgacgcagcacgcccaacaggttgatcggatcgagggtttccgggacgataatcgccggagacgccgaagcaatcgccgccacatcaacgccctcttccagcgccaccagcagttctttagcacgtacaataccgatgatttcatccagttcaccgcgacataccgggaacagactgtgcggtgaagagagcagttgctcgcggatttcatcgaccccgagattagcgtcaacccagcttatttcaccgcgcggcgtcatgatcccgcgcagagaacgcgacgccagcgtcagtacgccgttaatcatgtaacgttcttcttcggcaaatgcaccttccgggatcggcatcggcatcgggttatcggcatcgtgctgaacattggcctgacgtttcccgcccatcaaacgcaggatggcatcggcagtacgcgctcgcagcggcaaagtcgactggtggcgaataaagttgcgacgcgcaatctggttaaacacttcgatgatgatcgagaagccaatcgcggcatacaggtaacctttcggaatgtggaaaccgaaaccttctgccaccagactcagaccaatcattaacaggaagctcagacagagcaccaccaccgtggggtgctggttaacgaatcgcgtcagcggtttggatgccagcaacataaccgccatcgcaatcactaccgccgccatcatcaccggcagatggttaaccatccctactgcagtaattaccgcatccaacgagaagacggcgtcaaggatgacaatctgtgtgacgaccacccagaaactggcgtagcctttaccgtggccggaatcatgatcgcggttttccagccgttcatgcagttcggttgttgctttgaacagcaagaatatccccccgaacaacataatcaggtcgcgtccggagaaggagaaatccatgacggtaaatagcggtttggtcagcgtgaccatccatgaaatcagcgacagcagccccagacgcataatcagcgccagtgataaccccagcaaacgcgctttatcgcgttgttttggcggcagtttgtcagcaagaatggcgatgaagaccaggttatcgatacccagcacaatttcgagaacaacaagcgtgagtagccccgcccaaattgaggggtccattaagaattccatgacaagctcctgcttaaggaatagctattcgacgccagaaataatgcaggcgtaacgacaaaatgcaaacgaaaggtgcggcatagagtgccagaaaggcaggcgttaaaaggcctgatgctgaaatgacgtcggtgacgatccatactgcgggctactgccctatactccatggttgttaaacgggagttaaacatatcagagacgcctctgatttggcaaagatttaccttcctttgcaaacgaatgtgacaaggatattttacctttcgaaatttctgctaatcgaaagttaaattacggatcttcatcacataaaataattttttcgatatctaaaataaatcgcgaaacgcaggggtttttggttgtagcccttatctgaatcgattcgattgtggacgacgattcaaaaatacatctggcacgttgaggtgttaacgataataaaggaggtagcaagtgaccattgctattgttataggcacacatggttgggctgcagagcagttgcttaaaacggcagaaatgctgttaggcgagcaggaaaacgtcggctggatcgatttcgttccaggtgaaaatgccgaaacgctgattgaaaagtacaacgctcagttggcaaaactcgacaccactaaaggcgtgctgtttctcgttgatacatggggaggcagcccgttcaatgctgccagccgcattgtcgtcgacaaagagcattatgaagtcattgcaggcgttaacattccaatgctcgtggaaacgttaatggcccgtgatgatgacccaagctttgatgaactggtggcactggcagtagaaacaggccgtgaaggcgtgaaagcactgaaagccaaaccggttgaaaaagccgcgccagcacccgctgccgcagcaccaaaagcggctccaactccggcaaaaccaatggggccaaacgactacatggttattggccttgcgcgtatcgacgaccgtctgattcacggtcaggtcgccacccgctggaccaaagaaaccaatgtctcccgtattattgttgttagtgatgaagtggctgcggataccgttcgtaagacactgctcacccaggttgcacctccgggcgtaacagcacacgtagttgatgttgccaaaatgattcgcgtctacaacaacccgaaatatgctggcgaacgcgtaatgctgttatttaccaacccaacagatgtagagcgtctcgttgaaggcggcgtgaaaatcacctctgttaacgtcggtggtatggcattccgtcagggtaaaacccaggtgaataacgcggtttcggttgatgaaaaagatatcgaggcgttcaagaaactgaatgcgcgcggtattgagctggaagtccgtaaggtttccaccgatccgaaactgaaaatgatggatctgatcagcaaaatcgataagtaacgtattgtgttgattatcactcagttttcacacttaagtcttacgtaaacaggagaagtacaatggagattaccactcttcaaattgtgctggtatttatcgtagcctgtatcgcaggtatgggatcaatcctcgatgaatttcagtttcaccgtccgctaatcgcgtgtaccctggtgggtatcgttcttggggatatgaaaaccggtattattatcggtggtacgctggaaatgatcgcgctgggctggatgaacatcggtgctgcagttgcgcctgacgccgctctggcttctatcatttctaccattctggttatcgcaggtcatcagagcattggtgcaggtatcgcactggcaatccctctggccgctgcgggccaggtactgaccatcatcgttcgtactattaccgttgctttccagcacgctgcggataaggctgctgataacggcaacctgacagcgatttcctggatccacgtttcttctctgttcctgcaagcaatgcgtgtggctattccggccgtcatcgttgcgctgtctgttggtaccagcgaagtacagaacatgctgaatgcgattccggaagtggtgaccaatggtctgaatatcgccggtggcatgatcgtggtggttggttatgcgatggttatcaacatgatgcgtgctggctacctgatgccgttcttctacctcggcttcgtaaccgcagcattcaccaactttaacctggttgctctgggtgtgattggtactgttatggcagtgctctacatccaacttagcccgaaatacaaccgcgtagccggtgcgcctgctcaggcagctggtaacaacgatctcgataacgaactggactaacaggtgagcgaaatggttgatacaactcaaactaccaccgagaaaaaactcactcaaagtgatattcgtggcgtcttcctgcgttctaacctcttccagggttcatggaacttcgaacgtatgcaggcactgggtttctgcttctctatggtaccggcaattcgtcgcctctaccctgagaacaacgaagctcgtaaacaagctattcgccgtcacctggagttctttaacacccagccgttcgtggctgcgccgattctcggcgtaaccctggcgctggaagaacagcgtgctaatggcgcagagatcgacgacggtgctatcaacggtatcaaagtcggtttgatggggccactggctggtgtaggcgacccgatcttctggggaaccgtacgtccggtatttgcagcactgggtgccggtatcgcgatgagcggcagcctgttaggtccgctgctgttcttcatcctgtttaacctggtgcgtctggcaacccgttactacggcgtagcgtatggttactccaaaggtatcgatatcgttaaagatatgggtggtggcttcctgcaaaaactgacggaaggggcgtctatcctcggcctgtttgtcatgggggcattggttaacaagtggacacatgtcaacatcccgctggttgtctctcgcattactgaccagacgggcaaagaacacgttactactgtccagactattctggaccagttaatgccaggcctggtaccactgctgctgacctttgcttgtatgtggctactgcgcaaaaaagttaacccgctgtggatcatcgttggcttcttcgtcatcggtatcgctggttacgcttgcggcctgctgggactgtaagactgttgtacactaccggggccttttggccccgtttttttatctggaggattaatgacaatcacggacctggtactgattcttttcatcgccgcactcctggccttcgcgatctacgatcagttcatcatgccccgccgtaacggccccaccctgctggcaattcctttgctccggcgtggtcgcatcgatagcgttatcttcgtcggattgattgtcattcttatctataacaacgtcacgaatcatggtgcgttaataacgacatggttattaagcgcactggctctgatgggtttttatatattctggatccgcgttccgaagatcatctttaaacaaaaaggttttttcttcgccaatgtctggattgaatatagccgaatcaaagcgatgaacttgtcggaagatggcgtgttggtgatgcaattagaacagcgtcggctgttaatccgcgttcgaaatatcgacgatctggaaaaaatttataagcttctcgtttcaactcaataagttatgaatttagccaaagctatgtttagtgtatttttaataatcagacatagcttaggctatattacctcttcccttatttgttatttattttaacgtttcattgatatataaatccaaatgaaaatcgttatcaataaagcaatgaaataatatattccaacagttgttttatattctcaaaatatgttaaggttgcgccctcatttggggagtagccgatttccagattccggaaatgtacgtgtcaacatactcgttgcaaaacgtggcacgtacggactgaatactttcagtcaggcgagaccatatgcacatcaatcgctatgcctgcatgaacgcgaaaaccatcacggcttgttgttcatgtatgcatgtttgctgggggcgatgatgtgttttatggataccccggtcaggacattgtcatgaatatcactgctactgttcttcttgcgtttggtatgtcgatggatgcatttgctgcatcaatcggtaaaggtgccaccctccataaaccgaaattttctgaagcattgcgaaccggccttatttttggtgccgtcgaaaccctgacgccgctgatcggctggggaatgggcatgttagccagccggtttgtccttgaatggaaccactggattgcgtttgtgctgctgatattcctcggcgggcgaatgattattgagggttttcgtggcgcagatgatgaagatgaagagccgcgccgtcgacacggtttctggctactggtaaccaccgcgattgccaccagcctggatgccatggctgtgggtgttggtcttgctttcctgcaggtcaacattatcgcgaccgcattggccattggttgtgcaaccttgattatgtcaacattagggatgatggttggtcgctttatcggctcaattattgggaaaaaagcggaaattctcggcgggctggtgctgatcggcatcggcgtccagatcctctggacgcacttccacggttaataagaacgctgccagaggtgaatattaaagtccgtctggcagtcgaacacttcttttgctgccagtgtttgccagacttctggcttcgcacgccaggcaaacggcgtcatctgcaataatgcgacggcttcatcaccgcgaagacgcatcggataacacaactccgcactctgctgtaatgtaaaaccttccagttgttctgcatgaggtgcatgaagatgtacttcattgtaaatcagccccttcagctccatcaaatgtcgcggtcccggcgtggcagtaatgacccagccgccgggcttcactactcgtgctaattcttctgctttacacggcgcgtaaatacgtattatggcgtccatactggtatcggaaaacggcaaacggtggctggaagcgacacaaaaagtgacctgcggatagcgtttcgccgccgcttttatcgctaccttcgaaacatccagaccaaacgtggtgatttcgggcaacgcatcggcaaatgcgtgtgtgtaatacccttcaccacagccaatatccagcaccgccgtggccttatcatcaagccgttccctcagttgggcgacaattgcatcacgcagcggctgataatgtccggcatctaagaatgcgcggcgtgcttgcatcatttccgcgctgtcgcccggatcacgagaccgtttatgctgaacgggcagcagattgacatacccttctttcgccatatcaaactgatgtcgctggggacagatatagctgtttttttcacgcgaaagaggctgatggcaaagtggacaggaaaaagacatgacaactccggcaggatactaaaggccgcaagtgtaacgcgaatcacgcggcgggcaaatatccgaacgccaggagcgaagataaagcatagtaaaaagcctcgcattcgacgaggctttatagcgagattgaagcgtattcacacttcagatcagtggattcgatcagatagctgttacgttaacagctgccggacctttctggccgtcctgaatttcgaactcaacgttctgaccttcagccagagttttgaagccattaccctggatagcggagaagtgtacgaacacatctttgctgccatcagccggagtaatgaagccaaaacctttagactcgttgaaccacttaacctgacctttaatctttgccatttgaaaaattccttagattgttttcttcgcccgcaggcataacatagataaaactgacacattactgcatgaggcaccaatataaggctcggcagagaagcggtattcaacgtcaacgtgtttactcaggacttctttactgaaaatgccacacataaacagaactgtacctcgtttaacccgaaatctgttatcacatacaacgttaattatggcaagccatttttaaacatgtctcgatcagacgcacaaatctcgatacgtcttccactttttttgcacacttatgcaacggaatacgcgccgatatatcattgtgcttaaccttgccagttcaggcagatacttaaactggcgtattttctaacatagttcaataagttcagttgttccaggccagtgggagaagttattacatagtgcgtgcaatatcacattttttgctatgcaatgaataaaaagttatatcactttttctcataaaacagtcagttaacggctattaattaccctaaagagaagtcaatccccaaagggattgtaaatttaaaataagaaaaattgatgaatgagcaaaaaaatcaagagagaaacgtttcgctaataaataataccacgcttaatcacaaatccgatgtaaacatcctaataaattaatggggtaaatatctttttctgatatcccgttacgcaaataaataatatgataattatttgaagtcagaccagagttttaatttgaagcagttgcaccatgacagtgcgtataatcaggatgaattgagtaacccttcaacgacggggttactcaagattgaggaaggattatcgttcggcgaccagacgaataatatcttcgtcttcaaccgatttttgactctcaacggtctttttatctgctttctctggttcgtttgcttcgcacaaacgacgtaacagtgcattttgacgtttttgctgatccagcaacgcctcaagcagttcaatctgttcgttagtccgtgaactggcacgattgataaaaaaccacaagatgagcccgataagaagaaccaccaccgatacaaccaaagacgcaatgttcatcacgcctgaatttacaacttcgttcatttcaccacctctgagtagaggcgctattctaccactgctggagaggaagaaaatctagtgctgaaaaaatgatatcaccacgggataaactggttaatggcacaaattccgctgaaaaattgtacatcctgatcgcacatcatgttgaatacctgcgcccaaagcagcaagcaagccaacaccacgacaaccagaacgacccatcgaaactttttcactccaatctccgtttcacctaccttatgtcattaaactagcatgcgttagttaaacagcgcctaactatgtcgatattcgtgctttttcggaatgagtcgcttgcttcagcgcatattgccgctacgattaagcgaacataaaaagagaagaggttgtaatgcgattcatcattcgcacagttatgctgatagcactggtatggataggattattactcagcggatatggcgttttgattggaagcaaagagaatgccgcaggattaggtttgcaatgtacctatctgactgccagaggcaccagcacggtacaatacttgcacactaaaagtggttttttggggataacagattgcccgctgttacgcaaaagcaatatcgtggtcgataatggttaagggcaataaataaccagattctcactcctgagtaaaatactcttatagcaagcgcgtttaatataacgccaccttcaactttatttttctcatgctaaataaagaacctgtctgtttgatattccgacaggttcttactctcatcagaacggatagtcgtgataacccatttgggcagaaattttgcgcgctgcggtatgcaacattgcgacatattcctgtaaacgctcttcagagaaacgcaacgtcgggaaggagatgctcaaaccggcaatgaccacgccaaagcgatcaaataccggtaccgcaatgcatcgcagcccttcttcctgctcttcattatcttcgccatacccctgctcgcgcacctggtccagaacgggtaataacgcttctgtactggtgatggtccgctcggtactgcgtttatactccacgccctcaagaatttgcttcacttcatcgcgatcgcgccatgccagcagtaccttaccaatcgcggtgctgtacagcggattacgacgcccaatccgtgaatacatgcgcaaattgtacatagagtcaattttgtgaatgtaaacaatactgtcttcgtccagtgcgccgaggtggatagtttctttggtcaggcgggagagctcacgcatctggatatctgcgctacgaattaaatcgacgttttgtaacgcgcgagcgcccagttcaaacaatttcagggtcagggaatatttctccgactccccttcctgcgccacataacctaaggttttcatggtctgtaaaaagcgataaacggtgctttttgacatcatgacgcgctgcgacagctcggttatccctatttcgcgctcttcacccagcgcctgcaaaatgccaaaaacttttagcacggaagatacagaatcaggctgtttatccagatctgcgttagccatttatcacctcattgcgagtgttttataaaaatcagaactgttttttattataatttcgcaccagggtggtcgcaatccatcttttgccggttagttacaattctgcgacatccaccgtgaatatcagtgctagaatcatacccctgttgattattcaccaaagatataaaattcctatgccaaaagttcaggccgacggcctgccattgccccagcgatacggtgcgatattaaccattgtgattggtatttcgatggccgtccttgacggcgcaatcgccaacgtcgccctgccaacaatcgccacggaccttcatgccacgccagccagttccatctgggtagtgaacgcctatcaaatcgccattgtcatctccctgctctcgttttcgtttctgggcgatatgtttggctatcgacgtatttataaatgcggtctggtcgtttttctgttgtcttcactgttctgcgccctttctgattcgctgcaaatgctcacccttgcgcgtgtcatacaaggtttcggcggtgcagcgttgatgagcgttaataccgcacttatccgcctgatctatccacaacgttttctgggtagagggatgggcataaactcgtttattgttgccgtctcttctgctgccgggccgacaattgctgcagcaatcctctccatcgcatcctggaaatggttatttttaatcaacgtaccgttaggtattatcgccctgcttctggcgatgcgttttctgccacccaatggttctcgcgccagtaaaccccgtttcgacctgcccagcgccgtgatgaacgcgttaaccttcggcctgcttatcactgcgttgagtggtttcgctcaggggcaatcgctgacgttaattgctgcggaactggtggtaatggttgttgttggtattttctttattcgccgccagctttctcttcccgtaccgctgctaccggtggatttactgcgtatcccgctgttttcactttctatttgcacatctgtttgctctttctgcgcacaaatgctggcaatggtttccctgcccttttacctgcaaaccgtgctcgggcgtagtgaagtcgaaacaggtttacttctgacaccgtggccgttagcaacgatggtgatggctccgctggcaggctatttgattgaacgcgtacatgcaggattgctgggggctttagggttgttcatcatggctgcggggcttttttccctggttctgctgcccgcgtcacctgcggatatcaatattatctggccgatgatcttatgtggtgctggatttggcttattccagtcacccaataaccacaccattattacctccgcgcctcgcgaacgtagcggtggagccagtggcatgttaggaacggctcgtctactgggtcagagtagcggcgcggcgctggtggcgctgatgctaaatcagtttggagataatggtacacacgtctcgctgatggctgcggctattctggcagtgattgctgcctgtgtcagtggtttacgtatcactcagccacgatccagggcataaaaaaagcgcgtcgatcaggacgcgctttttagtatttacttcatattacttcaggtattcacccgtacgcagagcttcaattcgtttatccagcggcgggtgggtcatgaacaactcactgagcgatttcgacttaccgttaatgcagagagccatcatgctggttgcttcttgcggttcatagctggttttcaggcgctgcagcgcggcaatcattttctcgcgaccaaccagttttgccgaaccggcatcagcatggaattcacgatgacgcgagaaccacatggtgataatgctcgccagaataccaaacaccagttccagaaccgttgcaaccgcaaagtagatcagcgggttgccgttgctctcttcaccttcatcacgatttccgcccataaaacccgcggcaagctgcgccagaatacgggaaataaagataacgaaggtgttcaccacgccctgaatcagcgtcatggtgaccatatcaccattggcgatgtggctgatttcgtgagcaattaccgcctcggcttcatccgggctcatgttctgcagcaaaccggtgctgacagcaaccagagaggcatcacggcgcgcaccggttgcaaaagcgttgatgtccggcgcatggtagatagccacttgcggcatagcgatccccgcctgacgagcctgggttgctacagtattgaccagccaacgttccctttcgttacgcggttgctcgatcacttccccgccaacagatcgtaatgccatccatttggacatcagaagcgaaacgaaggaaccaccaaaaccgaacagcaaggccatgatcatcagcccctgaacgctgctcgactgtatccctgtcaggctcagtaccagcccgaaaacgaccattacggccaggttcgttagcaggaagagcgcgattcgcatcataattttctttttacctcagtttaacaaaacgcaatatgcgatacccacatcgtatgggttacgcgactattttcaagtctggatagtgcgtaagtcaccagaaagacacaactttacattttgtagcatctgatttacggcatcttgtcgctgttaaaaaatcaggcacaatttcttgtgcctgattgatattacttgacgggagcgggttgttccgcgggtctggctttttcaagcttcgccagatcgagtgcgatattcaccgtctcatccagataaggatccggctcctggtaatctttcggtagatcatccagtttcttcaactccggtttaccttcgcgtttaaagcgttcgttcaaacgcgccagacgcgtcgcatcatcttcattattctctttctcacgcacagcgtaattcagagaaacgatattgcgcttgtccttcatagcgttgaagcgcgcgatatccttcatgatgttctggaactcaggatctttcgcgatacgcgcattatgttccttcagcagctccggttcaaaggccgttaaatctcctgatttcacataagtcgcggcatcaatgctatcccacggcagcgcgttatcttcgaatttctcacccgtttccgtttcttcattacccgtcggcatgatgatgtctggcgttacgcctttacgttgcgtactgccgccgttaacgcgatagaatttctggatcgtgtactgcacagaacccagcgctggccattcaggacgtaacatctgatcgtaaatacggttcaatgaacggtattgctgaacggtgcctttaccaaacgtcggttcacccacaaccagcgcacgaccgtaatcctgcattgccgcggcaaagatttctgaagccgaagcactgaagcggtcaaccagcaccaccagcgggcctttatagaaaacctgtccgtcggtatcgctatcttcacgaaccttgccgttgttatcgcggacctgaacaatgggacccgcaggaataaacagaccggagagcgatacggcttcagttaacgccccaccgccattgctacgcaggtcgatgatgacgctgctgacattctgtttttccagtttctgcagttgcactttgacatcgtctgtcaaacccacatagaagcccggaatatccagcacgccgactttctctttaccgacggtcttcaccgacattttaaccgcgcggtcttcgagacgaatacgttcacgggtcaacgttacagtacgggtcttggtccctttaccagcaggtaaaatttccagacgaactttactgcccttcggccctttaattaaggcaaccacatcatcaagacgccagccaatcacgtcaaccatcggcttgcctgtttgaccaacaccgacaattttgtcaccaacgctgatagctttactcttcgctgccggaccacctgccaccatcgaattgataacggtgtagtcatcatccatttgcagcactgcgccaataccttccagcgacaaactcatttcagtgttgaactgttcggtattacgcggggaaagatagttggtatgcgggtcgatttcacgcgcaaacgccgtcattgccagcgagaaaacatcttcgctgttggtttgcgccagacgacgaatggcaaatttgtagcggcgagtcagggtttcacgaatttctttatccgtttttcctgtcagcttcaggcttaactcgtcgaatttgactttactgtcccacagcgcgttcaactcagcctcgtttttcggccagggcgctttgctgcggtcaaggttataagtgtcgttgccggtgaaatccatcggcttttccagtaccgacaaagcgtactggtaacgctcaaaacggcgcttttgcgccagattgtagagatcgtagaaaacgtcgagtttgcctgaacgcagttcatcgcctaactcggttttctttttcgcgaactgttcaacatcgcttgccagcagcacgttgtggctgtaatcgagcagattcaggtagcggtcaaagattttggccgaaaatgcctgatcgaggtcgaactggcgataatgagaacgggtgaagcgcgacgttacgcgctcacttaccgtcgcatgctgcgtctcttcctttaataccggaatttgatcagcacgcgtgatatcttctacagcgaaggtctggcctgctattgcaagcaggccagctaacgcggtaagcctaaaaaacatgttcatgcctggcccggcctccgtttcagaacaccaggtgttctgcgcgcacaatcaaagacatacccgaattcagctggacgcggacgccgtctttggtgatttctaatacggtggcatccatcgcgttttgacccgctttcaccttcagggcttgtccgacagtcagagctgaaatgtcagaaaccggggtgtgctgttcttcgcgaggtgcttttactgtttttggcgctttctctaccggcttttgcgcacgaggtttacgttcagcgccttctttgcggcgtggcgtagtcggacgtggcttgcgttcgcggcgcggtgcgtcttctttctcaccagcagttgcggcagcttcgcgttttttcgcttgctgttcagcacgctgtgcctgaacacgcgctttcgcttcttcaagctgcttgcgagcatgctctacatgttgctcgtccagctcaccgcatgggttgccgtcaagatcgacacgcgttgcgccgggtttaacaccgtaaagataacgccagctcgaagtgtagagacgtaaagcggatcgcaattgcgttttgctcaggttcatttccccagcaacacgatcgaccaaatcctgaaaaataccgattttcagcggacgcgcttcaccttccgcactgaaacagtggggaaaacgttcggccagaaacgcgattacttctttactgctattcaacttaggttgattttccatgaaatttcctgattacaacggacgtagccaacaagcgcaggcatgaacaggcgtcattataatgacgctatcagtaaatgctacgttatccgttgattatcctgcgacgctcgcaaagaattttttgtaatccgtcgttgcaagcactttttcaagctgtgccacaagctgacgtaagccttgctcgtcctcgtctgtaaagcgaccgaagacggtactatcgatgtcgagaacaccaataatctgatttttcaccaccagcggcagaacaatttcagaattactcgccgcatcacaggcaatatgcccgtcaaacacatgaacatcctcgatacgctgcacttgattgcgggcaaccgcagtgccgcacacgccgcgcccgacgggtatccggacacaggcaattttgccctgaaatggtccgagtaccagtgtatcgtcctcaagcaaataaaaacctgcccagtttatgtcagtgagacgctcatataacaacgcactggtgttcgcaagcgttgccagaaaactggtttctcccgccatcagcgcgttaaagtcgcgatttaaatccgcgtaaaattctgttttgttcattatataatcacttggttgtcttacctggatctgccagcctattaaaataagcattaaatgcgttaatgctcaagatcattcccatcatgggttaagattaatgttaattcttattacatttggcacgtcatggctcttaacacaccacaaattacgccgacaaaaaagataacagtgagggcaatcggcgaggaactgccgcgtggtgattaccaacgttgcccgcaatgtgacatgctgtttagcctgcccgagataaattctcatcaaagtgcctattgtccgcgctgtcaggcaaaaattcgtgacgggcgcgactggtcgctaacgcgcctggcggcaatggccttcaccatgctgttgcttatgccgtttgcctggggcgaaccgctgttgcatatctggctgttaggcattcgtattgacgccaacgttatgcaaggcatctggcaaatgaccaaacagggcgatgcgataacggggtcgatggtctttttctgcgttattggtgccccgctcattctggtgacctccatagcttatttatggtttggtaaccgactgggaatgaatttacgtccggtactgctgatgcttgagcgacttaaagagtgggtaatgctcgatatctacctggtcggcattggcgttgcttctataaaggtacaggattatgcccatatccaggctggtgtcggcttgttctcttttgtggcgttggtgattttaacgacggtgacgttgtcacatcttaatgtcgaagaactgtgggagcgattttatccgcagcgccccgctacgcgtagggacgagaaacttcgtgtctgtcttgggtgccattttaccggctatccagatcagcgtggtcgctgcccgcgttgccatatcccgctacgcctgcgtcgccgtcatagtctgcaaaaatgctgggcggcgctgttagcgtcaatcgttttattgttacctgccaacctgttgcctatttctatcatttatctgaacggaggacggcaggaagatacaattctttccggaattatgtcgctggcaagtagcaacattgcggttgcaggaatcgtgtttatcgccagtattctggtaccgtttactaaagtgatcgtcatgttcactttactgttgagcattcattttaaatgccagcaaggtttacgcacacgcattctgttactgcggatggtgacctggattggtcgctggtcgatgctcgacctgtttgtcatatctttaaccatgtcgctgattaatcgcgatcagatcctcgcttttactatgggaccggctgcgttttatttcggcgcagcggtaattttgactattcttgctgtggaatggctggacagccgcttactttgggatgcacatgagtcaggaaacgcccgcttcgacgactgaagcgcagattaaaaataaacgccgtatctcacctttctggctgctgccgttcatcgcgctaatgattgccagttggctgatttgggacagttatcaggaccggggtaataccgtcaccatcgactttatgtcggcggatggtattgttccaggccgtacgcctgttcgttatcagggcgttgaagtcggaacagtgcaggatatcagcctcagcgacgatcttcgtaagattgaagtcaaggtcagcatcaagtccgatatgaaagatgcgctgcgcgaagagactcagttctggctggtgacgccaaaagcatcgttggcaggtgtctccgggctggacgccctcgtcggtgggaactatatcggcatgatgccgggtaaaggtaaagagcaggatcactttgtcgcactcgatacccaaccgaaatatcggctggacaatggcgatctgatgatccacctgcaagcccccgatctcggttcgctgaacagcggttcattggtctatttccgcaagatcccggtgggaaaagtctacgactatgccatcaatcccaacaagcaaggcgtggtgattgatgtcctgatcgagcggcgttttaccgatctggtgaaaaaaggtagccgtttctggaacgtttccggcgttgatgccaacgtcagtatcagtggcgcgaaggtgaaactggaaagcctggcggcactggttaacggtgcgattgccttcgattcaccagaagagtcgaaacctgccgaggcggaagatacctttggtctgtatgaagatctggcccacagccagcgtggcgtaataataaaactggaactgccgagtggggccggattaaccgccgactcgacgccgttaatgtatcaggggctggaagtcggacagctgactaaactggatttaaatcctggtggtaaagtcacaggggaaatgaccgttgatcccagcgtcgttaccctgcttcgtgaaaatacccgcatcgaattacgcaacccgaaattatcccttagcgatgctaatctcagcgccctgctgaccggcaaaaccttcgagctggtgcccggcgatggcgagccacgcaaagagttcgttgttgtgccaggcgaaaaagcactgctgcatgaacctgatgttctgacgctgaccctgaccgcgccggaaagttacggtattgatgcgggtcagccgctcattcttcacggcgtgcaggtaggccaggttatcgatcgtaaactcaccagcaaaggcgtcacctttaccgtcgccatcgagcctcagcatcgcgaactggtaaaaggcgatagcaaatttgtcgtcaacagccgtgtcgatgtgaaggtggggctggatggcgttgagtttctcggtgccagcgcctcagaatggatcaatggcgggatacgtattctgccgggcgataaaggtgagatgaaagccagctatccactgtatgccaatttggaaaaagcgctggagaacagccttagcgatttacccaccacaaccgtgagtttgagtgcagagacgctgccggatgtgcaggcaggatcggtagtgctgtaccgtaaatttgaagttggtgaagtgattaccgtgcgtccgcgagctaacgcgtttgatatcgatctgcatattaagccggagtatcgcaaccttctgaccagcaatagcgtgttctgggcagaaggcggggcgaaagttcagctgaatggtagtggtctgaccgtacaggcatccccgctctccagagcattaaagggagccattagcttcgacaacctcagcggtgccagcgccagtcagcgtaaaggcgataagcgtattctgtatgcttccgaaacagcggcccgtgcggttggcgggcagattacgcttcacgctttcgatgccggaaaactggcggtcgggatgccaattcgctatctcggtattgatatcgggcaaatccagacgctggatctgattaccgcacgcaatgaagtacaggcaaaggcggtactttacccggaatatgtccagacctttgctcgcggtggtacgcgcttctcagtggtcacaccgcaaatttcggcagctggcgttgagcatcttgatactatcctccagccgtatatcaacgtcgaaccaggccggggcaatcctcgccgcgactttgaattacaagaggccaccattactgattcgcgttacctggatggcttaagcattattgttgaagcgccggaagccggttcgttaggcatcggtacgcctgtgctgttccgtggtctggaagtcggtacggttacaggaatgacgctggggacattgtcagatcgcgtgatgattgcgatgcgcatcagtaaacgctatcaacacctggtgcgtaacaattccgtcttctggttggcatcgggttacagtctggactttggtctgacgggcggcgtagtgaaaaccggcacctttaaccagtttatccgtggcggcatcgccttcgccacgcctccgggtacgccactggcaccgaaagcccaggaaggcaaacacttcctgttgcaggaaagtgaaccgaaagagtggcgtgaatggggaactgcgcttcccaaataatgcccactgctccggcgtgcctgcgccggagcgtttatgctaaactgcgcgcctgtttttttgccagtggtacatgctcgtggcccaacacaccgtttatttcccggacgcctttctgacacaaatgcgcgaagcgatgccttcgacgctctcatttgatgattttcttgccgcctgtcagcgcccgttgcgccgcagcattcgcgttaatacgctgaaaatctccgttgctgatttcctgcaattaaccgctccttatggctggacgcttacgccaattccgtggtgtgaagaaggtttctggattgaacgcgacaatgaagatgcattgccattgggtagtaccgccgagcatttaagtggcctgttttatattcaggaagccagttcaatgttgcctgttgccgccttgtttgctgacggtaatgcaccacagcgggtgatggatgtcgctgccgcgcctggctccaaaacgacgcaaatttccgcgcggatgaataacgaaggggcaatccttgccaatgagttttccgccagtcgggtaaaagtgttacatgccaatatcagccgctgtggtatcagtaatgttgcgctcacacattttgatggccgcgtgtttggtgcggcagtgccagaaatgttcgatgccattttgctggacgctccctgctctggcgaaggcgtggtgcgtaaagatcccgatgcgctaaaaaactggtcaccagaaagcaatcaggaaatcgcagctacacaacgggagcttatcgacagcgcctttcatgcattacgtcctggtggtacgctggtttactcgacctgtaccttaaaccaggaagaaaacgaagccgtttgcctgtggctgaaagagacttaccccgacgcagtagagtttttaccacttggcgatctcttccctggtgcaaacaaagcgctgaccgaagaaggctttttgcatgttttcccacaaatttacgactgcgaaggcttcttcgttgctcgtctgcgtaaaactcaggcgattcccgccttacccgcccccaaatacaaagtcggtaattttccgttcagcccggtgaaagatcgcgaagctggacaaattcgtcaggcggctacaggtgttggcttaaactgggatgaaaacctgcgcctctggcagcgtgacaaagaactgtggttgttcccggtgggcattgaagccctgatcggtaaagtccgattttctcggttggggattaaacttgccgagacgcacaacaaaggttatcgctggcagcatgaagcggttattgctcttgcctcacccgataatatgaatgcattcgagctgacaccgcaggaagcggaggagtggtatcgcgggcgcgatgtttacccgcaagccgcgccagtggcggatgatgtattggttactttccagcatcaaccgattggtttagccaaacggattggttcgcgattgaaaaacagctatccgcgtgaactggtgcgcgatgggaaactttttaccggtaacgcctgacagcgcacaaaaaaagcgcactttttgactggcacattcggctgcctcaactaggctgaaaaatggtgcgatcggactggtcgtaccacaatcggcagctaaatggagagcacgaagatgaaaaccagtgtgcgcataggcgcttttgaaatcgacgacggcgaattacacggtgaatcgccaggtgatcgaacgttaaccattccttgtaaatctgaccccgatttatgtatgcaactggatgcctgggatgctgaaaccagtatccctgccctgctaaatggcgaacactctgtcctttaccgtacccgttacgatcaacaatctgatgcctggattatgcgtcttgcctgatccaaaaagaacccgtcggcatggcgggttatttgtcctggttattcccccgttgtaaaatctctcctaaacttaacggtacggcaccacacttcggggatgaaatgttcgcgctggtactttttgtttgctacctggatggcggttgtgaagatattgttgtggatgtctacaacacggaacagcagtgtctttattctatgagcgatcaacggatccgccagggcggttgttttccgattgaggattttatagatggtttctggcgacctgcacaggagtacggtgatttttaattattgcaattgcacaagagtcagttcgcccccaaagacagcaccggtatcaatataatgcaggttgccaatatccacgcgatgtcgcaacggtgtatgaccaaaccagaaatgatcagcacctgtaattccctgccctttttggcgttcacctaatcgcgagcggctccacaagacctgatgcaaatcaacgtccttttgccattcataaacatcatctggataatcggcatgagcaataacatgcttgccggtgcgactgtgtacttcaagaataaagggcaaatgctgacatttttccagcgccgttttcgcttgtttctgttgattatctgccagcgcaataaaccagtcgccgccattcatcaaccacaaagacatctgctgggatgccagcgcatccatcgccatctgttcatgattgcctcttaccgcacaaacccaatgttgttccagtaactgcagacaacgtaaactttgcggcccacgatcgataacgtctcccactgagataagtaaatctcgccacggatcaaaacgacaatgccataatttgcggcgcaactgctcaagacaaccgtgtatatcgccagaaagccagatatgtcgccattgatgacccgcaattctctgataaacgggcgcaggctgtttcatcaatattttcctcccgcgctaaagatcacataatcttaacaagaatgttaaaaaacgctggactcagacagtagagtgtgtgttatggttgactataaagtcagcgaaggaaatgcttctggcttttaacagataaaaagagaccgaacacgattcctgtattcggtccagggaaatggctcttgggagagagccgtgcgctaaaagttggcattaatgcaggcttagttgccttgccctttaagaatagatgacgacgccaggttttccagtttgcgtgcaaaatggtcaataaaaagcgtggtggtcatcagctgaaatgttaaaaaccgcccgttctggtgaaagaactgaggcggtttttttattggaaatcaaaaggctattttaggtaattaacagagtttttcagctcgttctataaacggtgccagactcattttttcgccgggattgttaggatcatcaatctgaatcaccgaaatgggttgggcattggtcttcccactggcaacttccttttgtgcgatatcgtttaaaggatactgcacgagggtactcggattaataacatacaaagcattacccggtcggcaagtcagcatcacctcttcgcgattaaacgcccatttgtctttacccacttcaaaacgactgacggtaatcacctgcggtgcagccagcgccgctgcagaactggtgagtaacagaaacgccagaatactttttttcatcattttcgtaatccatcaaaaaggttcgagagtcgcaagcaggctgatgatcaccagcactaccgcacctatcgcccattcgagtttagtcatccacacaaaccagggtgccgcacgatcttcatcctgcctcatgcgcggtacaagaacataacgattagccagcgcaatgaccaccataatcatcaccaggatggctttgagcaataagagttggccccagtaagtcgtaagcgtggggggaaatccggtaatcaacaatgcattaagcacgccgcttgccagtacgccgatcaccgcaaaatgcccgcaccaggaaaaacgcatcagcgcctgaatagcctggtgtcgccaacggcctttgatgagttgcatacaccagagcaccggcagtaatcccccaaaccacgccgccgcacaaatcaggtgaatcgcgtgattagtctgatggattttcgctgttaccccttcattcagcgtcgcatgccccactcccgccagcagaataaattgcgcggtagtgagcataaacagcaaacgtggcatattccgcggttgcataagggcgacgatcaacgttacgagggcgagaacaatttgccataaccagatgccaccaaactgcgtttgcaaaacagcctgccaaatgtttggcgaaaatacatctgtccatcccgttcccatcaacccgccctgaacggcgagcattgcagtggcactgatcaaactccagacggcagcgtgctgttgtaaacgcagaaaacgcttcgccagcaagcgacgaatcgtcaagggggccagccaggcaccgtacattgcgaagccaaaaaccagcatcagcgaggtgaaatggataaatcgcagcgcgatccaggtaaacgccagcatgatttatttcacgctaaaggtgtagtgtcctttcgttttatgcccgtccaccgaaacaacatgccagtcaacggtgtaggttccgggtttcagcgaatcggccagtggaacaatcagttgcttttggtcctgctcatttcgcttcgccggtaatgttttaatattttcgttttttggccccgtgatttttgcaccactgaatcctgtttcaacaccttccgagaagtttaaagtgattgcctgcggtgcagctgtcacttgcgcgtttgccgcaggatactgatgcgttaaatgcgcatgtgcccagacggaaggtgtcaccaacgaagtggtcaggattgccagcgcgtagcgaagggagcgtgcagttgaagccatattatctattcctttttgtaataacttttttacagagcataaccttgtctaatgtctgagtcgaggatcatcaattccggcttgccatcctggctcactcttagtaacttttgcccgcgaatgatgaggagattaagaatgctgaagaatctggctaaactggatcaaacagaaatggataaagtgaatgtcgatttggcggcggccggggtggcatttaaagaacgctacaatatgccggtgatcgctgaagcggttgaacgtgaacagcctgaacatttgcgcagctggtttcgcgagcggcttattgcccaccgtttggcttcggtcaatctgtcacgtttaccttacgagcccaaacttaaataaaacttatacagagttacactttcttacataacgcctgctaaattatgagtattttctaaaccgcactcataatttgcagtcattttgaaaaggaagtcattatgtcgttctggaaagttgcagcagcgcaatatgagcctcgtaaaacctcactcaccgaacaggtagctcatcatctggagtttgtgagggccgccgccaggcaacaatgtcagctgttagtttttccatcgctttctttactggggtgtgattattcgcgacgtgcccttcctgccccacccgatctctcactgttagacccgctttgttatgccgcaacgacctggcgaatgaccatcattgccggccttcccgttgaatataacgatcgctttattcgtggaattgcggtgttcgcaccgtggcgaaaaacgcctgggatctaccatcagagtcatggtgcatgtctgggccgtcgttccagaaccatcacggtggtcgatgaacaaccgcaaggtatggatatggacccgacctgttcactgtttactacagggcaatgtctgggagaacccgacctgctggcgtcggcccgtcgcttacaatttttttcacatcagtactcgattgccgtgctgatggcaaatgcccgtggtaacagtgcactatgggatgaatatggtcgtctcatcgttcgcgccgatcgtggttcattattgttagtcggtcagcgttcatcacagggttggcaaggcgatatcattccattacgctaggctttttcggcctggagcatgccatgttgcgcattatcgatacagaaacctgcggtttgcagggagggatcgttgagattgcctctgttgatgtcattgacggaaaaatcgtcaaccccatgagccacctggtgcgccccgatcgtcctattagtccacaagcgatggcgattcatcgcatcaccgaagccatggtcgccgataaaccgtggattgaagatgtgatcccacactattacggtagtgaatggtatgtcgcgcataacgccagctttgaccgccgcgtactgcctgagatgcccggtgagtggatttgcactatgaaactggcccgtcgtttgtggcctgggatcaagtacagcaatatggcgttatataaaacacgcaagctcaatgtacagacgccgccgggcctgcatcatcaccgcgcgttgtatgactgttatatcaccgccgcgttgcttatcgatattatgaacacctccggctggacggcagaacagatggccgatatcaccggacgtccgtcgttgatgacgaccttcacctttggcaaataccgtggcaaagcggtttccgacgttgccgaacgcgatccgggctatctgcgctggttatttaataacctggacagcatgagcccggagctgcgtttaacactgaaacattatctggaaaatacttagtccgcaggcgtagcgggtaatgttccctgcgccagcgcgaccagaaaagcatattccatcgctacgccttcgtacgatttaaagcgaccagatttaccgccatggcctgagtccatgtcggtacagagcaataaaagatggtcatcggttttcagctcgcgcaatttagcgacccattttgccggttcccaatattgcacctgagaatcgtgcaaaccggtcgttaccagtaaatgcggataagcctgtgcggtgacgttgtcatacgggctgtagcttttcatgtactcgtaatattgcggatcctgcgggttaccccactcttcaaactcaccagtggtaagaggaattgattcatcaagcatcgttgttacaacatcaacaaacggtacctgggcgataacgccgtggaataattccgggcgttgattaattgcaacgcccatcaacatgccccccgcactcccgcccatcgcataacaaagcgaaggagagccatagcccagttttaacaatgcatcgcaggcatcaagataatcattaaacgtatttttcttcttcagaaattttccgtcttcgtaccattgttgccccagctcaccaccgccgcgaacatggacaatggcgtagacaaagccacgatctaacaaactcaagcggctaaaactgaaatcggcatcaatacttgcgccgtaagaaccatagccatacaccagcaacgggttgtgtcctttgcgaaaatgtttgcgatggtagaccaacgaaaccggaacttcgacgccatcacgggcgactatccacaggtgttcactgcggtaattcgccgcataaaaaccaggaacttccgtttgttttaatacacgacgctcaccggtatccatatccagttcaaacaaagtgtctggtgtagtcatggaagaataaccataacgcaatcgcgcggtttcaggttctggattgtaggcaatccaggtcacataggccggatcatcaaaggcaataccaatgacttcccgggtcttgcggttaatttggcgcaaactggttaacccgcgctgacgctcttcaaccaccagccagtcggtaaacagcgtaaacccttccagcatgatgttttcgcgtggcggaattaactcttcccactgttgctcatcacgcatacgggtacggtataagccaaagtttttgccgtggcggttggaacgcagataaaaacgatgctggtagtgatcaaggctgtattcgtgatctttgcggcgcggcagaaaaacaaacggctcggcatcggccatttccgcgtccagcaggcgaacttcactggtggtggcgctggccaaatgaatgactacatagtgcttcgaggtcgttttatgcaggctgacgtaataggtatcgtctttttcttcgtagatcagtttatcttgcgatgctggcgtaccgatggcgtgacgccagacctgataaggcagcagcgtcaccggatgcttgcgaacatagtagaaaatccaggagtcatttgcccagacaaagctgggttcaacgttatccagcagttccgggtaccagttaccagtttccagattacgaaaacgaatgccgtactggcgtcgggaaagaaaatcttctgccagcgccataatggtgttatcgggcgtaatcgccattccgcccatcgaataaaactcactatgagctgcgcgcttattggcatcgagcaatgtttcccactcatcccactcttcactgaatgccgattgacgctggtagatagcatattcacagcctggttcataaatatgccgatagcggtagccatttttgatgtagggcgcagaaacttctcgttgcggaatgcggtcgatgatttcctttaagatgcgatcctgcaaggcttgttgtgaggccatcacccgatgaccgtaactattttcttgttgcaggtagtccaggacttctggctgagaacgcgtatcgtcccgcagccagtagtaattatcgatgcgcgtatcgccatgaagcgtcatggcgtggggaatgcgggcggcttttggtagcatgttattgttctttctggttgaaacatcttataagggtggcaaaactcaccggggatgcaagcgaaacaggggagtcattgcttagatgatgacaggtaatggcgcggatatcgaatgttatgcagacagagaaaatcagcctgttcaaatggctgtgcgattctggatagcccgaaatagtcaacttcaggctatccagagagcggaattattccgccaaagtgcgtttttgctgttcgagatcgcgttcaatgccgtcacgaacatcctgggggattttcagcgcgtcacccagtgcattcaggtaactgcgttccataaaatggtcaatatcaatagccgcgcaactcaggaaatagatttccagcgcctcttcttcattgcggaccccggtagccaggcgttgtggatccagcggttgttcgattgcctgctcaatgagtacacgcccctgctcttccacgccggctccacgcaattgctggtcgattgccgcacgttctttggcatcaatatgaccatcacttttagcggcaaagaccagcgcaaggatcaaacgtgctgtacgctcatccagcggcgtactttgcgcgccaaactgcggttcgtcctgatgcgccgcgcgaattttatctttgtatttattccacagcaccgtacccgctaccgctccgccgccaaccagtaacgcgttggtgccatatttcgtaagaagtttacgtgctgatttatttgcgaccagcagcccagccagtccgcctaatgcgcctggcactaacagtttgaccaatccctgatccgcagacgaggaggtagaagaactgctttgcccaagcagggattgcagttgatttaaccagttagccatatttgctcctcaataaccatttttagtgcctgtagcatagcggatgaggatgtcagaaaatgtatatcgagacaaaagatgcgcaaataagcggggcggtaggccgttattcaaagaaattcgcgccaggtaaggtatttactgtatatcaggtgataagggtattttaggtgaaagtagtttgtcgttttgagtggcattgtttgatgctgattgcccgatgcgacgctgttgcgtcttctcaggcctacgattgtggtgcgttctggggcggacaaggcactcgcgccgcatccgccaacagtcaatcgaattatcagaagccattaacgccgctgatattccgccattcccgctttgcagtccacgctgacctggtaatgaatatcggcacttttaccacgcacggttagcggtactgaccatttatcatctttaccctgaatgtcctgcaaactgacccaagccacgggatcggcctgaccgacaattttttgatcatctgcccaacgcgccacgcgattttgttgataatcacgttttacgctcgcggcaattccggcagcatccagatcttcacactttgggaaagtgaccgacttgctggtttcattattggcagcgaaaactgatgcgcaggcagaaaccaacaacagccctaaaaacgcccctctttttttcatgtttttctccatagcacaatgattcaggagaaagcatggtacaaattgtcaggagcgcaagttgcttcaggccgcgtgtgaggcatcttcctcttcggattcagcaccgacgacctgtggggacggtaatttgccggttttcagaatggtgctcagcacatctttttgttctgccagccatagcgaaagggcttcacgttgctcgtcttccatttgcactggagaatttgtcagccaggtgtcaagcagatccgccgtatcaagcattttgtcataagcatcggcttcctttttgctggtaaacgacattttctcttcgccctcacgaatgactacgtatttaacttcaaccgccatttgcagcctctcataataactgtgattttatacagtatatttcttttcggttgagaaatcaacatcagcaataaagacacacgcaaacgttttcgtttatactgcgcgcggaattaatcaggggatattcgttatgacgttattaggcactgcgctgcgtccggcagcaactcgcgtgatgttattaggctccggtgaactgggtaaagaagtggcaatcgagtgtcagcgtctcggcgtagaggtgattgccgtcgatcgctatgccgacgcaccagccatgcatgtcgcgcatcgctcccatgtcattaatatgcttgatggtgatgcattacgccgtgtggttgaactggaaaaaccacattatatcgtgccggagatcgaagctattgccaccgatatgctgatccaacttgaagaggaaggactgaatgttgtcccctgcgctcgcgcaacgaaattaacgatgaatcgcgagggtatccgtcgcctggcggcagaagagctgcagctgcccacttccacttatcgttttgccgatagcgaaagccttttccgcgaggcggttgctgacattggctatccctgcattgtaaaaccggtgatgagctcttccggcaaggggcagacgtttattcgttctgcagagcaacttgctcaggcatggaagtacgctcagcaaggcggtcgcgccggagcgggccgcgtaattgttgaaggcgtcgttaagtttgacttcgaaattaccctgctaaccgtcagcgcggtggatggcgtccatttctgtgcaccagtaggtcatcgccaggaagatggcgactaccgtgaatcctggcaaccacagcaaatgagcccgcttgcccttgaacgtgcgcaggagattgcccgtaaagtggtgctggcactgggcggttatgggttgtttggtgtcgagctatttgtctgtggtgatgaggtgattttcagtgaggtctcccctcgtccacatgataccgggatggtgacgttaatttctcaagatctctcagagtttgccctgcatgtacgtgccttcctcggacttccggttggcgggatccgtcagtatggtcctgcagcttctgccgttattctgccacaactgaccagtcagaatgtcacgtttgataatgtgcagaatgccgtaggcgcagatttgcagattcgtttatttggtaagccggaaattgatggcagccgtcgtctgggggtggcactggctactgcagagagtgttgttgacgccattgaacgcgcgaagcacgccgccggacaggtaaaagtacagggttaaacccggcaaaaaaacgctacaaaaatgcccgatcctcgatcgggcattttgacttttacagcttagcgccttctacagcttcacgcgccagcttagtaatgcggtcgtaatcgcccgcttccagcgcatctgccggaaccagccaggaaccaccgatgcacagcacgcttttcagcgccaggtagtcacggtagttagccggagaaataccacccgtcgggcagaaacggacctgggagaacggacccgcgatcgcctgcagggctttcacgccgccgttagcttcagccgggaagaatttgaactctttcaaaccgtagtccatacccagcatcagttcggaaacagtgctgatccccggaatcagaggaatagtcccttcggtagcagctttcagcagcggctcggtcagacccgggctaattgcgaactgtgcacccgcttcagtgacttctgccagctgctgtggattcagcaccgtaccggcacccacaatcgcttcaggcacttctttggcgatagcacggatagcgtcaactgcacactcggtacgcagagtcacttccagaacgcgcaccccaccagcaaccaacgcttttgccatcggcaccgcgtgttccagtttttttaccacgataaccggtacaaccgggccggtggtcaggattgattctgcacttgttttccagtttttcatcagagttttctctcgcctgattacaaatttgtcgtcttaaaaagtgatacaggttgcgccctgttcggcaccggacagtttttcacgcaaggcgctgaataattcacgtcctgttcccacgcgtgacgcgctcaggtcaggaatgtgcggttcgcgagcagccagttccgcttcgtctaccagcagcgtcagttcgcctgtctgtccattcacacgaatgatgtccccgtcgcgcacttttgccagcagcccgccatcgtaggcttctggtgttacgtggatagctgacggcactttacctgaagcgccggagagtcgtccatcggtaactaacgcaattttgaaacaccggtccaataatacaccaagtggcggcatgagtttatgtaattctggcattccgttcgcttttggcccctgatgacggacaacaacgacacaatcgcggtccagcaaacccgcttcaaaggccggcataacgtcatgctggctttcaaaaacaaccgctggcgcttcaatcacctggttctcaaccggcacggcagaggttttcataaccgcacggcccaggttaccgcttaacacttttgtcccaccatgatgagagaaaggttgttcgaaggaagcgatcacattgctgtcgagtgatttttccgccccttcccgccagtccagttcaccattattcagccatggttcaagggtataacgagacagaccaaaacctgccaccgtattgacatcttcatgcagcaggcctgctttgagcagttcacgcaccagaaccggtacgccacctgccgcctggaagtggttaatatcggccggaccgttcgggtagagacgtgccatcagcggtacaacatcagaaaggtcagagaagtcatcccagttaatctgaataccggccgcgcgcgccatcgccaccaggtgcatggtgtggttagtggaaccaccggtcgccagcagtgcaacgataccgttcaccaccactttctcatcgatcatcttaccgatcggcatccattcattaccattaccggtcatgcgtgtaacctgacgcgcagctgcggcggtcaaagcatcgcgcagcggagaatccggatgaacaaaagaagagcctggcaactgcatccccataaactccaccaccatctggttggtgttggcagtaccgtagaaagtacatgttcccggcgcatggtaagacgcggcttctgactccagtaaggccatgcggtccactttaccttcggcataaagctggcgaatacgcactttttctttatttggcaaaccgcttgccatcggtccagacggcacaaacaccgcaggcaaatgaccaaacgacagggctgccatcgtcagacccgggacaatcttgtcgcacacaccgaggaacagagcaccatcaaacatgttatgggacagccccaccgccgcagacatcgctatcacttcgcggcttagcagcgacaattccattccatcctgcccctgggtgacaccatcacacatcgccggaacaccgcccgcaacctgaccaaccgcattcgcttcatgcagggctttacgaatgatttctggatagtgttcataaggctggtgcgcggagagcatgtcgttataggaggtgatgatggcgatattgttacgcaacatgcttttcaaagaggctttgtcttctggctggcaggcagcgaaaccgtgtgccaggttaccgcatgccaactgcgaacgatgaacggtcgaagttttcgcttgttctatccgggcgagataagcagagcgagtctcgcgcgaacgttcaatgattcgatttgttacgcgtaacaattgtggattcataaaggctcctgaaattgagttgtcagagcaggatgattcacaacgcgtttcattcagaggatttatgactgaaacgcctgtaaccggagctcatagggcaaaaacgtttcagtcagtgtaataaaaaaagcctcgtgggtgaatccgcacgaggcctgaaagtgtaaaaattgttctacaatctgcgcaagatcatgttaccggtaaaataaccataaaggataagcgcagatattactcaaactcattccaggaacgaccatcacgggtaatcatcgccaccgaggcaacgggtccccaggttccggcctgatacggtttcggcgcatcattgtccatcgcccacgcctcagtaatggagtctacccatttccaggcttcttccacttcgtcgcgacgtacaaacagtgcctgaataccacgcatggtttccagcagcaaacgttcataggcatccgccagatgcgtctgattaaaggtttctgaatagctcagatccagcttggtgatttgcaggttatgtttgtggtcaaggccaggaactttattcagtacctggatatccacgccttcatcaggttgcagacggatagtcagtttattctgcggcagatcctgccacgattctttaaacagattcagttcaggtgttttgaaatagaccacgacttcagaacatttggtcggcagacgtttaccagtacgcaggtagaatggcacaccggcccagcgccagttatcaatgtcgacgcggatcgccacgaaagtttctgtattgctgctcttgttcgcgccctcttcttccagatatcccggcacttttttgccctgggcgaagcccgcagtatattgcccgcgtacggttttttcgcgtacgttggagcggtcgatgcggcgcagagacttcagtactttcactttttcatcgcggatgctgtctgcgctcaggtcagacggcggagacatcgcaatcatgcaaagaatttgcagcaggtggttctggatcatgtcgcgcatctgaccggctttatcaaaatagccccagcgcccttcgatccccacttcttctgccacggtaatctcaacatgatcaatggtgcgattgtcccagttattcacaaacagggagttagcaaaacgcagcgccaacaggttcagcaccgtttctttaccaagatagtggtcgatacggtaaacctggcactcctcgaagtattcgccaacctgatcattgatttcctgcgaggtcgccagcgacgtccccagcggtttctccatgactacgcgtgccggtttagcattcagttttgcctcgccaagccctttgcaaattgcgccaaaagtgctgggcggcatggcaaagtagttaatggtgatacgatttttttgatccagcatcgcgccgagacggctgaatgcagcagtgtcattgacatcgagattacaaaaatccagacgtgcactcagggtgtcccataaaccttcatcaatggtttctttcatgaaagtttcgagcgcctcgcggacaactttggtatatgccgctttatcccagtcagcacgccctacgccgataatccgggtgtccgggttgagctgaccggctttttccagttgatacagggaaggcagcaatttacgacgcgcaaggtcgcctttcgcgccgaaaatgaccaggtcacaggcctgggctgtttgcgttaccgccatgtcattctccttaagttaactaacccggtacttaagccagggtatacttgtaattttcttacggtgcactgtactgcttttacgagcttgcgaaaactgtaaacgcttatccacccgtgcgattacgggaaaagcgcgcaaagtgcggcaaaactgataaaaaaatcatcgttttccattgggtaaaaatctgacactgatcatgttatgaaaaaaaataacaacttttttatctgcttttgtcattaacacggcacacaggcgtaatatctgacaaaactgcatttcgatttctttcagtgcggaaatcgtcattacccgtgagtctctttacatcatgaatatgctggaaaaaatccagtctcagctggaacatttgagcaaatcagagcgcaaagttgccgaggtcattctggcttcgcccgataacgcgatccattcgagtattgctgctatggcactggaagccaatgttagcgaaccgacggtgaatcgtttctgtcgcagcatggacacgcgcggttttcctgattttaaacttcatctggcacagagtctggcgaatggcactccctatgttaatcgcaatgtcaatgaagatgacagcgttgaatcatacacagggaaaatatttgagtccgcaatggcaacgcttgatcatgtccgtcattcactggataaatctgccatcaaccgcgccgtcgacttgctcactcaggcaaaaaaaatcgcctttttcggattaggctcttcagccgccgttgcccacgatgcgatgaataagttctttcgttttaatgttccggtggtgtactccgatgatatcgtgctgcaacgcatgagttgtatgaattgtagcgacggagacgtggtggtgctgatttctcacactggaagaacaaaaaatctggtcgagctggcgcagctggcacgcgaaaacgacgccatggtgattgccctcacctctgcgggtaccccgctcgcccgggaagcaacgctggcaattaccctcgacgtaccggaagatactgacatttatatgcccatggtttctcgacttgcacagctgaccgtgatagatgtgctggcgacaggatttactttgcgacgcggtgcaaaattcagagataacttgaagcgggtcaaagaagcgctgaaggaatcgcgttttgataagcagttacttaatttaagtgacgatcgctaaaaacgactgtcactgtcctaatcttatacgacatccgaatgagattaatttatcgccatcgcggcgttatttcattcggatttcatgttcaagcaacacctggttgtttcagtcaacggagtattacatgtccagaaggcttcgcagaacaaaaatcgttaccacgttaggcccagcaacagatcgcgataataatcttgaaaaagttatcgcggcgggtgccaacgttgtacgtatgaacttttctcacggctcgcctgaagatcacaaaatgcgcgcggataaagttcgtgagattgccgcaaaactggggcgtcatgtggctattctgggtgacctccaggggcccaaaatccgtgtatccacctttaaagaaggcaaagttttcctcaatattggggataaattcctgctcgacgccaacctgggtaaaggtgaaggcgacaaagaaaaagtcggtatcgactacaaaggcctgcctgctgacgtcgtgcctggtgacatcctgctgctggacgatggtcgcgtccagttaaaagtactggaagttcagggcatgaaagtgttcaccgaagtcaccgtcggtggtcccctctccaacaataaaggtatcaacaaacttggcggcggtttgtcggctgaagcgctgaccgaaaaagacaaagcagacattaagactgcggcgttgattggcgtagattacctggctgtctccttcccacgctgtggcgaagatctgaactatgcccgtcgcctggcacgcgatgcaggatgtgatgcgaaaattgttgccaaggttgaacgtgcggaagccgtttgcagccaggatgcaatggatgacatcatcctcgcctctgacgtggtaatggttgcacgtggcgacctcggtgtggaaattggcgacccggaactggtcggcattcagaaagcgttgatccgtcgtgcgcgtcagctaaaccgagcggtaatcacggcgacccagatgatggagtcaatgattactaacccgatgccgacgcgtgcagaagtcatggacgtagcaaacgccgttctggatggtactgacgctgtgatgctgtctgcagaaactgccgctgggcagtatccgtcagaaaccgttgcagccatggcgcgcgtttgcctgggtgcggaaaaaatcccgagcatcaacgtttctaaacaccgtctggacgttcagttcgacaatgtggaagaagctattgccatgtcagcaatgtacgcagctaaccacctgaaaggcgttacggcgatcatcaccatgaccgaatcgggtcgtaccgcgctgatgacctcccgtatcagctctggtctgccaattttcgccatgtcgcgccatgaacgtacgctgaacctgactgctctctatcgtggcgttacgccggtgcactttgatagcgctaatgacggcgtagcagctgccagcgaagcggttaatctgctgcgcgataaaggttacttgatgtctggtgacctggtgattgtcacccagggcgacgtgatgagtaccgtgggttctactaataccacgcgtattttaacggtagagtaagtacgttgccggatgcggcgaaaacgccacatccggcctacagttcaatgatagttcaacagatttcgaatattctgaagcaaacttgaacttatcatcaggcgaaggcctctcctcgcgagaggcttttttatttgatgggataaagatctttgcgcttatacggctggatttcgcccggtttgcgagttttcagcaattttagtatccaggtgtattgttctggtcgcggaccaacaaaaatctcgacttcttcattcatccgccgcgcaatcgtatgatcatccgcctctaacagatcatccatcggtgggcgcacctgaatcgtcagacgatgcgtcttgccatcataaatcggaaacagcggtacaacgcgcgcacggcacactttcatcaaacgaccaatcgcgggcaacgtcgctttataggtggcaaagaaatccacaaattcgctgtgctctgggccatgatcctgatcgggtaaataatatccccagtacccctgacgtaccgactggatgaatggtttaataccgtcatttctcgcatgcagacgaccgccaaagcgacgacgcaccgtgttccagacataatcaaaaaccgggttgccctgattatggaacatcgctgccattttctgcccttgcgaggccatcagcatggcaggaatatcgacggcccaaccgtgcggcaccagaaagataactttctcgttattacgccgcatctcttcgatgatctccagcccttgccagtcaacgcgcggctgaattttctccggcccgcgtattgccaactcagccatcattgccatcgcttgcggcgcggtggcaaacatctcatcaacaatcgcttcgcgttcagcttcactacgttctggaaagcagagcgacagattgattaacgcacgacggcgtgagctttttcccagtcgtccggcaaaacgtcccagccgtgccagaatgggatcacggaactttggcggcgttaaagcgatacccgccatcgctgctacgcccagccatgctccccagtagcgcgggtggcgaaaggatttatcaaactcaggaatgtattcgctattattttttttcgtttccatgcttttccagtttcggataaggcaaaaatcaatctggtgatagtgtagcggcgcaacttgccccgcaccaaataaaaaaagccggtactgactgcgtaccggctgcgaatggatgttaattaatcaaaccgtagctgcggcacaatctctttggcctgcgccaggaattcgcgacgatcggagccggtcagcccttcggtacgcggcagttttgccgtcagcgggtttacggcctgctggtttatccatacttcatagtgcagatgcggcccggttgaacgtccggtattaccggaaagcgcgatacggtcgccacgtttcaccttctgtcccggtttcaccagaatcttgcgcaagtgcatataacgcgtggtgtagctgcgaccatgacgaatagccacataataacctgctgcgccactgcgtttggcaaccaccacttcaccgtcacccactgaaagcactggcgtaccctgcggcatggcgaaatcaacacctctgtgtggtgcaacgcgaccggtcaccggattagtacgacgcgggttaaaattagacgagatacggaactgtttcgccgtcgggaatcgcaagaatcctttcgccagaccagtaccgttacgatcgtagaatttgccatcttcagcgcggatagcgtaataatctttaccttctgaacgcaaacgtacgcccagcagctggctttgctcacgtttaccatcaagcatttctcgagacattaacaccgcaaattcatcgccttttttcagtttgcggaaatccatttgccactgcatggctttaatcactgcgctcacttcggcgctggttaaaccggcgtttctggcgctggcaacaaagcttcccccgacggtacctttcagcagattgttaacccactctccttgctgcatttcgctggtcattttaaaaccgttagcggcagtacggtcataggttcgggtttcacgacgagacacttcccaggtgaggcgctgcagttcgccgtccgcggttaatgtccaggagagttgttgaccgattttcaggttacgcaattctttgtcggccgcagccagttgggtgatatcacccatatcaataccatactgattgagaatgctgcttagcgtatcgccagtggaaacaacatattcatgcacgcccgcttcaccggcgattttgtcatccagttcgtcctggggaatggcttcatcttcttgtgcagcttgatcaatcggctcactggcttcaggtaagagcgaacgaatttcgttctgttccagctcaatggttttgacaattggcgtggcatcacggtgataaacataaggccgccagacagcgacggccagagtaagaacggtgagcgaccccaacataacgcggtgtggtcgcggtaaattattaaacgccagggcgacagagcgggctatctgttgcacgtaatcacttcctcattaatctcctttcaggcagctcgcatactggttggctaattgactcaggaattctgaatagcttgttttacccagtttgatattcgtccccaggggatccaacgttcccatacgaacggatgtccctcgtgcgacgctctcaacgaccgctggcctgaactgtggctcagcaaaaacgcaggttgctttttgctcaaccaactgtgttcttatttcatgtaaacgctgcgcgccaggttgaatctcagggttaacggtaaaatgaccaagcggtgtcagtccaaactgtttttcgaaatagccgtaagcatcgtgaaaaacgaaataacctttccccttgagcggcgcgagctcgttaccaacctgcgtttcggttgaggctaattgtgcctcaaaatccttcaggttggcgtcaagtttggctcgactttgcggcataagttccactaattttccatggattgcaaccgctgtagcccgcgctatctctggggaaagccaaagatgcatgttgaaatcgccgtgatggtgatcttcgtcacttttttccgcgtggtcgtgatcatcatcatcgccgtgaatacttttcatcagtagcggtttcacatcttcaagctgcgcaatcgttacctgcttcgctcctggtaatttgcttaccggtttttgcataaacgcttccatctccgggccaacccaaacgactaagtccgcgttctgtaagcgttttacatccgatgggcgcagtgaataatcatgttctgaagcgccgtcaggaagtaaaacctctgtttctgttaccccatcagcaatggcagaagcgatgaacccaacgggtttaagcgaagcgacaacggcggcatctgcggcctgtgttgcacctccccagagagcggcggataatgctgcgaaaagaagcgtttttttatgtaacataatgcgaccaataatcgtaatgaatatgagaagtgtgatattataacatttcatgactactgcaagactaaaattaacatgacaagtctggtttccctggaaaatgtctcggtttcttttggccaacgccgcgtcctctctgatgtgtcgctggaacttaaacctggaaaaattttgactttacttgggccaaatggcgcaggtaagtcgacactggtacgggtagtgctcgggctggtaacacccgatgaaggggttatcaagcgcaacggaaaactgcgcatcggctatgtaccgcagaagctgtatctcgacaccacgttgccactgaccgtaaaccgttttttacgcttacgccctggtacacataaagaagatattttgcctgcactgaaacgtgtccaggccgggcacctgattaacgcaccgatgcaaaagctctctggtggcgaaacgcagcgtgtactattagcgcgagcattgttaaatcgcccgcaattattagtgctggatgaacccactcaaggcgtggatgtaaatggccaggtggcgttatatgaccttattgaccaactgcgtcgtgaactggattgtggcgttttaatggtttctcacgatctgcatctggtgatggcaaaaaccgatgaagtgctgtgcctgaatcaccacatttgttgttccggcacaccggaagttgtttccctgcatccggagtttatttcaatgtttggtcctcgtggtgctgaacaactgggtatctatcgccatcatcataaccatcgtcacgatttacagggacgaattgttttgcgtcggggaaatgatcgctcatgattgaattattatttcccggttggttagccgggatcatgctcgcctgtgccgcgggtccgctgggttcgtttgtagtctggcgtcgtatgtcttatttcggtgatacgctggctcatgcctcattacttggcgtcgcgtttggtttgttgctggacgtgaatccattctatgcggtgattgccgttacgctgctgctggcgggcggtctggtatggctggagaagcgtccacagctggcgatcgacacgttattagggattatggcgcacagtgccctgtcgctgggcctggtggtcgtgagtctgatgtctaatattcgtgttgatttgatggcttacctgttcggtgatttgctggcagtgacgccagaagatctcatctctattgcgattggcgtggtcatcgtggtggctattttgttctggcaatggcgcaatttgctgtcaatgacgataagcccggatctggcgtttgttgatggtgtgaaattacagcgagtgaaattgttgttgatgctggtgacggcattgacgattggtgtagcgatgaaatttgtcggtgcgttgattattacttcgttgctgattattcctgctgctactgcgcgtcgctttgcccgcacgccggaacagatggctggtgtcgctgttttggtggggatggtggcagtgactggcggtttaaccttttccgcggtttacgatacgccggcgggtccgtcggtggtgctatgtgcggcactgttatttattctcagtatgatgaaaaagcaggccagctaatctatcgctgaacacatttgtcggatgcggcgcgagcgccttatccgacctacggttcggtatctctggtagtcctggtaagacgcgaacagcgtcgcatcaggcatattgccagtgccggatgcggcgcgagcgaccaatccgacttacggcatttctggcggcgttatgccaaagtgattccacgcccgcgtcgtcgccatacgcccacgcggtgtacgctgcaaaaagccttgctgaatcaaataaggttccagcacatcctcaatggtttcacgttcttcgccaatggctgccgccaggttatccagacctacaggtccaccaaagaacttatcgattaccgccagcaacaatttgcggtccatataatcgaaaccttcagcatcgacattcaacatatccagcgcctgagcagcgatatctgccgagatggtgccatcgtgcttcacttcggcgaaatcacgcactcgacgcagcagacggttggcaatgcgcggcgtaccgcgagcgcgacgagcaacttccagcgcgccgtcatcactcatctcaagccccataaagcgtgcgctgcgactgacgatatattgcagatccggcacctgataaaactccagacgttgcacaataccaaaacggtcgcgcaacggtgatgtcagcgaacctgcgcgcgtggttgcaccaatcagggtaaacggcggcaaatcaattttaatggagcgtgccgccggaccttcaccaatcatgatatccagttggtagtcttccattgccgggtacagcacttcttcaacaactggcgatagacggtggatctcatcaataaacagcacgtcatgcggttcaaggttagtgagcatcgcagccaaatcgcccgccttttccagcaccggaccagaagtcgtgcgtaaattaacgcccatttcattggcgacaatgttggcaagcgtagttttacccaaccccggaggaccaaaaatcaacaaatgatcgagggcatcgccgcgcagtttcgctgctttgatgaaaatctccatctgtgaacgaacctgcggctgaccaacatactcttccagtaatttggggcgaatggcgcgatctgctacatcttccggcaaagtggtaccggcagaaatcagacggtctgcttcaatcatcctttacctcataacgcggcgcgtagggcttcgcgaattaaagtttcactgctggcgtcagggcgagcgattttgctcaccatgcggcttgcttcttgtggtttatagcccagcgccaccagcgcggcaaccgcttcttgttcagcatcgtcggtcgccgggctggcaggagacgtgagtaccaggtcggcggctggcgtaaagagatcgccatgcaaacctttaaatcggtctttcatttcaacaatcaagcgttcggcggtttttttgccaatacccggcagtttcaccagtgcccccacttcttcacgctcaacggcattaacgaactgctgcgctgacattccggagaggatcgccagcgccaacttcgggccgacgccgttggttttgatcaactctttgaacaatgtgcgctcttgtttattgttaaaaccgtacagcagttgcgcgtcttcacgcaccacaaagtgggtgaaaacgatcgcttcctgacccgcttcagggagttcataaaaacaggtcatcggcatatgcacttcatagcctacgccgcccacttcaattaacaccagcgggggttgtttttcaatgatgatgcctctgagtctgcctatcacatgacgctcctgcgtaatgaatcaaagataatgctgtatgataaaaaaatgctggatagatatccagcgaaggatgaagaaaacttgcgaggtgtctcgatgaactgaaaaatggcacagtataatttattctacaggttatattggaagcaaatattttaatattacatattcagtgaagaaatgcgtaataaaaatatacattgcgcctcctgaaaaaataaattttttatgctattacgtatatttgtatctatttcaatggaatgacaacgtgaatattaattaccctgctgaatatgaaattggagatatcgtctttacatgtataggtgctgccttatttggtcaaatatcagctgcatcaaattgctggagtaatcacgtcgggatcattatcggtcataacggtgaagacttcctggttgcagaaagccgggttcccctttcaaccatcaccacgctatctcgttttattaaacgttcgtctaatcaacgctatgctataaagcgattagacgctgggctgacagaacgacaaaaacaacgaattgttgaacaggttccctcccggctacgcaaactttaccacaccggttttaaatacgaatcttcgcgccagttctgttcaaaatttgtttttgatatttataaagaagcgctatgtattccggtgggtgaaatagagacgtttggagaattgttaaatagcaatccgaatgcaaaactcactttctggaaattctggttcctgggttctattccgtgggagcgtaaaaccgtcacgccagccagtttgtggcatcatccgggtttggtgttgattcatgcggagggagtggaaacgcctcagccggaactgaccgaggcggtataacttaacgcagtcgccctctcgccaggttcagccgcgattcgctcatctgcatcgcattctgactaacgtggcagtgggtgatagcaatcgccagcgcatcggcggcatccgcctgtggattagcgggcagtttcagcaaggtgcggaccatatgctgcacctggcttttttcggcactgccaatacctaccaccgtttgctttacctgacgtgccgcgtattcaaatactggcaactcctgattcaccgccgccacaatcgccacgccgcgcgcctggcccagtttcagggctgagtcagcgttctttgccataaagacttgttcaatggcgaaataatcaggctggaactgggtgatgatttccgtcacgcccgcatagatgagtttcagacgagacggtaaatcatccactttggtgcggatgcatccgctacccaggtaggacagttgcctacctacctggcggatgacgccgtagccggtcacgcgcgaacccggatcaatgccgagaataatagccatcacgcgtctccgttttgctgtttagcaggcctcatcagagagtcgctgcgacctcatcagagatttcaccgttatggtaaacttcctgcacgtcgtcgcaatcttccagcatatcgatcagacgcatcagtttcggtgcggtttctgcatccatatcagctttggtagacgggatcatggaaacttccgcgctgtctgctttcagacctgccgcttccagagcgtcgcgcactttacccatttcttcccatgcagtgtagacatcaatcgcgccgtcatcataggtcacaacgtcttcagcacctgcttccagtgctgcttccatgatggtgtcttcatcgcctttctcgaaggagatcacgccttttttgctgaacagataggcaacggaaccatcagtaccgaggttaccgccacatttgctaaatgcatgacgcacttcagcaacggtacggttgcggttgtcagacagacattcaatcatgattgccgtgccgccaggaccgtaaccttcgtagatgatggtttccatgtttgcatcatcatcaccgcccacaccacgtgcaattgcgcggttcagtgtgtcacgggtcatgttgttagacagtgctttatccaccgccgcacgcagacgcgggttagcgtccggatcgccaccgcccagcttagccgcggttaccagctcacgaatgattttagtgaagattttaccgcgcttagcatcctgcgcagctttacgatgtctggtgttggcccatttactatgacctgccataaaaatatctccagatagccctgcctgttcaggcagcgttaattacaaactgttcaatcgcctgccggttgctccaggacttagtgagcgccgccgcagcaggcgcatcaagccacttgtaagccagatgttcagtgaaaacgatctgccgctcgtgcggaagcgcaagacagaaccatgattccgtattacgcgtcacgcccggcgcatagcgatgacgtaaatgtgaaaaaatttcaaactctaccgtgcgctgacagtcaattaaggtcagttgttcagcgacaacatcaatggtgacctcttcctttacttcgcgcatggcagcttgcggcgcggtttcaccctcttccacgctgccggttaccgactgccagaaatcgggatcgtcacgccgctgcaacatcagcacccgtttcgtatcttgtgcgtagatgaccactaagatcgaaacgggacgcttatacactttatccttcacgctgcctcttcgttgactgccttcgctcatcccattcacatagttatctatgctcatgggagttcactcagttgccgcctcgatgcaacgcgaatgatttcgtgtatttgagtcatatcagttattctcagccttcttcacaacctgaatgctcagctcagccagtgcagtcgggttagcaaagctcggtgcttcagtcatcagacacgctgccgccgtggttttcgggaaggcgataacgtcacggatattgtcggtgccggtcagcagcatggtcagacggtcaagaccgaatgccagacctgcgtgcggcggagtaccgtatttcagagcgtcgagcaggaagccgaatttctcgcgctgttcctcttcgttgatacccagaataccaaacaccgtctgctgcatatcaccattatggatacgtactgaaccaccgcccacttcgtaaccattgatgaccatatcgtaagcgttcgccaccgcattttccggtgcagctttcagttctgcagccgtcatatctttcggtgaggtgaacggatggtgcattgccgtcaggccgccttcaccgtcgtcttcaaacatcgggaagtcgataacccacagcggtgcccatttgctttcgtcggtcagaccaaggtctttacccactttcaggcgcagtgcacccatcgcgtcggcaacaattttcttgttgtcggcaccgaagaaaatcatatcgccatcttgcgcggcagtacgatccaggatgtcttcgatgatttctgcattaaggaacttcgctaccgggctgttgataccttccagacctttcgcgcgttcgttaactttgatgtaagccagacctttcgcgccgtagattttaacgaagttaccgtattcgtcgatctgcttacgggtcagcgatgcgccgcccggaacgcgcagagccgctacgcgacctttcggatcgttcgccggacctgcaaatacagcaaactcaacagatttcagcagatcagcaacgtcagtcagttccatcgggttacgcagatccggtttatcagaaccataacggcgttctgcttccgcaaaggtcattaccgggaaatcgcccagatccacacccttcacttccagccacagatgacgcaccagcgcttccatcacttcacgcacttgcggcgcggtcatgaaagaagtttccacatcgatctgagtaaattcaggctgacggtcagcacgcaggtcttcgtcacggaagcatttaacgatctgatagtaacggtcaaaaccggacatcatcagcagctgtttgaacaactgcggggattgcggcagtgcgtagaatttacctttgtgcacacgagaaggcaccaggtagtcacgcgcgccttccggcgtggctttggtcagcatcggagtttcgatgtcgaggaagccgtggtcatccataaaacggcgcaccaggctggtgattttagcgcgggttttcaggcgctgagccatttccggacgacgcaggtcgaggtagcggtatttcagacgcgcttcttcggtgttgacgtggttagagtcaagcggcagaacatctgcgcggttgatgatagtcagcgaggacgccagcacttcgatttcgccggtcgccatatcgcggttaatatttttttcgtcacgcgcacgtacggtgcccgtgacctgaatgcagaactcattacgcagttcagaggccagctttaacgcgtccgcacgatccggatcgaaaaatacctgcacgataccttcgcggtcgcgcatatcgatgaagatcaggctaccaagatcacgacgacggttgacccaaccacacagagtcacctgctgccccacgtgggacaaacggagctgtccacaatattctgtacgcatgagatatcccttaacttagctgccggcggatgccccctgctgcgcaggtgaccaagtcgcagcgttagctgtatgtcacaactgaatgaaaaaaggcggctattatactggaaattctgccgcaccgtaagagcctggcccgcgctggaacgcctcgttaccactttatatcgggcctgaaatcagactctacgccagtttgctataaaggtgttgcccgaactcataaaaattaacaaaatttgtcgttccgccatcggctaatcgcattaaggtgtgaggcacgattttgttttttcaggagtcattatgcttgaacttaatgctaaaaccactgcgctggtggtgatcgatttacaagaaggcatcttaccttttgccggtggtccacatactgccgatgaggtagttaatcgcgccgggaagctggcggcgaaatttcgcgccagcggtcagcccgtgtttctggtgcgcgttggctggtctgccgattacgctgaagcattaaaacagccggtcgatgcgccctcaccggctaaagtgttgcccgaaaattggtggcaacatcctgctgcattaggtgcaaccgacagcgatatcgaaatcatcaaacgtcaatggggtgcgttttacggtacggatctggagttgcaattacgccgccgaggtatcgatacaatagtgttatgtgggatctcgaccaatatcggtgttgaatccaccgcccgcaatgcctgggaacttggctttaatctggtgattgccgaagacgcctgtagtgccgccagcgccgagcagcacaataacagtatcaaccatatctacccgcgcatcgcccgtgtgcgtagcgtggaagagatcctcaacgcgttatgatttacatcggtctaccgcaatggtcgcatcctaaatgggtgcggttggggatcaccagccttgaagagtatgcccgccactttaactgcgtggagggcaacaccacgctttacgccctgccgaaacccgaggttgtcctgcgctggcgtgagcagaccacagatgacttccgcttctgttttaagtttccggcgaccatttcgcatcaggcagcattacggcattgcgatgatttagtgactgaatttttgacccgcatgtcaccgttggctccgcgcattgggcaatactggctgcaactgcctgccacattcggcccacgggagctgcctgcgctttggcattttctcgattctcttcctggcgaatttaattatggcgtggaagtccgccatccacagtttttcgccaaaggagaagaggaacaaacgcttaatcgcggtttacatcagcgcggcgttaatcgggtgattttagacagccgcccggttcatgcagcacgtccacacagtgaagctattcgcgacgctcaacgaaaaaaacctaaagttccggtacatgctgtactgacggcgacaaatccgctgatccgttttatcggtagtgatgatatgacgcaaaaccgggaattatttcaggtctggttacaaaaattagcgcagtggcatcagaccactacgccttatctttttttacatacgccagacattgcccaggcaccggaactggtacataccctgtgggaagacttacgtaaaacgcttccagagatcggagcagttccggctattccacagcaatcttctcttttctgaatttgccacctatcatagacaggtgccatcggccattttaaagggagtttgtatggtaagcgcgctgtacgccgttttaagtgcgttgttattaatgaagttctcttttgatgtcgttcgcctgcgaatgcagtaccgcgttgcctatggcgacggcggttttagcgaactgcaaagcgctattcgcattcatggtaacgcggtggaatatattcccatcgcgattgtgctgatgctgtttatggaaatgaatggcgcagaaacctggatggtgcatatttgcggcatcgttttgcttgctggtcgtctgatgcattattacggttttcatcaccgtctgttccgctggcgacgttccggcatgagcgccacctggtgtgcgctgttgctgatggtgctggcgaatctttggtatatgccctgggagttggttttctccctgcgttagcgcacaatacgccactttctttttcccggatttttacgttatgtctcaccgcgacacgctattttctgcccctatcgccagactgggcgactggacctttgatgaacgggtagctgaagtcttcccggatatgatccagcgttccgtacccggctattccaatattatttccatgattggtatgttagccgagcgcttcgttcaacctggtacgcaggtttacgatctgggttgttctctgggcgcggcgacgctctcggtgcgtcgcaacattcatcatgataattgcaaaattattgccatcgacaactccccggcgatgattgaacgctgccgtcgtcatattgacgcctataaagcccctacgccagtagacgtcattgaaggtgatattcgcgatatcgccattgaaaacgcatcgatggtggtgctgaattttaccctgcaattcctggaaccttccgagcgccaggcgttactggataaaatttatcaagggctgaaccccggcggcgcgctggtgctttcggaaaaattcagtttcgaagatgccaaagttggtgaactgttgttcaacatgcaccacgactttaaacgtgccaacggttacagcgaactggagatcagccagaagcgcagcatgctggaaaacgtgatgctgaccgattccgtggaaacccataaagcacgcctgcataacgccggttttgagcatagtgagctgtggttccagtgctttaactttggttcactggtggcattaaaagcagaggacgctgcatgatcgactttggtaacttttattctctgattgccaaaaatcatctttcacactggctcgaaacgctgcccgcgcagattgctaactggcagcgcgagcagcagcacgggttgtttaagcagtggtcaaatgcggtggagtttctacctgaaattaaaccgtatcgtcttgatttattgcatagcgttacggcagaaagcgaagagccactgagcgcagggcaaattaaacgcattgaaacgctgatgcgcaacctgatgccgtggcgcaaagggccgttctcactgtatggcgtcaacatcgataccgaatggcgttccgactggaaatgggatcgtgttctgccccatctttctgatttaaccggacgcaccattctggatgtcggctgcggcagcggttatcacatgtggcgcatgattggcgcaggcgcgcacctcgcggtggggatcgaccctacgcaactgtttctgtgccagtttgaagcggtgcgtaaactactgggtaatgatcagcgcgcgcatttgttaccgttaggtattgaacaacttccggcactgaaagcctttgataccgtcttttcgatgggcgtgctttaccatcgccgttcaccgctggagcatctatggcagttgaaagatcaactggtcaatgaaggtgaactggtgctggaaacgctggttattgatggtgatgagaacacggtgctggtaccaggcgatcgttacgcgcaaatgcgtaatgtctatttcatcccttccgcgctggcgctgaaaaactggctgaagaagtgtggttttgtagatatccgcattgcggatgtgagcgttaccaccacagaagagcagcgacgcaccgaatggatggttaccgaatcgctggccgatttcctcgacccacatgatccgggtaaaacggtggaaggttatccggcacctaaacgcgcggtgctgattgcgcgcaagccgtaaaggtctggtattactgccggatgcggcgtgaacgccttatccggcctacaaaaccttgctaattcaatatattgcagggactatgtaggcctgataagcatagcgcatcaggcagctttacgtttgcataacctcagcgcccgtttccgggcgctattcacgtcttacgcctgaacagctggctgatcaaacgccgttaacttcggtgcattgcccgtatatttttcgatatacaccaacgctgagttaccggcacaggcatttgccagctgcgagctggggatatccgccgttaacacgttcgcactgccgtttttacacaagccattttccagatctggccatgcaccttcatgcacgcataccacgccttttttgatcccgtcagtcaccaccgcgcctgtcaaaatctgaccacgtttgttccagacacgcaccagatcgccattcgcaataccaaagcgtgcagcatcttcggtgtgaatagtgattggttcacgatcggcgatcgcatattttttacgcagttccgcatagttaagctgactgtgtaaacggtgtgccggatgtgcggtcagaagctgtaactgcttctcgtcggcggtacctttccattcatcaggagccagccaggttgggtgtgccgggcaatccttatagccaaatttttccaacgtttttgaatagatttcaattttgccgcttggcgtacccagcgcatttttcaccggatcggcgcggaaatcaccataacgaacgtactgttcgttcttctcgctgtggcgcatttcgatcagtttattttgctgccagaaggcattaaacattggcatagtgacgcgttgcgcacgggcacctttctgagcggcatcatagaaaaatttcagccacgccatttcatctttaccttcggtatagatctcttttccgccaggtttgagtaattccgcaagatcggcaaacacgtcaaaatcgttacgcgcttcaaattgcggagcaacagcctgcttcatcggcacaatatgctggttgctgtaatcaccggtcatcgtcaagtcattgcgctcaaacgatgtggtgatcggtaatacgatatctgcgtgtttggctgctgcggtccagtagcattcagaaacgacgatcatctccggtttctgccatgctttaatcagacgattagtatcctggtgatgggtaaagttaccgccacccgcccaccagatcattttgatattcggatacgtttgttctttaccgttatgctgatatttgccgccaggattttccagcgcatcgacgatacgggcaacaggaatcgccgtcattccgccatcatcagcggcctcgctggcatgtccggcaatcgccgcagacatttccggcagcacgccgccaacacgcgtcgggttgccaccgttggagtaatgataagagaaaccaaaaccgccgcccggtgtaccaatctgccctaacatcgccgccagcgtcaccagcatccagtgtttctgttcaccatattgctggcgctgaattccccagcctgccatcagcattgtgcgattcgccgccatcagttcagcgagtttgactatctgcgcttccggtacgccagtaatttccgccgcccagaccgcgctcttcggcgtattatcgctcttacctgtcagatactcttcaaactgcggatacccggtagtgtatttttcaaggaacactttatcgtgtttgccttgtgtcatcagggtatgcgcaatccctaacatcagtgccacgtcggtgcccatattcggcgcgatccaggtggcattatcgtcaaagaattcgatggtttcggagcggataggatcaatggcaatcactggtttgccagattttttcagctgatggaagtattccagcccttgctcatcggtactgctccaggcaatttttaaggtattcagcgggttcattccccacagcaccacaacctggctgttttccagaatcagcggccaggaggtctgctgttcatacacctctacagaaccgaccacatgcggcatgatcacctgtgctgccccggttgaataatcgccgctatgcccggaataaccgcccgccaggttcatataacgttgcagtaaggtttgcgctttatgcaacacgccagaagagcgccagccgtaagatccggcaaaaatggccgatggtccgttagctttacgaatacgatcatgttgctcatgaatcagttttaatgcctgttcccagctcacctgtacataggtatcttcgccacgacctttcgccggttgcagtggattatcgagatagctttttctcaccatcggatgctgaatacgcgccgtggtgtgtacctgatccgccgccgtagactgtaaggaattcggtatggttttcgccagcgcgcctgttgaagaaacaatcttgccgtccttcacttctacgttcatcgctccccaacgtcccgcggtgaggattttaccgcccttctcttctgcccatgcggggagcggtgctgccgatgtcaccaccagcgctccagcggcaataccgctgtgtttaataaattcacgtcttgttaatgtcataacttcctccctgatcaacgaggatcactgtttctcggtaatatctttggcgttgtactggaaataccgcgttaaaatgtccagttcgttttcgctcatgctggttcgtgcccccattcctttggcaatggacggccacgcattgacggtgtaatggtcggcggcaataggggcatgacaaccagcgcaataggtatcgtcaagtttttcagcgtattgccatagcggtttacggtccgctaatgcgggatcggtaagcgcaccctgtaaagacgcctgacgccattgattgccgtattcgtcagcctgccattccccgtttacagtgagcgccttgataccttcttcacttaatgtggctagcgccagccgttgacctgccgccaggtagagcgtgttttcactgccctgcatttgataaccctgcaacagaacgatcggctgtttgccactggcatcaacgacggtgagatcggttccaggattcacggtagccagctcgcctatgtgagaagttttgaaaggataaatatgtgcgccattagtaactgaagtagcggcctgactttccagctcatgcgccgcgttgtcatccatttttatttctggcggaaaatgggcaatgcctttatgacaatcgatacaggtttcgctgtccttttgtgctttgttatgcattttctgcgcagattcactttgcgaggcaatatccatggcatcaaaagaatggcaactacggcacgttgcagagtcagtggcttttaattctttccatactgtttcggccatttcctggcgatgagcttcgaacttatcgtcactgtctattttgccgctaacaaattcatgataaatatctttagatgcctttaatttagcaaataaataatccatccctgactttggaatatggcaatcggcacattccgcacgtatccctttctggttcgaaaagtggacagttccctgatattcctcaaaaggtttactcatcgagtggcaggaaaggcaaaatgctgtatccgacgttttatgtaagactttttgcgccagcaataacccgccgccaccaaccacaaccgctatcagcaaaaacaataacccaatgcgttttttccctcgcatagattcctctaattaaattactggacaccgaaatcattgtataattaaatatacaacgaattaaccgcttgcataattaggcacaacactgcctgaaacaatcgataaagaatatgatttattacaatgtaatcattaattgctaaggaataacccagttgctatttagaatatatatttatcagttttagtaatttaaatcccataattaatgtgaatatatacaatatttttagcacaacgctatgcgcactgtcacccgctcaacagatcacggttatcgttcgttttttatactgttcagggataaaaaaaggcccctgttgaaattgcaggggcctggtacgagcaagcatcatattgggcgacatgatgcaacggtaaaaatcatttggcctgatggcgttcaatgattcctttcatttcagcaaccgccgccccgtctacgatataacgcgaatactcgtccgcgtgttcatctgatgacatggacaatccttgattacgataacgcatcggtgaggcttgccacgctcccgcggagctatggacttccagcactccggcatcgaggaagtggtgcaggttttctgcacggactcctgctccggccataatgattggagcatcacgatgggcaataagttccataatttttgataaaccttgcagtgcgtctgatttttgccctgatgtcagtacccgggcaatgcccaattccgcaagattattgagtgtatataaagggttagcgcacatatcgaaggcgcgatgaaaagtcactgccagcggaccggcagcagccattattttttccattcgtggcatatcgacattcccgtcaacatcgagaacgcccgtcaccagtccaggaaaacctaattcgcggaccgtgcgcacatcctcaagaatggcggcaaactcaccgtcgctgtagcaaaaatcaccaccgcgtgggcgaattatcggatgcacagggatcgtcacccgctggcgcacggatttcagtacacccaacgacggcgttaagcccccctcttttggggctgcgcataattcaactctgtctgcgccgttttgctgcgccgttagtgcacattccatgctgtaacagcaaatttccagtaatgccatttttactccttaattacgccgactgctcgctggcaacgatctcttcaatggaccacggatgaaacttaatagttgttttgccatcggtgaccgccagcgtcggattcggtaatcgctcatgctcaccttttggcgaactggttttcactgagatccccggtaggctgagtccttcatcagaaagcaatgccagcgcacgggcattcagcgtttctggatcacccggcagaacgatttcaatatgttcccaaccttcgtgtgggtaacgtttttccccgggccacggtagctccacaatagaaaactgccagtgcgcaacctgtaccggttcatgcaatttaaacagacaaatcggtctgccattgatcatattttctgacaaaagctcgccacactgttcaaacccgcgacgccagcgttcagcagtggcgttttgatggcaacgcaaagaaatgtgatcggcagtcagcggagtgatattcaaccccagacggcgggaaagttcatctaatgcgtggataaatcgcggtaaatccgatgcaatatcctgcagctcgtcgatagattgccagttcgccataatcactcttcgtctttcagtaaaagcgttaatttaccctgttgccctgtgccaaccaaccgctgatttcacgccgcttctgatgcaatagtgaaaacggcaatacgccacgcgcacgttgctgacgaaaacagccatttgcagtatactcccgccctaatttctttaactggtgcgggcaatttttgctcgcttcatcaatgtaaggtattccggtgaatattcaggctcttctctcagaaaaagtccgtcaggccatgattgcggcaggcgcgcctgcggattgcgaaccgcaggttcgtcagtcagcaaaagttcagttcggcgactatcaggctaacggcatgatggcagttgctaaaaaactgggtatggcaccgcgacaattagcagagcaggtgctgactcatctggatcttaacggtatcgccagcaaagttgagatcgccggtccaggctttatcaacattttccttgatccggcattcctggctgaacatgttcagcaggcgctggcgtccgatcgtctcggtgttgctacgccagaaaaacagaccattgtggttgactactctgcgccaaacgtggcgaaagagatgcatgtcggtcacctgcgctctaccattattggtgacgcagcagtgcgtactctggagttcctcggtcacaaagtgattcgcgcaaaccacgtcggcgactggggcactcagttcggtatgctgattgcatggctggaaaagcagcagcaggaaaacgccggtgaaatggagctggctgaccttgaaggtttctaccgcgatgcgaaaaagcattacgatgaagatgaagagttcgccgagcgcgcacgtaactacgtggtaaaactgcaaagcggtgacgaatatttccgcgagatgtggcgcaaactggtcgacatcaccatgacgcagaaccagatcacctacgatcgtctcaacgtgacgctgacccgtgatgacgtgatgggcgaaagcctctacaacccgatgctgccaggaattgtggcggatctcaaagccaaaggtctggcagtagaaagcgaaggggcgaccgtcgtattccttgatgagtttaaaaacaaggaaggcgaaccgatgggcgtgatcattcagaagaaagatggcggctatctctacaccaccactgatatcgcctgtgcgaaatatcgttatgaaacactgcatgccgatcgcgtgctgtattacatcgactcccgtcagcatcaacacctgatgcaggcatgggcgatcgtccgtaaagcaggctatgtaccggaatccgtaccgctggaacaccacatgttcggcatgatgctgggtaaagacggcaaaccgttcaaaacccgcgcgggtggtacagtgaaactggccgatctgctggatgaagccctggaacgtgcacgccgtctggtggcagaaaagaacccggatatgccagccgacgagctggaaaaactggctaacgcggttggtattggtgcggtgaaatatgcggatctctccaaaaaccgcaccacggactacatcttcgactgggacaacatgctggcgtttgagggtaataccgcgccatacatgcagtatgcatacacgcgtgtattgtccgtgttccgtaaagcagaaattgacgaagagcaactggctgcagctccggttatcatccgtgaagatcgtgaagcgcaactggcagctcgcctgctgcagtttgaagaaaccctcaccgtggttgcccgtgaaggcacgccgcatgtaatgtgtgcttacctgtacgatctggccggtctgttctctggcttctacgagcactgcccgatcctcagcgcagaaaacgaagaagtgcgtaacagccgtctaaaactggcacaactgacggcgaagacgctgaagctgggtctggatacgctgggtattgagactgtagagcgtatgtaatcgatttttcgtgagagtgaagcctgatcagggttagccgatcaggcttttttattgccatctaaatgtattctgaaaatggacatgccattgttttctcactgttggataagaggccagaagcgtaatatccggccccagggaaacgataacggttgaatttaaggaataccgcagtgtttaaatttcttgtattaacattaggcattatctcttgccaggcttacgcagaagatacggttatagtaaacgaccatgacatttcagccatcaaagattgttggcaaaaaaattcagatgatgatactgacgttaacgtgatcaaatcatgcctgcgacaagaatacaatctcgtcgatgcgcaattaaataaagcctatggtgaagcttatcgttatatagaacaagtgccacgcacaggtgtaaaaaaacctgataccgaacaacttaacttgcttaaaaaatcacagcgagcctggctggattttagggacaaagaatgtgaattaatcctttcaaatgaggacgttcaggatttaagtgacccttattctgaatcagaatggctctcatgtatgatcatacagaccaatacgcgaactcgccagttgcagctataccgtaactctgaagatttttatccaagccctttgacaagaggataattcacatctttttggcatgttttgttgcaagctattcctgataaataattgcaacaagacatcgagcctttttcactgagttattaaacatactcgcgagcgcgtaatttttttgtccttcagcgataattcacaatcacttcattacgttgtacctttagcggtggaattaaccgcccaccgcctggcacttcccagataaatcgcaacggttctgctgccgctataccggaaaaggccacggtggttccgctctgcccctctaattcgacacaacgagattgcgaacacaagcgaacccgcagtcctgaaggtgtcgggccgataagctgataacgccacgctaccagcgtcatcaatcctgaagcaggttgtcgcgtagaaagaggcgcagacgacatcgactcaccgcgatgatttagcgtaattcctacactacttgcctgccacatcccctccccggcggcttgcaccagcagcggaaacaataatattgctaataaggttctcattatttgccgccaattgtcgccgtcatgcggatatgtcggttatcagacagttccagattcgacaggaccactaactgcggcaagctgcggcgcaggaagcgagacaataatggtcgcagcgcgtggttcaccaacaatactggcggcgcacccagcatctcctgacgggatagcgcttcctgagtttgcgccagtaaacgatccgccagccctggctccagtcctcccccgccctgcagcgcctgtagtaacaaacgttccagcggtgtatcgaggccaataacatggacttcatctttgccaggaaaccactgctgggtaatcgcccgtcccaacgccacgcgcacgacggcggttaattcatgtggatcgctttggatgggcgcatgttccgccagcgtttcgagaatggtgcgcatatcgcgaatcggtactttttcatcgaggagattttgcagcactttatgcagtgtggtgagcgtgacgacgccaggaacgagatcttccgtcagctttggcatctcctgggcgacgcgatccaacagctgttgcgcctcctgacgaccaaacagctctgcggcatgctggctaatgaggtggttaagatgcgttgctaccaccgtgctggcctcaaccactgtgtacccctgaatctgcgcctgttcttttagcgcactttcaatccagatagcattcaggccaaatgccggatcgacggtcgcctcaccaggtaacgtcccggcagcggttccagggttaatcgccagccagcgccccggataagcatcaccactgccaatctccacgcctttcatcaaaatgcgatagcgggcaggttgcagatccatattgtcgcgaatgtgcaccactggcggcagaaatcccatctcctgggcaaatttcttgcggatactgcgtatacggcccaacaactcaccatcctgctggaaatcgaccatcgggatcagtcgataacccacttccattcccagagaatcttccagttgtacatcgttccacgtcgcttcgacaacggtattattctctgccatttttaccggtttgggttcggcaggcgctttttgttcgcgtccgcgtatccaccaggccagcccgagcaatccggcagtgaacagcaaaaataccaggttcggcattccaggcaccaggccgagtaaaccgagcacggcggcgcttaacaacataacgcttgggttactgaaaagctgattcaccatctgctcgccaacatcctgatcggtgctgacacgcgtaacgatgacccccgcggcggtagaaatcaccagcgccggaatttgtgccaccagaccgtcgccaatggtcaatagcgtataactttccgccgcgtgtcccatgctcatgccatgttgcagcacgccgaccagcaacccgccgacaatgttaatgaccatgatgaggatcccggcgatggcatcgccgcgaacaaacttacttgccccgtccattgagccgtaaaaatcggcttcctgagtcacttcggagcggcgttttttcgcctcatcttcaccaatcaatccggcgttaaggtcggcgtcaatcgccatctgcttacccggcataccatcgagaacaaagcgcgcacccacttctgcgatacgcccggcacctttggtaatgaccataaagttgatgatcacgagaatgacaaacaccacgataccgatagcgaaattgccaccaacgaggaagtgaccgaacgcttcgaccaccttccctgccgccgccgcgccggtatgcccttccattaaaatgatacgggttgaagccacgttaagtgccagacgcaacagcgtggtaaacaacagaatggtcggaaacgcagcaaactcaagcgtgcgctgggtaaacatcgccaccagcaacaccatgatcgacaaggcaatattgaaggtaaacaacaggtcgagtatgaatgcgggcagtggcagcaccatcatcgacaagatcaacaggatcaaaatcggtccggcaaggatctgccattgtgtcgatttcaggtttgcgggcaggcgcagcatcgcggccagattactcatgggtcggtttctcgttaataaaatccagggcttccggcaccggaagatgagtaggttgtacagggcgctgtccaccagccagacgccagcgtttcagttgccagacccaggccagcacttccgccaccgcggcgtacagttgacccgggatttgttgaccaatctccgcatgtcgatacagcgctcgcgccagcggcggcgcttcaagcgtcgggacgttattttcagcgccaatttcacgaatgcgcagcgcgaccagccctgcacctttagcgaccactttcggtgcgctcattttgttttcgtcatactgcaacgctaccgaatagtgggtcgggttattgacaatgacatccgctttcggcacatcggccatcatccgacgccgtgcagcagctcgctgcatctgacggatccgccctttaacatgagggtcaccttcgctttgtttgaactcatcacgaatatcctgccgtgacatacgcagctttttcaggtggctgaatatttggaaaaagacgtcaaatcccaccattggaatgacaccaagcaccaccagcagtgcgcatagccctaccaaatccatcgcattacccatggcggtaatcggagactcggccatcaagcgcatcatctgcggccagtgatgccagagaaaaaaccccgtcacgctgccaaccaggatggttttcaaaattgctttaagcaactccgcgccagtctgagccgagaacatccgtttaatgcccggtagcgggttgagtttggaaaacttcggctgcaaggatttgccgctaaataccagccctcccagcatgaccggagaaatgagcgccaccagcaccacgccgctaatcagcggcagcagcgccagcatggcttctctgatcagcagaataatctgcccgaggatcagattcgggtcattgataatactgtgatcaaaatgcagcccagcggagagcatgcccgacaatcgacgggccagcgacacaccgccaaaccagataacactaacgcccaccagcaaaatcagcagtgaggtcagttcacgggaacgcgggatttgcccctcttcccgcgctttttctagtcggtgaggtgtgggggcttctgttttgtcgtcgctctcgtcagacacgtcgccaatcctggaaagagtattaagcgtgaatgatgccagagcgcaaagcgttcaatggtttgagtaaggggcaaaacaggcgggatttagggcttttgctgccacacatcaagcatagtgtgcgtttgtcggatgcggcgtcatcgccttatcagaccgcctgatatgacgtggtcacgccacatcaggcaatacaaatcaaaatccaagactatccaacaaatcgtccacctgatcctgactggctaccacaccggctttgctggtatcgacctgaggtccattaagcaaactctggttttcacgttttggacgcgactcctgttccgggatgttttccaacagcaccatcagcaactggcgttcgatctcctgaatgacatccatcatccgcttaatgacctgcccggtgagatcctgaaaatcctgcgccatcatgatttccagcagttgcgcgttagtaaagctggtatgcgcgggtacatctgccagaaattgtcgtgtatctgttaccagttcacgggcgtcggcaaggtcaatcggatcggcaaaccagtcatcccaacgttgggttaacgcttttgctgatttctccatttgatcctgatgcggttgtgacgcctcaacactgttcagcgcccgctccgcagcctgggcggtcatctgcacaacatagtacaaacgatcgcgcgcatcggggatggcttccgccgcttcggcaatggcctgatccagccccagttcccgcaaactgtcgcgcagcatacgcgtcaggctgccgatgcgcgcaatgatatcgccagctgaatgctcgtcagcaggtttgattgatggttgcatcatagtcgcatcctcacatgcccagtttctcaaagattttgttgagtttttcctccagcgtcgcggcggtaaatggcttcaccacatagccactggcccccgcttgcgccgcagcaatgatgttctctttcttcgcttctgcagtcaccattaacactggcaatgccgacatcgcgccatccgcacgaattgttttcagcaattccaggccatccatattgggcatgttccagtcggagataacaaatccataaccgcctgcctgcaacttattgagagcgtcgacgccatcttccgcttcctcaacattattgaatcccagctctttcagcaggttacgcactatgcgtcgcatggtggaaaagtcatccacaaccaaaaatttaagttctttatccgccatttcacactcctgatttaaatacgtatcgcctgtccggcactaatttttgccaacatttgctggcttacctggctaagatcgaccacttcgcagacaccacccatattgatggcctcgcgcggcatgccgaacaccacgcaacttgcttcgttttgcgcaagggtccatgcccccgcctgacgcatcgccaacattcccgccgcgccgtcgttgcccataccggtcaggatcaccccaaccgcattacgccccgcctgtttggcgacagaatggaacaacacatctaccgaaggccgatgacggttaaccgccgggccatcgtgaattttgatttggtaatttgcgccactacgcgacagctccatatgccgatcgcccggcgcaatataggcatgccccggcaagacacgttctccgtcttcggcttctttaaccccgatctggcaaagcttattaagtctgtcggcaaaagagcgggtgaaaccgggcggcatatgctgggtaattaacagtgccgggctggaaagcggcaacggttgcagtacgtgacgaattgcctcagttccacccgttgaagcaccaatcgcaatcagtttttcagaactcaacaacggccccgccttcagcgttgtcggtgccgacaatggcttatgtgctgcaaggctcgcctttgctgccgtacgcaccttttcagcaatcatttcgttatacgccagcataccttcgcgaatacccagttgcggtttggtgacaaaatctatcgcccccagctccagcgcgcgcagcgtgacttctgaccctttgccggtcagggaagaaaccatcacaacgggcattggacgcaaacgcattaatttttcgaggaaatccagtccgtccatccgcggcatttcaacatccagcgtcagcacatcgggattgaatttcttaatcaagtcacgcgcgaccagcggatcaggcgcggtcgccaccatttccatgtcgctatggctgttgatgatttctgtcatgatctggcgcatcagtgccgaatcatcgacagataacaccctgattttgctcatcgttaatccttacttagcgcatacaccgtctgaccacgcagcgtgaagcggcgctcaaggtggctaaagttttcagagtgacccgcaaacagcaatccgtcgggtttaaggagcggaacaaagcggcgcaaaatctcctgctgggtagtttgatcgaagtagatcatgacgttacgacagaagatcgcatcaaacggccccggcacggtgtactgtttcgccagtagattcagcggggcaaaatcaacatagttcgccagctcctgacgcacgcgtaccagcccttcatgcggccccgtccctcgcatgaaataccgttgcagttgctgcggcgtcaggtttttcaactcttcatggcgatagataccgcttctggctttttccagcacttcggtgtcgatatcactggcaaacactttccagcgtccgggcgcggtgcccaatgtgtcagccagcgtcatcgcaatgctgtacggctcttcgccggtcgaagccgccgcgctccatacgcgatactcgccagaacggcgacgtgcgtgatccgcgagcagagggaaatgatgtgcctcacggaaaaatgccgtcagattcgtggtcagcgaattgataaacgcctgccactcaccgctgtgctgattagattccagcaagttcagataatgaccgaaatccgtcagtcccagcgaacgcaaacgacgaaccagtcggttgtaaaccatgtcgcgtttatggtcagccagaacgatcccggctcgttgatagatcaattgacttatccgccgaaaatgcgcgtcggaaagcgccaggcgctcggtcatctgtaacaataaagacgtttgcccacagggcagagatgaagtcatagcgccttctcaatcacttcaggataccactggcgcaatttgtaactgcaccgactcatgtcgtgctacttcatgttcttcaagggtaaataccgccacacgcgacgaaagatggtcggcctgattcgccagttgttccgttgccaccgccgcttcttctaccagcgaggcgttctgctgagtcacctgatccatctggctgacagcctgtgcaacctgctcaatcccccgctgttgttcttccgacgcagaggcaatttctcccataatgtcgttcacgcgggtcaccgaactgacaatatcgatcatggtcgcggcggcgttattcaccagtttcgaaccctgctggacacgattgactgactcttcgatcagccctttgatctcttttgctgcctgcgcgctacggctggcaagattgcgcacttcacctgccactaccgcaaaaccacgcccctgctctccggcgcgagccgcttccactgccgcattcagggccagaatattggtctggaaagcaattccgtcgataacgctgataatgtcgccaattttttgcgagctggtggcgatctcctgcatggtgtgagtcatggtactgacctgaacaccgcccgcctgcgccgttgtcgcggcattttttgccagttccgacgcctgtcgtgcgttatcggcgttttgccctaccgtggcggttaattgctccatactggcggccgtttgtgccagcgatgccgcctgctgttcggtacgacttgagagatcgttattgcctgcgacaatctccgcgataccaatgtgcatctcctggcttcccttacgcacatcacttaccgtcccacgcaaagcctgctgcatggtcttcagactggcaaaaatggcggtgatctcattacgaccatataccgcaatcggacgcgccagattacccgcagcaatgctgtcaaaatggctaccgataatggccagtggttgaacaatcatcttgcgcgtccaccacagcgcactgctgatgtagatcgccgcaacaataatcatgctgataaacaccagtgccgaaatctgatagttacgctggctttgcgcactggcggcttccagcacatggttgatctccagctgccaggcctcaaagttaacgtcaaacgcattctgtgatccctgcaccggcgcagtgaggaaatccgaaagttgattactttcaagccaggtcgcctgatgttcgagatcgttgtgccagcgggcaaaacttttctccgtctctttttgcaatcccctgacgtgctcgttgcccgcagtcatcgccataaaacttttaaacagcgtggtggattgcgtcagactggcgcgcgccgtcgtcatcaacgttttaatgtcatccgccggatagctaagtgccgtcagagtgcccgctttgttcagcgcggtactggcctgtaacattaccgcccgagtttgcgctaatgccgcacgttgctgattgctctgctcgacctgattcagtcgttgcaaatcgtcgcgaaatgcccaaaaagacatgccgttactgccaatctgcaagatcccgcagagaatcaaaattaaaaacagcgtggtcgaaattcgaatacgattaaacatcaacgctccccatcaggcggcaatgaccgcgttagtaaatactcgtcaaaatgtttcccagtttggatcttgttcagcaattcgcagtcgtggctgagccggtggttgctcactggcaggacgggatggtgtttgcggtttattggtgagtgggctggctgccagacggaacgcggaaactgcttgcgttaaacgactcgcctgttcttccagcgcagcggcggcggcagctgattcctgcaccagcgatgcgttctgttgcgtgacgcgatccatttccgaaaccgccaatgcgacttgatcgatgccacggctctgttcatccgatgccgatgcaatctcgcccataatgtcagtcacgcgagtgacagcattgacgatattgttcattgtttccccggcgctttcgaccagcaccgaaccggtatcaacgcgtgagacggagtcttcaatgagggctttgatctcttttgccgcctgggcgctgcgactggcaagattacgcacttcacccgccaccacggcaaaaccacggccctgttcacccgcacgcgcggcttcaaccgcggcattcagcgcgaggatattagtctggaaggcaataccgtcgataacgctgataatgtcggcaattttcttcgaactatcggcgatctcatgcatcgttttcactacgccatccaccactttgccgccgtgctgggcggtgtcggaggcactttgcgccagttgcgaggcctggcgggcgttatcggcgttttgcttcactgtcgcggtgagctgctccatgctggcggcagtttcttccagcgcggatgcctgctgttcagtacgggaggaaagatcggtgttgcccgccgcaatttcacgggtaccggcatagatggcatctgaaccttcgcggacatgagtgacggtgtcagtcaaagagcgttgcatatgtgaaacgctctgcgccaggtcgcccatttcactgcgcccgtcaatggtcagggtattcgccaggttaccaccggcgatttcgcgaatgtgagcaataatttttgccagcggagtaagcaacatacggcgaatgccgtaccacgccaccagcagaatcaataccaccaccagcgcgataaccgccagttgccactgggcaaatcggtaatcatctgcgttgtcagtgacgatatcgcgatacagtttttcactgctgagggcgtactgagcaaacgcttcgcccattgcattttgcattccctgggttggctgagcgaaataagctccagtattgccataatctagataatcaatcagttcagttaacgctgtgtaatagtttttatatttttcatcaatattacgactggtagcgaccatttcaggtaacggtgccatgcttttgaattttttataatgcgtcgctgcctgcgccaatgttttcctggcgctatcgagcaattcaactttggcgttactttgttgattggaggaatccatcatcatccgtaccgctgaacgactcaggttaatgcgcgtttgcagcattaaatcccaggttgacgtcagctcgccctgctgttcccgtaattgattggaaaccacaaagctcttctggctatggtgaagggaagaaaaaaacagactgccggaaataagctgtaacagtgcgaatacccccagcaccattaccaacagcgtgactacgcggatacggttaatcataaggcaccttcctgaaaacaagttgatctcgttatcggcaaggaggggggaaactttattgctgatgccacccgccgcgaaattgaaataaaaaacccgatgcgcagatcatcgggttcatttcaattgaggaaatcgggagaattacgccacttctgacgccgcgctatctaacagcgccatctcttcgctgttcagcagtttttcgatgttcaccagaatcaacatccggtcgcccagtgcgcccagtccagtgagatattctgttgaaagcgtcacggcaaattccggtgccggacgaatttgctccgccgtcaatgaaagcacgtctgagacgccgtcaaccacgatgccgaccacccgctgtccgagattcaggacgataactaccgtgttgtcgttatagtccacatccacctggctgaacttaattcgtaagtcaacaatcggcacaataacgccgcgcagattcgtgacgcctttgataaacgctggcgtgttcgcaatccgtgttacctgatcgtagccacggatctcctgcactttcaggatatcaataccgtactcttcatcaccaagggtaaataccagaaattcctggcctgacggctcgctggccagctttgttacattcgtcataccggtcatattgttacctttttactcattcaggcggcggtgttcgccatacgttgttcgcggtttatcgcctgcaaggcggagacatcaacaatcagtgccacgctgccgtcgccaagaatggtcgcagcagaaatgccggggactttgcgatagttactttcaaggtttttaaccacaacctggtgttgaccaattaattgatccaccagcaaggcgtagcggcgaccgccactttgtaagatcaccacaattccctgggtggcttcggttttcgcgcccgcgacgttgaacactttccacagttcgacgatgggcagatattcaccccgcacttccagcacccgctcgccgccggccagtggatggagatcggcttcacggggttgcagtgattccataacagcattcagcggcagaatgaaaacttcatccgcaacgcgtacggacatgccgtcgaggatggccagcgtcagcggcagtaaaatgcggatcgtagtgccagtaccctgcttcgactggatttcgacatgaccgcccatcttctggatattacgtttaacgacgtccatgccgacgccgcgcccggagacgtcggtgacctgctctgccgtggagaagccaggtgcaaatatcagcatcgcgacttcgtcgtcgctcatgttttcgctgacagtcaaaccttgcgaggccgcttttgccagaattcgctcacggtttagccccgccccatcgtcggtcacttcaatgcaaatgttgccgccctgatgttcggcagacagaattaaatttccgacgctgtttttacctgcggcgagccgtttttctggcagttcaataccgtgatcgaggctattgcgtaccaggtgggtcagcgggtcgataatgcgttctatcaggcttttgtcgagttcagtagaactgcccaccagcgtcagttctacctgcttgccgagttttcccgccagatcacgcaccagccggggatagcgactaaaaacatattccatcggcatcatgcgaatcgacatcactgattcctgcaaatcacgggcgttacgttgtaactgccccatgctggttatcaaatcaccatgattaaccgggtccagttcgctggaacgctgggcaagcatggactgggtgataaccagctcgccgacgaggttaattaattgatcaaccttttctaccgctacacggatgctggtggattcattgctgcgcgtcgttttttcccgctccacgcggccggttggcgcttgttcggctgccagtttaagcactggtggggtggatatttttggcgagacttctactgtttcaaaggtaatctgatcggcttcaatcacaaaacagagtaccgctgtgatgtcatcttcggcgatgtcgcccggtaatattgccgagagcgaatccgcccctttcaccacgtcagttaacgttgtcagatgtcccagttcttcttccagcaggtcgacttccccggccttcaggcgcgaaaggataattcgtcgcggcgactgactgcgactctgctcatcttgcggttcacttttggcaaccacacttaatcgggtcactgcggatggcgtttcgcctttcgcttctaatgccagttgacgcaaggcctggcagatataatcgaagctggcggcatccggctcttgcgactgtttataagcgtcgagctgttcttgcatgatgtccttcgtttccaaaaacagattgataatgtcggtgttgagttgcatctcacctcgtctggcttcatcgagcaggttttccatcagatgcgtggtttcctgcaaaacgctgaagccaaaagttcctgcccctcctttgatcgagtgggcagcccgaaagatggcattcaattgttcggcatctggcgcttccggctgcaaaaccagcaaatgctgctccatgtcagccaacagttcgtccgcttcatcaaaaaatgtctgataaaaatcgcttatatccatgctcacgctgtcacctcggttcggctgatggcattgtgggaacactgacctgtggtgcaacctcaggtttttccagggcgcttactggctcattctggctttcggcgttttcatgcaaaatggcctgttcggcttgtttgttcagtaccagcaggctgatgcgacggttgacggcatcatcaggtccgcgatcgcttaagcgcatcgttgccgccatgccgacgacacgtaacactttgccgctatccaaccctccgaccatcagttcgcggcgggatgcattggcccgatcggcagaaagctcccagttgctatatcctttctcaccgctggcgtaggggaaatcatcggtatgacctgaaaggctaatacggttgggaataccgttcagtacaggcgcaatggcgcgcagaatgtcgcgcatatagggttcgacatcggcactgccggttctaaacatcgggcgattctggctatcgatgatctgaatacgtagaccttcctggaccagatcgattttgagatggggacgtaacgcccgcagtttcggatcggactctatcaactggtcgagatcaccccgcaatttccgcaatcgactttgctccatgcgttttttcagctcttcgatgttcggctgcttattcacttccccctggctttgggtgtaatcatcaccaccgccgggaattgggctttcactattagaaatgcgatcgccgcccgtaaccgcagtcgccagtggagtccggaagtactccgcaatctgaatcagctcttttgggctggagatggagatcagccacatcaccagaaaaaaggccatcatcgcagtcataaagtcggcataagcaatcttccacgatccatgtgctgccccgtggcttttggctttgcgtcgtttgacgacaataatcggatgcgcttgattcttcatgcttcctcggttgtcgtctgttgttgcggatttttcaccgcacgcacatgctcttccagttcaataaacgacggacgttcgctggaatagagcgttttgcgaccaaactcaacggcgataggcggtgcgtaaccgttcagattagaaagcagagtgactttgacgcactgcatcattttgctggtttcggcgcttttctgacgtaaaacagtcgctaatggggaaataaatccgtaagccaataaaatgccgaggaaagtccccaccatcgcatgtgcgataagcgcacccagctcggcggcaggacgatcggctgaacctaacgcgtgaacgacccccattacagccgcaacaataccaaacgccggaagtgagtccccgaccagcgccagactgttcgccgggacttctgcctcgctttcgtgcgtctcaatctcttcatccatcagagcttcgatttcgaaggtgttcatgtgaccgctgataatcaggcgcagataatcgacgataaaatcaagcatgacgctatccgcgaggatgcgtgggtagctggcgaagatctcgctctcacggggattttcaatatcacgttccagcgaaaacatccccatctgccgcgatttcgccatcaaccgataaagcagagccagcagatccatatacattgctttggtgtatttggagcgacgaaacagcaacggcagcgccttcagcgtgcctttaatcgctttgccattattgccgacgataaacgacccaatccctgcaccggcaataatcaccagttcagcgggttgatagagtgctccaaggcttccaccggtcatcaaataaccgccgaaaactgtaccgagaacaaccaggtaacctaataagataagcacgacatcatccttccactgttgaccatgacaggatgttcagtcgtcaggcgttaacgcgcgattggggcaaaaaaaagcagcggtacgtcgttaccgctgctggaatgttgcgcctcaccgtatcagttaaacagcctgtactctctgttcatccagcagttgtgggataatatcggcaggattctgggaaagtttacgtctttttactgcccgggatggcggttgacataagctgcaggcaaagctgccaacaggctggtgagcgtgggtaataaaattgccgccgcagcagttgcagctggaaagttgcagtaatccactttcaacaaaccgcaccaatgtccaggcacgggttaatgccagcagtggtccttcttctgcttgtgggcactgttcaaggtataaacggtaggctttgatcaccgcatcgacgccattacacaaaccggttttcagtaaaaactgccatgcattacagaacatcgaagcatgaacgttttgttcccaggtcataaaccagtcggttgagaatggcagcatgcctttcggcggtgggcttccgcgcagttctttataaagttttatcaggcgtccgcgacttaactgtgtttcgctttccagcatctgcaaacgagcgcccagggtgatcaattccattgccagctgaatatcccgcgcttcctgaacaatgcttttttcactcatgatcaggcccttttcttgcgcagcgcttcttcaggctgattaacatcattcagcaagcgtgttgagagcatgatgccggtatgaatttgctggagatcgtcaacgcgggaatcttgcgtcaactgagtaatcgtctggtggctgtcaaaacggaagtgacaaaccagttgattggtttctgccagcttaaccatttgcggaagagtcagtgccgctaacgttgtcgccatttcttcatttatgccgagacgaaacatagcggacgctttgtcctgaacaatcaaacgctgtgcaagtagtaaatatgacaagttgatgtcataaatgtgtttcagcaactcggaggtatgcattattcccacccagaataaccaactttatttttatgcggtttcaccgcaccccgtgatgtcgccgggaagccccggtaaaaaataattagcattagaatagttgcgataagctgcaataagcagaaccacctttttggtttaatatgtccttacaaatagaaatgggtctttacacttatctaagatttttcctaaatcgacgcaactgtactcgtcactacacgcacatacaacggaggggggctgcgattttcaataatgcgtgatgcagatcacacaaaacactcaattacttaacataaatgggtaatgactccaacttattgatagtgttttatgttcagataatgcccgatgactttgtcatgcagctccaccgattttgagaacgacagcgacttccgtcccagccgtgccaggtgctgcctcagattcaggttatgccgctcaattcgctgcgtatatcgcttgctgattacgtgcagctttcccttcaggcgggattcatacagcggccagccatccgtcatccatatcaccacgtcaaagggtgacagcaggctcataagacgccccagcgtcgccatagtgcgttcaccgaatacgtgcgcaacaaccgtcttccggagactgtcatacgcgtaaaacagccagcgctggcgcgatttagccccgacatagccccactgttcgtccatttccgcgcagacgatgacgtcactgcccggctgtatgcgcgaggttaccgactgcggcctgagttttttaagtgacgtaaaatcgtgttgaggccaacgcccataatgcgggctgttgcccggcatccaacgccattcatggccatatcaatgattttctggtgcgtaccgggttgagaagcggtgtaagtgaactgcagttgccatgttttacggcagtgagagcagagatagcgctgatgtccggcggtgcttttgccgttacgcaccaccccgtcagtagctgaacaggagggacagctgatagaaacagaagccactggagcacctcaaaaacaccatcatacactaaatcagtaagttggcagcatcacccataaatgtataagtcatacttttgttttgggtgtatttcaatctgttaaaaagtttttcgctacgctagcaagcaaaaatgaaacaggaataatcgaaatgggatgttgcgcacagtcaaaataactcaccgtaaataatcatctgctataaataatcactttcatgcaataccagataagctatttttaaacagacacttaccgcacaacaaactaattaaatacaaagaaaggcaacaatcaacttaatgttaatgaaatgttttacatatattaaccacttgtttaatgcggagaatcagtacactattttcttataattacatttgaaattatatgatcaccgggagtgattgattaattatctttactaataatcagactaatatttacctgtttgaccgagttgggattgcgtcgtttctccattaggagtaaagctttaatgtcacctgaagttcacagaataaggaacaggttatgagctatagcaatattcttgtcgctgttgcggttacaccggaaagtcagcaactgctggcaaaagcggtatctatcgccaggccagtaaagggacacatcagtttaattactctcgcttccgacccggaaatgtacaatcaattagctgcgccgatgcttgaagatttacgcagcgtgatgcatgaagaaacgcaaagctttcttgataagttaattcaggatgcggggtatcccgttgacaagacgtttattgcctacggtgagttaagcgaacatattctggaagtatgtcacaagcatcatttcgatttggtgatttgcggtaatcacaatcacagtttcttttcgcgagcatcctgctcggcgaaaagagttattgcctcaagtgaggtcgatgtgctgttagttccacttacgggagattaaccgctcctacgcaagctttggaaaggtagcaactttatcgcgctgctggctttccgcgcttcgcggaactatctgctttaggtcgctaatgaagcactcctgccagtggttaatatcgtttttcacgataacgtccagcatttctgcatgacgggaaatacgttccgccagcgacatagtcaatgcacgatccagcgcagctgcaacttcgtcacgatcgtaggggttaacaattaacgccgacgttaactcgtttgccgctcccgcaaattgcgaaagaacaagaacgcccggattggctgggtcctgagcagcaacatactcttttgctaccaggttcatcccgtcacgcagtggcgtcactaagcccacgtcagagtagcggaatattttcatcagtaatttacggtcaaaatgctgattcaaataataaagcggcgtccagcctaattgcccgtatttaccattaattcgtccagcttcattttcgagctgatgacgaatatcctgataggcttgcacatcaccacgcgacgttggtgcaatctgggtataacgaattttaccatgatgctgcggatatttttccagcaacgcttcataggcgagaaaacgctctggcaaacctttggaataatccagccgttcgacagaaaagatattttgtacgtttttcagttccgctttaagttgcgccagttttggcggcagtggcccggcagcctgtttggctatttctttcggttcaatgccgatcgggtagacttctgttcgaaatgctttgccccaggctgtatggctttttgcgctacgtgtcgtgacgcgggtcaggttagaaagacaatccaggaacgccagacgatcgttttctgtctggaaacccagcaaatcataatcacaaagctgttcaagcaaggtgtcatatgtcggcagcgcgttgaagatttccggtgtcgggaaaggaatatgcagaaagaaaccaatgcgattattcactccccgtttgcgtaattcatgcgcaaatggcaacaggtgataatcgtggatccagataatgtcatcgtcttgcaacagcggcagtaatttatctgccagcaacgcatttacgcgtagatagccgtcccaggcaggacgctgaaattgcaccagatcgagccgataatgaaaagcgggccagagaacggcattggagaattggttgtagtattcgtcaaggtcctgttcgctgaggttaaaagaggcccacgtaatgttaccttttttcaccttttttagcggctgatcctcattccctgtttcaccactccagccaaaccacagtccgcctgcggctttcagtgcccccagtatgccaacggcaaggccaccggcactggcggcgtgctcgtctggtggtgcaatccggttagatactacgactaaacgactcatagtcatcactcctgttattttctcttttttgttgtaatgcggtggttatcatttcaagccagctccagacatccggcacacccgccagtcgccatgatgcctgagttgcacctgtgccaatttttactgacattccgcccagtcggttaacgactgcgaagccagattcatcggttaaatcatcgcccagaaatacgggcgttcgcccgataaagggagcttcctgcataaaagctgcaattgcctcacctttactggtacctctcggtttgatctcgacaacacactttccctgctgtaacgccatttgtggccagatctgagtaatacgttgcgctaatgtcattaatgcgtcttcatgctgcggagcctgacgataatgcagcgcaaaagccatccctttcgcctccagctccgcgccgggatactgagcgatgactgtatgcagttgcacgctaatatcacgcgcaatcgcatccggcagatgaacgatatgtgttttaccattgatgtcacggcgctccgccccatgcacgcccgctaacgggaagcgataaggttttgccagtgcgtcaagctccaccattgagcgccctgatatcaatgccaatgcaccatcacttgcggttgccagtagctgtagtccttgcagaatattgtcaggcacgacgacctgatcgggatgcggtttgatttccgccagcgttccatcaagatcaaaaaaccaggcatatttcgcggatagttcaggggtttcggttaacggttctgtcacccggttctcctccttctcttttcttattgtgttgcgcagaacgcgctttacagacatgtaagtatagacagtgtgacgggggtcgccatttgcaacgaagaacagccaaccgttatggcggttggctatggtgggaaaaaacgctaaattgttgcagaaaaaagcatcagacagtgcgtttcgctttttgcttgtaacggtcgaagatcaccgctgccagcaggattaagccgcgaaccacgtactgcgcgaaaggagaaatattaagcaggttcatggcgttttccacggtgcctaaaattaagatacccgccaccacatatgagatttttccgatgccacctttcagagaaacgccacctaaaacgcaggcggagataacaatcagctcataaccaatcgacgtcattggctgcccactggtcatacgtgaagccagaataattccggctatcgctgataccaggcctgagagaacaaagataataattttggtgcgaacaaccggtacacccgccagacgcgcggcctcttcgttcccgccaatcgccagggtgttacgaccaaaggtggttttattcagcagcaaaccaaagataatcagacacgcgacggtgagccagattggcgcaggcagaccgaaccagttggcgtaaccaagggcaaagaagctttcatcttcgataccgaccgctttaccgtctgaaatgatgtacgccagacctcgaacaatctgcatcgttgccaatgtcgtgatcagagcatttattttcagtttggcgataacaaagccattgaccaggccacagagaacgcccagcaacaaccccgctgccacgccaatccacaggctttcagtcaggttaataaccaccgccgtggtgacacccgcacaggcaattacggaggcgacagaaaggtcaaagtcaccggaagcgaggcagaacaacatgccacaagccaccatccccgacatggaaattgccaggcccaaccctttcatattaatgaaggtggcaaaatttgggacaaaaatggcacaggcgataaagagcaccgcaaacaccaccagcatgccgtactgatcccagatacgcccgaagctgaatgacgacttaggtgcgccagaccccgatgtagaaacagaagacatcatactctccttactcaggcaacagcctggctgactttaggcatcgcaaggctcagtgcctgacgctcatctgcctgctcgtgtaacaattcaccggcgatttcaccttcccgcatcaccacaatccggtcggcaacgccgaggacttcaggtaagtcgctggaggcaaacagcaccgccacgccctgcgccgccagcgcataaattacgttatatatttcgtgcttagcgccaacatcaatgccgcgcgtaggttcatccagcaaaatgaccttcatctcttccgataaccagcggcccagaatggctttttgctgatttccgcctgagagattcatgatcagttgctccgcgcccggcgttttgatgttgagcgaacgaatgtggtgatcggcattgttttcttcccaaccgttgttgattacacaaccgccgagcacatgtttacgtctggcactgatgttgatattgtcgcgaacggagtgcacgggaataatgccttccgctttgcgatcttccgggcagagcatcatgcctgcggcaatggcgtggctcggtttacgaatatcgatcggctgttggtcgatataaacctgaccggcggtgatttgcgtcccgccaaacatgcctttcattaattcgctacgccccgcccctaccagaccaaacagcccaacaatttcaccactgcgaaccgccagacttattggcgtacgcacgcctggtgctttcacagcatcaagacgtaggcgctcctcgccataactacgcggttgccagccgtagatatcgccaatgtcgcgcccgaccatcgcctgcaccagcgcgtcgtggtcaacctgctgcatatcggtaaaggttttgacataacgtccatctttaaagacagtaatggcatcgctgagggcaaatatttcttccatacggtgagaaacgtataagattacccgcccctcttttcgcagttcacgaataacgcggaaaagattgtcgatttcacgggcagagagggagctggttggctcatcaaaggcgataattttggcgttacgcgccagcgctttggcgatttcaaccatctgccactgaccaatggagagatatttcagcggcgtgtccgggtcaatatccataccaagatgtttaagttgtaaacccgcctcataattcagcaatgagcgattcacaatgccgcctttatgcggcagctggccgagatagatgttttccgcgacggtcatttccggcacgagatgcagttcctggtaaataatcgccacgcccgcgttaagtgctgcggtcgtgtcggaaaaggacatttcctgcccattaatcactacagaacccgtggttggcgcatagttgccgctgaggatttttaagagagttgattttcctgcgccattttcacccatcaacgcatgaacctgaccggcatagcagtcaaaactaatatccgtcagcgccttaacgccgggaaacgttttaccgatgccgcgaaatgagagatacggggtagactgttgcataacgtctccgtgaatcactggtcgttcacaccccctctgcatcatgcagaggggaatttttccggcaaattacttaccgcctaaaccttttttctccagttcttctttaaagttgtcacgcgtgatcagtaccacgtcggtaacttcggtaaattttggcggttcaacgtcttttgctacccagttgtaaagcatttcgctggatttatagccatgtacgtccgggcttggcagcagggaaccgtagaagccggttgcctgtgctttagacagttcgctcaccgcatccacaccgttaatgccaatgccgatgatatcggccgctttaaagccctgaccttccgtcgcgcgtacgccgcccagcacggtgctgtcgttcataccgacgatcagccaatgtttaacttccggatgttgaaccagcattgagttggcagcgtcaaatgcccccgggatgtcgttagatttggtaggtacctgataaatttgtttttccgggaatccggccgctttcagcgcatccatagatcccgtagtacggcggcgggcggtatccagttcgttggcggtaatcgccatcaccgcgctttctttgacatcccagccacgtttctgcatctctttatacagttcctggccctgacgttcgccaattttagtcgccgccatcatcaccagcggaacggtatccattggcttacctttggcgttaacaaactggtcatccacggcaatgactttcatatcgtagccacgcgctttcgcgacgatggcagagccgagtttggggtccggagtacaaataacgaaaccttttgcgccactggcagccaggctgtcgatcgcgttcaatgttttttcgccatccggcacggcaatcttaataacctcaaaccctaaatccttcccggctttatcggcaaacttccattcggtctggaaccacggctcttccggttgcttcaccagaaaaccgagcttcaggttctccgccatagcggattgtgacataacggctgccagaccaatggctgccagggctttagtaaatttgtgcatggttctctccagctttagtgtcgttttgtgtagggcaaaaacgaatgacattcgttaaattaatcggaaaacaaagcattaccttttaactaaaagataagtgactgtgttgacatagttttagcgagaaattaattctccataggagagcaatatcacatcgcagaattacagtgagaacgtgcataaatttagcgggaaaagacataagggaaagccaatttgtcagacaaattgtcgaatgcacagcagattaatccataagattagcctggaaatccttgttgtctttggtacccatgcgggatgtcttctttttaaccagtcaataggccgcattacctggcgttgagtttttgaaatggtgtaataaccgcaactcaaagatgtggaaaatgcacgtcattcatttcgtcattaattatcactgtgctcattaattaacagaacacgtataatgagagccatctcgcaaaaatgaaaaaacgttttataaaatcatcacttcatcatgaattcaaattcattgattaatatcaacaagatacaaaaagcactatcattaaaattcattgcagttacattgatttcatcaatgaaatgtaaaaatatataaacttgatgatttaagcattttcttatacccgttcagacgttattcttatttcagatcatcgtcagaattgactccacgatcacatttcggaccggcagaaaggaattattctgcaaacagtaattatggtgttttgatttatcttgcacctctccacttctggatataaggatattaggtatggcaaccgctggaatgcttctcaaactcaactctcaaatgaaccgcgagttttacgcatccaatctctaccttcacctgagtaactggtgttctgaacagagtctgaacggcaccgccactttccttcgcgcccaggcacagagtaatgtgacccaaatgatgcgcatgtttaactttatgaagagtgtcggcgctacccccatcgttaaagccattgatgttcccggtgaaaaactgaactctctggaagaactgttccaaaaaacgatggaagaatacgagcaacgttctagtacgttggcacagttagccgatgaagcgaaagaactgaatgatgattcaaccgtcaatttcctgcgcgatctggaaaaagaacagcagcatgatggtctgttgctgcaaaccattcttgatgaagtgcgcagtgcgaaacttgcgggtatgtgccctgtgcagaccgaccaacatgttctgaatgtcgtgtcacaccagctgcattgatcatcatcggcgctaatgcattgcgccgatgaaggttttgagaaaccgctgcctcatctgtttgaagcagcggtttttttaatgggattcaccctgtggggtaaacttgagttcaataagcgcgatggctttttggattgcccgcatggtgaccgggtctgcggcggcgggatggttagtaaagtcgatattcttcagctgactggacattttttcacgaacttcaacgggcgcgattacatcgagaacatccagaatttgtttgataaccaactggcaagcaaccacatcagaaaccaattcctgatcggcattcagcggctgggacatcgtaaactcctgatagcattttgaaagccgttatagtagcgacttcacatcttcagcgatagtcacatccaccgtcatcaggacacaaaaaaacctgccggagcaggttttttgttatcggaacatattgcctggcggtacgtctttgaacgtcttgcaatagttattgaacatacttttcaggattttgcgcagtttcatcgcggcactccgaccatttgttatacaggtgttattgtctttgcgcttataatatgacaaccatcacaaaaatcaatctttatgtgatacaaatcacataaatacccctttaatgttataaaaatgataatcaaaaaacagcccccctatttctgacacctacagatggcaagaaatagcgcctgccaggcgtcttttccggccattgtcgcagcactgtaacgcgtaaaatagtgctttctcttactcttctggctggaccatgagacttctgattctgactctttcattaataacgctggcggggtgtacggttactcgccaagcccatgtgagcgaagttgacgcggcaacaggtattgtacggttagtttatgaccaggcttttttgcagcatgcccataccgatcgttatgtcagtcgcgggatcgccgatcgcgcatgccagcaggaaggctatacccacgcggtcccctttggtcagccagtaggcaactgtagcctttttgcgggttccttatgtttgaatacggaattcactttgtcatatcagtgccatcattccgccttccctgtctttctctaaatattttaatcagcgaggggatcttcgctgattaaagaaatagcggtaatgcgttttattcccattcgtatttttaataattgaagtttatattttaccttttgcaaataataaaataacaaattatagtgacgccacagcaacaaatataacctttgtggagcactatcatgctgaaaccagaaatgattgaaaaacttaatgagcagatgaacctggaactgtactcttcactgctttatcagcaaatgagcgcctggtgcagctatcataccttcgaaggtgctgccgcgttcctgcgccgtcacgcccaggaagagatgacgcatatgcagcgtctgtttgattacctgactgataccggcaatttaccgcgtattaataccgttgaatctccgtttgctgaatattcctcacttgatgaattattccaggaaacctataaacacgaacaattaatcacccagaaaattaacgaactggctcatgctgcaatgaccaatcaggactacccaacatttaatttcctgcaatggtatgtttctgagcagcatgaagaagagaaactgttcaaatcgattattgataaattaagcctggcaggcaaaagcggcgaaggtctgtattttatcgacaaagaactctctaccctcgacacacaaaactaatgctctccggcggcaggtttactgccgccgtttcaaatcagtgacggcaaatcttactctgatcggtcgaaaaaccgtctttcgaaggtataaatttgccttttgctgccagaaacgctaccagctctcccgctgtcatcccttctgccgagcaggtgtgaaaacgtgcctgttcaccaaaacgcgctttaatcgcagcttccagactggcatgcgtatattgctcgcctgattcaatcatcatatttaacacttcatgaccgtgaatagagtccatcgtccctcctcaaaaaaagcctagcgtagcgattgccgcttatgaagactttgcgccagcgcaggactgaatgctttttattgtacatttatatttacaccatatgtaacgtcggtttgacgaagcagccgttatgccttaacctgcgccgcagatatcactcataaagatcgtcaggacagaagaaagcgtgaaaaacagaaccctgggaagtgtttttatcgtggcgggaaccacaattggcgcaggcatgctggcaatgccgctggctgcggccggtgttggttttagcgttacgttaatcttgttgattgggctttgggcgttgatgtgctacacggcgctattactgctggaggtgtaccagcatgttccggcagataccggtctgggcacgctggcaaaacgctatctgggacgctacggtcaatggctgacgggcttcagtatgatgttcttaatgtatgctctgactgcggcatacatcagcggtgccggtgaattgttggcctccagcatcagcgactggacaggtatttctatgtcggcaaccgctggcgtgctgttgttcacttttgttgccggtggcgtggtttgtgtcggaacttcactggtcgatttatttaaccgttttctgttcagcgccaagattatttttctggtggtaatgctggtactactgctgccgcatattcacaaagtgaatcttttaaccctgccgttgcaacaggggctggctctgtctgcaatcccggtgatttttacgtcgtttggttttcacggtagcgtgccgagtattgtcagctatatggatggcaacattcgtaagctacgctgggtgtttataatcggtagtgcgatccccctggtggcatatattttctggcaggtggcgacgcttggcagcattgattcaacaacctttatgggattgctggctaatcatgctggattaaacgggctgttacaggcgttacgcgaaatggtggcctctccgcatgttgagctggcagtgcatttatttgctgatttagccctcgccacgtcatttctcggcgttgcgttaggcttatttgattatctggctgatttatttcagcgttcaaataccgttggtggacggttgcaaactggtgcaattacgtttctgccgccgttggcgtttgcactgttttatccacgaggatttgtgatggcgctgggttacgccggtgtggcgctggcggtactggcattgattatcccttcgctgttgacctggcaaagcagaaagcacaatcctcaggcgggttaccgggtcaaaggtggtcgtccggcgctggtggtggtgtttctctgtggtattgctgtgattggcgtgcaatttttgattgcggcagggttgttaccagaagtggggtgatcagatagcctcaaattccttattgggtgccagaattaacgctgacacccaatttggcctcttaatgcaggcagcactgcttaaatttcttaccactaccgcacgggcaaggatcgttacgccccggtttctcttctgctttgatcggttgctgaacagctttttcctgcggatgcgccatccagtacgcatgtagatcaagcgccgccagtcgaatggcatctacgctctcttcaaacgcttctggcgacatcttttctacccgctcgaagttttcctcagtaccgtgcagcgcaatcgcctccagcgctggttttaacgaatcgggcaacgttgaccagtcagaaagtgccacgccccgcatatagccaaagcaccactcctcaacaatcgtcagctcgctgccatcaacttctcgcaagccgaataacggctcaaactgctccgggaattcgttcagacgctctgcggtatcggccatatgttgaaaagccagattcataaagcgcgtcatctctttctctgacgcccagcgcggcacatagtcagccccaccccacacggcaaccagccactgttccggttcaatctcttgcggagaactcaacaccgccgtcaataaaccgtccagctccgccacatcaaggatggcgtggtcagtgttgtatttggtcagaatatcgtccagccattccaactcactttcgtttaacggtcccgttttcatacgcttttccttgtggatctcaactcgccagcacctatcttacatgccggtccgtatcagagatactttttgagtggctttgctggtgattaaaaattaaggagggtgtaacgacaagttgcaggcacaaaaaaaccacccgaaggtggtttcacgacactgcttattgctttgattttattcttatctttcccatggtacccggagcgggacttgaacccgcacagcgcgaacgccgagggattttaaatcccttgtgtctaccgattccaccatccgggctcgggaagaaagtggaggcgcgttccggagtcgaaccggactagacggatttgcaatccgctacataaccgctttgttaacgcgccaaattcttcaggcctttcagccagacatccgcttgacgccgatgtcttttaaactggagcgggaaacgagactcgaactcgcgaccccgaccttggcaaggtcgtgctctaccaactgagctattcccgcattcatcaagcaatcagttaatcacttgattttattatcgtctggcaatcagtgccgccgttcgatgcgttgcattctacttacctggcgcgatgagtcaacgatatttttcaccacttttgatcgtttgctgaaaattacgccgaaacgatcactgatcaagcaaatctgcacgcgcagcgctcaaatattgcaacattgaccacagagtcagtaccgcagccacaaagaaaagtgcaataccggcgtactcaacccaaatgttcggacgccacagcagccatgccaacgccaccatctgggcagtggttttcactttcccaatccaggagacggccacgctactgcgtttacccaactccgccatccattcgcgtagcgcagaaataataatttcacgggcgatcatcgttgccgccggtaatgtcacccaccagctgtgataatgctcggttaccagcaccatggcgatagccacgagaactttatctgccacagggtcaaggaaagcaccaaaccgggtactctggttccagcggcgtgccagaaaaccatcgaaccagtcagtcaccgccgcgacgcagaaaatgagcgcggcggcaaacggcgaccaggtgacaggcagataaaagaccaatacaaagaatgggataaggatgacacggaacagtgtaagcaacgtagggatattaaattgcataatgacgggtaactatctgttgtcagtaagattacccctatgttgctacagagacatcaatgtttcaacgaccagaagatcttttctgccagaccttgcgaaatacccggcacttttgcaatttcctcgacgctggcgttacgtaaaccttgcaaaccgcccatatatttcaacaacatttgccgacgttttggcccgacgccttcaatggtttccagggaactggtatttttgaccttcgcccgttttttacggtgcccgccaatcgcgtgatcatgtgattcatcgcgaatatgctggataacatgcagcgcgggtgaatctggcggcaaactaaatccctcaccttccggctcaaagaacagcgtttccagtccagccttacgatctgctcctttggcaacgccaagtagcagcggatgatttttatcccatgagacatccagttcggcgaagacatttttcgcctgcgcaagctggcctttgccgccgtcgataaggatcacatccgggatcttactgtcgtcaatggctttaccataacgccgacgcagcacctgattcatcgccgcataatcatcgcccggcgtgatgcctgtaatgttatagcgccgatactccgcacgcagcgggccgttagcatcaaacaccacacaggaagcgacggtttgttcgcccatggtatggctgatgtcaaagcactccatccgcttcacttccggcaatttcaacacgctggcaagcgcggtcagtcgctggtgaacggtagattgctgcgaaagtttgctggttaaggccgtcgccgcattggtgcgcgcgagtttcagataacgcgccctatcgccgcgaggtttggtttgaacattaatcttgcgtcccgccagttctgaaagggaatcggcgagcagcgttttatcgctaagattaaaatcgagcaggatctcacccggtaaggtgcgcatctggctgccttgtaaatagaactggcctacgaaggtttctaccacctcgctcagttccgtaccgccaggcactttcgggaaatagctgcggctgccgagcactttgccctgacgaatgaacaatacgtggacacaagccatgcccgcatcgaacgccacaccaataacgtcgaggtcgtcgccggtattggaaacgaattgtttttcggtgacgcgtcgcaccgcctgaatttggtcgcgaatacgtgcagcttcttcaaactccagattctggctggcagtttccatacgactaatgagttgcgtaagcacctgatcatctttgccagacaaaaacaggcgcacatactcgacctgctgagcgtattcttcttcactcaccagtccttcaacgcacggtcccagacagcgccctatctggtattgcagacacggacgcgagcgattgcgataaacactattttcgcactggcgaatggggaaaatcttttgcagtagcgccagtgtttcacgtacggcatagccattcgggaacgggccgaaatattcacctttggcatgcttcgcaccacgatgcatcgccagacgcgggtgggtatcaccactcaggaagataaaaggatatgatttatcatcgcgtagcaaaacgttgtaacgcggctgatagagtttgatgtagttgtgttccagcaacagcgcttcggtttctgtgtgagtaaccgttacatcaatttgctggatctgggcgaccagcgcttcggttttgcgcgaagcgaggttgctacggaaatagctggaaagccgttttttcaggtctttcgctttgccgacatagataaccgtaccaccagcatcgtacatgcgataaacgcctggctggctggttacggtttttaaaaacgcttttgcgtcaaactgatcactcactgacttgataatgtctccgcattacacagaccatggcgaattgccaggtgagtcagctcaacatcgccatgaatgtttagtttactgaacatacgatagcggtagctgttcaccgttttcggactgagattgagctgttctgagatctcattgaccttctggcccttggtgatcatcagcataatctgcaattcacgttcagacaaactggcaaatgggctttctgttttttctggttcgatctggcttaacgccatttgttgagcgatgtcagaagcaatgtaacgctgccctgaatagacagaacgaatcgcactcacgacttcctgcggagccgcgcctttgctgaggtagcccgcagcaccggcctgcatgactttcgctggtaaagggttttctgtatggacggtaagcatgatgattttgacatcagctgtggaacgcgcgattttacgcgtcgcctcaagaccgccaatgcccggcatactcatgtccattagcaccacgtcaacggcatttgtccggcaccacttaacggcgtcttcaccgcacgatgcctcaccgacgacttttataccctttatatcttccagaatgcgtcgtatccctgcgcgcaccagttcgtggtcatcaacaagtagaacgttgatcaaaggaatatctccagaaatagggataacgctactgatagttagtcattcgtatattagcggtttttattgcaactttgaaacgttaaaaatggtgggtattcgatttttctctcgtttttgtcaattcgattgtccacagttatggtcacgcccgtcaccaacggcttaccggatcgtttcacagtaagccctacgatgaaatgtgacaaaaattgactttattcagcaaaaatgaaaatcagcccgctgaatatgtaacattaattaacccgaacaatacgggcaaaaaacattcatgataaaaatatttattggtcattatattaacgtattttatagcactgccgatatcacgctcaaaaaacaaccactgctatttttagcaaagcttatggtatactccgccgccttaacatttttcaccgcaaattttcattgcaacatgacgaggaaaataaatgagtacgcctgatttttctactgccgagaataatcaagaactggcaaatgaagtctcctgcctgaaagcgatgctgacgctgatgctgcaggcgatgggacaagctgacgcgggccgcgtgatgttaaagatggaaaaacagcttgcgctgatcgaagacgaaacccaggctgcagtattttccaaaacggttaagcaaattaaacaagcctaccgtcagtaatataaaaccggctgatagcgtgcctttcagccggtttttgcatctggcacgcaggacagaaaagagatcaaattaagccagtagcggccgcgtaacaggcaacctgggtcttatttggtgcattaatttttttctgcatgtttttctggtggaaattgaccgtattctcagagattgacaaaatcatcgctatctctgctgatgttttcccttccgccgtccacctcagaatttctttttcgcgcttgctgaaattcatctctggcgtcatcactatttcatcatttaaacgcatcagagccatcagactttcgcgcaccagtaactgcatttttaattgcagttcatcactaagaatgggtatttcgcgcgcgctgcaacgggaaaaggacaaaaagcccagcgcccggtttggcagcattaaatactgagtgacaccgcggcgtaaaccatgtgcgcgcgcggcttcccataacggctgtgcttcgctgaataagtcatcattccacattaaatggccctgactaaagttttcagggttcagcaccggatcaattgcgagaaagttttttgcctgataataactaacccacgcctcagggtaattggtgtaaaaagccactttaggtcgagtgaatggtaccgggtggcggacacataacgaatagtaatcgtactccagctgctgagcctgaagctcaatttcatggtagacctcttctgcggtctccatcctctgaaaacgcaacagcatcgtgcgacgccagctgaaaaaatccttatcctgcatagtaaaccgcaacgcccctgagagtgagtatcatttataatgataattcaaactatcacataaataagatttatatataatttatattattcaggcaatgaattacttttgcaagccatcgcattctcttatgttattaatgagttatgctgatttgttaagcagttttatcaggcttgaaatggcgtccagccccgacaggtgaatcgtcggggctgattttttcttattattgcagcagaaacttctcgaggaactggcgggtgcgaggctgctcggggtcggcaaataacgcttttgcggccccctgctcgactatccgcccctggtccataaagatcgcccggtccgcaacatcccgggcaaagctcatttcgtgcgtcacaatcaccatcgtgcgcttttcctgcgccagctgacggatggtgttcaggacttcacccaccagctctggatccagcgctgacgttggctcgtcaaacaaaatcacctcaggacgcattgccagcgcacgcgcaatcgcaacacgctgctgttgaccgccagacaaacgacgtggatagctggtttctttacctgccagcccaacttttgccagcagctcgcgagcgcgcgccgtggcctcttctttcggttcacctttgacgatcaccggcccttcaataatgttctccagcaccgtacgatgcggaaacaaattaaagttctggaagacaaacccgacgtgctgacgcaactggcgaatcagagatttttgctgacttaatgaacgtgcagtatcaatagtgatatcgccaacggtgatcgttcccgcttcgggttgttccagcagatttatgctgcgtagcaacgtggttttgccggaaccactcggaccgataattgccaccacttcgccaggctttacctcaaggtcgataccgtgcagcaccgtctgaccgtggaattttttcaccaggttcttaacttcaatggcactcattttggttctctctcctggcgattaagttgattctcaaaatggttctgcaacgtcgataacacagtcgccatgatccagtagatgagcgaagccgccagatacatggtgaacacctccagcgtacgcgaggtaatcaactgcgcctgacggaacagctccggcacctggattgtcgcggccagcgacgtatcttttaccaggctaataaagctgttcgacagcggcggcaacgccacacgcgccgcctgtggcaaaatcgcgcgacgcatggtctgccacggcgtcataccaatactggctgccgcttcccactgacctttatcaatagaagaaatggcggcgcgcagcgtttcggcagcataggcggcagtgttcaacgacagaccaatcattgctgacggaatgggatctaattcgataccaaactgcggcaggccgtaatagatcataaacagttgtgcgatgagcggcgtaccacgaaaaatagagatataaaaacgcgccagccagcgcacgggccagattggcgacagacgcatcagcgcgagaataaacccgagcagtaagccaaaaaacatgccgccgatactgagttgcagcgtatacccagcccctttcagcaggaacggcaaggaatcaataaccagttgtatactttcttgcatgagcgtttccggagctaaacgtggggatgataggcgaacagcgcaggcgcaccgccggtatgaataaacagaatcggcccttcatctttgaagcgtttctgactgataccgtcaatcagccccgccatcgcttttccggtatacacaggatcaagcagaatgccttccagccgcgccagcaatttcactgcttccatgccttcgtcgttcggcacgccgtagccaggtgcaaaatagtcatcccagagtaaaatttccgctgatgcggtcagctccagttctttcgcaatcgcctgttgtaggttaaccactttcggcaattgatcggcaacggaacgcgacacggtcacgccaatcagttcgctttcaggcatcaggtgttccagcccaacagccagtccggcgtgagttccggcactgcccgatgcgactaccaccgatgaaatattaaccgccccttcacactgttgcgcgatttccagcgcactctccacataacctagcgcgccaagagcattagaaccgccaaccggaatgacatacgggcgaaagccttgtgcttcgactcgcgtcgccagctcttccagttgggcattgggatcggtcagtgcgtcgcacatttcaatctgggtattgaacagatccagcaacaagcgattgccgttggttaaatagttttctgcggttgtgccaataggattttccagcagcgccacgcagtgcagaccgagtttggcagcgactgcggcagtctgccgcacatggttagactggatcgccccggcagtaatcagcgtatcggcaccttcacgcagagcatctgccgcgagaaattccagcttacgtaatttattgccgcccattgccatgggggtgacgtcatcccgtttgatgaaaatttcccgtcctagataatcagaaaagcgcggcagatattcgagcggcgttggcgcgccgataaactccagccgtggaaaacgggttaaattatgcagtggcataacagcctccgatgtgtgttgttgtgattttcttattatgcacgctgaaaacgcgtaaataaaaaaggcgctagtgaaagcgcccttttttgtcattatgctgattatttggtcacatcagcaccaaaccatttttcggaaagggcttgcagagtgccatctttttgcatttccgcaattgcatcattcactgctttcagcaggtcctcatttcctttacgcagcgccacgccagactcctgacgggagaatgcttcaccggttactgccagcgtatcgttggttttcttcaccagatccagcgccgccagacgatcaacgaggatcgcatcgatacgccctacgcgcagatcctgatatttggtcgggtcatcatcataggtacgcacatcgacgccctgaacattctgccgcagccactcttcatagttggtgcccagaccgacccccacttttttgcctttcagatcatcggctgttttaatggtgccttcgttaccttttttcaccagcgcctgaataccagaaatggtgtacggggttgagaaatcgtattttttcttgcgctcatcagaaatggtgacctgattaatcaccacatcaatacgtttagagtccagcgacgccagcataccgtcccatttggtcggttttagtgacgcctcaacgccaagatgttttgccagctgttgggcaaattccacttcaaaaccggttaatttgccgtcatctccctgaaaactgaacggcggataagttccttccagccctaccagcagcgtgccgcgctctttaactttattaagcagaccttcatctgcaaaacttttaacgctcatgcccgcaaccagcgccacggccatcacacccatcaatgcctgacgtcccagatgtgctaatttcatattcaccccgaatgttgttatgtctgtttgcagtgtagagccattgtttgtaaacacaaaaacaactccgctacatcttattcttatttaatatatatcagaagaaggcaggctggaggatttctgcacaagtctggtacaggtttggcgctgatagtgttgatacttccgtaacgcgatgcggtaattgttggtgctggtggtgggcagccacggggcgaggatttcatcaaggaaaccgtcctgcagctgatcgagggaaatattttgctcgtgtagatgattccccaaacggcgcaaacgaacgacatattcacgcaccgtacctgggctcatttcagtttgctcaaaaagaaattgcttaaagccgataatatcgaaaaaatcactctgcgttttgcaatgtaaatcaccgcaaaatcggcacaatgccgcccatgatttttgttccgtttgccagccattttcatcaagcagcgtgtccaggcgggaaatctcgattttattcactattttgccgtcgcgaactaaggtaatgcgatcgagtaatttacggcaatgcgcgcaatgggtctggctgtgtttaaagtctttaagatagcggcttaatggccgtcttttcaggtgctgcaccatcattaagaactcctggtagtcaaagttaaagtgcggcatttactgacgttataacttacccagtttagtgcgtaaccgtttaatagcctggctgtgtaactgactgacccgcgattccccgacctccagcaccgcgccaatctctttgagattcagctcttcctggtaatagagggttaataccagtttttcgcgctccggcaacgtttcgatggcttccatcacccgctggcgcagattactgtccagtagttgttgtagcgggttttctcgctgatgatcatcagtaaccagttcgatgctatcgccgtgctcttcgcgccactcatcgtaggagaagagctggctgttattggtgtcgagcaacatttggcgataatcggcaatatcgatccctaaacgttccgctacctcagtttccgtggcgttgcggccaagttcctgctccagttgccctattgcctgtgccacttcacgcgcgttgcgtcgcacgctgcgcggcacccagtcacggctgcgaagttcatccagcatagcgccacggatacgctgcactgcgtaagttgtaaatgccgttccttgtagggcgtcatagcgttcgacggcattaagtaacccaatgccgcccgcctgtagcagatcgtcaagttccacgctcgcgggcagtcgaacctgcaggcgcaatgcttcgtgacgcaccagcgggacataacgctgccacagcgagtgtttatccattacaccttcagcggtatagagtgaattcacgataaacagccctgcgttatatgagttatcggcatgattatccgtttctgcagggtttttaatcggacgattagtgggtgaaatgaggggttatttgggggttacaggtaaattccaggcagaaaaaaaccccgccggtggcggggaagcacgttgctgacaaattgcgctttatgttgccggatgcggcgtaaacgccttatccggcctacaaaaatgtgcaaattcaataaattgcaattcaacttgtaggcctgataagcgcagcgcatcaggcaatttggcgttgccgtcagtctcagttaatcaggttacaacgattaaccctgcagcagagacagaacctgctgcggtacctggttagcttttgccaacacggagttaccggcctgctggatgatctgcgctttcgacatattggacacttcggtcgcatagtcggcgtcctgaatacgggactgcgcttcagacaggttggtagtggtgttgttcaggttggtaaccgcggaatccagacggttttgcaccgcaccgagggaagaacggaatttgtctacagatgcgatagcatcgtccagcgctttcagcggatccgtggttttaccatttgcaacagcagtcagagcctcaccaccagcagtcaaacctgtttgcagattaccgccatttaaatcggcagaatcgtatgttttaccatcaatatcgaccacttctgttttgccatcatctccgcccagtttgaccgcggttggagaactggcggcaccggaagagtcagtataggtaatagttttaacagaaacagcaccagtagtttcattcacatccgcagcgtaaagattgccatttgtatctttaagcgcatatgtatcggtatcattacccttggaatcctgcagttttactaagctaacagcaccaaggttggcagttgcggaacctgcagtattatcaatctgaacaggtgtaccgcctgaagtgatagttgtagctttagtagtatttgcatcagttacagttgcatttgccgttgctccagtcgccattgtcactgtaccatcattagcaactgttactgcgtaatacttcccatcgttatcaccaccggtgattttcgcatagtaatcattaccattatcagtataaacaccctcaattgaagctgggttagttccgccagtatcagtggctgcttccgtagaaagggtaattccagtaagtttaatattgtttgtggtggtagcaccaaaagcagttactggagcactagtggtaactgtatcgttatttttaacgctaaaaccatcaaggccaagagttttagcatcaatctgcttcagatcgatagtgatagtctggttatcatttgcgccaacctggattttcatggagccattttttgccagcacgttcacgccgttgaactgggtctgaccagatacgcggtcaatttcatccagacgggatttaatttcgtcctggatagaagacagatcagactcagagttagtaccggtagtggcctgtaccgtcagttcacgcacacgctgtaagttgttgttgatttcggacagcgcgccttcggtggtctgcgcaacggagataccgtcgttggcgttacgggccgcctgagtcaggcctttaatgttagaggtgaaacggttagcaatcgcctgacccgctgcgtcatccttcgcgctgttaatacgcaagccagaagacagacgctcgatagaactcgacagcgcagactggttcttgttgatattattttgagtgatcagcgagaggctgttggtattaatgacttgtgccatgattcgttatcctatattgcaagtcgttgattacgtattgggtttccacccgtcggctcaatcgccgtcaaccctgttatcgtctgtcgtaaaacaacctttagaatttttttcaaaaacagccattttttgttagtcgccgaaatactcttttctctgccccttattcccgctattaaaaaaaacaattaaacgtaaactttgcgcaattcagaccgataaccccggtattcgttttacgtgtcgaaagataaaaggaaatcgcatggcaagtatttcatcgctgggagtcgggtcaggtctggatttaagttccatccttgatagcctcaccgccgcgcaaaaagcgacgctaacccccatttcaaatcagcaatcgtcgtttaccgctaaacttagcgcctacggtacgctgaaaagcgcgctgacgactttccagaccgccaatactgcattgtctaaagccgatcttttttccgccaccagcaccaccagcagcaccaccgcgttcagtgccaccactgcgggtaacgccatcgccgggaaatacaccatcagcgtcacccatctggcgcaggcgcaaaccctgaccacgcgcaccaccagagacgatacgaaaacggcgatcgccaccagcgacagtaaactcaccattcaacaaggcggcgacaaagatccgattaccattgatatcagcgcggctaactcatcgttaagcgggatccgtgatgccatcaacaacgcaaaagcaggcgtaagcgcaagcatcattaacgtgggtaacggtgaatatcgtctgtcagtcacatcaaatgacaccggccttgataatgcgatgacactctcggtcagcggtgatgatgcgctacaaagttttatgggctatgacgccagtgccagcagcaacggtatggaggtctcggttgccgcccagaatgcgcagctgacagtcaacaacgtcgccatcgagaacagcagcaacaccatcagcgacgcgctggaaaacatcaccctgaacctgaacgatgtcaccacgggcaaccagacgctaaccatcactcaggacacctccaaagcgcaaacggcgattaaagactgggtgaatgcctacaactcgctaatagataccttcagcagcctgaccaaatacaccgccgtagatgcgggagctgatagccagagttctagcaatggtgcactgctcggcgactccacgctgcggacgattcagacgcagttgaaatcgatgctgagtaataccgtcagttcttccagctataaaacgttggcgcagattggtatcacgaccgatcccagcgatggcaaactggaactggatgccgacaaactcaccgctgcactgaaaaaagatgccagcggcgtaggtgcattgattgttggcgatggtaaaaaaaccggcatcacgaccaccatcggcagcaacctgaccagttggctttcgacaacgggcattattaaagccgctaccgatggcgttagtaagaccctgaataaattaactaaagactacaacgccgccagcgatcgcattgatgcgcaggtcgctcgctacaaagaacaatttacccaactggacgttttaatgacctcgttaaacagcaccagcagctacttaacgcagcagttcgaaaacaacagtaattccaagtaagcaatattcatcgggagacaggtcatgtacgcggcaaaaggcacccaggcctatgcacaaattggcgtcgaaagcgccgtaatgagcgccagccagcagcagctggtcaccatgctatttgatggagtgctgagcgcactggttagagcgagcctgtttatgcaggacaacaatcagcaaggcaaaggcgtctctttgtcaaaagcgatcaacatcattgagaacggactgcgggtgagtcttgatgaagagagcaaagacgaactaacccaaaacttgattgctctttatagctatatggtcaggcgcttgctgcaagccaatttacgcaacgatgtctccgcagtcgaagaagtggaagcattaatgcgcaatattgccgatgcctggaaagagtcgttactctccccttctttgattcaggacccagtctgatgaaccatgcaccgcatttatatttcgcctggcaacaactcgtcgaaaaaagccagctcatgttacgcctggcaacggaagaacaatgggacgaactcatcgccagcgaaatggcgtatgtgaatgcggtgcaggagattgcacatttgactgaagaggttgacccgtccaccacgatgcaggagcagctccgcccgatgctgcgcctgattctcgacaacgaaagcaaggtaaagcagttattacagattcggatggatgaactggcgaaactggtcggtcagtcatcggtgcaaaaatcggtgttaagtgcctatggcgatcagggcggctttgtgctggctccgcaggataacctcttttgaatctgaatgagtcgatggctcgcgaataatccgattacggctacgcttctaatgttccccttgaatggagtcgaagaatgcgtaatcccacgctgttacaatgttttcactggtattacccggaaggcggtaagctctggcctgaactggccgagcgcgccgacggttttaatgatattggtatcaatatggtctggttgccgcccgcctataaaggcgcatcgggcgggtattcggtcggctacgactcctatgatttatttgatttaggcgagtttgatcagaaaggcagcatccctactaaatatggcgataaagcacaactgctggccgccattgatgctctgaaacgtaatgacattgcggtgctgttggatgtggtagtcaaccacaaaatgggcgcggatgaaaaagaagctattcgcgtgcagcgtgtaaatgctgatgaccgtacgcaaattgacgaagaaatcattgagtgtgaaggctggacgcgttacaccttccccgcccgtgccgggcaatactcgcagtttatctgggatttcaaatgttttagcggtatcgaccatatcgaaaaccctgacgaagatggcatttttaaaattgttaacgactacaccggcgaaggctggaacgatcaggttgatgatgaattaggtaatttcgattatctgatgggcgagaatatcgattttcgcaatcatgccgtgacggaagagattaaatactgggcgcgctgggtgatggaacaaacgcaatgcgacggttttcgtcttgatgcggtcaaacatattccagcctggttttataaagagtggatcgaacacgtacaggaagttgcgccaaagccgctgtttattgtggcggagtactggtcgcatgaagttgataagctgcaaacgtatattgatcaggtggaaggcaaaaccatgctgtttgatgcgccgctgcagatgaaattccatgaagcatcgcgcatggggcgcgactacgacatgacgcagattttcacgggtacattagtggaagccgatcctttccacgccgtgacgctcgttgccaatcacgacacccaaccgttgcaagccctcgaagcgccggtcgaaccgtggtttaaaccgctggcgtatgccttaattttgttgcgggaaaatggcgttccttcggtattctatccggacctctacggtgcgcattacgaagatgtcggtggtgacgggcaaacctatccgatagatatgccaataatcgaacagcttgatgagttaattctcgcccgtcagcgtttcgcccacggtgtacagacgttatttttcgaccatccgaactgcattgcctttagccgcagtggcaccgacgaatttcccggctgcgtggtggtcatgtcgaacggggatgatggcgaaaaaaccattcatctgggagagaattacggcaataaaacctggcgtgattttctggggaaccggcaagagagagtagtgaccgacgaaaacggcgaagcaaccttcttttgcaacggcggcagcgtcagcgtgtgggttatcgaagaggtgatttaaattcatccccggcggcaagccggggagatttcattacggcagtggcgtcggtaacggcgctttatccagcgcggcggcacactctgctgtcgggcgatccacacgctccatcgtcataccatcgtactcaatggtgttaccgtcacgctcaacctcgtacagctcacgttttacggtaacgttagtgagatcatcagacatcaatgtcaacttacccggcacggcaatcacccgctgccactgacggcaatccagggtatcgccctctttagtgacaatcaggctgcctatcgcttccgggctgaccagcgcacgttgcggccctttggtctgccagtagcccgccagccagtccggcgcgggggttttcacgacattgttatagttttcgacttcggcacagcccgccagcaacaagagcgcgcctgcaattgcgagttttttcatcattcgtcctgcatgagaagaaaagaggattgtggcattaaagccctgatgtcgccagcctttcaaggttcagagagaaatttgatctaactattatttttgtgaattattaccccgaaaataaatttgcatggtgtatgattcgcgactcttgtttcaaaccttctgagttcagaggctacattcatgtcatggcagcaattcaaacacgcctggttgattaaattctgggcccccatccctgcggtcatcgcggcgggtattctctctacttactattttggcattactggcaccttttgggctgtcacgggtgaatttacccgttggggcggccagctcctgcaactgttcggcgtccatgctgaagagtggggttactttaaaattatccatctggaaggatcgccattaacccgcatcgacgggatgatgatcctcggtatgtttggcggctgctttgccgcagcgctgtgggccaacaatgtcaaactgcgaatgccgcgcagccgtatccgcattatgcaggccatcattggcggcattatcgccggttttggcgcgcgtctggcaatgggctgtaacctggcggcgttctttaccggtattcctcagttctcgctgcatgcctggttctttgccatcgccactgccattggttcatggtttggcgcgcgctttaccctgctgcccatcttccgtattcccgtgaaaatgcagaaagtttctgccgcctcaccgctgacgcaaaaaccggatcaggcgcggcgtcgttttcgtctcgggatgctggtctttttcggcatgctgggctgggcgctgctcacagcgatgaaccaacccaaactggggctggcaatgctgtttggcgtcggctttggtttactgattgaacgtgcgcaaatctgctttacttcagcgttccgcgatatgtggatcaccggacgtacccatatggcgaaagcaatcattatcggtatggcggtgagtgccatcgggatcttcagttacgtacagttaggcgttgaacccaaaatcatgtgggcgggaccaaacgcggtaattggtggtttactgtttggttttggcatcgtgctggctggcggctgcgaaaccggctggatgtaccgcgcggtagaaggccaggtgcactactggtgggtcggtctgggcaatgtgatcggctcaacgattctggcgtattactgggatgatttcgctccggcgctggccaccgactgggacaaaatcaacctgctgaaaacctttggtccgatgggtggcctgctggtgacatatttgctgttgtttgctgcgctgatgttgattatcggctgggaaaaacgcttcttccgccgtgcggcaccgcagactgctaaggagatcgcatgaaaaatatcgttcctgattaccgccttgatatggtgggtgaaccctgcccttatccggcagtcgcaacccttgaggcgatgccgcagttaaaaaaaggggaaatcctggaagtggtgagcgactgtccgcagtcgatcaataatattccactggatgcgcgtaatcacggctatacggtgctggatattcagcaagacgggccgaccattcgttatttaattcagaagtaatccctcattcccgctgtgacccacagcgggaacatcgttacctttgtatcacatagattttacccgcccccactcctattcttttcagtatgatctcaggaggtttctatgtgtggacgctttgcccaatcccaaacgcgtgaagattaccttgcgcttctcgcggaagatattgaacgcgatattccctatgatcccgaacccattggcagatacaacgtcgcgccgggaaccaaagtcctactgctcagtgaacgtgatgaacaccttcatctggatccggttttctggggatatgctcccggatggtgggataaaccgccgctgattaacgcccgcgtagaaactgcggcaaccagtcgtatgtttaaaccgctctggcaacatggtcgggcaatctgttttgccgatggctggtttgagtggaaaaaagaaggcgacaaaaaacagcctttttttatctatcgtgctgatggacaacctatttttatggccgcgataggtagcacaccatttgagcgtggtgacgaagccgaaggatttttgatcgtcactgctgcggcagatcaaggtctggtagatattcatgaccgccgcccactggtactgtcgccagaagctgcgcgggaatggatgcggcaagagattagcggtaaagaagcctcagaaatcgcggccagtggctgtgttccagcaaaccagttctcctggcacccggtatcgcgcgcggtgggtaatgttaaaaaccagggcgcggagttaattcaacctgtttgataagcctggagattattgatcaacaatactgcgtcataagaaatctctattagacaaagatttcattacctgttggcatattgcaaaaataacaccaatacggaatcgtcatgttcacgattaaaacagatgatctcacccatccagcagtgcaagcattagtggcttaccatatttccggcatgctgcagcagtctccccccgaaagcagtcatgctttagatgtgcaaaaattacgtaacccgacagtgacattctggtcagtatgggaaggcgaacaactcgcaggaattggtgcgctgaagttgctggatgataaacacggcgagctgaaatcaatgcgtaccgcgccaaattatttacgtcgtggtgtcgccagtctgattttacgccacattttgcaggtcgcccaggacagatgccttcatcgcctgagcttagaaacgggtacacaggctggatttacggcctgccatcaactttatttgaagcatggtttcgctgattgcgaaccgtttgctgattatcgacttgatccacacagtcgatttttatcattgacgctatgcgaaaataatgaattgccatgagccagacgcagcacattcttgcattcgacgtgctgcgcctttatttatcaccagcaggaaacgccttgtccatagacgccccttccacatgcgccacaagaaacctctattccagtgacacaattgcgcctaattaattacatttaatatttaattatgagttcctcaccatctattacatactttttaaccatatcggaatatttatcataatcagcgggattcgtaacaatatattttcgctgcgatctttcatagcaaatccctgtcaaagtccatgatataaaaatgtctcttcaaaagaattacattctttaaaaagtaattctttattgctatatatcgcagagacaacctcaatatcacactccatacgtgctttctccagatgatttgggaagtattgaatttcttttatcttattatcgccacaattaaacagcttagtagtctcaggcattgctggtatttaccatattttattgcgataaatagaaattgtcatagcctttgacggagatgagtcaacacgcgatatcagattattatctacggagacctgggtaattccatcggatacttttggaaataccatataattattgaaatcgagctctaattctttgcagaatttgggaatttgtattgtggcaaggccattatgacgaagataaagcacctcaatccaggatggaagaggtggcaaagaccccaagtgaagatctgttaagtcaagtttactattgtggagttcaacacatttaaacaatctcaccaatgctatatccacattttttttgaagtcattcgatgcgccttcttttactgaattagcccagtcgctgaaacctttgcaaagtctggaatctgtaattttcgtaaagttgtctagaaactctgcaatattagtcgatataaactctaatttatgccgaatgggtgggttaccagttccctgattttttctatcatgataaaacctatcttattataaatcgagaaatcttgaaaccagagactataatcaccccattcgaaatattctgagtgcaataacttaaattctgacagcatattaaataatttgctgtcttcactaattggtgtaaacttaccatttccaagacaactgactaactcacttgataattcatttatgattgcatcatcagatactaactcatgttgttttatcgtagattcagtattagatgtgactttatttaattgaaccggctgagtttttaacgaaagatcatttaatggaaacatttacactcctgtttaataaattatattgcccagggcgcattctaaaacacaataaaattaccactatcaaaaatcgctcatatccatcgcccggaatatgaataaaaacatcaacaaagattaaattatccagaggttactgttgcgtctgtggtcgtaacaacatccgacgtggtgatgtgtcaaatgagacgctctgatgttcaggggggttatcgcgtatacggatcgtggatggcagaaaacgttcaggatcaggtatccattttaaaccagaaattgagtgagtttgccccatccatgccccacgcggtgagatcggatgtaattaacaacaggttacaaaacctacacctgcatgctcatcacttcctgatacgccgccaccagcttattacgcacctgaatccccatttgcatagaaactgaggctttttgcatatcggtcatcacatcgtttaacgccacgccgggttcaccgagagtgaatttttctgcctgcgtgcgggcagctgtttgtgtatcactaatgcgatcgagcgcggcgtgcagctgcccggcaaaactaatggtcggttgcggcagtgattcctgcgcacgcgcactcatcgccgtagcctgtaactggctgataaccccttcaatcccctgtatcgctgacattctcgtctcccggataatttctggtagcaaagcctaccagtaagtcaataagacaaaggcgctaaatagcaacaaaaaaacgggtttattggcggatagaaaaaaacgaaagcacaaataatgggagcgtcaatttttcgagtttgctgacccgggagtgagtcttgttccactttgccaataacgccgtccataatcagccacgaggtgcgcgatgaatgcgactgcagcccagacaaaatctcttgagtggcttaatcgcctgcgtgcgaatccgaaaattccattgattgttgccggttccgcggcagtggcggtcatggtcgcactgatcctgtgggcgaaagcccccgactaccgcacattattcagcaatctttccgatcaggatggtggcgcaattgtcagccaactgacgcaaatgaatattccttaccgcttcagcgaagccagcggcgctattgaagttccggcagataaagttcacgaactgcgtctgcgcctggcacaacaaggtttgccaaaaggcggcgcggtcggtttcgaactgcttgatcaggaaaagtttggtatcagccagttcagcgaacaggtgaattatcagcgggcgctggaaggcgagctttctcgtaccatcgaaactatcggcccggtaaaaggggcgcgcgtacatctggcaatgccgaaaccgtctttattcgtccgtgaacaaaaatccccttctgcatcggtgacggtaaatctgttacccggccgcgcactcgatgaagggcaaattagcgccattgtgcatctggtttccagcgccgttgctggtctgccgccgggaaacgtcacgctggtggatcagggcggacatctgttaacccagtccaataccagcgggcgcgatcttaatgacgctcagttgaaatatgccagcgatgtcgaaggccgtattcagcggcgtattgaagcgatcctgtcgcctattgttggtaacggtaatattcacgcccaggttacggcgcagctggacttcgccagtaaagaacaaacggaagaacagtatcgccctaacggtgatgaatctcatgcggcgcttcgttcacgccagcttaatgagagcgagcaaagcggttccggttatccgggcggcgtaccgggggcgttgtcgaatcaaccggcacctgcgaataacgcgccaatcagcacgcctccggcaaatcaaaataaccgccagcagcaggcgagcaccaccagcaatagtgggccgcgtagcacacagcggaatgaaaccagtaactacgaagtcgatcgcaccattcgtcataccaaaatgaacgtgggcgatgtgcaacgtctgtcagtcgcggtcgtggtgaattacaaaaccttgccagatggcaaaccgttgcctctcagcaacgaacagatgaagcaaattgaagatctgacccgcgaggcgatgggcttttctgaaaaacgcggtgactcgctcaatgtcgttaactcgccgttcaatagcagtgacgaaagcggcggagaactgccattctggcaacagcaagcgtttatcgatcagttacttgctgccggtcgctggttgctggtactgctggtggcgtggctgctgtggcggaaagcggtacgtccgcagctaacacgtcgcgctgaggcgatgaaagctgtacagcaacaggcgcaggcccgcgaggaagtggaagatgcggtggaagtccgcctgagcaaagacgaacaactacaacaacggcgcgctaaccaacgtctgggggcagaagtcatgagccagcgtatccgtgaaatgtctgataacgatccgcgcgtggtggcgctggtcattcgccagtggataaataacgatcatgagtaacctgacaggcaccgataaaagcgtcatcctgctgatgaccattggcgaagaccgggcggcagaggtgttcaagcacctctcccagcgtgaagtacaaaccctgagcgctgcaatggcgaacgtcacgcagatctccaacaagcagctaaccgatgtgctggcggagtttgagcaagaagctgaacagtttgccgcactgaatatcaacgccaacgattatctgcgctcggtattggtcaaagctctgggtgaagaacgtgccgccagcctgctggaagatattctcgaaactcgcgataccgccagcggtattgaaacgctcaactttatggagccacagagcgccgccgatctgattcgcgatgagcatccgcaaattatcgccaccattctggtgcatctgaagcgcgcccaagccgccgatattctggcgttgttcgatgaacgtctgcgccacgacgtgatgttgcgtatcgccacctttggcggcgtgcagccagccgcgctggcggagctgaccgaagtactgaatggcttgctcgacggtcagaatctcaagcgcagcaaaatgggcggcgtgagaacggcagccgaaattatcaacctgatgaaaactcagcaggaagaagccgttattaccgccgtgcgtgaattcgacggcgagctggcgcagaaaatcatcgacgagatgttcctgttcgagaatctggtggatgtcgacgatcgcagcattcagcgtctgttgcaggaagtggattccgaatcgctgttgatcgcgctgaaaggagccgagcagccactgcgcgagaaattcttgcgcaatatgtcgcagcgtgccgccgatattctgcgcgacgatctcgccaaccgtggtccggtgcgtctgtcgcaggtggaaaacgaacagaaagcgattctgctgattgtgcgccgccttgccgaaactggcgagatggtaattggcagcggcgaggatacctatgtctgataatctgccgtggaaaacctggacgccggacgatctcgcgccaccacaggcagagtttgtgcccatagtcgagccggaagaaaccatcattgaagaggctgaacccagccttgagcagcaactggcgcaactgcaaatgcaggcccatgagcaaggttatcaggcgggtattgccgaaggtcgccagcaaggtcataagcagggctatcaggaaggactggcccaggggctggagcaaggtctggcagaggcgaagtctcaacaagcgccaattcatgcccggatgcagcaactggtcagcgaatttcaaactacccttgatgcacttgatagtgtgatagcgtcgcgcctgatgcagatggcgctggaggcggcacgtcaggtcatcggtcagacgccaacggtggataactcggcactgatcaaacagatccaacagttgttgcagcaagaaccgttattcagcggtaaaccacagctgcgcgtgcacccggatgatctgcaacgtgtggatgatatgctcggcgctaccttaagtttgcatggctggcgcttgcggggcgatcccaccctccatcctggcggctgtaaagtctccgccgatgaaggcgatctcgacgccagtgtcgccactcgctggcaagaactctgccgtctggcagcaccaggagtggtgtaatgaccacgcgcctgactcgctggctaaccacgctggataactttgaagccaaaatggcgcagttgcctgcggtacgtcgctacgggcgattaacccgcgctaccgggctggtgctggaagccaccggattacaattgccgctcggcgcaacctgtgtcattgagcgccagaacggcagcgaaacgcacgaagtagaaagcgaagtcgttggctttaacggtcaacggctgtttttaatgccgctggaggaagtcgaaggtgtcctgcccggcgcgcgtgtttatgccaaaaacatttcggcagaagggctgcaaagcggcaagcagttgccgctcggtccggcgttattaggtcgcgttctggacggcagcggtaaaccgctcgatggcctgccctcccccgatacgacggaaaccggtgcgctgattaccccgccatttaacccgttgcaacgtacaccgattgaacatgtgctggacaccggcgtgcgcccaatcaatgccctgcttaccgttgggcgtgggcagcgtatggggctgtttgccgggtccggcgttggtaaaagtgtgctgctggggatgatggcacgttacacccgcgccgatgtcattgtcgtgggtttgattggtgaacgtgggcgcgaagtaaaagattttattgagaacatcctcggtgccgaagggcgtgcacgctcagtggtgattgccgctccggcggatgtttctccgctcctgcgaatgcagggtgccgcctatgccacgcgcattgccgaagattttcgcgatcgtggtcagcatgtgttgctgattatggactccctcacccgctacgcgatggcccagcgtgaaattgcgctggcgattggcgaaccccccgccaccaaaggttatccaccgtcggtgtttgccaaattaccggcactggtcgagcgtgccggaaatggcattagcggcggcggctcgattaccgcgttttataccgtgctcactgaaggcgatgaccagcaggatccgattgccgactccgcgcgggcgatcctcgacggtcacattgtgctgtctcgccgactggcggaagccgggcactatccggctatcgatattgaagcgtcgatcagccgcgcaatgacggcgttgatcagtgagcaacattacgcgcgagtgcgcaccttcaaacagctgttgtcgagttttcagcgtaaccgcgatctggttagcgtcggcgcgtatgccaaaggcagcgatccgatgctcgataaagccatcgccctgtggccgcagctggagggctatttgcaacaaggcatttttgaacgcgcggactgggaagcgtctctccaggggctggagcgtattttcccgacagtgtcataacccaggagataacggcagatggcagaacatggtgcgctggcgaccctgaaagatctggcagaaaaagaggtagaggatgccgcgcgcctgctgggtgaaatgcgtcgcggatgtcagcaggcggaagaacagctcaaaatgctgattgattatcagaatgaatatcgcaataacctcaacagcgatatgagtgccgggataaccagcaaccgctggatcaactatcagcagtttatccagacgctggaaaaagccattactcagcatcgccagcaacttaatcagtggacgcagaaagttgacattgccctgaacagttggcgagaaaaaaaacaacgtttgcaggcctggcagacactgcaggaacggcaatccacggcggcactgcttgcagaaaaccgcctcgatcagaaaaagatggatgagttcgcccagcgcgccgccatgaggaaacctgaatgattcgcttagcgcccttgattaccgccgacgttgacaccaccacattgcctggcggcaaagccagcgatgctgcacaagattttctcgcgttgttgagcgaagcattagcaggcgagacaactaccgacaaagcggccccccagttgctggtggcaacagataagcccacgacaaaaggcgagccgctgatcagcgatattgtttccgacgcgcaacaagctaatttactgatccctgtggatgaaacaccgcctgtcatcaacgacgaacaatccacatcaacaccgttaaccaccgctcagacgatggcgttggctgcggtggctgacaaaaatacgacaaaagacgaaaaagcggatgatctgaatgaagacgtcaccgcaagcctgagcgccctttttgcgatgttgccgggttttgacaatacgcccaaagtgactgatgcgccgtcaaccgtgttaccgacagagaaaccaacgctcttcacaaaactgacttctgagcaactcacaacagcacagcctgatgacgcccccggcacaccagctcagccattaacaccgctggtagcagaagcccagagtaaagcggaagtcatcagcacaccttcaccggtgaccgctgccgccagcccgctaatcactccacaccagacacagccactgcccaccgtcgccgcacctgttttgagtgcaccgctgggttctcacgaatggcaacaatcattaagccagcatatttcgctgttcacccgccaggggcaacaaagtgcagagttgcgtctgcacccgcaggatttaggtgaagtgcaaatctccctcaaagtggatgataaccaggcgcaaatccagatggtttcaccgcatcagcatgtacgcgccgccctggaagcagcgctgccggtactgcgcacgcagctggccgaaagtggcattcagttagggcaaagcaacatcagtggcgaaagctttagtggtcagcagcaggccgcttcccagcaacagcaaagccaacgcacagcaaaccatgaacctctggcgggggaagacgacgatacgcttccggttcccgtctctttacaagggcgtgtaacaggcaacagcggcgttgatattttcgcctaacgtcagaggtagcaccgtaatccgcgtcttttccccgctttgttgcgctcaagacgcaggataattagccgataagcagtagcgacacaggaagaccgcaacacatgactgattacgcgataagcaagaaaagcaagcgatcgctttggatcccgattctggtattcattaccctcgcggcctgtgccagcgcaggttacagctactggcattcgcatcaggttgccgctgacgacaaagcgcagcaacgcgtcgtgccctcaccggtcttctacgcgctggataccttcacggtcaatttgggcgatgcggatcgcgtactttatatcggcataaccctgcgcctgaaagatgaagctacccgctcgcggctgagtgagtatttgccggaagtccgtagtcgcttgctgttactgttttcgcgtcaggatgctgccgtactggcgacagaagaaggcaagaaaaacctgattgccgagattaaaaccacactttccaccccgcttgttgccgggcaaccgaaacaggatgtcaccgacgtgctgtataccgcttttattctgcgataacgacatgggcgatagtattctttctcaagctgaaattgatgcgctgttgaatggtgacagcgaagtcaaagacgaaccgacagccagtgttagcggcgaaagtgacattcgtccgtacgatccgaatacccaacgacgggttgtgcgcgaacgtttgcaggcgctggaaatcattaatgagcgctttgcccgccattttcgtatggggctgttcaacctgctgcgtcgtagcccggatataaccgtcggggccatccgcattcagccgtaccatgaatttgcccgcaacctgccggtgccgaccaacctgaaccttatccatctgaaaccgctgcgcggcactgggctggtggtgttctcaccgagtctggtgtttatcgccgtggataacctgtttggcggcgatggacgcttcccgaccaaagtggaaggtcgcgagtttacccataccgaacagcgcgtcatcaaccgcatgttgaaactggcgcttgaaggctatagcgacgcctggaaggcgattaatccgctggaagttgagtacgtgcgttcggaaatgcaggtgaaatttaccaatatcaccacctcgccgaacgacattgtggttaacacgccgttccatgtggagattggcaacctgaccggcgaatttaatatctgcctgccattcagcatgatcgagccgctacgggaattgttggttaacccgccgctggaaaactcgcgtaatgaagatcagaactggcgcgataacctggtgcgccaggtgcagcattcacagctggagctggtcgccaactttgccgatatctcgctacgcctgtcgcagattttaaaactgaaccccggcgacgtcctgccgatagaaaaacccgatcgcatcatcgcccatgttgacggcgtcccggtgctgaccagtcagtatggcaccctcaacggtcagtatgcgttacggatagaacatttgattaacccgattttaaattctctgaacgaggaacagcccaaatgagtgacatgaataatccggccgatgacaacaacggcgcaatggacgatctgtgggctgaagcgttgagcgaacaaaaatcaaccagcagcaaaagcgctgccgagacggtgttccagcaatttggcggtggtgatgtcagcggaacgttgcaggatatcgacctgattatggatattccggtcaagctgaccgtcgagctgggccgtacgcggatgaccatcaaagagctgttgcgtctgacgcaagggtccgtcgtggcgctggacggtctggcgggcgaaccactggatattctgatcaacggttatttaatcgcccagggcgaagtggtggtcgttgccgataaatatggcgtgcggatcaccgatatcattactccgtctgagcgaatgcgccgcctgagccgttagtgatgaataaccacgctactgtgcaatcttccgcgccggtttctgctgcgccactgctgcaggtgagcggcgcactcatcgccattattgccctgatcctcgctgctgcctggctggtaaaacggttgggatttgcccctaaacgcactggcgttaacggtctgaaaattagcgccagtgcttcactgggcgcgcgtgaaagggttgtggtggtcgatgtggaagatgcacggctggtgctcggcgttaccgcaggtcaaatcaatctgctgcataaacttcccccttctgcaccaacggaagagataccgcagaccgattttcagtcggtcatgaaaaatttgcttaagcgtagcgggagatcctgatgcgtcgtttattgtctgtcgcacctgtccttctctggctgattacgcccctcgccttcgcgcaactgccgggtatcaccagccagccgctgcctggcggtggacaaagctggtcgctcccggtgcagacgctggtgttcatcacctcgttgacgtttattccggcaattttactgatgatgaccagtttcacccgcatcatcattgtttttggtttattgcgtaacgcgctgggaacaccctccgcgccacctaaccaggtattgctggggctggcactgtttttgaccttttttattatgtcaccggtgatcgacaaaatttatgtagatgcgtaccagccattcagcgaagagaaaatatcaatgcaggaggcgctggaaaaaggggcgcagccgctgcgtgagtttatgctgcgtcagacccgtgaggcagatttagggttgtttgccagactggcgaataccggcccgttgcagggacctgaagccgtgccgatgcgcattttgctcccggcctacgtgaccagcgagttgaaaaccgcatttcagataggcttcacgattttcatcccttttttgattatcgacctggtgatagccagcgtgttgatggcattggggatgatgatggttcccccagccaccattgctctgccctttaaactgatgctgtttgtactggtggatggctggcaattgctggtcggttcgctggcgcagagcttttacagctagagaggcaaaatgacacctgaatcggtcatgatgatggggactgaagcgatgaaagtcgcgctggcactggctgccccgctattgttggtagcgttggtcacgggccttatcatcagtattttgcaggccgccacgcagattaacgaaatgacgctgtcgtttattccgaaaatcatcgccgtatttatcgccattattattgccggaccgtggatgctcaatctgttgctggattacgtccgcaccttgttcactaacctgccgtatatcatcgggtagccgtactatgttgcaggtgacaagcgaacaatggctatcctggttaaacctgtacttctggccgttactgcgcgtgctggcgctgatctccaccgcgccgattctgagcgaacgcagcgtaccgaaacgggtaaaactgggtctggcaatgatgatcacgttcgccattgccccatcattacctgccaacgatgttcctgttttttcgttctttgctctgtggctggccgtgcagcagatcctgatcggcattgcgcttggttttaccatgcaatttgcctttgccgctgtgcgaaccgctggcgaaattatcggtctgcaaatggggctgtcatttgcgacgtttgtcgatccggccagccatcttaatatgcccgttttagcgcgtatcatggatatgctggcgttactgctgttcctgacatttaacggtcatttatggttgatttcactgctggtcgatacctttcacaccctgccgattggtggcgaaccgttgaacagcaatgcgtttctggcactcaccaaagcagggagtttgattttccttaacgggctgatgctggcgttaccgctcattactctgctgctgacactgaatctggcattaggtttacttaatcgtatggccccgcaattatccatttttgttattggatttccattaactctgactgtcggcatctctttaatggcggcattaatgccgttaattgcacctttttgcgaacatttattcagtgaaatttttaatttgctggctgatattattagtgaattgccattaatataattccgtaacgtttatcatgttatcctaaggattatccgaaaaataatacctacgaacatcttccaggatactcctgcagcgaaatatttgttttaagctcactcacatatcgcaacatttactttactttaagacaattccaggcaaattatacaacactttacgggatagtaagtccgcctgaaaaatcgcgagagtggcgcattaggtgacccatgttgttccgtttagtcatgatgaaatattcaggtaaggggaattatcgttacgcattgagtgagggtatgccatgtcaacgattattatggatttatgtagttacacccgactaggtttaaccgggtatctgttgagtagaggggttaaaaaaagagaaatcaacgacattgaaaccgttgatgaccttgccatagcttgtgattcacagcgcccttcagtggtgtttattaatgaggactgtttcatccacgatgcttctaacagtcagcgtatcaagctcatcattaatcaacatcccaatacgttatttatcgtttttatggcaattgccaatgttcattttgatgaatatctattggtcagaaaaaatttattgatcagttctaaatcgattaaaccggaatctctcgacgatatccttggcgatattctgaaaaaagagacaacgataacctcgtttttaaatatgccgacgttatcattgagccgaaccgaatcgagtatgttgcgaatgtggatggcaggtcagggaaccattcaaatctctgaccaaatgaatatcaaagccaagaccgtttcatcgcataaaggtaatattaaacgtaagatcaaaacgcataataaacaggttatctaccatgtcgtccgactgacggataatgtgactaatggtatttttgtcaacatgcgctaacacattctgactggtggtttcccaccagtcaggctgaataagattactctgctttctccacaaagataccgtcctgatgccctgcttcattaaagaaccagatgccgagcgggtagtcttccagcgaaaccaggtacattgtgccttcactaaactcctcaactgccagtaccacgccaggacgacgcggaccgccatccgttttgactgttacccgatcattcaccttcatcgttttcctcctgtggctttgtgccagtgtagaacaatttcgtttttctggcagcgccaggcgcgcgcgagtgctgattttctcgacggtctatacttaagagatgccaggcggacttaacgactggcggcaacaacagagtaacggttgcgaggaaagatgatgaaaaccgcaaaagagtacagcgataccgcaaaacgtgaggtcagcgtcgatgtcgatgccctgctggcggcgatcaatgaaattagcgaaagcgaagttcatcgcagccagaacgattctgaacacgttagcgtcgatggacgtgaatatcatacatggcgtgaattggcggatgccttcgaactggatattcatgacttcagcgtctctgaagtgaatcgttgaatgcacaataaaaaaatcccgaccctgagggggtcgggatgaaacttgcttaagcaagaagcacttaaaaaattcgttacaccaggaaatctgatgtgttcatcaccttatccgcaatttttttcgctgacaagaaaatattcgccatatgaatgattaacgctacttatgaatagaaatgtgacgcacgtcaccccttggtggctctggcgtcagcgggatcgctcccgaaaaaatcatctttgataatttgtgcggttttgagaatcatcctggtaagaggagtactgcgcgactatgttttcaattcaacaaccactactggtttttagcgatcttgatggcaccctgctggacagtcatagttatgactggcaaccggcagccccctggctcacccgtttacgcgaagcaaatgttcccgtcattctctgtagcagtaaaacatcagcggaaatgctgtacttgcaaaaaacgttggggctacaaggtttaccgctgattgccgaaaatggcgcagtgatccagcttgctgagcaatggcaggagatagacggttttccacgcatcatctcaggtattagccatggcgaaatcagcctggttttaaatacgctacgcgagaaagaacattttaaattcacgacttttgatgatgtcgacgatgcaaccatcgccgaatggacgggattaagccgtagccaggcggcgctgacgcagcttcatgaggcgtcggtaacgctaatctggcgcgacagtgacgagcgtatggcacaatttaccgctcgtctgaacgaactgggcttacagtttatgcagggtgcgcgcttctggcacgtactggatgcttctgccggaaaagatcaggctgccaactggattatcgcgacctatcaacaattgtcaggcaaacgcccaaccacacttggcctgggcgatgggccaaacgatgcgcccttactggaggtaatggattacgcggtgattgtgaaagggctaaatcgtgaaggggtgcatctgcatgatgaggatccggcccgcgtctggcgaacgcagcgtgaaggaccggaaggatggcgtgaagggctggaccattttttctccgcccgttaagcgttatcgctcgcgaatacccgattacgcccagcctgtttagcgagataaagccgacggtcggccagtgactggagttgttcaaaatcataatcaccggtttcctcgctgctgcttacccccagcgaggcactgatgcgtatcgtcgtactcttggcgatcaacatctctttttcatttaatttcagtcgaatacgttctgcgacctccgcagcctccgtcagactcgcgcctggcagaatcacacaaaactcctcaccaccgacccgcccggcaacgtcctgcgcacgcaaggaactgctaattaatccggcagcatgagaaagaacacggtcgcccgcctgatgaccaaagcggtcattaatcgctttaaaatggtcaagatcgacctgaatgacagaaaaaggatgttggtgcgtctgacacaatttagcgagcggacgggctttttcgaacagtgcgccacggttatataaacgcgttaaggtgtcgtgccacgcctgccactgcaacgagctttgcagaacatacatgttgctaaccatccggcgaatcacataccaggagatgagtaacatggtggtaaagagcgcccacagcagggttaatgcaatgctgatactgccgaaatcgccgcgcacgccttcgcttaacgtatggacacgcaccagcacaccgtcgaaatggtccagacgttcccagctaacatagcgactgtccatacgaatgccgccccgcgtgtcatgttccattgcctgcgccagcaaggccagttcacgaggatcaaaaatattccctgttggatggtcaggattggaagaggtcaaaaatctcagcttactgtcatagagctgatactcaccatcgaggtttttatcgatggcgtttcttaaaaattgctgcatagtacgcacgggaatactcatccccagcacgccataccagtagttattactgtctaccggaacactgacggtaacctgcggttcagtattgctggcgtgttccggttgcgaagtgaaccagcgtaccgcgcggtgacgattttctcgttgtgaatggccaataaaccagggttgggtgacatagccgtaataacgcgttggaacattgcgcgtaaacaaggtcggctgcgtcgaaacgtaaaatccggcacgcgagacatacatcgcctgttcaaccatcgacgaggagttgtgcgctagtcgcagcaagtaaccaacttccagtgcagcggtaatttcattgtcgaggctttcattttcgcgagacaggagattcccctcgctgactaatgcatccgacacaccattaactggcagagtgcgtcgtcggttgagttcgattttccaggcgtgctcgtcgcgatgctgttcgaactcggttacagcatcacgcagagaggtgaaatccagtggcgctacgagagcttcgcgcatgccattacgtaaaaagatcagtttgtcgacgttatactgcaaatgcttatcgagcgcgttggcaacgttttccagatgattacgctggctggagatataggcatcttccagcaccaccacttcacgccaggtgagcaaggtggaaaaaagcaataccacgataaagcagagattaacgacatgaccaggccccaggcggcgtgcgagttttttcaaccagctctggttttccatttttgtctcgtgctgcaccctgacgactcccaacctgcttttttatgattctggcataacctggcgatagcgtaccgcaaaacagcgataattttataatggtggcatgataagacgcgactatcattcattgcaggcattagcacaccaggccggatgtgatccggcctgatgttaatgataccctttcacacttcttccgcagaacgactcccctcccccggaacaagctcggtttcatgaaaagcttcccgcttgaccccgtaaccgtcataccaacgacactcaaccataccgctggagtatccagtgacaatcatccgcgggccgccctctttaaccgtaacttcctcactaaccataaagctcatactcgcctccttttttcgagtgaaacttgttcaccttagttgaagatggcgaattttgcataatagccagtgcgagtattaatgtgcctgaccgcgcattttctctacggctttcactcccagcaccacgatgccgccgatgataaatccaagaatcagatttaaaacagtcggtaatatcatcgccactactgcactttgctgcccggcgaaatgttcaatggcgtgatgcagcggcgcaattccatgtaccacaatcccaccgccgacgaggaacatcgccagcgtgccgacaatcgataacgctttcatcagccagggcgcgataatcaataaccctttacctaatgcctgcatcagcgcgctggatttttccgccagccaataccccaggtcatcaatcttaacgataacccctaccagaccgtagacgcccacggtcactaccagcgcgatgcctgaaagcaccagcacctgattaagcaacggcgcttcggccacaatccccagcgtgatggcgacgatttccgcagacaatataaaatcggtacgaatcgccccttttattttgtccttttcaaacttcagcggatcctgcgccgccagcttctccagacgctgctggctctgcgccggatcttctttatgtttacgcgcctccagcatatgcagcactttctctactccttcaaagcagagaaacgcgccaccaatcatcaacagaggcgtaatcgcccacgggataaacgcactgatgatcagcgccagcggcaccagaatcactttattaatcagcgatcctttcgccacgccccagaccacgggaagttcccggttggcccgcacgcctgaaacttgttgcgcattgagcgataagtcatcccctaatacaccggcggttttcttcgccgccagtttgcccatcacggagatatcgtccagtagtgtggcgatatcatcgagcaacgtcagtaaactactcccggccaaaagcattccctctcatttttattgttgaagggtgtaagtatgaagcaaaaacggcagctctgatacttgcttcacaggtcaacatttttttaacaatcaagtgcaattatatctctcgccagcagaatgattttcacgtttactatgaaccacctttttatttccaccgtgagggattatgcgtttccgccagttgttaccgctttttggcgcgctgtttgcgttgtatatcatttggggctcaacctattttgtcattcggattggcgtggaaagctggcctccgttaatgatggcgggcgttcgattcctggcagccggtattttattgctggcatttttgctactgcgcggacacaaactccccccgctacgtccgctgctcaatgccgcgctgattggcctgttattgctggctgtcggtaatggcatggtgacggttgccgaacatcaaaatgttccttccggcatcgccgccgtagtggttgcaaccgtgcccctctttaccctgtgcttcagccgcctgtttggcattaaaacgcgcaaactggaatgggtgggtattgccattgggcttgccggaatcatcatgctcaatagcggtggaaatttaagcggcaatccgtggggcgcgattctgattttaatcggctcgattagctgggcgtttggctcagtttatggctcgcgcattaccttacctgtagggatgatggcgggtgcgattgagatgctggcggcaggcgtggtgttaatgatcgcgtcgatgattgcgggtgaaaaactgacggcgctcccttccctttcaggcttccttgcggtcggctatctggcgctgtttggttcgattatcgccatcaacgcttatatgtatttaatccgtaatgtcagtccggctctcgccaccagctacgcttacgttaacccggtggtcgcggtcttgctgggtacgggactgggtggagaaacactgtcgaagattgaatggctggcgctcggcgtaattgtcttcgcggtggtactggtcacgttgggaaaatatctcttcccggcaaaacccgtagttgcgccagttattcaggacgcatcaagcgagtaaatgaatcccctgcgtgtcgatctgcgcgctggcaccttcgccgcagatccactcttccagacgctcggtaagcgcttcatccgtcagcttctcgcgcccacgtaacgcgcactcccagacaatcaatacgcgccagccgagttcctgcaagcgactgatatcgcggcgatcgcgctcaacatttttacctatcttctccagccagaactcggttcgagtcgcaggcactttaaacagatagcagtgatgatgatgccagaagcagccatgggtaaatatcacgcagcgatattcatcaacgacaaaatccggacgtccgggcagactggcgtcctgaacgcgaaatgccaggccctgcccggttaacagactggcgaggcgcttctctatcgccgtatcacgcgtggcaatcgcgcgcatatttttgctgcgagtggccttatcgtgaacgtcggccatgttgtgcctcttgctgacgcaacgccaccgcctgtttgatttttggctcaagcagttttgccaccgcggcaaagaccggcacgaccaccgagttaccgaactggcgataggcctgagtgtccgaaaccggaatacggaatttcgcttctcccggcgcttcaaaacccattaagcgcgcgcattcccgaggcgttaaccgacgtggacgatgttgctgattcagcggatcgtcaaagtctttctcacccgtggccatatcccagccgcgatcgattaaaatttccgcgccatctttgtaataacgcgcagacagcgtacgcgtgacgctttgcggattgttcggataaaccattccataaccgaagccgttaccgcgcgcctgatgttttttcgcatatcgatagaggtacttccacagcaccggcgtcaggatatatttcgcctcgaccatcgggtccaacagctgcgccagcgtcactcgctgcgcagggaaacattcgctgatatcacgcagggtaaaatcggctttcagattcagatcgcgacgaaaacccaccagcacgatgcgttcacggtgctgcggcagaaaatgtttgccgtcgatgattttcggatcgtctggcccattatcttctgcatcagccacgtcatagcccagttcgtccagcgtctgcatgatgatgcggaacgttttaccctggtcgtgacttttcaggtttttgacgttttcgagcacaaacatcgccggacgacgcgcgtcgataatgcgtaccacatcaaaaaacagcgtgccctgggtatcgcaggcaaaaccgtgcgcccgcccgagcgagttctttttcgatacgccagccagcgaaaatggctgacaagggaaaccggccagtaaaacatcgtgttcaggaatgtgttgacgaatatgttccgccgccgcctcatcactcacgccttctttatggctgagggtgatgtcgcggatatcttcattaaaatgatgcgtcgccggatcgcaataatggttggctttataagtgcgtaccgcatgtttgttccattcgctggtaaacacgcactgtccgccaatcgattcaaaaccgcgacggatgccgccaattccggcgaatagatcgataaagcgaaacgcataatgcggatgatgtgccggtggtttgggtaataacgtttgcagatgggcgaactctttctcacttaaacggtgccatgccgagtcattcgccagcgcacgttttaaaattgccgcgctccagtgattctcacctacaccattaagctgcgccaccaacgttttaacatcataaatttgcagcagtttctccagcattgcctgtgcggcattcccggtgctgtatgaatcggttactgatatattttcctgcatagatttcaccggccatctgagatggccgacaggttaacataattacagccatttagggccacgcgctcagccagcggatgaaaacgcatctatcaccttgtgatcgacaccttcattctcccccgccagttcggcactgagcttcgccataaactcgactaaaaaatgcgcgttgtgctgcgccagctgcttgcctcttgcggtttgcatggtttgcggtagcttcagcaacttagtctggaaatgatccagcgcgtagcgtttatcatcaagcgggcgatgctgtgcgaacggatcttcaccatcaaacagcgccacgcccaatgcccctgaaacggcaaacacgcgcgccaggccaatcgcccccagggcttccagccgatccgcatcctggacaattttagcttccgttgttaagggggcgatttgcgcgctgaaactgtgagcggcaatggcatgacaaacggcctcgattttctccgccggaaattgctcgaactcttcacggagcaggcgacgcgtctcttctgccgccaggattgaagaacgctgcctttgcggatgatttttcgccaggctcacaatatcgtgaaaataacaggcggttaaaatcaccagcatatcgacatcgtcatctgccgccagcttctgtgccgtagcccagacgcggcgaaaatgacacacgtcatgggccgcgtcctggtgctgatgatggtttttcaaccagttttcgaactgtgcctgccagtgttgtaagtccatacgcgctccgttgccaaagagtcgccaccttagcagtttttattcatagcgtctgctacgtgcgggacgaggtcgggtgtaccaggcaatgctgcctaacaatgccccgaccagagccataaataaaaatccgaccagtgcccctaaccactttcccgcggtagagcctaaatcgctttcaaatcccgacacgggggcatcgggaatccggctcatcacccagatgtaacgcgccattgcccagacgaaatagccacaccatgtatagaaagcccacaaagccagtttgccgccagggctgcgagagagtctctcttccatctttgtcgaaccgtattccattttgagataacccggaaaattcagacttagtactattatgtgataaaagtcacatttttccacattggatgagccagtcaagactcaatcattttttgaacaaatagataaattttgcgcaacggcagtgaatacaggaaaaatcgttttgagcgattttatttatctttgatatcggctttattaattcatttaatcaatatattagcactgattacaattatacctttttattattctgtgtcatgatgcttccgttattagccttttatcgtcttgtttatattttttgggccggcatgatgccggcttttttttatgccttcattaatgtgcgcctgatcacaccagccgtttggcgcaacaatcattgataccccctatgtttccgctcaactcataacatattgatatacatttataattttcatgaatatttatatttagaattcataattatgaattatattaaatagattagaaacattttgatatcttttaaatacatttgttacatgtaatccttaaaataaaatgaacttcatagaatagtatccaaatgtgcttttttttggataacggcacttattgatatattcatgaagattataatcacaagggaatacataatgaaaagaaaagttctggcaatgctggtcccggcgttattagttgctggcgcagcaaatgcggctgaagtctataataaagatggtaataaactggatttgtacggaaaagtagtgggtctgcactacttctctgatgattctggcagcgatggcgacatgtcatatgcccgtatcggtttcaaaggtgaaactcagatcgctgatcaattcactggttatggtcagtgggaatttaacattggcgcaaacggtcctgaaagcgacaagggtaataccgcaacgcgtctggcatttgcaggtttaggctttggtcagaatggtactttcgactatggtcgtaactacggtgtcgtatatgacgtagaagcatggaccgatatgctgccagaatttggtggcgatacctatgctggcgctgacaacttcatgaacggtcgtgctaatggtgttgcaacctaccgtaacaatggcttctttggttaggtcgatggcttgaactttgctttgcaatatcagggtaataatgaaagtggtggaccattcgggcaggaaggttccggtagtggtgatggccgtagcctttccaaagaaaatggtgatggtttcggtatgtcaacatcctacgacttcgacttcggtttaagtctgggtgctgcatatcaaactctgatcgttcagatcgtcaggttggagttggtttaaatgatcgtaaccatagcaacagaaatgctggtggtgaaaccgctgaagcatggactgttggtgcaaaatatgatgctaataatgtgtatttagcagctatgtacgctgaaactcgcaatatgaccccatatggtggtggcgagtttgataatggtgaatcaagatcagccatcgctaacaaaacccaaaactttgaagttgttgctcagtatcagttcgactttggcctgcgcccgtccatcgcttacctgcaatctaaaggtaaggatttaggcggttgggctcatgacggcaacggcgacccacgttacaccaataaagatctggttaaatacgttgatattggtgcgacctactacttcaacaaaaacatgtccacctatgttgattacaaaatcaacctgctggacaacgacgatgacttctacgaagcaaacggcatcgctaccgatgatatcgttgctgtgggcttagtctaccagttctaatcagtcaactcgctgcggcgtgttactgtaaaactgaacactagcctgagttcgtccctcatcgaactcaggcttttttattggcatttcatctccatctgcggcacacgcaattgccgaagcatatcgatacagcaccttaccctgcccctcctggcacaataacatcaaccagctactcttcaagctaacacccaaatgcatttctttatgaattaatccgtaacaaacacgcttcccatatagaaatatttgcaaaaatagtgcatgaaataagctttttctctaccaatccgggatataaatattcatcagcaccacaatattccacagcactaaatctctccccgccaccccgtacctctgataatggtctaaaatcattgaagccacttgcgacgacgttgctcaataaggaaaatttggcgtgaataatattcaacaccagtgcagcatcatcattacatacttacagccgccgactaccgctttcgatatattgactcaattttccagcctggttaaaaatagcgaccagctcagtcgcaaatatagtgactaccctaactaagcaacaataaggaatacactatgactgttcaaacaagtaaaaatccgcaggtcgatattgctgaagataatgcattcttcccttcagaatattcgcttagccaatataccagtcctgtctctgatcttgatggcgtggactatccaaaaccttatcgcggtaaacataaaattctggtgatcgccgcggacgaacgttatttgccgaccgataacggaaaactgttctcgaccggtaaccatccgattgaaacgttgctgccgttgtatcatctccatgctgcaggtttcgaattcgaagtggcgaccatttccggtctgatgaccaagtttgaatactgggctatgccgcacaaagatgaaaaagtaatgccattctttgagcagcataaatcgttgttccgcaatccgaagaaactcgcggatgttgttgccagcctcaacgctgatagcgaatatgcagcaatctttgttcctggtggtcatggcgcacttattggtttacctgaaagccaggacgtggctgccgctttacagtgggcaatcaaaaatgaccgttttgttatctccctttgccacggcccggcggcttttctggcgcttcgccacggcgataacccactgaatggttattccatttgcgcattcccagacgccgcagacaaacaaacgccagagattggctatatgccgggtcatctcacctggtacttcggcgaagaactgaagaaaatgggcatgaatatcattaatgacgacatcaccgggcgagtacataaggaccgtaaacttctcaccggcgacagtccttttgcagcgaatgcgttgggtaaactggcggcgcaggaaatgctggcagcttacgcgggttaatccctgttacgtttgaatgtaagcgcataatcaatcgcggccgcgttagtactcacgacgtggctgcgttttttcacggttaatttatggcgtactgaagccctatgttaatttctttgcggtaacgtaatccggaacacattatgcttattgagatagtgatacgtagcacttcccccatgcaattcggcaatcgctttgactaaagaaaggcctagtccctgacctacggaatgacgcgaattatctccccgccaaaatctacggaagagtttttcaggctcattaattttcgttccagggctggcgatatcaatattaagatagctgttggtatcaagaaaactggttatatgaatacgcgatttttctggcgaatatctaatggcattaacaataagattcgataacattcgttgtagtaaaattttatccgcaaagatttgctgattgcactcgaccttaaagcaaatctctttctcgtctgaaaggtattcaagatagtccaacaaattttcgacttccttattgagagaaagcgagtccagtttcaccaaaacattgtttttatctgccctggcaagaaacagtatgttctctgttaaccgcgaaatattttccagctcttcaatgtttccggcaattgttttttgatattcagcgatacttctggtttgactgagcgtaacctgattctgacccagtaatgcattaattggcgttctaagttcatgagcgagatcgtcagcaaactgacttagacgctcaaaatctttgactaaagcatgatgcattttattcaacgcctgcccaagaggttttagttctctcggtaatgcgctaacctcaacaggctctcggctatcgttataattcagcgcttccgttacaccactcaactttttgatctctcgtaatcccgttctgattaacagcggacttaatactgagcaaagtacaatggcgacaatgcaaattataatgctattaattttatactgttcaagcatgttatgtctggctgaagccaatttagccacagtaaccgttaatgatggcgaaacttcatcaatattaattcgtaaagcatctatctctgtatcattaataatgcttctgtaaatgccagctgcgctgattgtctcactagcaggtatgttatttaacatgccatcactgacatttgtccggttaacaattttattgatgctatcaccatgaataatcaagatatcctgactaacatccatcatccggttaaagtacacaggtaacgtatctggatttaccccatcaattaacaactgcttgatctgcgctgtccggttaatgagtgttgtatcatcgcgccatttcaactcacttgccaggccattatagagagtccagacaattccggcgccagcaacagacagtagcaatataaaaagcaaggttaaacggacggttatagatagtcttttcattatttttttaccgctacgaatgaatagcccatcccccggattgtggcaattagcttttcaggaaaaggatcatcaacttttgcgcggagcctgcgaatggcgacgtccaccgtattggtatcactatcaaagttgattccccaaatttcactcgcaataaccgttctgggtataatttcgccagctctggaggccagtagccaaagtaactgaaactccttgcgcgtcagtgtaatactgatattgtccctgctcacactatgactaacagagtccattcttaagccgctgatttctaatgttgaattcaaagcgtgatgttgccttaattgtgcccgaacccttgccagcaactcagaaaatgaaaaaggttttaccagataatcatttgccccactgtccagccctctgactctgtcatcgacagaatcccttgcagtaaggcaaataacaggggtttgctttgctgttcttaacgtttgtaagatctgccagccatccatacccggaagcataatatccagaatgatcaatgcataatcatccttcagcgcaagataaagcccatctctgccatcagaaacggcatcgatgacataacccgcttcggaaagcccctgcgttacccattcctgggtcctttgattatcttcaataagtagaatcttcatgaaaataatatgccataaatcatatgttatagaaacagcctggttcattacaaaattgtaatgctgctgtaaggttaccctggacgctttttcgctatcctcaaaactcattcacatgacaaggatataaacatgttaaagcgttatttagtactctcggtagcaacggcagcattttcattaccttctttggttaatgccgcacaacaaaacattcttagcgtgcacattttgaaccagcaaacaggaaaacccgctgctgacgtgacagtcactcttgaaaagaaggcggataacggctggttacaacttaataccgccaaaacagataaggatggacgaattaaggcactgtggcccgagcaaactgcaactacgggcgattaccgtgtcgtatttaaaaccggggactatttcaagaaacaaaatcttgaaagtttcttccctgagatccccgttgaatttcatattaataaagtgaacgagcattatcatgtgcctttattacttagccaatatgggtattcaacctatcgtggcagttaatgcataaatatgtaaaagcagatctctgctactgttagggaggacactccctgacagattaacagtaaacggctcttgctggctaacgacaaaaaagtgtgatggcttatgaaaaagaatcaatttttaaaagaatcagatgttacggccgagtcggtattctttatgaagcgtcggcaggtgttaaaagcactgggcatcagtgcaactgcactttctttgcctcacgctgcgcatgccgatctgcttagctggtttaaagggaacgatcgcccgcccgcccccgccggaaaagcgctggagttcagcaagcctgccgcctggcaaaataacctgccactgacgccagcagataaagtttccggttataataacttctatgaattcgggctggataaagccgatcccgccgctaatgctggtagcctgaaaaccgatccatggacactgaaaatcagcggcgaagtggcaaaaccattgaccctcgatcatgatgacttaacccgtcgcttcccgctggaagagcgtatttatcgtatgcgctgcgtggaagcgtggtcgatggtggtgccgtggattggttttccgctgcacaaattgctggcgcttgccgaacctaccagcaatgcgaagtatgtcgctttcgaaacaatttatgcaccggaacagatgccaggccagcaggaccgctttatcggcggtgggctgaaatatccttatgtcgaaggattgcgtctcgacgaagcaatgcatccgctcacactgatgaccgtaggtgtttatggcaaggcgttaccgccacaaaatggcgcgccggtgcgactgattgtgccgtggaaatatggctttaaagggattaaatcgatagtcagtattaagctgacccgcgagcgtccgccaaccacctggaatctggcagcgcctgacgaatacggtttttacgccaacgttaatccgtatgttgatcacccgcgctggtcacaggctaccgaacgatttattggttcaggcggcatcctcgatgtacagcgccagccaacgctactgtttaatggttacgccgcccaggtggcatcgctgtatcgtggcctggatttgcgggagaatttctaaatgcgtctgacagcaaaacaggtgacatggctgaaagtttgcctgcatcttgccggattgttgccgtttctctggctggtctgggcgatcaatcacggtggactgggtgccgatccggtgaaagatattcagcattttactggtcgcactgcactgaaatttttgctggcgaccttgttaatcacccctctggcacgctacgcaaaacagccgttattgatacgcactcgccgcctgttaggattatggtgctttgcctgggcgacactgcatttaacaagttacgcattgctggagctgggcgtgaataatctggcgttattaggtaaggagttaattacccggccttatttaacgttaggtattatcagctgggtaattttgcttgctttagcgttcacttcaacccaggcgatgcagcgaaaactcggcaagcactggcaacagttgcataatttcgtctatcttgtcgcgattctggccccaatacattatctgtggtccgtgaagattatttcaccgcagccgctcatctacgctgggctggctgtactgcttttagccttacggtataagaagttgcgttccctttttaaccggttacgcaagcaggttcacaacaaattatctgtataacttcatattgccgacaaagtacgcgttatccctgccggatgtggcgcgagcgccctatccggcatacacagatcgcatcaggttatgtttcgtttgtcatcaacctcaaatcaccaaaataatttattttatttcaataagatagataagtagaactgagaaagccatgctctcgtttcctaagagttgttgcattttgctatatgttacaatataacattacacatcatatacattaactctggaggaaactgttttggcgattcgtctttacaaactggctgttgctttaggtgtctttattgttagcgctcctgccttttcgcatggtcatcactcacacggcaaacccttaacagaggtcgaacaaaaagctgctaatggtgtttttgatgatgccaatgtacaaaaccgaacgctcagtgactgggatggagtctggcaatccgtttatcctttactgcaaagtggcaaacttgaccccgtctttcagaagaaagcggatgcagataaaactaaaacatttgctgaaattaaagattattatcacaaaggttatgcaacagatatcgagatgattggcattgaggacggcattgttgaattccatagaaataatgaaacaacatcgtgtaaatatgattacgatggatacaaaatactcacctataaatcaggcaagaaaggcgttcgttacttattcgaatgtaaagatcctgaaagcaaagcccctaaatatatacaatttagcgatcatataattgcaccacgaaaatcatctcattttcacatttttatgggtaatgattcacagcaatctttattaaatgaaatggaaaactggccaacgtattatccatatcagttgagtagcgaagaagtggtcgaggaaatgatgtctcattgagtattctcatgataacgcctcgatgccgctttagtaagttatcataactgccactggtccatccacaaacgccactgaacgcaagctagctacagacacgctcatcactatgacgtgtctgtatattaataagctaacccgcattgagttaaccaataacggattccatacacaatacggccaacagagaaagatacctgtgctcacgccattgcttatattggctggttacaatatgcactatcaattttttaaataacaaattattaaaaccacatctgtataaggaatttttaaggttcgtgggatagcttgactgtgaaaatcacaggagctacaaaaatgaaccgattctcaaaaactcaaatttatttacattggataacgctgcttttcgttgcaataacctatgccgcgatggaactccgtggctggtttcctaaaggtagtagtacttatctgctgatgcgagaaacacattacaatgcgggtatattcgtttgggtgttaatgttttcacgcctgattataaaacaccgttatagtgatccttctattgtgccaccgccacctgcctggcaaatgaaagcggcttcgctaatgcacatcatgctttatataaccttccttgcacttcctctgctggggattgctttgatggcttacagtggaaaatcgtggagtttccttggtttcaatgtgtctccctttgttaccccaaacagcgaaattaaagcactgataaaaaatattcacgaaacctgggcaaatataggctactttttaatcgcagctcacgctggcgcagcactctttcatcactacattcagaaagataatactctgttacgaatgatgcctcgccgcaaataagtcgatccccttacaaggaaatgtgaaccatggacatcaacgcgtcataaatgtttacgcaagtgcacaatgcaccctttccactatcaacaaggaggagcagaaactgtgtaaatcgtacaatggtaagacttatcaaaaatacaggttaattttggtatttaaaccttttttacttgttagtatgatacaaaggctttcaaaaaagctgcgaaattcaacaactcttggaaattatggactttgtcccgcggctttaatctgacggccgcgttccttttttgactcaattattgaacccttctctacgcaacttcagttcccaccaccaactttgcggcagtttcataggatgaatgtctaaaagaataatggtgagcgataagaaaacgactgaataactgcacattttcgctcgaaagcttcctgtcagatccatagcgaatcaagtgctgaatgtcacagtatcgaacagaaaacagtgacgatctaacccttcaagaatattctacgattgttctgtttaggaaaagcaaggcgggaagtcgggagataagtcattgataaagtggcggagagagggggatttgaacccccggtagagttgcccctactccggttttcgagaccggtccgttcagccgctccggcatctctccgttcagatggttgccatgatgccaggaaatttggcattttaacagtccctgtccgtgcaattttgttcaagtgacgagtttgcgagcaaaacgatgattaagtggccctggaaagtacaagaatcagcacatcaaactgcccttccctggcaggaagcactatcgatcccccttttaacgtgtctgacggaacaggaacaaagcaaattagtcactcttgccgaacgttttttacagcaaaagcggcttgttcctttacagggctttgaactggattcattaagaagctgccggatagcacttctattttgcctacccgttctggagttaggactggaatggctggatggttttcatgaagtcttaatttatcctgcgccatttgtggtcgatgatgaatgggaagacgatatcggtctggtgcataaccaacgtattgttcagtcaggtcagagctggcagcaagggcctatcgttttgaactggttggatatacaagattcttttgatgcttctggttttaacctgattattcatgaagtcgctcataagctggacacccgtaacggcgatcgcgccagcggagttccctttattccgttgcgtgaggttgctggctgggaacacgatcttcatgctgcaatgaacaacattcaggaagaaatcgaattggttggcgagaatgcggcgagcattgatgcttatgcagccagcgatcctgctgaatgttttgccgtactttctgaatatttctttagcgccccagaactttttgctcctcgtttcccttcattgtggcaacgtttctgccaattttatcaacaagatcctttgcagagactgcatcacgctaatgatacagactcgttttcggcgacgaatgttcattaattaacaactttgcagattaattaaccaattgaaatgacttatgaaatttagtgttgacagacaaggtaccgctaagtaatattcgccccgttcacacgattcctctgtagttcagtcggtagaacggcggactgttaatccgtatgtcactggttcgagtccagtcagaggagccaaattctaaaaattcgcttttttagcgcaatgtcactgaccttagttgaacattgttttttaacggatagcgggtttttaacatcttaagcgccctcgacctttatggttgagggcgttttgctatgaacgccatcaccattttcccctcgattataaaacttgagttattcagtagtctcccctcttgcaactcacacccaaaactgcctaacgaaaagttattaattttcaatcatattgctatcagtatttacattttttcgctgtgctagaaagggcgcatttatgttagctcgttcagggaaggtaagcatggctacgaagaagagaagtggagaagaaataaatgaccgacaaatattatgcgggatgggaattaaactacgccgcttaactgcgggtatctgtctgataactcaacttgcgttccctatggctgcggcagcacaaggtgtggtaaacgccgcaacccaacaaccagttcctgcacaaattgccattgcaaatgccaatacggtgccctacacccttggagcgttggaatcggcccaaagcgttgccgaacgtttcggtatttcggtggctgagttacgcaaactcaaccagtttcgtacgtttgctcgaggttttgataatgtccgccagggtgatgaactggatgtcccggcacaagttagtgaaaaaaaattaaccccgccgccgggtaatagcagtgacaacctcgagcaacagatagccagtacttcacagcaaatcgggtctctgctcgccgaagatatgaacagcgagcaagcggcaaatatggcgcgtggatgggcctcttctcaggcttcaggcgcaatgacagactggttaagccgcttcggtaccgcaagaatcacgctgggcgtggatgaagattttagcctgaagaactcccagttcgattttctccatccgtggtatgaaacgcctgataatctctttttcagtcagcatactctccatcgtactgacgagcgtacgcagattaacaacggcttaggttggcgtcatttcactcccacatggatgtcgggcatcaacttctttttcgaccacgatcttagccgttaccactcccgcgccggcattggcgcggagtactggcgcgactatctaaaattaagcagtaacggctatttgcgactgaccaactggcgcagcgcacctgaactggacaacgattatgaagcacgcccggccaatggctgggatgtacgcgcagaaagctggctacccgcctggccgcaccttggcggtaaactggtctatgaacagtattatggcgatgaagtggccctgttcgataaagacgatcggcaaagtaatcctcatgccataaccgctggacttaactatacccccttcccgctgatgaccttcagcgcggagcaacgccagggtaaacagggcgaaaatgacacccgttttgccgtcgattttacctggcaacctggcagcgcaatgcagaaacagcttgacccgaatgaagtcgctgcacggcgtagccttgcaggcagccgttatgatctggtggatcgcaacaacaatatcgttctggaatatcgcaaaaaagaactggttcgcctgaccctgacagaccccgtgacagggaagtcaggagaagtgaaatcactggtttcgtcgctacaaaccaaatatgccctgaaaggctataacgtcgaagccaccgcactggaagctgccggtggcaaagtggtcacaacgggtaaagatattctggttaccctgccggcttaccggttcaccagtacgccagaaaccgataacacctggccgattgaagtcaccgccgaagatgtcaaaggcaatttgtcgaatcgtgaacagagcatggtggtcgttcaggcacctacgctaagccagaaagattcctcggtatcgttaagtacccaaacattgaacgcggattcccattcaaccgccacactgacttttattgcgcatgatgcagcaggtaatcctgttgtcgggctggtgctctcgacgcgtcacgaaggtgttcaggacatcaccctttctgactggaaagataatggtgacggaagctatacccagatcctgaccacaggagcgatgtctggcacgctgacgctgatgccacagctgaatggtgtggatgcggctaaagcccccgccgtggtgaatatcatttctgtttcgtcatcccgaactcactcgtcaattaagattgataaggaccgttatctctccggcaatcctatcgaggtgacggtagaactgagagatgaaaatgacaaacctgttaaggaacaaaaacagcaactgaataacgcagtcagcatcgacaacgtgaaaccaggagtcactacagactggaaagaaaccgcagatggcgtctataaggcgacctataccgcctataccaaaggcagtggacttactgcgaagctattaatgcaaaactggaatgaagatttgcataccgctggatttatcatcgacgccaacccgcagtcagcgaaaattgcgacattatctgccagcaataatggtgtgctcgccaatgagaatgcagcaaacaccgtctcggtcaatgtcgctgatgaaggaagcaacccaatcaatgatcataccgtcacgtttgcggtattaagcggatcggcaacttccttcaacaatcaaaacaccgcaaaaacggatgttaatggtctggcgacttttgatctgaaaagtagtaagcaggaagacaacacggttgaagtcacccttgaaaatggcgtgaaacaaacgttaatcgtcagttttgtcggcgactcgagtactgcgcaggttgatctgcagaagtcgaaaaatgaagtggttgctgacggcaatgacagcgtcacaatgaccgcgaccgtccgggatgcaaaaggcaacctgctcaatgacgtcatggtcactttcaatgttaattcagcagaggcgaaactgagccaaaccgaagtgaatagccacgacgggatcgccacagctacgctgaccagtttgaaaaatggtgattatagggttacggcctctgtgagctctggttcccaggctaatcaacaggtgaattttatcggtgatcaaagtactgctgccctgaccctcagtgtgccttcaggtgatatcaccgtcaccaacacagctccgcaatatatgactgcaaccttgcaggataaaaatggcaacccactaaaagataaagaaatcaccttctctgtgccaaacgacgtcgcaagtaagttctcgattagcaacggaggaaaaggcatgacggatagtaacggggttgcaatcgcctccctgaccggcacgttagcgggcacgcatatgatcatggctcgtctggctaacagcaatgtcagcgatgcacagccaatgacgtttgtggcggataaagacagagcggttgtcgttttgcaaacatcgaaagcggaaatcattgggaatggcgtggatgagacaactctgacagcaacagtgaaagatccgtcgaatcatccggtggcggggataacggtaaacttcaccatgccacaggacgttgcggcaaactttacccttgaaaataacggtattgccatcactcaggccaatggggaagcgcatgtcacgctgaaaggtaaaaaagcgggcacgcatacggttaccgcaacgctgggtaataacaataccagtgattcgcagccggtaacatttgtggcggacaaagcctcggctcaggttgtcctgcagatatcaaaagatgagatcacaggtaatggcgtcgatagcgcaacgctaactgcaacggttaaagatcagttcgacaatgaggtgaataatcttccggtaacattcagctcagcctcttcaggactcaccctgaccccgggagtaagtaataccaacgagtctggcatcgcgcaggccactctcgcaggcgttgcctttggtgagaagacggttactgcatcactggctaataatggtgccagcgacaacaaaactgtgcattttattggcgacacagcggcggcaaaaattatcgagttggcgcctgtcccagacagcataatcgccggtaccccgcagaacagctccggcagcgtcatcaccgccacagtcgttgataataatggctttccggtgaaaggtgtgactgtgaacttcaccagcaacgcagcgacagccgaaatgacgaacggcggtcaagccgtgacgaacgaacagggtaaggctaccgtcacttataccaatacccgctcctcgatagaatcaggagcgagaccggataccgttgaggccagtctggaaaatggtagctccacgcttagcacatcaattaatgtcaacgctgatgcgtctacggcacatctcaccttgctacaggcactttttgatacagtctccgcaggcgagacaaccagtctgtatattgaggtgaaggataattacggcaacggtgtcccccagcaggaggtaaccctcagcgtttcaccaagtgaaggcgtgacccccagtaataacgctatatatactaccaaccacgacggcaatttttacgcaagctttaccgctacaaaagccggggtttatcaattgacggcaaccctcgaaaatggcgattcgatgcaacaaacagtgacctatgtgccgaacgtcgcgaatgctgaaatcacgctggcagcctcgaaggatccggtgattgccgacaataacgatctcacgacactaacagcaacagtcgctgatacagagggcaatgcgatagccaacactgaggtaacatttactctgccggaagatgtgaaggcgaacttcacgctgagcgatggcggtaaagtgattactgatgctgaaggcaaagcgaaagtcacgctgaaaggtacaaaagcaggcgctcatactgttacagcatcgatgactggcggtaagagtgagcagttggtggtgaactttattgcggatacgctcactgcgcaggttaatcttaacgttaccgaggacaattttatcgctaataacgtcgggatgaccaggctgcaggcaacagtgactgatggaaacggcaacccgttagccaatgaggcggtgacattcacgctaccggcagatgtgagcgcaagctttactctcggacaaggcggttccgccattactgatatcaacggcaaggctgaagttacactgagcggtacaaaatccggcacctaccccgtgacagttagcgtgaacaattatggtgtcagtgatacgaaacaggtgactttgattgccgatgctggtaccgcaaaactagcctccttaacctctgtatactcattcgtcgtcagcacgaccgagggcgcaaccatgacggcaagcgtcactgacgctaacggcaacccggtagaaggcataaaagttaatttccgcggaacctccgtcacgctaagcagcaccagcgttgaaacggatgatcggggtttcgctgaaattcttgtgacaagcaccgaggtcggactgaaaacagtttcagcctctctggcagataaacctactgaagtcatctcgcgattactgaatgccagtgcagatgttaattctgcgacgattaccagtctggagataccggaaggtcaggtaatggtcgcacaagacgtagcagttaaagctcacgttaacgaccagtttggcaacccggttgcgcatcaacccgtgacattcagtgcagagccatcctcgcaaatgatcatcagccagaatacggtctctactaatacgcagggtgtagccgaggtcaccatgacgcccgaaagaaacggttcgtatatggtgaaagcatccctgccgaatggagcctcacttgagaaacaactggaggctattgatgaaaaactgacactcacggcgtccagtccgcttatcggtgtctatgcccctacaggcgctactctgacggcaacgctaacctctgcaaatggcactccagtggagggtcaggtcatcaactttagcgtaacgccagaaggggcgacgttaagtggcggaaaagtgagaactaactcttcaggtcaggctccagtcgttttgaccagcaataaagtcggtacatatacggtgactgcatctttccataacggcgtaacaatacagacacagacaaccgtgaaagtcactggcaactcaagcaccgcccatgttgctagctttatcgctgatccatcgactatcgccgccaccaacactgatttaagtaccttaaaggcaacggttgaggatggcagtggtaacctgatcgaaggtctcactgtgtacttcgccttaaaaagcggctctgccacattaacgtcattaacagcggtgaccgatcaaaacggaatcgcgacaacaagcgtgaaaggagcgatgacaggtagcgtcacggtaagcgcagtcacgaccgctggtggaatgcaaacagtagatataacgctggtggctggcccggcagacacctcgcagtccgtccttaagagcaatcggtcatcactgaaaggggactataccgatagtgctgaattacgtcttgttctgcacgatatatcaggcaatccgatcaaagtttctgaagggatggaatttgtgcaatcaggtactaacgtgccctatataaaaattagcgcaattgattacagtctaaatatcaacggtgattacaaagccactgttacaggaggcggagagggtatcgcaacgctgatccctgtattgaatggtgttcatcaagctggtctgagtaccacaatacaattcactcgcgcagaagacaaaataatgagcggtacagtatcagtcaatggtactgacctaccgacaactacattcccttcgcaggggttcaccggggcgtattatcagttgaataatgacaactttgccccaggaaaaacggcggctgattatgagttttcaagctctgcctcctgggtcgatgttgatgctaccggtaaagtgacatttaaaaatgtcggcagcaattcggaaaggattacggcgacgccaaaatcaggaggccctagctatgtatacgaaatccgtgtgaagagttggtgggtgaacgccggcgaggctttcatgatatacagccttgctgaaaatttttgcagcagcaatggctacacgctccccagagcaaactatttaaaccactgtagttcccgaggcatcgggtcactgtacagtgaatggggagatatggggcattacacgactgacgctggttttcaatcaaatatgtattggtcatctagtcccgcaaactcaagcgaacaatacgtagtttccctggcaacaggtgatcaaagcgtatttgaaaagcttgggtttgcttatgcgacatgttataaaaacctgtgattttccgttataatttcttaaagagtgttccattcggggcactcttttttacattccctctacagaactagcccttctctcacagaaaatgaataaataaaaatgcggcaccgccagaatcgcgttcgatgtgactatgatcattttcggtgagtactgctttgatctaaaggctggttttctgtgatgattgaccagcctcagagtattgatgacaccaccgttcataacagatcggcattactatgcataagtactgtctcatattctcgccaaaacactttttaatgcctttgcgaattcatccagacttatattgtcaattttttgcccaacgacgactgactccgagacatcggccattgcgggccatcgcgttttgtaatcagcataaattgcaacaacaggggtattataggcacttgccatatgtaatattgaggtgtcaggagttattgcgatataagcatcttttatgattgctgctgaacgtttaatcgagggtggtaaggataaacggtagacattattataacaatccactaatgccctggctttatcttcacctttgggtccatgaacgatcactattggtatatctgtttcactttaaatttttgctattagattttctgcaatcgataatgaaaatgtacgttcctgcgagctaccttctaaattgaacgcaatgtaagatcctaacgatcgcatttcctcgcgcacctcatcgagtacatcctcacttagtggcaattcatatattggcctgactgctggaaaacccgcctcacgcatcataaatgcccatgtcataggtacgggagcccggagtttctgatccatactggacgcgttcttgcacaaaggggagaagcaattcatggttataccaacaacctgaaaattcgtttttgctttcaactgactgataaataacatcgttttcaggttctttttacgcatcccctcaatgcaaagatccggcgtaccgtattgctgtgttatgttctttgctaaatcttttatttcttttaatgttgcgtgatcctgcatagtcattgtgactaatgttaatttagtctgttcaagtttaagcgcattaaagacttctaaattaattgtcgacgttacaattaaaagatgcttaattttatgcaattcaagcgcccgaataacaggaaagatggccatagcatcgccaatctgatcgggaatatggatgacaacaaagtctgttttttcaatattgaaattataagctttataatcgtagtaactaaatgcaatacgtctcaacaatgatgctaaaaacatacctaacctcgcctccctactggttataatgcaatgcagtctatcagactcatcagggtgccattttgtgcatatgcggacttttatgtttcatatctctaacctgtgggtcctctgcttaatccttaaacaacaccagcaactcctgcgctttcatcttccatcgaatttttcatgttgccgctaatcagccataaaatcatttgcagatgcgctctgtcgaggtagtctcataaggttcgtttatagatcgacggcaatgtgagttaccttttccatactaattataaaaagacagtacaaacaggatcattatggactccacgctcatctccactcgtcccgatgaagggacgctttcgttaagtcgcgcccgacgagctgcgttaggcagcttcgctggtgccgtcgtcgactggtatgattttttactctatggcatcaccgccgcactggtgtttaatcgcgagtttttcccgcaagtaagcccggcgatgggaacgctcgccgcatttgctacctttggcgtcggatttcttttccgtccgctcggcggtgtcattttcggtcactttggcgaccgactgggacgtaagcgcatgttaatgctgaccgtctggatgatgggcatcgcgacagccttgattggtattcttccttcattctcgaccattgggtggtgggcacctattttgctggtgacactgcgtgccattcagggatttgcagtcggcggcgaatggggaggcgcggcgttgctttccgttgaaagtgcaccgaaaaataaaaaagccttttacagtagcggtgtacaagttggctacggtgtaggtttactgctttcaaccggactggtttcattgatcagtatgatgacgactgacgaacagtttttaagctggggctggcgcattcctttcctgtttagcatcgtactggtactgggagcattgtgggtgcgcaatggcatggaggagtccgcggaatttgaacaacagcaacattatcaagctgccgcgaaaaaacgcatcccggttatcgaagcgctgttacgacatcccggtgctttcctgaagattattgcgctacgactgtgcgaattgctgacgatgtacatcgttactgcctttgcacttaattattcaacccagaatatggggctaccgcgcgaacttttccttaatattggtttgctggtaggtggattaagctgcctgacaattccctgttttgcctggcttgccgatcgttttggtcgccgtagggtttatatcacaggtacgttaatcggaacgttgagcgcatttcctttctttatggcgcttgaagcacaatctattttctggatagttttcttctccataatgctggcaaacattgcgcatgacatggtggtgtgtgtgcaacaaccgatgtttaccgaaatgtttggtgccagttatcgctatagtggcgctggagtcggttatcaggttgccagtgtggttggcggtggatttacaccttttattgccgctgcactcatcacttactttgccgggaactggcatagcgtcgccatttatttgctggctggatgcctgatttccgcaatgaccgctttgttgatgaaagacagtcaacgcgcttgatagcctggcgaagatcatccgatcttcgccttacacttttgtttcacatttctgtgacatactatcggatgtgcggtaattgtatggaacaggagacacacatgaataataagggctccggtctgaccccagctcaggcactggataaactcgacgcgctgtatgagcaatctgtagtcgcattacgcaacgccattggcaactatattacaagtggcgaattacctgatgaaaacgcccgcaaacaaggtctttttgtctatccatcactgaccgtaacctgggacggtagcacaaccaatccccccaaaacgcgcgcatttggtcgctttacccacgcaggcagctacaccaccacgattactcgccctactctctttcgttcgtatcttaatgaacaacttacgttgctgtatcaggattatggtgcgcatatctcagtgcaaccctcgcagcatgaaatcccttatccttatgtcatcgatggctctgaattgacacttgatcgctcaatgagcgctgggttaactcgctacttcccgacaacagaactggcgcaaattggcgatgaaactgcagacggcatttatcatccaactgaattctccccgctatcgcattttgatgcgcgccgcgtcgatttttccctcgcacggttgcgccattataccggtacgccagttgaacattttcagccgttcgtcttgtttaccaactacacacgttatgtggatgaattcgttcgttggggatgcagccagatcctcgatcctgatagtccctacattgccctttcttgtgctggcgggaactggatcaccgccgaaaccgaagcgccagaagaagccatttccgaccttgcatggaaaaaacatcagatgccagcatggcatttaattaccgccgatggtcagggtattactctggtgaatattggcgtgggaccgtcaaatgctaaaaccatctgcgatcatctggcagtgctacgcccggatgtctggttgatgattggtcactgtggcggattacgtgaaagtcaggccattggcgattatgtacttgcacacgcttatttacgcgatgaccacgttcttgatgcggttctgccgcccgatattcctattccgagcattgctgaagtgcaacgtgcgctttatgacgccaccaagctggtgagcggcaggcccggtgaggaagtcaaacagcggctacgtactggtactgtggtaaccacagatgacaggaactgggaattacgttactcagcttctgcacttcgttttaacttaagccgggccgtagcaattgatatggaaagtgcaaccattgccgcgcaaggatatcgtttccgcgtgccatacgggacactactgtgtgtttcagataaaccgttgcatggcgagattaaacttcccggccaggctaaccgtttttatgaaggcgctatttccgaacatctgcaaattggcattcgggcgatcgatttgctgcgcgcagaaggcgaccgactgcattcgcgtaaattacgaacctttaatgagccgccgttccgataataagttctgaaccttcttatcagaaatagatgtgaaggagtaagtaagacacctggcaaatagcctgcaataatcgtgggctgtttgcttccttgggcggatacgagttttattatcgtcttaatgatttccacatattaaaagcaagtatgctttcaaaacacaattataaaaaatcccgccaacaatataagtttttataaaattaaatataagattatggctttagaatatttttatttctaatagacgagatttttcctgttatgatataatatgctgaattaacacatgttaacgatttaccagtaatgtaaataaattttcgaggagatcattccagtgggacgtaaatgggccaatattgttgctaaaaaaacggctaaagacggtgcaacgtctaaaatttatgcaaaattcggtgtagaaatctatgctgctgctaaacaaggtgaacccgatccagaattaaacacatctttaaaattcgttattgaacgtgcaaagcaggcacaagttccaaagcacgttattgataaagcaattgataaagccaaaggcggcggagatgaaacgttcgtgcagggacgttatgaaggctttggtcctaatggctcaatgattatcgccgagacattgacttcaaatgttaaccgtacgattgctaacgttcgcacaattttcaataaaaaaggcggcaatatcggagcggcaggttctgtcagctatatgtttgacaatacgggtgtgattgtatttaaagggacagaccctgaccatatttttgaaattttacttgaagctgaagttgatgttcgtgatgtgactgaagaagaaggtaacattgttatttatactgaacctactgaccttcataaaggaatcgcggctctaaaagcagctggaatcactgagttctcaacaacagaattagaaatgattgctcaatctgaagttgagctttccccagaagatttagaaatctttgaagggcttgttgatgcccttgaagatgacgacgatgtacaaaaagtttatcataacgtcgcaaatctctaattatcttttaaagaaatctgtctttacggcagatttctttaatctcatataattcttataaaaaatataatattcaactcgtcatattgattatacccccccgttcccagagaaataatatttattaaaattccagttcttctttttctgattacagaaggcaaagtggcaattacgcatagtttcccgataaagacgcgatagcgacatcccgcataaggcatttttctctttatctttgtacggtacttcatggaacagagtttttgaccttgcgaatcgtgatgtctgttggggagggacaatttgctcactgaagcgtgagactcgattaagcgcacgaaacacagaaatcaaaaaacccggtcacttttttacaaggtaaccgggtaaaaataatttttattttttaactgttttgagactcatagagatgtctcaaaactaaaatttggctcctctgactggactcgaaccagtgacatacggattaacagtccgccgttctaccgactgaactacagaggaatcgtgagaacgaggcgaatattagcgatgcccacccacaatgtcaaagcctgttttttaaatttgaaatcgtttgctgaaataatctgcattttgtcgtttattccgacacaactggctttttttcacacttttgcggctcgggtcgagggtatttccatagccaacgtccagtaaccattcgccagtaaaacagcacggcccgcacagcccagtcggcaaacattcccatccagacaccaaccacaccccagccaagcatgattcccagcacataaccgactacaacccgacaaccccacatgctcaacatcgaaacccacatggcgtaacgggcatcacgagcacctttaaatccagcgggtagcacccatgaggcggaccaaataggcataaataaagcatttagccaaatcagaatcacaacgacatgtttaacctgtggatcctgggtgtaaaacgatgccataaccccggcaaagggagccgttagccaggcgatggccgttaatccaagagtggaaagccagaacacatgccgcaactgaatctctgcttgcgctatctgccctacccccaaccttcggcctgtaatgatcgtagaagcagagccgagcgcacttccgggtaagttgataagagccgcaattgaaaacgcgataaaatttccggcaataacactggtccccatcccggcaacgaacatttgggttaataaccgaccactggtaaataacactgattcgacactcgcgggaataccaatccccatgacttcccagataatgctaaaattcagcggtttaaaatagctctttaacgaaatccttagcgcaggattaaaaccaatcgccagcacccacaaaattgcaactgcgccaatataacgagaaatggttaaacccagccctgccccgacaaatcccagtcccggccaggagaaaaggccgtaaatcaatatgccgctaataataatattaagaatattcaggctaccgttaatcaatagcggtattttcgtattccctgcaccacgaagtgccccgctaccaataagagtgatggcagctgctggataactgagtaccgtcagctccagataagtcaacgccagtgctttaacttctgtcgtggcatcacccgcgacgaaatcaataatttgttcgccaaaatgatgaataagcgttgccaacagtacggcaaacaacgtcatgatcaccaatgactgccgcgtcgccaccctcgctcgtcgtcgatcccgcttaccgagactaaatgccacaacgacagtagtaccaagatcgatagcagcaaaaaaagccataatgaccatattgaagctgtccgccaatcccacgccggccatcgcatcttttcccagccagctgaccagaaaagtgctcagaacccccatcaacaggacacaggcattctccatgaagataggaacagcaagcggggttatctcgcgccagaacaacactttgtagctcttgcgtttagcgtgccagcgagtgccgtgaacaacctggcgtaaagcagaggagatattcaaagccgaccttaattgcagaaagtgaaaccacatttcaaataatgagggagaatcagcaaagctgcaaagattttcgccaacaaattgtctgcaaatgcaacaaactgttgatagaaacggcaaacagttggggaatttaaaaatcgggtttgacaaaagatttttcgccgttaagatgtgcctcaacaacgattcctctgtagttcagtcggtagaacggcggactgttaatccgtatgtcactggttcgagtccagtcagaggagccaaattcctgaaaagcccgcttttatagcgggatttttgctatatctgataatcaatttcctcttcactgctttccatcacctgccgcttgatatcctcaactgacagtcctgcattacaaagttccagaaagcgccagacatagttacgctgaagttgtcctcgcttcagtcccaaccagacagtattagcatcaaaaagatgccgcgtatccaggcggattaaattctcttcctcttgttcgccactggattgctcggcaactaatccgatcccaagcccaagagcaacataggttttaatgacatcagaatcctgcgcacttaatacaatatctgccagcaaacctttgcgggcaaatgcgtcatcaatacgtgagcgccccgtaatcccctgtcggtaagtgattaacggccacttcgctattgattccagcgtcaatggtgaaatttgcgtcaagggatgatcgtgtggaacaagcaaactatggtgccaacgaaaccacgggaaggcgacgagctgcgggtcattactcaaacgctcgctggcgataccaatatcagcttcgccattttgcaacaatgtcgcaatttcctgtggcgtcccctggattagctcgagccgaacctccgggaaaagttcgcgaaaagctttaatgacctctggcaagctataacgtgcctgagtatgcgtcgttgcaatagtgagaacgccagacgtatcgttggtaaacaggtctgcaagccgacgaacattactggcttcattcagaatacgttctgcaatgaccagtaatgctttgcccggttcagtcatgcccagcagtcgcttacctcgtcgaacaaatatttcgatgccaagttcatcctccagttcccgaatatgacggctgacgcctgactgtgaggtaaaaagcatattcgcaacctctgtcaggttgtaatcctgacgtgcagcctcgcggattatctttagttgttggaaattcacggtaaactccgggcagttcagatttcccgttattgttaaagtctaatgcccggcataacaaataataaaaacccgcatcttattccatcccgatataacacttagctcaccaattgccactgccttttttccatcactggagaactaatcactgacattaacaactctttcactgcctgtgcctgtggcgataagttcgctctggcgggtaaatttaatgacaaagagagactcatggaaggagtggtaatgcgtgacatccacccatttactgcgccacataacgaacgcgcggccgattcgggtaatactgcaacgcccatgccgctggcaatcgctgcggtaagcgtggcaatagactcaatttcaccaataacttttgccgtgagtcgccgtagggaaaaagcctcatcaacacgaagtctaatagcactgtaatcactggggagaaagaggttcatttgcgcaatagcattcacatcaacgctttgccccgggcaatcttgagttcctaccagaaaaagatcttctttcagcaaagcctgactggatacaccagccacaggggaatgctcataaatcaccgccatatcgagttggtgatttatcaatttttcgttaagcactgcaccactattttcatgaagatagataacgatctccggaaattcagcgcgaaccgcctgtaataagggcatggtgatggatgacgcagcggttcctggtgcaaagccaatcgagacttgccccgataatgcctgaccaacgttatgcaccgccagttgggcctgttcacactgacgtaaaatggcccgcgcatgggtatagagaatttttccggcgtctgttggtgtaacgccccgctttgtacggatcaaaagttgttgatttaactcaccttccagtgtggcaacctgctggctgagcgctggttgtgcgatatgcaatacttcagcagcctgggtcaggctaccaatatctacaatttttacgaagtatttcaggcgtctgaagttcatgttgcctccggtttttaagaatcggcccaagtgccgccattacttacaaccagattgcaagatgcttgccagttttattttggtgttgatgtacaagctaaccaactgtcaaataagagattatgatagattcgtcatttgctcctttaatcagctgtcgcgttcccctgccctataaaaggagggtatgcaccacgatggttcattacccaataagattgaaagctcaccactttgttgaaattgacagcaaacaaacaaaaaaatgcatttcaccctttgacatcaccatgcactgccattaatatgcgccccgttcacacgattcctctgtagttcagtcggtagaacggcggactgttaatccgtatgtcactggttcgagtccagtcagaggagccaaattcaaaaaagcctgctttctagcaggctttttgctttctaattaccaacgctcttaaaacatctgtcttgaaccagaactaatttgcacaggcattcccgatcgacgttgcaacgcagcatttgcgcgatttacatcaacttcttgcccgttgataaacgcccgcaaagatggggttaccggcaatggcacttttcggtcagactcatattctgcacgattgcgcgacaatggctcatgaacttccagccagttcgagccatctggttcagtggtgtattttactggctggtcgataatttgcacacgcgtcccaacaggaacattatcaaacagatatttgatatcgtcattgcgcagacgaatacagccctgacttacccggagcccaataccaaaattggcattggtaccatggatggcatacaacctgccaatataaatcgcgtacagccccatgggattatcggggcccgcaggaacaaatgcgggcaaactctcccctcgtttcgcatattcgcgccgagtgttcggcgttggcgtccaggttggagcttcttgtttacgttcaacggtagtcacccagttacgcggggtttctcgcccagcctggccgataccaataggaaagacttccacagtattactgtctggtgggtagtaataaagacgcatctcagcgacgttaacaacaatccctttacgaacagtgtcgggcaaaatcagttgctgcggaatggtgagttgcgagccagacttcggcaaaaaaacatcagcgcccgggttcgcttccagcatgttacttaacccttgcccgtattgtgcggcaaaagtctccagcggctgggtattgtgatcaggaacagttacagtaaacgactgccccactaaacggctaccctctggaggtaatggataagttaccgccaggctagtatggctggcaaaaagcagagcaaatgagcaaagaatatttacacgacgcatcatgtccctttcctatgtcgcgaaagctatccgttaagtatagcttttatcagacttttcgtttttaactgttcaaatcagaagtcgtattccccggtagaacaatattactggcagcaagttcgcccatgttgttgtatatcgcacaggcagcttcgatgatgggcatcgccagagctgcgccactcccctcacctaaacgcatctccatattgagataaggctccagccccaaatgcgagagcgctatacgcgcgcctttttctgccgacaggtgagaaggaatgagatacggtttgatcgcaggagacatctggcaggctgcgagcgcagcagcataagaaagaaatccatccagcaacacgggtaaaccgcaggaagcagcacctaacatcactccagctattccgaccaaatcaaatccacccacttttgccaggacatcaacaccatcctgaggatttggttgattcaacgtaatcgcccgacgcacaacatcaattttattagccagtttatctgtcggcaggtttgcgccaatcccaaccacttcttcaggatcccggccagtgattgtgctgactattgctgctgccggtgtcgtgtttgccatccccagttcacctacaccaaacagcgtgacaccgttttttgccagctcctgcgtataacatatgacgtccaaaagcaacttttcagcctgacggcgactcattgccggagctgaagcaatattgccgctacctcgtgcgacacgcatgttgataagcccggggataggctcagcagtatcaataccaacatcaattacgtggacgttagcgcccgcttgttctgccagcacacacacgccggttgttccacgggtcatattttcagcctgtatggctgtcacttcttttggagaaatagcgaccccttcctcccagacgccgtgatcggcacacataaccagtaccgcttttttgcccacatgcggtatgccattcaaccccggcattcctgccagttgtatggcaagcacctccagctttcccaggctaccaacaggtttgagtaacccgtcaatatgccgttgtgcacgcgacatagcggtagaatcgatggctgggatcgtattcagtaaatcggcaagtatttgcatctcacgtctctttatagcagtgccagcaggaagaccagttcaccaagctctatggctgctcccagcgtatcgcccgtttgcccgcccagcgtacgtttgagaagctgaccgaggatgaaaatcgccaccatcgtcaccaccatagcagccacaccatgcatacccggcaataatacggcagcaaaaatagcggctaagccgagtgtgacgcaggtttgtcgcccatcaattttgccaatgaacacattgccaagcccttcttcccgcgcataacgatgacgatacatcaataatgcggcagtcccgcggctgaccgcacatgctgccgccagcgatgcaaggatcgattcgccacgcagagccaactcgcttaacaccagaatctttgccagtaccacaaaaatcaatgccagaccgccgtgggtgcctaaacggctatcacgcatgatttccaacatgcgatcgcggctacgtgcagaaaatacgccatcacaggtatcagcgaggccgtccagatggaatcccccggtcatcagcaccagcacaagtacgctaaacagtgccgccagtggtgcgccacaccatgcctgcagcaccatgaagaccagcccgctaatcgcgccaagcaataatccaatcaaaggaaaagtaataataccgcgagaataatgctcgaaatccagtccctgggaccagcgacgcggtacaggcagacgcgtaataaatgagagcatcgcccaaaataatttactcatttgatttttactccaatacccgaaaccaccagccatacttcatttgccgcagcggccaactgctgatttacccgcccggcaatatcacgaaaatgtcgtgccagacgactctccggcacaatccccattcccacttcgttagtcactaatacaacctttgcggggcaacgttggcaggcagcaatcaacgactgaatctcagcattaatcgcctgttccatcgcctgataatcccattcatcagggtctttatcgccgccataatcaaacaacagattagtcaccattgtggtaacgcattcaagcaacacaacctcattcgggttaatgtctgcatgaattaattcatcaagatgttgccagcgctccactgtgcgccagtgctccgggcggccttgccgatgatgttctatccgtgcagccatctcatcatcaaggatttgcgaggtagcgatatacagaacctgtgaagagtccccaataagcgcctctgcgtggcgactcttcccgctccgtgcgccccccgtcaccaaaatcatcataccgactcctgattcaaatgtatgatggtattcattgaacagaacaatggatcccccaccgttgctgaccgcaaaacatttacgcgattaatactgcgcgtaatataattaaaaatccagcattctcaatccattacgaaataagatggcattacggaatagccagactttctcgtgttaacgtccgacaaaatgcgtcattgacagcggtttctgtggattgacacatttcattcagataatgaattaatgctactgccggaacaaccagcaaacgggcattgtgttctgaaatccaggctattgattcaacgtcagcgacagatctgcgctgtaaaagaacttgtaaaacaacgtaatagaattatccggaatggtggcgactatgcactagggaaggtgcgaataagtggggaaattcttctcggctgactcagtcatttcatttcttcatgtttgagccgattttttctcccgtaaatgccttgaatcagcctatttagaccgtttcttcgccatttaaggcgttatccccagtttttagtgagatctctcccactgacgtatcatttggtccgcccgaaacaggttggccagcgtgaataacatcgccagttggttatcgtttttcagcaaccccttgtatctggctttcacgaagccgaactgtcgcttgatgatgcgaaatgggtgctccaccttggcccggatgctggctttcatgtattcgatgttgatggccgttttgttcttgcgtggatgctgtttcaaggttcttaccttgccggggcgctcggcgatcagccagtccacatccacctcggccagctcctcgcgctgtggcgccccttggtagccggcatcggctgagacaaattgctcctctccatgcagcagattacccagctgattgaggtcatgctcgttggccgcggtggtgactaggctgtgggtcaggccgctcttggcatcgacaccaatgtgggccttcatgccaaagtgccactgattgcctttcttggtctgatgcatctccggatcgcgttgctgctctttgttcttggtcgagctgggtgcctcaatgatggtggcatcgaccaaggtgccttgagtcatcatgacgcctgcttcggccagccagcgattgatggtcttgaacaattggcgggccagttgatgctgctccagcaggtggcggaaattcatgatggtggtgcggtccggcaaggcgctatccagggataaccgggcaaacagacgcatggaggcgatttcgtacagagcatcttccatcgcgccatcgctcaggttgtaccaatgctgcatgcagtgaatgcgtagcatggtttccagcggataaggtcgccggccattaccagccttggggtaaaacggctcgatgacttccaccatgttttgccatggcagaatctgctccatgcgggacaagaaaatctcttttctggtctgacggcgcttactgctgaattcactgtcggcgaaggtaagttgatgactcatgatgaaccctgttccatggctccagatgacaaacatgatctcatatcagggacttgttcgcaccttccctagaacaccacaatttcgctctctcggtaaggcactgtcacagcattcaacagaatgtgacttgccagatttattagcgccaccagatgtttaaccgggtaaccacgacccagtcggggatatattccatcttctcgctgacatcatcaagaataaaaaggtttatcacactcagagcaacgttcttcagcaggcgggataattcttcaacatttagaagatgtgttattaaaggcatacaaactggacgtattgtattttcttttggtggttgacctaaggtagcagtttatcctgatgcgctgagatttctgtaatatctacgtcaacattctcctcgaatagaaaatgcagccccggcaagtgattcacattttttaacaaaacgttgttagcgtgccattttcagaagctctccaagaaagcgaattcttttctcaaattctgcattctcagacacagctttctactccatggtaatggcccaaatacgaagttgctcaggatcattagtggtgctgagaagttaaataaccatgcggagtaccactcgtcatcacgtatttatatatcatgaagctattgttgtgttttgtacatcagtagatatattctgatatactccttttgctagacataacctttcacctgcttgcaaagcttctgtgttctgacattgccaaattgttgcaattctgtatccagccttctttcagtcatagcttcgggccgcgataagactcactgatctgaccctgattcctcttgcagactttatagaccaattaaaatgcagtttctgcaggtcaacgtctgaccatcattgtcatcactctggccattagagtaaccttctgcattcatccttttgtaaaaagtttatattagtatcagcaattaaccggacctgatactgatatgagtcttaccgcatatacggtcaatttcagcaattaattacattatccacgccaaagtatttgtcatcacaatgatggtaccttctttcagacaccattttttcaactccgttttccacggaccgcactcttatgtcaagagtgcggtccgtggatacaaccagagaccgactgacacgagtcagaggaaacgacggatatgttcagtcgtaaaatatctatcaaaaaacatgattaaggtcaaaaatgtttgatatttacaatttatgaagatgacaataattatagatatatgagaacataaatgaaaataattatcattacagtaatcatttgtactttgtattaatgagggatgaaatgttatataatataccttgtcgaatttatatcctttccactctgtcattatgcatttctgggatagtttctactgcaaccgcaacttcttcagaaacaaaaatcagcaacgaagagacgctcgtcgtgaccacgaatcgttcggcaagcaacctttgggaaagcccggcgactatacaggttattgaccaacaaacattgcagaactccaccaatgcctccatagccgataatttgcaggacatccccggagtagagataacagacaactccttggcaggccgtaaacaaatccgcattcgtggctggatttgcccctatatttccagacatctgttatcacttaacccattacaagcccgctgccgcagatattcccgtggcgagcgataacccagcgcactatgcggatgccattcgttataatgctcgaacgcctctgcaaggttctttgctgccgttaacccgtctggtttgggcatgatactgatgtagtcacgctttatcgttttcacgaagctctctgctattccgttactctccggactccgcaccgccgtgttcttcggttcaagtcccaacatccgggcgaactggcgtgtttcattagcccggtagcatgaaccattatccgtcagccactccactggagacgacggaagatcgttgccgaagcggcgttccaccgctcccagcatgacgtcctgtactgtttcactgttgaagccgccggtagtgaccgcccagtgcagtgcctcacgatcacagcagtccagcgcgaacgtgacacgcagtctctctccgttatcacagcagaactcgaacccgtcagagcaccatcgctgattgctttctttcacggccactctgcctgtatgtgcccgtttcgatggcggtacagcaggttttcgctcaagcaacagcgcattctggcgcatgatccggtaaacacgtttggcattgatcgcaggcataccatcaagttctgcctgtctgcgaagcagcgcccatacccgacgataaccatacgttggcagctctccgataacatggtgtatacggagaagcacatccgtatcatcagtgtgacgactgcggcggccatccatccagtcatcggttcgtctgagaatgacgtgcaactgcgcacgcgacacccggagacaacggctgactaagcttactccccatccccgggcaataagggcgcgtgcgctatccacttttttgcccgtccatattcaacggcttctttgaggagttcattttccatcgttttcttgccgagcaggcgctggagttctttaatctgcttcatggcggcagcaagttcagaggcaggaacaacctgttctccggcggcgacagcagtaagacttccttcctggtattgcttacgccagagaaataactggctggctgctacaccatgttgccgggcaacgagggagaccgtcatccccggttcaaagctctgctgaacaattgcgatcttttcctgtgtggtacgccgtctgcgtttctccggccctaagacatcaatcatctgttctccaatgactagtctaaaaactagtattaagactatcacttatttaagtgatattggttgtctggagattcagggggccagtctagtggcgaagcatcctcccgtgttttaattctcattgatggtcaggaggtaacttatcagcgcgccggagataattatggtgtgggactgttgatagatgagtctgcgctggagcgtgttgaggtagtgaaaggtccatattccgtactgtacggttcacaggcaattggcggtattgttaacttcatcaccaaaaagggtgaatctccggactccctatatcacttaaattgatacaactttttagagtagtcattagtgaacagataattgataactcagaaccagtaaaatgcaaaagacgcaccacgctgggaaaatcgctgctattcagcagagttttgtatcgagaatggtggccagccacttattgctctcgcgtaagcgggtaccgtgacattctgcctgaacttgacctggtactgtggctgattaaagccgatgaccgtgccctgtctgtggatgagtatttctggcgacacatcctgcagtgcggacatcagcaggtgctgtttgtggtgacgcaggccgacaaaacggagccctgccatgaatgggatatggccggtattcagccttctcctgcacaggcacagaatattcgcgaaaaaacggaggcggtattccgtctgttccggcccgtacatccggttgtggccgtatcggcccgcaccggctgggaactggatacgctggtcagtgcgctcatgacagcgcttcccgaccatgccgccagtcccctgatgacccgactgcaggacgagctgcgcacggaatctgtccggtctcaggcccgtgaacagtttaccggtgcggtggaccggatatttgacacggcggagagcgtctgtattgcctctgttgcacgcacggttctgcgtgccgtccgtgacacggtggtctctgttgcccgtgcggtatggaactggattttcttctgaacctgtcgtgactgatgccctccctgactctgagtctgctcacaaaagcactgttttcgttactgtctctcttgtccgtgcaatagctcaataatagaataaaacgatcaatatctattttatcgatcgtttatatcgatcgataagctaataataacctttgtcagtaacatgcacagatacgtacagaaagacattcagggaacaacagaaccacaattcagaaactcccacagccggacctccggcactgtaaccctttacctgccggtatccacgtttgtgggtaccggcttttttattcaccctcaatctaaggaaaagctgatgaaacgacatctgaatacctgctacaggctggtatggaatcacatgacgggcgctttcgtggttgcctccgaactggcccgcgcacggggtaaacgtggcggtgtggcggttgcactgtctcttgccgcagtcacgtcactcccggtgctggctgctgacatcgttgtgcacccgggagaaaccgtgaacggcggaacactggcaaatcatgacaaccagattgtcttcggtacgaccaacggaatgaccatcagtaccgggctggagtatgggccggataacgaggccaataccggcgggcaatgggtacaggatggcggaacagccaacaaaacgactgtcaccagtggtggtcttcagagagtgaaccccggtggaagtgtctcagacacggttatcagtgccggaggcggacagagccttcagggacgggctgtgaacaccacgctgaatggtggcgaacagtggatgcatgagggggcgatagccacaggaaccgtcattaatgataagggctggcaggtcgtcaagcccggtacagtggcaacggataccgttgttaataccggggcggaagggggaccggatgcagaaaacggtgataccgggcagtttgttcgcggggatgccgtacgcacaaccatcaataaaaacggtcgccagattgtgagagctgaaggaacggcaaataccactgtggtttatgccggcggcgaccagactgtacatggtcacgcactggataccacgctgaatgggggataccagtatgtgcacaacggcggtacagcgtctgacactgttgtgaacagtgacggctggcagattgtcaaaaacgggggtgtggccgggaataccaccgttaatcagaagggcagactgcaggtggacgccggtggtacagccacgaatgtcaccctgaagcagggcggcgcactggttaccagtacggctgcaaccgttaccggcataaaccgcctgggagcattctctgttgtggagggtaaagctgataatgtcgtactggaaaatggcggacgcctggatgtgctgaccggacacacagccactaatacccgcgtggatgatggcggaacgctggatgtccgcaacggtggcaccgccaccaccgtatccatgggaaatggcggtgtactgctggccgattccggtgccgctgtcagtggtacccggagcgacggaaaggcattcagtatcggaggcggtcaggcggatgccctgatgctggaaaaaggcagttcattcacgctgaacgccggtgatacggccacggataccacggtaaatggcggactgttcaccgccaggggcggcacactggcgggcaccaccacgctgaataacggcgccatacttaccctttccgggaagacggtgaacaacgataccctgaccatccgtgaaggcgatgcactcctgcagggaggctctctcaccggtaacggcagcgtggaaaaatcaggaagtggcacactcactgtcagcaacaccacactcacccagaaagccgtcaacctgaatgaaggcacgctgacgctgaacgacagtaccgtcaccacggatgtcattgctcagcgcggtacagccctgaagctgaccggcagcactgtgctgaacggtgccattgaccccacgaatgtcactctcgcctccggtgccacctggaatatccccgataacgccacggtgcagtcggtggtggatgacctcagccatgccggacagattcatttcacctccacccgcacagggaagttcgtaccggcaaccctgaaagtgaaaaacctgaacggacagaatggcaccatcagcctgcgtgtacgcccggatatggcacagaacaatgctgacagactggtcattgacggcggcagggcaaccggaaaaaccatcctgaacctggtgaacgccggcaacagtgcgtcggggctggcgaccagcggtaagggtattcaggtggtggaagccattaacggtgccaccacggaggaaggggcctttgtccaggggaacaggctgcaggccggtgcctttaactactccctcaaccgggacagtgatgagagctggtatctgcgcagtgaaaatgcttatcgtgcagaagtccccctgtatgcctccatgctgacacaggcaatggactatgaccggattgtggcaggctcccgcagccatcagaccggtgtaaatggtgaaaacaacagcgtccgtctcagcattcagggcggtcatctcggtcacgataacaatggcggtattgcccgtggggccacgccggaaagcagcggcagctatggattcgtccgtctggagggtgacctgatgagaacagaggttgccggtatgtctgtgaccgcgggggtatatggtgctgctggccattcttccgttgatgttaaggatgatgacggctcccgtgccggcacggtccgggatgatgccggcagcctgggcggatacctgaatctggtacacacgtcctccggcctgtgggctgacattgtggcacagggaacccgccacagcatgaaagcgtcatcggacaataacgacttccgcgcccggggctggggctggctgggctcactggaaaccggtctgcccttcagtatcactgacaacctgatgctggagccacaactgcagtatacctggcagggactttccctggatgacggtaaggacaacgccggttatgtgaagttcgggcatggcagtgcacaacatgtgcgtgccggtttccgtctgggcagccacaacgatatgacctttggcgaaggcacctcatcccgtgcccccctgcgtgacagtgcaaaacacagtgtgagtgaattaccggtgaactggtgggtacagccttctgttatccgcaccttcagctcccggggagatatgcgtgtggggacttccactgcaggcagcgggatgacgttctctccctcacagaatggcacatcactggacctgcaggccggactggaagcccgtgtccgggaaaatatcaccctgggcgttcaggccggttatgcccacagcgtcagcggcagcagcgctgaagggtataacggtcaggccacactgaatgtgaccttctgacagaaccatcgcctctctgtggtcccggtcatcatgaccgggacccggaccggcgcaacggatcttcaacgccacattcgctggcattaacaataacatgatattcatcacggagtgactatgttacagatagtcggcgcgctgatcctgctgatcgcaggatttgccattcttcgccttttgttcagagcattaatcagcacggcttctgcgctggcagggctcatattgctgtgtctgttcggcccggccttactggctggctatatcaccgaacgcataacccggttgttccatattcgctggctggcaggcgtatttctgacgattgccggaatgatcatcagcttcatgtggggacttgatggtaaacatatcgcgctggaggctcacacctttgactctgtgaaatttattctgaccaccgctctcgccggtggtctgctggctgttcccctgcagatcaaaaacattcagcagaacgggatcacaccagaagatatcagcaaggaaattaacgggtattactgctgtttttatactgcctttttccttatggcgtgttctgcatgcgcaccattgatcgcgttacagtacgatatttcaccgtcactgatgtggtggggcgggttgttgtactggctggctgcattagtgacgctgctatgggcggccagccagatccaggcgctgaaaaaactgacctgtgccatcagccagacactggaagaacaaccggtgctcaacagtaaatcgtggctgaccagtttgcaaaacgattacagccttcctgactcactgacggagcgcatctggctgacgctcatttctcaacggatttcccggggagagctgagggaatttgaactggcagacggaaactggttactgaacaatgcctggtatgaaagaaacatggcagggtttaacgaacagttgaaagagaacctgtcattcacacctgatgaactgaaaacgctcttccggaaccgcctgaatttatcaccggaagcgaatgacgattttctcgatcgttgcctggacggcggtgactggtatcccttttcagaaggtcgccgttttgtatcattccatcacgtggatgagcttcgtatctgtgcctcctgcgggctgacagaagtacatcatgccccggaaaatcataagccggatccggaatggtactgctcctctctttgtcgcgaaacagaaacactgtgtcaggaaatttatgaacgcccttacaacagctttatttccgatgcaacggcgaatggtctgattctcatgaaactgccggaaacctggagtacaaatgagaaaatgtttgcttccggagggcagggacatgggtttgccgctgaacggggaaaccatattgtcgacagagtccgtctgaaaaacgcacggatcctcggtgataataatgccagaaatggagcagacagactggtcagcggaacagaaatccagacgaaatattgttcaactgcagcccgtagcgtcggtgcggcattcgacggacaaaacggacagtatcgttacatgggaaataatggccccatgcaactggaagtcccccgtgatcagtatgccggcgctgttgaaaccatgaggaataagatccgcgaaggtaaagtagaggagagatgacgcccggcgagcgcagcctcattcaacgggccctgaaaaccctggaccgccatcttcatgaacccggcgtggccttcacctccacccgtgcagcacgggaatggctgattctgaacatggcgggactggagcgtgaagaattccgggtgctgtatctgaacaaccagaatcagctgattgccggtgaaaccctcttcaccggcaccatcaaccgcacggaagtccatccccgggaagtgattaaacgcgccctgtaccacaatgccgctgccgtggtactggcacacaatcacccgtccggtgaagtcacacccagtaaggcagaccggcttatcaccgaacgtctggtacaggcactgggcctggtggatatccgggtgccggaccatctgatagtcggtggcaaccaggttttctcctttgccgaacatggtctgctttaacccttcacaaccacatcacacctgttttcacttttatcttctgtcttcagaggtatcccattatgaaaattatcacccgtggtgaagccatgcgtattcaccaacaacatccgacatcccgtctttttccgttctgtaccggtaaataccgctggcacggcagtgctgaagcgtataccggtcgtgaagtgcaggatattcccggtgtgctggccgtgtttgctgaacgccgtaaggacagttttggtccgtatgtccggctgatgagcgtcaccctgaactgagtgggaattctgatgagcagaattatcgccactaccggaccattcttagccgattttctgtaaggattttatcgtgtcagacacactccccgggacaacacttcccgacgacaatcacgaccgcccctggtgggggctgccctgcaccgtgacgccctgtttcggggcacgtctggtgcaggagggtaaccggttgcattaccttgccgaccgcgccggtatcagaggcctgttcagcgatgcagatgcgtaccacctggaccaggcctttccgctgctgatgaaacaactggaactcatgctcaccagcggtgaactgaatccccgccatcagcataccgtcacgctgtatgcaaaagggctgacctgcaaagccgataccctcagcagttgtgattacgtttatctggctgtttatccgacgcccgaaatgaaaaattaactctccagaatagccttctgctacggcctggtgttttcaccacgccacttttccatttttatatctgcatatcaggaaaatcttcagtatgaaaacattacctgtattacccgggcaggcggccagttctcgcccgtctcctgttgaaatctggcagatactgctgtcccgactgctggaccagcactatggcctcacactgaatgacacaccttttgccgatgaacgtgtgattgagcagcatattgaggcaggcatttcactgtgtgatgcggtgaactttctcgtggaaaaatacgcgctggtgcgtaccgaccagccgggattcagcgcctgtacccgctctcagttaataaacagcatcgatatcctccgggctcgcagggcgaccggcctgatgacccgcgacaattacagaacggtaaataacattaccctgggtaagtatccggaggcgaaatgatgacactggaagccgacagcgttaacgtacaggcgctggatatggggcacattgtcgttgacattgatggtgttaatatcactgaactgattaataaggccgctgaaaacggttattcactccgcgtggtggatgaccgtgactctaccgaaacaccggcaacttatgccagccctcaccagttgctgtaagacaatgcagtgatacagggtatagtgccattaaccacagaaacagcactgttgtcctgtattaagcaggcaagagaagatgtccttaccctgcgccatctgcagcttctgcaccagaaccggtgaatctcactcaacaggcttcatttctcctgacgccagcctgaatacagctggcgttttcatttataaacagaaaggaaaaccgataataatggaatggacgccccgaccatgaagcaacggtaggatattactgataaaccttccagtggaggtgcgttatggccgttttaacgattagcattgacctgacaaaaaatgaattccaaatccacggtctgggtaggaacagaaaaatctaagctcagaaaacggattaaagtaagcgtcaacggagcaccgtattgacgcttatttattggtgagaactacgttccatggcaggagttcgtcaacacggttggagggccattccggcagtatgctcagaatatggcgcagatacgcttccggatcgataccgttcagacggcaggtgcctgcttttctggcaacaagcaggaatctcagcgctgaagcaggaattagaggtaaaaacgccctaccgggccatgaatcacccggtcattggagtagtaaccaaagcagatttagccagcatggaacaaatatctttggtgaaaagttggttacgggaagctggagcgcacaacgtgttagtaaccagtgcagttaataacaatggagttacagaactttttgccttgctgcatacagaagaaggctgttgttaatttcgattggttctcggatgagaatgatgacggtgatacacagataagaatcaatgagcaatgagggttgccgggcaaccctcattgaataaaacgggaattacttcgcttcgccgtttttcatttcgcccatagctttcagctttttggagatatcgcggcgttctttggagagctcggcatttttgatgatgtaatcgtcaacgcgatcttcatagtcacctttcatgctggcgatgatgccctggattgcttcaacgctcatccccggcttgatgtaatcgctcaggttgtccagcagcaggacgcgcttctggttgtcacggatctttttctcaacgtcctgaatttcacgttgcagtttgttcttacgacggaacagacgaacaaattccagtacgtcctggaatgaaggcttggtagtttccatttttatacccctgataatgtgagagtcggattcgtttaagcaaccgctattcgttagggccaacattactcatagctgccgcagatgacaatgcttttatcccttttcactatcataccctttatccttgctgaatcgaagcagcagcaagatgattctgaagttcaggaattatttgcgcaaggcccggcaaatcagattcgatagcaactcaagctgatgcgccgtttccatgttcagccacacataaccatagattggtgtttccacaaccttcaggtcatggtggttattgagcaactgacgcagctcttccacagcatcgttcaatttttccgtattggcaaaaaccggctgcggattaccttcgtacagcgcatgaacaaggctcagcagtatttgctgcatcatgtgctgggtatcacgaagtttttgcgcgttcaataacacgaaatggctggggcgcgtggcccagtatgcattgatttgcaactccagcatacaaaccagattgcggttaatggtctggataccttcatatatcgattttggaatacgggtttctttgctggcgggcgcaatcagtccacgcattttcacggcatcggtcaggagtttttgtagatggctttccagacgtgggcgttcgagtaagttcggtgagaatgcagattgatagacccgattatactcggtcagacttttcgccagttgaatgcgccagtggatgaacgcccgttgtggccagataccggtaaacaacattgccagtaaagagccgaggatcacatcgccgcttcgccataacgccgtatcaatttcacctgtcggggaacccacaacaattgccagcgtcaccccaatcaataaaccttgatacggtttcttgcccagcgccagccaaccgcaaaggaacatggccgccgcgcaccagactaacatcagcggtaacgagattaactccagttgcagagcgataagacctaaaatcgaacccaacaccgtaccgccaatacgctcaaaggcgcgagggacaacgttaccccagaacgagattggccccataatcaccaccatggtgaccagcggccaggtgctttccgggatagtaaacaggcggataatgagaaaagtgagcaggaatgccagcgcgacccgagtaccatgcacaatgcggtaatggcggtatacccggatttcaaacgggcttaatgacttatcggcacgcacgcagaaactccgtaatgagattaaaagcgctcataactcatctgtcggccagaaggcgcgcctctgaattatccgacggacaaaccgggaacagtgtaatttcccggcaggagcgaaaaaattgaaaggcgcatcttactcttttcgctttcaaaaaaaagagtggtcatcgcgttaacacaccgccctgagatgaattagtgatgttttggctgcaccgcaacatacatttcgatatcccagtacccatcttccgcgccattgttcaaataaacctcgaagcagggctttggtaacatttcataagcactgtcctgcaagagactattaaagaactgataccagggtttagcaaaatcatcaccgactacacgagctaccgccaccgcatactgaccacctgtaatttctgtcagaatgacgccctcactgttttcgggaagcgtaaagtaacccggcaccgtcacgacggtgtcgcagcgtaatttttcggcgggtgtttcatctggattgtcgtaatagacagcaacccactccttcggcacaatatttttgctatctacccacatcatcaactgctcaaagcctttctttaccgtctgttcccacgggccaacgagatggaaacctgcaacggtacgtttctcttcctgcttaatctcgtagttcatgacgcctccattgatactgtttttatatacagtatagttgcaaaattaaaaccacaaggaatgagtgttgattatgcgagcagactcgcactcctgccagtctgctgcaaaagaaaggtcaggccttatggtggaaataatcactcaggcgagaaaacatgctgccttccccgacagattccagggtaaccagcggccagtgcgccacctgtttatcacggtcgtaaagttcaatttcccctacccgctgatgggcgctaattggcgcggtgagttctttaccatcaagggtatatttggctttgatatgtggaatttcggctttcggtagcaccatccagaactcttgttccgttcccaggtcgatattttctttatcgccataccagatgcgttccgttccgacctttttcccacggtgcaaaatttgcaccgtagtaaagttttgttgcccccaacgcagtaattttcttgcctcttcctcacgaccttttgcactgtcagcccccattaccactgcaatgagacgacgctgcccatctacagccgaagcaatgagattaaacccggcaccagaagtatgacccgttttcaggccgtcaacattcatggttttatcccacaacaacccgttacggttttgctgggtgataccgttccaggtgagacttttctcactgtacatatgataaaactcgggctcgccgtggatgatagcacgagaaagcacagctaaatcataagccgagctatgctggccaggtgcatccagaccatgcactgtttcaaaatgcgtatccttgagatgcagcttctcggcatagttgttcatcatttcaacaaactgccgttgcccaccggcaatatagtcagccagagcaacacaagcgtcatttccggaatccacaattaaaccacggcttaaatcacgtaccgatacgcgatcgccctctttcaaaaacatcagtgaagaaccgacaaacaccggattatctttcgcccacgcatcgcgccccacggtgacaatatcgtctggcgtaatgcgatgactatcgatagcgcgatccacgacataacccgtcatcagctttgtcaggctggcgggattgcgctgttgatgctcattacccgcggtgaggatctgaccggtggtgtaatccatcaatacccaggacccggcatgaatctctggaggctgaggtgaaaaaggaatgttttccgccgcaaaaccagacgataagttaaaaacgaacaaagaagcagcaataataagacggcgtttcaacagcaaaccctcaggagtttcaaatagctgttctttttacggaaatacttatgaactggctggaataaagtgcaagaaaatgtgactaccctctcatttttatctgacatgatctgttgccactcgctgccaaattgtggcgctaaagctgattagcacggtgatatttgatactctggcagacagcagaaataacggatttaacctaatgatgaatgacggtaagcaacaatctacctttttgtttcacgattacgaaacctttggcacgcaccccgcgttagatcgccctgcacagttcgcagccattcgcaccgatagcgaattcaatgtcatcggcgaacccgaagtcttttactgcaagcccgctgatgactatttaccccagccaggagccgtattaattaccggtattaccccgcaggaagcacgggcgaaaggagaaaacgaagccgcgtttgccgcccgtattcactcgctttttaccgtaccgaagacctgtattctgggctacaacaatgtgcgtttcgacgacgaagtcacacgcaacattttttatcgtaatttctacgatccttacgcctggagctggcagcatgataactcgcgctgggatttactggatgttatgcgtgcctgttatgccctgcgcccggaaggaataaactggcctgaaaatgatgacggtctaccgagctttcgccttgagcatttaaccaaagcgaatggtattgaacatagcaacgcccacgatgcgatggctgatgtgtacgccactattgcgatggcaaagctggtaaaaacgcgtcagccacgcctgtttgattatctctttacccatcgtaataaacacaaactgatggcgttgattgatgttccgcagatgaaacccctggtgcacgtttccggaatgtttggagcatggcgcggcaataccagctgggtggcaccgctggcgtggcatcctgaaaatcgcaatgccgtaattatggtggatttggcaggagacatttcgccattactggaactggatagcgacacattgcgcgagcgtttatataccgcaaaaaccgatcttggcgataacgccgccgttccggttaagctggtgcatatcaataaatgtccggtgctggcccaggcgaatacgctacgcccggaagatgccgaccgactgggaattaatcgtcagcattgcctcgataacctgaaaattctgcgtgaaaatccgcaagtgcgcgaaaaagtggtggcgatattcgcggaagccgaaccgtttacgccttcagataacgtggatgcacagctttataacggctttttcagtgacgcagatcgtgcagcaatgaaaattgtgctggaaaccgagccgcgtaatttaccggcactggatatcacttttgttgataaacggattgaaaagctgttgttcaattatcgggcacgcaacttcccggggacgctggattatgccgagcagcaacgctggctggagcaccgtcgccaggtcttcacgccagagtttttgcagggttatgctgatgaattgcagatgctggtacaacaatatgccgatgacaaagagaaagtggcgctgttaaaagcactttggcagtacgcggaagagattgtctaatttgaagcctccgccgctggtacggcggaggacaatgttgagtcaggctttttgaacggtgatgctccacgctgcatcgccaatctgctgataatcggtgatggcatgtccttcttctgccgcccactgtgggattgcttcagttgcctgggtgcaatcaaactcaatcactaactcatcgccgctgaccatttctgccagagctgcttttgcttctatgagtggaaacggacagacctgcgtcaccacatccagctttttaatcaccatctttacaccttacttaatttgccgcagcagttgccagtcgcgccttacgctgcggtcgaacatacacaagccaggacgcagtccagactccgagaatcataaatacaaggccaatccagccctgccaggtcatcattgcagtcataaccagtccattaccgatagagcaaccacctgcaatactggcaccgaagcccatcagtacaccacctaacccgctacgtaatgttgtttgtgcatcagctgcgcgaacgcggaactcacggctcgctttggctgcaataaatgaccccacgaagatccctaacaccaggaaaacgccccagttaatgtatttcatgtcacccgcgaccagaaattgcagaatattggccgttggggaagtgattcctaacccaaacatgcgtccggttgcttcactcaggggccaggctaaaagcgcaatcaaaccgatgagtacagctgtgacaaagggatgccagcgtttttcaaacagaatatgagcgatcccggttcggcgcggcggtaaggtcgcgactttgagttttggcttcttcaactctttcatcaccacccagagcgttatcaccagcaaaacggcaaccaacggccacacagacaaattaaaagtctcagcaatagagttatgttcagtactgtagtgctgcaaggtttgatttaaaccactggcatgtggagaacgcatcaccgcactcatcaccatataagtgaaaagcgcgatccaactgccgatcaatccctcacccgcgcgataccaggtcccggtggcacatccacccgccagaacaattcccagcccgaagatatacccacctataacagtaccaagccacgggaacgccccggcttcgtaagtcagtaggcccgcctgaattaacgcaaaaacccccacgctttgtaccgaaattgcaatcagcaaggcgtaaaacatgcgattatttttcacgatatacatatcgcgaaaaccacctgtcaggcaaaaacgcccacgctgcatgacaaatcccagcagagcaccacaaattagcccgcttaatatcattgaaaacataaattaattaaccagatgaatgttaatgaggaaattattcatgactggtggaatgcagaccaataaccaaattctctaaattagaacaaatggttattaatgaggagttcgatacaaaagaataaaaaaaccggagccaaatgttcattcgactccggtttattattagaaaagatgattatgctacgtcttcgtactgcggaaccggattacggaagctcttggtgacgcaagccaggtaaatcagaccgatagcagcccagatcagacccagaaccattgagctttcttccaggttaacccacagcgcaccaacggtcagcgcaccacacatcggcaggaacagatactggaagtgatctttcagcgtcttgttacgcttctcacggatccagaactgcgagatgaccgacaggttaacgaaagtgaacgccaccagcgcaccaaagttaatcagcgccgttgccattaccaggtcgaagttgattgccagcagggcaatcgcgccaaccaggatgatgttcatcgccggagtacgccatttcgggtgtacataaccgaagaagcttttcgggaatacgccgtcacgacccattacgtacatcagacgcgctacgcctgcatgcgccgccataccggacgccagtacggtaatggtggagaagatcagcgcgccaacctggaacgctttacccgcaacgtacagcatgatttcaggctgtgacgcatccggatctttaaagcgagagatatccgggaagtacagctgcaggaagtaagttgcaaagatgaagatcatgccgccgatcagcgcggtcaggaaaatcgcacgcgggatcacgcgctctgcatctttggtttcttccgacaggttgctgatgccgtcaaagccggtaaaggagaagcacaggattgtcgccccggtaatcatcgggataacatgcgcatcgccagaccagaatggacgagtgctcgccagcgtaccagcgccttcaccttcaaatacgccataaacaaccatgcccagaatcaccgcgatcagcactacctgcaacacgacgattacagtgttgaagttcgctacggatttcagactacgcaggttaaaggcggtcataaaggccaccagcgccaccacaaacatccacgatgggatggaaggcaccagagcttcaaaatagattttcgccagtagaatgttgatcatcggcgcgaacagatagtcgagcagagaagaccaacccaccataaagccgacagtcgggctaatggatttctgggcgtaagtgtatgcagagccagcagaaggatagcggcgaaccagcttcccgtagctcagagccgtaaacaggatcgcaatcaatgcgaacgcataggctgtcggcacatgaccatccgtgaggcctgaaacgataccaaaagtatcaaacagcgtcatcggctgcatataggcaagacccatcattacaaccggaactaacgtaagcgttttacgcaattccacgcgagaggtgtttggagtaacgttatgcgacatggtcattctcctttacggtgataaccgtcgcgtaagcaaaaaattgccccatttttttggattcctcagcgacaacaactgtcgatttttagtaaatatctatccggtacgaagcccggcctcttggtatgaatgattggtttgaagcaaaaaataaccgacgctgatgaaacgtcggtttttagtcattttttgacagcggcgcattgtgcctaaatgggggggaaatgacaagagaatgagaggcttgtcagaataatttttctttaaatggctgattttccgtcatcagattttgcataaacaccggcgatcgcactatttgctaaaatttcatcccgccaccagccactggcaagtcctgcggtctgttcgttccagccaatccagacgggttcaaagagagtttgggcgaccactttcttctcgattaacgcgccactatcgagaaaacgttgcgccagataacggggtaaatagccgcagccgaggccgctaatttgcagctccagtttggttttaaaatcgaaaacggtaatggcttcttgttcgtcgagaagttgtgatgccgtagaagcgcctgcctgcgcagtatcccccaccacaatcgcccgatatcgcttaataatacgacgatttaacggctcttcttccagggctaacggatgatgaggcgcgaccgcaaagacttgttccagatcgcccaaccgtgaaaaaccaaactcactggaagatggtggctcatgcatcgcgccaacaataatatccgctcgcccctgagtcagggcatcccatgaaccaccgagtacgccattgataaacttcaggcgcgtcacgctatgatgttgataaaaagcttcaatgagtggcgcaagcagagaaaaaggaaacgtgtcgtccacgccaatcaccagctcgttttcccagccttcatgcagtttgatcgcctgcttttccagttcccgcacggtatgcagaacttcccgccctttctctaataacatttttccggtgcgggtgaatttagcgcggtgtccgctacgatcaagcaattgaatattaaggtcgctttccagcttgtgaacggtgtaactcagagcggacggcgtcttgtagagtttggccgacgccgccgcaaaactgccttctttttctaaggcatcgaggatcatcaacacatccagcagtggtttcatacacgcccccttgcagtgcatgcggcgtcctgctggcgtgatcgtttactccagcggcattaccagcggatcgggatactggtattcaaatcccagttcattacaaatccgactgccatcaataatcttacctttgccgctgtccagactatttctgaactgcggaggttccagccccagtaaacgggccatctgcggatagaaaacattacgcgcagggtgagctggcgcacatatattatagatgtgtccgcctttaggtgcctgtaacaacagagtgatagcgccaataacatcttctaaatggactaaattaacaccatgttcaccatcaggcgcggtttttccggcaaagaagcgtccgggatgacgtcccggtccgaccaggcccgcaagacgcagaatatcgaccgaagtaccgggtaaattgtgcagccagtcttcgagttcttctaatactcgtccactgttggttactggattacgcggggtggtttctttcaccgtgccttgcgcgtcgccatagacagatgttgagctggtaaaaataatgcggggaatacgatgggccagcgcgctatccactaactcttgtaccgcttgtaaatagaactcatcgccggggccgctacgacgtgccggaagcgtaatgaccagcgcatcggcatccatcagggcatccagatcgtcagaatcgcaaactagctcaggctccatgcgaagcagatagctatcaatgccactcattcgggccgcttcgacaccatcttgtgtggttttactcccggtgacttgccagcctcgcgctgaaagtgacatcgccagcggcatgcctaaccaccctaacccgacaattgcgacctttttcatccgttatctcctgatacaccttagatctataaggctacgctagcgtatcaaaactgacaattcattctatgaatgaatctgttcaataatgataacgacatgctgcaatgagcagtgaatcgtcggtaaccgcgtataccagacggtgctcctctgtaatgcgtcgggaccagaaacctgacaaattatgtttcaggggttctggcttccccttaccttcaaatggcgttctgcgggtatctttgataagttcattgatctttttaacaattcgcttatctgtttcctgccagtacagataatcgtcccatgattcctcagaccagattagtttcactcaatgatgtccttttccgttcctttgcctgatttcaggctatcgattgagtccatcaatctccgggcgttagcgggggagcgcagtagataagccgtctcttccagcgagttgtattcttcgagtgacatcagaacacaagcctctccattctgacgagtaataaggatcggggcatgatcttcaacggctttcatcattgttgccgacaaattctgacgcgcttcgctgtagctaattgtacgcatgtcaatctcctcttttgtacagttcattgtacaatgatgagcgttaattaactatttattaattagtttgtagatcaaggtattgtcagtgagacgaaaatccaggcttcgctatttttggtgccatcagctaagaggacagtcctcttagccccctcctttccccgctcattcattaaacaaatccattgccataaaatatataaaaaagcccttgctttctaacgtgaaagtggtttaggttaaaagacatcagttgaataaacattcacagagacttttatgacacgcgttcaatttaaacaccaccatcatcaccatcatcctgactagtctttcaggcgatgtgtgctggaagacattcagatcttccagtggtgcatgaacgcatgagaaagcccccggaagatcaccttccgggggcttttttattgcgcggttgataacggttcagacaggtttaaagaggaataacaaaatgacagacaacactcgtttacgcatagctatgcagaaatccggccgtttaagtgatgactcacgcgaattgctggcgcgctgtggcattaaaattaatcttcacacccagcgcctgatcgcgatggcagaaaacatgccgattgatattctgcgcgtgcgtgacgacgacattcccggtctggtaatggatggcgtggtagaccttgggattatcggcgaaaacgtgctggaagaagagctgcttaaccgccgcgcccagggtgaagatccacgctactttaccctgcgtcgtctggatttcggcggctgtcgtctttcgctggcaacgccggttgatgaagcctgggacggtccgctctccttaaacggtaaacgtatcgccacctcttatcctcacctgctcaagcgttatctcgaccagaaaggcatctcttttaaatcctgcttactgaacggttctgttgaagtcgccccgcgtgccggactggcggatgcgatttgcgatctggtttccaccggtgccacgctggaagctaacggcctgcgcgaagtcgaagttatctatcgctcgaaagcctgcctgattcaacgcgatggcgaaatggaagaatccaaacagcaactgatcgacaaactgctgacccgtattcagggtgtgatccaggcgcgcgaatcaaaatacatcatgatgcacgcaccgaccgaacgtctggatgaagtcatcgccctgctgccaggtgccgaacgcccaactattctgccgctggcgggtgaccaacagcgcgtagcgatgcacatggtcagcagcgaaaccctgttctgggaaaccatggaaaaactgaaagcgctgggtgccagttcaattctggtcctgccgattgagaagatgatggagtgatcgccatgagctttaacacaatcattgactggaatagctgtactgcggagcaacaacgccagctgttaatgcgcccggcgatttccgcctctgaaagcattacccgcactgttaacgatattctcgataacgtgaaagcacgcggcgatgaggccctgcgggaatacagcgcgaagtttgataaaaccacggttaccgcgctgaaggtgtctgcagaggagatcgccgccgccagcgaacgcctgagcgacgagctaaaacaggcgatggcggtggcagtaaagaatattgaaaccttccacactgcgcaaaaactgccgccggtagatgtagaaacgcagccaggcgtgcgttgccagcaggtcacgcgtccggtagcttcagttgggttgtatattcctggcggctccgccccgctcttctcaacggtattaatgctggcgactccggcgagtattgcgggctgtaaaaaagtggtgctgtgctcaccgccgccgattgccgatgagatcctttatgcggcgcagctgtgcggtgtgcaggacgtgtttaacgtcggcggcgcacaggccattgccgcactggcgtttggtacggaatctgtgccaaaagtggacaaaatcttcgggccgggtaacgcctttgtcaccgaagcgaaacgtcaggtgagccagcgtctggacggtgcggcgatcgatatgcccgcaggcccgtcggaagtgctggtgattgctgacagcggcgctacgccggatttcgtggcttctgatttgctctctcaggctgaacacggcccggactcacaggtgattttactgacgcccgctgctgatatggcgcgtcgcgttgccgaggccgtcgaacgccaactggcagaactgccgcgtgccgaaaccgcccgccaggcactgaacgccagccgcctgatcgtgactaaagatttagcgcagtgcgtggagatctccaaccagtacggcccggagcacctgatcattcagacccgcaacgcccgtgaactggtcgatagcatcaccagcgccggttcggtatttcttggtgactggtcaccggaatcggcaggtgattacgcctccggcaccaaccacgttctaccgacttacggttacaccgccacctgttccagcctcgggctggcagatttccagaagcgcatgaccgtacaggaactgtcgaaagaggggttctccgcgctggcttcaaccatagaaacactggccgccgccgagcgcctgaccgcccacaaaaatgccgttactttgcgtgttaacgcccttaaggagcaagcatgagcaccgtgactattaccgatttagcgcgtgaaaacgtccgcaacctgacgccgtatcagtcggcgcgtcgtctgggcggtaacggcgatgtctggctgaacgccaacgaataccccactgccgtggagtttcagcttactcagcaaacgctcaaccgctacccggaatgccagccgaaagcggtgattgaaaattacgcgcaatatgcaggcgtaaaaccggagcaggtgctggtcagccgtggcgcggacgaaggtattgaactgctgattcgcgctttttgcgaaccgggtaaagacgccatcctctactgcccgccaacgtacggcatgtacagcgtcagcgccgaaacgattggcgtcgagtgccgcacagtgccgacgctggacaactggcaactggacttacagggcatttccgacaagctggacggcgtaaaagtggtttatgtttgcagccccaataacccgaccgggcaactgatcaatccgcaggattttcgcaccctgctggagttaacccgcggtaaggcgattgtggttgccgatgaagcctatatcgagttttgcccgcaggcatcgctggctggctggctggcggaatatccgcacctggctattttacgcacactgtcgaaagcttttgctctggcggggcttcgttgcggatttacgctggcaaacgaagaagtcatcaacctgctgatgaaagtgatcgccccctacccgctctcgacgccggttgccgacattgcggcccaggcgttaagcccacagggaatcgtcgccatgcgcgaacgggtagcgcaaattattgcagaacgcgaatacctgattgccgcactgaaagagatcccctgcgtagagcaggttttcgactctgaaaccaactacattctggcgcgctttaaagcctccagtgcggtgtttaaatctttgtgggatcagggcattatcttacgtgatcagaataaacaaccctctttaagcggctgcctgcgaattaccgtcggaacccgtgaagaaagccagcgcgtcattgacgccttacgtgcggagcaagtttgatgagtcagaagtatctttttatcgatcgcgatggaaccctgattagcgaaccgccgagtgattttcaggtggaccgttttgataaactcgcctttgaaccgggcgtgatcccggaactgctgaagctgcaaaaagcgggctacaagctggtgatgatcactaatcaggatggtcttggaacacaaagtttcccacaggcggatttcgatggcccgcacaacctgatgatgcagatcttcacctcgcaaggcgtacagtttgatgaagtgctgatttgtccgcacctgcccgccgatgagtgcgactgccgtaagccgaaagtaaaactggtggaacgttatctggctgagcaagcgatggatcgcgctaacagttatgtgattggcgatcgcgcgaccgacattcaactggcggaaaacatgggcattactggtttacgctacgaccgcgaaaccctgaactggccaatgattggcgagcaactcaccagacgtgaccgttacgctcacgtagtgcgtaataccaaagagacgcagattgacgttcaggtgtggctggatcgtgaaggtggcagcaagattaacaccggcgttggcttctttgatcatatgctggatcagatcgctacccacggcggtttccgcatggaaatcaacgtcaaaggcgacctctatatcgacgatcaccacaccgtcgaagataccggcctggcgctgggcgaagcgctaaaaatcgccctcggagacaaacgcggtatttgccgctttggttttgtgctaccgatggacgaatgccttgcccgctgcgcgctggatatctctggtcgcccgcacctggaatataaagccgagtttacctaccagcgcgtgggcgatctcagcaccgaaatgatcgagcacttcttccgttcgctctcatacaccatgggcgtgacgctacacctgaaaaccaaaggtaaaaacgatcatcaccgtgtagagagtctgttcaaagcctttggtcgcaccctgcgccaggccatccgcgtggaaggcgataccctgccctcgtcgaaaggagtgctgtaatgaacgtggtgatccttgataccggctgcgccaacctgaactcggtgaagtctgccattgcgcgtcacggttatgaacccaaagtcagccgtgacccggacgtcgtgttgctggccgataaactgtttttacccggcgttggcactgcgcaagcggcgatggatcaggtacgtgagcgcgagctgtttgatctcatcaaagcctgtacccaaccggtgctgggcatctgcttagggatgcaactgctggggcggcgcagcgaagagagcaacggcgtcgacttgctgggcatcatcgacgaagacgtgccgaaaatgaccgactttggtctgccactgccacatatgggctggaaccgcgtttacccgcaggcaggcaaccgcctgtttcaggggattgaagacggcgcgtacttttactttgttcacagctacgcaatgccggtcaatccgtggaccatcgcccagtgtaattacggcgaaccgttcaccgcggcggtacaaaaagataacttctacggcgtgcagttccacccggagcgttctggtgccgctggtgctaagttgctgaaaaacttcctggagatgtgatgattattccggcattagatttaatcgacggcactgtggtgcgtctccatcagggcgattacggcaaacagcgcgattacggtaacgacccgctgccgcgattgcaggattacgccgcgcagggtgccgaagtgctgcacctggtggatctgaccggggcaaaagatccggctaaacgtcaaatcccgctgattaaaaccctggtcgcgggcgttaacgttccggtgcaggttggcggcggcgtgcgtagcgaagaagatgtggcggcgttactggaagcgggcgttgcgcgcgtagtggtcggctccaccgcggtgaaatcacaagatatggtgaaaggctggtttgaacgcttcggtgccgatgccttagtgctggcgctggatgtccgtattgacgagcaaggcaacaagcaggtggcagtcagcggctggcaagagaactcgggcgtttcactggaacaactggtggaaacctatctgcccgtcggcctgaaacatgtgctgtgtaccgatatctcgcgcgacggcacgctggcaggctctaacgtctctttatatgaagaagtgtgcgccagatatccgcaggtggcatttcagtcctccggcggtattggcgacattgatgatgtggcggccctgcgtggcactggtgtgcgcggcgtaatagttggtcgggcattactggaaggtaaattcaccgtgaaggaggccatcgcatgctggcaaaacgcataatcccatgtctcgacgttcgtgatggtcaggtggtgaaaggcgtacagtttcgcaaccatgaaatcattggcgatatcgtgccgctggcaaaacgctacgctgaagaaggcgctgacgaactggtgttctacgatatcaccgcttccagcgatggccgtgtggtagataaaagctgggtatctcgcgtggcggaagtgatcgacattccgttttgtgtggcgggtgggattaagtctctggaagatgccgcgaaaattctttcctttggcgcggataaaatttccatcaactctcctgcgctggcagacccaacattaattactcgcctggccgatcgctttggcgtgcagtgtattgtggtcggtattgatacctggtacgacgccgaaaccggtaaatatcatgtgaatcaatataccggcgatgaaagccgcacccgcgtcactcaatgggaaacgctcgactgggtacaggaagtgcaaaaacgcggtgccggagaaatcgtcctcaatatgatgaatcaggacggcgtgcgtaacggttacgacctcgaacaactgaaaaaagtgcgtgaagtttgccacgtcccgctgattgcctccggtggcgcgggcaccatggaacacttcctcgaagccttccgcgatgccgacgttgacggcgcgctggcagcttccgtattccacaaacaaataatcaatattggtgaattaaaagcgtacctggcaacacagggcgtggagatcaggatatgttaacagaacaacaacgtcgcgaactggactgggaaaaaaccgacggacttatgccggtgattgtgcaacacgcggtatccggcgaagtgctaatgctgggctatatgaacccggaagccttagacaaaaccctcgaaagcggcaaagtcaccttcttctcgcgcactaaacagcgactgtggaccaaaggcgaaacgtcgggcaatttcctcaacgtagtgagtattgccccggactgcgacaacgacacgttactggtgctggcgaatcccatcggcccgacctgccacaaaggcaccagcagttgcttcggcgacaccgctcaccagtggctgttcctgtatcaactggaacaactgctcgccgagcgcaaatctgccgatccggaaacctcctacaccgccaaactgtatgccagcggcaccaaacgcattgcgcagaaagtgggtgaagaaggcgtggaaaccgcgctggcagcaacggtacatgaccgctttgagctgaccaacgaggcgtctgatttgatgtatcacctgctggtgttgttgcaggatcaggggctggatttaacgacggtaattgagaacctgcgtaaacggcatcagtgagttgcggggtaagcggatgcgatattgttgccgcatccggcaaaaaaacgggcaaggtgtcaccaccctgccctttttctttaaaaccgaaaagattacttcgcgttgtaattgcgtagagcattacgccccagcacaatccccgcgccaaccatgccacccagcagcaccgccagaatcaaggtaattgcctttttcgggctatcacgacgaataggtaacatcggtttcatcacataacggtaagcatgaatatcaagatcatcaacttttaagctttcgatatccagcaggttttgacgagtctgatagtagtttggcgagaacaccaacggacgggtcgcctcatgcttaatcatcgactccagcgcttcgctccccaaaaggaacaacgtatcttgtgtgatatcttcgccagtctgttgaatctgcggttttgtcacctgcgcctgattcgcatactgcaacgcttcctgaatctgacggatacgcagatctttctgctcctgcgcgactacttcctgcgttcttaaagagtcctgcaagtttttccgtcccagagcaatgttgtctttgagatccttttctagctcttgattcactttatcgtcaacttgctgaatgtattgggccaacttcatttgtgcgccctctgcagtttgcccaacataagaaacagtcaatggtaattgctggttcttaacagaaggttcgatggtaagtttttctcgttcttcctgattatccagcgtttctgctaatgcagagaaggcagaactgaagcgaccaattaacgtctcctgcaaatccgatactttcggtgcagcctgaccatagataacattcatggcattgttatagccagcaatttgccccacgtcgggctgagtgataattgctgttgacgtccatttctccttcgctactgccaaatatccaatagccagggcaatagccacaatgacggaaatgatgattgtcatcttgccacgccacaactgcactagtaaatcaatcaaatcaatctgttccgggtcatggttttgcccagaaacattattattttctactctcatcattaccctaactgacggaaatttccaagtccgcatagtttagcgataatcctcgtgaatgctataggataagtgataaaaataatgaattgttgtgtaagtaacaaaagacaatcagggcgtaaatagccctgataacaagatgttagtcgctgccaaagagatcgcgggtgtataccttatctgccacatccttaagctcttctgccattcggttagagataatgacgtcggcttgttgtttgaaggtggcgagatcacgttccaggcgagagttgaagaatgagtcttctttcatcactggctcgtagatgatcacttcaacacctttcgccttgatacgtttcataatcccctgaatagaagacgcacggaagttatctgaaccgctcttcataatcagacgataaatacccaccacttgcggcttgcgtgacaaaatggcatcggcaataaaatctttacgcgtgcggttagcatcgacaattgccgagatcaggttattcggcacagactggtagttcgccagtaactgcttggtatctttcggcagacaataaccaccataaccaaacgacggattgttgtaatggttgccaatacgtgggtcgagacaaacgccttcgattatttgacgggaattcagacctaaactttctgcatagctatccagttcgttaaagtacgccacgcgcatcgccaggtaggtgtttgcaaaaagtttaatcgcttctgcttcagtggagtcggtaaacagcatcgggatattttgcttaatcgcgccttcctgtaacagagcagcgaaacgttctgcgcgttctgaacgctcaccgatgacaatacgtgaaggatggagattatcgtaaagggctttaccctcacggagaaattccggggagaatataatattttcagtgcgatatttcttatgcatcgctgcggtaaaaccaacgggaaccgttgatttgatgaccataaccgcataaggatttatctcaactacgtctttaattactgattctacactggatgtattgaaataattagttttaggatcatagtcggttggagtggcgatgatgacataatcagcatcccggtaggcttcatttttatctaatgtggcattaaagtgtattttatctgattgcaaaaactgctgaatttccttatcaacaataggagatatccgatcattcagcatagcaacgcgtgacggtaaaatatctaatgccacaacctcatgattttgtgcgattagaagcccgtttgacaagcctacatagccagtaccggaaatggtgattttcatttcatgctctcagaattaacttaactgtgaatcatgatgtttttagcatcctgataagagctaaaagttttaacgctacgttgttcgatggtcaacgcaacgaaaaacaattcagattttctttataagaatagctgatatttattaagttaatattaagcagtgaaatttagtctataagatatttggcaaaaaaaagcccggtgcaatatacgccgggcctcaattttattgttggttaaatcagattaatccagccattcggtatggaacacaccttctttatcaatacgcttataagtatgcgcaccaaaatagtcacgctgtgcctggatcaggttcgcaggcagaacagcagcacggtagctgtcgtaataggcaaccgctgcggagaaggtcggaaccggaataccgttctgtactgcataagcaacgacatcacgcagcgcctgctggtagtcatcggcaatttgcttgaagtacggagccagcaacaggttagcgatctgtggattttcggcataagcatcggtgattttctgcaggaactgcgcacggatgatgcagccagcacggaaaatcttcgcgatttcgccgtagttcagatcccagttgtactcttcagacgcagcacgcagctgagagaagccctgggcgtaagaaacgattttgcccagatacagcgcacgacgaactttttcgatgaactcagccttgtcgcctgctggctgtgcttgcggaccagagagaactttagatgcggcaacacgctgatctttcagagaagagatataacgtgcaaacacagactcggtaatcagcgacagcggttcgccgagatccagcgcgctctggctggtccatttaccggtacctttgttagccgcttcatccaggatcacatcaaccaggtagttaccgtcttcatcttttttggtgaagatatctttggtgatgtcgatcaggtaactgctcagttcaccgttattccactcggtaaaggtctgcgccagttcttcgttggtgaggttcaggccacctttaagcagagaataggcttcagcaatcagctgcatatcgccgtattcaataccgttgtgaaccatcttcacatagtgacctgcgccatcggcaccaatataggtaacgcatggttcaccgtcttcagctacggcggcgattttggtcaggatcggtgctaccaattcataggcttctttctggccaccaggcataatagaaggacctttcagcgccccctcttcaccgccagaaacaccggtaccgatgaagttaaagccctctgctgaaagctcacgattacgacgaatagtgtcctggaagaaggtgttaccaccatcaatgatgatgtctcctttatcgagatatggtttgagggaatcaatagcagcatccgtgcctgcacctgctttcaccattaacaggatgcgacgaggcgtttccagagattcgacaaactctttcaccgtatagtaaggaaccagtttcttgcctggattttcggcaatcacttcttccgtcttctcacgggaacggttgaaaatagagacggtataaccacggctttcgatgttgagcgcaaggttgcgtcccatcactgccataccgactacgccgatctgttgcttggacattacatactcctgtcaggtgtgatcaccgcgctgaatgctcgcggcctggaatgttcgcaaataagtatacaaagtacttattaaagtataaatagcttatccatgcttatatgcttacggctttatattacgggtgaaaaactgatgaaattcgatcaaagttgcgatttgataaaatacgttttctggctaaatatctaaaagtactttttaagtgccatctgaaggcttttgaaaaaaaacttcgattgtcatgatgagcataatgtatcgcatgaaaagcgggaacataatgaagtctgacaccagccaggctaagcctcaagcacaggtcaatatcttcacagtacataaagtaaccttgatcgaagccatttacacgcacaaaatctgaaaaacgtaccagcataaatgatcctgcgcaccaatcaacaaccgtatcagaatagatactttctttaggaatttttgttttattaaggaaggtgcgaataagcggggaaattcttctcggctgactcagtcatttcatttcttcatgtttgagccgattttttctcccgtaaatgccttgaatcagcctatttagaccgtttcttcgccatttaaggcgttatccccagtttttagtgagatctctcccactgacgtatcatttggtccgcccgaaacaggttggccagcgtgaataacatcgccagttggttatcgtttttcagcaaccccttgtatctggctttcacgaagccgaactgtcgcttgatgatgcgaaatgggtgctccaccctggcccggatgctggctttcatgtattcgatgttgatggccgttttgttcttgcgtggatgctgtttcaaggttcttaccttgccggggcgctcggcgatcagccagtccacatccacctcggccagctcctcgcgctgtggcgccccttggtagccggcatcggctgagacaaattgctcctctccatgcagcagattacccagctgattgaggtcatgctcgttggccgcggtggtgaccaggctgtgggtcaggccactcttggcatcgacaccaatgtgggccttcatgccaaagtgccactgattgcctttcttggtctgatgcatctccggatcgcgttgctgctctttgttcttggtcgagctgggtgcctcaatgatggtggcatcgaccaaggtgccttgagtcatcatgacgcctgcttcggccagccagcgattgatggtcttgaacaattggcgggccagttgatgctgctccagcaggtggcggaaattcatgatggtggtgcggtccggcaaggcgctatccagggataaccgggcaaacagacgcatggaggcgatttcgtacagagcatcttccatcgcgccatcgctcaggttgtaccaatgctgcatgcagtgaatgcgtagcatggtttccagcggataaggtcgccggccattaccagccttggggtaaaacggctcgatgacttccaccatgttttgccatggcagaatctgctccatgcgggacaagaaaatctcttttctggtctgacggcgcttactgctgaattcactgtcggcgaaggtaagttgatgactcatgatgaaccctgttctatggctccagatgacaaacatgatctcatatcagggacttgttcgcaccttccttaatccctaacataaatgacacaataaaatcagaaagcacaggaaattttcttacggaataatcatgtaaagatttcgcttcatctcggaacaggcataatgtactaaaagcataacgcttactttcgacatatttaatatatgtcagcaaatcatcatgcttcatgatgatatcgggattcaaaaacaaaatgtaatcatcatctgcgggtctatatttttcctttacatacgccaccgcaatattattattatgaccaaagccgtatacacctccactaatatagtccaggcctgcataatgctggcatatttgtttcaataatagagagtctttgttgtcgcgtacgataatcttgtagtgctcatcgtcagcattaagattttcgagtaattttttgatgtagtcttcatgtccgtgggaaacgattattatatataccatttcaatgttcttcagtaataaaattaactagttcatcaaacccaactaatacattttcattacgataaatgaaatttgcatcagagatatcttttttgaggttaccttttttgaagtcaataataagtttaactaacatgtcatcgttattagaatcaaaaaaagctttcttttcataactaccaagagtttctctagtaaatgggaaatctgatgctaatacccacttacctcgctctttagcttcagacaacggcaatccccatgtttctaacctagagggaaaacaaactatatctgaaatattataacaatgatcgattttttctttatccaagtacccgaggaaatgaacattatccagtccttctgcaagactgataatatattttgcatacgcattttctgtaccactgatagtaagcagaaatttaatattggattgttctttcaatttccttgctgcactaataataagctcgtaatttttaaatactcgtggaacagcagggtaaaatattgtcaactcagaagggttattcttaaattgagaatcatcatcagtaagttggcttttatcagataatttaatttctggccgactgacaatgatgttatttatagaatatttcttgataaatttttctttcatccagaattgttgaacaaacactgcagtattttttttaatgtttattttatatatcagcccgtatagcattttaaataagaaaaagctaggctccataagaatttcacggaataaaattcctttataaaaaggtgcagggttatgacaatacacatatctttttttagtgacgacattggccgtaatatcatgcagacaaatccaatgcgtagcattcagctcttttgaaagttttttacaaactacatattcaaagtgcaaacgttttagccacgaccctttaacctcaggaaactcaatgaatttaacccatggataactttcttttaactctttagcagaatggactaatgcgataaaactgacattttctttattattagttgctgccaaaaattttttcaaaatggtaaatggaccgccagtggtaaaattgaccgcagaaacaacgactatgctttttcccataatttggtctcatgattgtatttctttatgatttttgctggtactcccgcaatgacagtattttcgggaatagaacctctaacaacagaattggcgccgactacgactccattaccaataattgttccaggcaaaaccgtcacattctcacccaaccaaaccctctggccaattacaacagctgaagattccaacgtgcgcatgtctggaggtatatttggcgaactcattggatcagagtgcttaaaggaaccgtgattatgatcggtaataaatactttacttgcaataagcgtatcccgacctatcgtaacgctctcaattgaggcgatatgaacatagtcgttaacttgcacattatcggaaaaaaaaatcacgccacgtccaaatgcatccagcctgagaccgactccacttgtgaaattttcaccaaaattaatgctaccatcattgcgaatatagcagggaaatcgaataattctacagttccggtaaaatacacgagtcaataagacatctctaacaagccgaataaaaccacagagaccatatcgtttagcgagttttaagatcatcgatcacctcttcaagaacatccctgaagtaacttcctgttcgaattttctgagaaataatttttgtattctcactaatttgcttataagtttctattgtcatggagtcaacaatctcttgcatttctttgattgatcccactgcatatcctattctattatctacaatgaaatccgcaagggcggctttatcccatataaatactggaagttccattgaaagataaagagatgtcttatgagggttattaaactttaaatagtcgccaaaggcaccactacaggtttcgacagaatctccatcccaaatgagtccaaattgcatgcctgggaggttaatcttttccggagattgagcatcaaaacttccaagatatttaggattatctttattttcatagttgacaccaaagagagtaaaatcgcatccttcagtatatatgaaagaacatttatgcctagaaaggttgccagcatatatgacccctcgttgcttatccgtaacatctcgatgctccacatcagatgagacgaggtaatcaaatatttttatgtctttgattttatcctgagacatatatttactaaggtactttgtcatttgtggattgtgacttatgaccatatcacaggtagcaagccgcacagaatcactaccccctcctcctcttaattcatcaatatcatgaatcagaggtactattctaaattttagaaggcggtgaaagaatgacaatatatgccaaaatggtttggccatcgggaaattgaaaattaaaacatctttattttcaagaccgcagagaaatgtactaagcttaacagaactaataattctctggactactccaccccatagaggaatgttaacaacagaaatgttttcataatctgaagcaatgtccagtgcatcttttcttgctttaaatccagcatcgcgtctagagaaatttaaatcattcaaaaaatacattttcactttattttctgggccttaagaaattgagagaatactatgatacaaagagttatttgtatccaactgctaatattagtcatgaagctttcatgataaaaaatgaaagaaaaggtataaataaaatatgaataaaatattttcacagatatgtaatttcgagacaatctccataaaacacctgaaatacagccatgaataaccatcatcaaatagcttagctccgcggaaatataaacataatccgaaaaagcagtataaacatttgttggcaaacccacccacacaaattctttatgcaacgacatagagactccacctgttaatagccccatcagcctttcaaaaaaccaaaagacatgagaactggcagagttagatacttgctgaaaataaaactcctgaaacgcgattatagggctgaccaaatacatggatagataatatgccatccccccaggcagtccacgtaaaaagagcatatacaaggagaatagaacacctacagctgtaataagataaacataatgttttactctattaacacctacgatgaatgcataagagatgataaccataaagacaatttgcttaccagtattcagtataattgcaaagatgaatacaataaaaacaagtaaagtaaatgttttacttacctttgtattagtaaattttttagaccaaataaataaagcaaaagtagttagaatgattggctgcatgtatgctgagaaatttcttgatgtgtcttcaacatcagcatctcttatcaaattcatatagctaagtaagctagtcccgaactggtagttacttaacctcatgcatatatatatcatcgaaaaagaaataactaacaagcctacattatgcactttcttcgatggtatgctataaatagcattattgacttttctgatatttagatctaatacactttccgtcaataaacatgacagggtaaatgtcaaaacattgcaaagtagaaaaatcaacgtagcgtcatttaactgaaaagcatatatatctgacgttatttcatatcccaataagaccagtgcgaagatgatattaacgcatacggctggataaaatatatccttcttaagatataaacagataaatgctgtaatgagaaagacactaattacaagatagatcattaatccgtactcattatatttttcacttgataaagagcggcagatatcacttgatgcatatcataatatttatactcggccaaacgcccgccaaatataaccttgtcttctctgctagctaactctctatatttcttaaaaagctccatgtttttattatcattaactggatagtagggttcgtcgccaactttccactctaatggatattcttttgtaacaaccgtatgctttgtctcaacatagtcaaaatgtttatgctcaattattctggtatatggtacattagcatcagtgaaatttattactgcattcccttggaagtttggaaattcatggcgttccgtctcaaattttaaagagcgatattctaacgctccaaacctatagtcgaagtactgatcaatgggtccagtgtagatgattctatgggctttactcgctagagaatctttgtctttcaaaaaatcaatgcctaattttacgtccacaccttcaagcattttttcaataagcttagtgtagcctcccaccggaataccttgatagcgatcggaaaaataattgttatcaaacgtaaatctcactgggattcgcttaataataaatgcaggcaattcttttgcacttcttccccactgcttctccgtataaccctttatcaatgcttggtataagtcctccccaactaatgaaatcgcctgctcctccaaattttcaggtaccttgtcaccatacttttttttctgagcattaatgatattttgagcttcttgaggatctttaactccccacatttggtggaaagtattcatattaaaaggaaggttgaataatttgtctttataaatcgccagtggagaattagtaaaacgattaaattctactaaatcattaacgtaatcccatatatatttatcattggtatgaaaaatatgtgcaccatatttatgaatctggataccctcacagtcctctgtgtacgcatttccaccgatatgatttcttttctcaatcactaaaacttttttgtttagcttttttaactcattcgcacaaacggcaccaaacaaaccagaaccaacaatgatataatcgtacataaaatcctcagcaaaccagtaatttattatttcttacgaacatcagcatgagtgacgtaactaagcactctgttgcaagcaatgttattgctgcaccaatctctttaaaaagagttgttagcggaaaaatcaacaacaaactcaacaaacccgcagcgattaaaatcttactgaattctttcttataattatgggtcagcataacttgaatgccatagacattacttaatgaaataagaaaaggcagaggcgatataatcattagcacaatcactgcattatcatatcccggccctatacttatttttactagtatagatgcacccaagagcagaattaatgaaaaagcaccaccaatcaaactcaagcaggtcaatgattttttaattaaaatcacacccttcacacgattaagaacaagcgtacttgatattcttgggtatattgcttgggtgataggatttaatagcccttgaagcgcgtttcttatagtattggccgcattaaaattccctacggacgttggtccagatataaatcccaggataataactattcccgtagaatataaactaatagcagatgtggaaataaaaacatgaaaaccgtctgctaaagatcgacgcacattatgtaatgatagcgtaactttaccaatccaaccttcatgaacaacgatagctagtgcaataattccagcaaccagatttgcacttgactgaataaaaccggcaattgctatatctgactttgtgttcacaaaaataaatgttagagggataatagccaagcgggataaaatactacttaaagtcagccatttcattttttcttttccctgaaacagccagatagggtagattaaattcccgactaatgcaggaacaaacgaccatataattacggcatgcttgttatattcaggaacaagcaaggtcatcgacgttaagaaaatcaatgtaatgacgataagaactatttttgaaaatatcaccgcccaaaaaatagacgttactttatctttactatctgctgctttggcaatactctgagttgctgtgagattgaaaccatattcaacaaacattatcatatatagcatagtcgcttggcaaaaaccgaatataccgaaattttcaggaccaagtgttcttacaagatatggaaatgtaagcaatggtaaaagataattgctaccttgaacgacagccagatatataacgtttcttcttaaagataatttattcgtattcatgcaattaattttaatctgataagctcatctaacgtaaagagcctttcatcttttggcgaaaggattaaccctgatgtttggggccaatcaattgcaatgcgttcatcattccaacatattccacaatcgctttcaggatgataatagtttgtagttttatattgaaattcagcgatatcagacagaaccaaaaagccatgagcaaacccttttggtatccacaactgctgcttattatcagctgaaagcagaacaccaacccatttaccaaaggataccgaattgggtcgaatatcaacagcaacatcaaaaactgctccatgagtgcagcgtacaagtttatcttgtgcgtactcgccgcgttgaaagtgaaggcctctgagtacattttttgatgaacgtgagtgattgtcttgaacaaagctgaccggatagcctagaatatgttcaaatgctgattgattaaagctctcataaaagaaacctctatcatcaccaaatactcttggctccagaattagcacatcttcaatttcagttctaatcacattcattaatttgaatccttcgtcattttataaagatactgcccataattattctttattagtggtacagctaattttcttacttgctcaacatcaataaaacctttacgaaatgcaatctcttcaggacaggaaaccttcaatccctggcgctcttcaattgtcgcaataaaattacttgcttctatcagactctgatgagtccccgtgtccagccacgcgtagccacgccccatcatcgcgacagacagacgtccctgctcaagataaatacggttaatatctgtaatttctaactcaccacgtgcagacggcttcaagtttttcgccatctgaaccacgtcgttatcataaaagtacagacctgtaacggcgtaattactctttggttctaacggtttttcttccagactgattgccgtaccgtttttatcaaactcaacgacaccatagcgttctggatcattaacgtgataggcaaataccgttgcaccactttctttgttaacagcggcctccattagcttcggcagatcgtgaccgtaaaagatattatcaccaagaaccaaagcacaatcatcaccaccaataaactcttcaccgatgataaatgcctgcgcgaggccatctgggctaggttgcactttgtactgaagattcaggccccactggctaccgtcacccagcaattgttgaaaacgaggagtatcctgaggtgtactgataatcaaaatatcgcgaatacccgccaacatcagtgtagagagcgggtaatagatcatcggtttatcataaataggtaatagctgtttactgacagccatagtcacaggataaagacgtgtaccagaaccacccgctaaaataatacctttacgcattttcatttcatcattccttttaattcatcttgctccaccatcacgaacaagatgcaaaaactattaaattgctgtagtcgtaaataattcattgagcattcgtttcacgccaacctgccagtcaggcaagacaagcgcaaagttctgctgaaatttttctgtattaaggcgagagttatgtggacgacgagctggtgtaggataggctgttgttggtactgcgttgagcttgttgagtgcaaggggaatgcctgctttgcgcgcctcttcaaaaaccagcgcagcataatcgtaccaggttgtggtaccactggctaccaaatggtacaagcctgcgacatccggtttattcagtgcgacacgaatggcatgtgctgtacaatcagccagcagttcagcacctgttggcgcaccaaactgatcgttaataaccgctaattcttcacgctcttttgccagacgtaacatcgttttggcgaagttatttccttttcctgcatagacccagctggtccggaaaataagatgcttcgcgcaatattcctgtaacgctttttctccggctaacttggtttcaccgtaaacatttagtggtgcggttgcatccgtctccagccatggcatatcgccatttccagggaagacgtaatcagtcgagtaatggataacccaggctccaacttcatttgctgctttcgcaatcgcttcgacacttgttgcgttaattaattgtgcaaactccggttctgattctgctttgtctactgcggtgtgagcggctgcattgacaataatatccggccgaatgcttcttacggtttcagctacaccttcaggattactaaaatcaccgcaataatcagtagagtgaacatcaaaagcaatcaaattacccaaaggtgccagagcacgctgtagttcccaacctacctgccctgttttgccaaaaaggaggatattcattactggcggccctcatagttctgttcaatccacgattgataggcaccacttttcacattatcaacccattttgtattggacaggtaccattccaccgttttacgaatcccgctctcaaacgtttcctgtggtttccatcccaatgcgcgaccaatcttctcagcatcaatagcatagcggcgatcgtgtcccggacgatcagcaacataagtgatttgctcacgataagatttctctttcggtacaatctcatccagcaaatcacaaatagtgagcactacatcgatgtttttcttttcgttgtgcccaccaatgttataagtttcacccgctttaccttcggttacgacggtatataacgcacgcgcatgatcttcaacatacaaccagtcgcggatctgatctcctttgccataaataggtaatgccttaccttccagtgcattaagaataaccagtggaataagcttttccgggaaatgataaggaccatagttgttcgagcaattagtcacaattgtcggtaaaccatatgtacgtttccacgcgcggactaaatgatcgctggatgctttggatgcggaataagggctgcttggcgcgtaagctgtcgtctcagtaaataagggtaattcttctgtattatttacttcatctggatgaggcaaatcaccatagacttcgtcagtagaaatatgatgaaaacggaagctatttttcttgtcgctatcaagagcagaccagtaattgcgagcggcttccaaaaggacataagtaccaacaatattggtttcaataaatgccgcagggcctgtaattgaacggtcaacatggctttcagcagccaggtgcatcactgcatccggctgatgctgagcaaaaatccgtgccattgcaggtgcatcgcaaatatccgcatgttcaaaaacatagcgttcagaatcagaaacatcagcaagtgattcccggtttccggcgtacgttaatttatcgacattaacaacactatcctgcgtattatttataatgtgacgaactacagctgaaccaataaatcctgcgccaccagtaacaagtattttcacttaatttattccatattacttcagagcatgctgtgaaataagcggctctcagtttgattaatagaggtattaatgcacgctaccgcccctggctttacagctaccagagcactgcatgcatgcctatgatgtgacgagcgttacccactcgcgctaaacccgaaaaattcaaacgctaattgtcttaccaatccgctctggaaacaaggaaaatcctggaaaactttgaataaaaccctactgctaactcgttgttattctgatggtttatataaaacaacggcaggaagattcgcaacaaattacttttgctgcgaattttcactgccgttataattttcttatcaaccgttacatccggtcagattttcattattcgcttaacagcttctcaatacctttacggaacttcgccccttctttcaggttgcgtaggccatacttcacaaacgcctgcatatagcccatttttttgccgcagtcgtaactgtcgccggtcatcagcattgcatcaacggattgttttttcgccagctcggcaatagcatcagtcagctgaatacgtccccatgcaccaggctgagtacgttccagttccggccaaatatcggcagaaagcacatagcgacctacggccatgatgtctgagtccagcgtctgcggctgatccggtttttcgataaattcaacaatgcggctgactttaccctcacggtccagcggctctttagtctggatgacggagtattcagagaggtcacccggcatacgttttgccagcacctggctgcggcccgtttcgttgaaacgtgcaatcatggcagcaaggttgtaacgtagcgggtcggcgctggcatcgtcgatcacaacgtctggcagtaccacgacaaatgggttgtcaccaatggcaggtcgcgcacacaaaatggagtggcctaaacctaaaggttcgccctgacgcacgttcataatggtcacgcccggcggacagatggactgtacttccgccagcagttgacgcttcacgcgctgctcaaggagtgattctaactcataagaggtgtcgaagtggttttcgaccgcgttcttggacgcgtgagttaccaggaggatttctttgatccctgcagccacaatctcgtcaacaatgtactgaatcattggcttgtcgacgattggtagcatctctttgggtatcgccttagtggcaggcaacatatgcatcccgagacccgctacaggaataactgcttttaaattcgtcattatttcatccacctgtaaaatggttgctgaattatagcttgttcgatttttttcgccagcatcaattaccctgaattgattactgaattacttgtgatgttacgccgcttcgttgtggattgcagtagcattgttcctaagtatgactccatttttccaggaatggtcgcaaatctactccctcagttccggcaatctaaagttaatcttctccacattaacaatatggtgattaatcctgtcgatatcgacggagctttgtcctttttcattcaccgcatgaacatttgcaagagacagcagtgtttcttttttcgccataaaaacaccacgaacgtctttgcgcatgtcaaagttcatgctcaatgcgggtccaactgaggattcctgcatcacattgatatttcgcataaaaaaatgttgcggtttgttgtgtaactccagcgacgcacgcttcatctcaatgttagttagcgccacaaaggaaacagcattcccggcggagatttgaatgccgcgcaatttataagcaagatgagtattatccagttgaatatcattcacccggaaattttgcggtatcgagagatatttgcctttaattaccccatagccgattaacatcccggcgctattaatcatttcaatattatcaatcacgaaattgtcacaaccgtaaatagcgactgtcgcgttatcaatgcccgctttcttactgaaatccggcgtgatattgcgggctttgatattacgaataacaaaatgtttaccattttcaacatgtatcaactgccgacaatccgatcccgtgatattcgccacgacaaagtttttcactgcctggtcttccgggtagttgttatcataagtgcttcccgcaaggcctatgccgatgccccagttgattttgccgttggtacagttgatgcgctcgatgacatggtcagatatcaaaatatcacggtcgttaattgccacgttccattcaatggcgtcgccttgtaagtcgctgaacttacaattggtgatgttggcaccgataatctggttatgaaatccctggcgtaagatggcgtaattagcgtggctaacggtcaggttatcgatgatcaggttgcgcatgacccgtttgtttttgccgccgatataaatctgcgtcaccgggccaaagccgctcatagtcagccctttgatggtgcagtcagaaccacgcacatccagggtgatgttatgcatactgccgccatcctcccctgtcacctggctgccgtcctgtaagacaaatcgccctctgccgttgccgcgcaagcttccaagaatgtgtaacgttttaccgggagggataaagatgccggtgttgatattgtcacaaaccaatccggcaggcacgacgactgtttgcccttcgctgaaggcttgtttaaatgaggcgatccagtcgtgtgggttgtagtcgttaatgttaacgctttgtcgggcgggaagcgcgcgggcgaaaggggtatggaggaaggcaagcgccgagcttgccgtcaggaacgtgcgtcgggagagttttttaaatggcatgcgttctcctctataaagcctgcagcaagctggcgagttctcgattgatcacctgctggttaaaatcgtgttcaactttttcgcgcgcgcgtttgacgaccggagccaattcgtcggtgtccagttggctaaacgccgccagtcgttgcgccagtgcgcgagcatcgttctcaggcaccagccagccggatttgtcagcctccaccagttccggtattccactatgcagagtagaaaccaccggaataccgaccgccatcgcttccattagcgccaccggaataccttccatatcaccatccgcacctgtaaccgatggcaacaggaagacatccgcgtcgtcgagcatcgctttcacttcatggctcggtttaaagcccggcatctccaccacatcttccagttgatattgttcgatgagggtgcgcaggcgtctttcccacgggccaatgccgaggatgcgatagcgaaatgccacgccctgctctttcaactgacggcaggcttcgatcgccacatgcaggccttttttctcggttaagcgtgcgacggaaataatctccagcggcgttgcgggcgctttcacgggacgcgggctaaagcgcgtcatatctacgcccatgcgcgatacggcgattttttccctcgggcagcccattttttgcagccttccggcccacagatcgcttatcggtaacatcaggtcgccacggcgaaacagttgctgatattcgggagtgtagtggttgagcacttcccgactggagatatcaataccgtggaagatagtggcaattttgccgcgaatgacacccagttcgcggagttttgctgcggttacccccgcgggaccaaaatgagcgatgaacacatcggcgcgaaacggtgttgcgacctggccgcaaatggcagacaaaatcaggttccgcgactcggcaccatagcgtttgaggttgagcgcctgccaggtatttttacgatgaatgccgcgcaaggtctggctggctcggtggcgcagtttcgccactttgcccgtaggttcgtcctgtaaccagcgggttctggcagcaaggttgtatttcgtccatgccgcgtgggtgttttgtgtgtcgcctttttgcagcgcgagaatctctacctcaaatcccatatcaataaacgcggtaatttggttaaggacgaaggtttctgacgacagcgggaatttcagtaaaaagaagccgaccttcatttcacctccccgatgcgctcaagcacagactgcaccatctgcattcctgtctgacgctcacgactgacggcttcactaagtcgcgcattcagcgccggaagctggcctaaggtatccgcaaccatcgcttgcaggctgccgtctaataaatgacggatatcaattgccatctccggtagtcccagctgctgcataatcccggcggatttatgttcgtagttgatggcaattgccggagtggcaaaattcatcgagataatggcagagtgcaggcgcgtaccgacggtgagttcacaggcccccagaattttgcccatttccagatcgttgagttcatccatcactacgtggtaacgggcaggatcgctgatgtgctggcgcaggttgagcgccaccatgcggtcgtctttgttatagctgtcaatgcccgtacaggtggagagcgcaatcacctgatacccttcatcgagaatgcgattgaccaccccggcaaaggctttttcatacgcttgttgagtggtgccgagacgtttgtcaaacggtgccagttcgcgcagggtaatggccaccgttttctgttgtgcggcaacgtccagccagtgttgaacggcatagctggcggtgaagtcttctgtgtggtgatcgaccagccacgcggtatcgacgccatgttccacttttgcggtggtgatattgctgcgtttcatcagatcaaagctgaccgattcgcgcaggatcagcgcgtcgcagtgaccaaaaacgtagttcgccagttggttaaattgctcatcctggaacgggccaacactgtgaccaatcataaacagcggctttttcgccataaacgtgcaaagtgcatgttcaaactgcggcacgccatagagatcgacaaaaaacgatccgccgacctggataatggcgtcgtaacctgacagcaggcgcacgaagtcggtgaatccctgggcgatggcgatattgcgcagcttgccagtgtcggtgacgcgtgagagcaatacctgatgctggtagcggcgacggaggacttttttaacgcgcccgacaacgcccgccgcgctgttgtgttgtttcatttgcaggaacagcggatcgcccattaccgggcggttgagcagccaggaagaactgaccggatagcggctcatcacatccacttcggcgtgtggattgagaatgttgatggcatcaagtaagccgcgcaggatggcgctgtcgccacgattgccgcaagtgtggttgcccagaataagtaatttcattttttcctcataaatttgatgccaggtgaggctgcgtttgttttgttcgttgccgctttttgcctgatgcgacgctgacgcgtcttatcaggcctacaagacccgagcacagaaccgtaggacggataaggcgttcacgccgcatccggcattcagtgcctgatgcgacgctgacgcgtcttatcaggcctacaggtcccgagcacagaaccgtaggacggataaggcgttttacgccgcatccggcaaccgttgtcggaaccgaaaacagcaactcaccccgcccgtaaaagcattttcattttttcgctgcgacaaaactgacgcttcacttccaccaccagcggatggcgcgacagcacaatcatcaccacaaacgccagcacccccgtggctatttgcaccgccagcagcatccccagcgccagttgccctttcagcacaatgcccagcgcataactgaccaccagcgtcggcagcgagagataaaacggcagccataaactcaggatgtactggcgataactggaaccaagaaccggtttaatcatcacgaagtaactcagaatggtgttgataatttgcaccagcaggaagccaagcgtgacgccgatcgcgcccgccatctgcccacctataacaatcgccggaataaacagaaatgttttgaatacgttgaatttaaagctgatatcgacccgcgctttcgccatcagcagcgaaccaatcgggttacctacggagcgcagcagacccaccacacacagcaattgcagcaccggaataatgctgttccacttctcaccaaagaccagcggtacaaagttattcgacaccaccattagcccgagcagcgccggaaagttgataatccccactaccgacagcagcttgtagaagttaacacgcagcttttcggtatcgtcctgaattttggcgaatgccggaaacaacacgcgggtgatgattgggttcagcttcatcggtggcacaacggccacgttgtacgccaggttgtatccccctgccacgcccgcgccgagaatacgcgccagcacgagcgttgaaaggttggtattgagatagttgatgatgctgtccgccgtcagccaggcaccaaagcgtaagttcggtgccaccgacgccagcgagaaatgcagaccggggcgataaattttgcggccaaagtagccaaacagcagcgttctcaccgcactattgaccagataaccgaggatcgcggtcatcgccagcggccagaaatgggcgctaaccaccgtacaagtgaagcccgccagcaccgcgctggtttcgatcatgccgattttgttgaactccagctctttttgcatcaacgcgcggaactgttgcccgtgggggattaccacaaacgccagcgataatgttttaatcaacggtgccaggtccgggttattcagcacgtcgccgatgagatcactcaacaaaaacaccgccacgcacaccacgatccccagcccgacgttcagccagtacaacgtggtgagttcaaggtgactgatttcttttcgctgaataatcgagttagcgataccgaagtcagaaagcgtatctgccagcgcgataatcaccagcgacacggtaagcaggccgaactggtggttgtcgataatccgcgccagcacggtcatctgcaccagcccgaggccgatgatgatcaccgtggcaatcgccgaccacttcgcgccgctgatggttttttcacgtaagctcatatcaatatgccgctttgttaacgaaacctttgaacaccgtcaggaaaacgattttgatatcgaaccagacgctccattcgcggatgtactcaaggtcgaactcgacgcgtttttccattttctccagcgtgtcggtttcgccgcgccagccgttaatctgcgcccagccggtaatgcccggtttcaccttatggcgcagcatgtagccttcaatgagctgtcgatactgttcgttatgcgctactgcgtgcggacgtggaccgacaatcgacatccccccggtcagcacattgataaactgcggcaattcatccagcgaggtacggcgcagaaagttccccactttggtgacgcgcggatcgttctgcgtcgcctgggtcaccactttgtcgttctccatcactttcatggaacggaacttccacactttgatcggcttgccatccatgccgtagcgagtctggcggaaaataaccggccctggtgaactgagtttcaccgccagcgcaatacagcacagcaccggggagatcagcagcagaataagcgtcgccagcacaatgtcttccgcacgtttgagcaggcggttaaccccggaaagcggcgtgtcgtaaagcggcaccaccggtacgccgttcatctcttcgaggcgtgaatggagaatgttgaaggtaaagacgtcggggatcagcagcaccgaacaggtggtgtccgccagttgatggaccagttttttcactcgcgcgccgtcgcacatttgcatcgcgatatagacgttatgaatcttgcccgctttcgcgtcctcgaccagctgttgcaggttacccgcccagtcgttagaaacgccgcccggtttcgggtcgtggtaaacgcccaccacttcaaaccctaaccacggctggttacggaagctctccatcagcatttgcccggcggctaaatcccccgccaccgcgaccatgcgcttgttatagccatgattacgcagccagcccgccccaatgcgaatacacgaacggcaaaccaccagtccgatgctggtcagcgcataccacgccagccagattttcagttgcgtgtcgaaatcattgttgaacgccaccagtccggcgctgaaaatcacgcttaaggtccagttttgtagcaacagggcaaattctgtcgctgcccgaacaccgcgccatgagcgataaaaatcggtgatgccgcccagcatctggaacaccaccagcgtaatcagcgccaccaacaggtgcatgtagaggaatgacagtccgctgacttcgcaaaccagccatagtccggcaaacatgatggtgatatctgaaaagcgttgcaccatagagattaacgatgcattggttttcgctcgctcgcgcttttttagatttgtcatcgttgttcctgttattagccccttacccgcagtggggtaagggaagatccgacattactcgttcagcaacgtcagcagagttcgcgttcgcgcttccatcagcggcacatcaccgcgcgattccacattcaggcgcaccaccggttcggtattggaggtgcgcaggttaaagcgccagtcggcaaaggtcatgctgatgccatcggtgcgatccaccgccagcgcctcacggctaaaatgctgttccacgcggttaatcgcctcaacgggttgcgccagtttgctgttgatctcaccgcttgccggaaacgccgccatccggtcgcgtaccagttcgcccagcgttttatctttcaggcacaccagttcggcgaccagcagccacgggatcatgccgctgtcgcagtaagcgaaatcacggaagtaatggtgggcgctcatttcgccaccatagatggcgtcttccttgcgcatacgttctttaataaaggcgtgtccggttttcgacattaccggcgtgccacctgcggcagtcaccacatcaacggtgttccaggagagacgtggatcgtggatgatcttcgcgccgggatttttttcgaggaatgcttctgccaacaggccgacaatgtagtagccctcaataaactgccctttttcgtcaaacaggaaacagcggtcaaaatcgccatcaaaagcaatgcccatatccgcgccgtgtttgatgaccgcattgcgggtgtcgtcgcggcattccggcagtagtgggttaggaataccgttggggaaattgccgtccggcgtgttgtgcactttgattaattccacgggcgcgccgagggctttaaagcgggcttcaatggcgtccaccaccggacccgctgcgccgttcccggagttgatcaccagcttgagcggcgtgaggtttttgacattgatataaccgaacaggtgatcaacgtaagcgtcacgcaggttgatttgctgatagcgaccgcgtttggtttcatcgacgggaggaaagtcgttggcttcagccagacgctggacgtcgcgcagtccggtatctccgctgatcgggcgagccccctcgcgaaccagcttcatgccgttataatccatcggattatggctggcggtaacttcaatgccgccatccacgccgagatggaacgtggcgaaatagatctcttcggtgccggacataccaatatccagcacgtcaacgcccgcatcctgtaaacctttcgccagcgccagttttaaggtttcgctggtgaggcggacatcaccgcctaacacaatggttttcggtttgagaaattcgccataggcgcgaccaatgcgccaggcgatatcttcattcagttcttcgcctaatttcccgcgaatatcataggctttaaagcaggttaattttttcatatcgttaccctttttcaggcaatagttggccctgaccgaagcggccaattttatttttgtcgttatttacaccgcggtttcgcattcattgcctgatgcgacgtttacacccgtccgtagcgatccgcgaaacgcaccacatcatcctcttcgagataagagccggagcgcacttcaattaaatcgagcggaattttccccgggttttccaggcaatgcgtcgcccccagcggaatataaatggactcgttttcaccaagcagtttgatatcaccatcaatggtgacttttgccgttcccgcgacaaccacccagtgttccgcgcggtgatggtgcatctgtaccgacaagccctcgcccggtttcacggtgatgcgtttcacctggtagcggtcgcccgcgtcgatagagtcatatttgccccacggacgatacacttcgcgatgcacccgatgctcatggcgaccatcggctttgatctgctcgaccacttttttcacatcctgtaccgcgttacggtcggcaatcagcaccgcatctttggtctgcaccactaccagatctttcaccccgacggtggtgaccaggccagattcagcatacacatagctgttttcagttttgtgattaatcacatcgccgtggcaaacgttgccctcggcggtgtgggcgctgatctcccataatgaagaccaggagccaacatcgctccagcccgcatccatcggcaccacaacagcatctgccgtacgttccatgaccgcgtaatccaccgactcttccgggcaggcgagaaacgcttcttcatccacgcgaataaaattgagatccggatcgacggcgctcatcgctttttcacaggcatcgaggatatccgggcgatattttttcagttcttcgagatagcgtccggcgcggaacaggaacataccgctgttccagtaatattcgccgcttgccacataggcctgagcggtttccagattcggtttttcgacaaactgcgccacttcaaaggccaccatatcctgctcacccgcagacacttcaccgcgacgaatatagccataaccggtttctggtagatccggcacaatgccgaaggtcaccagcttgcccgcttcggcatatggcatggcattacgcacggcggcacggaacgcgtcttcatcggcaatcacatgatccgccgccaataccagcattaacgggtcgctctccgggctatgacgttttgccgccagcgccgccagcgcaatggcaggtgccgtgtttcgccctgccggttcgagaataatgttctcggtaagtttgttcagttgacgcagctgttccgcgacaataaagcggtgctgctcattgcaaatcaccaccgggctttcgcactccacgccgttcaggcggcagatggtggtttgcagcatggtgagatcgcctttcaggcataaaaactgcttgggataaagtacgcgggaaagcggccataagcggctaccggagccacctgccatcacaactggatagagtttcgactgcgccataattatccccgaatatcatttataaattgacgtaacacgttctctttatcgagcgtgcgttcggcatattcacgtgccaccgtgttgtgtttgggcagcaggagcgcctgacggatccccgccaccagcgcctcgaccgattccggttcaacgcaaaccgcaatgcccggaaaggtttcgcaaagctgccccagttctgtgtaggcttcagcagtaatcaccgcgttaccgcctactgccagaatattggtcagtttcgacggcaatacggcatctgccgcgccgcgtttttgcaccaccagatggcaatcgcccatcttcagcagtgcgggtaaagcgtcatacgattgcagcgggaaaaattgcatgttgcgcagtccacgctgctgcgccattttttccagccgcgctttgccgccgccctgcccgacaatggcaaaaatcagcggttcatcgcgcagacgatcggcagcttcaataacgttttccagcccctgcttttcaccaatattgccggagtaaagaatgatttttttgttatccggcaggtcaagctggttacgaagggcatcaacatcggcatctgcaacatgctgaaaacgggcaatttccgaccagttggggaagaagatgacgttttccgccgccacgcctttttcgatggctttattcatcatcgaacgcgaaatcgtggagacgttatcgacgttatgcagtccgctacgttcgaacgccgttgccagctgtgccactttgccgcctttgccttttccggcaaggcccagccccagcatggcgtccacttcgtaatcctgaatatgcagcacggtacgcgcaccagagagtttcgccagcaggcgcattcccggcgcgcaaaacagcgttggcaccacgccaataatgcgatccggcttccagcgacgttgcgccatcagcggaaagaaactgctgacggcaaaactgcccagatgcaacaggcgtttcagggtgctcggctgttttggcacatacagcgggcagcgccacaccgtggcggccccctcttctcgtttgtagcgccaggcggaatagttctcgcccacctgccattgcgggtagtaaggcggtgcggtaatgacccgcacctcatgaccttgtgccgccagccattccaccatctcgccggtgtatttgccgatgccggttaactccggcgagtagttaatgccgtagaccagtattttcataatccgggtactccggtacgcttctcagcgagaaaataggcgcggctgttagcatgaacattatcactggcgagcagcgcgtccgacgtcagccagcggtaatcgtcatgctgctcatccggcagtaacagctcttcttccgatactctgaagcgaaaaccgagcaccacatagtgagtggtgaaatccgtgccagagaagttatcgtcataaaagtgctgccagacaccgtaaaactggcctgctgttatcggcaaacgcagccccagttccgccatcgtcagccgctcaaatgcggcttccagcgtttcgtctttctgcacgcgccctcccggcacaaaccagtaaccctgcgccgggcggttggttcttttgccaagcagaaactcgccgcgactgttctcgacaataaagtcgagagagacaagcggagtggagcgcactaccgtggcaaagtcttcctgacgtaaaaacatcattacccccgaaagcggtcttgattctcaaggaaccactggtaagtgctggcaagccccgcttccagtgagatttcgtgataccagccaagctgatgcaggcgcgtcacatccagcagtttgcgcggcgtgccatccggtttgctggcatcaaaaaccacccggcctttgtaacccaccactttggcgatggtttgcgccagctcgcggatagtgcagtcaacgcccgtgccgacgttaatgtgcgacaacatcggctgggtgttctccagccagacttcatgcgccagctccatgacatgaatgctcgccgccgccatatcatcgacgtgcagaaattcgcgcatcggtgtaccgctgccccataccaccacgtccggcgcattctgtgccgtcgcctcgtggaagcgacgcagcaatgctgggatcacatgcgaattactcgggtggaagttgtcgtgtggcccgtacaggttggtcggcatgactgagcggtaatcgcgtccgtactggcggttgtatgattcgcacagtttgatcccggcgattttggcaatagcataaggctcgttagtcggctccagcgtgccctgcaacaactcgctttctgccatcggctgttttgccagtttcgggtagatgcaggacgatccgagaaacagcagtttgttcacgtcgttctgatgcgcggcgtgaatgatgttgctctcaatcatcatgttctggtagatgaaatccgccggataggtgttgttggcaacaatgccgcccactttcgccgccgccagatagacctggtcaatacgttcgctggcaaagaaatcatgcacggcgcggctgtccagcaggttcagctcgtcgcgggtgcgtaataccagttccacatcaccgcgctgttcgagctgccgcctgatggcggaaccgaccatcccgcgatgaccagcaataaaaactcgttgtttactcatgcttatgactccagcgcgatcgccacgtcgtagccgtgagatttcagcagagagtgttttttcgccgcttcgaggtcattagccaccatttcagacaccatctctctgagggtgatttccggtttccagcccagtttttcgtgcgctttggtcgggtcgccgagcagcgtttcaacttcagccggacggaagtaacgcgggtcaacagcgataatcacatcacccggtttaacgcccggcgcgtcatgcccggtgacggaaaccacaatgcccttctcttcaacgcccgtgccttcaaagcgcagtttgatgcccagctgtgctgccgccatttccacgaactgacgcacggagtactgaacgccggtcgcgataacgaaatcttccggctgttcctgctgcagcatcatccactgcatttttacgtagtctttggcgtggccccagtcacgcagggaatccatattgccgaggtacaggcacgactccagcccctgggcgatgttggcgattgcgcgggtgattttgcgggtaacgaaggtttcgccgcggcgcggggattcatggttgaagagaattccgttacaggcgtacatgccgtaggattcacggtagttaacggtgatccagtaggcgtacagtttggcgaccgcatacggagatcgcgggtagaacggcgtggtctctttctgcggaatttcctgcaccagaccatacagttcagaggtggaagcctgatagaaacgagttttcttttccagaccgaggaagcggatcgcctccagcaggcgcagcgtacccatcgcgtcgacgtcagcggtatattctggtgactcaaaagagaccgcaacgtggctcattgcgcccaggttgtacacttcatccggctgtacttcacgcaaaatgcgcgtcaggttagaggtatcactcaggtcgccataatgcagatggaatttcgggttgcaggtgtgcggatcctgataaatgtgatccacgcgctcggtgttgaatgacgatgcgcgacgcttaataccatgcacctcgtaacctttttccagcagaaactctgccaggtaagaaccgtcttgtccggttacaccggtgatgagagcgacttttgacatgtattattcctctgtatttttgaatttattcagtttcaacgcgttcgcgtatcaccactgcgggattcccccggcaaaccacatttgccggaagcgatttaaaaacactgcttcgtgcacccacgacggtgccgtcgccgattgtgacgcctggggcaacaaagacatcggttgccagccagcatttctcgccaatcacaataggcgtggcgttaatggtgaaatgttgacttgcatggtcgtggctaccggtgcataaataacttttttgcgatatcaccgaatgtgcgccaatggttatttcaccgagggtatataaattgacgtcatcgccgacccacgcgtaatcacctaaggttaatttccacggataggtaatttttactgacggacgaataactacgttttttcctatttttgctccgaataaacgtaataaaaaagcccgccagcgatacaatacttgtggcgaccaggcaaatattgttgcctgtactgcccaccataattgcactttaatagcgttgccgccccggaaccctttcggcaccgagaaaccgcttaaatcttgcattggttttccttatattcagactttgttatataaggctttcgtctttgaggtagtacgttggcgtaaatgccaggataattcagcccaaaagccaggcacatgtaatatttgtcgttggacttttttcgcgtcagcacacaattccatattattggtggtagataccccacccatggaaaattcagacaccaggccattgagttttttaaatgcataaccggctttatacattttggctgccagcgcgtagtcggaagaaactttatattccaggtcataacgccattttttcaagccggatacagggaaaaatatcgcctgatgactggcgggcaggctgtgataaatataccagcccggtttggcgctacgtttaattttatgcccgtcgccaaaatccagcagcgcatcgccggtgatcatcacgttatctttttgcatttttaacttacggacaaaatttgcggcattctgatgaaaaatatcgcccgaattgagaaacaacgcgaacttgccttgtgccatcgcaatgcctttgttcatggcgtcgtagataccgttatctggctcgctgacaaagcgtaggttaaagataccattgagattttccagatactcacgggtgccgtcgttggaaccgccatcgacaacaatccattcgaagctgatatcttccacctgcgccagatgcgccagcgaggcatgtgttttgactatcccttcgaggttacgaaacgcgacagtgattatgctaagcaacatgttcttattcttacctcgtaatatttaacgcttttcgcaaaataaacggacagacgattaaaaatgcatattccgggctaaatatcgaaccggtaaaaaacagcgataccggagtaaaaagatataattgcacgcgaaaattgcggttatcaccaaaagcgttgatcatcatttttatcactttccccatgtaccacagtgataaaaacaccgcgaaccaggaaaaataaataatcagcagatacaaaccattgtctatggtttttccgacatccgcaccgttaaatattccgaatgatgcgacatattcataaagtgagccaaatctgactacaccgtcaatatgggtcaaagaataaccgaccatcaccagcggaccgacaatacgataatatgatgacgatccttccgtacctaaatcgcccagacgggtggaaatataaggaaacgcgattaccacaccaaccaggaatacagccagagaaatcaatgctaacggtaactttttcttaatcgcctctttattcagatattgaaatgcccactccagcaaataaaacaggataaaggtcataacccctgaaaacgatccggataatattatccctgcgagaatcatagcatctgttttaggcgttttgataccaaactgtttgatgctgagccaaattgagattaatgccagagcgaaaaatgccggttcgaaataaagtgctgtcgtgcgcttgccgccgaatttaatgaaattcagcacatagctgttgctgtaaatcagatatttcgaaatcgactccataatactgctgccaccggtgaggataatttgtgccatctccaccgccgccagcgccaccaccagcccgaccaccagataaaagaaacgtaatatcttgcgatggttgtgtggcgaaattgttttaaaacgaatactccacaccatgccaataatgatcacaatatagacaaacagcatagttgaagtgacgtatttactggcatccagcgactgaccaaacagatagttaaacgccgtgagtcccgcgccaatccctaaggcaatcatcaattttttaacgctgatgcgttctaaaaacagcagtaacaagacaggtaaaaaagtgacgatggtgatggggaaactttcgccaagctgggcgattttgacgttaaccagcagataaatcagcggcagcaacaggtagctacagattctgatagaagttgacatactcctccagcatctgttgtccactgtaggcggcgcggctgcgttggctgaactcagccagcgtggtaccaaatatcgcctgcgcgatttccggtttgcttaactgcaccagttgcagcacctcttcttcgctgacggttttaccgccggatttttgcaacacttcccgcgccgcatcgctatgggtggcaatcaccggcacgccaatcgatagcgcctcacacaaaatcagcgggtagttatcgacgcgagaactgaataccagcgcatccatctgattgagcgcgctcatcagcttacgtttgtcggtttcaaagccgtgattaaccacgttgccagcggtgaacggcgagaacttaccaaaggtatgcagttcaattttgtcgcccagcgccatcatctcgcgtaccagttgctggttagttttgccgtcgtaacgcagatcatgcgccaccaccgcgattttcggcttgccctgggtttcgcgcaccggaggcaagtccgccagaatcgcttcagttgccatatcaatgccattattgataatccggcaacgccctggaccgtacaggctattgaaagcgtcagccacatgctggctgggggaaataaactgacagcccagcgccagcatctcacggaataactggcgtttgcccgccaccagttggtgtgcgcgatcaatcttcaccggcggatagttatttaaggtcgggcatttctggcagcctgttttccagccttcgcaaccgtcggtaaaggcgcagcgtccggtaacactccagtggtcgtgcagcgtccagaccagagtgacgtccggtttatggtttttcactttttcgcaaaagcgcaccacgctcttaagatttagccagtagctgtgcagcacatgaaaatgcaggaccaccggacccgctgtgcgagtaatggtgcgatataactcattgaaattgccaaacagatcgcgattaaacagacgaaacagagcaatattcgccatcgcggtcatccgcggcgtatgtttgatgacctgcggatagttctgatggctgacgctctctttgccgcctttgccgtaaccgtagacaaaatgtgacgccagcccctgttgcagcgcacgctggtggagatctaacgccacacctgctgccccgccttccgccagtcgcacattaaattgcaaaatattcatttaattaccttcactcgcgctttttctcccaccaccagcgcgttgtccgggacagagtcgagcaccacgctgcccgcgcccacggtgacgttgttaccaagcgtgatatcaccaagaataatgacgttggcaccgagttcgacgccgttgccaatgtgtggacatgccatgttatcggcaccacgattgccgatagtgacgccgtggcgaatggtaaaatcatcccccgctaccacgtttttattgatcacgacggcgtaaccgtgatggatagtaaagcggcggccaatggtcgcggcagcctggatttcataaccgaaaaagcattcggtgataatgcgatacagcaccagcagcggggccgcccacagattgttgaggacgttctttttgcgccacaccgaacaaaaatgagcaacacgataggcaagaaccatgcagcacgggcgtaaactccagctgttggcgcgcagatcttccagcatctttagcgcccccgaataccatcagccagacgtttgccgttacgcaccgacagcagcgtcagcaaagtgcgccaggtcatacgtttattgcggatctggtagagggtaaacagctgatattttttgctggcgcggtcgaatttgtctttgtgcttgcggtaaaagtggaagtacccggagaattttttcggtgacgaggtgatctgcatttcaccgtgattgatatgcaggatctgcgtcgcctcttctactttccacggttcgccgtactccaccaccatccgcaggaagatgtcgtaatcctgtgccgctttcagttcggtatcgaacaaacactctttgaaacgccatgcccaggtaaagacctggttgccaatgatattgcgtttgtagaacaggcggcgtgaatacggcgatttgggatacagcggcaagcttgccggttgggaatagacttcgccctggcaaacgtagtcgttagcgtacaaaaaggcgtgtgtgaccagttgctgtttatgggcgaggaagacgctcagacggttgggtgtccattcgtcatcgtcatcaatcccggtgatatattccccttgcgccagcataatcgcctggttacgtaccgcgcacgccccgctgttaatgtcgttgtgaatgtaagtgatacgcggatcgttgagggcggtgacgtactgttgcagttgttcccaggaggtggagcaatcatccacgatgatcatctcccagttgctgtagtcctggcgcaaaaccgattttattgcccgaatcgccagttgttggcggttccaggtcggcatatagattgagatcagcggattgtttttcataggttgttctcccggcttatgagctggtttgcttgccggatgcggcgtgaacgccttatccggcctacggggcggtgcgaatgcaggcgtcgttatttcgcatccgacttatattcgtattcgtaatagccataatcctgatacgcgctggcgcggcggaagatggagttcagaatcacccctttcaccggaataccgttttgctcaaagcggctcagactggtttccacttctttcaatgtgttgaccgcataacgcgccaccattaacgtggttccgacatgacgaccaacaattgccgcatcggtcactgccagaatcggcggcgtatcaatcaacaccaggtcatagtttttactcgcccagttcaccagttcggcaaagcgttcgctcatcaacagttcagaaggatttggcggcacctgaccgcgcgggatcaggtcaaatttggcaatagaggtcggtttagcagcggtagtaatatcgccctgaccaatcagaatttccgacaggccattaacgttattagtgcccaacagctcgtgggtgtagcctttgcgcatatcgcagtcgatcaacaacacgcgtttattggtctggctgatcaccgccgccaggttggcgcagacaaaggttttaccaattgacgggctaaccccggtcatcatcaacacattgttctgtgcctgcatcatcgcgaagtgcaaactggtacgcagactacggatggcttcaatcgccagatcggttggattccccaccgccagtagctggctctgtttatagcgtttaatccctttgatggttttgacgctatcacgcgctttctgccattccgacagcgggatgctggcatagacgctaataccgtgttcttccagtacttgcgggctttcaatgccgcgattaaacaacgagcgcagcagcacacccacgatagaaagcatcaggccaaggataatcgcgccgaggataatcagccctttcttcggtttcagcacgccaggctgagtgattgccgggtcaacaatgcgcacatcgccgacggtgctggcctcggtgattttcagctcctgctctttattcagcagttgcatatagacctgctgaccagactcgacatcgcgggtcagacggacaatctcctgctgggttttcggcatcgccgttacgcgaccgttaagtttggctttttcgtcttccagcgcctgacgtttctccagcagcgtgcggtacgccgggtgaactttggtgtacagcttggagatttccgcctctttaaaggtcagttcgttcaactgcgcatcgatgttcaccatcgaatcgagcaccgcttttgcttccagcggcagatcaacagaatctttatcctgacggaaggcattcagtttgttttcggcaacatccaagcggctacgtacttccggtaactgttgcgcgaggaaggcgaggcttttcgacgcttccgccgatttgcgctcaatattttgttcctgatagttacgggcgatgctgttaagaatgtcgcggatctgttcacgatcttcaccggtataagtcaggctcaaaacgccagcgtctttgccgttctccgttaccgtcaggctgttttgcagttggttgatcatccccagcgtggagtatttggtgacggtaaactcactgcccgggctggcgtgaatggcttcaaccatcagcgtgacgccttcttttttcagcatctggcccgcttgcccccgggcgctaaagccgccgtcgctgctcagggtgtagtttttgttgtccagcacattaagcgtaaacacctgatccgccatctctttcgggcggttaaaggtggtcactttcaccgtctcgttctgacgtcccatcaggcgatcccagcccgcaccgaaaatcgggaacgtgtttttgctcactgcaatatcgaggtcgagatcgtccaccgttttaccaagcaccagacgcgaacgaatcaactggatctcggcgtccgatgcaggcggtttgttggctaatgccgaaccaatgtcctgcactaacgaattgccgctgttttgctcgatttgtaccagtgcgtcggcactataaatcggcgtggcgaagaaggtgtaaaccacggcacagagggcgaatacggtggtgatgccaatcacccaccagcgcgcttcaatgacggtgccgaccaggcgaccaatatcgatttcatcactgcccgttaccggagcggcatgttgttttactttttctgtcattcttatacctgctctgcgttcaatgcctgcgcccactggcgggcagaccgttcaagtaatgtgtacaccgctgcaaacgtttcccggcttttgcgatacggatcggggatttcacattcgttatcccagtgaccaaacagcatcactttgccgcgcatctccggtgccatctcgcataagcgttcgatatggcgcttttccatggtcaaaatcaggtcgtagttgcgacacagacggcggctgatttgacgggcacagtgaccttccagagacagttgatgttctgcggcgacgctgatagcggtaggatcagcgcccttaccgaccagcgcgccgagtccagcggactccactttcagctccgggtgataacgttgcagtaagcgttccgccgtcggggaacggcaaatattgccgacacagacaactaagatgttgttaaacatgacgattaccagttatgaatgtcgctggctgtatccgtcatgtaacggacaccgctaatagttggcagcaactgattgatcagacggttccagcgggaaaccggggcggtggtgacatacaccacgtcataaggttgcaggcggaattctgtcgccatcaccagcgacgtggcatcggacatatccagctggtagatattggcaatcttgccgttacgcccgccctcgcctttcagcggacgaatgacaaagatgccgctggcgttggaggtggtcatgtcgatgccttcagcattgcccagggcttcagtcagggtcatgccgctaaagtccattttcagggtgctctgtttcttcacttcacccatcacaaatactttcagatcatcattacgtggcacgtagagaatatcgccggggtaaagcaggcgattctggttgaggtcgccgttttgcatcagcgcctgcaaagaaatgcgctcttcacgaccattgtgtgttagcaccacgttgcgccagtcagcggtgtcggtcaggccacctgcggcgttgatggcgtcgagaatagtcagtggcacgttggtgatcgcctgttgaccggatttattcacctgaccggagatataggccttttgtgagcggaaggcggcgatattaacgtccacctgcgggtcagcgatgtacgtcgctaagcgcccggtaatatcactgcggatttcagcgagcgttttcccgactacgtggaccttgccgatatacgggtaaaacatagtgccgtcaggctgtacccagttgccggtgtcgctggagctgcggtactgaccggctggcgtggtgagttccgggtgatcccagacggtgacattaagaacgtcccccggcccgacgcgatactggtaattcgcgatctcactttccagcgtcatattggggcgcgctacattcgggcgtgggcgtaattggtcaatcaggcgcggggtcagcggataaacattcaccattttgtcgagatcgaaatcagcgtcctgctgtttgatgacgtctttgcccatcgtcgacatattgctgcccggaagtactgtgcaaccgcttatcaaggttactgacaccaataatggcatcaatttcattttggatttcatcattgtttatttatcactttggcagagtaattatcctgtgcactattaatagcaatgtcgccatgcacatttaccttgcagttaattgaataaaaatttaactggcatcagtcctaaaaaaattgatttcatccgcaggctattgacagaataattcagactggtctttcaggcatccagacacgctaccgcccctggctttttagctaccaatacactgatttagtttaatttttcacaccctctcagcatgcagtcgttgatgagaaagggttattacggaaattaacttccgaatataaggtgacattatggtaattgaatattggctttccaataatgcaggaggaagtgttacagctaacggaatagcaggcaagataacaattcggtaattggctatttttaagaattatattaagtgtcattcaatatggtttttaggagtttctttaggttgacaatatttaatatagtgtctccacatgcgatatttcttaaataatgttttattattaccacttttaattcagggataatgtgaggttattaccctcaaataatatgagataaatagtgctgcaacattgcatttttgccccgatttatccatgatcgaattgtgacatttgtcatacaacgaataggttttgtacttactatggaatggattgccgatccgtctatctgggccgggttaatcacgctgattgtgatcgaactggtcctcggcattgataacctggtctttattgccatcctcgccgaaaaactaccgccgaagcagcgtgaccgcgcacgggttaccgggctgctgctggcaatgttaatgcgcctgttactgctggcgtcaatctcctggctggtcaccctgactcaaccgctgttcagcttccgctcgtttacctttagcgcccgcgacttaatcatgctgtttggtggtttcttcctgttgttcaaagccacgatggagctgaacgaacggctggaagggaaagacagcaataatcccacacaacgcaaaggtgcgaagttctggggcgtggtgacgcaaattgtggtactggacgccattttctcactcgactcagtgattaccgccgtcgggatggtcgaccatttactggtcatgatggccgccgtggttatcgctatcagcctgatgttgatggccagcaagccgttaacgcaatttgttaacagtcacccgacgatcgttattctctgcttaagcttcctgttgatgattggctttagcctggtggcagaaggtttcggcttcgtcattccgaaaggctacctgtacgctgccattggtttctcggtgatgatcgaggcgctcaatcagttggctatctttaaccggcgacgttttctttccgctaaccagacgctgcgccagcggactaccgaagcggtaatgcgcctgcttagcgggcaaaaagaagatgcggaactggacgccgaaaccgcgtccatgctggtggatcatggtaaccagcagatctttaatccgcaggaacggcggatgattgagcgggtacttaatcttaaccagcgtaccgtcagcagcattatgacgtcgcgccacgatattgagcatatcgatctcaacgcgccggaagaagaaatccgccagttgctggagcgaaatcagcatacgcggctggtggttaccgacggtgatgacgcagaagatttgctcggtgttgttcacgttatcgacctgctacaacagtctctgcgcggcgaaccgctcaacctgcgggtgttgattcgccagccgctggtgttcccggaaaccttgccgttgttacctgccctggagcagttccgtaatgcccgcacgcactttgcttttgtggtggatgagtttggctcggtggaagggattgtgacattaagtgacgtcactgaaaccattgccggtaacttaccgaacgaagtggaagagatcgacgcccgccatgatattcagaagaatgcggacggttcctggacggcgaatggtcatatgccgctggaggatctggtgcaatatgtgccgctgccgctggatgaaaaacgtgaatatcacaccattgccgggctgttgatggagtatttgcagcgtattccaaaacctggcgaagaagttcaggtgggggattatttgcttaaaacgttgcaggtagaaagccatcgcgtgcagaaggtgcagattataccgctgcgtaaggatggcgagatggagtacgaggtgtgatggtatcggtcattttacccaatagccgaaaggaataagatgagggaaccgcgccatcggcgatttaccgccgggagcccgggttgccagggtggtggagattgagccaccctggcacgttcaccggcttgagcgttccatagtagcgaggaacatcaagtgaacggaacagccttcgatcttacatattcagaatataatgatgccgccacgaacgcctgatgcgacgctttacgcgtcttatcaggcctacaggactggtcacctggtaacctacatcttctccagcaacttcttcacatctttgccattacgggaatctttattccgctcggcccagtcattcaggcgacgtttcgcttcgtcctgtagatgtttgcgcagtaactgatccacttgcaggctgtaattgagttgctgccagttgccataaacccgcagcggtactggcgtttctttcaggaaatcaatcagtttgctttccccgttccagccacccacgacccgaatatcaaactgggtgtcgcaggtttgatctgccagattcaacatgccttcccctgtcagcgccagcacaggcgattgaccttgcatgtcgtttaacgtcacgacgccatccttcaacgtcaaatcggtggtaaagcggtcaagccgcgtcacgttatcaaagttttcagcggccttcacatcaccgccattacgctctaccgcttgctgaatcatctgctggaagttcatcccttccatgcgcgtgtcggtcatttcgacatgtgcctgtccttgccagttgtggcggaatgcgtcggcatctatgtcagcaccggagaaatcaccagccagtgacatttttccggtcaacgaaatcggatagttaaacgccttcagaatggtaccaatctcaacgttttccagccgtggctggaagtttatccgcggatttattgatgtcgcgtccagcgtgcccggcagtgaaacctgtccaccgttaagtttgccctgcagttgagtaatttccagcaaacccgacttgttggtcatttgcgtggcaacatctgtaaaattcattccgcgccagcgcacgttactggcctgcaacaaaatatcagccgtaaagccttgcagtccctgataggccggttcatcaatacgcgaagaaatgaccgggcgcggcaacgttgattggctctgcccctgctgcgcggcaccgttttcaccattcgcggtttcattaagcgggatgaggttgtcaagattcagttgcgggaattgcagcctcagctgccattccggtttctctgtcagcgtaacctgtgcttgcccgcttagcgtactatcattggcggtcaaactaatttggttaaatgaaaggcgtttatgtgactcctgccactgggcctggaaactcccctgcccctgaataccttgttttggtaaatcggcaccctgcaactgccagttaatttgttcaatagccgccgttaaatcatgcggataatcagaagcatctaccgtaccgttaagggatatcgtgagatcgcgctgatcgcgattaacccgcccggagaactcaaatgaaccacgatgttggggatcttgttccatttgcaggcgaatattgcggattgtcacctgctcgtcatcttcatgctggaacaccagcacgctgtccgccaccttaagactggatatatcaaacgaccatccgcgatcgtctgacagatccggcaaggtattgtcgcgcggtgcaaccggagcgtcttcactgcgcaccgcttccgtctgcggcgtcagttggatcactgccccttttagcatcacctgcttaacgctcagttgatgactcagtagtggtaaaagcgccacgtccagacgcatgttgtcggcgcgaaccagtggctggcttgcgccctgggcggtgagagacattcgcccggagaggatactaagctgcggccagacgtgccaacgcagtggcccgtcgagctgcaattgataaccgctacgtgcagcaacttgcttgaccatatagtcgcggaaatcattcggattcaccagcaacactaacgcagataacccggccaccagcacgaccaggagtatcatcagcgtcgtcagaaatcgtctcatggtatcctcaatgggcctgaattagtctttatcgattcggctggctaccgcgccctgctggttgcgatatttcgcatcttcacggcggttgtaaggtcgcaccgccgggccggaaagcggctcaaagctcagcgcaccaattaacatgcccggacgcagcgccagcggcagcttaccggagttgtagaactccagcacaatgcaaccagaccagcccggatcgatgcggtgcgcggtgacgtgcaccatcagccccagacgcgccagtgaggaacgcccgtccagccagcccaccagatcggctggcagcgtcaccgactccagcgtcaccgccagcgccagctctcctgggtgaagatagaacgcctcgccctcgtcgagaacgatctcatcgctcatcacgcggtcaagcgcggcgctcacttcatctttgggaccgctcagatcgataaacgctgccgtgtgaccacggaaggtacgaaatttattgcccaggcgtacatccaccgtcgcgccgttaatacgctccactggcggacgtgggttgatcgacaaacggccttcatcaagccaggcttcaatatctcggtcacacagacgcatggcattttctcctttcgcgcatcactcccttaacgccaattacgtcaagggcatactaggttatcactgaacggtacacaatttatcaagcttattcaaagaactgacttattttcgctttcaatatatcgatcgcgatgcggtttttcccgccgcgcggcacgataatgtccgcatattgtttagaaggctcaatgaattgcaggaacatcgggcgcacggttttttgatattgcgccatcactgaatccattgaacgcccacgctcgttaacgtcacgcttgatgcggcgcatcaggcagatatccagcggggtatcaacgaaaatggagaagttaagttcgtcacgcaaacgcgcatccgtcagcaacaaaatgccttcgagaatgatgaccttcttcggctcaaccgtcaccgtttctttcatacgcgtatgttcaacatagctgtaaaccggcaggtcaattgccgagccgcgtttcaacgcttgtaaatgctcaagcagcagactgtgatccatcgcgctgggatggtcgtagttggtcttaacgcgttcttccatcgacagatggctttgatctttgtaatagcagtcttcgggaattacgccgatgtgttcatcaccgacttgctcacgcaattcacgataaagggtactggcaataagactcttgccggaagccgatgcgccagcgataccgataatgacgcactgatgagactgatcagtcatatatttagcgacctgattaacctggatgttaggaagggggcgacgaagcgccaaacgcggcaattatagggatttcatccgtctgataccagtcgaatagcgttgccgcgcgctcagagttaattgttgacaaagaattcccgggggcaaattacgttgatcagttttatgtaaggtaaaaaatgttaaacgcagttgcgcaaattatccgcctttacgtcactttatgagcaattcgcatataaaatgtaaaacttttgtactagcataaacacagaaacgaatactggcgaccaggtcttgcggataaagcggtaatgagcaaacaatcacagcatgtattaattgccctgccccacccgctgcttcacctggtcagtttaggtttagtctcgtttatctttacccttttctcgcttgagctttcgcagtttggcacccaactcgccccactgtggttcccgacgtccatcatgatggtggcgttttatcgccatgccgggcgcatgtggccgggaattgcgctgagctgttcgctgggaaatatcgccgcatccatcctgcttttttccaccagctcgctgaacatgacctggacgaccatcaatattgttgaagccgtggtcggggcagtgctgctacgtaaattgctgccgtggtataaccccttgcaaaatctggctgactggctgcgtctggcactcggcagcgccattgttccgcctctgttggggggtgttctggttgtcctgctgacgcccggagacgatcctctcagggcatttttgatatgggtactgtcagaatccatcggcgctctggcactggtgccgctgggattgttatttaaaccacactatctgctgcgccatcgcaacccacggttgctttttgagtcgctgctcacgttagccatcacactgacgttaagctggctttcgatgctgtatctgccgtggccttttactttcattattgtgctgttgatgtggagcgccgtgcgtctgccacgaatggaagcctttttgatcttccttaccacggtgatgatggtgtcgctgatgatggccgcggatccctccctgcttgctacgccgcgtacgtacctgatgagccatatgccgtggctaccgtttttgctgatcctgctgcccgccaacatcatgaccatggtgatgtatgcctttcgtgcggaacgcaaacacatttccgaaagcgaaacccactttcggaacgcgatggaatattccgctatcggtatggcgttagtgggcaccgagggacaatggctgcaaaccaacaaagcgctctgccagtttctcgggtacagtcaggaagagctgcgcggactcacctttcagcaactgacctggccggaggatctcaataaagatctccaacaggttgaaaagctgataagcggtgaaataaacacctattcaatggaaaaacgctactacaaccgcaatggcgatgttgtctgggcgttgcttgccgtctcactggtgcgccacacggatggcacgccgctctattttatcgctcagattgaagacattaacgagctaaaacgcaccgaacaggtcaatcagcaactgatggagcgcatcactctggctaacgaagcgggcgggattggcatctgggagtgggagttgaagccgaatatttttagctgggataagcggatgttcgagctgtatgaaattcctccacatatcaaaccgaactggcaggtgtggtacgagtgcgtgctgccggaagatcgccagcatgccgaaaaagtgattcgtgattcgttgcaatcacgctcgccctttaaactggaatttcgcattaccgtaaaagacggtattcgccatatccgcgccctcgccaaccgggtactgaataaagaaggcgaagtcgaacgtctcctcggcatcaatatggatatgaccgaagtgaaacagcttaacgaggcattgtttcaggaaaaagagcgcctgcacattacgcttgattccatcggtgaagccgtggtctgtattgatatggcgatgaaaattacctttatgaatccagtggcggagaagatgagcggctggacgcaggaagaagcgttaggtgttccgctcctgacggtgttgcatattacttttggcgacaacggaccattaatggagaacatttacagtgccgacacctcacgttccgcgatcgagcaagatgtggtgttgcactgtcggagcggcggcagttacgacgtgcattacagtattacgccgttaagtactctggacggcagcaatattggttcggttctggtgattcaggacgttaccgaatcacgcaaaatgctgcgccagctgagctacagcgcctcccatgatgcactgacgcatctcgccaaccgcgccagttttgagaaacaactgcgtatcctgctgcaaacggtaaacagtacacatcagcgacatgccctggtgtttatcgatcttgatcgctttaaagcggtgaatgacagcgccgggcatgcggcgggtgacgctttgctgcgcgaactggcgtcgttaatgctgagtatgctgcgttccagcgacgtgctggcgcgactcggtggggatgaatttggtctgctgctaccagactgtaatgttgaaagcgcgcgttttatcgctacacgcattatcagtgccgtgaatgactatcactttatatgggaaggccgtgtgcatcgggtaggtgccagtgccgggattaccttgattgatgacaacaatcatcaggcggcagaagtgatgtcgcaggctgatatcgcctgttatgcctccaaaaatggtggccggggccgggtgacggtttacgaaccgcagcaagctgccgcacatagcgaacgggcggcgatgtcgcttgatgaacagtggcggatgattaaagagaatcagttgatgatgctcgcccacggtgtcgcttcgccacggatcccggaagcgcgtaatttgtggctgatttcacttaagctctggagttgcgaaggcgagattattgatgaacaaacatttcgtcgtagcttcagcgatccggcgcttagccatgctcttgaccgccgggtattccacgaatttttccagcaggccgcaaaagcggttgccagtaaaggcataagcatctccctccccctttccgttgccggtttgagtagcgccacgctggtgaatgatctgcttgagcagctggaaaatagccctctaccaccacggttattacatctgattattccggctgaagcgattttagatcacgcagaaagcgtgcaaaaactgcggctggcgggatgtcggatagtgctcagccaggtgggccgcgatctgcaaatcttcaactcgctgaaagcgaatatggcagattacctgctacttgatggtgagttatgcgccaacgtgcagggtaatttgatggatgagatgctgattacgattattcaggggcacgctcagcgactcgggatgaaaaccatcgccgggccagtcgttttacccttagtgatggatacgctttctggcatcggcgtcgatctgatttatggtgaggtgattgccgatgcccaaccgctggatttgctggtgaatagtagttatttcgcgattaactgaggcgtgcttccccatcgcctgatgcgacgctaacgcgtcttatcatgcctacaaatcgctcattccccaggccggataaggcgctcgcaccgcatccggcgaccaacgtcatgcttcgtctggttgccagccttccgtataccagatatgcaacagcgcataagaacgccagggcttccagcgctcggcataacggcggatttgcgccggtgtcattcccggaaatcgctgtttaatcagataatcatccggcaggaaaacatctttcgcctgccagccacgcaaagcaaaataattcgccgtccagcgcccgatacccggaaaagtttgcagcgttttcatcgcctgctccacatcgcccggtattgtcattggtaaggtgccctccagcgccgcatttgccagatgaatcagcgcctctgcccgtttcaacggcatacctaacgcttttaatgcctgcgggtctgctgctgccagccgctgaggcgtcgggaagcagatatactccggaaaatcatccagccgttcgccataaagctgtgccactctggcggtcaattttgccgccatcgccacgctcaccagttggcctaaaatcgcccgcacgccctgctcaaaagcatcaacacagccgggtaaacgcaatccgggccgcgccgcgcctaacctgcccaacgcaccgttaacaatttgtgggttacattgcagatcaaacaggcggctcattttcgccagacactctgcggcaacaggttctaaacctgcacttaaatttatgtgcagagtatggcgggctatatccggaatagcagtcaccacgccgcgatattcgcccaccgccagactacgggcataataactgtccgcgaccgtttccacactgctcaccgcacgggcggcgagaaatcccaacatccacgaccagtcatacggcggctgccagttcagggtatacatcgcatctccttattcatccgctttcagcataaacgttattcagacgctgcgctttgctttcatattccggttgtcgcgacggcaacatttcgctaaagtcacgccccttcttcaccggcatggggattatttcgtgtttattggttttgattacggtacagcaaactgttcagtggcggtcatgcgtgacggtaaaccgcatttgctaaaaatggaaaacgacagcacgctgctgccttcaatgctttgcgcgccaacgcgtgaagcggtaagcgaatggctgtaccgccatcatgatgttccggcagacgacgatgaaacgcaggcgctgttacgtcgggcgattcgttataaccgcgaagaagatatcgatgttacggcgaaaagcgtgcagttcggtctttcctcactggcacagtacattgatgatccagaagaagtgtggtttgtgaaatcaccaaaatcgttcctcggtgccagcggcttaaaaccgcagcaggtagcgctgtttgaggatctggtctgcgcaatgatgttgcacattcgccagcaggcgcaggcacagctgccagaagcgattactcaggcggtgattggtcgtccgatcaacttccaggggctgggcggtgatgaagcaaacacccaggcgcaagggattctggaacgcgcggcgaagcgtgccggattcagggacgtggtattccagtacgagccggtcgcggctgggctggattacgaagccaccttgcaggaagaaaaacgggtgctggtggtggatatcggcggtggtacgactgactgttcattgctgctgatggggccgcagtggcgttcgcgtctcgatcgtgaagccagcctgctgggtcacagtggttgccgtattggcggtaacgatctggatatcgcgctggcgtttaaaaacctgatgccactgctgggtatgggtggcgaaaccgaaaaaggcatcgccctgccgatcctgccgtggtggaatgcggttgccatcaacgacgtacctgcgcagagtgatttctacagtagtgccaacggtcgtctgcttaacgatctggtacgcgatgcccgcgaaccggaaaaagtggccctgttacagaaagtctggcgtcagcgtttaagctatcgcctggtgcgtagcgcagaagagtgcaaaattgctctttcaagcgtagcggaaacccgcgcctcactgccgtttatcagcaatgaactggctacgctgattagccagcgagggctggaaagcgccctcagccagccactgacgcggattctggaacaggtgcaactggccctggataacgcccaggaaaaaccggacgttatctacctgaccggcggtagcgcccgttctccgctgattaaaaaagcgctggcagaacagttgccgggcattccgattgcaggcggcgatgactttggctccgtcaccgccgggctggcacgctgggcggaagtggtgtttcgttaattgaaaaatggctcagcagcggcttaaatctgcctgcgcctgagccagtttttctgctgcctgacgtaacggttccatcaacggcatggtccgtgctggagcatgaaggcggaatcgctgcaactctgtcgcgccgactgtcaacgccgattccagccgatgtcgtttggcggtcattttcgccattaccgcttgtctgtctgctggcgttatcgcttcattcggcctgaacacaaaacggcgttcacagctcgctttccagtcgataaccgcctgggtcagatggtcgccaaaccctttcacttgcttaacgccacgacgggtaacatctgcggctgtttcaataccaaaagaccgtaacgccgctttacgcgcagggccaacgccgggaatagaggcaacatcaataaaaaatccctccagaaacttctgcttctgccgttcccttgcagtgtcatgaagtgctgccagagcgcgtttctcttcttccggtaacccgagaatttcgtccttcattttttcgagcatcgtccgtttggcgataaaaccttccaggccgcctacctgctggatctggcggactaaatggtcatagtccattttcgcacgattaaatgcctcacggcgttgctgaacttctgctttgtacgctttgcttgtcagactgccaataatccagatagccgccagcacaggaaccaaaataatataacgcggttctgcctgaaggccgcaaagcagcagcgataatgctgacagtgcgatctcaagcagaatgatgtattcgcgccgtaacaggcctaaaggaagcggcctgccagtcggttggaaatgatcgggtaatggcagttgcaatgctggcggtgctactgacgccatcaccatcgcccagactttcgccagcacaaaattcccgccggtggtaatgacctcttcgccgagatcaataaaatagataacaccttgattatccagcgcacaccacgggcagtcagtcaaatgagcggggtaaacatgcattgctgaaacgatacatttctttaactgttggcgtagagagtccagtgccgctacccacgctttagccgtcggacgcccggttgccacgccactttccgtgaatgcctgctgaaacatggcttcaacatcactcggtaacatcgatagcggaatagatcgtggcggcggttttaaaccacgtcgctgattatctgacgcgtaggcataacggaaatgggtaatatccgtctccagcgcattacccgcatcagagataagcggcacaccagaataaggatgccgcccaccaaacaagacgtgaaaaattagcaacgcaaggccaaaattatcgtgattttctgtgcgttcaaaaccgacaaatgatggcaaggtttgtagctctggcggcgtaaaatgcgacacgccgacttcgcataaatgcagtgtgccattggcgttaatttgaaaggagtcgctatcaatcagtaccactttgctgtcgcgacctaccataaaactgttctggtttacgtcacccacgacgtgcccgtgctcgtgaaccgtagcaaaagatgaagcaatattgcgcgcaacatagagtagaaaatcccacgcacaatgagggtaactctggcgacgatgtgccgggctatagatcatatgaatcggttctttaccagaaacttttggcatcataaaaccgataacttttccgcctcgtccaccgtgaagcgttgcctgcggccaggcgacataattcaacaactgcgcgtcagctgtcgcagccataaaggcaagtttgtcctgttttaaggcgggtggcggcgtgtgataaatcttggcgacgctatcgacaaactcctcgatatcataaaccgcgccttcaccacctttgcccagttcacggccaagagtggtcaattcacctgtcgatgtaaatacttttatatttgttttcataatatttcgcgggtagttatattatatttcaatgaataataacaactaaccattaaaattatttctatatggggaaaacccactcaagaataaaaatgataatgcaattttatcaggatacaattcaatttcggcctgataatgattaacttccacaggtttttgctaactttgactacaaagggattctggagaaaaaatgaaaaagatattacttatgttgagtctgctattttttactaccgcgggctttagtgaagtttcggatacgttagtgacgggaggttatgataaacaagcgatgtctgacgcgattaaacatgcgcggaaagaaaccgataaattcatcgaggttatgaataaaaaagatgccgatactttcgcagtcaaagccccgataaccgatcacggaagaaccgagcatttctggcttacggatgtcacttattctaacggcatgtttattggcgtaatcagcaatgaccctggtattgttacaaacgtagaatatggccaggagtggaaaatcaagaaagaagatatttcagactggatgtatacgcgcggggataaaatttacggcggttataccattgatcctttattggtcacctatccaaaagaagaagccgacgagctaagagcaaaattagttcgctaatcagccgttatatttattgtttaaactggcggttgaattgttgtcttcaaccgccatgagaaactcactctgcccacagcgccagtgccaacgttttatcatcatccgtacgctcgtttaccgccgggctggacaaaaactgctttaacaattcaggtaataaatcgagttgttcctgcgttgctgccgccagtccattgaaaaacggggtaaagaaaggcacatgaggagaattatccagcatatttaacgccagtcgctggataccatccgtaaatgctgcaactttgtgcgcacgcccagtgctggtgaaagtttccagtctggaaacggcatcttcgtcggtaatgaagtgcgtcatgttggcatattcacccgccatcggcgtgagaggcaattgcagaccgtgacccaaatctaccaccacgccgccatcgccaatctgcataatcaaggtgccgtcaggcgatgaaatcagtcccagaaatgtgcaggcaaaatcgcgaaccgctaattctttggcttccgcctcggcaaaaagtcgttgacgaatggtcagtaccatatttgtggcgaggacatcattaagccccaattccccgccctgcactttttgcgacatataagccatcgcttcattgacggcgagcatcgcgccttcgccaccctgcgagacactgcctgcgccatcagcgacaaataccgacaataatggctgctggtcatttaaccaggcaatctgcatctggcaggcatcctgacaaggcaagtccgcgctgatgtgcgacgttccaacggttgatgcatagaccagacgccagctcacactgacgtccagccttttggcgcttccagcacaacttccgttcccggcgtggagcgggaaaccgaacgcagcgaactggataaccagctaaacagttcacggaattgtaatccttgcagaggcaaaggctgacgaacgctaatttgtgccagcgtcttcatatccgccccctgaacaccgatggaaaagaaagcaaaccttttatcttcttccccccgaaacactttgttggctgcagcctgccactcatcggttggtgcaccatcggtaatcaggaaaatccacgggcgataatacgaaataccatttgcacgatactcacgtttccgctcctctaccatatccagggctttggtaatggccgcacccattggtgtatcgccctgggcaaacaggatgggcggaaaaaaattagcggcgctggtaaagggttgttccacatgcaccgggccgaacgtcacaatgccgagttccactctttttaaagccagcggatcagcaagcagttcatcacgaaaggtaaccaatccggcgttaagttcattaataggtctaccgttcatagaaccagaaacatccagcagcaaaatgcaggggcaacgtggttccgggttactggcaaaatcgctggtggcaaacgtgatttgttcgctcataagaaatcctttcttagagaattatcgaggtccggtatcataccgactgcaataatgaaataagagcaaacgaagaaactttcagaattaggcccggcggcgcagaaaattttgctattcgcctcgcaagaacggagagccgtcgattgacactaagggcggagtgacataatttcaggagtgagggttagggagaggtttccccctccccctggtgttcttagtaagcctggaagctaatcactaagagtatcaccagtatgatgacgtgcttcatcataaccctttccttattaaaagccctcttctccgggagaggctttcccgtttcagcgtcccgctgaaatcatcggcttacctcctttcgccctgaatgcagtctatcgctaacgcgtgaataaaatagtttcctctgtgattattgcgtaacgactcgcaaagaatatttgctggcaggatcgcagactacaaagcctgcggattgacaatcttatcgtgaaggcatactttcaggagtgagggtagagcggggtttcccccgccctggtagtcttagtaagcggggaagcttatgactaagagcaccacgatgatgagtagcttcatcatgaccctttccttatttatggccccttcctcgggaggggctttcccgtttcagcgtcccgctgaaatcgtcggcttacctcctttcgccatgcaagcagtctatcgctaacgcgtagataaaatagtttcctgtgttattactggatgcgtgctcgcaaatgtgcccgtcattcagacgattccagacagtgtttcataattcctccatttttctcccttattggctggctacactagtatcattccgcgaaacgtttcaggaagagaaactcttaacgatgaaaggtagttataaatcccgttgggtaatcgtaatcgtggtggttatcgccgccatcgccgcattctggttctggcaaggccgcaatgactcccggagtgcagccccaggggcgacgaaacaagcgcagcaatcgccagcgggtggtcgacgtggtatgcgttccggcccattagccccggttcaggcggcgaccgccgtagaacaggcagttccgcgttacctcaccgggcttggcaccattaccgccgctaataccgttacggtgcgcagccgcgtggacggccaactgatagcgttacatttccaggaaggccagcaggtcaaagcaggcgatttactggcagaaattgaccccagccagttcaaagttgcattagcacaagcccagggccaactggcaaaagataaagccacgcttgccaacgcccgccgtgacctggcgcgttatcaacaactggcaaaaaccaatctcgtttcccgccaggagctggatgcccaacaggcgctggtcagtgaaaccgaaggcaccattaaggctgatgaagcaagcgttgccagcgcgcagctgcaactcgactggagccggattaccgcaccagtcgatggtcgcgttggtctcaagcaggttgatgttggtaaccaaatctccagtggtgataccaccgggatcgtggtgatcacccagacgcatcctatcgatttagtctttaccctgccggaaagcgatatcgctaccgtagtgcaggcgcagaaagccggaaaaccgctggtggtagaagcctgggatcgcaccaactcgaagaaattaagtgaaggcacgctgttaagtctagataaccaaatcgatgccactaccggtacgattaaagtgaaagcacgctttaataatcaggatgatgcgctgtttcccaatcagtttgttaacgcgcgcatgttagtcgacaccgaacaaaacgccgtagtgatcccaacagccgccctgcaaatgggcaatgaaggccattttgtctgggtgctgaatagcgaaaacaaggtcagcaaacatctggtgacgccgggcattcaggacagtcagaaagtggtgatccgtgcaggtatttctgcgggcgatcgcgtggtgacagacggcattgatcgcctgaccgaaggggcgaaagtggaagtggtggaagcccagagcgccactactccggaagagaaagccaccagccgcgaatacgcgaaaaaaggagcacgctcctgatgcaggtgttacccccgagcagcacaggcggcccgtcgcgcctgtttattatgcgtcctgtggccaccacgctgctgatggtggcgatcttactcgccgggattatcggttatcgcgccctgcccgtttcggcgctgccggaagtggactatccgaccattcaggtggtcacgctctacccaggtgccagcccggatgtcatgacctctgccgttaccgcgccgctagaacgccagttcgggcagatgtctggcctgaaacagatgtcgtcgcaaagttccggcggtgcgtcagttatcactttgcagttccagctaacattaccgctcgatgtcgccgagcaggaagtgcaggccgcgattaacgctgcgaccaacttgttgccgagcgatctgcctaacccgccggtttacagcaaagtgaacccggcagatccgccgatcatgacgctcgccgtcacctcaaccgccatgccgatgacgcaagtggaagatatggtggaaacccgcgtcgcgcagaaaatctcgcagatttccggcgtcggcctggtgacgctttccggcggtcagcgtccggctgttcgcgtcaaacttaacgctcaggcgattgccgccctcggcctgaccagcgaaaccgtgcgcaccgccattaccggcgctaacgttaactcggcaaaaggtagcctcgacggcccttcccgtgcggtcacgctttccgcgaacgaccagatgcaatccgccgaagagtatcgccagctaatcatcgcctaccagaacggcgcgccaattcgtctgggcgatgtcgcaactgtagagcaaggtgcagaaaacagctggctcggcgcgtgggcgaacaaagaacaggccattgtgatgaatgttcagcgccagcccggtgctaacattatctccaccgccgacagcattcggcagatgctgccacagctcactgagagtctgccgaaatcggtgaaggtgacagtgctttccgatcgcaccaccaatatccgcgcatccgtcgatgatactcagtttgaattgatgatggctatcgcgctggtagtcatgattatctacctgtttttgcgcaatattccggcgaccatcattcccggtgttgctgtaccgctgtcgttaatcggcactttcgcggttatggtgtttctcgatttttcaatcaataacctgacactgatggcgttaactatcgccaccggattcgtggtcgatgacgccatcgtggtgatcgaaaacatttcccgctatatcgaaaaaggcgaaaaaccgttggcggcggcgctcaagggcgcaggtgaaatcggctttaccattatctcgctgaccttctcactgattgcggtgttgatcccactgctgtttatgggcgatatcgtcgggcgactgttccgcgaatttgctattaccctggcggtagcgattttgatctcagcggtggtgtcgctgaccctgacaccgatgatgtgcgcgcggatgctcagccaggagtcgttgcgtaaacagaaccgcttctcccgtgcctcggaaaaaatgttcgacaggataatcgccgcctatggtcgtggactggcgaaagtgctgaatcatccgtggctgaccttaagcgtggcactcagcacgctgctgcttagcgtgctgctgtgggtgttcattccgaaaggtttcttcccggtacaggacaatggcattattcagggcactttgcaggcaccgcaatccagctcctttgccaatatggcccagcgacaacgccaggtcgcggacgtgattttgcaggatccggcagtgcaaagcctgacctcatttgttggcgttgatggcactaacccgtcgctgaacagtgcacgtttacaaatcaacctcaaaccgttggatgaacgtgatgatcgggtgcaaaaagtcatcgcccgtctgcaaacggcggtagataaagtgccgggcgtcgatctcttcctgcaaccaacgcaggatctgactattgatactcaggtcagccgcacccagtaccagtttaccttgcaggccacgtcactggatgcgctcagtacctgggtgccacagttgatggaaaaactccagcaactgccacagctttctgatgtctccagcgactggcaggacaaagggctggtggcgtatgtcaatgttgatcgcgacagcgccagccgtctggggatcagcatggcggatgtcgataacgccctgtacaacgcgtttggtcagcggctgatttccactatttatactcaggccaaccagtatcgcgtggtgctggagcacaacaccgaaaataccccaggcctcgcggcgctggataccattcgcctgaccagcagcgacggcggcgtggtgccgctaagctcaattgccaaaattgagcagcgttttgcgccgctctccatcaaccatctggatcagttcccggtaacgaccatctcctttaacgtgccggataactattcgctgggcgatgcggtgcaggcgattatggacaccgaaaagacgctgaatctgccggtggatatcaccacgcagttccagggcagcaccctcgccttccagtcggcgctgggcagcactgtctggctgattgtcgcggcggtggtggcgatgtatatcgtgctcggcattctgtacgagagctttattcacccgatcaccattctctcgacgctacccaccgcaggggttggcgcactgctggcgttgctgattgctggtagcgaactggatgtgattgcgattatcggcattattttgctgatcggtatcgtgaagaagaacgccatcatgatgatcgacttcgcgctggctgctgagcgcgagcaaggcatgtcgccgcgcgaggcaatctaccaggcttgtctgttgcgttttcgtccgatcctgatgaccactctggcggctctgcttggcgcgctgccgctgatgttgagtaccggggtcggcgcggaactgcgtcgtccgttaggtatcggcatggtcggcggtctgattgtcagccaggtgctgacgctgtttaccacgccggtgatttatttgctgttcgaccgcctggcattgtggaccaaaagccgctttgcccgtcatgaagaggaggcgtaagtgaagttttttgccctcttcatttaccgcccggtggcgacgattttactgtcggttgccattaccctgtgcggcatactgggcttccgtatgctgccggtcgccccgctgccgcaggtcgattttccggtgattatcgtcagcgcctcgctgcccggtgcgtcaccagaaacaatggcgtcttccgttgccacgccgctggagcgctcacttgggcgcattgccggagtcagtgaaatgacctccagcagttcgctcggcagcacgcgtattattttgcagtttgattttgaccgggatatcaacggcgcagcgcgtgatgtgcaggcggcgatcaacgctgcacaaagtttgctgcccagtgggatgcccagccgcccgacctatcgcaaagcgaacccgtcggatgcgccaattatgatcctcacgctgacgtccgatacttattcgcagggtgaactgtacgatttcgcctcgacgcagctggctccgacgatttcgcaaatcgacggtgttggtgatgtcgatgtcggaggcagctcactgcccgccgtacgcgtcgggctgaatccgcaggcgctgtttaatcagggcgtgtcgctggacgacgtacgcaccgccgtcagcaatgccaacgtgcgtaaaccgcagggcgcgctggaagatggcactcaccgctggcagatccagaccaatgatgagctaaaaaccgccgctgaatatcagccgttgattattcactacaacaacggcggcgcggttcgtctgggcgatgtggcgacggtgaccgactcagtgcaggatgtgcgcaacgccgggatgaccaacgccaaaccggctattttactgatgatccgcaaactgccggaagccaatattatccagacggttgacagcatccgggcaaaattaccggagttgcaggaaaccattccggcggcgattgatctgcaaattgcccaggatcgctcccccaccattcgcgcctcgctggaagaagtcgagcaaacgctgattatctcggtggcgctggtgattctggtggtgtttttattcctgcgctcgggtcgcgccactattattcccgccgtttcggtgccggtttcgctgattggtacgtttgcggcgatgtacctgtgcggattcagtctcaataacctttcgttaatggcgctcaccatcgctactggtttcgtggtggatgacgccatcgtggtgctggaaaacattgcacgtcatctggaagcgggaatgaaaccgttgcaagccgcactgcaaggtactcgcgaagtcggttttacggtgctgtcgatgagtctgtcactggtggcggtgttcctgccgctgctgttgatgggcggattgccgggccgactgttacgcgaatttgccgtgacgctttctgtcgccattggtatatcgttgctggtttctctgacattaacgccaatgatgtgtggctggatgctgaaagccagcaagccgcgcgagcaaaagcgactgcgtggttttggtcgcatgttggtagccctgcaacaaggctacggcaagtcactaaaatgggtgctcaatcatacccgtctggtgggcgtggtgctgcttggcaccattgcgctgaatatctggctgtatatctcgatcccgaaaaccttcttcccggagcaggacactggcgtgttgatgggcgggattcaggcggatcagagtatttcgtttcaggcgatgcgcggtaagttgcaggatttcatgaaaattatccgtgacgatccggcagtggataatgtcaccggctttacaggcggttcgcgagtgaacagcgggatgatgtttatcaccctcaagccacgcgacgaacgcagcgaaacggcgcagcaaattatcgaccgtctgcgcgtaaaactggcgaaagaaccgggggcgaatctgttcctgatggcggtacaggatattcgcgttggtgggcgtcagtcgaacgccagctaccagtacacgttgttatccgacgacctggcggcactgcgagaatgggagccgaaaatccgcaaaaaactggcgacgttgccggaactggcggacgtgaactccgatcagcaggataacggcgcggagatgaatctggtttacgaccgcgacaccatggcacggctgggaatcgacgtacaagccgccaacagtctgttaaataacgccttcggtcagcggcaaatctcgaccatttaccagccgatgaaccagtataaagtggtgatggaagtggatccgcgctatacccaggacatcagtgcgctggaaaaaatgttcgttatcaataacgaaggcaaagcgatcccgctgtcgtatttcgctaaatggcaaccggcgaatgccccactatcggtgaatcatcagggattatcggcggcctcgaccatttcgtttaacctgccgaccggaaaatcgctctcggacgccagtgcggcgatcgatcgcgcaatgacccagcttggtgtgccttcgacggtgcgcggcagttttgccggcacggcgcaggtgttccaggagacgatgaactcgcaggtgatcctgattatcgccgccatcgccacggtgtatatcgtgctgggtatcctttacgagagttacgtacatccgctgacgattctctccaccctgccctcggcgggcgttggagcgctgttggcgctggagctgttcaatgccccgttcagcctaatcgccctgatagggatcatgctattaatcggcatcgtgaagaaaaacgccattatgatggtcgattttgcgcttgaagcccaacggcacggtaacctgacgccgcaggaagctattttccaggcctgtctgctgcgttttcgcccgattatgatgactaccctggcggcgctgtttggtgcgctgccgctggtattgtcgggcggcgacggctcggagctgcggcaacccctggggatcaccattgtcggcggactggtaatgagccagctccttacgctgtataccacgccggtggtgtatctctttttcgaccgtctgcggctgcgtttttcgcgtaaacctaaacaaacggtaaccgagtaaatgacagatcttcccgacagcacccgttggcaattgtggattgtggctttcggcttctttatgcagtcgctggacaccaccatcgtaaacaccgcccttccctcaatggcgcaaagcctcggggaaagtccgttgcatatgcacatggtcattgtctcttatgtgctgaccgtggcggtgatgctgcccgccagcggctggctggcggacaaagtcggcgtgcgcaatattttctttaccgccatcgtgctgtttactctcggttcactgttttgcgcgctttccggcacgctgaacgaactgttgctggcacgcgcgttacagggcgttggcggcgcgatgatggtgccggtcggcagattgacggtgatgaaaatcgtaccgcgcgagcaatatatggcggcgatgacctttgtcacgttacccggtcaggtcggtccgctgctcggtccggcgctcggcggtctgctggtggagtacgcatcgtggcactggatctttttgatcaacattccggtggggattatcggtgcgatcgccacattgctgttaatgccgaactacaccatgcagacgcggcgctttgatctctccggatttttattgctggcggttggcatggcggtattaaccctggcgctggacggcagtaaaggtacaggtttatcgccgctgacgattgcaggcctggtcgcagttggcgtggtggcactggtgctttatctgctgcacgccagaaataacaaccgtgccctgttcagtctgaaactgttccgtactcgtaccttttcgctgggcctggcggggagctttgccggacgtattggcagtggcatgttgccctttatgacaccggttttcctgcaaattggcctcggtttctcgccgtttcatgccggactgatgatgatcccgatggtgcttggcagcatgggaatgaagcgaattgtggtacaggtggtgaatcgctttggttatcgtcgggtactggtagcgaccacgctgggtctgtcgctggtcaccctgttgtttatgactaccgccctgctgggctggtactacgttttgccgttcgtcctgtttttacaagggatggtcaactcgacgcgtttctcctccatgaacaccctgacgctgaaagatctcccggacaatctggcgagcagcggcaacagcctgctgtcgatgattatgcaattgtcgatgagtatcggcgtcactatcgccgggctgttgctgggactttttggttcacagcatgtcagcgtcgacagcggcaccacacaaaccgtctttatgtacacctggcttagcatggcgttgatcatcgcccttccggcgttcatctttgccagagtgccgaacgatacgcatcaaaatgtagctatttcgcggcgaaaaaggagcgcgcaatgaagttctggcgacccggtattaccggcaaactgtttctggcgattttcgccacctgcattgtcttgctgatcagtatgcactgggcggtgcgtatcagttttgagcgtggctttattgattacatcaagcatggtaatgaacagcgattacaactgttaagtgatgcgcttggcgagcagtatgcgcagcatggcaactggcgcttcctgcgcaacaatgatcgctttgtctttcagatcctgcgttcatttgaacacgataattcggaagataaacccggcccgggtatgccaccgcacggctggcgtacccagttctgggtggttgatcaaaacaacaaagtgctggttggtccgcgagcgccgattccacctgacggtacacggcgacccattctggtcaacggtgcggaagttggcgcggtgatcgcctcccccgttgagcggttaacgcgcaatactgatatcaatttcgataaacaacagcggcaaaccagctggttgattgtcgccctggcaacgttactcgcggcacttgccacttttctgctggcgcgcggtttactggcaccggtaaaacgacttgtcgatggcacgcacaaactggcggcgggcgatttcactacccgcgtaacgcccaccagtgaagatgaactgggcaaactggcgcaagacttcaaccagcttgccagcacactggagaaaaaccagcaaatgcggcgcgattttatggccgatatttctcacgaactgcgtacgccattagcggtgctgcgcggtgaactggaagccattcaggatggcgtgcgtaaattcacgccggagacggtggcgtctttacaggcggaggtcggtacactgaccaaactggttgacgatctccatcagttgtcgatgtctgatgaaggcgctctcgcctatcaaaaagcaccggtagatttgatcccactgctggaagtggcgggcggcgcatttcgcgaacgattcgccagtcgtggcctgaaactgcaattttccctgccagacagtattaccgtatttggcgatcgcgaccgtttaatgcagttattcaataacttactggaaaacagcctgcgctacactgacagcggcggcagcctgcaaatctctgccgggcagcgcgacaaaacggtgcgcctgacctttgccgacagtgcgccaggtgtcagtgacgatcagctacaaaaattgtttgaacgtttttatcgcaccgaaggttcccgcaaccgtgccagcggcggttccgggctggggctggcgatttgcctgaacattgttgaagcacataatggtcgcattattgctgcccattcgccttttggcggggtaagcattacagtagagttaccgctggaacgggatttacagagagaagtatgaccgagttaccaatcgacgaaaacacaccgcgtattttgatcgtggaagatgaaccgaagctggggcagttgctcattgattatctgcgtgctgcgagctatgcgccgacgcttatcagccacggcgatcaggtactgccgtatgtgcgccagacaccaccggatctgatcctgttagatctgatgctccctggcaccgatggcctgacgctgtgccgggaaattcgtcgtttttctgacattccgatcgtgatggtgacggcaaaaatcgaagagatcgatcgcctgctggggctggagattggcgcagatgattatatctgtaagccgtacagcccacgggaagtggtagcgcgcgtcaaaaccattttgcgccgttgcaaaccgcagcgcgagttgcagcaacaggatgctgaaagcccgttgattatcgacgaaggtcgttttcaggcttcatggcgcggtaaaatgcttgacctgacgcctgcggaatttcgtctgctgaaaacgctctctcacgaaccaggaaaagtgttctcccgcgagcaattgctcaatcatctttatgacgactaccgcgtagtaaccgaccgcaccatcgacagccacattaaaaacctgcgccgcaagctggaatctctcgacgccgaacagtcatttatccgcgccgtttatggcgtcggttaccgctgggaagccgacgcctgccgcatcgtttagttttagcgacattattttgttagccggagatggcgttcagaccagatccggcaacattatcccacgcatggtcagcaaactgacattatctctccgccctggcaggcatcagaaaatcgctcatactttaatcggtaaacagcacctttagatgctgttttcgatacacaatttcaatcaaggagtcattatggctggttggtttgaactcagtaagagcagtgataatcagttccggtttgtgctaaaagcgggcaatggtgagactatcctcaccagcgagctttatacctcaaaaacctctgcggaaaagggcatcgcgtcggtgcgtagcaacagcccgcaagaagaacgctatgagaaaaaaacggcaagtaacggcaaattctatttcaatctgaaagccgctaatcatcaaattatcggctccagccagatgtacgccaccgcgcaatctcgtgaaaccggaattgcctccgttaaagccaatggcacaagccagacggtgaaagacaatacgtaattacgatgccgggcgtgggttgttggcgtccggcgctttaccagagccccccacagcgctacaatgcccgcccttaaagtgggggcactcccctaaccgcttcatcaggtgaagcggatctgacctgtcatcagaacgagagaattatgtttaaaccggaactcctttccccggcgggaacgctgaaaaatatgcgttacgctttcgcttatggcgcagatgctgtttatgcgggccagccgcgttattccctgcgtgtgcgcaacaacgaattcaaccacgaaaatcttcagctcggcatcaatgaagcccacgcgctggggaaaaagttttatgtcgtggtcaacattgcaccgcacaacgccaagctgaaaacctttatccgtgacctgaaaccggtggtggaaatggggccggatgcgctgattatgtccgatccagggctgattatgctggtgcgtgagcacttccctgaaatgccgatccacctttcggtgcaggctaacgccgtgaactgggcgacggtgaaattctggcagcaaatgggcctgacccgcgtgatcctctctcgcgagctgtcgctggaagagattgaagagatccgcaatcaggtgccggatatggagatcgagatcttcgttcacggcgcgctgtgcatggcctactccggtcgctgcctgctctctggctatatcaacaagcgcgacccgaaccagggcacctgcaccaacgcctgccgctgggagtacaacgtccaggaagggaaagaagatgatgttggcaacatcgtacacaagtacgagccgattccggtgcaaaatgttgagccgacgctgggtatcggcgcaccaaccgacaaagtgtttatgatcgaagaggcccagcgtccgggcgagtatatgaccgcgtttgaagatgagcacggcacttacatcatgaactcgaaagatctgcgcgccatcgcccatgtagaacgcctgaccaaaatgggcgtgcattcgctgaaaatcgaaggtcgtaccaaatctttctactattgtgcacgcaccgcacaggtttaccgcaaagctatcgatgacgccgctgcgggaaaaccgttcgataccagcctgctggaaactctggaaggtctggcgcatcgtggctataccgaaggtttcctgcgtcgtcatactcacgacgattatcagaactacgaatacggttattcagtttctgaccgccagcagtttgttggtgagtttaccggtgagcgcaagggggacctcgcggcggtagcggtgaaaaataaattctccgttggcgacagccttgagctgatgacgccgcaaggcaacattaattttacccttgagcacatggaaaacgccaaaggcgaagctatgccgatagcaccaggcgatggttatactgtgtggctcccggtcccgcaggatcttgagctcaattacgcgctgctgatgcgtaatttctccggggaaaccacgcgtaatccccacggtaagtgattaatttcgattatttttcccggatggaaaattcttagaaaccgatcacatacagctgcatttattaaggttatcatccgtttcgctgaaaaacataacccataaaatgctagctgtaccaggaaccacctccttagcctgtgtaatctcccttacacgggcttattttttacgcgtaatacaatgaaataaaaggatttatttctggtcacgtccacacattgaccacatcgacaaaaaagcccctcgactgaggggcttcctgtttctaattacatccacataatttgctgccctgacggcaacgggtgcggccttacgacgtggacttctcccggcttcacaatgtatcgctgtaccgactcataagtgatgaacgtggcgctgcaattcacgttctgacactggtgataacgctcttttgtcgtgtcagtgatatagcggcttgtacgcgcatgtgcggcatgctggcataaaggacaatgaaacatcgcgagcacctcttccggttttgttgatggtgccattttagttaatttacccttacaaaacaaacagataaaataaaaacatcactcattatcttctgtttcgtaccccacatcagaaagcctgacctcaagctctaatgacgtcgtgaagccgctattattcagaaaatgtgtcaccttagtgattgtccagtcctgctcgtctatgacgcgcttaaagccagacactttgaccggtgtttccgtgtaaatatctgcccgaccggtagccaggctgatggagaactctgctacacgggcttatttttttatgcataagccctatctctggtaaccgtcttccattgaccacatcgatagaatcctccttcatagcacgatgcctttcacttatcggcatcgtgctcccacaggttccggctacgcacagccagaacgcgcatatttgacgcttaccaaaaaatattctcactctccacatttgaatgtcagacgagcgacaccatgtaatcctacaccttctgtcttcagctcaactatttgcatttttttgccctgagtaacacagaaatgagttgcatcattttttactatattttctgcaccagatattctacccctggctaaagaagcttcggcttcggtgtagtattggttatcgagtttacgctgaatattacttttatatgcaagaccaaatttaccgatacttgtctcatcattatgcacagcacaaccagacataataaaaatactaattaatgatatagcagctatctttttcatctcaccttcccccattaaataccaacgacactctctagtgtttaaatataataatggcatgattattataattgaataggattataataaatgttctgtacaacatttcctacataagtaggaattacggacattgaggcccttcagggtaactccatgggggctttaatatattatattgaagatgccactgtttagttgaatattaggtatatgctcttttttgaaatttatcggtggcagccgttagtattcgctgtccccattgcaagctcctggtggtaaccactgaatcctccatacttgaactgactttttatcctccgactttcatcctgttctgactccaccttttgttttctgctctacactatctacagaccaatcataaaggcacatacgatcatggcagaatttcccgccagcttactgattcttaatggcaaaagtactgacaatctacccttgcgcgaagcaattatgctgttgcgtgaggaaggaatgacgatccatgtgcgggtcacctgggagaaaggcgatgccgcacgatatgtagaggaggcccggaagtttggcgtcgcaacggtgattgccggtggtggcgatggcaccattaatgaagtttctacggcgttgattcagtgtgagggggatgacatacccgcgctgggaattttgccattaggaaccgccaatgattttgccaccagtgtagggattcctgaggcactggataaggcgctgaaactggcaattgccggtgacgccattgcgatagatatggcgcaggtcaacaaacaaacctgttttattaatatggcgacaggcggatttgggacgcgtattaccacagaaacgccggaaaaattaaaagccgcgctgggtagcgtctcttacatcattcatggcttaatgcgtatggatactctgcaaccggaccgttgtgaaatccgcggtgaaaactttcactggcaaggtgacgccctggtcattggtattggtaacgggcgtcaggccggtggcggtcagcaattgtgtccgaacgcgttaattaacgatggcttgctgcaactgcgcatttttaccggcgatgaaatacttccggctctcgtatcaaccttaaaatctgacgaagataacccgaatattatcgaaggcgcttcgtcgtggtttgatattcaggcaccacacgacatcacctttaatcttgatggcgaaccgttgagtgggcaaaattttcatattgaaatacttccggcagcgttgcgttgtcgattaccaccagattgtccactgttgcgttaatcaaactattctctcttgaaccagggagaatccgtaatgccggatgcggtgtaaacaccttatccggcatacagaacaatactacaccgtaattaattttacccgcgtcttctgcaatgccagtttatccacctctgacacagcatcatcggtaataataatgtcaattttttcgattggtagtacctgattaaaaccgcgacggttaaatttcgatgaatcgagaacggcaatcactttattagcggctgtgaccatcgcaccgctaatagaataaccttcattaaaggtcgtaataccattaaccgcatcaataccatcagcaccgacaaacattaaatcggcattaatatcctgtaatgaacgctcggcaatggaaccatgcatcgagcgcgttttatggcggaccgtgccaccacagacgaccagagtaatgtctttattttcggaaagggcaaacgctgccgggagactgttggtaatcaccgtgatatttttggcggtcattaatccttcggcgataagcattgtcgtacttccgctgtcgagaataacggtctgatcttacccagcaatagtggacacgcggctaagtgagtaaactctcagtcagaggtgactcacatgacaaaaacagtatcaaccagtaaaaaaccccgtaaacagcattcgcctgaatttcgcagtgaagccctgaagcttgctgaacgcatcggtgttactgccgcagcccgtgaactcagcctgtatgaatcacaactctacaactggcgcagtaaacagcaaaatcagcagacgtcttctgaacgtgaactggagatgtctaccgagattgcacgtctcaaacgccagctggcagaacgggatgaagagctggctatcctccaaaaggccgcgacatacttcgcgaagcgcctgaaatgaagtatgtctttattgaaaaacatcaggctgagttcagcatcaaagcaatgtgccgcgtgctccgggtggcccgcagcggctggtatacgtggtgtcagcggcggacaaggataagcacgcgtcagcagttccgccaacactgcgacagcgttgtcctcgcggcttttacccggtcaaaacagcgttacggtgccccacgcctgacggatgaactgcgtgctcagggttacccctttaacgtaaaaaccgtggcggcaagcctgcgccgtcagggactgagggcaaaggcctcccggaagttcagcccggtcagctaccgcgcacacggcctgcctgtgtcagaaaatctgttggagcaggatttttacgccagtggcccgaaccagaagtgggcaggagacatcacgtacttacgtacagatgaaggctggctgtatctggcagtggtcattgacctgtggtcacgtgccgttattggctggtcaatgtcgccacgcatgacggcgcaactggcctgcgatgccctgcagatggcgctgtggcggcgtaagaggccccggaacgttatcgttcacacggaccgtggaggccagtactgttcagcagattatcaggcgcaactgaagcggcataatctgcgtggaagtatgagcgcaaaaggttgctgctacgataatgcctgcgtggaaagcttctttcattcgctgaaagtggaatgtatccatggagaacactttatcagccgggaaataatgcgggcaacggtgtttaattatatcgaatgtgattacaatcggtggcggcggcacagttggtgtggcggcctcagtccggaacaatttgaaaacaagaacctcgcttaggcctgtgtccatattacgtgggtaggatcagtcatcccttcgtggatcattttgactgccgcctgcgctattctgttttttggcgcgctggcgagctgaaatcgctctttaaacccgacttcctgggtctcggtttcactattaccagacattattttcgccgcaccgccatgaaagcgcgtaaccacgcctttttgttcgagaaagcgcaaatcggcacggattgtcgcttccgaggcagcaaatactcccgccagatcctgaacaagcacggttccctgttcattcactaattggatgatcttattccttcgctcgaatgaattcatcgtcatttacccatattcaattgtggctagtgtaaacgaagggggaccattggtgaatgatctgttttgcacaataccgggccagcatcacgctggcccgcggtttcagggaatgagcaacactttgcccggcatagcattacgagcgatgtcacgcaccgcctgggcgaagctttcaaagcttccacggtgagcgattaatggctccaggcttaacttacgttctgtcagcaaccggctcgccgtttcccactcctgccccggccaagggctggagtagttcatccaactgccgataaccgtcagctctttacgcaatattttgccaaacgttgccgatgttaaatgcagatcctgatgcaacgtgcccaccagcgccagttgggcatgaggaccggcaatctctaccgccagttcgacagtttgcggtacgccagccgtctcgaggataagctgattaaagcgcagttcgcgtaaaacgctctgcatttgcggcgcgctcatttcgctactgttaaatgtttgcatcgcaccgaaagattttgccagtgccagtttttctgaactaatgtcgatcgccgtcacactctttgctcccagcgcgacagcgcactgaatggccagcaggccaatggttccggcaccaataataataacgtttttattctcacaaccttgcgctaaatgaaaagcatgcagaccaacggtaatcggctcaataaaagccccatcctcaataggcatatccgtgggtagagcaaagacattttttcgcttaacgacaatatattcagcaaatccaccatcacgccgcgagccaataaaatcatattttgcgcactgggaataaaaccctttcagacactctggacaagtaaaacagggtaataacggcacacaggcaaccgcatcgccagggtgtaaatcatcaacaccggatcccaccgcatcaatatagccgctaaattcatggcctaacgttattggataataatgtgcaccatttttaaatatcctgggtaaatcggaaccacataagcccgagctggcaatttttacccgcacctcatcctgatgtttaatttcaggaatgacgctttctgcaacgcgcacgataccatcagtatcattcaccactgatttcataaaaactcctgattgttaagggggataacctccccctcaggtaaaaattattctgcgagaacgactttctcttgtttaataaagccacgcgctctacgccaggtcatgaaaataccggtcagataaattgcaccgataataatgaaaccgggaatattttgcggggagaaaacctgaatcagtaaccaggtaatgggagaaccgccctgatccattgaagccaccatacccccggcttttaacgccccagcattagccgccagttgggtgtgcaaaccaatagtttgcgtcgcgatccacagggtgatgctcataatgatgacacccgagattaaggtgcggaacagatttccacgatgcacggcgaccgccatcgccacgaagaagccgatggtggcaagatcgccaaacggcagcacctgattacccggcacacaaacagcaattaaaatggtgagtgggataaaaatcaggcttgccgataccaccccgccgtatgtcccagcagcaacgccggatcaaggccaatcaggaactcctgaccgccgaacttcgcctgtaaacgactacgagcctgcttagcgatgggcgttaaaccatccatgatgggtttaatcacccgtggcattagcagcatcactgccgccgtttttaccgccagctgcaatacacctttgacatcgtaacccgcgaggatgccgataatcagccccatcacaaaacccacggtgacaggctcgccaaatggaccaaatttgcgctgaatatcgtcggcgctaaatttaattcggttaacgcctgggattttctcgatgatagcatcgaccagcaccgcaatcggccccatatacgccgacgtaccgtgcggaatagcaataccttccagctcaaagaaatttcgggtatcgcgggcaaaccagtcgccgagcttataaacaaacgccgcgtgaattaccacacctgccatccctatcatccatgaaccggttgccagatgcagcaacgcgccggtgaaggtcatatgccagatattccagatatcaacatttaccacccgcgtcatacgggtcagtaacatcgccacgttaaccagaatcgcaatcggaatcgccaccagcgcaatttgcgacgcccaggtcattggtgaagagcccggccagccaacatcgaccacatgcagattcaggtcgaaattttccgccatcgctttcgccgccgggccaatggaatccagcattaagccaatcacaaggccaatgccaacaaagccaatcccgatatgcagacccgctttaaagcaatcgcctgccttcatgcctaatattttagaaaaaataatgatgacaatcggcagcatcaccgtagggccgaggtcgagaatataacgcatgacttctgaaaacataggtcacccctgtaagatagtcagaattttattttgtaatgcttcgataccgataccagaaataaaaggcatgccgtgaactaacggaatatcgccaaaactacgatccactttggcagtggtgcatatcaaatgcacaccatccatataggtttctatttcattaacccgacactggattaattcaacaggaatattatgattctgacacaactctttaatttcttccgccgccatcgtagaggtcgcaaccgcgcctccgcaagcgacaataatcttgcgtttcataaatagtcctttttattgttacagagggatttattcgtctgaatctaaaacatactttgtgaagtattcctttaactgggtttcaggaagagtgattagtgtctcgacgatatcgggctgttgtaacttgccaaataaacagcgtaaaagtttcaattgctgctgcggattttccacaatcaacgcaataaccaacgataccgccacgtcgttatcatcatccgcttgctgaaaatgaactttatttgttggccttaacagataaatggctgacgacttagcatgaatcgcctcacaatgcggtattgcaatagcgtgctgctcaagcattatcccggtagggaattctgcttctctggcaattaatgcctgtggccaggtatcatgaaccacacctttggcgagcatctcattaccgatatgggttaaaacttcgctacgatcgacaaaagaaattccgctacgaacaaacaggttagtcatataccgtccttattccgcacagccgtagcgataggcgcgcaaaacatcataaattttatccataatcagctgatgcggtattgctgataattccccggactgaatgcgttcaaattgtttgggaagatactgactaatcatgcccagtgggatgtccacgccttcaagattcaccatcatcgtttcgacgctatttttaatccgactatgcggccagtaataacgaatacgatccgacaggctgtaacgaatatccagtaatgaatcgttaaaacccgtacgataatattttttccagtattgcggttcgtcgagcatcacttcttcaattaccgccaggcaaccgctgcgattttcaggggcgataagttcctgctcaatttgtgccagtgcaaatatcgcctcgcgtaaagcaaaggttaatgcgggaccgactttcaatattgcaaagtgatcgcggactaattcccaataagccgtccgggtctggtaatcggtagaatgtgcttcataaaccattcgggtgttttctatccattgcgccagcggctgcgcttcctgcggctgataatggataatattgctgtgatcaaattccacacccggctgcaccacgatggcaatcacacgtgttaacgcctctgtcagcccacgggcaataaaggccttttgatgcgtacgtaaagtattggcggcatcttcaacatgggtgatgtgtactgactgaatggcgctggcctcaccgcccggaaccggaacttcggtgccaatgacatagctcagttgctcacgctggcaatctgtcgccacactttccgcagcaaagcaaagcacagcagctcgttccgcaaccgtttctggtgctaacggtatgggatcccccgcgcaggacattgacgcatcaagatgaattttactgaagccggcacgaacatattcctttaccagctcgacggatttttccatcgccgcatccgcattttcttgctgccagcagtttggccccagatgatcgccgccgagaataatgcgttcgcgtgcaaacccaactttatcggcaatcgtaaaaacaaattcgcgaaagtctgccggtgtcattccggtataaccgccaaattgattgacctggtttgacgttgcttcaatcagcactttgcgcgtgctgttgcgatcaaatgccagcgccgcttcgataaccaacggatgggcagaacagactgaacatatgccgatatgttcaccagctttatgccgggcaattaacgttttcatgttttttccttgttaaatggcaggtgcgttatgccctgccctcgcagccacaatcggcaatcactttgctcaccacatcgcgcattgcggatttagccgactgcaaataatcccggggatcggtcgcttcagggtgctcggtcaggtaattttttaacgcctgcgagaaggcatttttcagctccgttgcaacgttgattttgcatatccccagtttgatggtttgctgaatatccttagtcgataaccctgacgcgccatgcagcaccagcggtaagttcacccactggcgaatgttctccagtctagaaaaatcaagcgccggtgcgctggcatacatcccatgagccgtgccgatggcgaccgccagggaatcaattccggttgcctcggcaaattcacgcgcctgagcggggttggtgtacaacgcatcggcttcattgacttgcacatcatcttcctggccgccaagttgccccagctccgcctcgacgctgacatcaaagcgatggcaaaaatccaccacctctttgacccgtgaaatattttgcgcaaaaggcaaatgcgaggcgtcaatcatgactgagcgcacgccagaacgaaccttctgagcgatatcgtcaaatttcgtgtgatggtcgagatgaattgccagtggatggtgatattgcttcgccatcgcgctgaccagcgccaacagattttctgtaccagcatgagtaaatgtgccaggcgttccggcgatgatgaccggcgcatgcaggttggcagcggtttctaccaccacttgcatcgtttcgagattgtgaatattgaatgccggaaccgcataaccgccgcgctgtgcgttgttcagcatctgctttgtcgataccacgtacattttcatatcctgtcgtttgttttcgatttcaaaatataatgaaattatttgtttttaaatatcgagataacgatcacaaaaacgacaatatgaaaattattcgaggagtgaaaggcaaaaaaacggcctcccgatagggaagccgtagcaaagtgcgcgtgtttttatgccggatgcggtgtaaacatacgtggcagtgctatgtaggcatgataagacgcttcagcgtcgcatcaggcataggttgccggatgcagcgtaaacgccttatccgtcctacggggtggtgttgttcgtataaggcgtatcaggcgatagtaattttgctatcgagataaacgtcctgcacggcgttaatcagtttcacgccgtcagccatcgatttcttgaacgctttacgtccaagaatcagccccattccgcctgcgcgtttgttgataaccgcagtacgcactgcatcgctgaggtcagtttcaccgcccgcagcaccgccggagtttatcaacccagcccgacccatatagcagttagctaactgataacgcaccagatcaatcgggttttcgctggtcaatttgctgtaaacacgatcgtcggtgtaaccgtaattaattgctttatagccgccgttattttccgccattttttgtttgacgatatctgcaccgatggttgccgccagatggtttgcctgaccggtcaggtcggcggaaacatggtaatcaacgccatctttcttaaaggcggagttacgcaaataggcccacagcactgtcaccatacccagctcgtgcgcacgttcaaaagccgcagaaatttcttcaatctggcgacgtgactcttccgagccaaaatagatagtcgcaccaaccgcaaccgcgcccatgttgaacgcctgctccacgctggcatacagcgtttgatcgtaggtattcgggtaacttagcgtctcgttgtgattaagtttgacgaggaatggaatgcgatgcgcataacgccgcgataccgacgccagcacgccgtaagttgacgccacacagttacagcccgcttcgatcgccagttcaacaatgtttttcgggtcaaagtagagcgggttagcagcaaatgaagctccggcagagtgctcaacgccctggtcaaccggcagaatagaaagatatcctgtgccagccagacgcccggtgttgtacaacgtctgcatattacgtaacaccgctggcgggcgattattgtcaatcattacgcggtctacgtagtcatgtccggggagataaagctggtcagaaggaattgtcatacaacggtgctgtaaaaggttgtcggcgtctttgccaagcaactgcgcaatatctgtcattactatgctcccgtaaattccgattggatatcggctatggattgtcctggcccgccttttgcgggcaatcataatcctggtcgttacgggcgagtttttccatcttttggatgttttttcagcgttttctgttggctcgattcatcagaaaaaatgttagcgcggtcaagttttcaccgcaaaggtatttaaaaggtattattaagtggtattgtcatcgcgtaccttacattacctgtcatgaaggaattaaaagatgaaaacaacagcaaagctgtcgttcatgatgtttgttgaatggtttatctggggcgcgtggtttgtgccattgtggttgtggttaagtaaaagcggttttagtgccggagaaattggctggtcgtatgcctgtaccgccattgcggcgatcctgtcgccaattctggttggctccatcactgaccgctttttctcggcgcaaaaagtgctggcggtattgatgttcgcaggcgcgctgctgatgtatttcgctgcgcaacagaccacttttgccgggttcttcccgttactgctggcctactcgctaacctatatgccgaccattgcgctgactaacagcatcgcttttgccaacgtgccggatgttgagcgtgatttcccgcgcattcgtgtgatgggcactatcggctggattgcctccggtctggcatgtggtttcttgccgcaaatactggggtatgccgatatctcaccgactaacatcccgctgctgattaccgccggaagttctgctctgctcggtgtgtttgcgtttttcctgcccgacacgccaccaaaaagcaccggcaaaatggatattaaagtcatgctcggcctggatgcgctgatcctgctgcgcgataaaaacttcctcgtctttttcttctgttcattcctgtttgcgatgccactagcgttctattacatctttgccaacggttatctgaccgaagttggcatgaaaaacgccaccggctggatgacgctcggccagttctctgaaatcttctttatgctggcattgccgtttttcactaaacgctttggtatcaaaaaggtattattgcttggtctggtcaccgctgcgatccgctatggcttctttatttacggtagtgcggatgaatatttcacctacgcgttactgttcctcggtattttgcttcacggcgtaagttacgatttttactacgttaccgcttacatctatgtcgataaaaaagcccccgtgcatatgcgtaccgctgcgcaggggctgatcacgctctgctgccagggcttcggcagtttgctcggctatcgtcttggcggtgtgatgatggaaaagatgttcgcttatcaggaaccggtaaacggactgactttcaactggtccgggatgtggactttcggcgcggtgatgattgccattatcgccgtgctgttcatgatttttttccgcgaatccgacaacgaaattacggctatcaaggtcgatgatcgcgatattgcgttgacacaaggggaagttaaatgaaaacagaacgtattctcggtgctctttatgggcaggcgttaggggatgcgatggggatgccctccgagctttggccacgcagccgcgttaaagcacactttggctggattgaccgttttcttcctggaccaaaggagaataacgcggcctgttattttaaccgcgccgaattcaccgacgatacctcgatggcgctgtgtctggcggatgcgttactggaacgtgaaggcaagatcgatccggatctgattgggcgtaatattctcgactgggcgctgcgtttcgacgcctttaacaaaaacgtactaggtccgacctcgaagattgcgcttaacgccattcgcgacggtaaacccgttgctgaactggaaaacaacggcgtgaccaacggcgcagcgatgcgcgtctcgccattaggttgtttgcttccggcgcgtgatgttgattcctttattgatgatgtagcgctggcgtccagcccgacccataaatccgatctggcggttgcaggcgcggtagtcatcgcatgggcgatttctcgtgccattgacggagaaagctggtcagcgattgttgattccctgccttcaattgcgcgacatgcacagcaaaaacgcatcactacgttcagcgcctcactggcggcgcggctggagattgcgctgaaaattgtgcgcaatgccgacggcaccgaatccgccagcgaacagctttaccaggtcgttggcgcaggtaccagcactattgagtccgttccgtgcgccattgcgctggttgaactggcacaaaccgacccgaatcgctgcgccgtcctgtgcgctaaccttggcggcgacacagacaccatcggtgctatggcgacggcaatttgcggcgcgttgcatggcgttaacgctatcgatcctgcgttaaaggcggaactggatgcggtaaatcagcttgatttcaaccgctatgccacagcgctggcgaaatatcgtcaacaacgggaggcggtatgagcggcgctcgattacacacgctgctgcctgaattaaccacgcgtcagtcggtgatggtcgtcggcgcggcggtcattgacgtgatcgccgacgcttatgccctcccctggcgtgggtgcgatatcgaactgaaacagcagagcgttaacgttggcggctgcgcactgaatattgccgtggcgttaaagcgcctcggcatcgaagcgggtaatgccttgccgctcggtcagggcgtgtgggcggagatgattcgcaaccggatggcaaaagagggcttaatcagcctgatcgataacgccgaaggtgataacggctggtgtctggcgctggttgagccggatggcgaacgcacttttatgtcattcagcggtgttgaaaatcagtggaatcgccagtggctggcgcgattaaccgttgcgcctggcagcctgctctatttttccggttatcaactggcctcgccctgcggcgaattgttagtggaatggctggaagagctgcaagacgtgacgccgtttatcgattttggcccacgtattggcgatatcccggatgcattactggcgcggatcatggcctgtcgacctttagtgtcgctcaatcgtcaagaggctgagattgccgccgaacgttttgctttatccgcagagataacaacacttggcaagcaatggcaggagaaatttgccgcgccgttgatcgttcgtctcgataaagaaggcgcatggtatttcagcaacgacgcttctggctgcattccggcatttccaacgcaagttgtcgacaccattggggcgggcgacagtcatgccggtggcgtacttgccgggctggcctctggtctgccactggcggatgccgtattactgggcaatgcagtggcgtcgtgggttgtcgggcatcggggcggtgattgtgcgccaacgcgcgaggaactactcctcgcacacaaaaacgtatagatcgctgcgacagtggctaatgctgtactcaataggccgttgctgttggtcaagcgccacttgcttgatcaccagcaccggtattttgctatctaactgaatatgtgactgaaactcggcatccggcatccgggcgctaacgcgggaacgcgtacgttgtgggtaaatgtgctggctgcggaaatagtcataaagtgaaatcccgatggcatcaacatcatgaattaaatgcgccggaacccacgattcctcaatcgataccgcttcttcatcgacatagcgaatacgcttaagcaaaaagacatcacttcctgcttcgaccgccagctgctgcgcgacttcttcgggacatttcacgacacgcttgttaacccatagcgtatcgggctttttcccgcgcaataccacctgctgagaaaaacctcgcgcttctttcaacgagtattcgaagatgttgttgatctgcgtgccgtaaccgcgcgaacgcgtcaccacaccctcttcttccagcgcctgcatcgccttgcgcaccgtaatgcgcgaaacgccggttaactgacttaaatcacgctcaccgggcaaaatattgccatgctccagcaccccgctgcgcacggcattttttaccgtttcggcaaacttaatataaagcggcgtgttatccgccgctaaaatacgctcgttcagttgggcaatcagctgggtatgcgcttgttccatttgtctttttcctgccggggagtctggtgggagtatatcactgcttcttatttaaggcgtttctttaatcccatcaacgaatgcctgcaactcctccaccgtgccattaaatacattaaaatccaccggaccattgatgccatctacctgtccacggtcggaatgctgccagaagcgccaggccattccgtcattgtccggacgacgttgatagtagtgagccacccaccacggatattcattgaaatagcccgccagattggtgtgataaaaaacggctcctgagtaaataatcggctttttccccgtacttttttcgaccatttttagccactgacttacccgcttgcgtaattcttttgccgataattttccccgttcttctacgtccagcacggcagggaaatcgccttgtgagaaatccaccgtttgcagaaataatctcgcctgaactgaagcggataccgacggggagaaataatgatacgccccacgcagcaggccattttcgcggcttagttgccagttacgcgaaaaataggggtccaccagcttttcgccttccgtcgccttaataaaagcaaactgtaagcggataccattgtcgcgcatttttgccacccgctgccagtcgatccgctcctgccagcgcgaaacatctattccgtgaatggtgtaactggcaggaatgcgaatagcgaaagatttaaccgggcgataaccgtagaagtggatgtagtctgtaatctgaactgctgtcgaatagaaaaaattcaccgtctgacgcggataaattgcaacgatggaaattagcccaagagcgcataatagagaggtgagtttttttcgactggtaattcttagctgcattggtttcatccctgaatgtcagtgccaaaggctgacaataaccaaagcagctatagtacggtgctcaccaccaggcgtggaagtggtgaaccggaccaataccgtgaccaacttccagcgtgtcggcctgggctaacgccgatgaaagccagctttttgcctcctgtacggtgtcagcccagtttgtatggcgcgggcgtagtgcagccaacgccgcagagagtgtacaaccagtgccgtgggtgtttttggtcataatgcgcggtgcggtaaaccgttgttcaccctcgcgggtaaacagccagtccgggctttgctcatcatccagatgaccacctttcattagcactgcgccacagcccatcgccaacagcgatcgcccttgttccagcatttcctgttcggtgcgcgcgtgtggcgcgtcgagcaaggcggcagcttcgggcaagtttggcgttattaatgaaacctgtggcaataatcgactgcgcagcgtagcaaccgccgaaggtgaaagcagcgggtcgccgctttttgccagcataacggtgtcgagtaccacgttttggatctgataacgttgcaaccgttctgccaccgcttcaacaatatcggtttccgccagcataccgattttagtggtatcgattcgcacatcgctgaacaccgaatcgagctgggcggcgacaaaatcaggctcaatgcgatacaccgactgtacgccacgggtattttgcgccaccagtgcagtaataactgagcaaccataagcgccaagtgccgagaaggttttaagatcggcctgaatccccgcaccaccactcggatcagtaccggcaatcgtcagagcgttaattcgtttcatgcctgcacctcctgcgtcaattgccagagcgcatcaaggaaatgtggaacaaaactgcctggcccctcgcttctggcgactgcgcgttctccggcttgtttcatccagtgacaggcagatgcgacattttccagcgtatcgcctggtaacgcacagcaggcagcgacaaccgccgataatgcacagccagttcctaccactttggtcattaacggatcaccaccgtgaataccaatgatacgatgtccatcggtaacataatccatctcgccagtgaccacgacgattgcgccagtttcccgtgccagtgtttgtgcagcgggtatcgcgttagctgcggcgtcagtggtatccactccccgtccgccattagcaatgccagctaatgccatgatttccgaagcattaccacgtatcgctgccggtttaaaagataaaagttcatgacaaaaatggcggcgataatcgagcgcacccaccgctactggatcaagcgtccagggtgtttgagagctttttgcttgctcaacggcagcacgcatcgcctgagcgcgtggctgcgtcagtgtgccaacgttaatcaacaaggcactggcgatagccgcaaactgactggcctcttcggtttcgataaccatcgctggcgatgcaccgagcgccagcaaggtattggcggtaaaggtttgcaccacatcattggtcatgcagtgcacaagaggggaatgttggtgaaaaaggtgtaacgcgtgcgcagattgcgctgaacccagcaggtcgacttgcatagtttgctcctgccataacgtgaagaagcaatgacctggtggtccgtgacttccctacgctggcattatccagatcaggtgatacgggtatttctcagccttcacgcagaagggcaccccgagtcgtttggttgcgatgataaatcgcagaggaggatggtaatgtccagcgcacgcgttgtaaacgaggaaaaacggcagttttacaatcgcgttaataaattatttgatatatgaatccagcaccttcagaacgacatccagatcttcttcacgttttagctcatccccctggtgaacgatgtgttccgtcagatgacctttaatcacttcccgcatcagaccgtttaccgcgccacggatagcagcaatctgttgtaaaactgcagcgcattcgtgcggctcgtcgagcattttcttgagcgccacgacctggccctgaatcttactggcacgcgctttcagtttctgtttatcacggattgtatgagacatggcaacacctggttaacaagaatatgaaaaatcatagcactattaatctactggggggtagtatcaggtactgggggggagtagaatcagattgccgaattaatactaagaattattatcatgaccgaatttacaactcttcttcagcaaggaaacgcctggttcttcatccccagcgccatcttacttggtgcgcttcatggcctggaaccagggcactcaaaaacgatgatggcggcgtttatcatcgccatcaaaggcaccattaaacaagcggtgatgctcggactggcagcaactatttcgcataccgcagtggtctggttaattgcctttggcgggatggtgatcagcaagcgctttactgctcaatcagcagaaccgtggctccagctgatttccgcagtgatcattattagcaccgcgttctggatgttctggcgtacctggcgcggcgaacgcaactggctggagaatatgcacgggcatgattatgagcatcatcatcacgatcacgaacatcaccacgaccatggacatcatcaccatcacgaacatggcgagtatcaggatgcccatgcacgagcccatgccaatgacattaaacgacgctttgatggtagagaggtcaccaactggcaaattttgttatttggcttaaccggtggccttatcccctgcccggcagcaattaccgtgctgttgatatgcattcagttgaaagccctgacactgggcgcaacactggtcgtcagtttcagcattggcctggcgttaacgcttgtcaccgtaggcgttggcgcagcaatcagcgttcagcaggtcgcaaaacgctggagcggatttaacactctcgctaaacgcgccccctatttttccagtctgttgattggcttagtcggtgtgtatatgggcgtacatggcttcatgggcataatgcgataactcaatcctttaggcttgcatgttatcttcagcccaggatgattcttaaatcagctatttccgctgactctctgctcgctaaggatgcttttagggcatcctttcatttacactttttacgaaatcatgggatcactaacaaaatatcgcttgtcagttatattgtatggcaggaaagatatgcgactgatattacagatccccaaagtggagagtttatgaccattaaaaataagatgttgctgggtgcgcttttgctggttaccagtgccgcctgggccgcaccagccaccgcgggttcgaccaatacctcgggaatttctaagtatgagttaagtagtttcattgctgactttaagcatttcaaaccaggggacaccgtaccagaaatgtaccgtaccgatgagtacaacattaagcagtggcagttgcgtaacctgcccgcgcctgatgccgggacgcactggacctatatgggtggcgcgtacgtgttgatcagcgacaccgacggtaaaatcattaaagcctacgacggtgagattttttatcatcgctaaaaaaagccccctcatcatgagggggaaatgcagacaccttgttattttttattattagccacttgctcgtcttgcttgttattagtcgtatttcacgttgattaatgcggttgcctccagtgcgccagatttaactttgtttgtatcgtagacgtagtaactggctgttatcggaattgaaaccgttgtatctgtaagttttgacttcgccgcaacttcctttaaatttgtatatcctttactgctgttagtgatatttaaaagtgtgactggcgaaccattactttcaagaataaatcctacgccattatcttccgcacctttcagtattgtgttgctgttggttaacaagtcagaacttgataaatacacctgcattttccgtgatgtttgattttgttgacctaataaatttttacaacgcagaataatatccccttgtttactatttattgttgctttgttacctgtggctggtaattgtgaaacgggaatactgtctaaagtaattaataaatcgtccggtttgcaggttgtggttatcgggttgtatgacaatgtcagattaaaggaatagacacctgcattttgtgccaatgcatttctgtagctatttacacatgcatcccatgacttgccacctaataaacacagtagaaattgtactgcggcactcccgcgtgtcgatgatgaagcactggataatgtcgcaacaccattaatcatcactgaaccgccgccccccgcagaaacattcacttttgcattactggccgcaggtgtcaccgtaactgaataaccactggtgaaactggtctgattatttgacaacgtgatgttgtttttattggtccattcaaaatgtaaatttaattttatggtatcgttataaagtccaacaataatatccgacgggctcataggggtgatagtatttgtacttacgcatgacgaatcattaaaattatgctcatatgtcgccatttgtgtttgagtaagtgcaaaatccccctgaacaaccaagttgtgctgaacagataactcactataacatgccgcatagctcacaggcataaccatcatcattaatataaatagcattatgcgaatttccatagaaccacctgactattactggcaaatataatttctactttcatcaatctctttaccgaaggtgattgtgcatgaaagtccttgttgcttatcaattgccacattaaccgatggcggtacttcattggtgcgaataaataactgacttccctggccgacaacgccaatattatgaccatggatatcattgacttcataaccaaacgttaatgattgcccatctgctcttaacgcttttataaaccatggcttgcgctgatcggtatcaaaattaaccagtacaaccgcgccgcgataaggggcggcaattttccggttgccacgtaattctgcttcgctatcgctttgcgacacatccagcatcaggtgattttcccgataaggtgtcattccgtcgtatatcaccactccattacggtttgttgtgcgatatttttgcccattgacataagcatctttaattcctggcgcattcatcacagcaaacgtttcggaaagacggttcgccagattaacgccacccgaccaggcgacaatgccccctgaaacactggctccagcctgtcgataagtactcgactgactataactgccattcactgtcgcaaccggcgcgttccaggtcaaattcgccccagctgtcgtttcatttccctgatgttgatgactcaggttgacaccataattgaactgatcccgactccctactgttcctgataatcccgtattatttgaggcaaacccctgatcatcaaacgtcgttgagttagacatatatatttgccgacgaggcgtcgaaacgtcatcaccccaatcaaagggaatcgatataaaaatattaaaacgtttctcttcatgatgattctcgtcataagcctggcttgccgcgagggtatagcttatccgtcgcaggttgttggaataactcaactgataatccttactactgccgctacgcccccagtaatctcgccataacgtacttaatgacacagacccccaaccttctggcaatgactggctcatattggcggaaaagctatttttgcggccaaaatcgttctggtaataatcggcaatgtcatagacatcgttttcatcacggcgataattatctttattgtttgcccaaacgtgatcgttaaatgtccggtaatcacgcgacgaataacgccaggccgccagaccaaaacgcgtcgacgtttggctcacaaatttgttgtaggcaatttgataactttgcccgtcaaacacatcgccgttgtcttgtttactatgcgacttagtggcatcgacggaaatggcaccaatgcgtgtattccagccagcccccaaagtaaacgcgtaataattattcgcgaccatcgagccaccatacagcgtcaataaattattaaaaccatactgataacccgcctggacaaaatcactttgtttgctcgccccttcaatatggctacgacccgccgctaaatcatatttcgacacgccgggttgcagcatatttggcaccgctgcataaggcaccagataggtggttaccgagccgtccgcctctttcacgctgacatcaagatctgctccaccaccggccaactgcaaatctgtaatcgcgaacgggccaggaggaacctctttctgataaaccacaaaaccattctgttcaatagttaccagcgcgttactctgagcaatcccctgcacccgtggcgtaaaattttgtttcgagttaggcaacatctgcatatcacgaaacaaccgcacacctctgaagcgaacagaatcaaaaatatcgcttgatgtgtacatatcacccacgcgaagcgtgccgagaagttgggcaaatccacgttccagatacagggtattgcttttccacacccctggattgttatttgttttactgaaactggcatcagaatgcagttgccaccccagtaaatttaacccgctgttaaaacgtacatatgtactcttgttattacccgacgctttatagtcgctgtaatactgactcagataataagaggtataaaacgcattaataccccgctcccagttttccggtggaacatagccactttccagttcttccacccaggcctgcgggacactgaaatcgagacgaaaaaccccgatatcccaggtatagctcccaccctgaacaagttgctcaaatgttaaacattgcttaccgctggcgaagttatcgctattaatgcctaaccgcttgataacttctcttgataaacatgtttcttgcgggttgtctttaacaataatctcatatttcccgcgccattgcttattgacataaatatcgatgtcatactgccccggtaagggttgattatcatcaagacgaatatttgcaacctgctggtctttcattccacctatcataaaatgggtatcaaaggtttcttcagctgcataagcttcaatgccgagcaataacgctacgattgctgatgcaagtggggtcattctcaacataggcagctcctgcaattaaattttgtcactaatatagttgccatggtcatcgataatggtcagatgccagttatttgcattattacttttgacattaacactctgactttctaagggggcaatcataatagtttcataattgactttgacattattagctttgacatccgaaatcgtcacccaattagctgagtcattttttatcaccaaaccattgccactgcgatttaccagcaattttttaaatgtcgctttatttaccggagcaatacccgctggccggtaaaacaacttaattctgttttgcatcgcaaacttcagtgcattcttaccttcttgctctggactatttggtggaatatccagaacattcagataaaaaatgctttctttattagtgggcagtttattcggcataattttgatttttacttgctgcccggaatttgcccctatttttgccactggtggcgttaacatgaaaggaacctgaattttttctggtggtaatgacgtatcgccatcatcaatccacgcctgcagcagcgaagaacggtttccctggttcatcaactgcaccatcacttctttattttctgccgggtaaataatgcgcgtcccgtagataacaattccggcatgtgcaggaaggaccatagaaaaaatgagtaaagataataatcctttcattttaatgcctcttaaattaaaaggccgccatgggatagcggccatgtttattacctggagaaacttacaattttatttattaatcctgcgccacacgcataaccagagaagataacacatcacctgattgcactgagttatctgtcagtttcaggtattttgctttaaacggaatagcatattgaccttccgctgttttataactctcaatgttaaaaggtgcagaaacatccaggacatcgctgttatcacctaaatagagatagtaacccacggtatcgttgctactggctatcgccttatcgttaccggttattttatcgttggtaatcaacgagagttttacaccagcaacttctttcgggcagctaatttttaacatgctgctggttacaccgactgcatcatcataggtagaatatttagctttaccttcaaagacactggttggtacagtcggcatattaatacttactgaatcaccacccgcttcgaatttacacggagattctgcaatattccccttaatagttaatgttccggtatcaacgtctgcagcaaatactccagcgctcataaaaaaagaagaaaagacagcggcagcaataattgaacgtttcataatatgttccttaataaaatttatttttggttgttaagagtctgtatctcttggaaacaaatttctcacatcaaaaaagttgccgcaatgtaaacacattgttttattgatttaaaacaaattaaccattgcaatataaatacaaaaaatatttaagagtattaactatttatcgcatctatcaattaatgtagatttatgtaaatggtattgttgatatcaataaaaaagccgaaatcatttatataaatgatttcggctttctaaatgcaattaaaatcaggttgccaaattaatcgtagcgatttaacacgattcgacgtttgctatcgctacctgcaacaaccacttctgtcgttacacctttgacgggcgaagaaaacagatgacgggtgtcaacattatacgttaactgaccacaatgctgttgaggttgaccattaaccatagccatactgcatgttgggggactgatcctgccattaatcgctaatgtggcagtctctgaagagaatgcgggagaagccaatccataggcaagaaaaataattcctgacagccaatacttattcattgaacgttatccctgtagtaaaggttatgcctggatagaatgagtgcataacaaactatagctgtacatccactacacagccacgaaggatgataatgaagcattgcctgtatgatcaatcgactttgtagagtttcggacgaaggtccgcagaatattcgcagtattaaataagtgttcattaatgcggcaaaaactaatacaccgcatcaatgtaacatctctgcggtgtatgaagaataaccagaatggttaataggcgttagaccgcgcggaaggaaatctcgcctggaatgacttcaccctgccagtagagctgagctgcaacgcggtcagccagctggcggtagatagcggtaaattcgctctccggacggctgataaccgttggcgtacctttatcgagatcctcacgtaaggagatgtgtaacggcatctgccccagcagctgtgtatggtatttttcagccagtttctctgcaccaccggtaccgaaaatcggttcatggtgaccacagttactgcaaatatgcacactcatgttctcgacaataccgagcaccggaacctcgactttctcgaacatcacaatgccttttttcgcatcgatcagcgcgatgtcctgcggggtggtgaccacgactgcaccggttactggaatgttttgcgccagcgtcaattgaatgtcaccggtgcctggcggcatatcaagcaccagatagtcgagatccggccacaaggtttcctgcaacatctgcattaacgccttgctcgccatcggtccacgccacaccatcgcattgtcgtcagtgaccagataaccaattgaattggttgccaggccatgagacataatcggtgccatatgggtaccgtccggcgaagttggacgctgattttctgcgcccaacattgttgggattgatgggccgtagatatcggcgtccagaatgccgactttcgccccttctgccgccagcgccagtgccaggtttaccgccgtggacgatttacccacgccgcctttaccggaactcaccgcgataatgttcttcacaccgttaattcccggctgattcttcacgcgtttcagagtggctatgttatgcgacagtttccagtcgatagctttcgccccggtgatgcgcagcagttcggcgctacattgctcttttaactcttcgaacgcgctatgccagacaaacggcataaccagttccacatgcaacgtgtcgtccatccaggcgacatggtgcaacgctttcagcgtggtgaggttatgcttcagggttgggtgctgaaaattggccagtgtcccggcgaccattgcgcgcaaggcttctggtgatttggcctgggattgttcgttcatcccgactccttttttgtatagataaaccatcagctgatagtttacctgaagaatatagagaagtacttacttaacattttcccatttggtactatctaaccccttttcactattaagaagtaatgcctactatgactcaagtcgcgaagaaaattctggtgacgtgcgcactgccgtacgctaacggctcaatccacctcggccatatgctggagcacatccaggctgatgtctgggtccgttaccagcgaatgcgcggccacgaggtcaacttcatctgcgccgacgatgcccacggtacaccgatcatgctgaaagctcagcagcttggtatcaccccggagcagatgattggcgaaatgagtcaggagcatcagactgatttcgcaggctttaacatcagctatgacaactatcactcgacgcacagcgaagagaaccgccagttgtcagaacttatctactctcgcctgaaagaaaacggttttattaaaaaccgcaccatctctcagctgtacgatccggaaaaaggcatgttcctgccggaccgttttgtgaaaggcacctgcccgaaatgtaaatccccggatcaatacggcgataactgcgaagtctgcggcgcgacctacagcccgactgaactgatcgagccgaaatcggtggtttctggcgctacgccggtaatgcgtgattctgaacacttcttctttgatctgccctctttcagcgaaatgttgcaggcatggacccgcagcggtgcgttgcaggagcaggtggcaaataaaatgcaggagtggtttgaatctggcctgcaacagtgggatatctcccgcgacgccccttacttcggttttgaaattccgaacgcgccgggcaaatatttctacgtctggctggacgcaccgattggctacatgggttctttcaagaatctgtgcgacaagcgcggcgacagcgtaagcttcgatgaatactggaagaaagactccaccgccgagctgtaccacttcatcggtaaagatattgtttacttccacagcctgttctggcctgccatgctggaaggcagcaacttccgcaagccgtccaacctgtttgttcatggctatgtgacggtgaacggcgcaaagatgtccaagtctcgcggcacctttattaaagccagcacctggctgaatcattttgacgcagacagcctgcgttactactacactgcgaaactctcttcgcgcattgatgatatcgatctcaacctggaagatttcgttcagcgtgtgaatgccgatatcgttaacaaagtggttaacctggcctcccgtaatgcgggctttatcaacaagcgttttgacggcgtgctggcaagcgaactggctgacccgcagttgtacaaaaccttcactgatgccgctgaagtgattggtgaagcgtgggaaagccgtgaatttggtaaagccgtgcgcgaaatcatggcgctggctgatctggctaaccgctatgtcgatgaacaggctccgtgggtggtggcgaaacaggaaggccgcgatgccgacctgcaggcaatttgctcaatgggcatcaacctgttccgcgtgctgatgacttacctgaagccggtactgccgaaactgaccgagcgtgcagaagcattcctcaatacggaactgacctgggatggtatccagcaaccgctgctgggccacaaagtgaatccgttcaaggcgctgtataaccgcatcgatatgaggcaggttgaagcactggtggaagcctctaaagaagaagtaaaagccgctgccgcgccggtaactggcccgctggcagatgatccgattcaggaaaccatcacctttgacgacttcgctaaagttgacctgcgcgtggcgctgattgaaaacgcagagtttgttgaaggttctgacaaactgctgcgcctgacgctggatctcggcggtgaaaaacgcaatgtcttctccggtattcgttctgcttacccggatccgcaggcactgattggtcgtcacaccattatggtggctaacctggcaccacgtaaaatgcgcttcggtatctctgaaggcatggtgatggctgccggtcctggcgggaaagatattttcctgctaagcccggatgccggtgctaaaccgggtcatcaggtgaaataatcccccttcaaggcgctgcatcgacagcgccttttctttataaattcctaaagttgttttcttgcgattttgtctctctctaacccgcataaatactggtagcatctgcattcaactggataaaattacagggatgcagaatgagacactttatctatcaggacgaaaaatcacataaattcagggcagttgagcaacagggaaacgagttgcatatcagttggggaaaagttggcaccaaagggcaaagccagataaaaagtttttcagatgctgcggcagcggcaaaagcggagcttaagctgattgcggagaaggtgaagaaggggtatgtggagcaagcgaaggataattctttgcaaccttcccaaacggtaacgggctctctcaaggtagcggacttatccaccattattcaggaacaaccctctttcgtagcagaaacccgtgcgcctgacaaaaatacagatgctgttttaccgtggctggcgaaagatattgctgtcgtttttccgcccgaagttgtacacaccacgttaagtcatcgccgctttcccggagttcctgttcagcaagcagacaaattgccccaattacgtcgcttagcctgtagtgtgtcgcaacgggataataaaacagccacatttgacttcagcgcctgttctttagaatggcaaaacaccgtcgcccaggcgatcagtcagatcgacggcctgaaaacaacacagttaccatcaccagtaatggctgtactcacggcacttgaaatgaaatgcacaagatataaagtgcgtgaggatgttatggatcagatcgtccaggaaggcggtctggaatatgctactgatgtaataatacaccttcaacagattgatattgaatgggattatgcgaataatgtcattattattctgccgtctggcattgcacctagctacttggagcaatattccagatttgaatgacgcctacgtaaacatttatcactgacggaagagtctctctggcaaaaatgtgcacaaaaacttattgccgcaattccacatattccagaatggcggcaaccattaattgctttgttattacccgaaaaaccagaaattgcacatgaaattgcccagcgtctactggggcaaaaaaaattaccctcgcttgagtggttaaaaatagtggcgactgatgagcacattcttgcctcattagaaaaatatcacgaaccatatgccatttttgatgattactattgtggtgcgatatggtcagccaccgtattacaggagcaaggtgttgcagccctgccccgatttgctccctatgccgcaagtgactactgcgccgatgtgttgcgtcatatcaatcatccgttcgcattgacactgcttatacgtgtagccgggcaaactaaacgctgtcacgatcggatgacgaaagccattgctgcgttcccacatgcagcaatggcggcactgacggaacttcttgggcaaaaagaagagaacagttggcgcattatgctaatgacaatgcttatctcacaaccagcactggcagaacaggtcattccctggctctcgacacccgcagttgccgtactgaaatcatgccagcaacaactgacacagccctcaaaccatgccagcgccgatctactgccagccgtagtagtctcccctccctggctttcgaaaaagaaaaaatcgccgattccggtgctggatttagcgccattaggcattgagccaatctgttatctgacagaagaaatcagtaatcaacttttggcgaaatatatctggtattcaaaacacatcacggttagccatgaagaaagtactaccaacctgttggcaaggatgggttttcaacgacggatcgctggtacatatattaaagctcccgaagcggtagttgaggcatggctaaatgaagattattcaaccttactaagtgaatttaaggtgtttcattcacctaccgggcattattggcagttggggattttgacaacattgccgctggagaaagcagtaaaagcatggaatgcccttaccctatctccacataccgataccgaatactccatgttacattttggactcaaagggttacctgggttagtaaactcacttgcacgctatccacaagaagccttgcccatcacgaattacttcgcagcgagtgagctggctcctgccgtcgcccgtgccttcaacaaactgaaaacgctacgcgaaaacgcccgtagctggctgttgaaatacccggaacatgcccttaccggcctgctgcctgcggcgctcggcaaagccggtgaagcacaggataacgcccgcgctgccttgcgtatgcttaccgaaaacggtcatcagccattactgcaagaaatcgcccgacgttataaccagccggaagtaaccgatgcggtgaacgctctgcttgcgctcgatcccttagataatcacccgacaaaaatccccactcttccggccttttatcagccatcgctctggacgcgcccggtattaaaagcaaatgcccaatcactgccagatagcgccctcctccacctcggtgaaatgctccgcttccctcaggaagaggctctgtatccgggattattgcaggtgaaagacgtctgttccgccgactcactggcgggatttgcctgggatctgtttaccgcctggcagaccgctggcgcgccgtcgaaagagagttgggcgttcactgcgttaggcgttctcggtaacgatgacaccgcccgcaaactgacgccattaatacgcgcctggcctggtgaatcccagcataaacgcgccaccgttgggttggatattctcgctgctatcggtagtgatatcgcccttatgcagcttaacggcatcgcccagaaactgaaattcaaagcattacaggagcgggcaaaagaaaaaattgccgacattgccgagagccgcgaactcacggtggcggagcttgaagatcgggttagcaccggatctcggtctggatgataacggttcgctgctgctggattttggcccacggcagttcaccgtcagctttgatgaaaccttaaaaccgtttgtgcgtgatgtttccggcagccgcctgaaagacctgcccaaaccgaacaaaagcgatgatgaaacgcgggcgaacgatgcggttaaccgctacaaattgctgaaaaaagatgcgcgtaccatcgccgcccagcaggtagcaaggctggaatccgccatgtgcctgcgccgccgctggtcgctggaaaacttccagctcttcctggttgagcatccgctggttcgtcacttaacccgccgtctgatttggggcgtttatagcgccgaaaaccagctactggcttgctttcgcgtagcagaagataacagctccagcaccgctgacgatgatcttttcaccctgccggaaggcgatatctctatcggcactcctcacgttctggaaatatcaccaacggatgctgccgcctttggtcagctttttgccgactacgaactgctaccaccgttccgccagctcgaccgtaacagctacgccctgacagaagccgagcgcaatgccagtgaactgacccgctgggcaggcagaaaatgcccgagtggtcgggtcatggggctggcgaataaaggctggataaagggcgaaccacaggatggaggctggatcggatggatgatcaaacctttgggtcgctggtcgttaatcatggaaatcgatgaaggctttgcggtaggcatgtcgccagccgaactcagcgctgagcagctcttaagcaagctgtggctatgggaaggcaaagcagaaagatatggctgggggagtaattcaacacaggaagcgcagttctccgtaatcgatgccatcaccgccagcgagctaattaacgatattgaagccctgtttgaataaggaaagagcatggacaaggaattaccgtggctggcggataacgcccaactggaactgaaatataaaaaaggcaaaacgccgctcagtcatcgtcgctggccgggcgaaccagtgtccgttatcactggaagtctcatccagacattgggtgatgaattgctacaaaaagctgagaagaaaaaaaacattgtctggcgttatgagaatttttcactggagtggcagtccgccatcacgcaggccatcaacttgatcggcgaacacaaaccctcaatcccggcccggacaatggcggcgctagcctgtatcgcgcaaaatgacagccaacagttgctcgacgaaatcgtccaacaagaggggctggaatatgcgactgaggtggtgattgcacgccagtttattgcgcggtgttatgagagtgatcctctggtagtgacattgcagtatcaggacgaggattatggctatggttatcgctcagaaacctataacgaattcgatctccgactgcgtaagcatctctctctggcagaggaaagctgctggcagcgttgcgccgacaaactcattgccgcactaccaggaataaacaaagttcgccgcccttttattgcgctgatcctcccggaaaaaccagaaatagccaatgagttggtaggccttgaatgcccgcgaactcattttcattctaaggagtggttaaaagttgttgctaatgaccccacagcggtgagaaaactcgaacactactggagccaggatatatttagcgatcgagaagccagctacatgtcgcatgaaaaccacttcggctacgcggcctgcgccgcccttttgcgcgaacaaggactggcagccattccgcgcctcgcgatgtatgcccataaagaagattgcggcagtctgctggtacaaattaaccatccgcaagtcatccgcaccttgctactggtggctgataaaaacaaacccagcctgcaacgtgtagctaaataccataaaaacttcccccatgcgacgctcgccgcactggcagaactgctggcgttaacagaaccaccagcccgccctggttatccaatcatcgaagacaaaaagctgcctgcacagcaaaaagcacgcgatgaatactggcgtacgctgttacaaacgctgatggcatcgcagccacaactggcagcagaagtgatgccgtggttaagtactcaaccccagtcagtgctgaagagttatttatcggcaccgcccaaaccggttattgatggcaccgataacagcaatctgccagaaatcctcgtttcaccaccgtggcgtagtaagaaaaaaatgacagctccacgtcttgatttggcaccgctcgaattaactccgcaagtttactggcaaccaggcgaacaagagaggcttgccgccactgagcctgcccgttatttcagcacggaatctcttgcgcaacgcatggaacaaaaaagtggacgagttgtattacaggaactgggttttggggatgatgtatggctgtttctgaattatatactccccggaaaactggatgctgcacgcaattcactctttgttcagtggcattactaccaggggcgggttgaagagatcctgaatggctggaactccccggaagcacaattagcagaacaggcgctccgcagcggtcacatagaagcgttaattaacatatgggaaaatgacaactactcacattatcgtccggaaaagagtgtctggaacctgtatttattggcacagttgccgcgtgagatggctttgaccttctggctgcgtatcaatgagaaaaagcatctgttcgcgggtgaggactattttctcagtatcctcggattggatgcgctaccaggtctgctgttggctttttcacatcgtccaaaagaaacatttccgttaattttaaattttggcgcaacagaactggcgctgcctgttgcccacgtctggcgacgtttcgcggcgcagcgtgatctggctcgccagtggattttacaatggccggaacatacggctagtgcacttatccctcttgtctttaccaaacccagcgataatagcgaagccgcattacttgccctgcgtttactgtacgaacagggacatggcgaattgctacaaaccgtggcaaaccgctggcagcgtacagatgtatggtctgccctggagcagttgcttaaacagggtccaatggacatttacccggcacgcattccaaaagcccctgatttctggcatccgcaaatgtggtccaggccgcgccttatcactaataatcaaactgttaccaatgacgctctggaaattatcggcgaaatgctgcgctttacccaggggggacgtttttatagcgggctggaacaactgaaaacgttctgccagccacaaacgctggcagcttttgcctgggatctcttcactgcgtggcaacaagctggtgcccccgcaaaagacaactgggcatttctggcgttaagtctctttggtgacgaaagcacggcacgggatctgacgacacagatcctcgcctggccacaagaaggcaaatctgcccgtgctgtcagcggcctgaacatccttaccctgatgaataatgatatggcgctgatacagctgcatcatatatcgcaacgggctaaatcccgccccttacgtgataacgcggcggaatttcttcaggtggtcgcagaaaatcgcgggctaagccaggaagagctagcggacagattagtcccaaccctgggccttgatgatccgcaggcgttgagttttgattttggtccccggcagtttaccgttcgcttcgatgaaaatctcaacccggttatctttgatcagcaaaacgttcgccagaaaagcgttccccgtttgcgcgccgatgacgatcaactgaaagcgcccgaggcactggcccgactaaaagggctaaaaaaagatgctactcaggtgagcaaaaacctgctcccgcgtcttgaaacggccctacgtaccacccgacgctggtcgctggcagattttcattctctgtttgttaatcatccctttacccgtctggttacccagcgattaatatggggggtttatccggcaaatgaaccgcgttgtttactcaaagcctttcgtgtggccgcagagggggagttctgcaatgcgcaagatgagccaattgacctgcctgcggacgctctgattggcattgcccacccgttagaaatgacagcagaaatgcgcagtgaatttgcacagctttttgccgattacgaaattatgccgccttttcgccagttgtcgcgccgcacggtgctgctcacacctgacgagtcaaccagtaacagcctgactcgctgggaaggtaaatccgctaccgttgggcaacttatgggaatgcgatacaaaggctgggagtcaggctatgaggacgcatttgtctataacctgggtgagtaccggctggtccttaagttttcacccggttttaaccactacaatgttgatagcaaagcgctaatgagcttccgttctcttcgagtgtaccgtgacaataaatccgtcacttttgccgaacttgatgtgtttgatttgagtgaggcgttaagcgcacctgacgtcattttccattaaaacacagcgggcagtgatgcaactgcccgttatcaacacgacttaccagcggggaaagcgatgatcgtgcaaaaagagctggttgctatttacgattatgaggtccctgtacctgaagatccgttttccttcagacttgagatccataaatgctctgaattatttacaggttccgtctatcgactggagcgattccggctacgtccaacatttcatcaacgtgatcgagaagatgctgacccgctaataaatgatgcgttgatttatataagagatgagtgtattgatgagcggaaattacgaggtgaatcacctgaaactgtaatagcaatttttaatcgtgaactacagaatatattcaaccaagaaatagaataatatactctaaataattcaaattggtccgatccggcgcaacgtcccaatggcctggattataaatctcattatcttaattgcaacggggtccagccgtggttataattcgttcgttggaacacgatgttgcacaggctgtggtgttaggcctgaaaatagtaaataaaagaacctgcctcaccagcaggtttttttatttactgtgatctgctttccagatatttttcgctcaaacaactaatgcgccaaacatttattgcgcgtaaaatatcgtttatttcattaatacatttcagggatgaatatatgtcaccgcagaataatcatctgcagcgtccgcctgctgctgtgttatacgccgatgaactggcaaaattaaaacaaaatgataacgcaccttgcccgcccggttggcagttaagtttgcctgcggcccgtgcttttatccttggcgacgaagcgcaaaatatcagccgtaaagtggtgattagcccctccgctgtcgaacgtatgttagtcactcttgctaccggccgcggtttgatgttggtgggggaaccgggtaccgcaaaatctcttctttctgaattactggcaaccgctattagcggcgatgccgggttaaccatccagggcggggcatctaccaccgaagatcaaatcaagtatggctggaactacgccctgcttatcaatcatggtccgtcaacggaagcgctggtccctgccccgctttatcagggaatgcgcgacggcaaaatcgtccgtttcgaagagataacgcgtacaccgctggaagtgcaggactgtctgttaggtatgctttctgacagggtgatgacggggccggaactcactggtgaagccagtcagctctatgcgcgagaaggctttaatattattgccactgccaatacccgcgatcgcggcgtcaatgaaatgagtgctgcgctaaagcgtcgcttcgattttgaaacggtttttccgattatggatttcgcccaggagttggaactggtcgccagtgcttcggcgcgtttgctggcccatagcggtattccgcataaagtgcctgacgcggtactggaattactggtccgcaccttccgcgatctgcgtgccaacggcgaaaagaaaacgtcaatggatacactgacagcgattatgtccaccgctgaagccgtgaacgtggcccatgctgtgggcgtccgcgcctggtttttagcgaatcgcgcgggggagcctgccgacctggtggaatgtattgccggaaccatcgtcaaagataacgaagaagatcgcgcgcgtctgcgccgttacttcgaacagcgtgtcgccacacataaagaagctcactggcaggcttattatcaagcccgccaccgcctgccgtgaggaaagatgcatgagcgagccgttaattgtcggcatccggcatcatagtccggcctgcgcccggctggtgaaatcgttaatcgaaagccagcggccacgatacgtgttgattgaaggcccggctgattttaatgaccgggtagacgaactgtttttagcccaccagcttccggtagctatttacagttattgccagtatcaggacggtgcagcccccgggcgtggtgcctggacgccatttgctgaattttcgccggagtggcaggcgctacaagccgcacgtcgcattcaggcacaaacttacttcatcgatttgccttgctgggcgcagagtgaagaagaggacgattcgcctgatacgcaagatgaaagccaggccttactgctgcgtgccacccgcatggataacagcgataccctgtgggatcacttgttcgaagatgaaagccagcaaactgcattaccctctgcgctggcgcactattttgcccaactgcggggcgacgcctccggcgatgcgctcaatcgtcagcgcgaagcctttatggcccgctggattggatgggcgatgcagcaaaataatggcgacgtgttagttgtctgcggtggctggcacgctccggcactggcaaagatgtggcgcgaatgccctcagaaaattaacaagccagaattgccctcgctggcagatgccgttacaggttgttatctcacaccctacagtgaaaagcgccttgatgtgctggcaggatacctttcaggaatgcctgccccggtatggcaaaactggtgctggcagtggggcttgcagaaggccggtgaacaactgctaaaaactatccttacccgtttgcgccagcacaaattgcccgcttctaccgcggatatggctgccgctcatctgcatgcgatggcgctggcacagttgcgcggtcatacactaccgttacgcactgactggctggatgccatagcaggctcgctgattaaagaagccctgaacgcgccgttgccgtggagctatcgcggcgttattcatcccgataccgatccgattctgctaacgttgatagacacattagcgggtgacggattcggtaaacttgccccttctacgccacaaccgcctctgccaaaagatgtcacctgcgaactggaacgtaccgcaatctcccttccggcggagcttaccttaaatcgctttacccccgatgggctggcgcaaagtcaggtgttacatcggctggcaatactggagatccctgggattgtacgccagcagggaagtacactgacacttgcaggcaacggtgaagaacgctggaaattaacccgcccgcttagccagcatgcggcattgattgaggccgcctgttttggtgccacactccaggaagccgcacgcaataaattagaagccgatatgctggacgcgggcggaatcggcagtatcaccacatgtcttagccaggcggcgttagcgggtctggcgtccttcagtcaacaattactggagcaactcacactattaatcgcccaggaaaatcaatttgccgaaatgggccaggcgctggaagtgctttatgccttatggcggctggatgaaattagcggtatgcaaggcgcgcagatattacaaacgacgttatgcgcgactatcgatcgcacgctgtggctgtgtgaatctaacggcagaccggatgaaaaggagtttcacgctcacctgcatagctggcaagcgctttgccatattctgcgcgatctacatagcggcgttaatttacccggcgtttctctttctgcggcggtagccttactggagcgacgcagtcaggcaattcatgccccggcgctggatcgcggcgcggctcttggcgcactaatgcgtctggaacatcccaacgccagtgccgaagcggcgctgacgatgctggcgcagttatccccggcacaatctggtgaggcgctgcacggtttgctggcgctggcccgccatcaactggcctgtcagccggcatttatcgccggtttcagcagtcatttaaatcaactgagtgaagccgattttattaacgccctgcccgatttacgcgcggcgatggcctggctaccaccacgagaacgcgggacgctggcgcatcaggtgcttgagcattatcaactggcgcaacttcccgtttcggcgctgcaaatgccgttgcattgtccaccacaggccattgcacatcatcaacaactcgaacagcaggcactggcatcgctgcaaaactggggagttttccatgtctgaactgaacgatcttctgaccacccgtgagctacaacgctggcgattaattcttggcgaagcggcagaaacgacgctttgtgggctggatgacaacgcccggcagatagaccacgcgctggagtggctgtatgggcgcgatcctgaacggctccagcgtggtgaacgttccggtggattaggtggctcaaatctcaccacccctgagtggatcaacagtattcacacgctgtttccgcagcaggtgattgagcggctggaaagcgatgccgtgctgcgctacggcattgaagatgtggtgacgaatctcgacgtgctggaacgtatgcagccttctgaaagcctgctacgcgctgttttgcacaccaaacatctgatgaaccccgaagtactggctgccgcccgccggatagtgtgccaggttgttgaagaaattatggctcgactggcaaaggaagttcgtcaggctttttctggtgtccgcgatcgccgtcgccgttcatttattccactggcgcgaaactttgatttcaaaagtactctgcgcgccaacctgcaacactggcacccgcaacacggcaagttgtatatcgaatccccccgctttaacagccgcattaaacgccaaagcgaacaatggcaactggtcttactggttgatcaaagcggatcgatggtcgattcggtgatccactctgcggtgatggcggcctgtttgtggcagttacccggcattcgtacccatctggtggcgtttgacacaagcgtcgttgatctcacggcagacgttgccgatccggtagagttattaatgaaagtacagttgggcggcgggaccaatatcgccagtgccgtggagtatggtcggcaacttattgaacaaccagcgaaaagcgtcattatcctcgtgagcgatttttacgaagggggttcatcatcattactgacgcatcaggtgaaaaagtgtgtccagagcggcatcaaagtgctgggactggcagcgctcgatagcaccgcaacaccttgctatgaccgcgatacggcccaggcgctggttaatgtcggcgcacaaatagccgccatgacgccgggcgagctggcatcatggcttgcggagaatcttcagtcatgaattcactacgtccggaattattagaactgacaccgcaggccctgacggcgttaagcaatgccggttttgttaagcgcagtcttaaggaactggaaaatggcaacgtcccggagatcagccatgagaacgacgctttaatcgccaccttcagtgacggtgtccgtacccagctggcgaacggccaggcactgaaagaggctcagtgcagttgcggggccaacggtatgtgccgtcatcgcgtgatgctggtgttaagttatcaacgactttgtgccaccactcagtctacggaaaaagaagaagagtgggatccggcaatctggctggaagaactggctacccttcccgatgctacccgcaaacgcgcacaggcgctggtcgctaaaggcatcaccattgagttgttctgtgcgccgggtgaaattccctctgcccgcttaccgatgagcgatgtgcgtttttattcccgcagcagtattcgtttcgcccgttgtgattgtattgaaggcacactttgcgaacatgtcgtactggcggtacaggccttcgtcgaggccaaagcgcagcaagcagaatttaaccatttaatctggcagatgcgcagcgaacacgtcacatcatctgacgatccgtttgccagcgaagaaggcaacgcgtgtcgtcaatatgttcagcaattaagccagacattatggcttggcggcatcagccagccgctcatccattacgaggcagcattcaaccgcgcattgcaggcggcagagacctgcaactggcgctgggtgagtgaatcgctacggcaactgcgcgccagcgttgatgccttccacgcccgcgccagccactataatgccggagaatgcttacatcagcttgcggcattaaacagtcgattaaattgcgcacaagagatggcccggcgcgacagtattggtgaagttcctcctgtgccgtggcgcacggtcgttggctctggcattgccggagaagcaaagcttgatcatctgcggctggtgtctttaggtatgcgttgctggcaggatattgagcattatggtttacgcatctggtttaccgatcccgacaccggcagtattttgcacctttcgcgcagttggccgcgaagtgaacaggaaaactcaccggcagctacgcgtcggctgtttagttttcaggctggcgcactggcgggcgggcaaattgtttcacaagcagcaaaacgcagtgccgatggcgagctgctgttagctacccgcaaccgcttaagcagcgttgtgccgctgtcgcctgatgcctggcaaatgttgagcgcgccgttacgccagccgggcattgtggctttgcgggaatatttacgccagcgtccccccgcctgcatacggcctcttaatcaggtcgataacttatttattctgccggtcgctgagtgtatttcgctcggttgggacagcagccgccagacgctggatgcgcaggtcattagcggcgaaggggaagataatgtgctgacgttatcattaccagcctcagccagcgcaccttatgccgttgaacgcatggcggcgcttttgcaacaaacagacgaccccgtgtgtctggtttctggctttgtcagttttgttgaagggcaattgacactggaaccacgggtgatgatgacaaaaacccgtgcctgggcgctggacgcagaaactacgcctgtggcaccgctaccttctgccagcgttttgcctgtgccgtctactgctcatcagttgctgatacgctgccaggcgttacttattcaactgctccataacggctggcgctatcaggaacagagtgctattggtcaggcatagttgctggcgaatgacctcaccgcggtgggtttttatcggctggcacatgtgttgggacaatttcgtaatacagaaagcgaggcacgggtagaagcaatgaataacggtgttttgctttgcgaacaattattccccatgcttcagcaacaaggatgaaatagtgctttttactaagagttctactccagttccggactgctcacgccacggtattaggcatatcctatatagcccctggtgagagtcaccagttccttgattaaataaaatggagttttacatgaaggctttcaataagctgttttccctcgttgttgcatctgttctggttttctctcttgctggctgcggtgacaaagaagaatcgaagaaattcagcgccaatctgaacggcactgaaattgccattacctatgtctacaaaggtgacaaggtgcttaagcaatcttctgaaaccaaaattcaatttgcctccattggtgcaaccaccaaagaagatgctgccaagacacttgagccgttaagcgccaaatacaaaaacatcgcgggtgttgaagaaaaattaacctataccgatacctacgcgcaggaaaacgtgactatcgatatggaaaaagtggattttaaagccctgcagggtatttcaggaatcaacgtttctgctgaagatgccaaaaaaggtatcactatggcgcaaatggaactggtgatgaaagccgctggttttaaagaagtgaaataatcggttggcggtcatgctctaaacatgaccgccaattttttagccttttttcacatgctggcgcgctgccagtccacgcagaaaataacgtaaaaattgatcgccgcattcgcggaagtttttatgatccggtgcgcgcatcatcgctgtaatttccggcatcgaaacgcggaactgctgttcggtgaggatagccagaatgtcatcggttttcagcgaaaacgcgatgcgtaattttttcagcacgatgttgttattaatgcgacgttccggctccagtgccggagcagactcatccttgccgcgtttttcataaatcaggccattgaggaatgacgacaaaacaatgtccggacaacgctgaaaaccctcttcgtcttctttacgtagccagacggcgatctgttccgcggtggcttcgacattacccagcgccagaatacgcaccaggtcattattattggctttcaaaatgtagcgcacgctgcgcagaatatcgttacttagcatgaggccttcaggtgttgatgaggcaaaaagccattttagcagtcttttacaggccaatcgcctcttttaagcttttcagataacggcggctgaccggcacggttaagccattacgcaaaatcaactcggcctggccgttatcttccagacgaatctcctgtaaatgcgcgaggttaaccagatactgacgatggcagcgcagtagtggtgtacgactttccagggtacgtaatgtcaattcggtaaagccctctttcccttcgtggctggtaacgtagacaccgctcatccgactgctgacaaatgccacatctttcatttgcagcaaataaatccgactatgccccgtacaagggataaatttcagcgcctgttgattttccggtaacagcgaaacatcctgcttgctgcgctcctgacgcaatcgcgccagcgttttctccagtcgcgcttcatcaattggcttcagcagataatcaaaggcatgttcttcaaaggctttaattgcgtattcgtcaaacgcagtgagaaaaacaatatacgggcgatgttccgggtcaagcatccccaccatttccagaccactgatgcgcggcatctggatatcgagaaacagcacatccgggcgcagtttatgcaccgcgccgatcccttccacggcgtttgaacactctccaacgatttcaatatcgctctgctcctgcaaaaatacacgcaggttctcccgtgctaacggttcatcatcgacaattaagactttaatcatgcctcgtccctccatggtagtcgtaacgttattcgggtgtaactatcaggctcacaggcgacgcttattccatagtcatcgccaaaccgttcacgtaaacgcttatccaccagattcatccccagcccactggcattggttaccggttgatacaaaccggcattgtcttcgatctccagcatcaaatgttgcccctcacgtcgggcgctgattgccactcgccctgtatccagcagttgtgatgtcccatgtttaatggcgttttccactatcggttgcagggtaaacgcgggcaattgctgctgggataattcttgcggaatagcaatgttgacctgcaaccgcgactggaagcgcgccttttcaatttgcagataagcattcacatgttcaatttcgtcggcgagagtaacaaactccgaaggccgctttaagtttttgcggaaaaaagtggaaagatactgcaccagctggctggcctgttcgctgtcgcggcggatcaccgctttaatggtgttaagcgcattaaacaaaaaatggggattcacctgggcgtgaagcagtttgatctctgactgggtgagcatcgctttttgccgctcatattgcccggcaaggatctgcgccgaaagcaattgcgcaatcccctcacccaacgtgcggttgattgaactgaataaacggtttttggcttcatacaatttgatggtgcccatcacccgctgattttcaccacgcaacggaattaccagcgtcgaccccagtttgcattgcggatgcaaagagcaacggtaaggtacttcgttgccatcagcgtagaccacttcaccggtttcaatcgcttttaaagtataagttgaagaaatcggtttgccgggtaaatggtggtcgtcaccaattccggtaaaggccagcaatttctctcgatcggtaatcgcgactgcaccaatatccagttcctgatacagcacctgagccactttcatgctgttcacttcgttaaacccctggcgcaaaatgccttccgtcgaggctgccactttcagcgcagtggcagaaaaagccgaagtgtatttttcaaacatcgcgcgtttatcgagcaatatacgcataaacagcgccgcgccgacggtattggtgaccatcattggcgcagcaatattactcaccagacgcaccgcatcttcataaggtcgggcgatcgcaaggatgatcagcatttgcaccatttcagcgacgaacgtgacggcaccggcggtaatggggttaaagactttatcagtgcgcccgcggcggatcaggatgctgtgtaccaggccaccgagtaatccttcaacgatggtcgagatcatgcaacttaacgcggtcatgccccccatcgaatatcgatgtaagccgccggtcagcccaaccagcccaccgacgaccggaccgccgagtaagccgcccattaccgcgcctatcgcacgggtattggcaatagaatcgtcaatgtgcaacccaaaccaggtgcccatgatgcagaagatggaaaagacgatgtagcagagaaatttatgcggcagacgaaccgtgacctgcattaacggtatgaataatggcgttttactcattaaccatgcaatgactaaaaaaacgcacatctgctgaagcagcagcaacaccagattaaaatcgtacatacccgcaaaccacacttccctttaaaacgcgtaacatacattgcctgcgtttaactttctttgaactcttgcagaaaaatgagaattcgtgagtacgatcactcaaaatcgcctggcaaaaataaaatcaccctatagatgcacaaaaaacgggcaaaactacctggttcgcaaaactgcgtctaaagttaaaccgggacctcgcgagcaagggtgagacgatggcgctttacacaattggtgaagtggcgttgctttgtgatattaatcctgtcacgttacgcgcgtggcagaggcgttacggattgctgaaaccgcaacggacagacggcggtcatcggctgttcaacgatgccgatattgaccggatccgcgagatcaaacgctggatcgacaacggcgtgcaggtcagcaaagttaaaatgctgctcagtaatgaaaatgttgatgtgcagaacggctggcgcgatcagcaagaaacattactgacttacctgcaaagcggcaatctacatagcctgcgaacgtggatcaaagagcgcggtcaggattaccccgcccagacactcaccacacatctgtttattcctctgcgccgacggcttcagtgccaacaaccgactctccaggcgctgctggcgatcctcgacggcgtactgatcaactacatcgccatttgtctggcttcggcacgtaaaaaacagggtaaagatgcgctggtggttggctggaatattcaggataccacccgtctgtggctggagggctggattgccagtcaacaaggatggcgcattgatgtcctcgcccactcgctcaatcaactacgccctgaactattcgaaggccgtacattgctggtgtggtgcggtgaaaatcgaacctccgcccaacagcagcaactcaccagttggcaagaacaaggccatgatattttcccactcggcatttaatgattcgttaacaaatgcgctttactgtacaatcctttcgttaacataaggagtgcattatgcgcatagctaaaattggggtcatcgccctgttcctgtttatggcgttaggcggaattggtggcgtcatgctcgcaggttatacctttattttgcgtgctggctaagcgcctgcaccagcctttcaaacaggcggtctgcgatgatcgccgccagtgccaccagtaacgccccctggatcacatacgcggtattaaatccgctaagcccgatgatgatgggcgtacccagcgtgctggcccctaccgttgaggcgatcgtcgccgtaccaatgttgataatcaccgaagttcgcacgcccgccagaatcaccggagccgccagcggtagctcgaccttacgcactcgctgaccacgactcattcccatacctttcgcaacttctgtcacgctggcatcaatcgctcccagcccggcaagtgtcgcctgcaggacgggcagcacaccgtaaaggatcaaggcgataatcgctggttgcagaccaaagccgatcaccggaacggcgatcgccagcactgcgacgggcggaaaagtctgtccaacggcggcaatagtttccaccagtgggcgaaattccgcgccccacgggcgagtgacagcaattccggcaccagtgccaatgatcaccgcaaacaaactcgaaattcccaccagccagaaatgagccagtgccagagctgcaaaactttcttgctgataaacgggtcgtggcagttgtgggaacaaggcagcaaacagcggctggctgtaaggcagccagaaaatcagcgccacaaacagagcaatgagccagaacagcggatcgcgcaacatcttcatacgcttacgcctccaccagcagatcctgaaaatgcagcgtgccgcaaggctggccctgcatgttcaccaccggcagcacctcgcatccccgcgcaacaaacagagagagcgcatcgcgtagcgtcatctcttctgccagtgcctcaccatctgctcgttcttcgcgacgcacgtaatccgccacactacgtaacgaaagcaggcgcacacccagttcactacgtccaaaaaactggcggacaaaatcattcgccggacgagtcagcatcgtcagcggattgccctgctgcactacttcaccgtgatccatcaataccagatgttctgccagccgtagcgcctcatcaatatcatgagtgaccagcacaatggtacgccccagcaaacggtgaatgcgcgtcatctcttgttgcaacgcgccgcgcgttaccgggtccagtgcgccaaaaggttcatccattagtaagacttgcggatcggcagccagtgcacgcgccactcccacacgttgctgctgaccaccggaaagctgatgcggataacgctcacgcaaatttgactccagccccagtagcgccattaattcgtcgatacgatcgtcaatccgcgcccgcgaccatttttgtaattgcggcacggtagcgatgttttgcgccacgctccagtgggggaacaggccaatagattgaatggcatagcccatccggcggcgcaactccagtactggcagcgagcgaatttcttctccggcaaagcggatctctccgctgtcatgctccaccaggcggttaatcattttcagggtggtggatttgccggagccagatgtgccaatcagcaccgaaaaactcccttcctgaaaattgagattgagatcgttaacggctttttgtgcgccgaacagtttgctgacatggctaaattcaatcattacgtttcaccttcagcagtgcgataagcaaatcgaacagcgcgtcggtaagcaccgccagaacaattaccgggatcacccccagcaacactaaatcaatggcgctgcttagcagcccctggaaaaccagcgcaccaaaaccgcctgcgccgattaacgccgcaatcaccgccatacctacagtttgcaccatcaccacccgcaggctgcgcagaaataccggtaacgccagcggtaactgaacatgcaggaaacgctgcgccccgctcatccccatcgctctggcgctttccagcacatcgcgcgggatctggttcaaaccgactaccacgccgcgcaccagcggcagcaaggcatagagcaccagcgcaatcagtgcgggtgtcattccggttcctgctatgccgagcgtccccagccacggaaaggccgtaaccagcgcggcaagcggcgcaatcaacaggccaaagagcgccaccgaaggcacggtctgaatcacattgagcagagaaaaaattgccccctgccgagcagtggaaaagtagcaccagatgcccaacggcacaccaatcactaacgcaggcagcaccgcaccaaacagcaacgtcagatgttgtgccagcgcgtcgtcaaacacatcctgacggttggcgtattctttcattagtgagagatcgttaagcgtgccggagtacagcaaccacagcggaataatggcaatctgcatatgcaacaaccagcgccacagcggatgcgtggagattcggcggatggcatcgctacaggccagcaatgccagcgccgcagccagccagaaaccactgccgaggctggtacgcgccagcgcactgccattttgcgccagttgggtcgccgcctttccagctccccacaccagcaatacgaagacgaattgcgccagaatgagtgcacaaatgctgccttttttaccgggaataaaacaggccgtcagccaggcgcaaccaacgcccaccagcatccagatcgtttgcggccacagctgccagagatgacgcccctcacccgaaactaaacgattaggcgcgtaactgataaacggcagcgccgctgcgattgccgtcagcaacagcagcagcgccagaacaggattaatacggaaataagtcacgggaaattacttcgtccaccctttttgtttcaggtagtcggcagccacttttttggcatccagtccttccacagcaatgctggcattcagttgctgcaatgtttttgcatcgaggctggcgaagactggctgtagccactgtgccatttgcggatactccctcaacaccgactcacgcaccactggtgcaggcgcgtagataggttgcacaccttgcggatcgcttaaggtttgcagccccagcgccgctaccgggccgtcagtgccgtaagccattgcagcattaacgccagaggtttgctgggcagcggctttgatcgtcaccgccgtgtcgccaccagccagtgacagcaactgatcctgaccgagcttaaagccataggctttttcaaacgcgggtaacgcatcggcgcgttcgataaactctgccgaggctgccagtttgaaggtgccgccctcttgcagataacgactcaggtcggcaagcgaagtgagtttatttttctctgccacatcctgacgcacggcgatagtccaggtgttatttgcaggcgcgggcgtcagccagattaacttgttgtgctccgaatcgagctttttgactttctcgtaaccttgctgcgcgtttttccacgctgcatcgttttcatctttaaagaagaaagcgccattgccggtatattccggatagatatccagttcaccggaagtaatcgccccgcgcaccacaggagtcgttccgagttgcactttattcaccgtcggtacgccgtggctttccagcacctgcaaaatgatattgccgagtagcgcaccttcggtatcgatttttgaaccgactttaacgggggaagccgcctgtagcggcaggctcacggctgccaacataaccagtgaacctgcccagagctttaagagtggcatgatgctttcctcattcttttactgttgttttcagcgaattaagagaaaagcatagttgataatggcggggttagcttgagcggaaggattcagttgcagaatcagataaatacttaagaggcatattcggtccggcgtttcctgccggatgcggcgcgagcgccttatccggcctacaaagggcgcaaacgtcgcgcccttactaaagcattacagcaactcaaactcgcctttcttaacgcgtgcggaatcagtgccgataaagacattgaacttgccaggctcggcgtcatatttcatctgttgattccagaacttcagcgcctcaatatcgatcgggaagctgacagtctgagtttcgcccggtttcagggtgattttctcaaagcctttcagctgtttcacagggcgactcatggaagccgtcacatcctgcaagtacatctgcactaccgtggcaccctcgcgcttaccggtgttcgtcacctgcacgctggcagtcactttgccgtcacgcttcatggtcggcgcagaaagtttcacatcagagacggtgaaagtggtgtagctcagcccatagccgaacggatacaacgccccgttagcttcatcaaaataacgcgaagtgtatttgttcggcttgtcggcattatacgggcgaccggtattcagatggctgtagtacaccgggatctgcccgacagaacgcgggaaggacattggcagcttgccggacgggttgtaatcgccaaacaatacatcggcaattgcattaccgccttcagtccccgcaaaccaggtttccagaatcgcatcagcctgctgatcttctttcaccagcgccagcggacgcccgttcatcagcaccagcaccagcggtttaccggtggctttcagcgccgcaatcaagtcacgttggctttgcggaatagtgatatcggtccggctggaggcttcgtgcgccatcccctgtgcttcaccgactacagccaccaccacatcagattgtttcgccgtctgcaccgcttcatcaatcatctcttgcggcgaacgcggatcgactttgaccgcttcttcatactgattcaggaaatcgataatgcctttgtcactggtaacgttcgcccctttggcatacagcactttaccgttttcaccgacggcatttttaatcccggtcagtacggtcacggattgatcggcaacaccggctgcggaccagctgcccatcacgtcacgtttactgtccgccagtggcccaaccaccgcaatggtggccgattttttcagcggtaacgtttcgagacggtttttcagcaacaccaagctttcgcgcgccacttcacgcgcttctttacggtgcaggcggctttcggcattggtatccaccgggtcagactctttcggccccaaatggctgtatgggtcgttaaacaaccccatatcatatttaacgttcagtacatggcgggcagcatcgtccagctctgccatcgtcactttgccggatttaatcaacccaggcagatacttcgagtagtactcgtcgctcatgctcatgttgattccggatttcagcgccacgcgcaccgcatcttccgggtctgccgccgtgccatgtttaatcagctctttgattgcaccgtgatcggaaacggtgatgcctttaaagccccactggtcgcgcagaacatctttcagcagccaggaatcggaggtggctggcgtgccgttcagcgagttcagcgccaccatcaccgcgccgctgcctgcgtccagccccgctttgtacggcggcatataatcattaaacaggcgctgcggactcatatcgacggtgttgtactctttaccgccttctaccgcgccgtatgcggcaaagtgtttgacgctggtcatcaccgagtagcgatctgccgggcttttaccctgcatcgcttccaccatggttttacccattgttgaggtgagatacgtatcttcgccaaaaccttcggaagcacgtccccagcgcggatcgcgcgagacatcgaccatcggtgcccaggtcatattcaggccatcatctgccgcttcataagcagagacacgtccgaccgttttcactgcatcgaggttaaaagacgaggccagaccgaggctaatcgggaacaccgtgcgctgaccgtgcagcacgtcgtaagcaaagaaaagaggaattttcaggcggcttaattccatcacctgatcctgcatggcgcggatatcctgacgggttacggtgttgaaaatcgccccaacctgaccgtctttgatcatctcgcggatcgcctctttcgggttatccgggccgacgctgattaagcgcagctgaccaattttctcatcaactgtcattttcttaagcagttcggtgacgaacgcatcccgcgcttcgggcgttaatggatggttgccgaataaatcatccgccagtgctggctgcagggccagactcaccgcgattcctactgaacatagccatttcatatggatttttcttcctttgttgcccgacgtggcagcgaaaatggtgcaaaaaccgtagtttgccataagcatgatggagagagaaaaagaatgctcagtttattgtctgaattttcaaaatattcactcgctgaattgttatacaaggcgctattctagtttgtgatattttttcgccaccacaaggagtggaaaatgtcttccatgacaacaactgataataaagcctttttgaatgaacttgctcgtctggtgggttcttcacacctgctcaccgatcccgcaaaaacggcccgctatcgcaagggcttccgttctggtcagggcgacgcgctggctgtcgttttccctggctcactactagaattgtggcgggtgctgaaagcctgcgtcaccgccgacaaaattattctgatgcaggccgccaatacaggcctgaccgaaggatcgacgccaaacggtaacgattatgatcgcgatgtcgttatcatcagcaccctgcgtctcgacaagctgcacgttcttggcaagggcgaacaggtgctggcctatccgggcaccacgctctattcgctggaaaaagccctcaaaccgctgggacgcgaaccgcactcagtgattggatcatcgtgtataggcgcatcggtcatcggcggtatttgtaacaactccggcggctcgctggtgcaacgtggcccggcgtataccgaaatgtcgttattcgcgcgtataaatgaagacggcaaactgacgctggtgaaccatctggggattgatctgggcgaaacgccggagcagatccttagcaagctggatgatgatcgcatcaaagatgacgatgtgcgtcacgatggtcgtcacgcccacgattatgactatgtccaccgcgttcgtgatattgaagccgacacgcccgcacgttataacgccgatcctgatcggttatttgaatcttctggttgcgccgggaagctggcggtctttgcagtacgtcttgataccttcgaagcggaaaaaaatcagcaggtgttttatatcggcaccaaccagccggaagtgctgaccgaaatccgccgtcatattctggctaacttcgaaaatctgccggttgccggggaatatatgcaccgggatatctacgatattgcggaaaaatacggcaaagacaccttcctgatgattgataagttaggcaccgacaagatgccgttcttctttaatctcaagggacgcaccgatgcgatgctggagaaagtgaaattcttccgtccgcattttactgaccgtgcgatgcaaaaattcggtcacctgttccccagccatttaccgccgcgcatgaaaaactggcgcgataaatacgagcatcatctgctgttaaaaatggcgggcgatggcgtgggcgaagccaaatcgtggctggtggattatttcaaacaggccgaaggcgatttctttgtctgtacgccggaggaaggcagcaaagcgtttttacaccgtttcgccgctgcgggcgcagcaattcgttatcaggcggtgcattccgatgaagtcgaagacattctggcgttggatatcgctctgcggcgtaacgacaccgagtggtatgagcatttaccgccggagatcgacagccagctggtgcacaagctctattacggccattttatgtgctatgtcttccatcaggattacatagtgaaaaaaggcgtggatgtgcatgcgttaaaagaacagatgctggaactgctacagcagcgcggcgcgcagtaccctgccgagcataacgtcggtcatttgtataaagcaccggagacgttgcagaagttctatcgcgagaacgatccgaccaacagcatgaatccggggatcggtaaaaccagtaaacggaaaaactggcaggaagtggagtaaaaattacggatggcagagtatcgccatccgaattcacttaatcgttctgtgccgtctgccccgccgccgccatttgggcggctttttgttttttatagctcaacgctgctgccggcacaggcatcactttaccggtttcaatccaggtacgcaggcggctggcatcggcaaaatgggtatatttgccaaacgcgtccatcactaccagcgccaccggtttattattgataaccgtacgcatcaccagacaatggcccgccgcattggtaaagccggttttggttaactgaatattccagttatcgcgatacaccagatgattagtattgcggaacggcagcgtatacgtcggattagagaaggttgccatatcttcccgggtagtacttaactgcccgatcaacggatattgtttgctggcaatgagcagtttggttaagtcacgggcagttgaaacgttatgcaccgacaatccggtaggttcaacaaagcgcgtgttgttcattccgagcgatttcgctttcgcattcattgccttaataaaggctttgtaaccaccgggataatggtgcgcaaggcttgccgccgcgcggttttctgaagacatcagcgccagcaacagcatatctttacggctgatttcgctattcagtcgtacgcgcgaatagacccctttcatctccggcgtctggctgatatccacttttagtttttcatccagcggcagtcgtgcatccagcacaaccatcgcggtcattaatttgctgatagacgcaatcggacgcaccagatccgggtggttcgaatagatcactttgttggtattcagatcaacaatcatcgcgctaccggaggcaatttccggttgtgaagcggtggtagcggctgccgttttcgcaacggcctgcggtgcaaaaggcacagccagcatcagggccaggctaaataaagaaactcgaaatttcggcatgatgagcattcagatagtggttcacgcgcacgggttgcgcaccgccggagtaaggatttactgaggctagcgacgccatcataacgagcaaaaagtgcgatcgtcaaaggagaatcgtgaggaaatgctgcattgctgacatttacgccagcaatgcaacgtcaaagaactttctagaacaaacgataaccgtagccccatagtataacggttagggcgagcagcacttccagtaccagcacgccaatcgccagcgtcgaactagagaagctaaggccttcctctttgttgatattcaggaagctcggaataccaaggtaaagcaggtagccggtgtaaaacagcgccaccgtgccgaccagcgcacacaaccagaccagtggataaagcgccaccagaccgcttaaaaacagcggagttgcaacgtagcccgcgaagaccatgcagtgcgcaagtgacggacgctgcggataattacgcgccatccaccagatgacccgccccatcaccgcgaccccagccagcataacgccgtaaaacaagacagccagcgccagtccggtaaaccaggataacttcaggatagtgccatcgccaaaattccagccaatctgtgtagtgccaatgaaggcgcaaatcaccggaatcgccgccatcagcaaaacgtggtgggtgtaatggtgagaaatcgtttcgttttcgcgattaatcacctgcatttcacgatcgggatgggaaaacagtccccagacatggctcataccgcccccttgttgtgagttcatgaacctgacagttcaagtataagtcagcttgtgattattttttgttcgcccatgtaattttcactgtctgatgaacgtcctttttcagcgtgaatgattcacagggtgtatgcttactggcaaccaaagggagacagactggcctatggatctcaatacacttatctcacaatatggttatgccgcgctggtgatcggtagcctggcggaaggtgaaaccgtgactttgctgggaggcgttgcggcgcatcaggggctattaaagttcccgctggtggtactttctgtggcgcttggcggcatgattggcgaccaggtgctctatctgtgcgggcggcggtttggcggcaagctgttacgccgtttctcgaaacatcaggataaaattgagcgggcgcagaaacttatccaacgccatccgtatctgtttgtcattggtacgcgctttatgtatggctttcgggtgattggcccgacgctgattggtgccagccagctgccgccgaaaatctttctgccgctgaatattctcggcgcatttgcctgggcgttgatttttaccactattggttacgctggtggtcaggtgattgcgccgtggttgcacaatctcgaccagcatttgaagcactgggtctggttgattctggtcgtggttctggtggtgggcgtgcgctggtggctgaaacgacgcgggaagaaaaagccggatcatcaggcgtaaaaccattgccctggataaggcgttcgcgccgcatccgacatccggagtaccatgcctgatacgacgcttgtgcgtcttttcatgccgaccaaaatattacccaatgaaatatccacgcacctcactgcgctattctgggttgaactgtggattcgccaacataaagccgccatccactatcaacgactgcccggtggtgtaatttgcgccctccgaacaaagccacaccaccaggctggcaatctcatgcgttgcgccaaaacgccgcaagggaatcgaaggctccgcgtcgggcttcacgtcgctgtcatccatgccattcattggcgtggcgatcgccccaggcgcgactgcgttcaccaaaatcttatgcctgaccagctccagcgccatcgctttggttaacccaccgagcgcatgtttagcggctgtgtaggcgctggcatccggcagcggcgtatgttcatgtaccgacgtaatgttgatgatgcgaccgccctgcccttgtttcaccatctgacgagccgcaatttgcgagcataagaatgcaccatcgacatcaacggtaaaaatcttgcgccactcatcaaaagccatatcaagaaacggcgctttggtcattgcacccgcattattcaccagcacatcaatgcgccccagccgttgaatgagtttctccagcgccagtgccccttctggtagattgccgagatccagctgcacgatctccgcacgtacgccgtggctaactacctcacgcgcggtatcttttgccccttcttcatctgagtgccaggtaataccaatatcaaacccctgctgcgccagtaataacgcgcactctttgccgatccccgaatcggaggcggtaataatcgcaacctgtgccatcgagttctccacttaacgctgaataaacgttaagtatagaaggcgcatatcatcagcgtttgtaccccccgcccaacgcaccagtgagttgaatggaggcatccagccactgcccttgcaataacaggccattggcccgctcacgcagcgcggggattctggcttcgctgacgcgggaaccagcaatgatgcccgcgttaaagcgcgcctgcgcaagacctaccacacgcaaggcatcgcgctcaatttgcgcctgatgctggtttttctccgccagtgtctgaacctgactggctgcccgcgccacgtcattcaccgcttcaaccaccgctttgttgtagctggcgatagacaagttgctttcggcttttgcgatatcgagattggcgttaagacgaccactatcgaaaatgggtagcgtcaggcctgccgtaacgcccatttgctgcgcggaatgacggaacagatcgcttaagtgcaacgcatcctgttgcaggaaggccatcaggttgatgtcaggataaaatgccgcttttgccgcatcaatggtgcttagcgatgactcaacgtaccagtgcgccgcctgcaaatctgcccgccgggccagtaaggagtaccccagttcatcaggaagctggcttgccactttcggcaacgcgaccggtttaagcttcaatgactttgtctggttatttgtaagtgcgcttaaccgtgcctcaataattttcattttccccgcgacatcgttgagctgctgccgggttttgctggcattaatatcggtttccacaccttcaactgaagaagtaatcccgttctgatatagctggcgatcggtcgcgataatggtgttctgctctttttctatttgctgcaagaccgtgtttaacgccgcctgggtttgccactcccagtacaggcgggctacgctgccagccagcaattggcgggtttgctcgcgttccgccgcccgtgctttaaccgtacccaggcgggcagtaacctccgcccgattctttccccagatatcgagatgccagcccgccgttaagccaaaagtaccgttggtgtaccacgggccggtcgtacctgcggccggatcgttcagagcaaacggccccattaagccttctgccgacattttttgccgctccatatccgccgaaaagtcgatctgcggaccatcctgagtggcaactgccttcgcctgggcttcagctagctgaatgcgctgttcagccacctgcatatccggtgcgttctgtagtgcattgttaattaaggaagtgagttgattatcgtgatactccagccaccattggctgtctggccaaccattttcagcgccgtgggtaatgcggtgtcaacttgtgcagcgggcgtttgctggcttaacgcctggcgggtttcatgcataggcgcacacccggccagcatcagtaacagcggaaaacaggcgatggctggataaaaggaatcacgattcatgggggaataatcaggtaagaaaaggtgcgcggagattaccgtgtgttgcgatatattttttagtttcgcgtggcaatacatcagtggcaataaaacgacatatccagaaaaatatacactaagtgaatgatatcttccgatttatcttaatcgtttatggataacggcaaagggcttcgttttttcctatacttattcagcactcacaaataaaggaacgccaatgaaaattatactctgggctgtattgattattttcctgattgggctactggtggtgactggcgtatttaagatgatattttaaaattaattaatgtcatcaggtccgaaaataacgagaatatttcagtctctcatcctgttgcgctcctgtcatgtgcattgcttcatataatcactggcgcaaggagcgcgcagggggcggccaatcgccgccgccccctgcacccccgggctctggcgaacaaaatcgccgctgcgcggtgccctcggcttatcccttacggctaccgggtcgggcgcgaggtaacatccctgtaaaacgcgccctcagcccacatccatgtgggctgccccggccttcagggaacgcctcggcaattttgacgccaccaaacaaccgtgcggcctattgataaagagctaacacattgtcaaaaaacatcactatggttttttagagtttctcgatatcaattgcctgaatagcccttgcaatatcaggggaattattcaacacccgaacatgctgaaataattccgttgcttcatcgtattctttacgcaaataactcaaccactgtttaatccgcgcaacgtgatataacccggtatcgccctgcttttccagacgggtatatttttgcagcaaagcaaccacctccggccacggcattcgcggttcgttatattttaccacccggctcaggttgggaatattgagcgccccgcgaccaatcatcactgcgtcgcagccgctgatcgccatgcattgttgcgcgctctgccagtcccagatttcaccgttggcaatcaccggaatattcagccgctggcgaatatcgccaatcgcctgccagtcaatatgctccgcgcggtaaccctgctctttcgtccgcccatgcaccaccagctccgtagcgccagcctgttgaaccgcatcggcgatttcaaatttcttctcaccgctgtcccagcccagacgcactttcacgctgacgggcaaatgcgccggtacagcttcacgcatcgcttttgcaccctggtagatgagttcaggatctttgagtaacgtcgccccgccgccgctaccgttaaccgttttcgacgggcagccgcaattgagatccacgccccaggaacctaactccaccgcacgggcggcgttctctgccagccattgtgggaactgacctaacaactgcacgcgcaccagcgtaccagatggtgtccggctggcgttttgtagctcagggcaaatgcgatgaaagacttttaccggcagcagttgatccaccacgcggacaaactcggtgatgcacagatcgtagtcgttaacttcggtcagcaattcacgcaccagagagtcaagcactccctccatcggtgccagtaacacacgcatatcatcacccgcaaaaaaatgaggcgctatgttagcgcctatggtcagcggattaaaggtctgcaaagagggattgctgcaaactgcaatccctctctatgcttgatgtatgcctgagttcgctgcgcattgcgtaatgccggggagcgaaaaaataagcgctgatttcttaatgtgatcggtagcacgttttacgaattaattgtatgatgaatccatctcatctggggtgttgattatgagtaagacactgaacattatctggcaatatttacgcgctttcgtcctgatttatgcctgcctgtatgcaggcattttcattgcttccctgctaccggtaaccattccgggcagcatcatcgggatgctgatcctgtttgtcctgctggccttgcaaattcttccggcaaaatgggtcaatccggggtgctacgtactgattcgctatatggcgctattgtttgtgccgattggcgtaggcgtcatgcaatattttgatttgctccgcgcacagtttggcccggtagtggtttcctgtgcagtcagtacgctggtggtttttctggtggtgagctggagttcgcaactggtacacggtgaacgtaaagtcgtaggtcagaaaggatcagaagaatgatggcgaatatctggtggtcattaccgctgacattgattgtcttttttgccgcccgcaaactggcggcacggtataagtttcccttgcttaacccgttgctggtagcaatggtggtgatcattccttttttaatgctgactggcatctcttacgacagctactttaaaggtagcgaagtgctaaacgatctgctgcaaccggcggtcgtcgcgctggcctatcctttatatgagcagctacaccagatccgcgcgcgctggaaatcgatcatcaccatctgttttatcggcagcgtggttgcgatggtgacggggacttccgtggcattgttgatgggcgcttcaccggaaatcgccgcgtcaatcctgccgaaatcagtcaccacgcctattgcaatggcggttggcggcagtattggcggtattccggcaatcagcgcagtttgcgtgattttcgtcggcatcctcggcgcggtatttggccatacattgcttaatgcgatgcgtattcgtaccaaagctgcgcgcggtctggcaatggggactgcctcgcacgccctcggtacggcgcgctgcgccgagctggattatcaggaaggtgcatttagttcgctagcgctggtgttatgcgggataattacttcgctgatcgcaccgttccttttcccgattattctggcagtaatgggctaaaatttgcgatgcgtcgcgcatttttgatgtatgtttcacgcgttgcataattaatgagattcagatcacatataaagccacaacgggttcgtaaactgttatcccattacatgattatgaggcaacgccatgcatccacgttttcaaaccgcttttgcccaacttgcggataacttgcaatctgcactggaacctattctggcagacaagtacttccccgctttgttgaccggggagcaagtctcatcgctgaagagcgcaacggggctggacgaagacgcgctggcattcgcactacttccgctggcggcggcctgtgcgcgtacgccattgtcgaattttaatgttggcgcaattgcgcgcggtgtgagcggaacctggtatttcggtgccaatatggaatttattggtgcgacaatgcagcaaaccgttcatgccgaacaaagcgcgatcagccacgcctggttgagtggtgaaaaagcgcttgcagccatcaccgttaactacacgccttgtggtcactgccgtcagtttatgaatgaactgaacagcggtctggatctgcgtattcatctgccgggccgcgaggcacacgcgctgcgtgactatctgccagatgcctttgggccgaaagatctggagattaaaacgctgctgatggacgaacaggatcacggctatgcgctgacgggtgatgcgctttctcaggcagcgattgcggcggcaaaccgttcgcacatgccttacagtaagtcgccaagcggtgtcgcgctggaatgtaaagacggtcgtattttcagtggcagctacgctgaaaacgccgcattcaacccgactctgccaccgttgcagggagcgttaattctgttgaatctcaagggttatgattacccggatatccagcgcgcggttctggcagaaaaagccgatgcgccgttgattcagtgggatgccacctccgcaacgctgaaagctctcggctgtcacagtatcgaccgagtgcttctcgcttaagcctggtgccggatgcggcgtgaacgccttgtccggcttgccagccctctcctggtgtcgaaattcccggcaaacagtttgccgtttcttgcgcaaaaccagcgggtaaagtagcctgatggaaattttccttagatcgagtctcctgcatgttaaagcgcgtgttcctcagcctgttagtcctgatcggcttgctgctgttgactgtgctcggcctcgatcgctggatgagctggaaaaccgcgccttatatctacgacgaattgcaggatctcccctaccgccaggtcggtgtggtgctcggaacagcaaaatattatcgtactggcgtaattaatcagtattatcgctaccgcattcaaggagcgattaatgcctataacagcggtaaggtaaattatctattactgagcggcgataacgcattgcaaagttataatgagccgatgaccatgcgcaaagatttaatcgctgctggtgtcgacccatcagatattgttctcgattacgcaggctttcgtacgctggattccatcgtgcgtacacgcaaagttttcgatactaatgatttcattattatcacccaacgtttccactgtgagcgagcattatttattgcgctgcatatggggattcaggctcagtgttatgccgtaccgtcaccgaaagatatgctgtcagtacgtattcgtgaatttgccgcccgtttcggtgcgctggctgacctttatatttttaaacgtgaaccgcgttttttagggccgctggtccctattccggctatgcaccaggtaccggaagatgcgcaggggtatcccgccgtcacacccgaacagttacttgaattacaaaagaaacaaggaaagtagttatggatgtacagcagttttttgtcgttgccgtttttttccttatcccgatattttgtttccgcgaagcatggaaaggctggcgcgcaggcgcgattgataaacgggttaaaaatgcaccggaaccggtgtatgtctggcgagcaaaaaatcccggactctttttcgcttatatggtggcatatatcggcttcggaattttatctatcggcatgattgtttatcttattttctatcgttaatattcccctctccagttaattattgagaataattattacttcacctgataagctgcggatatcacattcctaaccgcagctatttgtgaatcttttcacagtttaaattcccccgcacgcttagccttaatatcagtacattattatttactaaacgctcgccttaattacctatagcattaaggaagatcacatgccgcaacaaaattatctggatgaactcactccggcttttacgtctttactggcgattaaagaagcctctcgctgtttattatgtcacgacgctccctgtagtcaggcttgcccggcacagaccgatccggggaaatttattcgctcaatctactttcgtaattttaaaggcgctgccgagacaattcgcgaaaataatgccctcggtgccgtttgtgccagagtgtgcccgacggagaaattatgccaaagcggttgtacccgtgccggtgttgatgctcccattgatatcggccgcttacagcgttttgttactgattttgaacaacaaaccggaatggaaatttatcagcccggtactaaaacgctcggcaaagtcgcgattattggcgcaggtcctgccggattgcaggccagtgtgacactgacaaaccagggttatgacgtcacgatttatgagaaagaagcgcaccccggtggctggttgcgtaacggtattccgcaattccggttaccgcaatcagtgctggatgcagagatcgcccgtattgaaaaaatgggcgtgaccattaagtgcaacaacgaagtcggtaacacactcacccttgagcagctgaaagcagaaaaccgcgcggtactggtcaccgtggggttatcaagcggttccgggctaccgctgtttgagcatagtgacgttgagattgccgtcgacttcttgcaacgtgcacgacaggcgcaaggcgatatcagcattccacaaagcgcattaattatcggcggcggtgatgtcgcgatggacgtagccagcacgctgaaagttctcggctgtcaggcggtaacttgcgtagcgcgtgaagagttagatgagtttccggcaagcgaaaaagagtttaccagcgcccgggagctgggcgtttcgatcatcgatggattcacgccagtagccgtggaaggcaataaagtcacgtttaagcatgtacggttatcgggcgaactgacgatggcggcagataaaattattctcgccgtcggtcagcatgccagactagatgcctttgcggagttagagccgcagcgtaacaccatcaaaacacaaaattaccagacccgcgacccgcaagtctttgctgctggcgatattgttgagggtgacaaaaccgtggtctatgccgtgaaaaccgggaaagaagccgccgaggcgattcatcactatttagagggagcttgctcatgttaacgaaagatctttcgattactttttgcggcgtgaagtttcccaacccgttctgcctctcttcttcgccggtaggcaactgctatgagatgtgtgccaaagcctacgacacaggttggggcggtgtggtgtttaaaacgatcggcttttttatcgccaacgaagtctcgccgcgttttgatcatctggtgaaagaagataccggttttatcggcttcaaaaatatggagcagattgctgaacatccgttggaagagaatctggccgccctgcgtcggctgaaggaagattacccggacaaagtattgatcgcttcgatcatgggggaaaatgagcagcaatgggaggagctggcgcgcctggtgcaagaagctggcgcggatatgatcgagtgtaacttctcctgtccgcaaatgacttctcatgcgatgggtagcgatgtcgggcaaagcccggagctggtagaaaaatattgtcgggcagtgaaacggggttccacgctgccaatgctggcgaagatgacgccgaatatcggtgatatgtgcgaagtggcgctggcggcgaagcgcggcggcgcagatggcattgcggcgattaacaccgttaaatccatcaccaatatcgatcttaatcagaaaatcggtatgccgatcgttaacggaaaatcgagtatttccggatattccggtaaagcggtaaaaccgatcgccctgcgcttcattcagcaaatgcgcacccatccagaactgcgcgatttcccaatcagcggtatcggcggcattgaaacctgggaggatgcggctgagtttttattgctcggcgcagcaacgttacaggtgaccaccggcatcatgcagtacgggtatcggatagtggaagatatggcaagcgggttgtcgcattatctcgccgatcagggatttgattcgctgcaggagatggtaggtctggcgaataacaatattgtcccggcggaagatttagaccgcagttatattgtctatccccgtatcaatcttgataaatgtgttggctgtggacgctgttatatttcctgttacgacggcggtcaccaggcgatggaatggagcgagaaaacccgcacaccgcattgtaataccgagaaatgtgtgggttgtctgctttgtggtcacgtctgcccggtgggttgtattgagctcggggaagtgaagtttaagaaaggcgagaaagaacacccggtaacgttgtaaaaccagagacgcatccggcatttggttcctgtcgccggatgcggcttgaacgccttatccggcctacaaaaccatacaaatcagtatgttgagcttattgtaggccggataaaacgcgccagcgttgcatccggcatttggctcctgttgccggatgcggcgtgaacgccttatccggcctacaaaaccacacagatcatgatgttatgtgcgtttatgaccgaatgcggaccacattcacatcatttcttacgcgcgtatttcagtgaatccagcgctacggcgaagataataatcgcccctttgatgatgtactgccagtatgggtttacgccgatatacgtcaggccatagttgatgacggtaaaaataattaccccggtcaccacgccaatcaccgtccccacaccgccgctgaacgatacaccgcctaccacgcacgccgcgatagcatccagctcatacataaagccgaggttgttggtggcagagccgatacgtccggcttctaacatcccgccaaaggcatagaacacgccagacaacgcgtagatcatcagcaggttcaggccgacgttgacaccagatacttttgccgcttccgggttaccgccaatggcaaaaatgttcttaccgaagcgggttttgttccacaacacccagacgaacgccaccgcaatcaacgcgtagaaggtgatgtaagagagacggaaactccccagcgcgacaaagccctgagcaaaggtagagaagccactgtcaaaaccagaaattggcgacgccccgacaaagtcgtaatagagcgagttgatgccatagacgatgatcatcgtgccgagcgtggtaatgaacggcgtcacgttgagataagcgataatcagaccgttgatcaaaccgatcaccgcaccaatggcacagacaatcagaataaccagcgcaatcggcatcgtcgccatttccgggaacactttgttggcgttatccatggactgcaataatgtcgcagccaccactgccgccagccctacctgacgaccagcagaaagatcggtcccctgggtgacaattaaccctgccacaccgagcgcgataataatacgcaccgatgactgggtgagaatattacttaagttcaacagacttaaaaatgttgggtcctggaaaataataatcgccagcaaaactaaaagaacgacgtaaataccgccctctttcaggtaagtaagaaaacttttcttatttaacgcactcatgggaagcccctaatcttaaaggtgcaaagacgcaagacgcagaatttcgttttgcgttgttgtttttgtatcgacaattccggaaacgagaccattgctcatgaccagaatacggtctgttatccctaacaactcaggcatttcagaggagataataataatccccttgcctttcttcgccagttcggcaattaactgataaatttcaaacttcgccccgacatcaataccgcgcgtcggttcatcgagcattaatatttctggttgcgttagtagccagcgaccaataatcaccttttgctgattaccaccggagagcgaaccaatttgcgtccgatgacccggcgtttttacccgcatcgaatcaatcacccactgggtatcgcttttcatccgcgagttatccagtaaaccaactttatttttgtagttgcgaatattggaaattaacgagttaaaaccaatatccagataggcataaattcccgttgagcggcgctcctcagttaccagtgcaaatccatggtttatggcttcgttggcattatggttattgatctgtttgccgtgcaacgttatggtgccagccgatttctcgcgaataccaaataacgtctcaacaatatcggtacgtttcgcccccaccagaccggcaataccgaggatctcccctttatgcagatcaaacgagacatcgcgaatcgacggctggcgcagtgacgtcaggttacgtacctcgaggatgacttcgcccggtttgttttctttgtcagggaaacgctggttaagagaacgcccaaccatcatggcgatgatcttgtccatcgtcagtcctgccagcggttcggtggcgatccactgaccgtcgcgcaatacggtaacttcatcacataactggaagatttcttccattttatgcgagatataaacaataccgcagccgcgctcttttaatttacgaataatagtgaacagatgattgacctctttttcggttaacgaagaagtcggttcatccataatcacaattttcgcgttataggaaaacgctttggcgatttcgatcatctgcatttgcgaaacggataatgtgccgacgcgcgcacgcggatcgatatcaatatccagttcgtcaaaaatcgctttggtttcgcggtacattttgtcctgatcgacaaacatgcctttggtgggatatcgccccagccacatgttatccatcaccgaacgttgtaataccaggtttaactcctggtgtaccatcgaaataccattttccagggcttcttttgcagaatggaaatcgatctctttaccctggaataaaatggtgccggagtctttttgataaataccaaacaggcattttaataatgtcgattttcctgcaccgttttcccccattaatgcatggatagaatgtggccggacttttaaattaacgttatcaagtgccttaacaccaggaaaggacttgttgataccgctcatttccaacaagtattccccggaggacggagtcgttgagctgaccatataattttaccttgttggccatacaataagggcgcagtaatagactgcgcccaatcagtcttatttcttgctgaattcagccaggttgtctttatctacgccaacataaggtacgcggaccactttgttgtcgattttccagttggtgccatcagccgcacctttaccatcggccaggtttttcgccagatcaaaggtcgctttcgcctggttgttagcatcgttcagtacggtgcccgccagtgcaccggatttcaccagcgccagcgcttctggcagcgcatcgacgccaaacaccggaatgctggacttgttgtgtgctttcagcgcttcaaccgcgcccattgccatcgcatcgttgttggcgataaccacttcgattttgttggcgttcgggccagacagccaggcgtccatcttatctttcgcctgagcggtgtcccacattgcggtatctaactgtaactgttcagttttgatgcctttatcgttcaattctttaatcacgtaagtggtacgtgcttctgcatccggatggcccggttcacctttcagcagtacgaactgaatctgaccgtctttgttcagatcccaaccctgattcgccgcccagtgtttagcaatcaaatcgccttgaataatgccggactctttggagtcagtgccaacgtagtaggctttgtcgtagctatccagcgccttacgagacggttctttgttgaagaaaaccaccggcacgttttgcccacgcgctttctcaatcaccgtacccgcagctgccgggtcaaccaggttgattgccagtgccttcacccctttcgccagcaatacgtcgatctgatcgttctgcttggactggtcattctgagaatcattcatcagcagctgaacatctggcgcggctttcgcatcttgctcaatagccttgcgcactacagacataaagttatcgtcgtacttatagattgttacaccaatgcgagtatcagcagcgtgtgcagcggcaccgaataacatgctggccatcacagcagacagggttaacaccttcttattcatggtatctccggtttttcttatgcagggtagtgcttgagataaatgctcggcggggcagtagagttaatgaagtgttactgaacgccgaagctcactttttaaaattcgttcttccatgcccggtaacgctccagaaaacggctttaattgttgttatgacgctgttacctcggcaaaagtgattattcactgttacatacgggttacaacgttaaaacggtgcaatcatagctatcacattgttaagatactgtgaaatcactcacagattgaaagcggttacatcgcctgatttgttgagttagtgatcgccgccgcattctggcgtgttgcgacagaatggcgacgcactaacgtcggcataaaacagtggctggcacgaggatcaatattgcctgctgccccctgcaaggccagttcggtggctaatttcgccattgaagcaatgggataacgcacggtcgttaattgcgggtcggtgtaacgggcgatgggaatatcatcgaaaccgatgattgagagatgtaacggaatcgcaatgccattatcttttaatgctgtcagtgcgccagcggccatattgtcgttataagcaaatacagcggtaagttgtagattgcgccccagcagttcaaccatcgccgcctcaccgcccggcatgtccggcgtaccagcgccaatccagctttccggcggaataatatcctgctctttcaacgcactcatccagcctgctttacgcatggcgtcatcttcaatgccgtggctggaagaaagataaccaatacgttgatgaccgttattcagcaacatgcgcgtcgccattcgggcaccgctgagattatccaggcaaacgcaacgatgggcgtaccccggcacaacgcggttgattaacaccataccgggaatgttatccataaattgcgccagttcatcgtcactcaatgcttttgagtgaacaatcaacgcattacaacgctggcgaattaacacctcaatggcgtgacgctctttttccgcttcatgatagctattgccgattagcacgtatttctgatgctgctgagcgaccagatccaccgcttttaccagcgcgccgaaaaacgcatcagaaacgtccatcaccaccacgccaatggtgtcgctaacctgagttgccagcgcctgggcattggcgtttggccgataatccagctcactcacggctttcattactgcttcacgcgtgtcggcactgaccagcgtgctgttattgagcacccgggaaaccgttgccacagagacgccagcctgacgcgctacatcacgaatggtgatcatattcactacctgttatgagattgcagtaaatgactgcttgctggcggctattttgtcagcactgaatacaggacttcgtgaatcgagtcacagcaatggaaacggttacagccgttttgttaacgaatgtgatccagatcgttatcttgatgttttagatattgccggtccggcagcacgcaaagttaactgacgccagagccattccaccggcccctggcggaagtaacgcagccagataacagagaagaggatattcgccagccataccggaataacaaacgccagcagctccaggcggtcaaaatgcataaacaaaccgaggtggtaaaaaagcgtggtacaaatcagcgtttgcaatagatagttggtcagcgccatccgtccgacgcaggcgatcgcaagcaccagcttaaagcggctcaattgcggccagaagccataaaacagcgacgcatagccaatcgcctgaaacggcgcactcagttcccgcggcatttgaagtaagaaggcacaccagcgatacgcccagtccagctgccattgcagggcgatggcaggaaggttaatggtcaccccaatcgccaccagcacaaaaccagtacgacgatagtgacgtaagctgaactgccctttcagccagccgctgcgcatcagcgccgcaccaatgagcatcatccctgccagttgccagccatactgtgcgcccagtgccagtaaactgttgccaacaccatcggcacgattactgatcgcttcaacgccgccgtgaagcttccagtatttttcatacaaaatagccgatgcatccggcgtccaggcgcggctggtctggctgtcggaaatcagccccaataacagcaaaacgccaagccccaccagataaagcatgacgcctgtattaaacaggctttttaccgatggcgcatcgcgcaccagccgccagcagattaagcccaccagcccgtaagccagcaaaatatcgccgtcccagaacaataaaccgtgaataaagcccaacaagactaacagcgttaaccgcgactggatccagcgtctgccacggggcagcaacatttgcaggcccgcaccaaacagtagcgcaaaaagcgtgaggaatttcacctggccgatgagatcaagaaatgcccaagtccatgcatcccgcggcgtaatagcaccgtaccaggcgggattgagataagccgcctttggtagcccaaaggcgctgatgtttaatagcaggatccccagaatggcgacgccgcgaacaaaatcgagcgtgacgttgcgctccatggttcctgccttttaatcagttgtgatgacgcacagcgcgcagaaactcgtggcgcgtattctgactggatttgaacaatccaccaagagaggtcgttgtcgtggcactggttgcatcgcggatgccacgcgccttcacgcagtaatgcaccgcgtcgatcgagacagccacgttattggtgcccagcagcgtttgtagcgcaataagaatttgctgcgtcagacgttcctgcacctgcggacgctgggcaaagaactgcacaatgcggttaatttttgacagaccgatcaccgaatctttcgggatataggccaccgtcgctttgccatcgatggtaacaaaatggtgttcacaggtgctggtcagagtgatatcgcgcacggtgaccatttcatcgaccttcattttgttttcaatgagggtgattttcgggaaattggcgtaatccagaccggagaaaatttcatcgacatacattttagcgatgcgatgcggcgtttccatcaaactgtcatcagccaggtcgagattcagcagctgcatgatttcggtcatatgaccagcaataaggcttttgcgcgtttcgttatccatttcatgcacgggcgggcgcagcggtgtttccagtcctcgcgcaactaacgcttcatgaaccagggccgcttctttactgagtgatggcatttatgatttctcctgcaggtgtgacgcctccgccctgcgtgggggcaaagttattaagctgatttacagcctgattattgtgcgtgaggcggcgcacataatccagtattcacagcgataattattgtaattgccgctgcctttcatcagcagatgttaaaacatcgttatgcaaatacggaagtgaaagttactcacagcacattgaataaacggtatgatgaagaaattgcaaacaacacaacaaggagccacgcatggaaatgctcgaagagcaccgctgttttgaaggctggcagcaacgctggcgacacgactccagtaccttaaactgcccgatgacgttcagtatctttctccctccacctcgtgatcacactccgccaccagtgctgtactggctttccggattaacctgcaatgacgagaacttcaccaccaaggcgggtgcccagcgggtagcggcggaactggggattgtactggtgatgccagacaccagcccgcgcggcgaaaaggttgccaacgacgatggctacgatttaggccagggcgcaggcttttatcttaatgccacgcaaccgccgtgggcgacgcattaccggatgtatgattatctgcgcgatgaattaccggcgctggttcagtcgcaatttaatgtcagcgaccgctgcgccattagcggtcactcaatgggtggtcacggtgcgctgattatggcgctgaaaaatccgggtaaatacaccagcgtttcggcctttgcgccaattgtgaatccgtgcagcgtcccgtggggaatcaaagcgtttagcagctatttaggtgaggacaaaaatgcatggctggaatgggacagttgcgcactgatgtatgccagtaacgcgcaggatgcgatcccgacgcttatcgatcagggcgataatgatcagtttcttgccgaccagttgcaacctgcggtactggcagaagccgcgcgccagaaagcgtggccgatgacgctgcgtattcagccgggatatgatcacagttactacttcatcgcctcttttatagaggatcacctgcgcttccatgcgcagtatttactgaagtgaaagtccgcccggttcgccgggcatcttctcatcagaagcgataatccactgccataaagtaacgacgtccgtcttcgttatagctgtagtcgtcacgactgagatccttgtcgccaaggttcagcacgcctgcgcgcagtttgacgtctttagtcacctgccaggccgcgccggtattccagatggtataaccgcccggtgttttagccgtcgcgctgtcggcgcgtttctgcccggtatagtgcccagaaacatagaatgaccagtcttccagcgccagcggtttccagtccagcgtaccgttagcagtatggaacggcagatcggatagcggtttgttttcgccgttgctgacatcacgaccatcgttgtaggtgtagttgatcgacagtttccattcatcgttgaacggaattttcagttcggtttccacgccctgaatacgagctttgttaacgttgtagtagctaaataccggtatgcgccgtccgttagcgcccgtctcaaaaccaacaaagttttggtagcccggtgcagcgttgacgtcagacgtacggctgatgctgatacgatctttcacatcgttacggaaaacggtaacgctggattcaaccccttccagccagccttcttcacccatgtagtaaagccccagctcccaactttcgctggtttctggtttcagatccgggctacccacaatcttacatgcgccacggcaggaattgctcgtccagtcagggctaagttgcaacagagaaggtgctttaaatgccgtcgcccagccccctttcaccgttacggtgtcggtggcgttataaaccaggtaggcacgcggactccagtgttcaccgtaggtttcgtgatcgtccatacgcacgccggtcgtcagcgccagcggctcgaagatccgccattcatcttccacaaacagcgcgtactggctggcagacgttttggagctggttcccccggtcaggttcaccgcatcgctaagtttgtcgtgacgccattcaccgccaaccgtgagaaactgattaatcgccgtcagcggcaacgtgtatttgccgtcgaccgtattgctttcggaagttatcgggctgctgttgccagggtttttgttctcgactttctcaccgtagtatttcagttcgctggtgccgtaatcccaacgcccattatggctgacggagtagttctggcgttccaggcggtttttgtccagcgagtcggaatcacgatcctgacggtcgaaaccgtatccggcagtaaaatcgtgattttgattcggtgtccaggcaaattcgacattgccgtcgcggctggagaatccttcaatacgcggcgtttctccggtatcggtggtcgttgagttttgcgggtcatccttttcacgttttgccaggctgccgtaagctttcattcccagcacaccatcaattaatggtccactggtaaagaactgaccgttataggtgtcaccgcgatcgcgatgttcctgaatggtggtatcgacggtaacggtacccgaccatttctgaccgatttttttggtgatgatattcactacaccgccgagcgcatcggaaccgtacagcgacgacatcgggccacggaccacttcaatacgttcgatggaatcgaccgggatccagttcagatcgaaatcattgtggcggaagacggcattgcgggagttcacgcgtttaccgtcgacgagaatcagggtatagctgctgtccagaccacgaatactaacgcccttacggttatccccttcgttcgtcagttgtacgccaggcacttctttgaggacatccttcagattctgtaccggttttcgctgcaggtcttcctgggtaatgacgctgatactggcaggtgcatctttaagattttgttccacggaagatgcagtgacaaccatcgtttcgccatcatcatcgaccgctaacacaggccatgcacaagaaatagcggacaaacacagcccgacccgtacgaaagggttcaacctaaacattccatatctccatgaggtaactacgaaaataaaatgggttatcgctcacatcttcttcacgtccccttgcgtacggcagcatcgcggtggacttattttttatgcaggtgatcatcccagaaagccggaacagcctctgatttgtcagccttttttgattgcggcgtaacgataatgcaaacgataacaattatcaatccaaatgttaaattttatatccgcatgatttgtcagggaaatggaattgaaaaagccctctcggttgagagggcttagcaaggaagggaggaaacttatttcttatcgttctgcgggaacttcatttcgctgtagcgtacgaagtgagttcctttaatcagcttgtagccgaaccaaataatcaggaacagcgggataccaatatacgttgccgctacgccgccccagtcaatagtatctttcaggaacgcttcgtagttctggcccaaagtgataatcagacacagaatgaatgcgaagatcggccccagtgggaagaaacctgaacggtacggcagatcgttaatgtcgtgtccctgcaatacgtaaccgcgacggaagcgatagtggctaatggcaatccccagccaggcgataaaacccgtcatcccggaggtgttcagcagccacaggtataccgtctggttgccaaacatggaggtcaggaagcacagaccggcaatcaccgtcgtcgcatacagcgcattacgcggcacgccaccacgcgacagtttagcgaaaatgcgcggcgctttaccgtcacacgccagggtgtacagcatacgagtagacgcatacataccggagttacccgctgacagcaccgccgtcagaataactgcgttcatcaccgccgccgcagagagcagacccgcgtgctggaacaccagggtgaacggactaacgctgatgtctttaacatcgttacgcagcaggctcggatcggtgtacggaataatcaggctgataatcaggatcgcgaacacatagaacaacaggattcgccagaacacctgacgtaccgcgcgtggaatgtttttcgccggatcttcggactcgcctgcagcaataccgatcagctcggttccctggaaagagaagccgacaatcatagctacgccgatcatcgccgcaaaaccaccagcaaacggcgcttcgccgattgtccagttgctccagcccgcaggctgcgcgcctttgaagataccgataatcatcagcacgccaacgatgataaagacaataactgtcgtgactttgatcagtgagaaccagtattccgcttcaccaaagccacgaactgagatgtagttcagcaggaagataacgccgaggaacaacgcactccagatccagcccggtgtatccgggaaccaccagctcatgaccagctgagctgcaaccaggtcaacggcgatagtcaccgcccagttgtaccagtagttccagcccagcgcgaagccaaagccttcttcaacatagttctgaccgtaagtggcaaacgaaccggaaaccggcatatatgcagccagttcaccgagactggtcatcaggaagtaaaccatcaggccaatcagcatatacgagagcaatgccccgcccggacctgcctgagaaatcgttgcgccagaggcaacaaaaagacctgtaccgatggaaccgccaatggcaatcatcgtcaggtgacgcgcctttaattcacggcgtaagcccggcgcttctgtggttttagtttcggaaaccatacaaaaatgctatccatcttaaaaatgaggcgcgattgtagcagacgattggcaatccttccggcagaaatacacggttataagacaccttcatgatcgcccagggattataagtaaagcagccaatctcttttctggcgaatgcatgctgaaggcgctgcgtcacgaaatcgacacagcaccagcatgttcttgtacagcaacttaacgcggcacatttgcgggatcgcaatagtccagaaagcgccgtagcgcgttggaaaggtgtttttgccgatgatgtatacgccacaacgtacgcatcaggcgcggcagagggaccgcaacttcacttaatgtgcctgcctgcaattgatcttcaatcacacgtcgcgacaggcaactaattcccaacccatgacgcaccgcatgtttgattgcctcggagttacctaattccatcgccatctcaaacttcggtaaatgtgacagcaacagataatcgacaatctcccgcgtgccggaaccgcgttcacgcaggatccacggcgcagcggccagctgttctaaggtgaccggaccacgggccaacggcgaagtcggcgcggcgaaaaccaccagctcgtcttccagccacggttcagaaatgatttcagtgctgtggcacggtccttcaataaagccaatatcaacgcggaaatccagcaccgcttgcatcacgtcctggctattcccaacgctaagttcaatcggcaactgcggataatcatggcgataacgggcgataactgcaggcagaatgtagttaccgatggtactactggcatagatacgaatcgcgccgttgtcttcgcgaaacagttgttcgatttcaaccgcctgttcaagcaatgccaacgcacgcggatagagcagccgcccgtgttcattaacaaccagtcttttccccacgcgatcaaacagttgcacgccaagctgcccttccaggtcggtcaaggctgcgctcactgctgattgcgacaacgccagcatcaccgacgcctgggtggttgatccacttttcaatacttctgcaaaaacttccaactgccggagggtgatgtgcatagtcgcttaccacttataaagattaattataaatatataatcaattttatttttaaaccagttagtcgtaaccttatgcccggttaaaggagagggttatgacgaatatcaccttacagaaacaacatcgtacactgtggcattttattccggggttagccctgagtgcagttatcaccggggtcgccctgtggggtggttccattcccgcggttgcgggtgccgggtttagtgccctcaccctcgcaatcttgttggggatggttttaggcaacaccatctatccgcacatctggaaaagctgtgacggtggtgtgctgtttgccaagcaatatttattacgtctgggtatcattctttatggcttccgtctgacgttctcgcaaattgccgatgtcggtatcagtgggatcatcattgacgtgttgacgctgtccagtaccttcctgctggcttgcttcctggggcagaaagtgtttggtctggataagcacaccagctggttgatcggtgccggtagcagtatctgtggtgctgccgcggtactggcgactgagccggtagtgaaagcggaagccagtaaagtaaccgtggctgttgcaaccgttgttatcttcgggaccgtcgcgattttcctctacccggcgatatatccgctgatgtctcaatggtttagtccggaaactttcggtatctacattggttctactgtgcacgaagtggcgcaggtggtggcggcaggtcatgccatcagcccggatgcggaaaacgcagcagttatttccaaaatgctgcgcgtgatgatgctggctccgttcctcatcctgctggcggcgcgtgttaaacagctgtctggggcgaacagcggcgagaaaagcaaaatcactattccgtggtttgccatcttgttcatcgtagttgccatctttaactcgttccacctgttaccgcagagcgtggtgaacatgctggtaacgctggataccttcctgctggcaatggcgatggcggcgctgggtctgaccactcacgtcagcgcgctgaaaaaagctggggcgaaacctctgctgatggcactggtactgtttgcctggctgattgttggtggtggtgcgattaactatgtgattcaaagcgtcatcgcataaaccactacatcttgctcctgttaacccgctatcattaccgttttcctccagcgggtttaacaggagtcctcgcatgaaatacattggagcgcacgttagtgctgctggcggtctggcaaatgccgcaattcgcgccgccgaaatcgacgcaaccgcgtttgccttgttcaccaaaaaccaacgtcagtggcgtgccgcaccgctcacgacgcaaaccatcgatgaattcaaagccgcctgtgaaaaatatcactacacatcggcgcaaattcttccccacgacagttatctgattaacctcggacatccggtcactgaagctctggaaaaatcgcgcgatgcctttatagatgaaatgcagcgttgcgaacagctggggctttctttgctcaacttccaccctggcagccatctgatgcagatttcagaagaggattgccttgcgcgtattgccgaatccatcaacattgcgctggataaaactcaaggtgtgacagcggtgatagaaaacaccgccggtcagggcagtaacttagggtttaaattcgaacatctcgcggcgattatcgacggcgtggaagataaatcccgcgtcggcgtctgcattgatacctgccatgctttcgctgccgggtatgatttgcgtactccagccgaatgcgagaaaacattcgcggattttgcccgtactgtcggctttaagtatctgcgcgggatgcaccttaacgatgcgaaaagcacctttggcagccgcgttgaccgccatcatagcctcggtgaaggcaatatcggtcatgatgcgttccgctggatcatgcaggacgaccgtttcgacggcattccgctgatcctcgaaaccatcaacccggatatctgggcagaagagatcgcctggctgaaagcgcaacaaactgaaaaagcggtagcctgaagatgaataaccgggaaaaggagatccttgcaattttacggcgtaacccgctgattcagcagaacgaaattgcggacatgctgcaaatcagccgttcgcgcgttgcggcgcatattatggatttaatgcgcaaaggccggattaaaggcaaaggttacattctcaccgagcaggaatactgcgtagtggtggggacaatcaatatggatattcgcgggatggcggatatccgttacccgcaatcggcttctcatcccggtacaattcattgctcagcgggcggcgtgggacgcaacatcgcccacaatctggcgctgttaggccgtgacgtccatttgctttcagtgattggcgatgacttttatggcgaaatgctcctggaagaaacgcgccgtgccggcgtgaatgtctccggctgcgttcgtttgcatggtcaaagcacatcgacgtatctggcaattgccaatcgagacgatcaaaccgtgctggcgattaacgatacccatctgctggaacagttgacaccgcaactactgaacgggtcgcgcgatttacttcgtcatgcgggcgtggtactggctgattgcaacctgacagccgaggcgctggaatgggtctttaccctcgctgatgaaatcccggtgtttgtcgataccgtttcagaattcaaagcgggcaaaatcaaacactggctggcgcatattcacaccctgaaacccactttaccggagctggaaattttatggggacaggcgatcaccagcgatgctgaccgtaataccgcagtgaatgcattgcatcagcaaggtgttcagcaactgtttgtttatttgcccgatgagtcagtttattgcagcgaaaaggatggagaacaatttttgctgaccgcgccagcgcatacgacagtagacagttttggtgctgacgatggttttatggcgggcctggtatatagctttcttgaaggatacagtttccgcgacagcgcccgttttgcggtagcctgcgcggcaatttcgcgcgccagcggcagcttaaacaaccctaccctgtctgccgataacgcgctttcattagtgccaatggtgtaacaatgttgccggatgcgacgcttaacgcgtcttatccggcctacaaatcaggcaatttcagcaagtaaatgtaggcctgataagcttgcgcatcaggcaatgacactcaagctaaaccaataaagaacccggcaatggtcgcactcatcaagttggaaagcgtcgccgccgccagcgcccgtaaaccaagctgggcgatttccggcgcacggtgtggcgcaaccgcagaaaacgcccccaccaccaccccgatagaaccaaagttagcgaaaccgcacaacgcgaaggaaataatcgccacagttttagcatcgagagtgccagccgtttgcagatagggtgagaaattgagataagcgacaaattcatttattgccagtttctgtccaatcaaactcccggcaagattcgcatcactccagtccacacccatcacccacgccagtggagccagcaggtaacctaaaatggactccagcgaggcatgttcaaaaccaaaccagccaccaacgccgccgataataccgttaatcaacgcaattattgcaacaaatgccatcaccactgttgccacacctgcggcgattttcagcccggtcattgcccctgtcgcagcggcttcaataatgctttttggcggtgtttcggtgaaagagaggttattaaaggaaacctgcgaagattccgttgccgggcttaacaggcgggcaaacaagatcccgccagggatcgccattaatgatgccgccagcagatattccacaggcacgcccagtgcggcgtaaccaatcattgtcgaaccagcaatcgaggccatgccactacaaatcgctgtaaataattcattgcgattcagacgatcgataaagggtttgacgattgccggaatttcgttttgcccgaggaaaatggtggtgaccgcgacgaatgactcgatcttgctgatatttaatgctttctggaagataccgccgagaattcgaattaaaatccccatcacaccgatgtagtagagaatactcaccagcgcggtgacgaagataattgccggtaacaccctgaaaccaaagataaatcctgcaccatcaaataaggtatccattttcggtccgaccagagaaccgaagataaatgcgctacccgcgtcgctgtacgccatcactttatgcacgccaaaagcgactttttcagcgacccaacgccctggcggtaaccaaagcataatgccgccaatcacgacctgtaacactaacgccgcgccaacggtacgcaggctgatcttcttcttgtttactgacagtaaaaacgcaatcgtcagcaataccaccattcccagaacacttctcatgacatccatagtgattatctcttcatgtcatattgggcgacggctttctgcccatcagaaatagccaggcctgcatcttgcgataccggcccggcttgttatcaacacttaatgggttttgatgtagccgcgcacgcactcttcgactaatccccagaaccagtctgtatcaatagtgatgccgactttggtattggcgggcttgccaagaacgcccagctcgtcgcagacggtacgcccatagcaagggccactgttgacgtccacttcgacgtacatctcctgggttttaatgccatcagggttaatcagataaccgatgcaggtggcgtcgtgcaccgggccgccagcaaggccgtagttttcgaactgcgttttgagagtgaagttcatgatgtcgctgaacagctctccggcggggccgcctgccctttccatccgagcaatcacgtccggggtgcaaacggtctggttggtgagatcgaggcccatcatcactaatggaacgccggaggtgaacactacgcgtgcggcttccgggtcggcaaagatgttgaactcggcagatggcgtgaagttgcctgtaccgtaagcgccgcccattagcacaatttcacggattttgggcaggatcgcgggttgcatacgcattgccaccgcgatatttgaaagcggaccaaccggcaccagagtgatatcgccatcgcttgccatcagggtatcaatgatatatttcaccgcatgagtgctttctgcctggcgggtcagcggctcgaataccgggccatccagtccggtttcaccgtgaatattatcggcaacgatttgttgacgcataatgggctgcggcatccccgcataaaccggaacattaatctccagtttctggcaaacattcaggccattaattaatgttttatcaagcgtctgattacccgctacaatagtgatgcctaataaatctattgccggatgtttcgccgccatcattatagcaatagcatcatcatgacccggatcacaatccagaataatttttctcttttccattgtttatttcctctgtttccagttgcgttattttttctacagcaaagaaaattcgaccgggccgatgattgaatcttaacaacagcgtacgtatgctaaatatgagaaatctcatagcggataaacatcgtgaaagaaatccacaataatgatcttaagcagcaattgatgagtgaatccgcgtttaaggattgctttttaacggatgtttcagccgatacgcggctgtttcattttttagcgcgtgactacattgtgcaggaagggcaacagccgtcctggctgttttacctgacgcgaggccgcgccaggctttacgccacgctagctaatggtcgcgtgtcgctgatcgatttctttgccgccccctgttttattggcgagattgagttaatcgataaagaccatgaaccgcgtgcggtgcaggctattgaagagtgttggtgccttgcgctccctatgaaacattaccgtccgctgttattaaacgacacgctatttttacgaaaactctgcgtcaccttaagtcataaaaattatcgtaatattgtttctttaactcagaatcaatcatttccgttagtgaatcgcctggcagcatttatattactctcgcaggaaggtgatctttatcacgaaaagcatacgcaagcggcagagtatttaggcgtttcttatcgacatcttttatatgttctcgcgcagttcattcacgacggtttattaattaaaagcaagaaagggtatctcattaaaaacagaaagcagttgtcaggactggcgctggagatggacccggagaataaattctccgggatgatgcagtaaaaattattttcaatagcgcgattgccggatgcaacgcttaatacgttttatccggtctacaaatcgagcattacgccagaccaataaagaacccggcaatagtcgcactcatcaggttggaaagcgttgctgctgccagcgcccgtaaaccaagctgggcgatttccggcgcgcgttttggcgaaatagccgaaaatgcgccaacgacaacaccgatagaaccaaagttagcaaaaccacaaagcgcaaaggagataatcgcaatggttttcacttccagcgtgccgcccgtttgcaggtatggggagaaactcaggtaagcgacgaattcgttaatcgccagtttctgcccaatcaggctacccgcaagattggcatcactccagtccacacccatgatccacgccagcggtgccagcacatagccaaaaatactttccagagaggcattggcgaaaccaaaccagccgccaattccgccgataatgccgttgatcagcgcaataattgcgacaaacgccattaccaccgtcgccacaccagcggcgatttttagcccggtcatcgcaccgctcgccgccgcttcgataaagctttttggcggcgtttcgctgaacgacagattttcaaatgtgacctgcgaaggctcggttgccgggctaagaatacgtgcaaacaaaatcccgccagggatcgccatcagcgatgccgctaacaggtagtcaattggtacgcccattccggcataaccaatcatcatcgaaccagcaatggacgccatcccgctacaaattgcggtaaacaactcgttgcgattcatgcgatcgataaacggtttaacgatcgccgggatctcattttgcccgaggaaaatagtagtaaccgcaacaaaagattcgattttgctgatgttgagggctttctggaaaatgctgccaaggatgcgaatcagcagccccatcacgccaatgtagtacagcagactgatgagcgcagtaacgaaaataatcgccggaagtacgcgaaaggcgaagataaaacccgcaccgtcaaacaggacatccattttcggcccaaccagcgaaccaaaaatgaaggcgctaccggcatcactgtaagacatcactttatgaacgcctaatgccgcctgttctactgcccattttcccggtgggaagtagagcatgatgccaccaatagcgatttgcagcagcagtgcggctccaaccgtgcgcaaactgatgctctttttattcactgacaacagaaatgctattgccagtaacaccaccatccccacaacacttctcattatatccataatgattttcccttcatgccggtaaacccggcgtcagcgccaggttttggtatgcttgatgagtacgggcgacggctttctgcccgtcagaaattaacccgcgagacgctgatattctttggcaatttcgctcgccagaatggcgttgttgaacaccagctggatgttggatttcaggctgtcaccgccggtcagttcagcaacgcgcgccagcaggaatggcgtactttctttaccaatgactccctgagcttcagcttcagctaccgcctgatcgatcgccgcattgatagtgtgttccggcatagcaaactgttccgggatcgggttcgctaccacgaggccaccgttcagaccgctttgccatttcaccaccattgcacgggcaatttcgctggcgctgtcgagacgaatgctgacgtcaaacgggctggtgcggcagaaaaacgcaggcagcgctttagtctgatagccaattaacggcacaccgaaggtttctaaatactcagtggttaatcctaaatcgagaatagatttcgccccggcacaaacaacggtgacattagtatttgccagttcttgcaaatcggcagaaatatcgaaggtatgttccgccccgcgatgcacaccaccaattcccccggtggcaaatactttaattccggcaagcgccgcaataatcatcgttgaagccacagtggttgcgccattttttccggcggcaacaacaaaaggtaaatcgcgacgactaactttggtcacgttatgcccttcacgacccagtaattcaatttcttctttgcttaaccccactttcatcacgccgccaataatggcgatcgtggcaggtacagcgccctgtttacgaatagtttcttcaacttcaattgcggtctgggcattttgtgggaacggcatcccgtgagaaataatggtcgattccagcgccacaaccggttttttgttttttaaagcgtcctgcacttccggggaaatttgtaataattcaggggaaatttttaattcagacattctgcgttctccactaacgatataacgttggcaatcgataaatcggggttattggtgtattcacaggagagcgccattgacgaacatccctgtgcgaaacgaacagattcggcaaacggcattccgtctacccaacacgaagcaagtcccgccatcatggcatcgcccgctccggtaacattaataacattggttttgatcggcgcagaccagccactttcaccgctgatatcgctgtaataaacgccgtcgccgcccatgctcaataccagtcggttcaggccatgttgatggaaccaggcagcaacttttgccacatcttcacgccctgacagcgcaatcccactcagggtttccgcttcaaggcggtttggcttgagagtgtggatctgatttagacggtcgcgcactttgacacatttccatgccgaaaccggatcgacaaatacgggtacgttggcggcattatccagaatccatgccagtgcctcttcactgatattacagtccgcgacaatgacctttgccctctgaataaattcaccgtgctgtgcgagatattcagctgtaatagcgttgctaatattcatgtcatttatagcaaccagcatttcaccggtattatcgagtaatgataaataactcgacgtattttctcccggcacaatcaggcatttatcgacataaacgccagattgattggtttgcgttagcagcgattgaccataaaaatcactgcctacggcgctcagtagccaggctttgttacccagcaacgccaggttttgtgcaatattgcgccctactccaccaggcgtaaattttattttacctggatttgaatccgcataatttaatgattcatgtgaatatccggcgacatcaatattcgccgaacctataattacgacataatccttttcgcgcatagcacgtcctctggtaaaaaattaccaaccctgtcaatccacaagaatatagatactgcaaagacggtttaaacatgtgttcatatttaaacatgtgctcatagtatgcatgttttacgtaaagtaaattaccgccagagaggcaaaatgggcagatttgagcaggctcacaaaatgcgattaaatgcctgaattacaaaagcgaggaatttgtgacgggatgcacagaacagaacaataaaaaagggcagaaaataatctgcccttgaggaaataacctgagtgtttgatgaacgtttgaagtttctactgaaagataaaaccatttaaattcataaaattacattcacaaaccggtcattctctttgcgctcatcaaatgttacaggacaggaaatttctgccctgtaacacaccttttattacgctgctttcgctactgcgtccacttccggacgtttcaggaaggcataggccaaacccgccaccagcgtaccggcaataattgctaccaggtaacccaataccggcgtaatagcgccagggatcagcagaacaaacagaccaccgtgcggtgccatcagtttcgcaccaatcgccattgagattgcgccagtcagcgccccacccacgatacagcacggcagcacacgcatcggatcacgagcagcaaacggaattgcaccttccgaaatgaagcacagtcccaataccagagcggctttgccaccttcctgctgcgctttgtcgaatttgcgacgcgccaccattgttgccagacccattgccagcggtggcaccatacctgccgccataatcgccgccatcgggccataggtttgagtactcagcagacccacaccgaatgcgtacgctgctttgtttaccggaccgcccatgtcagtacacatcatgccaccgaggatcgcccccagcagaaccgcattcgcagtccccatggtctgcagccagtgagtcagcccttcgagaatgccagcaactggtttaccgatcaggtagatcatcgccagaccgaccaccagactggaaattagcggaatgatcaggatcggtttcagcgcctccatactctgtggcagtttcaattgcgtactgattaacttcgcaatgtaaccagccaggaagcccgcaataataccaccaatgaagccagaaccggtgctgaccgccagcataccgccaatcagacccggagtgaggcccggacgatcggcaatggaaaaggcaatataacctgccagtaccggcaccatcagcgcaaaggctgaaccaccaccaatctgcatcagcgccgcagccaacgtacccggctctttaaacgcttcgataccaaaagcaaaagaaagcgcgatacacagaccacctgcaacgaccatcggcagcatgtaagaaacgcccgtcagcaagtgacggtatgcgcctgcactctctttcttactttcagtggtcgccgtttgagctttgcccgccggttcatacggcgttgcttcagcaaccgctttatccagttcctgcgcggttttcttcagcgccagaccggtagaggtacgatacatcggtttaccagcaaatttcgccagatccacttcgatatctgccgccacaatcaccagatccgctgctgcgacttcttcgggagtgattgcattacccgcgccaacagaaccacgggtttcaactttcacccaccagccacgttttttcgcttcggtttcaatggcttcagccgccataaaggtgtgtgctacgccagtcgggcaagcagtcaccgcaactacgcgtttcggaccgctggcggcaactggtgctgtcgcagcgaccggcgcagtgtaaggtttcgcatggcctttggcttcactcaggaacagctcagggtgcgcaactgcccgggaaatatcgcccagccagacatttttaccgttcagcgcgctgtcgttcgggatggaatcaccgagaacaatcgccatttcagcgtcgttcggattgtcgatgatttccagttttgcttttcgcgccgccgcgcccagcagggtcttcgccatataggcgcgtgcctgaccgagattagcgtcaataatcagcagcgttttcattatgcctctcctgctgtcagttaaaaggttgtaagtcgacgcgcgccatcattgcggccaactgcggacgatcggtaatacccacattgctttgacttaccgccagggctgcaacagctgtcgccagacgcagtgtgtgttcactggattcacgcatcagcaagccataaatcaggccaccaaccatagaatcccctgcgccaacggtgcttacgacatcgactgacggtggtttggcgatccattcgccggaggcattaacccaaagcgcgccttcggcacccagtgaaataacaacatgcgcgatgccttgttcacgtagcgcatgtgcagcttcaatcacatctttcatttcaggcagtttacggcctgcccagatttccagctcgcggcggttaggtttcaccagccacggtgccgctttcaaacctgctactaacgcttcacggctactatcaaagataatgcaaggacactgactacgcaggcgagtcatccagtcggtgaacgcttccgggctgacgcctgacggtaagcttccgctgacacagaccatatcgaactgaccgagccagctcagagaatcagtcacaaagcgttcccagtcggcgggggtgacttcaaaacccgagaagttgaagtcggtcacttcgccgtctttttccgtcagcttaacgttaattcgggtgcgcccctgtacaacctggaaacggttggcaatgcccagctcgctgaacagttgctgaaaaccatcctgattgtctttacccaggaagccgccaacggtgacatcaattcccaggtcttttaatactttggccacgttgatgcctttacccgccgcatgcagaccggtggttttcaccaggttcacttcgccgcgttcaatttccgggcagaaaccaacaaggtcataagccggattaagggtgatagtagcaacacgtctgctcattatgcgccctccccaagaccagcagcgatagcgtcgccgattgctttcagcgcctgttcagcatctgcaccctgggcggtaaagcgtaggcgatgacctttcttaacgccaagtgccacaactttcatcagactacgtccgtttgccggtttgccggtaccatcaaggtttgtcacggtaatatcactgttaaattgtttaatggtattgaccagcatggtacctggacgagcatgcaggccgtgttcattgcgcaccacaaactccgcgcttaacacgtcgtcggtcggcgcatcatcgctggtcagcagcgccagcaacgttgccgcatccgctttcagcaagcggtcagctttattgtcgagcaataaatcagcgagacgcttaagaaccgcgatgggctgatcgtcattcatcgccacactcaccagcatggctgccgtttcgccgtccacatcaaaagcatttgccgcacggcttaccgcaatcgcgctacgcagattgccttcggcgctatcgctcagccagataccctgtccgagattcagcggttgttcattgatggctttggtgacgaaagtggcgtcaactgcccccgcctctttcagacgcgcagcgttcagcgcctgaagagtcagcagatcgctggcgacgatatccagtgtcagcatttcgttgtcgagcttcagctgctcactctgcttttcgcccatcagtaatgcgcgaagttcttctgctgttgttgctgacttcagttgttcagcaacggaatcatcgctcagtacgtgggtcagctggcgtagcaggcccagatgttcatccgagctggcagcaataccgattgccacgtacgctacctgaccgtcaccccaggtgacgccttccgggaactgaaatacctgaacgccggttttcagcacctgatcgcgggtgtcggtagtgccgtgtggaatagcaataccattgccgaggaacgttgaggtttgctgttcgcgcgccagcatgccattgacgtagccttctgctacattaccggcctgcaccagcgccgcagcgacctggcgaatcgcctcttctttgtctccggccttttcgcccggatggatgtcctgtacggataactggaacatagttctcctctcttgctgaattgaaacgattcagcctctatgagaaaaaaagcgccaacctggcttagggttaaagacaagatcgcgctgaaacgtttcaagaaagcataatacttctgtttcagcacgcaaggaaagccgtaaagttatgagcaaaagtttgatgtgctgcacaattttttgccatttttcctaattgctgatgggaaaatccgttatcagcaatttcatttcagcagcgtcagcagccaatcagcaacagtgaaatggcattttgactattcgtggcgcttttgatttcgctgtctgtttattttctgacaagcagcgtaaactccgcgtcttcctcttccagtgatcgaccagcatgcataactcccccgcagtctccagcgcgaaatcgtttgacctgacctcgacggcgtttttaatcgttgcctttctcaccggtattgcgggcgctctgcaaaccccgacactcagtatttttcttaccgatgaagtacatgcccgtccggcgatggtgggattcttctttaccggcagcgctgtcattgggattctggtaagtcagtttctcgccgggcgctctgataagcgcggcgatcgcaaatcgctgattgtcttttgctgcctgttaggcgtgctggcctgcaccctttttgcctggaatcgcaactactttgttttgctattcgttggcgtctttcttagcagctttggctcgaccgctaacccgcaaatgtttgcccttgcccgtgaacatgccgacaaaaccggacgtgaggcggtgatgttcagctcttttttacgcgctcaggtttcactggcatgggtcattggcccaccgctggcttatgccttagcgatgggtttcagctttacggtaatgtatctgagcgcagcggtagcgtttattgtttgcggtgtgatggtgtggctgtttttaccgtcgatgcgaaaagagcttccgctggcgaccggcacgatcgaagcgccgcgccgtaaccgtcgcgatacgctgctgctgtttgtcatttgtacattgatgtggggctcgaacagcctgtacatcatcaacatgccgctatttattatcaacgaactgcatcttcccgagaaactggccggtgtgatgatggggaccgccgccgggctggaaatcccgacgatgttgattgccggatatttcgccaaacgtctgggtaagcgtttcttaatgcgcgttgctgccgtgggtggcgtctgtttttacgcaggaatgctgatggcgcattcacctgtcattctgttgggcttgcagctgctaaatgctatttttattggcattctgggcggcatcgggatgctctattttcaggatctgatgcccggtcaggcgggttcagccaccacgctctataccaacacttcgcgcgtgggctggatcatcgcaggatcagtggcgggcatcgtcgccgagatctggaattatcacgctgtgttctggtttgcgatggtgatgattatcgccactctgttttgcttactgcggattaaagatgtttaaggcgcggtcagcatttccagatcgataagccaggtcatggcctgctgacgcgagttaccgcacatttcagcgctggcttgtaagcctgcacagactttcggtcgcagtggcgaggtgaaaattttacagcgttgctgttcatcaagctgaatgcagggcgtattggcgggcttgccatctggcataccgggaatagggctggaaattgaaggggcagtgcaacacgccccgcaacccggacggcattccatacgttgttctcttaaggttaaccaccggattgatgagcgcgcacagtaccaccttttttgcaccagcaaaagtgcgaataccacttgcccgaaaggcccgtcgcgagtactttgtcgcgatatttttgacattttcgactacaggaatttttcgatgccaagagcgaacgaaattaaaaaaggtatggtactgaattacaacggcaaactgctgctggttaaggatattgatattcagtcgcccactgcccgcggtgccgctacgctgtacaaaatgcgtttttctgatgtccgtaccgggctgaaagtagaagagcgtttcaaaggtgatgatatcgttgacaccgtgacgctgacccgccgttacgttgacttctcctatgtcgatggcaacgaatatgtctttatggataaagaagactataccccgtataccttcaccaaagatcagattgaagaagagttgctgtttatgccagagggcggcatgccggacatgcaggtgctgacctgggacggtcaactgctggcgcttgagctgccgcagaccgttgatctggaaatcgttgaaaccgcaccaggcatcaaaggggcatctgccagcgcccgtaacaaaccggcgacattgagcactggtctggtgattcaggtaccagaatacttaagcccgggcgaaaaaattcgtatccatatcgaagaacgccgttatatggggcgtgctgactaacttcagccgcatgcagaaaagggatagctcaggctgtcccttttttaatttattataccaatcttctattttgcgcttcctgaacaccttacgccctcaattttcactcgttgattgatcgccctcacacttcatcgcattaacaatccagaccaatttcaattgctgtcatataactttacactgtcgttgttaattaatcgttactaagacgtgactcctatgaatacaatcgcctccgttacgctcccgcatcatgtacacgctccacgctatgatcgccagcagttgcaatcacgtatcgttcattttggctttggagcctttcaccgcgctcatcaggcgttactgaccgatcgtgtgctgaatgcccagggcggcgactgggggatctgtgaaatcagcttgttcagcggtgatcaactgatgagccagctccgcgcacagaaccatttatataccgtgctggagaaaggtgcggacggcaatcaggtgataattgtcggtgccgttcacgaatgccttaatgcaaaactggattccttagcggcaattattgagaaattttgcgagccacaggtggcaattgtttccctgacgattaccgaaaaaggctattgtattgacccggccaccggtgcactcgacaccagtaatccgcggattattcacgatctacaaacccctgaagaacctcactccgcaccgggtattctcgtcgaagcactgaaacgccgccgtgagcgcggccttacaccgtttaccgtgctctcctgcgacaatattcccgacaatggtcatgtggtgaaaaacgcggtgctgggaatggcagaaaaacgttcgccagaactcgccgggtggataaaagagcacgtcagttttccgggaaccatggtcgaccgcattgttccggctgcaaccgacgaatcactggtggaaatcagccagcatctgggggtgaatgatccctgcgcgattagctgcgaaccgtttatccagtgggtggtggaagataacttcgtcgctgggcgtcctgcctgggaagtcgcaggtgtacaaatggtgaatgatgtcctgccatgggaagagatgaaactgcggatgcttaatggcagccactcttttctcgcttatctgggttacctctcaggattcgcccatatcagtgattgcatgcaggatcgcgcatttcgccatgccgccagaacattaatgctggatgagcaagcgccgacactgcaaattaaagatgtcgatttaacacaatatgcggataagttaattgcacgttttgctaatccggcgctgaaacataagacctggcaaatcgcgatggatggcagccagaaattaccgcaacgcatgctggcaggtattcgcatacatcaggggcgcgaaacggactggtcgttgctggcattaggcgttgcaggctggatgcgttacgtcagcggcgttgatgatgccggaaatgccattgatgttcgcgatccgcttagcgataaaattcgcgaacttgttgcgggcagcagcagtgaacaacgcgtaaccgccctgctttccctgcgtgaagttttcggtgatgatctgccagataacccgcattttgtgcaggccatcgaacaagcctggcaacaaatcgtacaattcggcgcacatcaggcgctattaaacaccctcaaaatttaacgatttctgcggttaaagcggatgaagctcaccttcgtccgctctccccttctcttttctgccttttttagccaggattaacgctcagttaacttaccagagtattgcggagccgttgtgaccaggaccaacctcatcaccggttttctcggcagcgggaaaaccacgtcgattcttcatctgttagcccataaagatcccaacgaaaaatgggcggtactggttaatgaatttggggaagtcggaattgatggtgctttgctcgccgatagcggcgcattgctgaaagagatccccggcggctgcatgtgctgcgttaatggtttacccatgcaggtagggttgaataccttactgcgtcagggaaaaccagaccgcttgttgatagagccgaccgggctgggccatccgaaacagatcctcgatctgttaaccgcaccagtctatgaaccgtggatagatctgcgcgccaccttgtgcattctcgatccgcgcttgctgctggacgaaaaaagcgccagcaatgaaaacttccgtgaccagctggctgccgcagacatcattgtcgccaataaatccgaccgtacgacgcccgaaagtgagcaagcgctacagcgttggtggcagcaaaatggtggcgatcgacaattaattcacagtgagcatgggaaagttgacggtcatcttctggatttgccgcgtcgcaatttagccgagttgcccgccagcgccgcgcattctcatcagcatgtcgtgaaaaaagggttagcagcgttaagcctgccagagcatcaacgctggcgtcgcagtctgaacagcgggcaaggatatcaggcctgcggctggatattcgacgctgatacggtattcgacaccattggcattctggaatgggcgcgacttgcaccggtggaacgcgtcaaaggcgtgctgcgtattcccgaagggctggtgcgaatcaaccgtcagggcgatgacctgcacattgaaacgcaaaacgttgcgccaccggacagccgtattgagctgatttccagcagcgaagctgactggaatgccttgcagagcgcgctgttgaagcttcgtttagcgactaccgcgtaaggttgcctgcgtttttcagtaagataattagagaaaatatgattaaaaatttgccgcaaatagtgttgttgaatattgtcggcctcgcgctgtttctttcctggtatatccccgttaatcatggattctggttgccgattgatgcggatattttttatttctttaatcagaaactggtcgaaagtaaggcctttttgtggctggttgcattgaccaacaatcgcgccttcgacggttgttcactgctggcgatgggtatgttgatgctgagtttctggctgaaagaaaacgcccctggcagacgacgtatcgtgattattggtctggtcatgctattaactgcagtggtattaaaccagctgggtcaggcattaattcctgtaaaacgggccagcccaacattgacttttaccgatattaaccgcgtcagcgaactgctctctgttcccacgaaagatgcctcacgagatagctttcccggcgatcacggcatgatgctgcttattttttcggcattcatgtggcgttatttcggcaaagttgcaggccttatcgcccttattatttttgtggtttttgcatttcccagagtaatgattggcgcacactggtttactgacatcattgtcggttcgatgaccgtgatattgatcggtttgccctgggtgttgctgacgccattaagtgatcgattaatcaccttttttgacaaatcactaccaggaaaaaacaaacatttccaaaacaaataactcacagtaattaacatcatcagggttatttttatagtgaggataatcctgatgatgcgcaccgtgctttcatctatcgaacgcaaaaatcattctctaagtaaatgaatggattgcatgcgtttcactcaattgtactttaattgaccaaccccgcttattaactttctgtatcactttttcttataaaaaatcatgtaaaaccgctcgccaagaccgcaccaatcgggtaatctcgaactcgttttgcctcggcggtagattatcctcacagcatataattttgtgcgttagtccacagatttggccttaaggaattgtttcaacatgcccaggtaattagtctcgtgtcgcttggcatttttttataacgatatttgtcgttaaggacttcaagggaaaacaaacaacatggtcaaatctcaaccgattttgagatatatcttgcgcgggattcccgcgattgcagtagcggttctgctttctgcatgtagtgcaaataacaccgcaaagaatatgcatcctgagacacgtgcagtgggtagtgaaacatcatcactgcaagcttctcaggatgaatttgaaaacctggttcgtaatgtcgacgtaaaatcgcgaattatggatcagtatgctgactggaaaggcgtacgttatcgtctgggcggcagcactaaaaaaggtatcgattgttctggtttcgtacagcgtacattccgtgagcaatttggcttagaacttccgcgttcgacttacgaacagcaggaaatgggtaaatctgtttcccgcagtaatttgcgtacgggtgatttagttctgttccgtgccggttcaacgggacgccatgtcggtatttatatcggcaacaatcagtttgtccatgcttccaccagcagtggtgttattatttccagcatgaatgaaccgtactggaagaagcgttacaacgaagcacgccgggttctcagccgcagctaataaaccgtttggatgcaatcccttggctatcctgacgagttaactgaaagcactgcttaggcagtgcttttttgttttcattcatcagagaaaatgatgtttccgcgtcttgatccaggctatagtccggtcattgttatcttttaaatgttgtcgtaatttcaggaaattaacggaatcatgttcatacgcgctcccaattttggacgtaagctcctgcttacctgcattgttgcaggcgtaatgattgcgatactggtgagttgccttcagtttttagtggcctggcataagcacgaagtcaaatacgacacactgattaccgacgtacaaaagtatctcgatacctattttgccgacctgaaatccactactgaccggctccagccgctgaccttagatacctgccagcaagctaaccccgaactgaccgcccgcgcagcgtttagcatgaatgtccgaacgtttgtgctggtgaaagataaaaaaacattctgttcatctgcgaccggtgagatggacattccactcaatgaattgattccggcgctcgacattaataaaaacgtcgatatggcgatcttacccggcacgccgatggtgccgaacaaacccgcaatcgtcatctggtatcgcaaccctttgctgaaaaatagcggcgtctttgccgctctgaatctcaacctgacgccttcactcttttatagttcacggcaggaagattacgatggcgtcgccctcattattggcaatactgcgctatctaccttttcttcacgtttgatgaacgttaacgaattaaccgacatgccagtccgtgaaactaaaattgcgggcattcctctgaccgttcggctttatgcagatgactggacatggaacgatgtgtggtacgcatttttactgggcggcatgagtggaactgtcgttggcctgctctgctattacctgatgagcgtacgtatgcgccccggcagagaaatcatgaccgccatcaagcgcgaacaattttacgtggcgtatcaaccggtggtggatacacaagctttgcgagtaacgggcctggaagtactgctacgctggcggcatcctgtcgcgggagaaattcccccggatgccttcattaactttgccgaatcgcaaaagatgattgtgccgctgactcagcacctgtttgagttaattgcccgcgatgccgcagaattagaaaaagtgctgccggtaggcgtcaaatttggtattaacattgcgccggaccatctgcacagcgaaagctttaaagcagatatccagaaactgctcacttccctgcccgcacaccatttccagattgtgctggaaattaccgagcgcgatatgttgaaagagcaagaagccacacaactcttcgcctggctgcactcggtcggcgtagaaattgctattgatgacttcggcaccgggcacagcgcgcttatctatcttgagcgttttacgctcgattatctgaaaattgaccgtggatttatcaacgccatcggtacggaaacgatcacttcccccgtacttgacgcggtgctgacgctggcgaaacgcctcaatatgctgacggttgctgaaggggtcgaaacgccggaacaggcgcgatggctaagcgaacgcggcgttaatttcatgcaaggctactggattagccgcccgttaccgctggacgattttgttcgctggctaaagaaaccgtatacgccgcagtggtaaggtgtgcttacgtcccttattattcatagtgaaagcatgccggattgcggctaatgatgagtaaaaggaaatccgttgcagatgattgtgcgcatactgctgctgtttatcgctctgttcacctttggtgtgcaggcgcaggctatcaaggaaagctatgcctttgccgtgctgggcgaaccccggtacgcgtttaatttcaaccattttgattatgtgaaccccgccgcgccaaaaggtgggcagataacgttgtcagccctcggcaccttcgataatttcaaccgctatgcactgcgcggcaacccgggcgcacgcaccgagcagctgtacgacacgctatttacgacttccgatgacgaaccaggcagttattacccgctgattgctgaaagcgcacgctatgctgacgattattcctgggtggaggtcgctattaatccgcgcgcccgttttcatgatggttcgcccattactgcccgcgatgtagagtttacttttcaaaaatttatgaccgaaggcgtgccgcaatttcgtctggtctacaaaggcaccaccgtcaaagccattgcaccgttaaccgtgcgcattgagttagctaaacccggcaaagaagatatgctgagtctgttttcgctgccggtatttccagaaaagtactggaaggatcacaaacttagcgacccgctcgccacgcctccgcttgccagtggtccgtaccgcgttacgtcctggaaaatggggcaaaatattgtctattcccgtgtgaaagattactgggcagcaaacttaccggtaaaccgtggacgctggaatttcgacaccattcgctacgattattacctcgatgataatgtcgcctttgaagcgtttaaagcaggtgcctttgatttgcgtatggaaaacgacgccaaaaactgggccacgcgttataccggtaaaaatttcgataaaaaatacatcatcaaagatgagcaaaagaacgaatcagcccaggatacgcgttggctggcgtttaatatccaacgtccggtattcagcgatcgccgggtccgggaagctatcactctcgcctttgactttgaatggatgaacaaggcgttgttttacaatgcctggagtcgcacgaacagttattttcagaataccgaatacgcggccagaaattaccccgacgccgcggagctggtgcttctggcaccaatgaaaaaagatctaccgtcagaagtcttcacacaaatctaccagccgccggtatccaaaggcgatggctacgatcgtgacaacctgttaaaagccgacaaacttctcaacgaagcgggctgggtgctgaagggtcagcaacgcgttaatgccacaacgggtcagccactcagctttgaattattgcttcccgcaagcagcaatagtcagtgggtattgccgttccagcacagcctgcaacggctgggtatcaacatggacattcgcaaggtggataactcgcaaatcactaaccgcatgcgcagtcgcgactatgacatgatgccgcgcgtatggcgggcgatgccgtggcccagttccgatttacagatttcctggtcatcggaatatatcaattccacttataatgcccccggcgtgcaaagcccggttatcgactcgctgatcaaccaaattattgccgcgcagggaaataaagaaaaattactgccgttggggcgagcactggatcgcgtattaacgtggaattattacatgctgccaatgtggtacatggcggaagaccgtctcgcctggtgggataaattctcccagccggccgtgcgccccatctatagcctcggtatcgatacctggtggtatgacgtcaataaagcggccaaactgccgtccgccagcaaacagggagagtagatgggcgcttacctgattcgccgtctgttgctggtgatcccaacattatgggcgattatcaccatcaactttttcatcgtgcaaattgcgcctggcggtccggtcgaccaggccatcgccgccattgagtttggtaatgccggagtattacccggcgcaggcggtgaaggtgttcgtgccagccatgcgcaaacgggtgtcggcaatatcagcgacagtaattaccgtggcggacgcggattagatccagaagtgatcgctgagatcactcatcgctacggttttgataagccgatccacgaacgttacttcaaaatgctctgggactacatccgctttgattttggcgatagcctgtttcgcagcgcctcggtgctgacgctgattaaagacagtctgccggtttccatcaccctcggattgtggagcacgctgattatctatctggtgtcgattccgttaggcattcgcaaagctgtttataatgggagccgctttgacgtctggagtagcgcatttatcatcatcggctacgccattccggcctttttgtttgccatcctgctgattgtcttcttcgcgggcggcagctatttcgacctgttccctctacgcggcctggtttccgctaactttgattcgctgccgtggtatcagaaaatcaccgattatctgtggcatatcacgctgccggtgctggcgacagtgattggtggctttgcggcgctgaccatgctgacaaaaaactcattccttgatgaagtgcgcaagcaatacgtggtgaccgcgcgtgcgaaaggggtaagtgaaaaaaatattctctggaaacatgtgttccgcaacgccatgctgctggtgattgccggttttccggcgacgtttatcagcatgttttttaccggctcgctgctgattgaggtgatgttttcactcaatggtctgggcttactgggctacgaagcgaccgtctcgcgcgattatcctgtaatgtttggtaccttgtatattttcaccctgattggcctgctgctgaatattgtcagtgatatcagctatacgctggttgatccgcgtattgattttgagggacgttaatgtcgcgactcagccccgtcaatcaggcccgttgggcgcgttttcgtcataaccgtcgcggctactggtcgttatggattttcctcgtcttgtttggtttgagtttgtgttctgaacttatcgccaacgataaaccgttgctggtgcgttatgacggcagttggtatttcccgttattgaaaaactacagcgaaagcgattttggcggcccgctggcaagtcaggctgattatcaggacccgtggctgaaacaacggctggaaaataacggctgggtactgtgggcaccgattcgctttggtgctaccagtatcaactttgctaccaataagcccttcccttctccaccctcccggcaaaactggctgggaacggatgccaacggcggcgatgtgctggcacgcattctctatggcacgcggatctcggttctgtttggcctgatgctgactctctgttccagcgtgatgggcgtgctggcgggggcgctacaaggctattacggcggtaaagtcgatctctggggacaacgctttattgaagtatggtcggggatgccgacgctgtttttgattattttactttccagcgtcgtacagcctaacttctggtggctgctggcaattactgtcttgtttggctggatgagtctggtcggcgtggtgcgggcggagtttttacgtactcgtaatttcgactacattcgtgcggcacaggcgcttggcgtcagcgatcgcagtatcatcctgcgtcatatgttgcctaatgccatggtcgcgaccctcacctttttaccgtttattttatgtagttcgataaccaccctgacctcgctcgatttcctcggcttcggtctaccgctcggttcaccgtcactcggtgaactgctgttacaagggaaaaataaccttcaggccccgtggcttgggatcaccgccttcttgtcggtggcgatattattgtctttgctgatctttattggtgaagccgtccgcgacgcatttgatcctaataaggcggtgtagcatgacgcaaactctgttagcgattgaaaatttgtcggtgggttttcgccatcagcaaaccgtacgtacagtagtcaatgatgtttcactacagattgaggctggcgaaacgctggcgctggtgggtgagtcaggttcaggcaaaagcgttaccgcgctgtcaattttacgcctgctcccttccccgccggttgaatatctctccggcgatattcgttttcatggcgaatcgctgcttcacgccagcgatcaaacgttgcgcggtgtacgcggtaataagatcgccatgatttttcaggaaccgatggtgtcgttaaatccattgcataccctggaaaaacagctttatgaagtgctttcactccaccgcgggatgcgtcgggaagcggctcgtggcgaaattcttaactgccttgatcgcgttggtatccgccaggcggcaaaacggctgacagattatccgcatcagctctccggcggcgaacggcagcgggtgatgattgcgatggcgctgttaacgcgaccggaattattaattgccgatgaaccgaccaccgcactggacgtctctgtccaggcgcagattttacagctgttgcgcgaactgcaaggcgagctgaatatgggcatgctgtttattactcataacctcagcattgtcagaaaactggcccaccgcgtggcggtaatgcaaaacggtcgctgtgtcgagcaaaattacgccgctacgctatttgcatcacccactcatccttacacacaaaagctactcaacagtgaaccgtcaggcgatccagtgccgttgccagaacctgcctcaacgttgctggatgttgaacagcttcaggttgccttccccattcgcaaagggattttgaagcgcattgtggatcataatgtggtggtgaaaaacatcagttttacgctacgagcgggtgaaacactgggtttagtgggcgagtccggttccgggaaaagtacgacgggactggcgctgctgcgactgattaattctcagggcagcatcatctttgacggtcagccactgcaaaatttaaatcgccgccagctgttacctattcgtcatcgcattcaggtggtatttcaggatccaaactcctcgctcaacccacgactcaacgttttgcagattattgaggaaggcttacgggttcaccagccgacgctttctgccgcacaacgcgaacaacaagtgatagccgtgatgcatgaagtgggattagatcctgaaacacgccaccgttatccggcggagttctctggtggtcagcgacaacgtattgcgattgccagggcattaattcttaagccctcgctgatcatacttgatgaaccgacatcatcactcgacaaaacggtacaggcgcaaatattgacgctattgaaatcattgcaacaaaagcatcaactggcctatttgtttatcagccacgatttgcacgttgtccgcgcgttatgtcatcaggttatcatactgcgacaaggggaagtagtggaacaaggaccgtgcgcgcgcgtgtttgccacaccgcagcaggagtatacgcgtcagctactggcgttgagctgacgcttaaaaaggattgtagtttgaaaagggttcggcaattgccacaccaaaatttttcaatcggcatgttgcagcaaactcgtcctggcgatttacaaacaggcacggctcaccttcacactccagcaccgaacatggaacttcgatgtcgcttaacgcctggcttagtttatacatcaccgaccatgcattatcaccatccgggctaagcaatttaagcgccaccaggctgttgtcaccgcacggtccattttgcggaatcggttcaaccttcgaacctgcgaaaccagcagaccagcgatagttctgcggcagtcgatggacgattgagagttgtaatgaagtcacttattttccccggaagcacattcacttcacaatttgtttacatcaattttaacacatcatcaacaatccgtctttatacagatcgtaaagattgatgcctcgcctgcgtggcctctatggctctgatttaagtaatatctgcgggcgtggtcacgtttgcggggctatatgtacccgtttctgcgatctaactcaacctttttaactacaatgatgtgactttttacataaattgattttacataaaataaacatatatcgggggaatgatagatttgtggttgacatgcatcaacaaaggaagccttttagcttcctcgttgtgcaatagatcaccgttttttcggccgactggcgtacagacagaagagaatggagctggttgcgcagaatgcaattgaccaaatcatcggccatgcagagttaaaggtcgcaagagaaagcaatgcgccaacaattgcccctatgccaaaacggaaggttcctgccagcgaagatgccgttcccgccatatggggaaactcatcaagaatgaccgccatcgcattggatgacaccatcgacacgcagcccacaaacgccgcaacgccaaccaccagcgaccaaaatcccagccccagcagcgcactgatgaccatccacgctgccataataaattgtatccacaaccccgagcggaacatatttaacgcgccaatgcggcggacgaagcggctgttaaagatggtcatcacgaacagaaaaacaatgtttagcgcaaagtaataaccaaagttttccggcgcgacgtggttaatttcaatataaacaaacggtccggcgcttaagaatgagaacatcccggcaaagctgaaaccactggcaagcatgtagctcaggacacgtttatggcggaacagcgccgcaaagttaccaatagtggtacgaatgtgaaatggctgacgacgctccggtggtaaggtttctttaatcaggaagaaaatcattgccgaagccagaatcgccgctaatgccaggatccagaagatgtaatgccagctcagccacaccagcacccagccgccaactatcggtgccatcagcggtgcaatggttgtcaccagcatgacaaacgacatcatccgcgagaactcttctttcgggtaaatatcgcgcatcagggcgttaatgaccacgctggccgcagccgcagccagcccgtggaagaaacgcatcacaatcagctgatcgatggtgtttgccaacgcacacgccaccgcggcggcggcaaacaccagcgtaccgccgagcaccaccggcttacgcccgaagctgtctgccatcggcccgtagattaactgccccaacgcaaagcccagaatataagtactgagggtcatctgcgtactgcccgccggtacgccaaactgcgctgaaattaccggtagcgcgggcagatacatatcaatcgacagcggcatcaacatggccagcaggccaaggataaaaacaatagcaaacgacgaatgctgtcgggtggtcacaacgggctcctgaaagtcattgaaaagttagacgacgctggcaatttcttcttcagttaacggacgatattcaccgggggctaaatcagcatccagcgtaataccgccaatacgttcacgatgcagctcaaccacgtggttacccacggcggcgaacatgcgtttcacctgatgataacgcccttcgctgatggtcagacgaacctgcgttggggtaatcacttccagcaccgcaggcttagtgagatctttttcgttatgcagctgcacgcctttagcaaattgctctgccgtatcgtcagctacaggtgattccagtgtcaccagataggtcttctcgcaatgatggcgcggagaagtaatgcggtgcgaccactgaccatcatcagtcatcagcaccagaccggtggtatcaatatccaaccgccccgccgcatgcagtttccacgctaccggttcatcaagaaaatagagcaccgttgggtgatcagggtcgtccgtggagcaaacatagccctgaggcttattgagcatgaagtaacgtggaccgtgttgctgcgccagcgggttgccatcgtaagcgacatcatgttcaggaagcagtttgaacgctgcattacggacgatttcgccatcgacggtgacacgattgccgcggatttcacgcccggcaatagcacggctaacgccgagttgctgtgcgataaatttatcaagtcgcatgtgtgtgattttgcctgtaaaaacggaggtcgggcattgacccgaaaatctgaactgttgtctgcccagtatagcggtctaataacatccctcaagggaaaaagatccatggcatactattagcagaataatctacctacgcgagaccatgatttttacacttcgcccatatcagcaagaagccgtggatgccacgctcaaccattttcgtcgtcataaaacccctgccgttatcgtgctgcccaccggcgcaggtaaaagcctggtgatagcggaactggcacggctggctcgtggtcgcgtgctggtgctggcacacgttaaagaactggtggcgcaaaaccatgcaaagtatcaggcgctggggctggaagccgatatttttgccgccgggctaaagcgcaaagagagccacggtaaagtggtatttggcagcgtgcagtctgtcgcccgtaatcttgatgcctttcagggtgaattttcgctgttgattgtcgatgaatgtcaccgtattggtgacgatgaagagagccagtatcagcaaatcctcactcacctgacaaaagtgaatccccacttacgcctgctggggctgactgccacgccttttcgattgggcaaaggctggatctaccagtttcattatcacggcatggtacgcggcgatgagaaagcccttttccgtgactgcatttatgagctgccgctgcgttatatgattaaacacggctatctgacgccgccagaacgactggatatgccagtagtgcaatacgatttcagccgcttgcaggcacagagtaacgggctgttcagcgaagccgatctcaaccgtgagctgaaaaaacaacaacgtattaccccgcacatcatcagccagattatggagtttgctgcaacgcgcaaaggggtgatgatttttgccgcgacggttgaacacgcaaaagagattgtgggattactgcctgccgaagatgcagcactgattactggcgacacccccggcgctgagcgcgatgtgttaattgaaaattttaaagcccagcgttttcgctatctggtcaacgtcgcggtactgaccaccggatttgacgccccgcacgtcgatcttatcgccattctgcgccctaccgaatcagtgagtctttaccaacaaattgtcgggcgcggtctgcgtctcgctccgggcaagactgattgcttaattcttgattatgcgggtaatcctcacgatctctacgcgccggaagttggtacaccaaaaggcaaaagtgacaacgttccggtacaggttttctgccctgcctgcggttttgccaacaccttttgggggaaaacgaccgccgacgggacattgattgaacactttggtcgtcgctgtcagggatggtttgaagatgacgacggtcatcgcgaacaatgtgacttccgtttccgttttaaaaattgcccgcaatgtaacgcggaaaacgatattgccgcccgccgctgccgcgaatgtgacaccgtactggttgatccggacgatatgttaaaagcggcgctacgactgaaagacgcgctggtattacgctgtagcggcatgtctttgcaacatgggcacgacgagaaaggcgaatggttgaaaatcacctattacgatgaagacggcgcggatgtgagtgagcgtttccgtctgcaaacacctgcccagcgtaccgccttcgagcagctttttatccgcccgcatacgcgcacaccgggcatcccgctgcgctggatcaccgccgccgatatcctcgcccagcaagccttattgcgacacccggattttgtcgtcgcccgcatgaaaggccagtactggcaggtgcgtgaaaaagtgttcgattacgaaggtcgttttcgtctggcgcacgaattacgcggttaatggtagttttgattgatgtataaggcgattgagtatagaatctcgcccgcttttgcatacgcaaagcagatcacttacctgttgctgggtcgcctgtagcaggattaatttaagagagaaagaaatgtttactatcaacgcagaagtacgtaaagagcagggtaagggtgcgagccgccgcctgcgtgccgctaacaagttcccggcaatcatctacggtggcaaagaagcgccgctggctatcgagctggatcacgacaaagtcatgaacatgcaagctaaagctgaattctacagcgaagttctgaccatcgttgttgacggtaaagaaatcaaagttaaagctcaggacgtacagcgtcacccgtacaaaccgaagctgcagcacatcgacttcgttcgcgcttaattgctgaataagttgtaaaaaaccccgctccggcggggttttttgtatctgcagattatgcctgattacggtattgctattttttgcaggccagataaggcgttcacgccgcatctggcattcagaacacaaaaccgattaattgccgccagacgtccggcgctgcaattggtcgcgcaaattcggcggcgtgcctttaatggtcaaggtatcggttgctggatcccagaagatgcgttcacctaacagcatcgcatcaaagttaatagtcaagccaccgccgctaccggcaaacttcgtcaactgacgcagtgtgctacggtctgccgggaagctctcttccagttcgtagcctttttcagccgcaaactccgtgaagctcacttcgcttacgcctgccagctctttcgacagcgatttcagttcgatctcttcgcctgcctgcagctgctcattacagtagctataaacctgctggcgcacgttctgtcgctctgctttatccagttgtgcttcggcagtgaaatcatcaaccgcttgcaacagcccacggttttgcgctttcgcgtttaacccttcgctggccccgaggaaatccataaagaaatccgccactttgcgccctactcgccctttcaggaaagtgagatagcgggtggactctggattggtttcccattcggttaaatcgatacgcgcaacaatatccgcatgattgatatcaagataatgggttgggttgatgtcgagattttcgttaacgcgcatactgctcaggttgctcagaactgccaccagcaaatactccaccgccagatagcgatagtggcaaaacagcacgaatccaccgtcagcaaaaggatatttcgctaattcgtcacgcaggcggccggttgccgcgcggctaaatgccaggaagtcctcttcgccctgacgctgtaagcgcagcgtctgcgccagttcactctcttcgctaaacaagccgtaagctttatttttggcgctatagacccgatgcagttctgccaccatctcaacgacggtttctgtcggttccagcaatgaatcgcgcaacaccagctcaaggttctgctcatcacgcttgataagctggtgcagagcaatctggttgatatccagactcatgataaactctcctttaagaccgggcggtattcaaccaccgccggttaagcgacgcaataaaagatggcggtcattttacagaaggcagcgtaacgagaatgatttaacgcataaaaaagcagaaaaaaaaccgttgctacggtaatatgttgccctttcatcaactaactgatttcgatttatgccacaaatttcccgctacagtgatgaacaggttgaacaattgctcgcagagctgctcaacgtactggaaaaacataaggctccgaccgacctttccctgatggtgttaggcaacatggtcactaaccttatcaacaccagcattgccccggcccaacgccaggcaattgccaactcttttgcccgcgccttacagtcctctatcaacgaagacaaagcgcactaagggaaacagataacaggttatggtaactcatcgtcagcgctaccgtgaaaaagtctcccagatggtcagttgggggcactggtttgcactgttcaatattctgctttcgctcgtcattggcagccgttacctgtttatcgccgactggccgacaacgcttgctggtcgcatttattcctacgtaagcattatcggccatttcagcttcctggtgttcgccacctacttgctgatcctcttcccgctgacctttatcgtcggctcccagaggctgatgaggtttttgtccgtcattctggcaacggcgggaatgacgctattactgatcgatagcgaagtctttactcgtttccatctccatcttaatcccatcgtctggcaactggttatcaacccagacgaaaatgagatggcgcgcgactggcagctgatgttcatcagcgtgccggttattttattgcttgaactggtgtttgcgacgtggagctggcaaaagctgcgcagcctgacgcgtcgtcgacgcttcgcgcgcccgctggccgcattcttatttatcgcctttatcgcctcgcatgtggtgtatatctgggccgatgccaacttctatcgcccgatcaccatgcagcgcgctaacctgccgctttcgtacccgatgacggcgcgacgttttcttgagaagcatggtctgcttgatgcgcaggagtatcaacgccgtcttattgagcaaggtaatccagacgccgtttccgttcagtatccgttaagcgaactgcgctatcgcgatatgggcaccgggcagaatgtgctgttgattactgtcgatggcctgaactactcacgcttcgagaagcagatgcctgcgctggcaggttttgctgagcaaaatatttcgttcacgcgccatatgagctccggcaacactacagacaacggcatctttggcctgttctatggcatctcgccgagctatatggacggcattctgtcgacccgtacgcctgcggcattaattactgcgcttaatcagcaaggctatcagctggggttattctcatcagatggctttaccagcccgctgtatcgccaggcattgttgtcagatttctcgatgccgagcgtacgcacccaatccgacgagcagaccgccacgcagtggatcaactggctgggacgctacgcacaagaagataaccgctggttctcgtgggtttctttcaatggtactaacattgacgacagcaatcagcaggcatttgcacggaaatatagccgggcggcaggcaatgtcgatgaccagatcaaccgcgtgctcaatgcactgcgtgattctggcaaactggacaatacggtggtgattatcactgccggtcggggtattccactgagcgaagaggaagaaacctttgactggtcccacggtcatctgcaggtgccattagtgattcactggccaggcacgccggcgcagcgtattaatgctctgactgatcataccgatctgatgacgacgctgatgcaacgcctgctacatgtcagcacacctgccagcgaatattcgcaaggtcaggatttgttcaaccctcaacgccgtcattactgggttaccgcagcggataacgatacgctggcaattaccaccccgaaaaagacgctggtactgaacaataacggtaaataccgcacttacaacttacgtggtgaaagagtgaaagatgaaaaaccacagttaagtttgttattgcaagtgctgacagacgagaagcgttttatcgctaactgattaattataaatcagttagcgaaatatcttacttgcaatcggtgtggaaaacggtagtattagcagccacgagtcggcacgtagcgcagcctggtagcgcaccgtcatggggtgtcgggggtcggaggttcaaatcctctcgtgccgaccaaaaatcccaagaaaaaaccaacccttacggttggtttttttatatctgcaattaattcgataaacagaccgtgacacatcacagcctgtttattttctgttatcagaacgtccagaccacacccgcctgagtattccacggcgattctacccctgcgccattgccatagctgactgacaaatgaccgcttaacgtcggggtaaacgatgaccttataccagcctgataaacgccactggttccagccacatcattattaaatttgccatcgtcattaactttcacctggttagaatcggcgtattcctgacgcacggccgctttcagccagggttccagcgtcgtaccgttttgcaggtccatgtgatagcttaccgccgttcccgcttcagcgcgtaatatccgggtatttcccacatccgcgcgcatgccgtttgataacgtgtagtcctgaccatctgtggtaaagccggtaaaggccagatagggtctaacactccacaatccgtcaacccaacggaacccgctctcaacatgagcacccgcgccgttactattgtaatcgccaaacgctgttgccccattactcatcttgccatggatggtgttggcaaaacggtcaactttcaccaccccatcaacataggcaccgttctgatgctcccaaccggcataagcccccagggtatagctatcgatattacctttgccgccgcgatcaaaaccaatatcagaatgagagtaaccaaagatcaagccgcgaattgtactgctttcttcacgggagaaacggctatcgataccgagcgtcaggcccgtcaatgtttgctcaaaaccagctcccgcatcagtggtcacgttgttgcgggtgttaattgccgaactccacatcgccgtatcgtaactaacgccttttacgctaccaagacgctcacgcacggtgtccagttctgcatcaaataccagcggttgtgcggccgccatattcagcacatcagtggttgaaggggtaatttgcgcgcgattctctgccagactccagctatggttgccattatccagcaaggtatattcatacgtaccgatatcaacaacgcctccggcattgcccaacgtaaatgcagcatcaccgccgcccgttgttaccagtgtaaggctatctcctgctgccgggctggcaccggtgtccgtcacgaatattttgaaatcacctgttgcctgaccggtgacgttgagctgatcgctctgatgattagccatatcggtacgcatataaaaattgccgtttcccgacagggtattggtggtcaacgtaatgaaattttccgcacttgccgtcactgatgaacgagtcactggctcatccatcataatcacatttgcgtcagacatcgcaaggttggctaagttgaggagggtgttttggttcgtcgtagtgatatcggcaatgatggtccatacgctattttcgagcgaaacgtccgctttgctggtatccacggcaccatgcgttctaaaagaagcgccctcagaaaccactaccttacccaccaacattgcgggtgcataatttatttgcggcttcatgacctcaagaatgccatcattccctctgactgaaacgttaaccattgtgccagcccagacgttagcgcggccattgttgataaccatattttcagagatggcttttgaggaatacgtgatacttccattctgatatgatcgaccgagatcatataccgcatttgcctgcactttcgtaccagtatcctttcccagcgattgcatagtggcatgcttatcaaggatagtatcaatggcctgcgtgtcctccataacaatgagcccggaaccatcatccagttcataattttttgacacaccatcttttatactaaattggcctttactgtttggaccactcacttccagcgcattcgttgagacaattaattttccgcctgcttttttatcaacgccagttacagtcccgccatccataacctccagtaagccgccactatctacagtggtattataagcgaagtcattttcttcaactcgcaaacttccgccgttttccaacaacatattattagcaataccattcttgatatcgaactgaccgagacggtttgttccgaatacctccatggcccgcgtggttgttttaatagcaccgcctgctttctgatctaccgcaaatgcaaatcccccctctttaacctccagtagtcctcccttttcgatagcgacaaagacggcccccccatctttttcaacgattaagcgcccgcctttaatcgtggtatcattcgctgcgccataaacctgtagcacaccattattgagcgtagtctggtttgccgcgccacccatttgaacaatttgataaccgtcatttaatactgagtattctgcggcgccattcatttcaatgtactgataccctccgttaatttcagtattattacttacaccaaattcttttatatgctgttctccgccaggattgattttcgtattattggcggtcccataaaccagctggatatctttttccaggacaacaccatcaactgtctcaccatactcaacagttgatgccaatgctatgggtgaatataaggaaggtgcgaataagcggggaaattcttctcggctgactcagtcatttcatttcttcatgtttgagccgattttttctcccgtaaatgccttgaatcagcctatttagaccgtttcttcgccatttaaggcgttatccccagtttttagtgagatctctcccactgacgtatcatttggtccgcccgaaacaggttggccagcgtgaataacatcgccagttggttatcgtttttcagcaaccccttgtatctggctttcacgaagccgaactgtcgcttgatgatgcgaaatgggtgctccaccctggcccggatgctggctttcatgtattcgatgttgatggccgttttgttcttgcgtggatgctgtttcaaggttcttaccttgccggggcgctcggcgatcagccagtccacatccacctcggccagctcctcgcgctgtggcgccccttggtagccggcatcggctgagacaaattgctcctctccatgcagcagattacccagctgattgaggtcatgctcgttggccgcggtggtgaccaggctgtgggtcaggccactcttggcatcgacaccaatgtgggccttcatgccaaagtgccactgattgcctttcttggtctgatgcatctccggatcgcgttgctgctctttgttcttggtcgagctgggtgcctcaatgatggtggcatcgaccaaggtgccttgagtcatcatgacgcctgcttcggccagccagcgattgatggtcttgaacaattggcgggccagttgatgctgctccagcaggtggcggaaattcatgatggtggtgcggtccggcaaggcgctatccagggataaccgggcaaacagacgcatggaggcgatttcgtacagagcatcttccatcgcgccatcgctcaggttgtaccaatgctgcatgcagtgaatgcgtagcatggtttccagcggataaggtcgccggccattaccagccttggggtaaaacggctcgatgacttccaccatgttttgccatggcagaatctgctccatgcgggacaagaaaatctcttttctggtctgacggcgcttactgctgaattcactgtcggcgaaggtaagttgatgactcatgatgaaccctgttctatggctccagatgacaaacatgatctcatatcagggacttgttcgcaccttccataacgctgtagccaccagaacagatattgcggaacgacaaagagaaacagaaccagattgatgcattgagctttcatcctatgaaattaattgctgttaaaagcattgggtacagaaaatacccatagctccatacccggagtcagtttttaaaaactgtttaaagaaatgcacaagtattgtgattgattttttagttgtttttcttgatgagaagctgatgcaaaattccgtctttataatgaaaatgatgccaaagcgaacgacaaggttgtagttttcactacatgtccatacataaaatggggtaacattcacgcgcctggtagcgttaccaacgctacgctcaaacataatgattctaataaaacctcaggagactactatgcctgaagcaacaccttttcaggtgatgattgtggatgatcatccacttatgcgacgcggtgttcgtcagttactggagcttgatcctggctctgaagtggtcgccgaagcgggcgacggcgcgagcgctatcgatctggcgaatagactggatatcgacgtgatcttgctggatctcaatatgaaaggtatgagtggcctggatactctcaatgccttgcgcagggatggcgttaccgcgcaaattattatcctgaccgtatccgatgcctccagcgatgtctttgcgctgatagacgcaggcgcagacggttatctgttgaaagacagcgacccggaagtattgctggaagcgattcgtgccggagcgaaaggcagcaaagtctttagcgaacgcgtcaatcagtacttacgtgaacgtgaaatgtttggcgcggaagaagatcccttcagcgtgctgacggagcgcgagctggatgttctgcacgagctggcacaggggctgtcaaataaacagattgcctcggtgttgaatatttccgagcagacagtaaaagtacatattcgcaatctgctgcgtaaactcaatgtccgctcacgcgtggcggccaccattctgttcctgcaacaacgcggggcacaataaaaatagcccgatggatttatcatcgggctgagatttatgacaaacgcaaaactgcctgatgcgctacgcttatcaggcctacgtggatcgatcaatttattgaatttacacaattttgtaggccggataaggcgttcacgccgcatccggcataaactaagcgcactttgtcaacagtctagcccgatggcatcaccatcgggcctctttttatttactctcctgcggcgacaaatgttgcatcgcctgcgcgatactacgttcaatcaccgcacggcgagtatcgttggcaggtaagagtttcaacatcatctcccacgcggcaacggcttcgccaaatcgctgctgctcaaaggcattaaacgcatacatgcttagcacacggatattgctatggtccgttctcaccagctgacgtagcagttcaccgccgaggcggttgtcgttgggatcagatgaacgagtcaacgcttcagcgtatcccagtgcagcatcactgtttttcggatcgaggcgatacgcagtggcgtatgcatcggtggcgatactggcgttacccagcgccatgccaacgcggcccaacataatccagccttctatatctcccggatttttttgcagttgagtacgcatccccagcgcaagacgcgacatctcttcttcgttgagcggatcggctttcggatccagcgccctgtccagcaacgccggagcctgtgccgtggcctgctgccagattttcacctgctgataattgccagtctggtagtagctgacgccagccacaattaacgccaccacaatacccggcagataaacaacatatccggcacgcttaccttccggcacgctttgttcaggaaacgcttccggcaccacgcgtacccgacgccgcgagcgggcgtatatgacccaaccgccaatgccaatagccactactggcagcacccacagcagcacggtcagcggcgttaacggcggatcgtaagtgacgaagttgccgtaacgcgccaccatataatcgacaatctcttttttacttttaccttcctgcatcagttcatacactttctgacgcaggtcggtggcaatcatcgagttggaatcggcaatgctgttgttctggcatttcgggcagcgcagttcttcagtgagctgacggaactgttgttcctgtgcttcatctttaaactgcaacacatcgatggtcgccagcgctgagccggagatcatcagcatcagcacgcccaataaaaacctcattgtgcggcctccttactgtatttctcccacagcggcttgatctcttcttcccagacgcgaggattcagatcgcccgcatggcgatagcgaatgatgccgttgccgtcaataagaaacgtttctggcgcgccatagacaccgagatccagccctaacatgccatcgccatcaaacaggcttagcgcgtaaggattgcccagctctttcagccagctgattgccttctggcgatcgtctttatagttcatgccgaccacgcggatgccctgcgcagaaagctgattcagatattgatgttccgcacggcaggtcggacaccaggtcgcccagacgttaagcagtactggtttgccctgagtcagcacatccgcctgataaaactgccccggattgtccagtgattcgagacgaaacttcggcacaggcttgccaatgagcgccgattccagattggtcggatcatccccttcggcattacgcgccagctgccacagcagcgccgcggcaatcgccaggaagataatcaacggaattaacaatactttgcgcttcatacggcctccggcgcagttttttgcggactcacgcgcttacgatagcgaggatcaaacagacacagcagtccgcccaacgccatcatcagcccgcccgcccaaatccagcgaacaaatggtttgtagtaaagacgcacggcccacgcgccgttttccagctcttcaccgagggccgcgtacaggtcacgcgtgatgccgccgtcaattgccgcttcggtcatcatcgacccggcagtgttgtaataacgtttttccgcatacagcaccgtttccggcttgccatcgcgcgttacgccgatagtcgccacaccgccacgccagttcgggccagtcacctctttgacatcacggaaggtgaagcgatattcatgaatatcgacgctatcgccggacttcatgcgcacatcacgctcaacgctatagttctggctaaaggcaatgccaacaattgtcactgccagcccaaggtgagccgccaccatcccccaataactgaaggtggttttcgtgccgcgtgaaatacgtagcgcagcttccgcaattgccagcaccgcaatccagcaggccattgccaggccgagcaccgtcatcgccacaactttgctttcgaacagccacggcaacagcagcgacagcaccagcgtagagatgaaggcgataatcaataaattgcggatcttacgcgggcgatcccgcccccagcgcaccagaggaccgacaccaagcagtagcgcaaacggcaccatcagccaggtaaacatggtgttgaagaacggttcgccaatcgaaatactgcccagtcccagttgcttatgcaccaacggcagcagcgtccccagcaacaccaccagcatcgcagcgaccagcaaaacattgttcgctaacagcaaagattcccgcgaccacagcgcattgtttacgcgtgagcgaactttgtgtccacgcgcggcaaacagcagcagcgaaccgccaatcaccagcaccataaaggcgaggataaacataccgcgcgccggatcagacgcaaacgcgtgtaccgataccagcacgccggaacgcacgaggaaagtccccaacagacacaacgagaaggcactgattgccagcagtaatgtccacgctttgaagctggcgcgttgttcagtgaccgccagtgagtgcatcagcgcagtccccaccagccacggcataaacgaggcgttttctaccggatcccagaaccaccagccaccccagccgagttcgtaataggcccatgcggaaccgagcacgatgccgagcgtcaggaagatccacgctgccagcgtccacggacgagtaaaacgcgcataagtgctgtccagacgcccgctcagcaaagaagcaatggcaaaagcaaacgccaccgagaaacccacgtaccccatataaagcagaggcggatggaagatcagccccggatcctgcaatagcgggttaagatcgcgaccttcaatcgggaagttcggcaacgtgcgagagaacgggttagaggtaaagagaatgaacagcaaaaagccgacactgaccatccccattatcgccagtacacgggccacaatatccagcggaatacgctgactaaaaatcgccaccgcaaaggtccagccgctcatcagcagcacccacagcagtagcgagccttcatgcgcgccccaggtagccgccacgcgataccacaccggaagctgggtattggagttgctggcaacataggtgacggtgaagtcgttgaccacgaaagcattgaccagcaccagaaatgcgccagccacagacataaacagcagccaggcaaacaagcgggaagacgccatcatgcgcgcatctccgcgcgccacgccccatagcggatacacggacagcagcagcgcaattcccagcgccaggcacagcagtccgttaccaatttctggcatcatgatgctgggtccttataaacactcgccgggcgacggtggttagcttccatcgctttctcaacttctggcggcgtatagttttcatcgtgtttcgccagcacttctttcgcgaggatatgattgcctttttccagttcgccctgcaccacaacgccctgcccttcacggaacagatccggcaaaatgccttcgtaagagacatccactgagccttcagcatcgtaaatggtgaaggtcactttcagcgaattgggatcgcgctgcacactacccggcatcaccatcccgccaacgcgcagacgctgaccgacttccggcatttgctgagtttcacgcttgccgtagagaatttcccccggcgtataaaagagatcgatattcgagcgcagcgcatatagcaccagaccgatagtcagcgccagccctgccaacacggcacaggcaatccacaagcggtttttacggcgaatattcatgcagcctcctgctgttgcgcagcacgtaaacgcgcctcacgcgcccgctgttgcgccacgccacgcagaattgcgcgatgttgcatcaccgagtgcacgaccaaaaccaccagcggaataacggtcatcaccaccgccagccagacaaaaaaggcgtaaccgcccattgcgaaaaattcattccaggaagcaaatgcaggggtcatttacggcctcttttcagtatcagttcactcacccacggacggcgtttttccatcagcaaaatcaaattacgcatccgcatcagcgtcagcgtggcagacaggagcaggaagccaaaaatcgaccagcgcagcggcgaacgcatcgccggatcgatactttgctgcatccgcgttgatccctgatgcagggtgttccaccactccacggagtaatgaataatcggcagattcaccacgccaatcagcaccaggatacctgccgcacggcccgccagacggcggtcgtcgaaggcgtgccacagggcaatcacacccacatacaaaaacagcagcaccagttcagaagtcagacgtgcatcccatacccaccaggtgccccacatcggttttccccatgcagagccggtaaccagggcaataaaggtaaacacggcaccaatgggggccatcgccgccaccgccaggttggccattttcatctgccagacaaggccaataaacgctgccactgccattgatgcataaatgcccatcgaccagatcgccgcaggcacatgcaggtagataatgcggtagctatttccctgctgataatcagccggagcaaagccgaatccccagatccagccgacggtaagcacgaccacactggcaattgccagccacggtataaaccagccacagatttgatacagccgtggtgggatcgccagttgatgcagtgttttccacatagtttcgataccagactcgaacaaaaatcagtaatccagcgttattgaatgctgattcgtaacgctgccgccgtcgcaaaaggacttaatgtcgcggtgcctgccagcaacgcgcctaaaattgccagatacccgtcaacgggcaaatgcatagaagccgcgtccatcgcggcggtggcaaagatgagtaatgggatagtcagcggtaacaccagtatgctgagcagcacaccaccgcgcttaagtcccactgtcagcgccacgcccggtgcaccgagaaagccaagcgtaggcgttcccagcagcagcgtcagcgccatcacttgccagccataaacatccattcccagtagcattgctaccagtggcgaaaggatgagtaacggcagaccggttaccatccagtgcgccatcaccttcgccagcacaacggcgggcaagggtaacggcaacaacatcaattgttcaagactgccgtcctgcaaatcgtcacggaacagtcgttccagcgccagcaaggatgaaagcagcgcagcaacccagataatgcccggtgcaatacgcgccagcagttgcggctccggaccgatactgagcggaaaaagggtaattacaatcaggaagaaccacagcgggttggcgatttcggcgctatggcgaaacgctacacgcagctcaagacggaaaatgcgccagaacatcatgcggccctcgtttgcgtcagtgaaatgcggcgaattttactttcagcaacgttgagcggctggtgggtagtcagaatcacaatccccccctgctccgtatgctgcgccatacgctgggtcagacgatcgacaccgttaacgtcaatcgcggtaaaaggctcgtcgaggatccataacgtggcacgggtcagccacagacgcgctaaagcgacgcggcgttgttgcccggccgagagctgatttacaggaatatcttcgaatccggcaagcccggcctgcgccagggcttccagacattgtgcggtatcgccatcgcgatgataaaagtgcagattttctaacgccgtcagccgggttttgatccccggctgatggcctatccataacaggttttgatggtagctgtcgcgtacctgatgcaagggctgcccttgccagagaacctcgcctgcgtcagggcgagacaaccccgtcagcaaacggagaagcgttgtcttccccgcgccgttgctaccggtgatttgtacccactctcctgcgttcagcgtaaatgacaagccactaaataaggttcgttcatcccgctcacaaagtaactctctggcttcaagcatacccacgcaataaccctgttaaaaacctggctcgacttcacgcatatcgggcagcttgtgcgctatccctttatggcaatcaatacaggtttgcccatctttcaccgcctggtcatgcatcttcgcggcaaccgatttctgggcggttgtatccatatactcgaagttgtgacagttacggcactcctgcgagttattgtccttcatgcgccgccactcattctgtgccatcgtcagacgatgagcttcaaatttctgcggcgtgtcaataacgccaaaaattttaccatacagctctttacttgctttgagcttgcgtatcatcttcggcacaaactcgtgcggaacgtgacaatccggacaggtcgcacggacgccgctacggttgttgtagtgcacggaatccatgtattcctgatacaccgtgttgcgcatttcgtggcagctaatgcagaactcttcggtattggctttttccatcccggtgttaaagccaccccagaagacgatgccgccaacaaaaccgatcaacagcagcgtccccagcgccagacggctgggggtacgccaccatttccacaggcgcttaatcagaccaggcttacggtcagaatttcccataataacctcttatttcccgtaaccttttgatggggtaaaggtattccccacgattggcgcggtatcggcctgcggtacgtgacattgcagacagaaataacgacgcggagccacttccgcgcccactttgccgtcgctgtccataaagtgagtaggactgatacgcggcgcgccagtggtgcgatagctttcgacaccgtggcactgcaagcagcgattggtattggtcgttacctgataaccttcaacgctatgcgggatcattggcggctgattcacatagttcagcggcatccgatcctgctcttttggcatccgaatggccccttcctgtgtcccggatacttccggcgactggctaaaatcgacgccattagccgcccaaaccgcgccgcttaccaccagggccagcatcgccgtccattgacacagcgctttcttcaggtcatggcttttcatgatttcgctcccgaactccatcgtgtagttattgtaaatacatcctcagaacagacatccacgcagcgaccgcacgtcatgcaatcgcggctggtgacctgcaccgggctttgttcatccagcaccggggcacgtagcacatgcggttccgggcaaacatgaaaacaatccatacagcggttacatttctgccgatcggtggccgcaacggtaatcacacctttgctacccagcacgccatacagcgcgccaaccggacaaatgtgcccgcaccagccgtgttcaacgaccagtagatcaaataaaaacagcgcgagaataagcagcgcgccgctgccgaagcccattaccaggctacgccccatcagagaaacggggttgatccattcccaaatgagcgtgccagttaaggctgatcccaccagaatgaccaccaacagcacgtagcgaatgtggcgagggatcgtcgcagactgattgaggtcaaagcgcctgcgtaaccagttcgctaagtcggtaatcgggttcagcgggcagacccagctgcaaaataatcgctttcccgccagggcgtagagcacggtgataatcaccgcaccggtcaacgccaccgtggcaggcagatgaccactggcaagactttgcagcgtcatcagcggatcggtcagcggaacggtgtcgaataacaggctactgctgtagttgccgtgcaagatccacacaccaaaccatggaccgctcaaaaacatccccagcacgaagaactgacaaaggcgacgtaacaccagccaacggtgactgcgccaccagccttttttctccagcgcctcgcgcccggcgtcacgtttacgatttgccattgttcccctccagccagccgaagcggtaatggtgacctaactcccctttcgccagtgacagcggtaacaccttgattgccggttgttccagcacgcatactttttcgcacttaccgcaaccggtacaggcgtcgctgtgaaccgtcggcagaaagcgggcgtgcttaccggtacgcgtgttgcgctccagctccagggtgatggcctcatcaattttcgggcattcgcgataacaaacatcgcagcgcagcccctgaaagttgagacagttttcctggtccaccagtaccgccagccccatccgcgcgtcgtcgatcgattcaatctcacgatccagcgcaccgcttgggcacactttggcgcacggaatgtcctcacacatttcgcaaggaatatcccgtgcgacaaaatatggcgtgcccgccgacagaccagaggccagcgtcgccagttttaaggtgtcgtaagggcaagcctgaacacactgaccgcaacgcacacaggcactggcaaaggcgttctcgtttatggctccgggcgggcgcaaccgcacgccagatgcgcgtgcggtttgctgttgtaaccccagcgccacacccacggcagccagcccgcctgctgtgcgaacgacatcgcgcagaaagcggcggcgaccattttgaggtttcgctgaccgggacataatggcttacaccttctccagtttgaccgcgcacttcttgaagtccgtctctttcgagagcggatcggtcgcatccagcgtcagtttgttaaccaactgtgcggcgtcgaagaacggcatgtacaccaggccctgtggcggacggttacgaccgcgcgtttcaacaatcgagatcacttcgccacggcgagaaaccactttcactttgtcgccacggcgcagatcgcgcgctttcgcatccagcgggtgaataaacaggaccgcttccgggaaggcgcggtgcagttctggtacacggcgagtcatactgccggtgtgccagtgctccagaacgcgtccggtagagagccacaggtcgtactcttcatccggtgcttccgccgccggttcgaatggcagtgcgaagatcaccgctttgccatccggtttaccgtagaacttatagccttcgcccgctttcacgtacgggtcgttaccttcgctgtaacgccactgcgtttctttaccgttcaccaccggccagcgcagaccgcgcgctttgtggtagtcatcgaacggtgccagatcgtgaccgtgaccgcgaccaaaccatgcgtactcttcgaacagccctttttgcagatagaagcccagctcgcgggattcatcgttcagctgatcttccgccagttcggataccgggaatttgctcacttccggtgtggcatacagcacttcgtacagcgttttgccacgcagttccggtttcttcgccagcagatcttccggccatacttcttcagttttgaagcggcgggagaactggactaactgccagagatccgatttcgcttcgcccggtgcctgtacctgttgacgccagaactgagtacggcgttcggcgttaccgtaagcgccctctttctctacccacattgcggtcggcaggatcaagtcggcggccagcgcactgactgtcggatacggatcggagacgatgatgaagttgcgcggatcgcgccagcccggcatacgctcttcattgatgttcggcccggcctgcatgttgttggtacacatggtccagtaaacattcagtttgccgtctttcagcgcacggtcttgtgccaccgcgtgcagaccgattttcgccggaatggtgccgctcgggatattccacttcttctcgcagatatcacggtgtttctcgttggtcaccaccatgtccgcaggcagacggtgagcaaaggtgcccacttcacgcgcagtaccacacgcagaaggttgcccggtcagggagaacggaccgcaacccggctgggaaattttgccggtcagcaggtgcaggttgtagaccaggttgttagcccacacgccacgagtatgctggttgaagcccatcgtccagtaggagatgactttcttgttcggatcggcatacagctgcgccagttgttctaactggtctttcggcacgccggtcatttcggcagttttttccagcgtatactcggcaacgaaggctttgtaatcttcaaagctcatcggttcggaggcgtcagaacccggattcttcgctgctttttccagcggatgggtcggacgtaaaccgtagccgatgtccgtcgcccctttgcgcaggttaacgtgcttgctgaagaagtcctgatttatcgcattgttttgaatgatatagttggcgatgtagttcaggatcaccaggtcagattgcggcgtaaagatgatgccgttatccgccagctcgaagctacgatgctggtaggtagaaagcaccgccacggtgacgttctggttagagagacgacggttagtgatgcgcgaccagaggatcgggtgcatttccgccatgtttgcgccccacagcacaaacgcgtcagcctgctcgatgtcgtcatagcagcccatcggctcatccataccaaaggtacgcataaagccaactactgccgacgccatacagtgacgcgcgttcgggtcgatgttgttcgaacggaagcccgctttaaacagcttggacgcggcataaccttcccagatagtccactgaccagaaccgaacataccgatcgattccggccctttttctttcagggcggttttgaatttctcttccatcacatcgaaggcctgatcccaggtgattggggtaaattcgccttctttgtcatatttaccgtttttcatacgcagcagcggctgcgtcaaacggtctttaccgtacatgattttgggcaggaaatagcccttaatgcagttcaggccacggttaaccggtgcgtccgggtcgccctgacaggccaccacacgtccctgctgcgttccgaccagaacgccgcaaccagtaccgcagaaacggcacggcgctttatcccatttgatggcttcctgctgaccaacaacggcgcgggcaacgcccggcacgctgagaccggcagccgccgcagcggccgcaacggcgttagctttcataaagctacgacgactgagtttcatggtgtttcctcaccttgctcttcctgctggtgataaaccagcgacaccgccagcacgccctctacgttgcgtactgactcaatggtttggatcagcgtttcgctgtcttctgcttccaccaccacaatcaactgaccgctcggcgcgtcgctgacagcaacttcacagccgggaaaggcgttcagttgggtgctgatgtctgaaattcgttcgcttttggcctgcacgaccaggctgcaaacttgccagttagtgtgcatggagatactccgcagttatggctgataccggacagctggctgcacatgctccacatccgttgcaaagttggctattaagttgcggctggtagatcccggagagcgtcgggcgaaagataattgccattggctcacagctatcctgacagcggcggcattcaactgactgatacgccaggcacgcgtccccgatggtgaactgcaaatcccaggccctggtgtggcgcggagaaaatagcgattcggggcaagcctgcgcgcaggcgtaacagaagctgcactcgttatttttgaaattaacgctcggatagccgcccgcgccgcgttgcagaatgttgttttcacaagcattaatacaggcgtcgcagcgggtgcaatgggtcagaaaatgagattcatcaccggaccagggcggacggataccgttactggctttgcgccagcgaccagtgagtatgccccgacgggatgcatcaatcttcacattgaccttccatcattaacgcgctctgaaaattgagagcgaccaaataaaccgcataattaataagccatttttatagccgctaagatattaaaggatgtgtcaaagatgcataccccgatcggggtaaaacctgtagcaggatcaaaagagtggcgggaagcgtggcaaaaacgggcttttgctcacatttcaaatggttataaatatatttatatagcgattgattcaccagagatatttctgctggtttgctctctcattagaatttaacactaaaagagcaggtaaaattgtctgaatgttctttaagttattcataaagcaaattaataaatctgatgaatatgttaaccttcagcgacatcatcggtgaaaacctataaatgaagaaggaaagcaaaaaaatgaagaccattctacctgcagtattgtttgccgctttcgctaccacttccgcctgggcggcagaaagcgtccagccactggaaaaaatcgcgccttatccacaagctgaaaaagggatgaagcgtcaggtgattcagttaaccccgcaagaagatgaatctaccctgaaagtagaactgttaatcggtcagacgctggaagtcgattgcaatttgcatcgtctcggcgggaagctggaaaacaaaacgctggaaggctggggctatgattattatgtctttgataaagtcagttccccggtttcaacgatgatggcctgcccggatggcaagaaagagaagaaatttgtcaccgcgtatctgggcgatgctggaatgctgcgttacaacagcaagctgccgatcgtggtgtatacgccagacaatgtagatgtgaagtaccgcgtctggaaggcggaagagaaaattgacaacgcggtagttcgctaaactgccgtgaagtgcggcaccccgtaggtcagacaaggcggtcacgccgcatccgacatccaacgcccgagccggttgcctgatgcgacgctggcgcgtcttatcaggcctacaccgctgtgaagtgcggcaccccgtaggtcagacaaggcggtcacgccgcatccgacatccaacgcccgagccggttgcctgatgcgacgctggcgcgtcttatcaggcctacaccgctgtgaagtgctccaccccgtaggtcggataaggcggttacgccgcatccgacatctaacgcccaagccggttgcctgatgcgacgctggcgcgtcttatcaggcctacaccgctgtgaagtgctccaccccgtaggttggataaggcggttacgccgcatccgacatccaacgtccgagccggttgcctgatgcgacgctggcgcgtcttatcaggcctacaccgctgtgaagtgctccaccccgtaggtcggataaggcggttacgccgcatccgacatctaacgcccaagccggttgcctgatgcgacgctggcgcgtcttatcaggcctacaccgctgtgaagtgctccaccccgtaggttggataaggcggttacgccgcatccaacatctaacgcccgagccggttgcctgatgcgacgctggcgcgtcttatcagcatacgccacatccggcataccatgccggatgtggcgtatcattacaacgcaatatccgccacttctttttgaacgggttgcggtttcaactgcggtttcggcgtactatctgctgcctgcggcttgtcgtagttcaaccccagcacttcgctggtgtactgcaactcgcgttctgttgccgctacatcaccgttcagcttgcgtccataagacggaacgatcgctttcaacgtagcctgccattgcgggctggaaacacgatcgccaaatactttttccagcagattcaacataatcggcgcggcggttgacgcccctggcgatgcccccaggagcgcggcaatggttccttgctggtcactgacgacttcagtacccagacgcagtacgccacctttctcggcatcacgcttgataatctgcacgcgctgccccgcttgccacaaacgccagtcctcttttttcgcctgcggatagtactctttcaacgcttcaaaacgatcctcttcactcaacatcacctgactcaccagatatttcaccagatcgaaattatccagcccgacgtgcatcatcggcatcacgttagaggtggtggtggaactcattagatcccacaatgaaccgtttttgaggaatttggttgagaaggtggcaaatggcccaaacagcactacgcgtttaccgtccagaacgcgggtatcgatatgcggaaccgacatcggtggtgcgccaacggatgctttaccgtaaaccttcgccagatggtgattaaccacgtccgggttttccgaaacaaggaactgtccgcccaccgggaaaccggcgtagtctttcgcttccggaatccccgattcctgtaacagcttcagcgccgcaccgcccgcgccgataaagacaaatttggcacgaatgttctgtgcagtgccatttttcagatcggcaacggtaacggtccaggtgttatcgtcattacgctttagggcgcggacttcgctgctgagttgcagcgagaagttagatttcttctgcaaggaagcaattaactggcgggtgatctcgccgtagttcacatcggtaccaatttccgtacgcgtggctgccactttctgttgcggatcgcgcccttccatcactaacggtgcccactctttgatctgcgcgtgatcttcagagtaacgcataccgcgaaacagcgagctttgttgcaacgcggcgtaacgggcgcgcaggaaattgacgttatcctcgccccagacaaagctcatatgcggaacggtattgataaatgaacgcggagtacgcagcacgccgcgctcaacctggtgcgcccagaactggcgggaaatctgaaatgcttcgttaatggcgactgctttttcaatactgatgctgccatcggcgttttgcggggtgtagttcagttccatcagtgcagaatgcccggttccggcgttattccagccgttcgaactctcctgcgcgacaccctccaggcgctccaccatggtcatcgaccattcaggctccagctcgcgtaaataggtccccaacgtggcgctcataatgccgccgccaatcaacagtacatcagtttcctgctcctcggacgctttcgcttttgccgccatcgaaacggcattaagccccacggccatcgagaagagcatggcagtcacttttttcatcttgttaatgccttacttttagtcgctttattgcaggtgagatttgcgcggcatcaacggtaacacttaagtaacaacatttaaataatgtttataaattatattctaattttagaaacattataatttcgttgattaattatagggttattagaaatgaagggatttttagcatattgacctgacggcagcagtccgccaggtcagcgtcgtaatattatgccgtccgggcaacggcatcacgcgaagcggcatcgcgctcttcgcccgtcagctcgctaagttgcccattgcgcatttccagcaggcggtcggcgtggataaagtaatgatcatcatgactgatagcgaaaatagttttacccatctcctgcatcagcggcagcaacacctgataaaactcacgacggaagtgtggatcctgatccgccgcccattcatccagcaggataatatcgcgttcttctgccagcgccagcaacagcgccacgcgttttttctgcccttttgataacttcaggttaacaatacgcccgttgcttaactcaagcttatgagccattttcagctgcgccagccacttctcaaccagttgcgggttagcgggtttaccctccggccccagcagttgatcaaacagccagacatcggtaaacactgccgaaaacagtttgcgataatcttccggttgttcgccgctgacaggtttgccatccagcaagatttcgccgctttgtggctgatacaagcccgtcaacaacatcgccagcgtcgattttccgctaccgttgccgccaatcagaaacagcagctcgccacgtttgatggtgagattaatcggaccaacggaaaacgcgttatcctgataagcaaacgtcacgttacgcagctccagcgtttgccagttgggaaacgcctgcgggcgcggaaactctgctttgaaaggcgcgagcgcgaatttgttcagcttgttaaacgccacctgcgccgtcagcagcgtcggcaatgcgccaaccgccgaaagcagcggcgtacgcaggaataaaagcgtcaacgaataggtcgcggcaacgttggtatcagcccaaccgaggctgttcgccatccagaacaccaggccgattgcgcccagcatcatgatgtttgaccagttcacggcactaagatggaaggtgtctgcgcgaataatatggtggcgatactcttgcgcatcaggaatgtagaggttgttaaacacatactcggcgcgttcccggttcagagtcagctctttgcgcccttcaagtacagtttgaaaatccgtgtacagcttgtcttcggtttcacgcagggtcgccatatgtttgtacacccgcgccaccagcacaaaaccgccccagatggtgatcgccatccagatagccgttaccagcaacattttgcccgacagcatccacagatacgccgctgaaccgatagtgagaatgatcccctgcaccagttccggcagacgcacaaaagcaatggtgatattgcgcacatcgctggttaaccccgccagcaacgaggcgctaccgagttgttcaatgcgctcgacgtgagtatccagaatccgcttgataaattcactacgcagtcggtaaacgaagtgatgccccaaagtggtgagcgccagttgcgatccgagagtgactgccatcaacagcagcaataatcccagaaactccggcaacaccagcagactggtatccgccgtttcgataaggcgctgattgataaaagcaattaagccaatgcctaatgccgcactggcgaggcttagcgccatcacactgataaatggccagcgatactgccgccagacaagtacaagaagttccatgcagaaaacccggacaatgaattacagcccgcagtttaaacatcttcgcgcgcacagcaataataattcttatttttattcttttttacctgcctgacggaatgtcaggttgtagcggcagtcgatggtgagtggatgaaaccccgctttcaacggttgaataccgtgataaaacagccgcgattcaccgccccataccaccacatcgccatgttccaacaacaaacgtttgagcggatcatttcgtttcaggccgccaaattgaaaaatcgcgggtaagcccagagaaacagaaacaattggcgcgcgcagatccggttcgtctttatcctgatgcagcgacagtttcgcgccaggagcgtagcggttgataagacaagcatctggctggaaatctggatagcccgccgccgtagccgcacgttgacataaattatgaaaactctgtggcatggcgggccacggtttatttgtttgcggatcaatgggcgaatagagataaccttgccgatgggtcgtccagcccagatgcccacagttggtcatcgccaccgacatggtatatcccccgggggtgaccatctggcgaaacggcgactggctggcaacgtcattaatatcgcggatcagttgctccgcagcgttaaaagcaaaacgccgtaaaattaccgcaccagccgccagtggctcttgccacggttcagcatcggcaaacagatccaacattacctctcctcattttcagcttcgcggcgcagcagttgcgctttacgcgacacgccccagcggtaaccggaaagtgtgccatcaccacggaccacccgatgacagggtattatgatagccagcttgttggcggcacaggcgctggcaacggcccgtaccgctttcggtttgccgatggcgttagccagttgctgataactgacggtttcaccgcaaggtatcgtgcgcagtgcctgccagacttgttgctgaaaagcagtgccgcgaatgtccagcggtaacgtcagcggcgtatcgcgttgattgaggctggcgatcacttcacgcacatgttgctgaaacatcagatcggcaggcgcgttgtcggcagcgggaaacatctgctgcaactcgctgattagtgtcgcgtcatcatcgcccagcaatatcgcgcaaatcccccgctcgctttctgccaccaggcaacgacccagctcacaatcagccagcgcgtaacgcaccgccagattttcgccaccgtgacggaattgtttagccgtcatgcccagcgtttcgtcagctttgcgatagtaactgctgctgtcggggaatccggcgttaagaatagacgtcgtcacgctctcccctttcgccagcgattcgcgcaaacggcgagcgcgccaggcctgttgccaggctttaggcgtcattccggtagtcgctttaaacaaccgatgtagatgaaatggactcatcgccacctggtcggctaaggcttccagcgttacaggcgtttcctgttccagcagtcgacacgcgtgggtgattttatccaaccgatgttgctgggcattggctttttctggctgacaacgtttgcaggggcgaaagccagcggcgagtgcctcgctggcatttgcgtagaaggagacgttttcccgcaaagcatgtctggcgcggcaagacggacggcaaaagatgcctgtggtacgcacggcgaaaacgaattcgccgtcggcattcgggtcgcgggctaagacagattgccagcgttgatcgtcagttaagcatgtggcttttttcataatcagctccctggttaaggatagcctttaggctgcccggtcaccatcacgcaaaaaccaacaatcttgcgctttaatttttttcgctgacaaggaagcttttaaactgtggtgacatccaggttttaaagctatcgccttctttggtgatcatataaaccgccagcccttcccggcgaacaacctctttagctttctccggcccgagtaccatcaagccagtatcccaggcatcggcttccagcgccgtcggagcaatcaccgtcacggataccagattgtgttcgatgggacgcccggtttgcggatcgataacatgggaaagacgtttgccgtccagttcgtaatagttacggtagctgccagaggtgctaatcccatgaccgttgatatccaccacagcctgaaccgcgttttctttatcggttggtttttgaatcgctacccgccacggcaggccttcaccgttcataccacggctgttcagcgcgccgcccaccgacaccagatagcgggaaatcccttcctgctccatcaagcgtgccaaatgatcggccgcatagccttcgccgacggtggagagatcgacatataaatccggcaggtctttttgcagatattgctgatgcgactgattgatgaccgtcaggtgctgtaagccggttttggctttcatcgcatcgatctgttcctggctcggaatttgaaccggctgttgttccgggccaaagccccacagattcaccagcggcccgacggttatatccatcgcgccatcggtcttcgcgccaatgcgcagcgaggtggtgacgatatcggccatcgcttcacttaccggccacggcgataaactttgcgagtcgttaaagcgcatcagcgcggaatcttttttataggtcgaaagcagctgatcgtcggcgtccagttgggtctgaatcttttctttaagttcggcgctgcgtttggcgtcaatgcccgggatgctggcacgccagaaggtacccatagttttgccttcaagaacggtaacttcagtagcgtgggttttggcgggttgtggtttttgatcgcaaccaacaaagaagagcgcggcagccagcagtgccacgcgggtaaagcttatttccatacgtgattatcctcatgcgaacggtcgcaagagtacaccaaaaaactgagtttgtacgctgaaaacaatgaaaaaagggcccgcaggccctttgttcgatatcaatcgagattagaactggtaaaccagacccagagctacgatgttatcagtgttgatgccagcgtcacgagtgaactggttgtcgtccagcaggttgattttgtagtcaacgtaggtggacatgtttttgttgaagtagtaggtagcaccaacatcaacatatttcaggatatcttcgtcgtcgtagccacgacccaggtttttacctttagactgcaggtaagccagggacggacgcagaccgaagtcgaactggtactgagcaacagcttcgaagttctgtgctttgttcgcccaacccagggaacctacgcgagttgcgttgtaggtctgggtgtactgagcagccaggtagatgttgttagcgtcgtatttcagaccaccagtgtaggtttcagcacggtcgccgttaccgatgtaagcagcggtgttctgagcatcagtacgtttggagctggagatcgcaccaccgataccgaaaccttcgtaatcataagtgatagaaccgccgacgccgtcgccgttttgacgcagtgcgtcacgaccgttgttagttacgccactagtaaagccttcaccagatgggttgccgtttttaccctggtactgaacagcaaagttcaggccgtcaaccagaccgaagaagtcagtgttacggtaggtcgcgaagccgttaccacgctgctgcatgaagttgtcagaaccgtaggtgtcaccaccgaattctggcagtacgtcggtccaggaagttacgtcataaacaacgccgtagttacgaccgtagtcgaaagaacccacatcctggaatttcagacctgcgaatgccacacgggtccaggagttgttttcgttttcagcgctgttgccctggatctgatattcccactggccgtaaccggtcagctggtcagtaacctgagtttcacctttgaagccaagacgcatgtaggtctggtcgccatctacatctttgttgtcagagaaatagtgcaggccgtctactttaccgtacagatctaatttgttgccgtctttgttgtaaacttcagcagcgtttgctgcgcctgctaccagcagagctgggaccaggagggacagtactttaactttcatgttattaaccctctgttatatgcctttatttgcttttttatgccactgcatactgattaaccctcattaatcagtcggcaagtccattctccccaaaaatgcagaataatccaacacgaatatgatactaaaacttttaagatgtttcatttatcgctatagatgtttcaaaatgtaaatgcaagggaactttttaagattattgcggaatggcgaaataagcacctaacatcaagcaataataattcaaggttaaaatcaataacttattcttaagtatttgacagcactgaatgtcaaaacaaaaccttcactcgcaactagaataactcccgctatcatcattaactttatttattaccgtcattcatttctgaatgtctgtttacccctatttcaaccggatgcctcgcattcggttttttttacccttctttacacacttttcattattctgtgctaccacagaaaaactataacgcttgttaactatttcacaaataattaacatccgcataatttccagcaatctttgtttatttgcaattatttttgttgggctttttgtaggttatttgtacagcaaaatggcgcttgtacatctatttcccccaatgcaggatgataaatatcacgggagaatagagaatcatcaatcaggtaagagtctggaatttcacactgtaccctttatactgccctatcacttcgcgaagttttaacaggtcataaacacgaatgcgtcagaaagagacaacggccacgacccgcttttcactcctaccggggagcattacccgcttctttttactgttgatcattgtgttactggtgacgatgggtgtaatggtacaaagcgccgttaacgcctggctgaaagataaaagttaccagattgtcgacattacccatgctatccaaaagcgcgtcgataactggcgttacgtgacctggcagatctacgacaacattgccgcgacgacctccccctcctccggcgaaggtttacaagagacgcgcctgaaacaggatgtctactatctggagaaaccacgccgcaaaacggaagcgttaatctttggctctcacgacaactcaacgcttgagatgactcagcggatgtccacttatctggatacattgtggggcgcagaaaatgtaccgtggtcgatgtattacctgaatggtcaggataacagtctggtgctgatctcaaccctaccccttaaagatctcacctccggatttaaagaatcgaccgtcagcgacattgttgattcacgtcgtgcagagatgttgcaacaggccaacgccctcgatgaacgcgaaagcttttctaacatgcgccgcctggcctggcagaacggtcattactttacattgcgtactacctttaaccagccaggacatctggcaacggtcgtggcttttgatctgccgattaatgatttgatcccaccgggtatgccgctggacagtttccgccttgagccagacgcgacggcaacgggaaacaatgataatgagaaagaagggacggatagcgtcagtatccactttaacagtacgaagattgaaatctcctcggcactcaactctaccgatatgcgcctggtctggcaggttccttatggcaccttattgctggatacgttgcaaaacattctgctgccactgctgctgaacatcggtttgctggcgctggcgttatttggctataccacattccgccatttctccagccgcagtacagaaaacgtccccagcacggcggtcaataacgaattgcgcattttacgggcaatcaatgaagagatagtctcactgctgccgctcggcctgctggttcacgatcaggaatcgaaccgcactgtcataagtaacaaaattgccgatcatttgctgccgcatttgaatctgcaaaacatcaccaccatggcggaacagcatcaggggattattcaggcgacgatcaataacgagctgtatgagatccgcatgttccgcagccaggtcgcgccgcgcacacaaattttcattattcgcgatcaggatcgcgaagtgctggtaaacaagaaactcaagcaggcgcagcgtctgtatgagaaaaaccagcaggggcggatgatctttatgaaaaacattggcgatgcgctgaaagaacccgcacagtccctggcggagagcgcggctaaactcaacgccccggaaagcaaacaactggcgaatcaggcagatgtgctggtgcggctggttgatgaaatacagttagcgaacatgcttgcggatgatagctggaaaagtgagacggtgctgttctccgtgcaggatttaattgatgaagttgtgccttcagtgttgcctgccatcaagcgtaaaggtctgcaactgctgattaacaatcatctgaaagcacacgatatgcgccgcggcgatcgcgatgccttacgacgtattttgctgctactgatgcaatatgccgtgacctcaacgcaattgggaaaaatcacccttgaggttgatcaggatgagtcctccgaagaccgcctgacgttccgcattctggacacgggagaaggcgtaagtattcatgaaatggataatttgcacttcccgtttatcaaccagacccaaaacgatcgctatggcaaggcggacccgctggcattctggctgagcgatcaactggcacgtaaactgggcggtcatttaaacatcaaaacgcgggatgggcttggtacacgctactctgtgcatatcaaaatgctcgcagctgacccggaagttgaagaggaagaagagcgtttactggatgatgtctgcgtaatggtggatgttacttcggcagaaattcggaatattgtcactcgccagttagaaaattggggtgcaacctgtatcacacccgatgaaagattaattagtcaagattatgatatctttttaacggataatccgtctaatcttactgcctctggcttgcttttaagcgatgatgagtctggcgtacgggaaattgggcctggtcaattgtgcgtcaacttcaatatgagcaacgctatgcaggaagcggtcttacaattaattgaagtgcaactggcgcaggaagaggtgacagaatcgcctctgggcggagatgaaaatgcgcaactccatgccagcggctattatgcgctctttgtagacacagtaccggatgatgttaagaggctgtatactgaagcagcaaccagtgactttgctgcgttagcccaaacggctcatcgtcttaaaggcgtatttgccatgctaaatctggtacccggcaagcagttatgtgaaacgctggaacatctgattcgtgagaaggatgttccaggaatagaaaaatacatcagcgacattgacagttatgtcaagagcttgctgtagcaaggtagcctattacatgaacaatatgaacgtaattattgccgatgaccatccgatagtcttgttcggtattcgcaaatcacttgagcaaattgagtgggtgaatgttgtcggcgaatttgaagactctacagcactgatcaacaacctgccgaaactggatgcgcatgtgttgattaccgatctctccatgcctggcgataagtacggcgatggcattaccttaatcaagtacatcaagcgccatttcccaagcctgtcgatcattgttctgactatgaacaacaacccggcgattcttagtgcggtattggatctggatatcgaagggatcgtgctgaaacaaggtgcaccgaccgatctgccgaaagctctcgccgcgctgcagaaagggaagaaatttaccccggaaagcgtttctcgcctgttggaaaaaatcagtgctggtggttacggtgacaagcgtctctcgccaaaagagagtgaagttctgcgcctgtttgcggaaggcttcctggtgaccgagatcgctaaaaagctgaaccgcagtattaaaaccatcagtagccagaagaaatctgcgatgatgaagctgggtgtcgagaacgatatcgccctgctgaattatctctcttcagtgaccttaagtccggcagataaagactaatcacctgtaggccagataagacgcgttagtgtcttatctggcatttgcaccgattgccggatgcggcgtaaacgccttatccggcctacgattcccattatttcaacaaattacattaaagtaggccagataagacgcgtcagcgtcgcatctggcatttgcactgaatgccggatgcggcgtaaacgccttatccgtcctacgaatcccgcgatttcctgaccctctcggcatataacgtcagcgtctgttttatcacatccagcgttaccggcttcgacaggcagctgtccataccggactccagacaccgctgcttctcttcagccaacgcattagcagttactccgattaccggcaacgtcagtcccaactgacgaatgcgttgcgtcaagcggtaaccatccatatttggcatgttgacgtcgctaagcacgatatcaatatgattcttgctaagtacattaagcgcatcgacgccatcattcgcggttttacattgatagcccaacgatcccaactgatctgccagcaaacgccggttaatcggatgatcatccacgaccagaatcatcatatcgtcattatcgctgaccgctttgtccgttgacggcagagcgttagcaggatcgtcgctctccatctcgatcaaataaatacgcgccaacaatgccggtagctcatgcggagcagccacactgtgtacccactcccctggcgctttctccagcggaataccaatatggcgacgacagaaggtcactaccgctctgccctgccattttttactcactacctcgtcagtgatcaacacatcttcgggagtcggttcctgcccttcgtatgttgtaacgacgatgccgctgcgctgcaaactggtttccaggaactgacagagcgacgcattgcggaccgccagccagcagcgtttaccactcaacccttccacgccttttttctgcgggtactgagcgccgtacaacggaatacgcacggtaaactggctgcccattcccggttctgaatctaccgagatatcgccgtccatcatgctgatcagtttttcacaaatcgccagacccagaccggtcccctggaaattacgctgtacgcccgttccgacctggaagaagggatcaaacaagcgcaccacttctttcgccggtatccccacgccggtatcgcgaacacggatagagagataatcgccatccgcgcgaacatgcaaaactatacagccggtatcggtgaattttatggcgttactcaacaggttggagatgacctgctgtaaacgcatcgggtcgccatttaaggccactggcacatccggttcaataaagcagtacaagcctaactgcttgcgtaccaccagcggtaaatagttggcggtgatgtggttcatcacttcacgcggtgaaaactcacgcggttcgatcttcaactgttccgattcaatcttcgagaaatcgagaatatcgctgataattttcaacaacaggctggaagagttgttcattgccgtcaccagccgatcgacgcctttcggtaactctttggtttgcaacagatccaggttaccgataatgccatacagcggcgttcgcagctcatgactgacggtggcaaggaacatcgattttgactggctcgcctgttccgctgcttgtgccatctcctgcaacgactcttccatcttcacgcgcgaagaaacatccaccagcacacaaatggccacgttttcattacgatagcgcgaatggacgaagctgatttgcagattggtattgttgctggtcaggacatcaacaaaattgacctgctgcccacagataatttgcgtcagtcgttggcggtcctcatgcgtaagcatattgagataggtatgcgccagttcgttacttaaaatattgacgccatcagcggtacgcaaaatgcagatacccactggcgcggaggcgacaatcttgcgattgaactgctcatgttcttccagtcgcagggcgtcgctttccgccggaatgaaaatacgtcgctcgtacatccgtgcgagagtaaacaatgcagctccggcaagcacattcagcaaaattgcgttaaggatcaacatgcgaatgcgttccagcaccttatcaaccggcaccgaatacacgatgcttagcgatgagggtggcagatttttcttcagcaccagctcccggaacccttccgtatagccaaaccaggagcgttcctgcatccagcgaggatcgcccttaattttactttctggtccggtaagcgaaatcagggtatgaccattttcatcaagaatggtaacccccatcggcaacgtacccggtaagaaaaagttctccatccggatggtctgctcgacacccaaaagcgcctgcaaccggttcgccagataaactggcgtcaacgcgtaaaaatacccgacgccagggcgcggaccttcgctgatccagtagaggttactgccgctatcatcttgtggtgcatttcgatatttattgatgcgttcatgcaaagctttcaacgcggtatcgcgttccactggcatatcacgcagaccgaaattggccatgcagaggttatcgctgccgattaaaaatacccggtttagatcgtaagccgcagaaaaattatcgcgccagtagcgcataaaccacgccaatgactccagagaacctcgccaggtgttactcattgcggaacaatcggagtcggcaaacagcggttcaaacgcaggcacatccgcctgcgtttctcgtccacgcggggaaagcacaccgttttctgccgataagcgattttcggcgatgtacttcagctctttcatcacatcagaggtgcgttgaataaagcgctgagcctgatcggaactcagattaaattcctgacgaatttccgattctcgctgatgtaacgcattaacgatgtaaaaaacggatgaaaaagcaatcaacagccagagcactaacgccaatgctctgaacatgtagcgcgaggctttcagggttgtacgaaaagaagcaaggtatttcaaaggggcgaagctccgcctcaggtgaccgatggagtgtggttaaggtagcggtaaaagcgtgttaccgcaatgttctctcttctctggaatatgatacaccgccgagaaatcatcaccttaacctctgataatcgtcatataccggacaagactagtggatttcagcatgcattatatgaagtggatttatccacgccgcttacgcaatcaaatgatcctgatggcaatcctgatggtcattgtcccaacgcttactattggttatatcgtagaaacggaaggacgttcagcagtcttatctgaaaaagagaaaaaactttctgccgtggtcaacctgcttaatcaggcactaggcgatcgctatgatctctacatcgacttaccacgtgaggagcgtatccgcgcattaaatgcagaacttgcccccattaccgaaaatatcactcacgccttccctggcatcggtgctggttattacaacaaaatgctggatgcgataatcacctacgcgccttcagcgctatatcagaataatgtcggcgttaccattgccgcagatcaccctggtcgcgaagtgatgcgtacaaatacccctttagtttattcaggcaggcaggtgcgcggcgatattttgaattcaatgctccccattgagcgtaatggtgaaatcctcggctatatctgggccaatgaattaaccgaagatattcgccgccaggcctggaaaatggatgtgaggattatcattgtgctcaccgctggtttgctgataagcctgctgttgattgtccttttctcccgtcgcctgagcgccaatattgatatcatcaccgatggcctctcgactctggcacaaaatattcccactcgattaccacaattgcccggtgaaatggggcaaatcagtcagagtgttaataacctcgcccaggcactgcgtgaaacgcgga

(The sequence listing continues in the following parts.)